European Patent Application EP 4 600 357 A1, published August 13, 2025. Title: Delivery system for gene editing tools. Applicant: Technische Universität München. The sequence listing filed with the application follows.

SEQUENCE LISTING (324 sequences)

SEQ ID NO: 1 - protein, 676 aa, Synthetic construct
MGARASVLSGGELDRWEKIRSRPGGKKKYKLKHIVWASRELERFAVNPGLLETSEGCRQILGQLQPSLQTGSEELRSLYNTVATLYCVHQRIEIKDTKEALDKIEEEQNKSKKKAQQAAADTGHSNQVSQNYPIVQNIQGQMVHQAISPRTLNAWVKVVEEKAFSPEVIPMFSALSEGATPQDLNTMLNTVGGHQAAMQMLKETINEEAAEWDRVHPVHAGPIAPGQMREPRGSDIAGTTSTLQEQIGWMTNNPPIPVGEIYKRWIILGLNKIVRMYSPTSILDIRQGPKEPFRDYVDRFYKTLRAEQASQEVKNWMTETLLVQNANPDCKTILKALGPAATLEEMMTACQGVGGPGHKARVLAEAMSQVTNSATIMMQRGNFRNQRKIVKSFNSGKEGHTARNSRAPRKKGGSGGVSGWRLFKKISGGSGPAAKRVKLDSGLQLPPLERLTLGAAPAAKKKKLDYKDDDDKGGASSKTIVLSVGEATRTLTEIQSTADRQIFEEKVGPLVGRLRLTASLRQNGAKTAYRVNLKLDQADVVDSGLPKVRYTQVWSHDVTIVANSTEASRKSLYDLTKSLVATSQVEDLVVNLVPLGRGGSGGTERQANFLGKIWPSYKGRPGNFLQSRPEPTAPPEESFRSGVETTTPPQKQEPIDKELYPLTSLRSLFGNDPSSQ

SEQ ID NO: 2 - protein, 631 aa, Synthetic construct
MGARASVLSGGELDRWEKIRSRPGGKKKYKLKHIVWASRELERFAVNPGLLETSEGCRQILGQLQPSLQTGSEELRSLYNTVATLYCVHQRIEIKDTKEALDKIEEEQNKSKKKAQQAAADTGHSNQVSQNYPIVQNIQGQMVHQAISPRTLNAWVKVVEEKAFSPEVIPMFSALSEGATPQDLNTMLNTVGGHQAAMQMLKETINEEAAEWDRVHPVHAGPIAPGQMREPRGSDIAGTTSTLQEQIGWMTNNPPIPVGEIYKRWIILGLNKIVRMYSPTSILDIRQGPKEPFRDYVDRFYKTLRAEQASQEVKNWMTETLLVQNANPDCKTILKALGPAATLEEMMTACQGVGGPGHKARVLAEAMSQVTNSATIMMQRGNFRNQRKIVKSFNSGKEGHTARNSRAPRKKGGSGGVSGWRLFKKISGGASSKTIVLSVGEATRTLTEIQSTADRQIFEEKVGPLVGRLRLTASLRQNGAKTAYRVNLKLDQADVVDSGLPKVRYTQVWSHDVTIVANSTEASRKSLYDLTKSLVATSQVEDLVVNLVPLGRGGSGGTERQANFLGKIWPSYKGRPGNFLQSRPEPTAPPEESFRSGVETTTPPQKQEPIDKELYPLTSLRSLFGNDPSSQ

SEQ ID NO: 3 - protein, 676 aa, Synthetic construct
MGARASVLSGGELDRWEKIRLRPGGKKKYKLKHIVWASRELERFAVNPGLLETSEGCRQILGQLQPSLQTGSEELRSLYNTVATLYCVHQRIEIKDTKEALDKIEEEQNKSKKKAQQAAADTGHSNQVSQNYPIVQNIQGQMVHQAISPRTLNAWVKVVEEKAFSPEVIPMFSALSEGATPQDLNTMLNTVGGHQAAMQMLKETINEEAAEWDRVHPVHAGPIAPGQMREPRGSDIAGTTSTLQEQIGWMTNNPPIPVGEIYKRWIILGLNKIVRMYSPTSILDIRQGPKEPFRDYVDRFYKTLRAEQASQEVKNWMTETLLVQNANPDCKTILKALGPAATLEEMMTACQGVGGPGHKARVLAEAMSQVTNSATIMMQRGNFRNQRKIVKSFNSGKEGHTARNSRAPRKKGGSGGVSGWRLFKKISGGSGPAAKRVKLDSGLQLPPLERLTLGAAPAAKKKKLDYKDDDDKGGASSKTIVLSVGEATRTLTEIQSTADRQIFEEKVGPLVGRLRLTASLRQNGAKTAYRVNLKLDQADVVDSGLPKVRYTQVWSHDVTIVANSTEASRKSLYDLTKSLVATSQVEDLVVNLVPLGRGGSGGTERQANFLGKIWPSYKGRPGNFLQSRPEPTAPPEESFRSGVETTTPPQKQEPIDKELYPLTSLRSLFGNDPSSQ

SEQ ID NO: 4 - protein, 631 aa, Synthetic construct
MGARASVLSGGELDRWEKIRLRPGGKKKYKLKHIVWASRELERFAVNPGLLETSEGCRQILGQLQPSLQTGSEELRSLYNTVATLYCVHQRIEIKDTKEALDKIEEEQNKSKKKAQQAAADTGHSNQVSQNYPIVQNIQGQMVHQAISPRTLNAWVKVVEEKAFSPEVIPMFSALSEGATPQDLNTMLNTVGGHQAAMQMLKETINEEAAEWDRVHPVHAGPIAPGQMREPRGSDIAGTTSTLQEQIGWMTNNPPIPVGEIYKRWIILGLNKIVRMYSPTSILDIRQGPKEPFRDYVDRFYKTLRAEQASQEVKNWMTETLLVQNANPDCKTILKALGPAATLEEMMTACQGVGGPGHKARVLAEAMSQVTNSATIMMQRGNFRNQRKIVKSFNSGKEGHTARNSRAPRKKGGSGGVSGWRLFKKISGGASSKTIVLSVGEATRTLTEIQSTADRQIFEEKVGPLVGRLRLTASLRQNGAKTAYRVNLKLDQADVVDSGLPKVRYTQVWSHDVTIVANSTEASRKSLYDLTKSLVATSQVEDLVVNLVPLGRGGSGGTERQANFLGKIWPSYKGRPGNFLQSRPEPTAPPEESFRSGVETTTPPQKQEPIDKELYPLTSLRSLFGNDPSSQ

SEQ ID NO: 5 - protein, 505 aa, Synthetic construct
MGARASVLSGGELDRWEKIRLRPGGKKKYKLKHIVWASRELERFAVNPGLLETSEGCRQILGQLQPSLQTGSEELRSLYNTVATLYCVHQRIEIKDTKEALDKIEEEQNKSKKKAQQAAADTGHSNQVSQNYPIVQNIQGQMVHQAISPRTLNAWVKVVEEKAFSPEVIPMFSALSEGATPQDLNTMLNTVGGHQAAMQMLKETINEEAAEWDRVHPVHAGPIAPGQMREPRGSDIAGTTSTLQEQIGWMTNNPPIPVGEIYKRWIILGLNKIVRMYSPTSILDIRQGPKEPFRDYVDRFYKTLRAEQASQEVKNWMTETLLVQNANPDCKTILKALGPAATLEEMMTACQGVGGPGHKARVLAEAMSQVTNSATIMMQRGNFRNQRKIVKSFNSGKEGHTARNSRAPRKKGGSGGVSGWRLFKKISASGGTERQANFLGKIWPSYKGRPGNFLQSRPEPTAPPEESFRSGVETTTPPQKQEPIDKELYPLTSLRSLFGNDPSSQ

SEQ ID NO: 6 - protein, 505 aa, Synthetic construct
MGARASVLSGGELDRWEKIRSRPGGKKKYKLKHIVWASRELERFAVNPGLLETSEGCRQILGQLQPSLQTGSEELRSLYNTVATLYCVHQRIEIKDTKEALDKIEEEQNKSKKKAQQAAADTGHSNQVSQNYPIVQNIQGQMVHQAISPRTLNAWVKVVEEKAFSPEVIPMFSALSEGATPQDLNTMLNTVGGHQAAMQMLKETINEEAAEWDRVHPVHAGPIAPGQMREPRGSDIAGTTSTLQEQIGWMTNNPPIPVGEIYKRWIILGLNKIVRMYSPTSILDIRQGPKEPFRDYVDRFYKTLRAEQASQEVKNWMTETLLVQNANPDCKTILKALGPAATLEEMMTACQGVGGPGHKARVLAEAMSQVTNSATIMMQRGNFRNQRKIVKSFNSGKEGHTARNSRAPRKKGGSGGVSGWRLFKKISASGGTERQANFLGKIWPSYKGRPGNFLQSRPEPTAPPEESFRSGVETTTPPQKQEPIDKELYPLTSLRSLFGNDPSSQ

SEQ ID NO: 7 - protein, 623 aa, Synthetic construct
MHGLQDDPDLQALLKGSQLLKVKSSSWRRERFYKLQEDCKTIWQESRKVMRSPESQLFSIEDIQEVRMGHRTEGLEKFARDIPEDRCFSIVFKDQRNTLDLIAPSPADAQHWVQGLRKIIHHSGSMDQRQKLQTGARASVLSGGELDRWEKIRLRPGGKKKYKLKHIVWASRELERFAVNPGLLETSEGCRQILGQLQPSLQTGSEELRSLYNTVATLYCVHQRIEIKDTKEALDKIEEEQNKSKKKAQQAAADTGHSNQVSQNYPIVQNIQGQMVHQAISPRTLNAWVKVVEEKAFSPEVIPMFSALSEGATPQDLNTMLNTVGGHQAAMQMLKETINEEAAEWDRVHPVHAGPIAPGQMREPRGSDIAGTTSTLQEQIGWMTNNPPIPVGEIYKRWIILGLNKIVRMYSPTSILDIRQGPKEPFRDYVDRFYKTLRAEQASQEVKNWMTETLLVQNANPDCKTILKALGPAATLEEMMTACQGVGGPGHKARVLAEAMSQVTNSATIMMQRGNFRNQRKIVKSFNSGKEGHTARNSRAPRKKGGSGGTERQANFLGKIWPSYKGRPGNFLQSRPEPTAPPEESFRSGVETTTPPQKQEPIDKELYPLTSLRSLFGNDPSSQ

SEQ ID NO: 8 - protein, 764 aa, Synthetic construct
MHGLQDDPDLQALLKGSQLLKVKSSSWRRERFYKLQEDCKTIWQESRKVMRSPESQLFSIEDIQEVRMGHRTEGLEKFARDIPEDRCFSIVFKDQRNTLDLIAPSPADAQHWVQGLRKIIHHSGSMDQRQKLQTGARASVLSGGELDRWEKIRSRPGGKKKYKLKHIVWASRELERFAVNPGLLETSEGCRQILGQLQPSLQTGSEELRSLYNTVATLYCVHQRIEIKDTKEALDKIEEEQNKSKKKAQQAAADTGHSNQVSQNYPIVQNIQGQMVHQAISPRTLNAWVKVVEEKAFSPEVIPMFSALSEGATPQDLNTMLNTVGGHQAAMQMLKETINEEAAEWDRVHPVHAGPIAPGQMREPRGSDIAGTTSTLQEQIGWMTNNPPIPVGEIYKRWIILGLNKIVRMYSPTSILDIRQGPKEPFRDYVDRFYKTLRAEQASQEVKNWMTETLLVQNANPDCKTILKALGPAATLEEMMTACQGVGGPGHKARVLAEAMSQVTNSATIMMQRGNFRNQRKIVKSFNSGKEGHTARNSRAPRKKGGSGGVSGWRLFKKISGGASSKTIVLSVGEATRTLTEIQSTADRQIFEEKVGPLVGRLRLTASLRQNGAKTAYRVNLKLDQADVVDSGLPKVRYTQVWSHDVTIVANSTEASRKSLYDLTKSLVATSQVEDLVVNLVPLGRGGSGGTERQANFLGKIWPSYKGRPGNFLQSRPEPTAPPEESFRSGVETTTPPQKQEPIDKELYPLTSLRSLFGNDPSSQ

SEQ ID NO: 9 - protein, 764 aa, Synthetic construct
MHGLQDDPDLQALLKGSQLLKVKSSSWRRERFYKLQEDCKTIWQESRKVMRSPESQLFSIEDIQEVRMGHRTEGLEKFARDIPEDRCFSIVFKDQRNTLDLIAPSPADAQHWVQGLRKIIHHSGSMDQRQKLQTGARASVLSGGELDRWEKIRLRPGGKKKYKLKHIVWASRELERFAVNPGLLETSEGCRQILGQLQPSLQTGSEELRSLYNTVATLYCVHQRIEIKDTKEALDKIEEEQNKSKKKAQQAAADTGHSNQVSQNYPIVQNIQGQMVHQAISPRTLNAWVKVVEEKAFSPEVIPMFSALSEGATPQDLNTMLNTVGGHQAAMQMLKETINEEAAEWDRVHPVHAGPIAPGQMREPRGSDIAGTTSTLQEQIGWMTNNPPIPVGEIYKRWIILGLNKIVRMYSPTSILDIRQGPKEPFRDYVDRFYKTLRAEQASQEVKNWMTETLLVQNANPDCKTILKALGPAATLEEMMTACQGVGGPGHKARVLAEAMSQVTNSATIMMQRGNFRNQRKIVKSFNSGKEGHTARNSRAPRKKGGSGGVSGWRLFKKISGGASSKTIVLSVGEATRTLTEIQSTADRQIFEEKVGPLVGRLRLTASLRQNGAKTAYRVNLKLDQADVVDSGLPKVRYTQVWSHDVTIVANSTEASRKSLYDLTKSLVATSQVEDLVVNLVPLGRGGSGGTERQANFLGKIWPSYKGRPGNFLQSRPEPTAPPEESFRSGVETTTPPQKQEPIDKELYPLTSLRSLFGNDPSSQ

SEQ ID NO: 10 - protein, 779 aa, Synthetic construct
MHGLQDDPDLQALLKGSQLLKVKSSSWRRERFYKLQEDCKTIWQESRKVMRSPESQLFSIEDIQEVRMGHRTEGLEKFARDIPEDRCFSIVFKDQRNTLDLIAPSPADAQHWVQGLRKIIHHSGSMDQRQKLQTGARASVLSGGELDRWEKIRSRPGGKKKYKLKHIVWASRELERFAVNPGLLETSEGCRQILGQLQPSLQTGSEELRSLYNTVATLYCVHQRIEIKDTKEALDKIEEEQNKSKKKAQQAAADTGHSNQVSQNYPIVQNIQGQMVHQAISPRTLNAWVKVVEEKAFSPEVIPMFSALSEGATPQDLNTMLNTVGGHQAAMQMLKETINEEAAEWDRVHPVHAGPIAPGQMREPRGSDIAGTTSTLQEQIGWMTNNPPIPVGEIYKRWIILGLNKIVRMYSPTSILDIRQGPKEPFRDYVDRFYKTLRAEQASQEVKNWMTETLLVQNANPDCKTILKALGPAATLEEMMTACQGVGGPGHKARVLAEAMSQVTNSATIMMQRGNFRNQRKIVKCFNCGKEGHTARNCRAPRKKGCWKCGKEGHQMKDCGGSGGVSGWRLFKKISGGASSKTIVLSVGEATRTLTEIQSTADRQIFEEKVGPLVGRLRLTASLRQNGAKTAYRVNLKLDQADVVDSGLPKVRYTQVWSHDVTIVANSTEASRKSLYDLTKSLVATSQVEDLVVNLVPLGRGGSGGTERQANFLGKIWPSYKGRPGNFLQSRPEPTAPPEESFRSGVETTTPPQKQEPIDKELYPLTSLRSLFGNDPSSQ

SEQ ID NO: 11 - protein, 809 aa, Synthetic construct
MHGLQDDPDLQALLKGSQLLKVKSSSWRRERFYKLQEDCKTIWQESRKVMRSPESQLFSIEDIQEVRMGHRTEGLEKFARDIPEDRCFSIVFKDQRNTLDLIAPSPADAQHWVQGLRKIIHHSGSMDQRQKLQTGARASVLSGGELDRWEKIRSRPGGKKKYKLKHIVWASRELERFAVNPGLLETSEGCRQILGQLQPSLQTGSEELRSLYNTVATLYCVHQRIEIKDTKEALDKIEEEQNKSKKKAQQAAADTGHSNQVSQNYPIVQNIQGQMVHQAISPRTLNAWVKVVEEKAFSPEVIPMFSALSEGATPQDLNTMLNTVGGHQAAMQMLKETINEEAAEWDRVHPVHAGPIAPGQMREPRGSDIAGTTSTLQEQIGWMTNNPPIPVGEIYKRWIILGLNKIVRMYSPTSILDIRQGPKEPFRDYVDRFYKTLRAEQASQEVKNWMTETLLVQNANPDCKTILKALGPAATLEEMMTACQGVGGPGHKARVLAEAMSQVTNSATIMMQRGNFRNQRKIVKSFNSGKEGHTARNSRAPRKKGGSGGVSGWRLFKKISGGSGPAAKRVKLDSGLQLPPLERLTLGAAPAAKKKKLDYKDDDDKGGASSKTIVLSVGEATRTLTEIQSTADRQIFEEKVGPLVGRLRLTASLRQNGAKTAYRVNLKLDQADVVDSGLPKVRYTQVWSHDVTIVANSTEASRKSLYDLTKSLVATSQVEDLVVNLVPLGRGGSGGTERQANFLGKIWPSYKGRPGNFLQSRPEPTAPPEESFRSGVETTTPPQKQEPIDKELYPLTSLRSLFGNDPSSQ

SEQ ID NO: 12 - protein, 366 aa, Synthetic construct
MGARASVLSGGAQQAAADTGHSNQVSQNYSPTSILDIRQGPKEPFRDYVDRFYKTLRAEQASQEVKNWMTETLLVQNANPDCKTILKALGPAATLEEMMTACQGVGGPGHKARVLAEAMSQVTNSATIMGGSGGRMKQLEDKVEELLSKNYHLENEVARLKKLVGERGGSGGVSGWRLFKKISGGASSKTIVLSVGEATRTLTEIQSTADRQIFEEKVGPLVGRLRLTASLRQNGAKTAYRVNLKLDQADVVDSGLPKVRYTQVWSHDVTIVANSTEASRKSLYDLTKSLVATSQVEDLVVNLVPLGRGGSAGGLQSRPEPTAPPEESFRSGVETTTPPQKQEPIDKELYPLTSLRSLFGNDPSSQ

SEQ ID NO: 13 - protein, 411 aa, Synthetic construct
MGARASVLSGGAQQAAADTGHSNQVSQNYSPTSILDIRQGPKEPFRDYVDRFYKTLRAEQASQEVKNWMTETLLVQNANPDCKTILKALGPAATLEEMMTACQGVGGPGHKARVLAEAMSQVTNSATIMGGSGGRMKQLEDKVEELLSKNYHLENEVARLKKLVGERGGSGGVSGWRLFKKISGGSGPAAKRVKLDSGLQLPPLERLTLGAAPAAKKKKLDYKDDDDKGGASSKTIVLSVGEATRTLTEIQSTADRQIFEEKVGPLVGRLRLTASLRQNGAKTAYRVNLKLDQADVVDSGLPKVRYTQVWSHDVTIVANSTEASRKSLYDLTKSLVATSQVEDLVVNLVPLGRGGSAGGLQSRPEPTAPPEESFRSGVETTTPPQKQEPIDKELYPLTSLRSLFGNDPSSQ

SEQ ID NO: 14 - protein, 403 aa, Synthetic construct
MGARASVLSGGAQQAAADTGHSNQVSQNYSPTSILDIRQGPKEPFRDYVDRFYKTLRAEQASQEVKNWMTETLLVQNANPDCKTILKALGPAATLEEMMTACQGVGGPGHKARVLAEAMSQVTNSATIMGGSGGRMKQLEDKVEELLSKNYHLENEVARLKKLVGERGGSGGVSGWRLFKKISGGSGPAAKKKKNGSGLQLPPLERLTLGAADYKDDDDKGGASSKTIVLSVGEATRTLTEIQSTADRQIFEEKVGPLVGRLRLTASLRQNGAKTAYRVNLKLDQADVVDSGLPKVRYTQVWSHDVTIVANSTEASRKSLYDLTKSLVATSQVEDLVVNLVPLGRGGSAGGLQSRPEPTAPPEESFRSGVETTTPPQKQEPIDKELYPLTSLRSLFGNDPSSQ

SEQ ID NO: 15 - protein, 401 aa, Synthetic construct
MGARASVLSGGAQQAAADTGHSNQVSQNYSPTSILDIRQGPKEPFRDYVDRFYKTLRAEQASQEVKNWMTETLLVQNANPDCKTILKALGPAATLEEMMTACQGVGGPGHKARVLAEAMSQVTNSATIMGGSGGRMKQLEDKVEELLSKNYHLENEVARLKKLVGERGGSGGVSGWRLFKKISGGSGPKKKRKVSGLQLPPLERLTLGAADYKDDDDKGGASSKTIVLSVGEATRTLTEIQSTADRQIFEEKVGPLVGRLRLTASLRQNGAKTAYRVNLKLDQADVVDSGLPKVRYTQVWSHDVTIVANSTEASRKSLYDLTKSLVATSQVEDLVVNLVPLGRGGSAGGLQSRPEPTAPPEESFRSGVETTTPPQKQEPIDKELYPLTSLRSLFGNDPSSQ

SEQ ID NO: 16 - protein, 511 aa, Synthetic construct
MGARASVLSGGAQQAAADTGHSNQVSQNYPIVQNIQGQMVHQAISPRTLNAWVKVVEEKAFSPEVIPMFSALSEGATPQDLNTMLNTVGGHQAAMQMLKETINEEAAEWDRVHPVHAGPIAPGQMREPRGSDIAGTTSTLQEQIGWMTNNPPIPVGEIYKRWIILGLNKIVRMYSPTSILDIRQGPKEPFRDYVDRFYKTLRAEQASQEVKNWMTETLLVQNANPDCKTILKALGPAATLEEMMTACQGVGGPGHKARVLAEAMSQVTNSATIMGGSGGRMKQLEDKVEELLSKNYHLENEVARLKKLVGERGGSGGVSGWRLFKKISGGASSKTIVLSVGEATRTLTEIQSTADRQIFEEKVGPLVGRLRLTASLRQNGAKTAYRVNLKLDQADVVDSGLPKVRYTQVWSHDVTIVANSTEASRKSLYDLTKSLVATSQVEDLVVNLVPLGRGGSAGGLQSRPEPTAPPEESFRSGVETTTPPQKQEPIDKELYPLTSLRSLFGNDPSSQ

SEQ ID NO: 17 - protein, 556 aa, Synthetic construct
MGARASVLSGGAQQAAADTGHSNQVSQNYPIVQNIQGQMVHQAISPRTLNAWVKVVEEKAFSPEVIPMFSALSEGATPQDLNTMLNTVGGHQAAMQMLKETINEEAAEWDRVHPVHAGPIAPGQMREPRGSDIAGTTSTLQEQIGWMTNNPPIPVGEIYKRWIILGLNKIVRMYSPTSILDIRQGPKEPFRDYVDRFYKTLRAEQASQEVKNWMTETLLVQNANPDCKTILKALGPAATLEEMMTACQGVGGPGHKARVLAEAMSQVTNSATIMGGSGGRMKQLEDKVEELLSKNYHLENEVARLKKLVGERGGSGGVSGWRLFKKISGGSGPAAKRVKLDSGLQLPPLERLTLGAAPAAKKKKLDYKDDDDKGGASSKTIVLSVGEATRTLTEIQSTADRQIFEEKVGPLVGRLRLTASLRQNGAKTAYRVNLKLDQADVVDSGLPKVRYTQVWSHDVTIVANSTEASRKSLYDLTKSLVATSQVEDLVVNLVPLGRGGSAGGLQSRPEPTAPPEESFRSGVETTTPPQKQEPIDKELYPLTSLRSLFGNDPSSQ

SEQ ID NO: 18 - protein, 499 aa, Synthetic construct
MHGLQDDPDLQALLKGSQLLKVKSSSWRRERFYKLQEDCKTIWQESRKVMRSPESQLFSIEDIQEVRMGHRTEGLEKFARDIPEDRCFSIVFKDQRNTLDLIAPSPADAQHWVQGLRKIIHHSGSMDQRQKLQTGARASVLSGGAQQAAADTGHSNQVSQNYSPTSILDIRQGPKEPFRDYVDRFYKTLRAEQASQEVKNWMTETLLVQNANPDCKTILKALGPAATLEEMMTACQGVGGPGHKARVLAEAMSQVTNSATIMGGSGGRMKQLEDKVEELLSKNYHLENEVARLKKLVGERGGSGGVSGWRLFKKISGGASSKTIVLSVGEATRTLTEIQSTADRQIFEEKVGPLVGRLRLTASLRQNGAKTAYRVNLKLDQADVVDSGLPKVRYTQVWSHDVTIVANSTEASRKSLYDLTKSLVATSQVEDLVVNLVPLGRGGSAGGLQSRPEPTAPPEESFRSGVETTTPPQKQEPIDKELYPLTSLRSLFGNDPSSQ

SEQ ID NO: 19 - protein, 544 aa, Synthetic construct
MHGLQDDPDLQALLKGSQLLKVKSSSWRRERFYKLQEDCKTIWQESRKVMRSPESQLFSIEDIQEVRMGHRTEGLEKFARDIPEDRCFSIVFKDQRNTLDLIAPSPADAQHWVQGLRKIIHHSGSMDQRQKLQTGARASVLSGGAQQAAADTGHSNQVSQNYSPTSILDIRQGPKEPFRDYVDRFYKTLRAEQASQEVKNWMTETLLVQNANPDCKTILKALGPAATLEEMMTACQGVGGPGHKARVLAEAMSQVTNSATIMGGSGGRMKQLEDKVEELLSKNYHLENEVARLKKLVGERGGSGGVSGWRLFKKISGGSGPAAKRVKLDSGLQLPPLERLTLGAAPAAKKKKLDYKDDDDKGGASSKTIVLSVGEATRTLTEIQSTADRQIFEEKVGPLVGRLRLTASLRQNGAKTAYRVNLKLDQADVVDSGLPKVRYTQVWSHDVTIVANSTEASRKSLYDLTKSLVATSQVEDLVVNLVPLGRGGSAGGLQSRPEPTAPPEESFRSGVETTTPPQKQEPIDKELYPLTSLRSLFGNDPSSQ

SEQ ID NO: 20 - protein, 536 aa, Synthetic construct
MHGLQDDPDLQALLKGSQLLKVKSSSWRRERFYKLQEDCKTIWQESRKVMRSPESQLFSIEDIQEVRMGHRTEGLEKFARDIPEDRCFSIVFKDQRNTLDLIAPSPADAQHWVQGLRKIIHHSGSMDQRQKLQTGARASVLSGGAQQAAADTGHSNQVSQNYSPTSILDIRQGPKEPFRDYVDRFYKTLRAEQASQEVKNWMTETLLVQNANPDCKTILKALGPAATLEEMMTACQGVGGPGHKARVLAEAMSQVTNSATIMGGSGGRMKQLEDKVEELLSKNYHLENEVARLKKLVGERGGSGGVSGWRLFKKISGGSGPAAKKKKLDSGLQLPPLERLTLGAADYKDDDDKGGASSKTIVLSVGEATRTLTEIQSTADRQIFEEKVGPLVGRLRLTASLRQNGAKTAYRVNLKLDQADVVDSGLPKVRYTQVWSHDVTIVANSTEASRKSLYDLTKSLVATSQVEDLVVNLVPLGRGGSAGGLQSRPEPTAPPEESFRSGVETTTPPQKQEPIDKELYPLTSLRSLFGNDPSSQ

SEQ ID NO: 21 - protein, 536 aa, Synthetic construct
MHGLQDDPDLQALLKGSQLLKVKSSSWRRERFYKLQEDCKTIWQESRKVMRSPESQLFSIEDIQEVRMGHRTEGLEKFARDIPEDRCFSIVFKDQRNTLDLIAPSPADAQHWVQGLRKIIHHSGSMDQRQKLQTGARASVLSGGAQQAAADTGHSNQVSQNYSPTSILDIRQGPKEPFRDYVDRFYKTLRAEQASQEVKNWMTETLLVQNANPDCKTILKALGPAATLEEMMTACQGVGGPGHKARVLAEAMSQVTNSATIMGGSGGRMKQLEDKVEELLSKNYHLENEVARLKKLVGERGGSGGVSGWRLFKKISGGSGPAAKRVKLDSGLQLPPLERLTLGAADYKDDDDKGGASSKTIVLSVGEATRTLTEIQSTADRQIFEEKVGPLVGRLRLTASLRQNGAKTAYRVNLKLDQADVVDSGLPKVRYTQVWSHDVTIVANSTEASRKSLYDLTKSLVATSQVEDLVVNLVPLGRGGSAGGLQSRPEPTAPPEESFRSGVETTTPPQKQEPIDKELYPLTSLRSLFGNDPSSQ

SEQ ID NO: 22 - protein, 536 aa, Synthetic construct
MHGLQDDPDLQALLKGSQLLKVKSSSWRRERFYKLQEDCKTIWQESRKVMRSPESQLFSIEDIQEVRMGHRTEGLEKFARDIPEDRCFSIVFKDQRNTLDLIAPSPADAQHWVQGLRKIIHHSGSMDQRQKLQTGARASVLSGGAQQAAADTGHSNQVSQNYSPTSILDIRQGPKEPFRDYVDRFYKTLRAEQASQEVKNWMTETLLVQNANPDCKTILKALGPAATLEEMMTACQGVGGPGHKARVLAEAMSQVTNSATIMGGSGGRMKQLEDKVEELLSKNYHLENEVARLKKLVGERGGSGGVSGWRLFKKISGGSGPAAKKKKNGSGLQLPPLERLTLGAADYKDDDDKGGASSKTIVLSVGEATRTLTEIQSTADRQIFEEKVGPLVGRLRLTASLRQNGAKTAYRVNLKLDQADVVDSGLPKVRYTQVWSHDVTIVANSTEASRKSLYDLTKSLVATSQVEDLVVNLVPLGRGGSAGGLQSRPEPTAPPEESFRSGVETTTPPQKQEPIDKELYPLTSLRSLFGNDPSSQ

SEQ ID NO: 23 - protein, 534 aa, Synthetic construct
MHGLQDDPDLQALLKGSQLLKVKSSSWRRERFYKLQEDCKTIWQESRKVMRSPESQLFSIEDIQEVRMGHRTEGLEKFARDIPEDRCFSIVFKDQRNTLDLIAPSPADAQHWVQGLRKIIHHSGSMDQRQKLQTGARASVLSGGAQQAAADTGHSNQVSQNYSPTSILDIRQGPKEPFRDYVDRFYKTLRAEQASQEVKNWMTETLLVQNANPDCKTILKALGPAATLEEMMTACQGVGGPGHKARVLAEAMSQVTNSATIMGGSGGRMKQLEDKVEELLSKNYHLENEVARLKKLVGERGGSGGVSGWRLFKKISGGSGPKKKRKVSGLQLPPLERLTLGAADYKDDDDKGGASSKTIVLSVGEATRTLTEIQSTADRQIFEEKVGPLVGRLRLTASLRQNGAKTAYRVNLKLDQADVVDSGLPKVRYTQVWSHDVTIVANSTEASRKSLYDLTKSLVATSQVEDLVVNLVPLGRGGSAGGLQSRPEPTAPPEESFRSGVETTTPPQKQEPIDKELYPLTSLRSLFGNDPSSQ

SEQ ID NO: 24 - protein, 749 aa, Synthetic construct
MGARASVLSGGELDRWEKIRSRPGGKKKYKLKHIVWASRELERFAVNPGLLETSEGCRQILGQLQPSLQTGSEELRSLYNTVATLYCVHQRIEIKDTKEALDKIEEEQNKSKKKAQQAAADTGHSNQVSQNYPIVQNIQGQMVHQAISPRTLNAWVKVVEEKAFSPEVIPMFSALSEGATPQDLNTMLNTVGGHQAAMQMLKETINEEAAEWDRVHPVHAGPIAPGQMREPRGSDIAGTTSTLQEQIGWMTNNPPIPVGEIYKRWIILGLNKIVRMYSPTSILDIRQGPKEPFRDYVDRFYKTLRAEQASQEVKNWMTETLLVQNANPDCKTILKALGPAATLEEMMTACQGVGGPGHKARVLAEAMSQVTNSATIMMQRGNFRNQRKIVKSFNSGKEGHTARNSRAPRKKGGSGGVSGWRLFKKISGGSGPAAKRVKLDSGLQLPPLERLTLGAAPAAKKKKLDYKDDDDKGGASPGGGSGGTERQANFLGKIWPSYKGRPGNFLQSRPEPTAPPEESFRSGVETTTPPQKQEPIDKELYPLTSLRSLFGNDPSSQGGGGGMDHYLDIRLRPDPEFPPAQLMSVLFGKLHQALVAQGGDRIGVSFPDLDESRSRLGERLRIHASADDLRALLARPWLEGLRDHLQFGEPAVVPHPTPYRQVSRVQAKSNPERLRRRLMRRHDLSEEEARKRIPDTVARALDLPFVTLRSQSTGQHFRLFIRHGPLQVTAEEGGFTCYGLSKGGFVPWF

SEQ ID NO: 25 - protein, 747 aa, Synthetic construct
MGARASVLSGGELDRWEKIRSRPGGKKKYKLKHIVWASRELERFAVNPGLLETSEGCRQILGQLQPSLQTGSEELRSLYNTVATLYCVHQRIEIKDTKEALDKIEEEQNKSKKKAQQAAADTGHSNQVSQNYPIVQNIQGQMVHQAISPRTLNAWVKVVEEKAFSPEVIPMFSALSEGATPQDLNTMLNTVGGHQAAMQMLKETINEEAAEWDRVHPVHAGPIAPGQMREPRGSDIAGTTSTLQEQIGWMTNNPPIPVGEIYKRWIILGLNKIVRMYSPTSILDIRQGPKEPFRDYVDRFYKTLRAEQASQEVKNWMTETLLVQNANPDCKTILKALGPAATLEEMMTACQGVGGPGHKARVLAEAMSQVTNSATIMMQRGNFRNQRKIVKSFNSGKEGHTARNSRAPRKKGGSGGVSGWRLFKKISGGSGPAAKRVKLDSGLQLPPLERLTLGAAPAAKKKKLDYKDDDDKGGASPGGGGMDHYLDIRLRPDPEFPPAQLMSVLFGKLHQALVAQGGDRIGVSFPDLDESRSRLGERLRIHASADDLRALLARPWLEGLRDHLQFGEPAVVPHPTPYRQVSRVQAKSNPERLRRRLMRRHDLSEEEARKRIPDTVARALDLPFVTLRSQSTGQHFRLFIRHGPLQVTAEEGGFTCYGLSKGGFVPWFGGSGGTERQANFLGKIWPSYKGRPGNFLQSRPEPTAPPEESFRSGVETTTPPQKQEPIDKELYPLTSLRSLFGNDPSSQ

SEQ ID NO: 26 - protein, 500 aa, Synthetic construct
MGARASVLSGGELDRWEKIRLRPGGKKKYKLKHIVWASRELERFAVNPGLLETSEGCRQILGQLQPSLQTGSEELRSLYNTVATLYCVHQRIEIKDTKEALDKIEEEQNKSKKKAQQAAADTGHSNQVSQNYPIVQNIQGQMVHQAISPRTLNAWVKVVEEKAFSPEVIPMFSALSEGATPQDLNTMLNTVGGHQAAMQMLKETINEEAAEWDRVHPVHAGPIAPGQMREPRGSDIAGTTSTLQEQIGWMTHNPPIPVGEIYKRWIILGLNKIVRMYSPTSILDIRQGPKEPFRDYVDRFYKTLRAEQASQEVKNWMTETLLVQNANPDCKTILKALGPGATLEEMMTACQGVGGPGHKARVLAEAMSQVTNPATIMIQKGNFRNQRKTVKCFNCGKEGHIAKNCRAPRKKGCWKCGKEGHQMKDCTERQANFLGKIWPSHKGRPGNFLQSRPEPTAPPEESFRFGEETTTPSQKQEPIDKELYPLASLRSLFGSDPSSQ

SEQ ID NO: 27 - protein, 1435 aa, Synthetic construct
MGARASVLSGGELDRWEKIRLRPGGKKKYKLKHIVWASRELERFAVNPGLLETSEGCRQILGQLQPSLQTGSEELRSLYNTVATLYCVHQRIEIKDTKEALDKIEEEQNKSKKKAQQAAADTGHSNQVSQNYPIVQNIQGQMVHQAISPRTLNAWVKVVEEKAFSPEVIPMFSALSEGATPQDLNTMLNTVGGHQAAMQMLKETINEEAAEWDRVHPVHAGPIAPGQMREPRGSDIAGTTSTLQEQIGWMTHNPPIPVGEIYKRWIILGLNKIVRMYSPTSILDIRQGPKEPFRDYVDRFYKTLRAEQASQEVKNWMTETLLVQNANPDCKTILKALGPGATLEEMMTACQGVGGPGHKARVLAEAMSQVTNPATIMIQKGNFRNQRKTVKCFNCGKEGHIAKNCRAPRKKGCWKCGKEGHQMKDCTERQANFFREDLAFPQGKAREFSSEQTRANSPTRRELQVWGRDNNSLSEAGADRQGTVSFSFPQITLWQRPLVTIKIGGQLKEALLDTGADDTVLEEMNLPGRWKPKMIGGIGGFIKVRQYDQILIEICGHKAIGTVLVGPTPVNIIGRNLLTQIGCTLNFPISPIETVPVKLKPGMDGPKVKQWPLTEEKIKALVEICTEMEKEGKISKIGPENPYNTPVFAIKKKDSTKWRKLVDFRELNKRTQDFWEVQLGIPHPAGLKQKKSVTVLDVGDAYFSVPLDKDFRKYTAFTIPSINNETPGIRYQYNVLPQGWKGSPAIFQCSMTKILEPFRKQNPDIVIYQYMDDLYVGSDLEIGQHRTKIEELRQHLLRWGFTTPDKKHQKEPPFLWMGYELHPDKWTVQPIVLPEKDSWTVNDIQKLVGKLNWASQIYAGIKVRQLCKLLRGTKALTEVVPLTEEAELELAENREILKEPVHGVYYDPSKDLIAEIQKQGQGQWTYQIYQEPFKNLKTGKYARMKGAHTNDVKQLTEAVQKIATESIVIWGKTPKFKLPIQKETWEAWWTEYWQATWIPEWEFVNTPPLVKLWYQLEKEPIIGAETFYVDGAANRETKLGKAGYVTDRGRQKVVPLTDTTNQKTELQAIHLALQDSGLEVNIVTDSQYALGIIQAQPDKSESELVSQIIEQLIKKEKVYLAWVPAHKGIGGNEQVDKLVSAGIRKVLFLDGIDKAQEEHEKYHSNWRAMASDFNLPPVVAKEIVASCDKCQLKGEAMHGQVDCSPGIWQLVCTHLEGKVILVAVHVASGYIEAEVIPAETGQETAYFLLKLAGRWPVKTVHTDNGSNFTSTTVKAACWWAGIKQEFGIPYNPQSQGVIESMNKELKKIIGQVRDQAEHLKTAVQMAVFIHNFKRKGGIGGYSAGERIVDIIATDIQTKELQKQITKIQNFRVYYRDSRDPVWKGPAKLLWKGEGAVVIQDNSDIKVVPRRKAKIIRDYGKQMAGDDCVASRQDED

SEQ ID NO: 28 - protein, 2136 aa, Synthetic construct
MDKKYSIGLDIGTNSVGWAVITDEYKVPSKKFKVLGNTDRHSIKKNLIGALLFDSGETAEATRLKRTARRRYTRRKNRICYLQEIFSNEMAKVDDSFFHRLEESFLVEEDKKHERHPIFGNIVDEVAYHEKYPTIYHLRKKLVDSTDKADLRLIYLALAHMIKFRGHFLIEGDLNPDNSDVDKLFIQLVQTYNQLFEENPINASGVDAKAILSARLSKSRRLENLIAQLPGEKKNGLFGNLIALSLGLTPNFKSNFDLAEDAKLQLSKDTYDDDLDNLLAQIGDQYADLFLAAKNLSDAILLSDILRVNTEITKAPLSASMIKRYDEHHQDLTLLKALVRQQLPEKYKEIFFDQSKNGYAGYIDGGASQEEFYKFIKPILEKMDGTEELLVKLNREDLLRKQRTFDNGSIPHQIHLGELHAILRRQEDFYPFLKDNREKIEKILTFRIPYYVGPLARGNSRFAWMTRKSEETITPWNFEEVVDKGASAQSFIERMTNFDKNLPNEKVLPKHSLLYEYFTVYNELTKVKYVTEGMRKPAFLSGEQKKAIVDLLFKTNRKVTVKQLKEDYFKKIECFDSVEISGVEDRFNASLGTYHDLLKIIKDKDFLDNEENEDILEDIVLTLTLFEDREMIEERLKTYAHLFDDKVMKQLKRRRYTGWGRLSRKLINGIRDKQSGKTILDFLKSDGFANRNFMQLIHDDSLTFKEDIQKAQVSGQGDSLHEHIANLAGSPAIKKGILQTVKVVDELVKVMGRHKPENIVIEMARENQTTQKGQKNSRERMKRIEEGIKELGSQILKEHPVENTQLQNEKLYLYYLQNGRDMYVDQELDINRLSDYDVDHIVPQSFLKDDSIDNKVLTRSDKARGKSDNVPSEEVVKKMKNYWRQLLNAKLITQRKFDNLTKAERGGLSELDKAGFIKRQLVETRQITKHVAQILDSRMNTKYDENDKLIREVKVITLKSKLVSDFRKDFQFYKVREINNYHHAHDAYLNAVVGTALIKKYPKLESEFVYGDYKVYDVRKMIAKSEQEIGKATAKYFFYSNIMNFFKTEITLANGEIRKRPLIETNGETGEIVWDKGRDFATVRKVLSMPQVNIVKKTEVQTGGFSKESILPKRNSDKLIARKKDWDPKKYGGFDSPTVAYSVLVVAKVEKGKSKKLKSVKELLGITIMERSSFEKNPIDFLEAKGYKEVKKDLIIKLPKYSLFELENGRKRMLASAGELQKGNELALPSKYVNFLYLASHYEKLKGSPEDNEQKQLFVEQHKHYLDEIIEQISEFSKRVILADANLDKVLSAYNKHRDKPIREQAENIIHLFTLTNLGAPAAFKYFDTTIDRKRYTSTKEVLDATLIHQSITGLYETRIDLSQLGGDAYPYDVPDYASLGSGSPKKKRKVEDGEGPAAKRVKLDSGAAPAAKKKKLDTGGPGSEPATSGSETPGTSESATPESGPGASTLNIEDEYRLHETSKEPDVSLGSTWLSDFPQAWAETGGMGLAVRQAPLIIPLKATSTPVSIKQYPMSQEARLGIKPHIQRLLDQGILVPCQSPWNTPLLPVKKPGTNDYRPVQDLREVNKRVEDIHPTVPNPYNLLSGLPPSHQWYTVLDLKDAFFCLRLHPTSQPLFAFEWRDPEMGISGQLTWTRLPQGFKNSPTLFNEALHRDLADFRIQHPDLILLQYVDDLLLAATSELDCQQGTRALLQTLGNLGYRASAKKAQICQKQVKYLGYLLKEGQRWLTEARKETVMGQPTPKTPRQLREFLGKAGFCRLFIPGFAEMAAPLYPLTKPGTLFNWGPDQQKAYQEIKQALLTAPALGLPDLTKPFELFVDEKQGYAKGVLTQKLGPWRRPVAYLSKKLDPVAAGWPPCLRMVAAIAVLTKDAGKLTMGQPLVILAPHAVEALVKQPPDRWLSNARMTHYQALLLDTDRVQFGPVVALNPATLLPLPEEGLQHNCLDILAEAHGTRPDLTDQPLPDADHTWYTDGSSLLQEGQRKAGAAVTTETEVIWAKALPAGTSAQRAELIALTQALKMAEGKKLNVYTDSRYAFATAHIHGEIYRRRGWLTSEGKEIKNKDEILALLKALFLPKRLSIIHCPGHQKGHSAEARGNRMADQAARKAAITETPDTSTLLIENSSPGTPKKKRKVD

SEQ ID NO: 29 - protein, 1946 aa, Synthetic construct
MDKKYSIGLDIGTNSVGWAVITDEYKVPSKKFKVLGNTDRHSIKKNLIGALLFDSGETAEATRLKRTARRRYTRRKNRICYLQEIFSNEMAKVDDSFFHRLEESFLVEEDKKHERHPIFGNIVDEVAYHEKYPTIYHLRKKLVDSTDKADLRLIYLALAHMIKFRGHFLIEGDLNPDNSDVDKLFIQLVQTYNQLFEENPINASGVDAKAILSARLSKSRRLENLIAQLPGEKKNGLFGNLIALSLGLTPNFKSNFDLAEDAKLQLSKDTYDDDLDNLLAQIGDQYADLFLAAKNLSDAILLSDILRVNTEITKAPLSASMIKRYDEHHQDLTLLKALVRQQLPEKYKEIFFDQSKNGYAGYIDGGASQEEFYKFIKPILEKMDGTEELLVKLNREDLLRKQRTFDNGSIPHQIHLGELHAILRRQEDFYPFLKDNREKIEKILTFRIPYYVGPLARGNSRFAWMTRKSEETITPWNFEEVVDKGASAQSFIERMTNFDKNLPNEKVLPKHSLLYEYFTVYNELTKVKYVTEGMRKPAFLSGEQKKAIVDLLFKTNRKVTVKQLKEDYFKKIECFDSVEISGVEDRFNASLGTYHDLLKIIKDKDFLDNEENEDILEDIVLTLTLFEDREMIEERLKTYAHLFDDKVMKQLKRRRYTGWGRLSRKLINGIRDKQSGKTILDFLKSDGFANRNFMQLIHDDSLTFKEDIQKAQVSGQGDSLHEHIANLAGSPAIKKGILQTVKVVDELVKVMGRHKPENIVIEMARENQTTQKGQKNSRERMKRIEEGIKELGSQILKEHPVENTQLQNEKLYLYYLQNGRDMYVDQELDINRLSDYDVDHIVPQSFLKDDSIDNKVLTRSDKARGKSDNVPSEEVVKKMKNYWRQLLNAKLITQRKFDNLTKAERGGLSELDKAGFIKRQLVETRQITKHVAQILDSRMNTKYDENDKLIREVKVITLKSKLVSDFRKDFQFYKVREINNYHHAHDAYLNAVVGTALIKKYPKLESEFVYGDYKVYDVRKMIAKSEQEIGKATAKYFFYSNIMNFFKTEITLANGEIRKRPLIETNGETGEIVWDKGRDFATVRKVLSMPQVNIVKKTEVQTGGFSKESILPKRNSDKLIARKKDWDPKKYGGFDSPTVAYSVLVVAKVEKGKSKKLKSVKELLGITIMERSSFEKNPIDFLEAKGYKEVKKDLIIKLPKYSLFELENGRKRMLASAGELQKGNELALPSKYVNFLYLASHYEKLKGSPEDNEQKQLFVEQHKHYLDEIIEQISEFSKRVILADANLDKVLSAYNKHRDKPIREQAENIIHLFTLTNLGAPAAFKYFDTTIDRKRYTSTKEVLDATLIHQSITGLYETRIDLSQLGGDAYPYDVPDYASLGSGSPKKKRKVEDGEGPAAKRVKLDSGAAPAAKKKKLDTGGPGSEPATSGSETPGTSESATPESGPGASTLNIEDEYRLHETSKEPDVSLGSTWLSDFPQAWAETGGMGLAVRQAPLIIPLKATSTPVSIKQYPMSQEARLGIKPHIQRLLDQGILVPCQSPWNTPLLPVKKPGTNDYRPVQDLREVNKRVEDIHPTVPNPYNLLSGLPPSHQWYTVLDLKDAFFCLRLHPTSQPLFAFEWRDPEMGISGQLTWTRLPQGFKNSPTLFNEALHRDLADFRIQHPDLILLQYVDDLLLAATSELDCQQGTRALLQTLGNLGYRASAKKAQICQKQVKYLGYLLKEGQRWLTEARKETVMGQPTPKTPRQLREFLGKAGFCRLFIPGFAEMAAPLYPLTKPGTLFNWGPDQQKAYQEIKQALLTAPALGLPDLTKPFELFVDEKQGYAKGVLTQKLGPWRRPVAYLSKKLDPVAAGWPPCLRMVAAIAVLTKDAGKLTMGQPLVILAPHAVEALVKQPPDRWLSNARMTHYQALLLDTDRVQFGPVVALNPATLLPLPEEGLQHNSRK

SEQ ID NO: 30 - protein, 2138 aa, Synthetic construct
MTLNIEDEYRLHETSKEPDVSLGSTWLSDFPQAWAETGGMGLAVRQAPLIIPLKATSTPVSIKQYPMSQEARLGIKPHIQRLLDQGILVPCQSPWNTPLLPVKKPGTNDYRPVQDLREVNKRVEDIHPTVPNPYNLLSGLPPSHQWYTVLDLKDAFFCLRLHPTSQPLFAFEWRDPEMGISGQLTWTRLPQGFKNSPTLFNEALHRDLADFRIQHPDLILLQYVDDLLLAATSELDCQQGTRALLQTLGNLGYRASAKKAQICQKQVKYLGYLLKEGQRWLTEARKETVMGQPTPKTPRQLREFLGKAGFCRLFIPGFAEMAAPLYPLTKPGTLFNWGPDQQKAYQEIKQALLTAPALGLPDLTKPFELFVDEKQGYAKGVLTQKLGPWRRPVAYLSKKLDPVAAGWPPCLRMVAAIAVLTKDAGKLTMGQPLVILAPHAVEALVKQPPDRWLSNARMTHYQALLLDTDRVQFGPVVALNPATLLPLPEEGLQHNCLDILAEAHGTRPDLTDQPLPDADHTWYTDGSSLLQEGQRKAGAAVTTETEVIWAKALPAGTSAQRAELIALTQALKMAEGKKLNVYTDSRYAFATAHIHGEIYRRRGWLTSEGKEIKNKDEILALLKALFLPKRLSIIHCPGHQKGHSAEARGNRMADQAARKAAITETPDTSTLLIENSSPGSTPPKKKRKVEDGEGTGGPGSEPATSGSETPGTSESATPESGPGGSGDKKYSIGLDIGTNSVGWAVITDEYKVPSKKFKVLGNTDRHSIKKNLIGALLFDSGETAEATRLKRTARRRYTRRKNRICYLQEIFSNEMAKVDDSFFHRLEESFLVEEDKKHERHPIFGNIVDEVAYHEKYPTIYHLRKKLVDSTDKADLRLIYLALAHMIKFRGHFLIEGDLNPDNSDVDKLFIQLVQTYNQLFEENPINASGVDAKAILSARLSKSRRLENLIAQLPGEKKNGLFGNLIALSLGLTPNFKSNFDLAEDAKLQLSKDTYDDDLDNLLAQIGDQYADLFLAAKNLSDAILLSDILRVNTEITKAPLSASMIKRYDEHHQDLTLLKALVRQQLPEKYKEIFFDQSKNGYAGYIDGGASQEEFYKFIKPILEKMDGTEELLVKLNREDLLRKQRTFDNGSIPHQIHLGELHAILRRQEDFYPFLKDNREKIEKILTFRIPYYVGPLARGNSRFAWMTRKSEETITPWNFEEVVDKGASAQSFIERMTNFDKNLPNEKVLPKHSLLYEYFTVYNELTKVKYVTEGMRKPAFLSGEQKKAIVDLLFKTNRKVTVKQLKEDYFKKIECFDSVEISGVEDRFNASLGTYHDLLKIIKDKDFLDNEENEDILEDIVLTLTLFEDREMIEERLKTYAHLFDDKVMKQLKRRRYTGWGRLSRKLINGIRDKQSGKTILDFLKSDGFANRNFMQLIHDDSLTFKEDIQKAQVSGQGDSLHEHIANLAGSPAIKKGILQTVKVVDELVKVMGRHKPENIVIEMARENQTTQKGQKNSRERMKRIEEGIKELGSQILKEHPVENTQLQNEKLYLYYLQNGRDMYVDQELDINRLSDYDVDAIVPQSFLKDDSIDNKVLTRSDKNRGKSDNVPSEEVVKKMKNYWRQLLNAKLITQRKFDNLTKAERGGLSELDKAGFIKRQLVETRQITKHVAQILDSRMNTKYDENDKLIREVKVITLKSKLVSDFRKDFQFYKVREINNYHHAHDAYLNAVVGTALIKKYPKLESEFVYGDYKVYDVRKMIAKSEQEIGKATAKYFFYSNIMNFFKTEITLANGEIRKRPLIETNGETGEIVWDKGRDFATVRKVLSMPQVNIVKKTEVQTGGFSKESILPKRNSDKLIARKKDWDPKKYGGFDSPTVAYSVLVVAKVEKGKSKKLKSVKELLGITIMERSSFEKNPIDFLEAKGYKEVKKDLIIKLPKYSLFELENGRKRMLASAGELQKGNELALPSKYVNFLYLASHYEKLKGSPEDNEQKQLFVEQHKHYLDEIIEQISEFSKRVILADANLDKVLSAYNKHRDKPIREQAENIIHLFTLTNLGAPAAFKYFDTTIDRKRYTSTKEVLDATLIHQSITGLYETRIDLSQLGGDGSTPPKKKRKVEDGEGPAAKRVKLDSGAAPAAKKKKLDYKDDDDK

SEQ ID NO: 31 - protein, 1956 aa, Synthetic construct
MTLNIEDEYRLHETSKEPDVSLGSTWLSDFPQAWAETGGMGLAVRQAPLIIPLKATSTPVSIKQYPMSQEARLGIKPHIQRLLDQGILVPCQSPWNTPLLPVKKPGTNDYRPVQDLREVNKRVEDIHPTVPNPYNLLSGLPPSHQWYTVLDLKDAFFCLRLHPTSQPLFAFEWRDPEMGISGQLTWTRLPQGFKNSPTLFNEALHRDLADFRIQHPDLILLQYVDDLLLAATSELDCQQGTRALLQTLGNLGYRASAKKAQICQKQVKYLGYLLKEGQRWLTEARKETVMGQPTPKTPRQLREFLGKAGFCRLFIPGFAEMAAPLYPLTKPGTLFNWGPDQQKAYQEIKQALLTAPALGLPDLTKPFELFVDEKQGYAKGVLTQKLGPWRRPVAYLSKKLDPVAAGWPPCLRMVAAIAVLTKDAGKLTMGQPLVILAPHAVEALVKQPPDRWLSNARMTHYQALLLDTDRVQFGPVVALNPATLLPLPEEGLQHNSGSTPPKKKRKVEDGEGTGGPGSEPATSGSETPGTSESATPESGPGGSGDKKYSIGLDIGTNSVGWAVITDEYKVPSKKFKVLGNTDRHSIKKNLIGALLFDSGETAEATRLKRTARRRYTRRKNRICYLQEIFSNEMAKVDDSFFHRLEESFLVEEDKKHERHPIFGNIVDEVAYHEKYPTIYHLRKKLVDSTDKADLRLIYLALAHMIKFRGHFLIEGDLNPDNSDVDKLFIQLVQTYNQLFEENPINASGVDAKAILSARLSKSRRLENLIAQLPGEKKNGLFGNLIALSLGLTPNFKSNFDLAEDAKLQLSKDTYDDDLDNLLAQIGDQYADLFLAAKNLSDAILLSDILRVNTEITKAPLSASMIKRYDEHHQDLTLLKALVRQQLPEKYKEIFFDQSKNGYAGYIDGGASQEEFYKFIKPILEKMDGTEELLVKLNREDLLRKQRTFDNGSIPHQIHLGELHAILRRQEDFYPFLKDNREKIEKILTFRIPYYVGPLARGNSRFAWMTRKSEETITPWNFEEVVDKGASAQSFIERMTNFDKNLPNEKVLPKHSLLYEYFTVYNELTKVKYVTEGMRKPAFLSGEQKKAIVDLLFKTNRKVTVKQLKEDYFKKIECFDSVEISGVEDRFNASLGTYHDLLKIIKDKDFLDNEENEDILEDIVLTLTLFEDREMIEERLKTYAHLFDDKVMKQLKRRRYTGWGRLSRKLINGIRDKQSGKTILDFLKSDGFANRNFMQLIHDDSLTFKEDIQKAQVSGQGDSLHEHIANLAGSPAIKKGILQTVKVVDELVKVMGRHKPENIVIEMARENQTTQKGQKNSRERMKRIEEGIKELGSQILKEHPVENTQLQNEKLYLYYLQNGRDMYVDQELDINRLSDYDVDAIVPQSFLKDDSIDNKVLTRSDKNRGKSDNVPSEEVVKKMKNYWRQLLNAKLITQRKFDNLTKAERGGLSELDKAGFIKRQLVETRQITKHVAQILDSRMNTKYDENDKLIREVKVITLKSKLVSDFRKDFQFYKVREINNYHHAHDAYLNAVVGTALIKKYPKLESEFVYGDYKVYDVRKMIAKSEQEIGKATAKYFFYSNIMNFFKTEITLANGEIRKRPLIETNGETGEIVWDKGRDFATVRKVLSMPQVNIVKKTEVQTGGFSKESILPKRNSDKLIARKKDWDPKKYGGFDSPTVAYSVLVVAKVEKGKSKKLKSVKELLGITIMERSSFEKNPIDFLEAKGYKEVKKDLIIKLPKYSLFELENGRKRMLASAGELQKGNELALPSKYVNFLYLASHYEKLKGSPEDNEQKQLFVEQHKHYLDEIIEQISEFSKRVILADANLDKVLSAYNKHRDKPIREQAENIIHLFTLTNLGAPAAFKYFDTTIDRKRYTSTKEVLDATLIHQSITGLYETRIDLSQLGGDGSTPPKKKRKVEDGEGPAAKRVKLDSGAAPAAKKKKLDYKDDDDK

SEQ ID NO: 32 - protein, 2206 aa, Synthetic construct
MTLNIEDEYRLHETSKEPDVSLGSTWLSDFPQAWAETGGMGLAVRQAPLIIPLKATSTPVSIKQYPMSQEARLGIKPHIQRLLDQGILVPCQSPWNTPLLPVKKPGTNDYRPVQDLREVNKRVEDIHPTVPNPYNLLSGLPPSHQWYTVLDLKDAFFCLRLHPTSQPLFAFEWRDPEMGISGQLTWTRLPQGFKNSPTLFNEALHRDLADFRIQHPDLILLQYVDDLLLAATSELDCQQGTRALLQTLGNLGYRASAKKAQICQKQVKYLGYLLKEGQRWLTEARKETVMGQPTPKTPRQLREFLGKAGFCRLFIPGFAEMAAPLYPLTKPGTLFNWGPDQQKAYQEIKQALLTAPALGLPDLTKPFELFVDEKQGYAKGVLTQKLGPWRRPVAYLSKKLDPVAAGWPPCLRMVAAIAVLTKDAGKLTMGQPLVILAPHAVEALVKQPPDRWLSNARMTHYQALLLDTDRVQFGPVVALNPATLLPLPEEGLQHNCLDILAEAHGTRPDLTDQPLPDADHTWYTDGSSLLQEGQRKAGAAVTTETEVIWAKALPAGTSAQRAELIALTQALKMAEGKKLNVYTDSRYAFATAHIHGEIYRRRGWLTSEGKEIKNKDEILALLKALFLPKRLSIIHCPGHQKGHSAEARGNRMADQAARKAAITETPDTSTLLIENSSPGSTPPKKKRKVEDGEGTGGPGSEPATSGSETPGTSESATPESGPGGSGDKKYSIGLDIGTNSVGWAVITDEYKVPSKKFKVLGNTDRHSIKKNLIGALLFDSGETAEATRLKRTARRRYTRRKNRICYLQEIFSNEMAKVDDSFFHRLEESFLVEEDKKHERHPIFGNIVDEVAYHEKYPTIYHLRKKLVDSTDKADLRLIYLALAHMIKFRGHFLIEGDLNPDNSDVDKLFIQLVQTYNQLFEENPINASGVDAKAILSARLSKSRRLENLIAQLPGEKKNGLFGNLIALSLGLTPNFKSNFDLAEDAKLQLSKDTYDDDLDNLLAQIGDQYADLFLAAKNLSDAILLSDILRVNTEITKAPLSASMIKRYDEHHQDLTLLKALVRQQLPEKYKEIFFDQSKNGYAGYIDGGASQEEFYKFIKPILEKMDGTEELLVKLNREDLLRKQRTFDNGSIPHQIHLGELHAILRRQEDFYPFLKDNREKIEKILTFRIPYYVGPLARGNSRFAWMTRKSEETITPWNFEEVVDKGASAQSFIERMTNFDKNLPNEKVLPKHSLLYEYFTVYNELTKVKYVTEGMRKPAFLSGEQKKAIVDLLFKTNRKVTVKQLKEDYFKKIECFDSVEISGVEDRFNASLGTYHDLLKIIKDKDFLDNEENEDILEDIVLTLTLFEDREMIEERLKTYAHLFDDKVMKQLKRRRYTGWGRLSRKLINGIRDKQSGKTILDFLKSDGFANRNFMQLIHDDSLTFKEDIQKAQVSGQGDSLHEHIANLAGSPAIKKGILQTVKVVDELVKVMGRHKPENIVIEMARENQTTQKGQKNSRERMKRIEEGIKELGSQILKEHPVENTQLQNEKLYLYYLQNGRDMYVDQELDINRLSDYDVDAIVPQSFLKDDSIDNKVLTRSDKNRGKSDNVPSEEVVKKMKNYWRQLLNAKLITQRKFDNLTKAERGGLSELDKAGFIKRQLVETRQITKHVAQILDSRMNTKYDENDKLIREVKVITLKSKLVSDFRKDFQFYKVREINNYHHAHDAYLNAVVGTALIKKYPKLESEFVYGDYKVYDVRKMIAKSEQEIGKATAKYFFYSNIMNFFKTEITLANGEIRKRPLIETNGETGEIVWDKGRDFATVRKVLSMPQVNIVKKTEVQTGGFSKESILPKRNSDKLIARKKDWDPKKYGGFDSPTVAYSVLVVAKVEKGKSKKLKSVKELLGITIMERSSFEKNPIDFLEAKGYKEVKKDLIIKLPKYSLFELENGRKRMLASAGELQKGNELALPSKYVNFLYLASHYEKLKGSPEDNEQKQLFVEQHKHYLDEIIEQISEFSKRVILADANLDKVLSAYNKHRDKPIREQAENIIHLFTLTNLGAPAAFKYFDTTIDRKRYTSTKEVLDATLIHQSITGLYETRIDLSQLGGDGSTPPKKKRKVEDGEGPAAKRVKLDSGAAPAAKKKKLDYKDDDDKGGSGGATVKFKYKGEEKEVDISKIKKVWRVGKMISFTYDLGGGKTGRGAVSEKDAPKELLQMLEKQKK

SEQ ID NO: 33 - protein, 1629 aa, Synthetic construct
MKRTADGSEFESPKKKRKVSEVEFSHEYWMRHALTLAKRARDEREVPVGAVLVLNNRVIGEGWNRAIGLHDPTAHAEIMALRQGGLVMQNYRLIDATLYVTFEPCVMCAGAMIHSRIGRVVFGVRNSKRGAAGSLMNVLNYPGMNHRVEITEGILADECAALLCDFYRMPRQVFNAQKKAQSSINSGGSSGGSSGSETPGTSESATPESSGGSSGGSDKKYSIGLAIGTNSVGWAVITDEYKVPSKKFKVLGNTDRHSIKKNLIGALLFDSGETAEATRLKRTARRRYTRRKNRICYLQEIFSNEMAKVDDSFFHRLEESFLVEEDKKHERHPIFGNIVDEVAYHEKYPTIYHLRKKLVDSTDKADLRLIYLALAHMIKFRGHFLIEGDLNPDNSDVDKLFIQLVQTYNQLFEENPINASGVDAKAILSARLSKSRRLENLIAQLPGEKKNGLFGNLIALSLGLTPNFKSNFDLAEDAKLQLSKDTYDDDLDNLLAQIGDQYADLFLAAKNLSDAILLSDILRVNTEITKAPLSASMIKRYDEHHQDLTLLKALVRQQLPEKYKEIFFDQSKNGYAGYIDGGASQEEFYKFIKPILEKMDGTEELLVKLNREDLLRKQRTFDNGSIPHQIHLGELHAILRRQEDFYPFLKDNREKIEKILTFRIPYYVGPLARGNSRFAWMTRKSEETITPWNFEEVVDKGASAQSFIERMTNFDKNLPNEKVLPKHSLLYEYFTVYNELTKVKYVTEGMRKPAFLSGEQKKAIVDLLFKTNRKVTVKQLKEDYFKKIECFDSVEISGVEDRFNASLGTYHDLLKIIKDKDFLDNEENEDILEDIVLTLTLFEDREMIEERLKTYAHLFDDKVMKQLKRRRYTGWGRLSRKLINGIRDKQSGKTILDFLKSDGFANRNFMQLIHDDSLTFKEDIQKAQVSGQGDSLHEHIANLAGSPAIKKGILQTVKVVDELVKVMGRHKPENIVIEMARENQTTQKGQKNSRERMKRIEEGIKELGSQILKEHPVENTQLQNEKLYLYYLQNGRDMYVDQELDINRLSDYDVDHIVPQSFLKDDSIDNKVLTRSDKNRGKSDNVPSEEVVKKMKNYWRQLLNAKLITQRKFDNLTKAERGGLSELDKAGFIKRQLVETRQITKHVAQILDSRMNTKYDENDKLIREVKVITLKSKLVSDFRKDFQFYKVREINNYHHAHDAYLNAVVGTALIKKYPKLESEFVYGDYKVYDVRKMIAKSEQEIGKATAKYFFYSNIMNFFKTEITLANGEIRKRPLIETNGETGEIVWDKGRDFATVRKVLSMPQVNIVKKTEVQTGGFSKESILPKRNSDKLIARKKDWDPKKYGGFDSPTVAYSVLVVAKVEKGKSKKLKSVKELLGITIMERSSFEKNPIDFLEAKGYKEVKKDLIIKLPKYSLFELENGRKRMLASAGELQKGNELALPSKYVNFLYLASHYEKLKGSPEDNEQKQLFVEQHKHYLDEIIEQISEFSKRVILADANLDKVLSAYNKHRDKPIREQAENIIHLFTLTNLGAPAAFKYFDTTIDRKRYTSTKEVLDATLIHQSITGLYETRIDLSQLGGDGSTPPKKKRKVEDGEGPAAKRVKLDSGAAPAAKKKKLDYKDDDDK

SEQ ID NO: 34 - protein, 1413 aa, Synthetic construct
MDKKYSIGLDIGTNSVGWAVITDEYKVPSKKFKVLGNTDRHSIKKNLIGALLFDSGETAEATRLKRTARRRYTRRKNRICYLQEIFSNEMAKVDDSFFHRLEESFLVEEDKKHERHPIFGNIVDEVAYHEKYPTIYHLRKKLVDSTDKADLRLIYLALAHMIKFRGHFLIEGDLNPDNSDVDKLFIQLVQTYNQLFEENPINASGVDAKAILSARLSKSRRLENLIAQLPGEKKNGLFGNLIALSLGLTPNFKSNFDLAEDAKLQLSKDTYDDDLDNLLAQIGDQYADLFLAAKNLSDAILLSDILRVNTEITKAPLSASMIKRYDEHHQDLTLLKALVRQQLPEKYKEIFFDQSKNGYAGYIDGGASQEEFYKFIKPILEKMDGTEELLVKLNREDLLRKQRTFDNGSIPHQIHLGELHAILRRQEDFYPFLKDNREKIEKILTFRIPYYVGPLARGNSRFAWMTRKSEETITPWNFEEVVDKGASAQSFIERMTNFDKNLPNEKVLPKHSLLYEYFTVYNELTKVKYVTEGMRKPAFLSGEQKKAIVDLLFKTNRKVTVKQLKEDYFKKIECFDSVEISGVEDRFNASLGTYHDLLKIIKDKDFLDNEENEDILEDIVLTLTLFEDREMIEERLKTYAHLFDDKVMKQLKRRRYTGWGRLSRKLINGIRDKQSGKTILDFLKSDGFANRNFMQLIHDDSLTFKEDIQKAQVSGQGDSLHEHIANLAGSPAIKKGILQTVKVVDELVKVMGRHKPENIVIEMARENQTTQKGQKNSRERMKRIEEGIKELGSQILKEHPVENTQLQNEKLYLYYLQNGRDMYVDQELDINRLSDYDVDHIVPQSFLKDDSIDNKVLTRSDKNRGKSDNVPSEEVVKKMKNYWRQLLNAKLITQRKFDNLTKAERGGLSELDKAGFIKRQLVETRQITKHVAQILDSRMNTKYDENDKLIREVKVITLKSKLVSDFRKDFQFYKVREINNYHHAHDAYLNAVVGTALIKKYPKLESEFVYGDYKVYDVRKMIAKSEQEIGKATAKYFFYSNIMNFFKTEITLANGEIRKRPLIETNGETGEIVWDKGRDFATVRKVLSMPQVNIVKKTEVQTGGFSKESILPKRNSDKLIARKKDWDPKKYGGFDSPTVAYSVLVVAKVEKGKSKKLKSVKELLGITIMERSSFEKNPIDFLEAKGYKEVKKDLIIKLPKYSLFELENGRKRMLASAGELQKGNELALPSKYVNFLYLASHYEKLKGSPEDNEQKQLFVEQHKHYLDEIIEQISEFSKRVILADANLDKVLSAYNKHRDKPIREQAENIIHLFTLTNLGAPAAFKYFDTTIDRKRYTSTKEVLDATLIHQSITGLYETRIDLSQLGGDGSTPPKKKRKVEDGEGPAAKRVKLDSGAAPAAKKKKLDYKDDDDK

SEQ ID NO: 35 - protein, 1401 aa, Synthetic construct
MDKKYSIGLDIGTNSVGWAVITDEYKVPSKKFKVLGNTDRHSIKKNLIGALLFDSGETAEATRLKRTARRRYTRRKNRICYLQEIFSNEMAKVDDSFFHRLEESFLVEEDKKHERHPIFGNIVDEVAYHEKYPTIYHLRKKLVDSTDKADLRLIYLALAHMIKFRGHFLIEGDLNPDNSDVDKLFIQLVQTYNQLFEENPINASGVDAKAILSARLSKSRRLENLIAQLPGEKKNGLFGNLIALSLGLTPNFKSNFDLAEDAKLQLSKDTYDDDLDNLLAQIGDQYADLFLAAKNLSDAILLSDILRVNTEITKAPLSASMIKRYDEHHQDLTLLKALVRQQLPEKYKEIFFDQSKNGYAGYIDGGASQEEFYKFIKPILEKMDGTEELLVKLNREDLLRKQRTFDNGSIPHQIHLGELHAILRRQEDFYPFLKDNREKIEKILTFRIPYYVGPLARGNSRFAWMTRKSEETITPWNFEEVVDKGASAQSFIERMTNFDKNLPNEKVLPKHSLLYEYFTVYNELTKVKYVTEGMRKPAFLSGEQKKAIVDLLFKTNRKVTVKQLKEDYFKKIECFDSVEISGVEDRFNASLGTYHDLLKIIKDKDFLDNEENEDILEDIVLTLTLFEDREMIEERLKTYAHLFDDKVMKQLKRRRYTGWGRLSRKLINGIRDKQSGKTILDFLKSDGFANRNFMQLIHDDSLTFKEDIQKAQVSGQGDSLHEHIANLAGSPAIKKGILQTVKVVDELVKVMGRHKPENIVIEMARENQTTQKGQKNSRERMKRIEEGIKELGSQILKEHPVENTQLQNEKLYLYYLQNGRDMYVDQELDINRLSDYDVDHIVPQSFLKDDSIDNKVLTRSDKARGKSDNVPSEEVVKKMKNYWRQLLNAKLITQRKFDNLTKAERGGLSELDKAGFIKRQLVETRQITKHVAQILDSRMNTKYDENDKLIREVKVITLKSKLVSDFRKDFQFYKVREINNYHHAHDAYLNAVVGTALIKKYPKLESEFVYGDYKVYDVRKMIAKSEQEIGKATAKYFFYSNIMNFFKTEITLANGEIRKRPLIETNGETGEIVWDKGRDFATVRKVLSMPQVNIVKKTEVQTGGFSKESILPKRNSDKLIARKKDWDPKKYGGFDSPTVAYSVLVVAKVEKGKSKKLKSVKELLGITIMERSSFEKNPIDFLEAKGYKEVKKDLIIKLPKYSLFELENGRKRMLASAGELQKGNELALPSKYVNFLYLASHYEKLKGSPEDNEQKQLFVEQHKHYLDEIIEQISEFSKRVILADANLDKVLSAYNKHRDKPIREQAENIIHLFTLTNLGAPAAFKYFDTTIDRKRYTSTKEVLDATLIHQSITGLYETRIDLSQLGGDAYPYDVPDYASLGSGSPKKKRKVEDPKKKRKVD

SEQ ID NO: 36 - protein, 815 aa, Synthetic construct
MVSKGEAVIKEFMRFKVHMEGSMNGHEFEIEGEGEGRPYEGTQTAKLKVTKGGPLPFSWDILSPQFMYGSRAFIKHPADIPDYYKQSFPEGFKWERVMNFEDGGAVTVTQDTSLEDGTLIYKVKLRGTNFPPDGPVMQKKTMGWEASTERLYPEDGVLKGDIKMALRLKDGGRYLADFKTTYKAKKPVQMPGAYNVDRKLDITSHNEDPGASASGSGSGSETPGTSESATPESGSGATNFSLLKQAGDVEENPGPGSADYKDDDDKGSGSETPGTSESATPESGGGGLLEKFVGTWKIADSHNFGEYLKAIGAPKELSDGGDATTPTLYISQKDGDKMSVKIENGPPTFLDTQVKFKLGEEFDEFPSDRRKGVKSVVNLVGEKLVYVQKWDGKETTYVREIKDGKLVVTLTMGDVVAVRSYRRATERQRRYQLFTAQAGRGRRGKSWTSLPLRRARLRWLRQRNTRHQRVCYPRIRWRRPAREVCWNMEDCRQSQFWGVSQGYRSPKRTVRRRRRYNPNSVHLSKGRGQDVCDRKRAANIPGYASQIQTRRRVRVPIRQKKGRQERGQSRGRKTGLRPKVGRERNHIRAGNQGRKARGHTHNGRRRGCAVLQTRYRMTDLALPISAFSSKQATWRKTQGLLESPFQILCWASTAPAVVPKLPEQARAPHQNLAVVDCWRNLSVLGKSPTATTSENTSKLLGHPKSFPTAGTQLLPHCIFPKRMGTKCPSKSRMDRRLFSTHKSSSNWEKSSMNFPATAAKASNLWSTLSGKSSFTFKNGTEKKRPMSAKSKTGSLLLLLRWAMWSPSGLIGEPQS

SEQ ID NO: 37 - protein, 802 aa, Synthetic construct
WFLKARPSKSSGSRCTWKAATATSSRSKAKARADLTRELRPPSKPKAALCLSAGTSCLHSLCTAAGPSSSTPLTSPTTTSSLSQRASSGRETSRTAEPLHRTHLWKMGPSTKSCGAQTSLQTALCRKRQWAGKPAPRDCTLKMACRATSRWPDRTAADTWPTSRPPTRPRNLCRCLAPTTWTESWTSPPTTKTDRALPPPVPAADPRHLAQASLPHQSLEAAPQTSACSNRLATWKRTLDLALPTTRTTTTKALAAKPLAHPKALHQKAEAADCWKSSSAPGRSPTLTTSASTSRPSALQKSCQTEATPPHLHCTSARKTATKCPSRSRTALLPSWTPKSSSSWARSSTSFQATDGRESSPWSTSWERSWCTCRSGTAKRQPTSERSRTASWWSPSLWATWWPCGATEGPQSEGSGATNFSLLKQAGDVEENPGPAYPYDVPDYAGSGSETPGTSESATPESGGGGLLEKFVGTWKIADSHNFGEYLKAIGAPKELSDGGDATTPTLYISQKDGDKMSVKIENGPPTFLDTQVKFKLGEEFDEFPSDRRKGVKSVVNLVGEKLVYVQKWDGKETTYVREIKDGKLVVTLTMGDVVAVRSYRRATERIWRYQFQPSQASRRRGGKPRACWKAHSKSSAGPRQHRQWFRNSRNKRERHTRIWRWWTAGEICRYLENRRQPQLRRIPQSYWGTQRAFRRRGRNYSHTVYFPKGWGQNVRQNREWTADFSRHTSQVQIGRRVRISQRPPQRRQICGQPCRGKARLRSKMGRKRNDLCPRNQRREACCYSYDGRCGRRQVLSESHRV

SEQ ID NO: 38 - protein, 815 aa, Synthetic construct
GFRRGRDQRVHEVQGAHGRQHERPRVRDRRRRRGQTLRGNSDRQAESDQRRPSAFQLGHPVSTVYVRQQGLHQAPRHPRLLQAVFPRGLQVGESDELRGRRSRDCDTGHISGRWDPDLQSEAAGHKLPSRRPCDAEKDNGLGSQHRETVPRWRAEGRHQDGPETEGRRQIPGRLQDHLQGQETCADAWRLQRGQKAGHHLPQRRLTGRFRLRFRQRIRDTWHKRVCHTRVWKRRHKLQPAQTGWRRGREPWTWLCRLQGRRRQRLWQRNPWHIRKRYTRKRRRRTAGKVRRHLEDRRLSQLRRVPQGHRRSKRVVRRRRRHHTYTVHQPERRRQNVRQDRERPSYLPGHPSQVQAGRGVRRVSKRQTEGSQVRGQPRGREAGVRAEVGRQRDNLRQRDQGRQAGGHPHYGRRGGRAELQKGHRVKAAALPTFHCSSRPGTSRKILDQLTPTTCQITLAPAAKHQAPASLLPQNQVAEACSRSLLEHGRLPTVTILGSISRLSEPQKNCPTAATLQPQLCTSLKRTGTRCLLRSKTGRQHSWIRKSNSNSAKSLTSSHPTEERASRAWSISWAKNWSTSKSGTGKKPHTCGKSRTESSWSHSQWATSWLCGLTDALPNDGSGATNFSLLKQAGDVEENPGPAGKPIPNPLLGLDSTGSGSETPGTSESATPESGGGGLLEKFVGTWKIADSHNFGEYLKAIGAPKELSDGGDATTPTLYISQKDGDKMSVKIENGPPTFLDTQVKFKLGEEFDEFPSDRRKGVKSVVNLVGEKLVYVQKWDGKETTYVREIKDGKLVVTLTMGDVVAVRSYRRATE

SEQ ID NO: 39 - protein, 1367 aa, Synthetic construct
DKKYSIGLDIGTNSVGWAVITDEYKVPSKKFKVLGNTDRHSIKKNLIGALLFDSGETAEATRLKRTARRRYTRRKNRICYLQEIFSNEMAKVDDSFFHRLEESFLVEEDKKHERHPIFGNIVDEVAYHEKYPTIYHLRKKLVDSTDKADLRLIYLALAHMIKFRGHFLIEGDLNPDNSDVDKLFIQLVQTYNQLFEENPINASGVDAKAILSARLSKSRRLENLIAQLPGEKKNGLFGNLIALSLGLTPNFKSNFDLAEDAKLQLSKDTYDDDLDNLLAQIGDQYADLFLAAKNLSDAILLSDILRVNTEITKAPLSASMIKRYDEHHQDLTLLKALVRQQLPEKYKEIFFDQSKNGYAGYIDGGASQEEFYKFIKPILEKMDGTEELLVKLNREDLLRKQRTFDNGSIPHQIHLGELHAILRRQEDFYPFLKDNREKIEKILTFRIPYYVGPLARGNSRFAWMTRKSEETITPWNFEEVVDKGASAQSFIERMTNFDKNLPNEKVLPKHSLLYEYFTVYNELTKVKYVTEGMRKPAFLSGEQKKAIVDLLFKTNRKVTVKQLKEDYFKKIECFDSVEISGVEDRFNASLGTYHDLLKIIKDKDFLDNEENEDILEDIVLTLTLFEDREMIEERLKTYAHLFDDKVMKQLKRRRYTGWGRLSRKLINGIRDKQSGKTILDFLKSDGFANRNFMQLIHDDSLTFKEDIQKAQVSGQGDSLHEHIANLAGSPAIKKGILQTVKVVDELVKVMGRHKPENIVIEMARENQTTQKGQKNSRERMKRIEEGIKELGSQILKEHPVENTQLQNEKLYLYYLQNGRDMYVDQELDINRLSDYDVDHIVPQSFLKDDSIDNKVLTRSDKNRGKSDNVPSEEVVKKMKNYWRQLLNAKLITQRKFDNLTKAERGGLSELDKAGFIKRQLVETRQITKHVAQILDSRMNTKYDENDKLIREVKVITLKSKLVSDFRKDFQFYKVREINNYHHAHDAYLNAVVGTALIKKYPKLESEFVYGDYKVYDVRKMIAKSEQEIGKATAKYFFYSNIMNFFKTEITLANGEIRKRPLIETNGETGEIVWDKGRDFATVRKVLSMPQVNIVKKTEVQTGGFSKESILPKRNSDKLIARKKDWDPKKYGGFDSPTVAYSVLVVAKVEKGKSKKLKSVKELLGITIMERSSFEKNPIDFLEAKGYKEVKKDLIIKLPKYSLFELENGRKRMLASAGELQKGNELALPSKYVNFLYLASHYEKLKGSPEDNEQKQLFVEQHKHYLDEIIEQISEFSKRVILADANLDKVLSAYNKHRDKPIREQAENIIHLFTLTNLGAPAAFKYFDTTIDRKRYTSTKEVLDATLIHQSITGLYETRIDLSQLGGD

SEQ ID NO: 40 - protein, 1367 aa, Synthetic construct
DKKYSIGLDIGTNSVGWAVITDEYKVPSKKFKVLGNTDRHSIKKNLIGALLFDSGETAEATRLKRTARRRYTRRKNRICYLQEIFSNEMAKVDDSFFHRLEESFLVEEDKKHERHPIFGNIVDEVAYHEKYPTIYHLRKKLVDSTDKADLRLIYLALAHMIKFRGHFLIEGDLNPDNSDVDKLFIQLVQTYNQLFEENPINASGVDAKAILSARLSKSRRLENLIAQLPGEKKNGLFGNLIALSLGLTPNFKSNFDLAEDAKLQLSKDTYDDDLDNLLAQIGDQYADLFLAAKNLSDAILLSDILRVNTEITKAPLSASMIKRYDEHHQDLTLLKALVRQQLPEKYKEIFFDQSKNGYAGYIDGGASQEEFYKFIKPILEKMDGTEELLVKLNREDLLRKQRTFDNGSIPHQIHLGELHAILRRQEDFYPFLKDNREKIEKILTFRIPYYVGPLARGNSRFAWMTRKSEETITPWNFEEVVDKGASAQSFIERMTNFDKNLPNEKVLPKHSLLYEYFTVYNELTKVKYVTEGMRKPAFLSGEQKKAIVDLLFKTNRKVTVKQLKEDYFKKIECFDSVEISGVEDRFNASLGTYHDLLKIIKDKDFLDNEENEDILEDIVLTLTLFEDREMIEERLKTYAHLFDDKVMKQLKRRRYTGWGRLSRKLINGIRDKQSGKTILDFLKSDGFANRNFMQLIHDDSLTFKEDIQKAQVSGQGDSLHEHIANLAGSPAIKKGILQTVKVVDELVKVMGRHKPENIVIEMARENQTTQKGQKNSRERMKRIEEGIKELGSQILKEHPVENTQLQNEKLYLYYLQNGRDMYVDQELDINRLSDYDVDAIVPQSFLKDDSIDNKVLTRSDKNRGKSDNVPSEEVVKKMKNYWRQLLNAKLITQRKFDNLTKAERGGLSELDKAGFIKRQLVETRQITKHVAQILDSRMNTKYDENDKLIREVKVITLKSKLVSDFRKDFQFYKVREINNYHHAHDAYLNAVVGTALIKKYPKLESEFVYGDYKVYDVRKMIAKSEQEIGKATAKYFFYSNIMNFFKTEITLANGEIRKRPLIETNGETGEIVWDKGRDFATVRKVLSMPQVNIVKKTEVQTGGFSKESILPKRNSDKLIARKKDWDPKKYGGFDSPTVAYSVLVVAKVEKGKSKKLKSVKELLGITIMERSSFEKNPIDFLEAKGYKEVKKDLIIKLPKYSLFELENGRKRMLASAGELQKGNELALPSKYVNFLYLASHYEKLKGSPEDNEQKQLFVEQHKHYLDEIIEQISEFSKRVILADANLDKVLSAYNKHRDKPIREQAENIIHLFTLTNLGAPAAFKYFDTTIDRKRYTSTKEVLDATLIHQSITGLYETRIDLSQLGGD

SEQ ID NO: 41 - protein, 1367 aa, Synthetic construct
DKKYSIGLDIGTNSVGWAVITDEYKVPSKKFKVLGNTDRHSIKKNLIGALLFDSGETAEATRLKRTARRRYTRRKNRICYLQEIFSNEMAKVDDSFFHRLEESFLVEEDKKHERHPIFGNIVDEVAYHEKYPTIYHLRKKLVDSTDKADLRLIYLALAHMIKFRGHFLIEGDLNPDNSDVDKLFIQLVQTYNQLFEENPINASGVDAKAILSARLSKSRRLENLIAQLPGEKKNGLFGNLIALSLGLTPNFKSNFDLAEDAKLQLSKDTYDDDLDNLLAQIGDQYADLFLAAKNLSDAILLSDILRVNTEITKAPLSASMIKRYDEHHQDLTLLKALVRQQLPEKYKEIFFDQSKNGYAGYIDGGASQEEFYKFIKPILEKMDGTEELLVKLNREDLLRKQRTFDNGSIPHQIHLGELHAILRRQEDFYPFLKDNREKIEKILTFRIPYYVGPLARGNSRFAWMTRKSEETITPWNFEEVVDKGASAQSFIERMTNFDKNLPNEKVLPKHSLLYEYFTVYNELTKVKYVTEGMRKPAFLSGEQKKAIVDLLFKTNRKVTVKQLKEDYFKKIECFDSVEISGVEDRFNASLGTYHDLLKIIKDKDFLDNEENEDILEDIVLTLTLFEDREMIEERLKTYAHLFDDKVMKQLKRRRYTGWGRLSRKLINGIRDKQSGKTILDFLKSDGFANRNFMQLIHDDSLTFKEDIQKAQVSGQGDSLHEHIANLAGSPAIKKGILQTVKVVDELVKVMGRHKPENIVIEMARENQTTQKGQKNSRERMKRIEEGIKELGSQILKEHPVENTQLQNEKLYLYYLQNGRDMYVDQELDINRLSDYDVDHIVPQSFLKDDSIDNKVLTRSDKARGKSDNVPSEEVVKKMKNYWRQLLNAKLITQRKFDNLTKAERGGLSELDKAGFIKRQLVETRQITKHVAQILDSRMNTKYDENDKLIREVKVITLKSKLVSDFRKDFQFYKVREINNYHHAHDAYLNAVVGTALIKKYPKLESEFVYGDYKVYDVRKMIAKSEQEIGKATAKYFFYSNIMNFFKTEITLANGEIRKRPLIETNGETGEIVWDKGRDFATVRKVLSMPQVNIVKKTEVQTGGFSKESILPKRNSDKLIARKKDWDPKKYGGFDSPTVAYSVLVVAKVEKGKSKKLKSVKELLGITIMERSSFEKNPIDFLEAKGYKEVKKDLIIKLPKYSLFELENGRKRMLASAGELQKGNELALPSKYVNFLYLASHYEKLKGSPEDNEQKQLFVEQHKHYLDEIIEQISEFSKRVILADANLDKVLSAYNKHRDKPIREQAENIIHLFTLTNLGAPAAFKYFDTTIDRKRYTSTKEVLDATLIHQSITGLYETRIDLSQLGGD

SEQ ID NO: 42 - protein, 1367 aa, Synthetic construct
DKKYSIGLDIGTNSVGWAVITDEYKVPSKKFKVLGNTDRHSIKKNLIGALLFDSGETAEATRLKRTARRRYTRRKNRICYLQEIFSNEMAKVDDSFFHRLEESFLVEEDKKHERHPIFGNIVDEVAYHEKYPTIYHLRKKLVDSTDKADLRLIYLALAHMIKFRGHFLIEGDLNPDNSDVDKLFIQLVQTYNQLFEENPINASGVDAKAILSARLSKSRRLENLIAQLPGEKKNGLFGNLIALSLGLTPNFKSNFDLAEDAKLQLSKDTYDDDLDNLLAQIGDQYADLFLAAKNLSDAILLSDILRVNTEITKAPLSASMIKRYDEHHQDLTLLKALVRQQLPEKYKEIFFDQSKNGYAGYIDGGASQEEFYKFIKPILEKMDGTEELLVKLNREDLLRKQRTFDNGSIPHQIHLGELHAILRRQEDFYPFLKDNREKIEKILTFRIPYYVGPLARGNSRFAWMTRKSEETITPWNFEEVVDKGASAQSFIERMTNFDKNLPNEKVLPKHSLLYEYFTVYNELTKVKYVTEGMRKPAFLSGEQKKAIVDLLFKTNRKVTVKQLKEDYFKKIECFDSVEISGVEDRFNASLGTYHDLLKIIKDKDFLDNEENEDILEDIVLTLTLFEDREMIEERLKTYAHLFDDKVMKQLKRRRYTGWGRLSRKLINGIRDKQSGKTILDFLKSDGFANRNFMQLIHDDSLTFKEDIQKAQVSGQGDSLHEHIANLAGSPAIKKGILQTVKVVDELVKVMGRHKPENIVIEMARENQTTQKGQKNSRERMKRIEEGIKELGSQILKEHPVENTQLQNEKLYLYYLQNGRDMYVDQELDINRLSDYDVDAIVPQSFLKDDSIDNKVLTRSDKARGKSDNVPSEEVVKKMKNYWRQLLNAKLITQRKFDNLTKAERGGLSELDKAGFIKRQLVETRQITKHVAQILDSRMNTKYDENDKLIREVKVITLKSKLVSDFRKDFQFYKVREINNYHHAHDAYLNAVVGTALIKKYPKLESEFVYGDYKVYDVRKMIAKSEQEIGKATAKYFFYSNIMNFFKTEITLANGEIRKRPLIETNGETGEIVWDKGRDFATVRKVLSMPQVNIVKKTEVQTGGFSKESILPKRNSDKLIARKKDWDPKKYGGFDSPTVAYSVLVVAKVEKGKSKKLKSVKELLGITIMERSSFEKNPIDFLEAKGYKEVKKDLIIKLPKYSLFELENGRKRMLASAGELQKGNELALPSKYVNFLYLASHYEKLKGSPEDNEQKQLFVEQHKHYLDEIIEQISEFSKRVILADANLDKVLSAYNKHRDKPIREQAENIIHLFTLTNLGAPAAFKYFDTTIDRKRYTSTKEVLDATLIHQSITGLYETRIDLSQLGGD

SEQ ID NO: 43 - protein, 63 aa, Synthetic construct
ATVKFKYKGEEKEVDISKIKKVWRVGKMISFTYDEGGGKTGRGAVSEKDAPKELLQMLEKQKK

SEQ ID NO: 44 - protein, 63 aa, Synthetic construct
ATVKFKYKGEEKEVDISKIKKVWRVGKMISFTYDLGGGKTGRGAVSEKDAPKELLQMLEKQKK

SEQ ID NO: 45 - protein, 677 aa, Synthetic construct
TLNIEDEYRLHETSKEPDVSLGSTWLSDFPQAWAETGGMGLAVRQAPLIIPLKATSTPVSIKQYPMSQEARLGIKPHIQRLLDQGILVPCQSPWNTPLLPVKKPGTNDYRPVQDLREVNKRVEDIHPTVPNPYNLLSGLPPSHQWYTVLDLKDAFFCLRLHPTSQPLFAFEWRDPEMGISGQLTWTRLPQGFKNSPTLFNEALHRDLADFRIQHPDLILLQYVDDLLLAATSELDCQQGTRALLQTLGNLGYRASAKKAQICQKQVKYLGYLLKEGQRWLTEARKETVMGQPTPKTPRQLREFLGKAGFCRLFIPGFAEMAAPLYPLTKPGTLFNWGPDQQKAYQEIKQALLTAPALGLPDLTKPFELFVDEKQGYAKGVLTQKLGPWRRPVAYLSKKLDPVAAGWPPCLRMVAAIAVLTKDAGKLTMGQPLVILAPHAVEALVKQPPDRWLSNARMTHYQALLLDTDRVQFGPVVALNPATLLPLPEEGLQHNCLDILAEAHGTRPDLTDQPLPDADHTWYTDGSSLLQEGQRKAGAAVTTETEVIWAKALPAGTSAQRAELIALTQALKMAEGKKLNVYTDSRYAFATAHIHGEIYRRRGWLTSEGKEIKNKDEILALLKALFLPKRLSIIHCPGHQKGHSAEARGNRMADQAARKAAITETPDTSTLLIENSSP

SEQ ID NO: 46 - protein, 495 aa, Synthetic construct
TLNIEDEYRLHETSKEPDVSLGSTWLSDFPQAWAETGGMGLAVRQAPLIIPLKATSTPVSIKQYPMSQEARLGIKPHIQRLLDQGILVPCQSPWNTPLLPVKKPGTNDYRPVQDLREVNKRVEDIHPTVPNPYNLLSGLPPSHQWYTVLDLKDAFFCLRLHPTSQPLFAFEWRDPEMGISGQLTWTRLPQGFKNSPTLFNEALHRDLADFRIQHPDLILLQYVDDLLLAATSELDCQQGTRALLQTLGNLGYRASAKKAQICQKQVKYLGYLLKEGQRWLTEARKETVMGQPTPKTPRQLREFLGKAGFCRLFIPGFAEMAAPLYPLTKPGTLFNWGPDQQKAYQEIKQALLTAPALGLPDLTKPFELFVDEKQGYAKGVLTQKLGPWRRPVAYLSKKLDPVAAGWPPCLRMVAAIAVLTKDAGKLTMGQPLVILAPHAVEALVKQPPDRWLSNARMTHYQALLLDTDRVQFGPVVALNPATLLPLPEEGLQHNS

SEQ ID NO: 47 - protein, 426 aa, Synthetic construct
DTSNLMEQILSSDNLNRAYLQVVRNKGAEGVDGMKYTELKEHLAKNGETIKGQLRTRKYKPQPARRVEIPKPDGGVRNLGVPTVTDRFIQQAIAQVLTPIYEEQFHDHSYGFRPNRCAQQAILTALNIMNDGNDWIVDIDLEKFFDTVNHDKLMTLIGRTIKDGDVISIVRKYLVSGIMIDDEYEDSIVGTPQGGNLSPLLANIMLNELDKEMEKRGLNFVRYADDCIIMVGSEMSANRVMRNISRFIEEKLGLKVNMTKSKVDRPSGLKYLGFGFYFDPRAHQFKAKPHAKSVAKFKKRMKELTCRSWGVSNSYKVEKLNQLIRGWINYFKIGSMKTLCKELDSRIRYRLRMCIWKQWKTPQNQEKNLVKLGIDRNTARRVAYTGKRIAYVCNKGAVNVAISNKRLASFGLISMLDYYIEKCVTC

SEQ ID NO: 48 - protein, 22 aa, Synthetic construct
PPKKKRKVEDGEGPAAKRVKLD

SEQ ID NO: 49 - protein, 35 aa, Synthetic construct
PPKKKRKVEDGEGPAAKRVKLDSGAAPAAKKKKLD

SEQ ID NO: 50 - protein, 9 aa, Synthetic construct
PAAKKKKLD

SEQ ID NO: 51 - protein, 7 aa, Synthetic construct
PKKKRKV

SEQ ID NO: 52 - protein, 9 aa, Synthetic construct
PAAKRVKLD

SEQ ID NO: 53 - protein, 9 aa, Synthetic construct
PAAKKKKLD

SEQ ID NO: 54 - protein, 9 aa, Synthetic construct
PAAKKKKNG

SEQ ID NO: 55 - protein, 27 aa, Synthetic construct
GPGSEPATSGSETPGTSESATPESGPG

SEQ ID NO: 56 - protein, 121 aa, Synthetic construct
SKTIVLSVGEATRTLTEIQSTADRQIFEEKVGPLVGRLRLTASLRQNGAKTAYRVNLKLDQADVVDSGLPKVRYTQVWSHDVTIVANSTEASRKSLYDLTKSLVATSQVEDLVVNLVPLGR

SEQ ID NO: 57 - protein, 247 aa, Synthetic construct
SKTIVLSVGEATRTLTEIQSTADRQIFEEKVGPLVGRLRLTASLRQNGAKTAYRVNLKLDQADVVDSGLPKVRYTQVWSHDVTIVANSTEASRKSLYDLTKSLVATSQVEDLVVNLVPLGRGGSGGSKTIVLSVGEATRTLTEIQSTADRQIFEEKVGPLVGRLRLTASLRQNGAKTAYRVNLKLDQADVVDSGLPKVRYTQVWSHDVTIVANSTEASRKSLYDLTKSLVATSQVEDLVVNLVPLGR

SEQ ID NO: 58 - protein, 129 aa, Synthetic construct
ASNFTQFVLVDNGGTGDVTVAPSNFANGVAEWISSNSRSQAYKVTCSVRQSSAQKRKYTIKVEVPKVATQTVGGEELPVAGWRSYLNMELTIPIFATNSDCELIVKAMQGLLKDGNPIPSAIAANSGIY

SEQ ID NO: 59 - protein, 8 aa, Synthetic construct
DYKDDDDK

SEQ ID NO: 60 - protein, 500 aa, Synthetic construct
MGARASVLSGGELDRWEKIRLRPGGKKKYKLKHIVWASRELERFAVNPGLLETSEGCRQILGQLQPSLQTGSEELRSLYNTVATLYCVHQRIEIKDTKEALDKIEEEQNKSKKKAQQAAADTGHSNQVSQNYPIVQNIQGQMVHQAISPRTLNAWVKVVEEKAFSPEVIPMFSALSEGATPQDLNTMLNTVGGHQAAMQMLKETINEEAAEWDRVHPVHAGPIAPGQMREPRGSDIAGTTSTLQEQIGWMTNNPPIPVGEIYKRWIILGLNKIVRMYSPTSILDIRQGPKEPFRDYVDRFYKTLRAEQASQEVKNWMTETLLVQNANPDCKTILKALGPAATLEEMMTACQGVGGPGHKARVLAEAMSQVTNSATIMMQRGNFRNQRKIVKCFNCGKEGHTARNCRAPRKKGCWKCGKEGHQMKDCTERQANFLGKIWPSYKGRPGNFLQSRPEPTAPPEESFRSGVETTTPPQKQEPIDKELYPLTSLRSLFGNDPSSQ

SEQ ID NO: 61 - protein, 500 aa, Synthetic construct
MGARASVLSGGELDRWEKIRSRPGGKKKYKLKHIVWASRELERFAVNPGLLETSEGCRQILGQLQPSLQTGSEELRSLYNTVATLYCVHQRIEIKDTKEALDKIEEEQNKSKKKAQQAAADTGHSNQVSQNYPIVQNIQGQMVHQAISPRTLNAWVKVVEEKAFSPEVIPMFSALSEGATPQDLNTMLNTVGGHQAAMQMLKETINEEAAEWDRVHPVHAGPIAPGQMREPRGSDIAGTTSTLQEQIGWMTNNPPIPVGEIYKRWIILGLNKIVRMYSPTSILDIRQGPKEPFRDYVDRFYKTLRAEQASQEVKNWMTETLLVQNANPDCKTILKALGPAATLEEMMTACQGVGGPGHKARVLAEAMSQVTNSATIMMQRGNFRNQRKIVKCFNCGKEGHTARNCRAPRKKGCWKCGKEGHQMKDCTERQANFLGKIWPSYKGRPGNFLQSRPEPTAPPEESFRSGVETTTPPQKQEPIDKELYPLTSLRSLFGNDPSSQ

SEQ ID NO: 62 - protein, 186 aa, Synthetic construct
MQRGNFRNQRKIVKSFNSGKEGHTARNSRAPRKKGGSGGVSGWRLFKKISGGASSKTIVLSVGEATRTLTEIQSTADRQIFEEKVGPLVGRLRLTASLRQNGAKTAYRVNLKLDQADVVDSGLPKVRYTQVWSHDVTIVANSTEASRKSLYDLTKSLVATSQVEDLVVNLVPLGRGGSGGTERQAN

SEQ ID NO: 63 - protein, 201 aa, Synthetic construct
MQRGNFRNQRKIVKCFNCGKEGHTARNCRAPRKKGCWKCGKEGHQMKDCGGSGGVSGWRLFKKISGGASSKTIVLSVGEATRTLTEIQSTADRQIFEEKVGPLVGRLRLTASLRQNGAKTAYRVNLKLDQADVVDSGLPKVRYTQVWSHDVTIVANSTEASRKSLYDLTKSLVATSQVEDLVVNLVPLGRGGSGGTERQAN

SEQ ID NO: 64 - protein, 187 aa, Synthetic construct
MDHYLDIRLRPDPEFPPAQLMSVLFGKLHQALVAQGGDRIGVSFPDLDESRSRLGERLRIHASADDLRALLARPWLEGLRDHLQFGEPAVVPHPTPYRQVSRVQAKSNPERLRRRLMRRHDLSEEEARKRIPDTVARALDLPFVTLRSQSTGQHFRLFIRHGPLQVTAEEGGFTCYGLSKGGFVPWF

SEQ ID NO: 65 - protein, 11 aa, Synthetic construct
LQLPPLERLTL

SEQ ID NO: 66 - protein, 123 aa, Synthetic construct
QVQLVESGGGLVQAGGSLRLSCAASGYFSSYAMGWFRQAPGKEREFVAAISWIESTTDYADSVKGRFTISRDNAKKTLHLQMNSLKPEDTAVYYCAACDIPFGQAFCALYDYWGQGTQVTVSS

SEQ ID NO: 67 - protein, 11 aa, Synthetic construct
VSGWRLFKKIS

SEQ ID NO: 68 - protein, 132 aa, Synthetic construct
HGLQDDPDLQALLKGSQLLKVKSSSWRRERFYKLQEDCKTIWQESRKVMRSPESQLFSIEDIQEVRMGHRTEGLEKFARDIPEDRCFSIVFKDQRNTLDLIAPSPADAQHWVQGLRKIIHHSGSMDQRQKLQ

SEQ ID NO: 69 - protein, 33 aa, Synthetic construct
RMKQLEDKVEELLSKNYHLENEVARLKKLVGER

SEQ ID NO: 70 - protein, 33 aa, Synthetic construct
RMKQIEDKIEEILSKIYHIENEIARIKKLIGER

SEQ ID NO: 71 - protein, 238 aa, Synthetic construct
VSKGEELFTGVVPILVELDGDVNGHKFSVRGEGEGDATNGKLTLKFICTTGKLPVPWPTLVTTLGYGVACFARYPDHMKQHDFFKSAMPEGYVQERTISFKDDGTYKTRAEVKFEGDTLVNRIVLKGIDFKEDGNILGHKLEYNFNSHKVYITADKQKNGIKANFKTRHNVEDGGVQLADHYQQNTPIGDGPVLLPDNHYLSHQSKLSKDPNEKRDHMVLKERVTAAGITHDMDELYK

SEQ ID NO: 72 - protein, 232 aa, Synthetic construct
MVSKGEAVIKEFMRFKVHMEGSMNGHEFEIEGEGEGRPYEGTQTAKLKVTKGGPLPFSWDILSPQFMYGSRAFIKHPADIPDYYKQSFPEGFKWERVMNFEDGGAVTVTQDTSLEDGTLIYKVKLRGTNFPPDGPVMQKKTMGWEASTERLYPEDGVLKGDIKMALRLKDGGRYLADFKTTYKAKKPVQMPGAYNVDRKLDITSHNEDYTVVEQYERSEGRHSTGGMDELYK

SEQ ID NO: 73 - protein, 129 aa, Synthetic construct
MGARASVLSGGAQQAAADTGHSNQVSQNYSPTSILDIRQGPKEPFRDYVDRFYKTLRAEQASQEVKNWMTETLLVQNANPDCKTILKALGPAATLEEMMTACQGVGGPGHKARVLAEAMSQVTNSATIM

SEQ ID NO: 74 - protein, 245 aa, Synthetic construct
PIVQNIQGQMVHQAISPRTLNAWVKVVEEKAFSPEVIPMFSALSEGATPQDLNTMLNTVGGHQAAMQMLKETINEEAAEWDRVHPVHAGPIAPGQMREPRGSDIAGTTSTLQEQIGWMTNNPPIPVGEIYKRWIILGLNKIVRMYSPTSILDIRQGPKEPFRDYVDRFYKTLRAEQASQEVKNWMTETLLVQNANPDCKTILKALGPAATLEEMMTACQGVGGPGHKARVLAEAMSQVTNSATIM

SEQ ID NO: 75 - protein, 52 aa, Synthetic construct
LQSRPEPTAPPEESFRSGVETTTPPQKQEPIDKELYPLTSLRSLFGNDPSSQ

SEQ ID NO: 76 - protein, 343 aa, Synthetic construct
MSNLLTVHQNLPALPVDATSDEVRKNLMDMFRDRQAFSEHTWKMLLSVCRSWAAWCKLNNRKWFPAEPEDVRDYLLYLQARGLAVKTIQQHLGQLNMLHRRSGLPRPSDSNAVSLVMRRIRKENVDAGERAKQALAFERTDFDQVRSLMENSDRCQDIRNLAFLGIAYNTLLRIAEIARIRVKDISRTDGGRMLIHIGRTKTLVSTAGVEKALSLGVTKLVERWISVSGVADDPNNYLFCRVRKNGVAAPSATSQLSTRALEGIFEATHRLIYGAKDDSGQRYLAWSGHSARVGAARDMARAGVSIPEIMQAGGWTNVNIVMNYIRNLDSETGAMVRLLEDGD

SEQ ID NO: 77 - protein, 121 aa, Synthetic construct; identical to SEQ ID NO: 56

SEQ ID NO: 78 - protein, 247 aa, Synthetic construct; identical to SEQ ID NO: 57

SEQ ID NO: 79 - protein, 247 aa, Synthetic construct; identical to SEQ ID NO: 57

SEQ ID NO: 80 - protein, 665 aa, Synthetic construct
MARSTLSKPLKNKVNPRGPLIPLILLMLRGVSTASPGSSPHQVYNITWEVTNGDRETVWATSGNHPLWTWWPDLTPDLCMLAHHGPSYWGLEYQSPFSSPPGPPCCSGGSSPGCSRDCEEPLTSLTPRCNTAWNRLKLDQTTHKSNEGFYVCPGPHRPRESKSCGGPDSFYCAYWGCETTGRAYWKPSSSWDFITVNNNLTSDQAVQVCKDNKWCNPLVIRFTDAGRRVTSWTTGHYWGLRLYVSGQDPGLTFGIRLRYQNLGPRVPIGPNPVLADQQPLSKPKPVKSPSVTKPPSGTPLSPTQLPPAGTENRLLNLVDGAYQALNLTSPDKTQECWLCLVAGPPYYEGVAVLGTYSNHTSAPANCSVASQHKLTLSEVTGQGLCIGAVPKTHQALCNTTQTSSRGSYYLVAPTGTMWACSTGLTPCISTTILNLTTDYCVLVELWPRVTYHSPSYVYGLFERSNRHKREPVSLTLALLLGGLTMGGIAAGIGTGTTALMATQQFQQLQAAVQDDLREVEKSISNLEKSLTSLSEVVLQNRRGLDLLFLKEGGLCAALKEECCFYADHTGLVRDSMAKLRERLNQRQKLFESTQGWFEGLFNRSPWFTTLISTIMGPLIVLLMILLFGPCILNRLVQFVKDRISVVQALVLTQQYHQLKPIEYEP

SEQ ID NO: 81 - protein, 649 aa, Synthetic construct
MARSTLSKPLKNKVNPRGPLIPLILLMLRGVSTASPGSSPHQVYNITWEVTNGDRETVWATSGNHPLWTWWPDLTPDLCMLAHHGPSYWGLEYQSPFSSPPGPPCCSGGSSPGCSRDCEEPLTSLTPRCNTAWNRLKLDQTTHKSNEGFYVCPGPHRPRESKSCGGPDSFYCAYWGCETTGRAYWKPSSSWDFITVNNNLTSDQAVQVCKDNKWCNPLVIRFTDAGRRVTSWTTGHYWGLRLYVSGQDPGLTFGIRLRYQNLGPRVPIGPNPVLADQQPLSKPKPVKSPSVTKPPSGTPLSPTQLPPAGTENRLLNLVDGAYQALNLTSPDKTQECWLCLVAGPPYYEGVAVLGTYSNHTSAPANCSVASQHKLTLSEVTGQGLCIGAVPKTHQALCNTTQTSSRGSYYLVAPTGTMWACSTGLTPCISTTILNLTTDYCVLVELWPRVTYHSPSYVYGLFERSNRHKREPVSLTLALLLGGLTMGGIAAGIGTGTTALMATQQFQQLQAAVQDDLREVEKSISNLEKSLTSLSEVVLQNRRGLDLLFLKEGGLCAALKEECCFYADHTGLVRDSMAKLRERLNQRQKLFESTQGWFEGLFNRSPWFTTLISTIMGPLIVLLMILLFGPCILNRLVQFVKDRISVVQAL

SEQ ID NO: 82 - DNA, 2031 bp, Synthetic construct
  source 1..2031: mol_type = other DNA
atgggcgctagagcctctgttctgtctggcggcgaactggacagatgggagaagatcagaagcagacctggcggcaagaagaagtacaagctgaagcacatcgtgtgggccagcagagagctggaaagattcgctgtgaaccccggcctgctggaaacaagcgagggctgtagacagatcctgggccagctccagccatctctccagacaggatctgaggaactgagaagcctgtacaacaccgtggccacactgtactgcgtgcaccagagaatcgagatcaaggacaccaaagaggccctggacaagatcgaggaagaacagaacaagtctaagaagaaggcccagcaggctgccgccgatacaggccactctaatcaggtgtcccagaactaccccatcgtgcagaacatccagggccagatggtgcatcaggctatcagccccagaacactgaacgcctgggtcaaagtggtggaagagaaggctttcagccctgaagtgatccccatgttcagcgccctgtctgagggtgccacacctcaggacctgaacaccatgctgaacacagtcggcggacaccaggccgctatgcagatgctgaaagagacaatcaacgaagaggccgccgagtgggacagagtgcatcctgttcatgctggccctatcgctcccggccagatgagagaacctagaggctctgacattgccggcaccaccagcacactgcaagagcagatcggctggatgacaaacaaccctcctattcctgtgggcgagatctacaagagatggatcatcctgggactgaacaagatcgtgcggatgtacagccccaccagcatcctggacattagacagggccccaaagagcccttcagagactacgtggacagattctacaagaccctgagagccgagcaggccagccaagaagtgaagaactggatgaccgagacactgctggtgcagaacgctaaccccgactgcaagaccatcctgaaggctctgggacctgccgccacactggaagagatgatgacagcctgtcaaggcgtcggaggacctggccataaggctagagttctggccgaggccatgagccaagtgaccaacagcgccacaatcatgatgcagagaggcaacttcagaaaccagcggaagatcgtgaagtccttcaactccggcaaagagggccacaccgcccgcaattctagagcccctagaaagaaaggtggatccggcggcgtttctggatggcggctgttcaagaagatcagcggcggttccggacctgctgccaaaagagtgaaactggactccggactgcaactgcctccactggaaagactgacactgggagctgccccagccgccaagaagaaaaagctggactacaaggacgacgacgacaagggcggagctagctctaagacaatcgtgctgtctgtgggcgaagccaccagaacactgaccgagatccagagcacagccgacagacagatcttcgaggaaaaagtgggccctctcgtgggcagactgagactgacagcttccctgagacagaacggcgccaagaccgcctacagagtgaacctgaagctggaccaggccgacgtggtggattctggccttcctaaagtgcggtacacccaagtgtggtcccacgacgtgaccatcgtggccaattctaccgaggccagcagaaagagcctgtacgacctgaccaagagcctggtggccacaagccaggtggaagatctggtcgtgaacctggtgcctctcggacgtggcggatccggtggaaccgagagacaggccaacttcctgggcaagatctggcctagctacaagggcagacccggcaacttcctccagagcagaccagagcctaccgctcctcctgaggaatccttcagatccggcgtggaaaccaccacacctccacagaagcaagagcccatcgacaaagagctgtaccctctgaccagcctgagatccctgttcggcaacgaccctagctctcaatga

SEQ ID NO: 83 - DNA, 1896 bp, Synthetic construct
  source 1..1896: mol_type = other DNA
atgggcgctagagcctctgttctgtctggcggcgaactggacagatgggagaagatcagaagcagacctggcggcaagaagaagtacaagctgaagcacatcgtgtgggccagcagagagctggaaagattcgctgtgaaccccggcctgctggaaacaagcgagggctgtagacagatcctgggccagctccagccatctctccagacaggatctgaggaactgagaagcctgtacaacaccgtggccacactgtactgcgtgcaccagagaatcgagatcaaggacaccaaagaggccctggacaagatcgaggaagaacagaacaagtctaagaagaaggcccagcaggctgccgccgatacaggccactctaatcaggtgtcccagaactaccccatcgtgcagaacatccagggccagatggtgcatcaggctatcagccccagaacactgaacgcctgggtcaaagtggtggaagagaaggctttcagccctgaagtgatccccatgttcagcgccctgtctgagggtgccacacctcaggacctgaacaccatgctgaacacagtcggcggacaccaggccgctatgcagatgctgaaagagacaatcaacgaagaggccgccgagtgggacagagtgcatcctgttcatgctggccctatcgctcccggccagatgagagaacctagaggctctgacattgccggcaccaccagcacactgcaagagcagatcggctggatgacaaacaaccctcctattcctgtgggcgagatctacaagagatggatcatcctgggactgaacaagatcgtgcggatgtacagccccaccagcatcctggacattagacagggccccaaagagcccttcagagactacgtggacagattctacaagaccctgagagccgagcaggccagccaagaagtgaagaactggatgaccgagacactgctggtgcagaacgctaaccccgactgcaagaccatcctgaaggctctgggacctgccgccacactggaagagatgatgacagcctgtcaaggcgtcggaggacctggccataaggctagagttctggccgaggccatgagccaagtgaccaacagcgccacaatcatgatgcagagaggcaacttcagaaaccagcggaagatcgtgaagtccttcaactccggcaaagagggccacaccgcccgcaattctagagcccctagaaagaaaggtggatccggcggcgtttctggatggcggctgttcaagaagatcagcggcggagctagctctaagacaatcgtgctgtctgtgggcgaagccaccagaacactgaccgagatccagagcacagccgacagacagatcttcgaggaaaaagtgggccctctcgtgggcagactgagactgacagcttccctgagacagaacggcgccaagaccgcctacagagtgaacctgaagctggaccaggccgacgtggtggattctggccttcctaaagtgcggtacacccaagtgtggtcccacgacgtgaccatcgtggccaattctaccgaggccagcagaaagagcctgtacgacctgaccaagagcctggtggccacaagccaggtggaagatctggtcgtgaacctggtgcctctcggacgtggcggatccggtggaaccgagagacaggccaacttcctgggcaagatctggcctagctacaagggcagacccggcaacttcctccagagcagaccagagcctaccgctcctcctgaggaatccttcagatccggcgtggaaaccaccacacctccacagaagcaagagcccatcgacaaagagctgtaccctctgaccagcctgagatccctgttcggcaacgaccctagctctcaatga

SEQ ID NO: 84 - DNA, 2031 bp, Synthetic construct
  source 1..2031: mol_type = other DNA
atgggcgctagagcctctgttctgtctggcggcgaactggacagatgggagaagatcagactgagacctggcggcaagaagaagtacaagctgaagcacatcgtgtgggccagcagagagctggaaagattcgctgtgaaccccggcctgctggaaacaagcgagggctgtagacagatcctgggccagctccagccatctctccagacaggatctgaggaactgagaagcctgtacaacaccgtggccacactgtactgcgtgcaccagagaatcgagatcaaggacaccaaagaggccctggacaagatcgaggaagaacagaacaagtctaagaagaaggcccagcaggctgccgccgatacaggccactctaatcaggtgtcccagaactaccccatcgtgcagaacatccagggccagatggtgcatcaggctatcagccccagaacactgaacgcctgggtcaaagtggtggaagagaaggctttcagccctgaagtgatccccatgttcagcgccctgtctgagggtgccacacctcaggacctgaacaccatgctgaacacagtcggcggacaccaggccgctatgcagatgctgaaagagacaatcaacgaagaggccgccgagtgggacagagtgcatcctgttcatgctggccctatcgctcccggccagatgagagaacctagaggctctgacattgccggcaccaccagcacactgcaagagcagatcggctggatgacaaacaaccctcctattcctgtgggcgagatctacaagagatggatcatcctgggactgaacaagatcgtgcggatgtacagccccaccagcatcctggacattagacagggccccaaagagcccttcagagactacgtggacagattctacaagaccctgagagccgagcaggccagccaagaagtgaagaactggatgaccgagacactgctggtgcagaacgctaaccccgactgcaagaccatcctgaaggctctgggacctgccgccacactggaagagatgatgacagcctgtcaaggcgtcggaggacctggccataaggctagagttctggccgaggccatgagccaagtgaccaacagcgccacaatcatgatgcagagaggcaacttcagaaaccagcggaagatcgtgaagtccttcaactccggcaaagagggccacaccgcccgcaattctagagcccctagaaagaaaggtggatccggcggcgtttctggatggcggctgttcaagaagatcagcggcggttccggacctgctgccaaaagagtgaaactggactccggactgcaactgcctccactggaaagactgacactgggagctgccccagccgccaagaagaaaaagctggactacaaggacgacgacgacaagggcggagctagctctaagacaatcgtgctgtctgtgggcgaagccaccagaacactgaccgagatccagagcacagccgacagacagatcttcgaggaaaaagtgggccctctcgtgggcagactgagactgacagcttccctgagacagaacggcgccaagaccgcctacagagtgaacctgaagctggaccaggccgacgtggtggattctggccttcctaaagtgcggtacacccaagtgtggtcccacgacgtgaccatcgtggccaattctaccgaggccagcagaaagagcctgtacgacctgaccaagagcctggtggccacaagccaggtggaagatctggtcgtgaacctggtgcctctcggacgtggcggatccggtggaaccgagagacaggccaacttcctgggcaagatctggcctagctacaagggcagacccggcaacttcctccagagcagaccagagcctaccgctcctcctgaggaatccttcagatccggcgtggaaaccaccacacctccacagaagcaagagcccatcgacaaagagctgtaccctctgaccagcctgagatccctgttcggcaacgaccctagctctcaatga

SEQ ID NO: 85 - DNA, 1896 bp, Synthetic construct
  source 1..1896: mol_type = other DNA
atgggcgctagagcctctgttctgtctggcggcgaactggacagatgggagaagatcagactgagacctggcggcaagaagaagtacaagctgaagcacatcgtgtgggccagcagagagctggaaagattcgctgtgaaccccggcctgctggaaacaagcgagggctgtagacagatcctgggccagctccagccatctctccagacaggatctgaggaactgagaagcctgtacaacaccgtggccacactgtactgcgtgcaccagagaatcgagatcaaggacaccaaagaggccctggacaagatcgaggaagaacagaacaagtctaagaagaaggcccagcaggctgccgccgatacaggccactctaatcaggtgtcccagaactaccccatcgtgcagaacatccagggccagatggtgcatcaggctatcagccccagaacactgaacgcctgggtcaaagtggtggaagagaaggctttcagccctgaagtgatccccatgttcagcgccctgtctgagggtgccacacctcaggacctgaacaccatgctgaacacagtcggcggacaccaggccgctatgcagatgctgaaagagacaatcaacgaagaggccgccgagtgggacagagtgcatcctgttcatgctggccctatcgctcccggccagatgagagaacctagaggctctgacattgccggcaccaccagcacactgcaagagcagatcggctggatgacaaacaaccctcctattcctgtgggcgagatctacaagagatggatcatcctgggactgaacaagatcgtgcggatgtacagccccaccagcatcctggacattagacagggccccaaagagcccttcagagactacgtggacagattctacaagaccctgagagccgagcaggccagccaagaagtgaagaactggatgaccgagacactgctggtgcagaacgctaaccccgactgcaagaccatcctgaaggctctgggacctgccgccacactggaagagatgatgacagcctgtcaaggcgtcggaggacctggccataaggctagagttctggccgaggccatgagccaagtgaccaacagcgccacaatcatgatgcagagaggcaacttcagaaaccagcggaagatcgtgaagtccttcaactccggcaaagagggccacaccgcccgcaattctagagcccctagaaagaaaggtggatccggcggcgtttctggatggcggctgttcaagaagatcagcggcggagctagctctaagacaatcgtgctgtctgtgggcgaagccaccagaacactgaccgagatccagagcacagccgacagacagatcttcgaggaaaaagtgggccctctcgtgggcagactgagactgacagcttccctgagacagaacggcgccaagaccgcctacagagtgaacctgaagctggaccaggccgacgtggtggattctggccttcctaaagtgcggtacacccaagtgtggtcccacgacgtgaccatcgtggccaattctaccgaggccagcagaaagagcctgtacgacctgaccaagagcctggtggccacaagccaggtggaagatctggtcgtgaacctggtgcctctcggacgtggcggatccggtggaaccgagagacaggccaacttcctgggcaagatctggcctagctacaagggcagacccggcaacttcctccagagcagaccagagcctaccgctcctcctgaggaatccttcagatccggcgtggaaaccaccacacctccacagaagcaagagcccatcgacaaagagctgtaccctctgaccagcctgagatccctgttcggcaacgaccctagctctcaatga

SEQ ID NO: 86 - DNA, 1518 bp, Synthetic construct
  source 1..1518: mol_type = other DNA
atgggcgctagagcctctgttctgtctggcggcgaactggacagatgggagaagatcagactgagacctggcggcaagaagaagtacaagctgaagcacatcgtgtgggccagcagagagctggaaagattcgctgtgaaccccggcctgctggaaacaagcgagggctgtagacagatcctgggccagctccagccatctctccagacaggatctgaggaactgagaagcctgtacaacaccgtggccacactgtactgcgtgcaccagagaatcgagatcaaggacaccaaagaggccctggacaagatcgaggaagaacagaacaagtctaagaagaaggcccagcaggctgccgccgatacaggccactctaatcaggtgtcccagaactaccccatcgtgcagaacatccagggccagatggtgcatcaggctatcagccccagaacactgaacgcctgggtcaaagtggtggaagagaaggctttcagccctgaagtgatccccatgttcagcgccctgtctgagggtgccacacctcaggacctgaacaccatgctgaacacagtcggcggacaccaggccgctatgcagatgctgaaagagacaatcaacgaagaggccgccgagtgggacagagtgcatcctgttcatgctggccctatcgctcccggccagatgagagaacctagaggctctgacattgccggcaccaccagcacactgcaagagcagatcggctggatgacaaacaaccctcctattcctgtgggcgagatctacaagagatggatcatcctgggactgaacaagatcgtgcggatgtacagccccaccagcatcctggacattagacagggccccaaagagcccttcagagactacgtggacagattctacaagaccctgagagccgagcaggccagccaagaagtgaagaactggatgaccgagacactgctggtgcagaacgctaaccccgactgcaagaccatcctgaaggctctgggacctgccgccacactggaagagatgatgacagcctgtcaaggcgtcggaggacctggccataaggctagagttctggccgaggccatgagccaagtgaccaacagcgccacaatcatgatgcagagaggcaacttcagaaaccagcggaagatcgtgaagtccttcaactccggcaaagagggccacaccgcccgcaattctagagcccctagaaagaaaggtggatccggcggcgtttctggatggcggctgttcaagaagatcagcgctagcggtggaaccgagagacaggccaacttcctgggcaagatctggcctagctacaagggcagacccggcaacttcctccagagcagaccagagcctaccgctcctcctgaggaatccttcagatccggcgtggaaaccaccacacctccacagaagcaagagcccatcgacaaagagctgtaccctctgaccagcctgagatccctgttcggcaacgaccctagctctcaatga

SEQ ID NO: 87 - DNA, 1518 bp, Synthetic construct
  source 1..1518: mol_type = other DNA
atgggcgctagagcctctgttctgtctggcggcgaactggacagatgggagaagatcagaagcagacctggcggcaagaagaagtacaagctgaagcacatcgtgtgggccagcagagagctggaaagattcgctgtgaaccccggcctgctggaaacaagcgagggctgtagacagatcctgggccagctccagccatctctccagacaggatctgaggaactgagaagcctgtacaacaccgtggccacactgtactgcgtgcaccagagaatcgagatcaaggacaccaaagaggccctggacaagatcgaggaagaacagaacaagtctaagaagaaggcccagcaggctgccgccgatacaggccactctaatcaggtgtcccagaactaccccatcgtgcagaacatccagggccagatggtgcatcaggctatcagccccagaacactgaacgcctgggtcaaagtggtggaagagaaggctttcagccctgaagtgatccccatgttcagcgccctgtctgagggtgccacacctcaggacctgaacaccatgctgaacacagtcggcggacaccaggccgctatgcagatgctgaaagagacaatcaacgaagaggccgccgagtgggacagagtgcatcctgttcatgctggccctatcgctcccggccagatgagagaacctagaggctctgacattgccggcaccaccagcacactgcaagagcagatcggctggatgacaaacaaccctcctattcctgtgggcgagatctacaagagatggatcatcctgggactgaacaagatcgtgcggatgtacagccccaccagcatcctggacattagacagggccccaaagagcccttcagagactacgtggacagattctacaagaccctgagagccgagcaggccagccaagaagtgaagaactggatgaccgagacactgctggtgcagaacgctaaccccgactgcaagaccatcctgaaggctctgggacctgccgccacactggaagagatgatgacagcctgtcaaggcgtcggaggacctggccataaggctagagttctggccgaggccatgagccaagtgaccaacagcgccacaatcatgatgcagagaggcaacttcagaaaccagcggaagatcgtgaagtccttcaactccggcaaagagggccacaccgcccgcaattctagagcccctagaaagaaaggtggatccggcggcgtttctggatggcggctgttcaagaagatcagcgctagcggtggaaccgagagacaggccaacttcctgggcaagatctggcctagctacaagggcagacccggcaacttcctccagagcagaccagagcctaccgctcctcctgaggaatccttcagatccggcgtggaaaccaccacacctccacagaagcaagagcccatcgacaaagagctgtaccctctgaccagcctgagatccctgttcggcaacgaccctagctctcaatga

SEQ ID NO: 88 - DNA, 1872 bp, Synthetic construct
  source 1..1872: mol_type = other DNA
atgcacggcctgcaggacgaccctgatctgcaggccctgctgaagggcagccagctgctgaaagtgaagtccagcagctggcggcgggaaagattctacaagctgcaagaggactgcaagaccatctggcaggagtctagaaaggtgatgcgctccccagaaagccaactgttcagcatcgaggacatccaggaggtgcggatgggccacagaacagagggactggaaaagttcgccagagatatccccgaggatagatgttttagcattgtgttcaaggaccagcggaacaccctggacctgatcgcccctagccctgctgatgcccagcattgggtccagggcctcagaaagatcatccaccacagcggctctatggaccagagacagaaactgcagaccggtgctagagcctctgttctgtctggcggcgaactggacagatgggagaagatcagactgagacctggcggcaagaagaagtacaagctgaagcacatcgtgtgggccagcagagagctggaaagattcgctgtgaaccccggcctgctggaaacaagcgagggctgtagacagatcctgggccagctccagccatctctccagacaggatctgaggaactgagaagcctgtacaacaccgtggccacactgtactgcgtgcaccagagaatcgagatcaaggacaccaaagaggccctggacaagatcgaggaagaacagaacaagtctaagaagaaggcccagcaggctgccgccgatacaggccactctaatcaggtgtcccagaactaccccatcgtgcagaacatccagggccagatggtgcatcaggctatcagccccagaacactgaacgcctgggtcaaagtggtggaagagaaggctttcagccctgaagtgatccccatgttcagcgccctgtctgagggtgccacacctcaggacctgaacaccatgctgaacacagtcggcggacaccaggccgctatgcagatgctgaaagagacaatcaacgaagaggccgccgagtgggacagagtgcatcctgttcatgctggccctatcgctcccggccagatgagagaacctagaggctctgacattgccggcaccaccagcacactgcaagagcagatcggctggatgacaaacaaccctcctattcctgtgggcgagatctacaagagatggatcatcctgggactgaacaagatcgtgcggatgtacagccccaccagcatcctggacattagacagggccccaaagagcccttcagagactacgtggacagattctacaagaccctgagagccgagcaggccagccaagaagtgaagaactggatgaccgagacactgctggtgcagaacgctaaccccgactgcaagaccatcctgaaggctctgggacctgccgccacactggaagagatgatgacagcctgtcaaggcgtcggaggacctggccataaggctagagttctggccgaggccatgagccaagtgaccaacagcgccacaatcatgatgcagagaggcaacttcagaaaccagcggaagatcgtgaagtccttcaactccggcaaagagggccacaccgcccgcaattctagagcccctagaaagaaaggtggatccggtggaaccgagagacaggccaacttcctgggcaagatctggcctagctacaagggcagacccggcaacttcctccagagcagaccagagcctaccgctcctcctgaggaatccttcagatccggcgtggaaaccaccacacctccacagaagcaagagcccatcgacaaagagctgtaccctctgaccagcctgagatccctgttcggcaacgaccctagctctcaatga

SEQ ID NO: 89 - DNA, 2295 bp, Synthetic construct
  source 1..2295: mol_type = other DNA
atgcacggcctgcaggacgaccctgatctgcaggccctgctgaagggcagccagctgctgaaagtgaagtccagcagctggcggcgggaaagattctacaagctgcaagaggactgcaagaccatctggcaggagtctagaaaggtgatgcgctccccagaaagccaactgttcagcatcgaggacatccaggaggtgcggatgggccacagaacagagggactggaaaagttcgccagagatatccccgaggatagatgttttagcattgtgttcaaggaccagcggaacaccctggacctgatcgcccctagccctgctgatgcccagcattgggtccagggcctcagaaagatcatccaccacagcggctctatggaccagagacagaaactgcagaccggtgctagagcctctgttctgtctggcggcgaactggacagatgggagaagatcagaagcagacctggcggcaagaagaagtacaagctgaagcacatcgtgtgggccagcagagagctggaaagattcgctgtgaaccccggcctgctggaaacaagcgagggctgtagacagatcctgggccagctccagccatctctccagacaggatctgaggaactgagaagcctgtacaacaccgtggccacactgtactgcgtgcaccagagaatcgagatcaaggacaccaaagaggccctggacaagatcgaggaagaacagaacaagtctaagaagaaggcccagcaggctgccgccgatacaggccactctaatcaggtgtcccagaactaccccatcgtgcagaacatccagggccagatggtgcatcaggctatcagccccagaacactgaacgcctgggtcaaagtggtggaagagaaggctttcagccctgaagtgatccccatgttcagcgccctgtctgagggtgccacacctcaggacctgaacaccatgctgaacacagtcggcggacaccaggccgctatgcagatgctgaaagagacaatcaacgaagaggccgccgagtgggacagagtgcatcctgttcatgctggccctatcgctcccggccagatgagagaacctagaggctctgacattgccggcaccaccagcacactgcaagagcagatcggctggatgacaaacaaccctcctattcctgtgggcgagatctacaagagatggatcatcctgggactgaacaagatcgtgcggatgtacagccccaccagcatcctggacattagacagggccccaaagagcccttcagagactacgtggacagattctacaagaccctgagagccgagcaggccagccaagaagtgaagaactggatgaccgagacactgctggtgcagaacgctaaccccgactgcaagaccatcctgaaggctctgggacctgccgccacactggaagagatgatgacagcctgtcaaggcgtcggaggacctggccataaggctagagttctggccgaggccatgagccaagtgaccaacagcgccacaatcatgatgcagagaggcaacttcagaaaccagcggaagatcgtgaagtccttcaactccggcaaagagggccacaccgcccgcaattctagagcccctagaaagaaaggtggatccggcggcgtttctggatggcggctgttcaagaagatcagcggcggagctagctctaagacaatcgtgctgtctgtgggcgaagccaccagaacactgaccgagatccagagcacagccgacagacagatcttcgaggaaaaagtgggccctctcgtgggcagactgagactgacagcttccctgagacagaacggcgccaagaccgcctacagagtgaacctgaagctggaccaggccgacgtggtggattctggccttcctaaagtgcggtacacccaagtgtggtcccacgacgtgaccatcgtggccaattctaccgaggccagcagaaagagcctgtacgacctgaccaagagcctggtggccacaagccaggtggaagatctggtcgtgaacctggtgcctctcggacgtggcggatccggtggaaccgagagacaggccaacttcctgggcaagatctggcctagctacaagggcagacccggcaacttcctccagagcagaccagagcctaccgctcctcctgaggaatccttcagatccggcgtggaaaccaccacacctccacagaagcaagagcccatcgacaaagagctgtaccctctgaccagcctgagatccctgttcggcaacgaccctagctctcaatga

SEQ ID NO: 90 - DNA, 2295 bp, Synthetic construct
  source 1..2295: mol_type = other DNA
atgcacggcctgcaggacgaccctgatctgcaggccctgctgaagggcagccagctgctgaaagtgaagtccagcagctggcggcgggaaagattctacaagctgcaagaggactgcaagaccatctggcaggagtctagaaaggtgatgcgctccccagaaagccaactgttcagcatcgaggacatccaggaggtgcggatgggccacagaacagagggactggaaaagttcgccagagatatccccgaggatagatgttttagcattgtgttcaaggaccagcggaacaccctggacctgatcgcccctagccctgctgatgcccagcattgggtccagggcctcagaaagatcatccaccacagcggctctatggaccagagacagaaactgcagaccggtgctagagcctctgttctgtctggcggcgaactggacagatgggagaagatcagactgagacctggcggcaagaagaagtacaagctgaagcacatcgtgtgggccagcagagagctggaaagattcgctgtgaaccccggcctgctggaaacaagcgagggctgtagacagatcctgggccagctccagccatctctccagacaggatctgaggaactgagaagcctgtacaacaccgtggccacactgtactgcgtgcaccagagaatcgagatcaaggacaccaaagaggccctggacaagatcgaggaagaacagaacaagtctaagaagaaggcccagcaggctgccgccgatacaggccactctaatcaggtgtcccagaactaccccatcgtgcagaacatccagggccagatggtgcatcaggctatcagccccagaacactgaacgcctgggtcaaagtggtggaagagaaggctttcagccctgaagtgatccccatgttcagcgccctgtctgagggtgccacacctcaggacctgaacaccatgctgaacacagtcggcggacaccaggccgctatgcagatgctgaaagagacaatcaacgaagaggccgccgagtgggacagagtgcatcctgttcatgctggccctatcgctcccggccagatgagagaacctagaggctctgacattgccggcaccaccagcacactgcaagagcagatcggctggatgacaaacaaccctcctattcctgtgggcgagatctacaagagatggatcatcctgggactgaacaagatcgtgcggatgtacagccccaccagcatcctggacattagacagggccccaaagagcccttcagagactacgtggacagattctacaagaccctgagagccgagcaggccagccaagaagtgaagaactggatgaccgagacactgctggtgcagaacgctaaccccgactgcaagaccatcctgaaggctctgggacctgccgccacactggaagagatgatgacagcctgtcaaggcgtcggaggacctggccataaggctagagttctggccgaggccatgagccaagtgaccaacagcgccacaatcatgatgcagagaggcaacttcagaaaccagcggaagatcgtgaagtccttcaactccggcaaagagggccacaccgcccgcaattctagagcccctagaaagaaaggtggatccggcggcgtttctggatggcggctgttcaagaagatcagcggcggagctagctctaagacaatcgtgctgtctgtgggcgaagccaccagaacactgaccgagatccagagcacagccgacagacagatcttcgaggaaaaagtgggccctctcgtgggcagactgagactgacagcttccctgagacagaacggcgccaagaccgcctacagagtgaacctgaagctggaccaggccgacgtggtggattctggccttcctaaagtgcggtacacccaagtgtggtcccacgacgtgaccatcgtggccaattctaccgaggccagcagaaagagcctgtacgacctgaccaagagcctggtggccacaagccaggtggaagatctggtcgtgaacctggtgcctctcggacgtggcggatccggtggaaccgagagacaggccaacttcctgggcaagatctggcctagctacaagggcagacccggcaacttcctccagagcagaccagagcctaccgctcctcctgaggaatccttcagatccggcgtggaaaccaccacacctccacagaagcaagagcccatcgacaaagagctgtaccctctgaccagcctgagatccctgttcggcaacgaccctagctctcaatga

SEQ ID NO: 91 - DNA, 2340 bp, Synthetic construct
  source 1..2340: mol_type = other DNA
atgcacggcctgcaggacgaccctgatctgcaggccctgctgaagggcagccagctgctgaaagtgaagtccagcagctggcggcgggaaagattctacaagctgcaagaggactgcaagaccatctggcaggagtctagaaaggtgatgcgctccccagaaagccaactgttcagcatcgaggacatccaggaggtgcggatgggccacagaacagagggactggaaaagttcgccagagatatccccgaggatagatgttttagcattgtgttcaaggaccagcggaacaccctggacctgatcgcccctagccctgctgatgcccagcattgggtccagggcctcagaaagatcatccaccacagcggctctatggaccagagacagaaactgcagaccggtgctagagcctctgttctgtctggcggcgaactggacagatgggagaagatcagaagcagacctggcggcaagaagaagtacaagctgaagcacatcgtgtgggccagcagagagctggaaagattcgctgtgaaccccggcctgctggaaacaagcgagggctgtagacagatcctgggccagctccagccatctctccagacaggatctgaggaactgagaagcctgtacaacaccgtggccacactgtactgcgtgcaccagagaatcgagatcaaggacaccaaagaggccctggacaagatcgaggaagaacagaacaagtctaagaagaaggcccagcaggctgccgccgatacaggccactctaatcaggtgtcccagaactaccccatcgtgcagaacatccagggccagatggtgcatcaggctatcagccccagaacactgaacgcctgggtcaaagtggtggaagagaaggctttcagccctgaagtgatccccatgttcagcgccctgtctgagggtgccacacctcaggacctgaacaccatgctgaacacagtcggcggacaccaggccgctatgcagatgctgaaagagacaatcaacgaagaggccgccgagtgggacagagtgcatcctgttcatgctggccctatcgctcccggccagatgagagaacctagaggctctgacattgccggcaccaccagcacactgcaagagcagatcggctggatgacaaacaaccctcctattcctgtgggcgagatctacaagagatggatcatcctgggactgaacaagatcgtgcggatgtacagccccaccagcatcctggacattagacagggccccaaagagcccttcagagactacgtggacagattctacaagaccctgagagccgagcaggccagccaagaagtgaagaactggatgaccgagacactgctggtgcagaacgctaaccccgactgcaagaccatcctgaaggctctgggacctgccgccacactggaagagatgatgacagcctgtcaaggcgtcggaggacctggccataaggctagagttctggccgaggccatgagccaagtgaccaacagcgccacaatcatgatgcagagaggcaacttcagaaaccagcggaagatcgtgaagtgcttcaactgcggcaaagagggccacaccgccagaaactgtagagcccctagaaagaaaggctgctggaagtgtggaaaagaggggcaccagatgaaggactgcggtggatccggcggcgtttctggatggcggctgttcaagaagatcagcggcggagctagctctaagacaatcgtgctgtctgtgggcgaagccaccagaacactgaccgagatccagagcacagccgacagacagatcttcgaggaaaaagtgggccctctcgtgggcagactgagactgacagcttccctgagacagaacggcgccaagaccgcctacagagtgaacctgaagctggaccaggccgacgtggtggattctggccttcctaaagtgcggtacacccaagtgtggtcccacgacgtgaccatcgtggccaattctaccgaggccagcagaaagagcctgtacgacctgaccaagagcctggtggccacaagccaggtggaagatctggtcgtgaacctggtgcctctcggacgtggcggatccggtggaaccgagagacaggccaacttcctgggcaagatctggcctagctacaagggcagacccggcaacttcctccagagcagaccagagcctaccgctcctcctgaggaatccttcagatccggcgtggaaaccaccacacctccacagaagcaagagcccatcgacaaagagctgtaccctctgaccagcctgagatccctgttcggcaacgaccctagctctcaatga

SEQ ID NO: 92 - DNA, 2430 bp, Synthetic construct
  source 1..2430: mol_type = other DNA
atgcacggcctgcaggacgaccctgatctgcaggccctgctgaagggcagccagctgctgaaagtgaagtccagcagctggcggcgggaaagattctacaagctgcaagaggactgcaagaccatctggcaggagtctagaaaggtgatgcgctccccagaaagccaactgttcagcatcgaggacatccaggaggtgcggatgggccacagaacagagggactggaaaagttcgccagagatatccccgaggatagatgttttagcattgtgttcaaggaccagcggaacaccctggacctgatcgcccctagccctgctgatgcccagcattgggtccagggcctcagaaagatcatccaccacagcggctctatggaccagagacagaaactgcagaccggtgctagagcctctgttctgtctggcggcgaactggacagatgggagaagatcagaagcagacctggcggcaagaagaagtacaagctgaagcacatcgtgtgggccagcagagagctggaaagattcgctgtgaaccccggcctgctggaaacaagcgagggctgtagacagatcctgggccagctccagccatctctccagacaggatctgaggaactgagaagcctgtacaacaccgtggccacactgtactgcgtgcaccagagaatcgagatcaaggacaccaaagaggccctggacaagatcgaggaagaacagaacaagtctaagaagaaggcccagcaggctgccgccgatacaggccactctaatcaggtgtcccagaactaccccatcgtgcagaacatccagggccagatggtgcatcaggctatcagccccagaacactgaacgcctgggtcaaagtggtggaagagaaggctttcagccctgaagtgatccccatgttcagcgccctgtctgagggtgccacacctcaggacctgaacaccatgctgaacacagtcggcggacaccaggccgctatgcagatgctgaaagagacaatcaacgaagaggccgccgagtgggacagagtgcatcctgttcatgctggccctatcgctcccggccagatgagagaacctagaggctctgacattgccggcaccaccagcacactgcaagagcagatcggctggatgacaaacaaccctcctattcctgtgggcgagatctacaagagatggatcatcctgggactgaacaagatcgtgcggatgtacagccccaccagcatcctggacattagacagggccccaaagagcccttcagagactacgtggacagattctacaagaccctgagagccgagcaggccagccaagaagtgaagaactggatgaccgagacactgctggtgcagaacgctaaccccgactgcaagaccatcctgaaggctctgggacctgccgccacactggaagagatgatgacagcctgtcaaggcgtcggaggacctggccataaggctagagttctggccgaggccatgagccaagtgaccaacagcgccacaatcatgatgcagagaggcaacttcagaaaccagcggaagatcgtgaagtccttcaactccggcaaagagggccacaccgcccgcaattctagagcccctagaaagaaaggtggatccggcggcgtttctggatggcggctgttcaagaagatcagcggcggttccggacctgctgccaaaagagtgaaactggactccggactgcaactgcctccactggaaagactgacactgggagctgccccagccgccaagaagaaaaagctggactacaaggacgacgacgacaagggcggagctagctctaagacaatcgtgctgtctgtgggcgaagccaccagaacactgaccgagatccagagcacagccgacagacagatcttcgaggaaaaagtgggccctctcgtgggcagactgagactgacagcttccctgagacagaacggcgccaagaccgcctacagagtgaacctgaagctggaccaggccgacgtggtggattctggccttcctaaagtgcggtacacccaagtgtggtcccacgacgtgaccatcgtggccaattctaccgaggccagcagaaagagcctgtacgacctgaccaagagcctggtggccacaagccaggtggaagatctggtcgtgaacctggtgcctctcggacgtggcggatccggtggaaccgagagacaggccaacttcctgggcaagatctggcctagctacaagggcagacccggcaacttcctccagagcagaccagagcctaccgctcctcctgaggaatccttcagatccggcgtggaaaccaccacacctccacagaagcaagagcccatcgacaaagagctgtaccctctgaccagcctgagatccctgttcggcaacgaccctagctctcaatga

SEQ ID NO: 93 - DNA, 1101 bp, Synthetic construct
  source 1..1101: mol_type = other DNA
atgggagctagagcatctgttctgtctggcggagcacagcaggccgctgctgatacaggccactctaatcaggtgtcccagaactacagccccacctccatcctggacatcagacagggccccaaagagcccttccgggactacgtggacagattctacaagaccctgagagccgagcaggccagccaagaagtgaagaactggatgaccgagacactgctggtgcagaacgccaatcctgactgcaagaccatcctgaaggctctgggacctgccgccacactggaagagatgatgacagcctgtcaaggcgttggcggccctggacacaaagctagagttctggccgaggccatgagccaagtgaccaactccgctaccatcatgggaggatccggcggcagaatgaagcagctggaagataaggtggaagaactgctgagcaagaactaccacctggaaaacgaggtggcccggctgaagaagctcgttggagaaagaggtggcagcggcggagtttctggatggcggctgttcaagaagatcagcggcggagctagctctaagacaatcgtgctgtctgtgggcgaagccaccagaacactgaccgagatccagagcacagccgacagacagatcttcgaggaaaaagtgggccctctcgtgggcagactgagactgacagcttccctgagacagaacggcgccaagaccgcctacagagtgaacctgaagctggaccaggccgacgtggtggattctggccttcctaaagtgcggtacacccaagtgtggtcccacgacgtgaccatcgtggccaattctaccgaggccagcagaaagagcctgtacgacctgaccaagagcctggtggccacaagccaggtggaagatctggtcgtgaacctggtgcctctcggacgtggcggcagcgctggcggactccagagcagacctgaacctacagctccaccagaggaatccttccgcagcggcgtggaaaccacaacacctccacagaagcaagagcccatcgacaaagagctgtaccctctgaccagcctgagaagcctgttcggcaacgatcccagcagccagtaa

SEQ ID NO: 94 - DNA, 1236 bp, Synthetic construct
  source 1..1236: mol_type = other DNA
atgggagctagagcatctgttctgtctggcggagcacagcaggccgctgctgatacaggccactctaatcaggtgtcccagaactacagccccacctccatcctggacatcagacagggccccaaagagcccttccgggactacgtggacagattctacaagaccctgagagccgagcaggccagccaagaagtgaagaactggatgaccgagacactgctggtgcagaacgccaatcctgactgcaagaccatcctgaaggctctgggacctgccgccacactggaagagatgatgacagcctgtcaaggcgttggcggccctggacacaaagctagagttctggccgaggccatgagccaagtgaccaactccgctaccatcatgggaggatccggcggcagaatgaagcagctggaagataaggtggaagaactgctgagcaagaactaccacctggaaaacgaggtggcccggctgaagaagctcgttggagaaagaggtggcagcggcggagtttctggatggcggctgttcaagaagatcagcggcggttccggacctgctgccaaaagagtgaaactggactccggactgcaactgcctccactggaaagactgacactgggagctgccccagccgccaagaagaaaaagctggactacaaggacgacgacgacaagggcggagctagctctaagacaatcgtgctgtctgtgggcgaagccaccagaacactgaccgagatccagagcacagccgacagacagatcttcgaggaaaaagtgggccctctcgtgggcagactgagactgacagcttccctgagacagaacggcgccaagaccgcctacagagtgaacctgaagctggaccaggccgacgtggtggattctggccttcctaaagtgcggtacacccaagtgtggtcccacgacgtgaccatcgtggccaattctaccgaggccagcagaaagagcctgtacgacctgaccaagagcctggtggccacaagccaggtggaagatctggtcgtgaacctggtgcctctcggacgtggcggcagcgctggcggactccagagcagacctgaacctacagctccaccagaggaatccttccgcagcggcgtggaaaccacaacacctccacagaagcaagagcccatcgacaaagagctgtaccctctgaccagcctgagaagcctgttcggcaacgatcccagcagccagtaa

SEQ ID NO: 95 - DNA, 1212 bp, Synthetic construct
  source 1..1212: mol_type = other DNA
atgggagctagagcatctgttctgtctggcggagcacagcaggccgctgctgatacaggccactctaatcaggtgtcccagaactacagccccacctccatcctggacatcagacagggccccaaagagcccttccgggactacgtggacagattctacaagaccctgagagccgagcaggccagccaagaagtgaagaactggatgaccgagacactgctggtgcagaacgccaatcctgactgcaagaccatcctgaaggctctgggacctgccgccacactggaagagatgatgacagcctgtcaaggcgttggcggccctggacacaaagctagagttctggccgaggccatgagccaagtgaccaactccgctaccatcatgggaggatccggcggcagaatgaagcagctggaagataaggtggaagaactgctgagcaagaactaccacctggaaaacgaggtggcccggctgaagaagctcgttggagaaagaggtggcagcggcggagtttctggatggcggctgttcaagaagatcagcggcggttccggacctgctgccaagaagaaaaagaacggctccggactgcaactgcctccactggaaagactgacactgggagctgccgactacaaggacgacgacgacaagggcggagctagctctaagacaatcgtgctgtctgtgggcgaagccaccagaacactgaccgagatccagagcacagccgacagacagatcttcgaggaaaaagtgggccctctcgtgggcagactgagactgacagcttccctgagacagaacggcgccaagaccgcctacagagtgaacctgaagctggaccaggccgacgtggtggattctggccttcctaaagtgcggtacacccaagtgtggtcccacgacgtgaccatcgtggccaattctaccgaggccagcagaaagagcctgtacgacctgaccaagagcctggtggccacaagccaggtggaagatctggtcgtgaacctggtgcctctcggacgtggcggcagcgctggcggactccagagcagacctgaacctacagctccaccagaggaatccttccgcagcggcgtggaaaccacaacacctccacagaagcaagagcccatcgacaaagagctgtaccctctgaccagcctgagaagcctgttcggcaacgatcccagcagccagtaa

SEQ ID NO: 96 - DNA, 1206 bp, Synthetic construct
  source 1..1206: mol_type = other DNA
atgggagctagagcatctgttctgtctggcggagcacagcaggccgctgctgatacaggccactctaatcaggtgtcccagaactacagccccacctccatcctggacatcagacagggccccaaagagcccttccgggactacgtggacagattctacaagaccctgagagccgagcaggccagccaagaagtgaagaactggatgaccgagacactgctggtgcagaacgccaatcctgactgcaagaccatcctgaaggctctgggacctgccgccacactggaagagatgatgacagcctgtcaaggcgttggcggccctggacacaaagctagagttctggccgaggccatgagccaagtgaccaactccgctaccatcatgggaggatccggcggcagaatgaagcagctggaagataaggtggaagaactgctgagcaagaactaccacctggaaaacgaggtggcccggctgaagaagctcgttggagaaagaggtggcagcggcggagtttctggatggcggctgttcaagaagatcagcggcggttccggacctaagaagaaaagaaaggtgtccggactgcaactgcctccactggaaagactgacactgggagctgccgactacaaggacgacgacgacaagggcggagctagctctaagacaatcgtgctgtctgtgggcgaagccaccagaacactgaccgagatccagagcacagccgacagacagatcttcgaggaaaaagtgggccctctcgtgggcagactgagactgacagcttccctgagacagaacggcgccaagaccgcctacagagtgaacctgaagctggaccaggccgacgtggtggattctggccttcctaaagtgcggtacacccaagtgtggtcccacgacgtgaccatcgtggccaattctaccgaggccagcagaaagagcctgtacgacctgaccaagagcctggtggccacaagccaggtggaagatctggtcgtgaacctggtgcctctcggacgtggcggcagcgctggcggactccagagcagacctgaacctacagctccaccagaggaatccttccgcagcggcgtggaaaccacaacacctccacagaagcaagagcccatcgacaaagagctgtaccctctgaccagcctgagaagcctgttcggcaacgatcccagcagccagtaa

SEQ ID NO: 97 - DNA, 1536 bp, Synthetic construct
  source 1..1536: mol_type = other DNA
atgggagctagagcatctgttctgtctggcggagcacagcaggccgctgctgatacaggccactctaatcaggtgtcccagaactaccccatcgtgcagaacatccagggccagatggtgcatcaggctatcagccccagaacactgaacgcctgggtcaaagtggtggaagagaaggctttcagccctgaagtgatccccatgttcagcgccctgtctgagggtgccacacctcaggacctgaacaccatgctgaacacagtcggcggacaccaggccgctatgcagatgctgaaagagacaatcaacgaagaggccgccgagtgggacagagtgcatcctgttcatgctggccctatcgctcccggccagatgagagaacctagaggctctgacattgccggcaccaccagcacactgcaagagcagatcggctggatgacaaacaaccctcctattcctgtgggcgagatctacaagagatggatcatcctgggactgaacaagatcgtgcggatgtacagccccacctccatcctggacatcagacagggccccaaagagcccttccgggactacgtggacagattctacaagaccctgagagccgagcaggccagccaagaagtgaagaactggatgaccgagacactgctggtgcagaacgccaatcctgactgcaagaccatcctgaaggctctgggacctgccgccacactggaagagatgatgacagcctgtcaaggcgttggcggccctggacacaaagctagagttctggccgaggccatgagccaagtgaccaactccgctaccatcatgggaggatccggcggcagaatgaagcagctggaagataaggtggaagaactgctgagcaagaactaccacctggaaaacgaggtggcccggctgaagaagctcgttggagaaagaggtggcagcggcggagtttctggatggcggctgttcaagaagatcagcggcggagctagctctaagacaatcgtgctgtctgtgggcgaagccaccagaacactgaccgagatccagagcacagccgacagacagatcttcgaggaaaaagtgggccctctcgtgggcagactgagactgacagcttccctgagacagaacggcgccaagaccgcctacagagtgaacctgaagctggaccaggccgacgtggtggattctggccttcctaaagtgcggtacacccaagtgtggtcccacgacgtgaccatcgtggccaattctaccgaggccagcagaaagagcctgtacgacctgaccaagagcctggtggccacaagccaggtggaagatctggtcgtgaacctggtgcctctcggacgtggcggcagcgctggcggactccagagcagacctgaacctacagctccaccagaggaatccttccgcagcggcgtggaaaccacaacacctccacagaagcaagagcccatcgacaaagagctgtaccctctgaccagcctgagaagcctgttcggcaacgatcccagcagccagtaa

SEQ ID NO: 98 - DNA, 1671 bp, Synthetic construct
  source 1..1671: mol_type = other DNA
atgggagctagagcatctgttctgtctggcggagcacagcaggccgctgctgatacaggccactctaatcaggtgtcccagaactaccccatcgtgcagaacatccagggccagatggtgcatcaggctatcagccccagaacactgaacgcctgggtcaaagtggtggaagagaaggctttcagccctgaagtgatccccatgttcagcgccctgtctgagggtgccacacctcaggacctgaacaccatgctgaacacagtcggcggacaccaggccgctatgcagatgctgaaagagacaatcaacgaagaggccgccgagtgggacagagtgcatcctgttcatgctggccctatcgctcccggccagatgagagaacctagaggctctgacattgccggcaccaccagcacactgcaagagcagatcggctggatgacaaacaaccctcctattcctgtgggcgagatctacaagagatggatcatcctgggactgaacaagatcgtgcggatgtacagccccacctccatcctggacatcagacagggccccaaagagcccttccgggactacgtggacagattctacaagaccctgagagccgagcaggccagccaagaagtgaagaactggatgaccgagacactgctggtgcagaacgccaatcctgactgcaagaccatcctgaaggctctgggacctgccgccacactggaagagatgatgacagcctgtcaaggcgttggcggccctggacacaaagctagagttctggccgaggccatgagccaagtgaccaactccgctaccatcatgggaggatccggcggcagaatgaagcagctggaagataaggtggaagaactgctgagcaagaactaccacctggaaaacgaggtggcccggctgaagaagctcgttggagaaagaggtggcagcggcggagtttctggatggcggctgttcaagaagatcagcggcggttccggacctgctgccaaaagagtgaaactggactccggactgcaactgcctccactggaaagactgacactgggagctgccccagccgccaagaagaaaaagctggactacaaggacgacgacgacaagggcggagctagctctaagacaatcgtgctgtctgtgggcgaagccaccagaacactgaccgagatccagagcacagccgacagacagatcttcgaggaaaaagtgggccctctcgtgggcagactgagactgacagcttccctgagacagaacggcgccaagaccgcctacagagtgaacctgaagctggaccaggccgacgtggtggattctggccttcctaaagtgcggtacacccaagtgtggtcccacgacgtgaccatcgtggccaattctaccgaggccagcagaaagagcctgtacgacctgaccaagagcctggtggccacaagccaggtggaagatctggtcgtgaacctggtgcctctcggacgtggcggcagcgctggcggactccagagcagacctgaacctacagctccaccagaggaatccttccgcagcggcgtggaaaccacaacacctccacagaagcaagagcccatcgacaaagagctgtaccctctgaccagcctgagaagcctgttcggcaacgatcccagcagccagtaa

SEQ ID NO: 99 - DNA, 1500 bp, Synthetic construct
  source 1..1500: mol_type = other DNA
atgcacggcctgcaggacgaccctgatctgcaggccctgctgaagggcagccagctgctgaaagtgaagtccagcagctggcggcgggaaagattctacaagctgcaagaggactgcaagaccatctggcaggagtctagaaaggtgatgcgctccccagaaagccaactgttcagcatcgaggacatccaggaggtgcggatgggccacagaacagagggactggaaaagttcgccagagatatccccgaggatagatgttttagcattgtgttcaaggaccagcggaacaccctggacctgatcgcccctagccctgctgatgcccagcattgggtccagggcctcagaaagatcatccaccacagcggctctatggaccagagacagaaactgcagaccggtgctagagcatctgttctgtctggcggagcacagcaggccgctgctgatacaggccactctaatcaggtgtcccagaactacagccccacctccatcctggacatcagacagggccccaaagagcccttccgggactacgtggacagattctacaagaccctgagagccgagcaggccagccaagaagtgaagaactggatgaccgagacactgctggtgcagaacgccaatcctgactgcaagaccatcctgaaggctctgggacctgccgccacactggaagagatgatgacagcctgtcaaggcgttggcggccctggacacaaagctagagttctggccgaggccatgagccaagtgaccaactccgctaccatcatgggaggatccggcggcagaatgaagcagctggaagataaggtggaagaactgctgagcaagaactaccacctggaaaacgaggtggcccggctgaagaagctcgttggagaaagaggtggcagcggcggagtttctggatggcggctgttcaagaagatcagcggcggagctagctctaagacaatcgtgctgtctgtgggcgaagccaccagaacactgaccgagatccagagcacagccgacagacagatcttcgaggaaaaagtgggccctctcgtgggcagactgagactgacagcttccctgagacagaacggcgccaagaccgcctacagagtgaacctgaagctggaccaggccgacgtggtggattctggccttcctaaagtgcggtacacccaagtgtggtcccacgacgtgaccatcgtggccaattctaccgaggccagcagaaagagcctgtacgacctgaccaagagcctggtggccacaagccaggtggaagatctggtcgtgaacctggtgcctctcggacgtggcggcagcgctggcggactccagagcagacctgaacctacagctccaccagaggaatccttccgcagcggcgtggaaaccacaacacctccacagaagcaagagcccatcgacaaagagctgtaccctctgaccagcctgagaagcctgttcggcaacgatcccagcagccagtaa

SEQ ID NO: 100 - DNA, 1635 bp, Synthetic construct
  source 1..1635: mol_type = other DNA
atgcacggcctgcaggacgaccctgatctgcaggccctgctgaagggcagccagctgctgaaagtgaagtccagcagctggcggcgggaaagattctacaagctgcaagaggactgcaagaccatctggcaggagtctagaaaggtgatgcgctccccagaaagccaactgttcagcatcgaggacatccaggaggtgcggatgggccacagaacagagggactggaaaagttcgccagagatatccccgaggatagatgttttagcattgtgttcaaggaccagcggaacaccctggacctgatcgcccctagccctgctgatgcccagcattgggtccagggcctcagaaagatcatccaccacagcggctctatggaccagagacagaaactgcagaccggtgctagagcatctgttctgtctggcggagcacagcaggccgctgctgatacaggccactctaatcaggtgtcccagaactacagccccacctccatcctggacatcagacagggccccaaagagcccttccgggactacgtggacagattctacaagaccctgagagccgagcaggccagccaagaagtgaagaactggatgaccgagacactgctggtgcagaacgccaatcctgactgcaagaccatcctgaaggctctgggacctgccgccacactggaagagatgatgacagcctgtcaaggcgttggcggccctggacacaaagctagagttctggccgaggccatgagccaagtgaccaactccgctaccatcatgggaggatccggcggcagaatgaagcagctggaagataaggtggaagaactgctgagcaagaactaccacctggaaaacgaggtggcccggctgaagaagctcgttggagaaagaggtggcagcggcggagtttctggatggcggctgttcaagaagatcagcggcggttccggacctgctgccaaaagagtgaaactggactccggactgcaactgcctccactggaaagactgacactgggagctgccccagccgccaagaagaaaaagctggactacaaggacgacgacgacaagggcggagctagctctaagacaatcgtgctgtctgtgggcgaagccaccagaacactgaccgagatccagagcacagccgacagacagatcttcgaggaaaaagtgggccctctcgtgggcagactgagactgacagcttccctgagacagaacggcgccaagaccgcctacagagtgaacctgaagctggaccaggccgacgtggtggattctggccttcctaaagtgcggtacacccaagtgtggtcccacgacgtgaccatcgtggccaattctaccgaggccagcagaaagagcctgtacgacctgaccaagagcctggtggccacaagccaggtggaagatctggtcgtgaacctggtgcctctcggacgtggcggcagcgctggcggactccagagcagacctgaacctacagctccaccagaggaatccttccgcagcggcgtggaaaccacaacacctccacagaagcaagagcccatcgacaaagagctgtaccctctgaccagcctgagaagcctgttcggcaacgatcccagcagccagtaa

SEQ ID NO: 101 - DNA, 1611 bp, Synthetic construct
  source 1..1611: mol_type = other DNA
atgcacggcctgcaggacgaccctgatctgcaggccctgctgaagggcagccagctgctgaaagtgaagtccagcagctggcggcgggaaagattctacaagctgcaagaggactgcaagaccatctggcaggagtctagaaaggtgatgcgctccccagaaagccaactgttcagcatcgaggacatccaggaggtgcggatgggccacagaacagagggactggaaaagttcgccagagatatccccgaggatagatgttttagcattgtgttcaaggaccagcggaacaccctggacctgatcgcccctagccctgctgatgcccagcattgggtccagggcctcagaaagatcatccaccacagcggctctatggaccagagacagaaactgcagaccggtgctagagcatctgttctgtctggcggagcacagcaggccgctgctgatacaggccactctaatcaggtgtcccagaactacagccccacctccatcctggacatcagacagggccccaaagagcccttccgggactacgtggacagattctacaagaccctgagagccgagcaggccagccaagaagtgaagaactggatgaccgagacactgctggtgcagaacgccaatcctgactgcaagaccatcctgaaggctctgggacctgccgccacactggaagagatgatgacagcctgtcaaggcgttggcggccctggacacaaagctagagttctggccgaggccatgagccaagtgaccaactccgctaccatcatgggaggatccggcggcagaatgaagcagctggaagataaggtggaagaactgctgagcaagaactaccacctggaaaacgaggtggcccggctgaagaagctcgttggagaaagaggtggcagcggcggagtttctggatggcggctgttcaagaagatcagcggcggttccggacctgctgccaagaagaaaaagctggactccggactgcaactgcctccactggaaagactgacactgggagctgccgactacaaggacgacgacgacaagggcggagctagctctaagacaatcgtgctgtctgtgggcgaagccaccagaacactgaccgagatccagagcacagccgacagacagatcttcgaggaaaaagtgggccctctcgtgggcagactgagactgacagcttccctgagacagaacggcgccaagaccgcctacagagtgaacctgaagctggaccaggccgacgtggtggattctggccttcctaaagtgcggtacacccaagtgtggtcccacgacgtgaccatcgtggccaattctaccgaggccagcagaaagagcctgtacgacctgaccaagagcctggtggccacaagccaggtggaagatctggtcgtgaacctggtgcctctcggacgtggcggcagcgctggcggactccagagcagacctgaacctacagctccaccagaggaatccttccgcagcggcgtggaaaccacaacacctccacagaagcaagagcccatcgacaaagagctgtaccctctgaccagcctgagaagcctgttcggcaacgatcccagcagccagtaa

SEQ ID NO: 102 - DNA, 1611 bp, Synthetic construct
  source 1..1611: mol_type = other DNA
atgcacggcctgcaggacgaccctgatctgcaggccctgctgaagggcagccagctgctgaaagtgaagtccagcagctggcggcgggaaagattctacaagctgcaagaggactgcaagaccatctggcaggagtctagaaaggtgatgcgctccccagaaagccaactgttcagcatcgaggacatccaggaggtgcggatgggccacagaacagagggactggaaaagttcgccagagatatccccgaggatagatgttttagcattgtgttcaaggaccagcggaacaccctggacctgatcgcccctagccctgctgatgcccagcattgggtccagggcctcagaaagatcatccaccacagcggctctatggaccagagacagaaactgcagaccggtgctagagcatctgttctgtctggcggagcacagcaggccgctgctgatacaggccactctaatcaggtgtcccagaactacagccccacctccatcctggacatcagacagggccccaaagagcccttccgggactacgtggacagattctacaagaccctgagagccgagcaggccagccaagaagtgaagaactggatgaccgagacactgctggtgcagaacgccaatcctgactgcaagaccatcctgaaggctctgggacctgccgccacactggaagagatgatgacagcctgtcaaggcgttggcggccctggacacaaagctagagttctggccgaggccatgagccaagtgaccaactccgctaccatcatgggaggatccggcggcagaatgaagcagctggaagataaggtggaagaactgctgagcaagaactaccacctggaaaacgaggtggcccggctgaagaagctcgttggagaaagaggtggcagcggcggagtttctggatggcggctgttcaagaagatcagcggcggttccggacctgctgccaaaagagtgaaactggactccggactgcaactgcctccactggaaagactgacactgggagctgccgactacaaggacgacgacgacaagggcggagctagctctaagacaatcgtgctgtctgtgggcgaagccaccagaacactgaccgagatccagagcacagccgacagacagatcttcgaggaaaaagtgggccctctcgtgggcagactgagactgacagcttccctgagacagaacggcgccaagaccgcctacagagtgaacctgaagctggaccaggccgacgtggtggattctggccttcctaaagtgcggtacacccaagtgtggtcccacgacgtgaccatcgtggccaattctaccgaggccagcagaaagagcctgtacgacctgaccaagagcctggtggccacaagccaggtggaagatctggtcgtgaacctggtgcctctcggacgtggcggcagcgctggcggactccagagcagacctgaacctacagctccaccagaggaatccttccgcagcggcgtggaaaccacaacacctccacagaagcaagagcccatcgacaaagagctgtaccctctgaccagcctgagaagcctgttcggcaacgatcccagcagccagtaa

SEQ ID NO: 103 - DNA, 1611 bp, Synthetic construct
  source 1..1611: mol_type = other DNA
atgcacggcctgcaggacgaccctgatctgcaggccctgctgaagggcagccagctgctgaaagtgaagtccagcagctggcggcgggaaagattctacaagctgcaagaggactgcaagaccatctggcaggagtctagaaaggtgatgcgctccccagaaagccaactgttcagcatcgaggacatccaggaggtgcggatgggccacagaacagagggactggaaaagttcgccagagatatccccgaggatagatgttttagcattgtgttcaaggaccagcggaacaccctggacctgatcgcccctagccctgctgatgcccagcattgggtccagggcctcagaaagatcatccaccacagcggctctatggaccagagacagaaactgcagaccggtgctagagcatctgttctgtctggcggagcacagcaggccgctgctgatacaggccactctaatcaggtgtcccagaactacagccccacctccatcctggacatcagacagggccccaaagagcccttccgggactacgtggacagattctacaagaccctgagagccgagcaggccagccaagaagtgaagaactggatgaccgagacactgctggtgcagaacgccaatcctgactgcaagaccatcctgaaggctctgggacctgccgccacactggaagagatgatgacagcctgtcaaggcgttggcggccctggacacaaagctagagttctggccgaggccatgagccaagtgaccaactccgctaccatcatgggaggatccggcggcagaatgaagcagctggaagataaggtggaagaactgctgagcaagaactaccacctggaaaacgaggtggcccggctgaagaagctcgttggagaaagaggtggcagcggcggagtttctggatggcggctgttcaagaagatcagcggcggttccggacctgctgccaagaagaaaaagaacggctccggactgcaactgcctccactggaaagactgacactgggagctgccgactacaaggacgacgacgacaagggcggagctagctctaagacaatcgtgctgtctgtgggcgaagccaccagaacactgaccgagatccagagcacagccgacagacagatcttcgaggaaaaagtgggccctctcgtgggcagactgagactgacagcttccctgagacagaacggcgccaagaccgcctacagagtgaacctgaagctggaccaggccgacgtggtggattctggccttcctaaagtgcggtacacccaagtgtggtcccacgacgtgaccatcgtggccaattctaccgaggccagcagaaagagcctgtacgacctgaccaagagcctggtggccacaagccaggtggaagatctggtcgtgaacctggtgcctctcggacgtggcggcagcgctggcggactccagagcagacctgaacctacagctccaccagaggaatccttccgcagcggcgtggaaaccacaacacctccacagaagcaagagcccatcgacaaagagctgtaccctctgaccagcctgagaagcctgttcggcaacgatcccagcagccagtaa

SEQ ID NO: 104 - DNA, 1605 bp, Synthetic construct
  source 1..1605: mol_type = other DNA
atgcacggcctgcaggacgaccctgatctgcaggccctgctgaagggcagccagctgctgaaagtgaagtccagcagctggcggcgggaaagattctacaagctgcaagaggactgcaagaccatctggcaggagtctagaaaggtgatgcgctccccagaaagccaactgttcagcatcgaggacatccaggaggtgcggatgggccacagaacagagggactggaaaagttcgccagagatatccccgaggatagatgttttagcattgtgttcaaggaccagcggaacaccctggacctgatcgcccctagccctgctgatgcccagcattgggtccagggcctcagaaagatcatccaccacagcggctctatggaccagagacagaaactgcagaccggtgctagagcatctgttctgtctggcggagcacagcaggccgctgctgatacaggccactctaatcaggtgtcccagaactacagccccacctccatcctggacatcagacagggccccaaagagcccttccgggactacgtggacagattctacaagaccctgagagccgagcaggccagccaagaagtgaagaactggatgaccgagacactgctggtgcagaacgccaatcctgactgcaagaccatcctgaaggctctgggacctgccgccacactggaagagatgatgacagcctgtcaaggcgttggcggccctggacacaaagctagagttctggccgaggccatgagccaagtgaccaactccgctaccatcatgggaggatccggcggcagaatgaagcagctggaagataaggtggaagaactgctgagcaagaactaccacctggaaaacgaggtggcccggctgaagaagctcgttggagaaagaggtggcagcggcggagtttctggatggcggctgttcaagaagatcagcggcggttccggacctaagaagaaaagaaaggtgtccggactgcaactgcctccactggaaagactgacactgggagctgccgactacaaggacgacgacgacaagggcggagctagctctaagacaatcgtgctgtctgtgggcgaagccaccagaacactgaccgagatccagagcacagccgacagacagatcttcgaggaaaaagtgggccctctcgtgggcagactgagactgacagcttccctgagacagaacggcgccaagaccgcctacagagtgaacctgaagctggaccaggccgacgtggtggattctggccttcctaaagtgcggtacacccaagtgtggtcccacgacgtgaccatcgtggccaattctaccgaggccagcagaaagagcctgtacgacctgaccaagagcctggtggccacaagccaggtggaagatctggtcgtgaacctggtgcctctcggacgtggcggcagcgctggcggactccagagcagacctgaacctacagctccaccagaggaatccttccgcagcggcgtggaaaccacaacacctccacagaagcaagagcccatcgacaaagagctgtaccctctgaccagcctgagaagcctgttcggcaacgatcccagcagccagtaa

SEQ ID NO: 105 - DNA, 2250 bp, Synthetic construct
  source 1..2250: mol_type = other DNA
atgggcgctagagcctctgttctgtctggcggcgaactggacagatgggagaagatcagaagcagacctggcggcaagaagaagtacaagctgaagcacatcgtgtgggccagcagagagctggaaagattcgctgtgaaccccggcctgctggaaacaagcgagggctgtagacagatcctgggccagctccagccatctctccagacaggatctgaggaactgagaagcctgtacaacaccgtggccacactgtactgcgtgcaccagagaatcgagatcaaggacaccaaagaggccctggacaagatcgaggaagaacagaacaagtctaagaagaaggcccagcaggctgccgccgatacaggccactctaatcaggtgtcccagaactaccccatcgtgcagaacatccagggccagatggtgcatcaggctatcagccccagaacactgaacgcctgggtcaaagtggtggaagagaaggctttcagccctgaagtgatccccatgttcagcgccctgtctgagggtgccacacctcaggacctgaacaccatgctgaacacagtcggcggacaccaggccgctatgcagatgctgaaagagacaatcaacgaagaggccgccgagtgggacagagtgcatcctgttcatgctggccctatcgctcccggccagatgagagaacctagaggctctgacattgccggcaccaccagcacactgcaagagcagatcggctggatgacaaacaaccctcctattcctgtgggcgagatctacaagagatggatcatcctgggactgaacaagatcgtgcggatgtacagccccaccagcatcctggacattagacagggccccaaagagcccttcagagactacgtggacagattctacaagaccctgagagccgagcaggccagccaagaagtgaagaactggatgaccgagacactgctggtgcagaacgctaaccccgactgcaagaccatcctgaaggctctgggacctgccgccacactggaagagatgatgacagcctgtcaaggcgtcggaggacctggccataaggctagagttctggccgaggccatgagccaagtgaccaacagcgccacaatcatgatgcagagaggcaacttcagaaaccagcggaagatcgtgaagtccttcaactccggcaaagagggccacaccgcccgcaattctagagcccctagaaagaaaggtggatccggcggcgtttctggatggcggctgttcaagaagatcagcggcggttccggacctgctgccaaaagagtgaaactggactccggactgcaactgcctccactggaaagactgacactgggagctgccccagccgccaagaagaaaaagctggactacaaggacgacgacgacaagggcggagctagccccgggggcggatccggtggaaccgagagacaggccaacttcctgggcaagatctggcctagctacaagggcagacccggcaacttcctccagagcagaccagagcctaccgctcctcctgaggaatccttcagatccggcgtggaaaccaccacacctccacagaagcaagagcccatcgacaaagagctgtaccctctgaccagcctgagatccctgttcggcaacgaccctagctctcaaggcggaggaggtggtatggaccactacctggacatcagactgcggcccgatcctgagtttcctccagctcagctgatgagcgtgctgttcggcaaactgcaccaggctctggttgcccaaggcggcgatagaatcggagtgtcattccccgacctggacgagagcagaagcagactgggagagagactgagaatccacgccagcgccgatgatctgagagccctgcttgctagaccttggctggaaggcctgagagatcacctccagtttggagagcctgccgtggtgcctcatccaacaccatatagacaggtgtccagagtgcaggccaagagcaaccccgaaagactgcggagaaggctgatgcggagacacgacctgtctgaggaagaggcccggaagagaatccccgacacagtggctagagccctggacctgcctttcgtgacactgagaagccagagcaccggccagcacttccggctgtttatcagacacggccctctgcaagtgaccgccgaagaaggcggctttacctgttacggcctgagcaaaggcggattcgtgccctggttttga

SEQ ID NO: 106 - DNA, 2244 bp, Synthetic construct
  source 1..2244: mol_type = other DNA
atgggcgctagagcctctgttctgtctggcggcgaactggacagatgggagaagatcagaagcagacctggcggcaagaagaagtacaagctgaagcacatcgtgtgggccagcagagagctggaaagattcgctgtgaaccccggcctgctggaaacaagcgagggctgtagacagatcctgggccagctccagccatctctccagacaggatctgaggaactgagaagcctgtacaacaccgtggccacactgtactgcgtgcaccagagaatcgagatcaaggacaccaaagaggccctggacaagatcgaggaagaacagaacaagtctaagaagaaggcccagcaggctgccgccgatacaggccactctaatcaggtgtcccagaactaccccatcgtgcagaacatccagggccagatggtgcatcaggctatcagccccagaacactgaacgcctgggtcaaagtggtggaagagaaggctttcagccctgaagtgatccccatgttcagcgccctgtctgagggtgccacacctcaggacctgaacaccatgctgaacacagtcggcggacaccaggccgctatgcagatgctgaaagagacaatcaacgaagaggccgccgagtgggacagagtgcatcctgttcatgctggccctatcgctcccggccagatgagagaacctagaggctctgacattgccggcaccaccagcacactgcaagagcagatcggctggatgacaaacaaccctcctattcctgtgggcgagatctacaagagatggatcatcctgggactgaacaagatcgtgcggatgtacagccccaccagcatcctggacattagacagggccccaaagagcccttcagagactacgtggacagattctacaagaccctgagagccgagcaggccagccaagaagtgaagaactggatgaccgagacactgctggtgcagaacgctaaccccgactgcaagaccatcctgaaggctctgggacctgccgccacactggaagagatgatgacagcctgtcaaggcgtcggaggacctggccataaggctagagttctggccgaggccatgagccaagtgaccaacagcgccacaatcatgatgcagagaggcaacttcagaaaccagcggaagatcgtgaagtccttcaactccggcaaagagggccacaccgcccgcaattctagagcccctagaaagaaaggtggatccggcggcgtttctggatggcggctgttcaagaagatcagcggcggttccggacctgctgccaaaagagtgaaactggactccggactgcaactgcctccactggaaagactgacactgggagctgccccagccgccaagaagaaaaagctggactacaaggacgacgacgacaagggcggagctagccccgggggcggtggtatggaccactacctggacatcagactgcggcccgatcctgagtttcctccagctcagctgatgagcgtgctgttcggcaaactgcaccaggctctggttgcccaaggcggcgatagaatcggagtgtcattccccgacctggacgagagcagaagcagactgggagagagactgagaatccacgccagcgccgatgatctgagagccctgcttgctagaccttggctggaaggcctgagagatcacctccagtttggagagcctgccgtggtgcctcatccaacaccatatagacaggtgtccagagtgcaggccaagagcaaccccgaaagactgcggagaaggctgatgcggagacacgacctgtctgaggaagaggcccggaagagaatccccgacacagtggctagagccctggacctgcctttcgtgacactgagaagccagagcaccggccagcacttccggctgtttatcagacacggccctctgcaagtgaccgccgaagaaggcggctttacctgttacggcctgagcaaaggcggattcgtgccctggtttggcggatccggtggaaccgagagacaggccaacttcctgggcaagatctggcctagctacaagggcagacccggcaacttcctccagagcagaccagagcctaccgctcctcctgaggaatccttcagatccggcgtggaaaccaccacacctccacagaagcaagagcccatcgacaaagagctgtaccctctgaccagcctgagatccctgttcggcaacgaccctagctctcaatga

SEQ ID NO: 107 - DNA, 4307 bp, Synthetic construct
  source 1..4307: mol_type = other DNA
atgggtgcgagagcgtcagtattaagcgggggagaattagatcgatgggaaaaaattcggttaaggccagggggaaagaaaaaatataaattaaaacatatagtatgggcaagcagggagctagaacgattcgcagttaatcctggcctgttagaaacatcagaaggctgtagacaaatactgggacagctacaaccatcccttcagacaggatcagaagaacttagatcattatataatacagtagcaaccctctattgtgtgcatcaaaggatagagataaaagacaccaaggaagctttagacaagatagaggaagagcaaaacaaaagtaagaaaaaagcacagcaagcagcagctgacacaggacacagcaatcaggtcagccaaaattaccctatagtgcagaacatccaggggcaaatggtacatcaggccatatcacctagaactttaaatgcatgggtaaaagtagtagaagagaaggctttcagcccagaagtgatacccatgttttcagcattatcagaaggagccaccccacaagatttaaacaccatgctaaacacagtggggggacatcaagcagccatgcaaatgttaaaagagaccatcaatgaggaagctgcagaatgggatagagtgcatccagtgcatgcagggcctattgcaccaggccagatgagagaaccaaggggaagtgacatagcaggaactactagtacccttcaggaacaaataggatggatgacacataatccacctatcccagtaggagaaatctataaaagatggataatcctgggattaaataaaatagtaagaatgtatagccctaccagcattctggacataagacaaggaccaaaggaaccctttagagactatgtagaccgattctataaaactctaagagccgagcaagcttcacaagaggtaaaaaattggatgacagaaaccttgttggtccaaaatgcgaacccagattgtaagactattttaaaagcattgggaccaggagcgacactagaagaaatgatgacagcatgtcagggagtggggggacccggccataaagcaagagttttggctgaagcaatgagccaagtaacaaatccagctaccataatgatacagaaaggcaattttaggaaccaaagaaagactgttaagtgtttcaattgtggcaaagaagggcacatagccaaaaattgcagggcccctaggaaaaagggctgttggaaatgtggaaaggaaggacaccaaatgaaagattgtactgagagacaggctaattttttagggaagatctggccttcccacaagggaaggccagggaattttcttcagagcagaccagagccaacagccccaccagaagagagcttcaggtttggggaagagacaacaactccctctcagaagcaggagccgatagacaaggaactgtatcctttagcttccctcagatcactctttggcagcgacccctcgtcacaataaagataggggggcaattaaaggaagctctattagatacaggagcagatgatacagtattagaagaaatgaatttgccaggaagatggaaaccaaaaatgatagggggaattggaggttttatcaaagtaagacagtatgatcagatactcatagaaatctgcggacataaagctataggtacagtattagtaggacctacacctgtcaacataattggaagaaatctgttgactcagattggctgcactttaaattttcccattagtcctattgagactgtaccagtaaaattaaagccaggaatggatggcccaaaagttaaacaatggccattgacagaagaaaaaataaaagcattagtagaaatttgtacagaaatggaaaaggaaggaaaaatttcaaaaattgggcctgaaaatccatacaatactccagtatttgccataaagaaaaaagacagtactaaatggagaaaattagtagatttcagagaacttaataagagaactcaagatttctgggaagttcaattaggaataccacatcctgcagggttaaaacagaaaaaatcagtaacagtactggatgtgggcgatgcatatttttcagttcccttagataaagacttcaggaagtatactgcatttaccatacctagtataaacaatgagacaccagggattagatatcagtacaatgtgcttccacagggatggaaaggatcaccagcaatattccagtgtagcatgacaaaaatcttagagccttttagaaaacaaaatccagacatagtcatctatcaatacatggatgatttgtatgtaggatctgacttagaaatagggcagcatagaacaaaaatagaggaactgagacaacatctgttgaggtggggatttaccacaccagacaaaaaacatcagaaagaacctccattcctttggatgggttatgaactccatcctgataaatggacagtacagcctatagtgctgccagaaaaggacagctggactgtcaatgacatacagaaattagtgggaaaattgaattgggcaagtcagatttatgcagggattaaagtaaggcaattatgtaaacttcttaggggaaccaaagcactaacagaagtagtaccactaacagaagaagcagagctagaactggcagaaaacagggagattctaaaagaaccggtacatggagtgtattatgacccatcaaaagacttaatagcagaaatacagaagcaggggcaaggccaatggacatatcaaatttatcaagagccatttaaaaatctgaaaacaggaaagtatgcaagaatgaagggtgcccacactaatgatgtgaaacaattaacagaggcagtacaaaaaatagccacagaaagcatagtaatatggggaaagactcctaaatttaaattacccatacaaaaggaaacatgggaagcatggtggacagagtattggcaagccacctggattcctgagtgggagtttgtcaatacccctcccttagtgaagttatggtaccagttagagaaagaacccataataggagcagaaactttctatgtagatggggcagccaatagggaaactaaattaggaaaagcaggatatgtaactgacagaggaagacaaaaagttgtccccctaacggacacaacaaatcagaagactgagttacaagcaattcatctagctttgcaggattcgggattagaagtaaacatagtgacagactcacaatatgcattgggaatcattcaagcacaaccagataagagtgaatcagagttagtcagtcaaataatagagcagttaataaaaaaggaaaaagtctacctggcatgggtaccagcacacaaaggaattggaggaaatgaacaagtagataaattggtcagtgctggaatcaggaaagtactatttttagatggaatagataaggcccaagaagaacatgagaaatatcacagtaattggagagcaatggctagtgattttaacctaccacctgtagtagcaaaagaaatagtagccagctgtgataaatgtcagctaaaaggggaagccatgcatggacaagtagactgtagcccaggaatatggcagctagtttgtacacatttagaaggaaaagttatcttggtagcagttcatgtagccagtggatatatagaagcagaagtaattccagcagagacagggcaagaaacagcatacttcctcttaaaattagcaggaagatggccagtaaaaacagtacatacagacaatggcagcaatttcaccagtactacagttaaggccgcctgttggtgggcggggatcaagcaggaatttggcattccctacaatccccaaagtcaaggagtaatagaatctatgaataaagaattaaagaaaattataggacaggtaagagatcaggctgaacatcttaagacagcagtacaaatggcagtattcatccacaattttaaaagaaaaggggggattggggggtacagtgcaggggaaagaatagtagacataatagcaacagacatacaaactaaagaattacaaaaacaaattacaaaaattcaaaattttcgggtttattacagggacagcagagatccagtttggaaaggaccagcaaagctcctctggaaaggtgaaggggcagtagtaatacaagataatagtgacataaaagtagtgccaagaagaaaagcaaagatcatcagggattatggaaaacagatggcaggtgatgattgtgtggcaagtagacaggatgaggattaa

SEQ ID NO: 108 - DNA, 6411 bp, Synthetic construct
  source 1..6411: mol_type = other DNA
atggacaagaagtacagcatcggcctggacatcggcaccaactctgtgggctgggccgtgatcaccgacgagtacaaggtgcccagcaagaaattcaaggtgctgggcaacaccgaccggcacagcatcaagaagaacctgatcggagccctgctgttcgacagcggcgaaacagccgaggccacccggctgaagagaaccgccagaagaagatacaccagacggaagaaccggatctgctatctgcaagagatcttcagcaacgagatggccaaggtggacgacagcttcttccacagactggaagagtccttcctggtggaagaggataagaagcacgagcggcaccccatcttcggcaacatcgtggacgaggtggcctaccacgagaagtaccccaccatctaccacctgagaaagaaactggtggacagcaccgacaaggccgacctgcggctgatctatctggccctggcccacatgatcaagttccggggccacttcctgatcgagggcgacctgaaccccgacaacagcgacgtggacaagctgttcatccagctggtgcagacctacaaccagctgttcgaggaaaaccccatcaacgccagcggcgtggacgccaaggccatcctgtctgccagactgagcaagagcagacggctggaaaatctgatcgcccagctgcccggcgagaagaagaatggcctgttcggcaacctgattgccctgagcctgggcctgacccccaacttcaagagcaacttcgacctggccgaggatgccaaactgcagctgagcaaggacacctacgacgacgacctggacaacctgctggcccagatcggcgaccagtacgccgacctgtttctggccgccaagaacctgtccgacgccatcctgctgagcgacatcctgagagtgaacaccgagatcaccaaggcccccctgagcgcctctatgatcaagagatacgacgagcaccaccaggacctgaccctgctgaaagctctcgtgcggcagcagctgcctgagaagtacaaagagattttcttcgaccagagcaagaacggctacgccggctacattgacggcggagccagccaggaagagttctacaagttcatcaagcccatcctggaaaagatggacggcaccgaggaactgctcgtgaagctgaacagagaggacctgctgcggaagcagcggaccttcgacaacggcagcatcccccaccagatccacctgggagagctgcacgccattctgcggcggcaggaagatttttacccattcctgaaggacaaccgggaaaagatcgagaagatcctgaccttccgcatcccctactacgtgggccctctggccaggggaaacagcagattcgcctggatgaccagaaagagcgaggaaaccatcaccccctggaacttcgaggaagtggtggacaagggcgcttccgcccagagcttcatcgagcggatgaccaacttcgataagaacctgcccaacgagaaggtgctgcccaagcacagcctgctgtacgagtacttcaccgtgtataacgagctgaccaaagtgaaatacgtgaccgagggaatgagaaagcccgccttcctgagcggcgagcagaaaaaggccatcgtggacctgctgttcaagaccaaccggaaagtgaccgtgaagcagctgaaagaggactacttcaagaaaatcgagtgcttcgactccgtggaaatctccggcgtggaagatcggttcaacgcctccctgggcacataccacgatctgctgaaaattatcaaggacaaggacttcctggacaatgaggaaaacgaggacattctggaagatatcgtgctgaccctgacactgtttgaggacagagagatgatcgaggaacggctgaaaacctatgcccacctgttcgacgacaaagtgatgaagcagctgaagcggcggagatacaccggctggggcaggctgagccggaagctgatcaacggcatccgggacaagcagtccggcaagacaatcctggatttcctgaagtccgacggcttcgccaacagaaacttcatgcagctgatccacgacgacagcctgacctttaaagaggacatccagaaagcccaggtgtccggccagggcgatagcctgcacgagcacattgccaatctggccggcagccccgccattaagaagggcatcctgcagacagtgaaggtggtggacgagctcgtgaaagtgatgggccggcacaagcccgagaacatcgtgatcgaaatggccagagagaaccagaccacccagaagggacagaagaacagccgcgagagaatgaagcggatcgaagagggcatcaaagagctgggcagccagatcctgaaagaacaccccgtggaaaacacccagctgcagaacgagaagctgtacctgtactacctgcagaatgggcgggatatgtacgtggaccaggaactggacatcaaccggctgtccgactacgatgtggaccatatcgtgcctcagagctttctgaaggacgactccatcgacaacaaggtgctgaccagaagcgacaaggcccggggcaagagcgacaacgtgccctccgaagaggtcgtgaagaagatgaagaactactggcggcagctgctgaacgccaagctgattacccagagaaagttcgacaatctgaccaaggccgagagaggcggcctgagcgaactggataaggccggcttcatcaagagacagctggtggaaacccggcagatcacaaagcacgtggcacagatcctggactcccggatgaacactaagtacgacgagaatgacaagctgatccgggaagtgaaagtgatcaccctgaagtccaagctggtgtccgatttccggaaggatttccagttttacaaagtgcgcgagatcaacaactaccaccacgcccacgacgcctacctgaacgccgtcgtgggaaccgccctgatcaaaaagtaccctaagctggaaagcgagttcgtgtacggcgactacaaggtgtacgacgtgcggaagatgatcgccaagagcgagcaggaaatcggcaaggctaccgccaagtacttcttctacagcaacatcatgaactttttcaagaccgagattaccctggccaacggcgagatccggaagcggcctctgatcgagacaaacggcgaaaccggggagatcgtgtgggataagggccgggattttgccaccgtgcggaaagtgctgagcatgccccaagtgaatatcgtgaaaaagaccgaggtgcagacaggcggcttcagcaaagagtctatcctgcccaagaggaacagcgataagctgatcgccagaaagaaggactgggaccctaagaagtacggcggcttcgacagccccaccgtggcctattctgtgctggtggtggccaaagtggaaaagggcaagtccaagaaactgaagagtgtgaaagagctgctggggatcaccatcatggaaagaagcagcttcgagaagaatcccatcgactttctggaagccaagggctacaaagaagtgaaaaaggacctgatcatcaagctgcctaagtactccctgttcgagctggaaaacggccggaagagaatgctggcctctgccggcgaactgcagaagggaaacgaactggccctgccctccaaatatgtgaacttcctgtacctggccagccactatgagaagctgaagggctcccccgaggataatgagcagaaacagctgtttgtggaacagcacaagcactacctggacgagatcatcgagcagatcagcgagttctccaagagagtgatcctggccgacgctaatctggacaaagtgctgtccgcctacaacaagcaccgggataagcccatcagagagcaggccgagaatatcatccacctgtttaccctgaccaatctgggagcccctgccgccttcaagtactttgacaccaccatcgaccggaagaggtacaccagcaccaaagaggtgctggacgccaccctgatccaccagagcatcaccggcctgtacgagacacggatcgacctgtctcagctgggaggcgacgcctatccctatgacgtgcccgattatgccagcctgggctccggatcccccaagaagaaacgcaaggtggaagatggcgagggcccagccgctaagagagtgaaactggattccggagctgctcctgccgccaagaagaagaaactcgacaccggtggacctggaagcgagcctgctacatctggctctgagacacctggcacctccgagtctgctacacctgaatctggacctggcgctagcaccctgaacatcgaggacgagtaccggctgcacgagacaagcaaagaacccgatgtgtccctgggcagcacctggcttagtgatttccctcaggcctgggccgagacaggcggaatgggacttgctgttagacaggcccctctgatcatccctctgaaggccacaagcacccctgtgtccatcaagcagtaccccatgagccaagaggcccggctgggaatcaagccccacattcagagactgctggaccagggcatcctggtgccttgtcagagcccttggaatacccctctgctgcccgtgaagaagcccggcaccaacgattacagacccgtgcaggacctgcgggaagtgaacaagagagtggaagatattcaccccaccgtgccgaatccttacaacctgctgtctggcctgcctcctagccaccagtggtacacagtgctggacctgaaggacgccttcttctgtctgcggctgcaccctacaagccagcctctgtttgcctttgagtggcgggaccctgagatgggcattagcggacagctgacctggaccagactgccccagggcttcaagaacagccccacactgttcaacgaggccctgcatagggacctcgccgacttcagaatccagcatcctgacctgatcctgctccagtacgtggacgatctgctgctggccgctacaagcgagctggattgtcagcagggaacaagagccctgctgcaaaccctgggcaacctgggctatagagcctctgccaagaaggcccagatttgccagaaacaagtgaagtatctgggctacctgctgaaagagggccagcgttggctgaccgaggccagaaaagaaaccgtgatgggccagcctacacctaagacacccagacagctgagagagttcctgggcaaagccggattctgtcggctgttcatccctggctttgccgagatggctgcccctctgtacccactgacaaagcccggaactctgttcaactggggcccagatcagcagaaggcctaccaagagatcaagcaggctctgctgacagcccctgctctgggactgcctgatctgaccaagcctttcgagctgttcgtggacgagaagcagggctatgccaaaggcgtgctgacacagaagctcggcccttggagaaggcctgtggcctacctgagcaagaaactggaccctgtggctgccggatggcctccttgtctgagaatggtggccgccattgccgtgctgaccaaggatgccggaaagctgacaatgggacagcctctggtcattctggcccctcatgccgtggaagccctcgtgaaacagcctcctgatcggtggctgagcaacgccaggatgacacactatcaggcactgctgctcgacaccgacagagtgcagtttggacctgtggtggccctgaatcctgccacacttctgcctctgcctgaggaaggcctccagcacaattgcctggacatcctggccgaggctcacggcacaagacccgatctgacagatcagccactgcctgacgccgaccacacctggtatacagatggcagctctctgctgcaagaaggacagagaaaagccggggctgccgtgaccaccgagacagaagtgatttgggccaaagctctgcccgctggcacatctgctcagagagccgaactgatcgccctgacacaggccctgaaaatggccgagggcaagaagctgaacgtctacaccgactccagatacgccttcgccaccgctcacatccacggcgaaatctatcggcggagaggatggctgaccagcgagggcaaagagattaagaacaaggacgagattctcgccctgctcaaggccctgttcctgcctaagcggctgagcatcatccactgtccaggccaccagaagggccactctgctgaagctagaggcaacagaatggccgaccaggctgccagaaaggccgccatcacagagacacccgataccagcacactgctgatcgagaacagcagccctggtacccctaagaagaagcggaaagtggactga

SEQ ID NO: 109 - DNA, 5841 bp, Synthetic construct
  source 1..5841: mol_type = other DNA
atggacaagaagtacagcatcggcctggacatcggcaccaactctgtgggctgggccgtgatcaccgacgagtacaaggtgcccagcaagaaattcaaggtgctgggcaacaccgaccggcacagcatcaagaagaacctgatcggagccctgctgttcgacagcggcgaaacagccgaggccacccggctgaagagaaccgccagaagaagatacaccagacggaagaaccggatctgctatctgcaagagatcttcagcaacgagatggccaaggtggacgacagcttcttccacagactggaagagtccttcctggtggaagaggataagaagcacgagcggcaccccatcttcggcaacatcgtggacgaggtggcctaccacgagaagtaccccaccatctaccacctgagaaagaaactggtggacagcaccgacaaggccgacctgcggctgatctatctggccctggcccacatgatcaagttccggggccacttcctgatcgagggcgacctgaaccccgacaacagcgacgtggacaagctgttcatccagctggtgcagacctacaaccagctgttcgaggaaaaccccatcaacgccagcggcgtggacgccaaggccatcctgtctgccagactgagcaagagcagacggctggaaaatctgatcgcccagctgcccggcgagaagaagaatggcctgttcggcaacctgattgccctgagcctgggcctgacccccaacttcaagagcaacttcgacctggccgaggatgccaaactgcagctgagcaaggacacctacgacgacgacctggacaacctgctggcccagatcggcgaccagtacgccgacctgtttctggccgccaagaacctgtccgacgccatcctgctgagcgacatcctgagagtgaacaccgagatcaccaaggcccccctgagcgcctctatgatcaagagatacgacgagcaccaccaggacctgaccctgctgaaagctctcgtgcggcagcagctgcctgagaagtacaaagagattttcttcgaccagagcaagaacggctacgccggctacattgacggcggagccagccaggaagagttctacaagttcatcaagcccatcctggaaaagatggacggcaccgaggaactgctcgtgaagctgaacagagaggacctgctgcggaagcagcggaccttcgacaacggcagcatcccccaccagatccacctgggagagctgcacgccattctgcggcggcaggaagatttttacccattcctgaaggacaaccgggaaaagatcgagaagatcctgaccttccgcatcccctactacgtgggccctctggccaggggaaacagcagattcgcctggatgaccagaaagagcgaggaaaccatcaccccctggaacttcgaggaagtggtggacaagggcgcttccgcccagagcttcatcgagcggatgaccaacttcgataagaacctgcccaacgagaaggtgctgcccaagcacagcctgctgtacgagtacttcaccgtgtataacgagctgaccaaagtgaaatacgtgaccgagggaatgagaaagcccgccttcctgagcggcgagcagaaaaaggccatcgtggacctgctgttcaagaccaaccggaaagtgaccgtgaagcagctgaaagaggactacttcaagaaaatcgagtgcttcgactccgtggaaatctccggcgtggaagatcggttcaacgcctccctgggcacataccacgatctgctgaaaattatcaaggacaaggacttcctggacaatgaggaaaacgaggacattctggaagatatcgtgctgaccctgacactgtttgaggacagagagatgatcgaggaacggctgaaaacctatgcccacctgttcgacgacaaagtgatgaagcagctgaagcggcggagatacaccggctggggcaggctgagccggaagctgatcaacggcatccgggacaagcagtccggcaagacaatcctggatttcctgaagtccgacggcttcgccaacagaaacttcatgcagctgatccacgacgacagcctgacctttaaagaggacatccagaaagcccaggtgtccggccagggcgatagcctgcacgagcacattgccaatctggccggcagccccgccattaagaagggcatcctgcagacagtgaaggtggtggacgagctcgtgaaagtgatgggccggcacaagcccgagaacatcgtgatcgaaatggccagagagaaccagaccacccagaagggacagaagaacagccgcgagagaatgaagcggatcgaagagggcatcaaagagctgggcagccagatcctgaaagaacaccccgtggaaaacacccagctgcagaacgagaagctgtacctgtactacctgcagaatgggcgggatatgtacgtggaccaggaactggacatcaaccggctgtccgactacgatgtggaccatatcgtgcctcagagctttctgaaggacgactccatcgacaacaaggtgctgaccagaagcgacaaggcccggggcaagagcgacaacgtgccctccgaagaggtcgtgaagaagatgaagaactactggcggcagctgctgaacgccaagctgattacccagagaaagttcgacaatctgaccaaggccgagagaggcggcctgagcgaactggataaggccggcttcatcaagagacagctggtggaaacccggcagatcacaaagcacgtggcacagatcctggactcccggatgaacactaagtacgacgagaatgacaagctgatccgggaagtgaaagtgatcaccctgaagtccaagctggtgtccgatttccggaaggatttccagttttacaaagtgcgcgagatcaacaactaccaccacgcccacgacgcctacctgaacgccgtcgtgggaaccgccctgatcaaaaagtaccctaagctggaaagcgagttcgtgtacggcgactacaaggtgtacgacgtgcggaagatgatcgccaagagcgagcaggaaatcggcaaggctaccgccaagtacttcttctacagcaacatcatgaactttttcaagaccgagattaccctggccaacggcgagatccggaagcggcctctgatcgagacaaacggcgaaaccggggagatcgtgtgggataagggccgggattttgccaccgtgcggaaagtgctgagcatgccccaagtgaatatcgtgaaaaagaccgaggtgcagacaggcggcttcagcaaagagtctatcctgcccaagaggaacagcgataagctgatcgccagaaagaaggactgggaccctaagaagtacggcggcttcgacagccccaccgtggcctattctgtgctggtggtggccaaagtggaaaagggcaagtccaagaaactgaagagtgtgaaagagctgctggggatcaccatcatggaaagaagcagcttcgagaagaatcccatcgactttctggaagccaagggctacaaagaagtgaaaaaggacctgatcatcaagctgcctaagtactccctgttcgagctggaaaacggccggaagagaatgctggcctctgccggcgaactgcagaagggaaacgaactggccctgccctccaaatatgtgaacttcctgtacctggccagccactatgagaagctgaagggctcccccgaggataatgagcagaaacagctgtttgtggaacagcacaagcactacctggacgagatcatcgagcagatcagcgagttctccaagagagtgatcctggccgacgctaatctggacaaagtgctgtccgcctacaacaagcaccgggataagcccatcagagagcaggccgagaatatcatccacctgtttaccctgaccaatctgggagcccctgccgccttcaagtactttgacaccaccatcgaccggaagaggtacaccagcaccaaagaggtgctggacgccaccctgatccaccagagcatcaccggcctgtacgagacacggatcgacctgtctcagctgggaggcgacgcctatccctatgacgtgcccgattatgccagcctgggctccggatcccccaagaagaaacgcaaggtggaagatggcgagggcccagccgctaagagagtgaaactggattccggagctgctcctgccgccaagaagaagaaactcgacaccggtggacctggaagcgagcctgctacatctggctctgagacacctggcacctccgagtctgctacacctgaatctggacctggcgctagcaccctgaacatcgaggacgagtaccggctgcacgagacaagcaaagaacccgatgtgtccctgggcagcacctggcttagtgatttccctcaggcctgggccgagacaggcggaatgggacttgctgttagacaggcccctctgatcatccctctgaaggccacaagcacccctgtgtccatcaagcagtaccccatgagccaagaggcccggctgggaatcaagccccacattcagagactgctggaccagggcatcctggtgccttgtcagagcccttggaatacccctctgctgcccgtgaagaagcccggcaccaacgattacagacccgtgcaggacctgcgggaagtgaacaagagagtggaagatattcaccccaccgtgccgaatccttacaacctgctgtctggcctgcctcctagccaccagtggtacacagtgctggacctgaaggacgccttcttctgtctgcggctgcaccctacaagccagcctctgtttgcctttgagtggcgggaccctgagatgggcattagcggacagctgacctggaccagactgccccagggcttcaagaacagccccacactgttcaacgaggccctgcatagggacctcgccgacttcagaatccagcatcctgacctgatcctgctccagtacgtggacgatctgctgctggccgctacaagcgagctggattgtcagcagggaacaagagccctgctgcaaaccctgggcaacctgggctatagagcctctgccaagaaggcccagatttgccagaaacaagtgaagtatctgggctacctgctgaaagagggccagcgttggctgaccgaggccagaaaagaaaccgtgatgggccagcctacacctaagacacccagacagctgagagagttcctgggcaaagccggattctgtcggctgttcatccctggctttgccgagatggctgcccctctgtacccactgacaaagcccggaactctgttcaactggggcccagatcagcagaaggcctaccaagagatcaagcaggctctgctgacagcccctgctctgggactgcctgatctgaccaagcctttcgagctgttcgtggacgagaagcagggctatgccaaaggcgtgctgacacagaagctcggcccttggagaaggcctgtggcctacctgagcaagaaactggaccctgtggctgccggatggcctccttgtctgagaatggtggccgccattgccgtgctgaccaaggatgccggaaagctgacaatgggacagcctctggtcattctggcccctcatgccgtggaagccctcgtgaaacagcctcctgatcggtggctgagcaacgccaggatgacacactatcaggcactgctgctcgacaccgacagagtgcagtttggacctgtggtggccctgaatcctgccacacttctgcctctgcctgaggaaggcctccagcacaattcgcgtaaatga

SEQ ID NO: 110 - DNA, 6417 bp, Synthetic construct
  source 1..6417: mol_type = other DNA
atgaccctgaacatcgaggacgagtaccggctgcacgagacaagcaaagaacccgatgtgtccctgggcagcacctggcttagtgatttccctcaggcctgggccgagacaggcggaatgggacttgctgttagacaggcccctctgatcatccctctgaaggccacaagcacccctgtgtccatcaagcagtaccccatgagccaagaggcccggctgggaatcaagccccacattcagagactgctggaccagggcatcctggtgccttgtcagagcccttggaatacccctctgctgcccgtgaagaagcccggcaccaacgattacagacccgtgcaggacctgcgggaagtgaacaagagagtggaagatattcaccccaccgtgccgaatccttacaacctgctgtctggcctgcctcctagccaccagtggtacacagtgctggacctgaaggacgccttcttctgtctgcggctgcaccctacaagccagcctctgtttgcctttgagtggcgggaccctgagatgggcattagcggacagctgacctggaccagactgccccagggcttcaagaacagccccacactgttcaacgaggccctgcatagggacctcgccgacttcagaatccagcatcctgacctgatcctgctccagtacgtggacgatctgctgctggccgctacaagcgagctggattgtcagcagggaacaagagccctgctgcaaaccctgggcaacctgggctatagagcctctgccaagaaggcccagatttgccagaaacaagtgaagtatctgggctacctgctgaaagagggccagcgttggctgaccgaggccagaaaagaaaccgtgatgggccagcctacacctaagacacccagacagctgagagagttcctgggcaaagccggattctgtcggctgttcatccctggctttgccgagatggctgcccctctgtacccactgacaaagcccggaactctgttcaactggggcccagatcagcagaaggcctaccaagagatcaagcaggctctgctgacagcccctgctctgggactgcctgatctgaccaagcctttcgagctgttcgtggacgagaagcagggctatgccaaaggcgtgctgacacagaagctcggcccttggagaaggcctgtggcctacctgagcaagaaactggaccctgtggctgccggatggcctccttgtctgagaatggtggccgccattgccgtgctgaccaaggatgccggaaagctgacaatgggacagcctctggtcattctggcccctcatgccgtggaagccctcgtgaaacagcctcctgatcggtggctgagcaacgccaggatgacacactatcaggcactgctgctcgacaccgacagagtgcagtttggacctgtggtggccctgaatcctgccacacttctgcctctgcctgaggaaggcctccagcacaattgcctggacatcctggccgaggctcacggcacaagacccgatctgacagatcagccactgcctgacgccgaccacacctggtatacagatggcagctctctgctgcaagaaggacagagaaaagccggggctgccgtgaccaccgagacagaagtgatttgggccaaagctctgcccgctggcacatctgctcagagagccgaactgatcgccctgacacaggccctgaaaatggccgagggcaagaagctgaacgtctacaccgactccagatacgccttcgccaccgctcacatccacggcgaaatctatcggcggagaggatggctgaccagcgagggcaaagagattaagaacaaggacgagattctcgccctgctcaaggccctgttcctgcctaagcggctgagcatcatccactgtccaggccaccagaagggccactctgctgaagctagaggcaacagaatggccgaccaggctgccagaaaggccgccatcacagagacacccgataccagcacactgctgatcgagaacagcagccctggatccacgccgcccaagaagaagagaaaggttgaggacggcgagggcaccggtggacctggaagcgagcctgctacatctggctctgagacacctggcacctccgagtctgctacacctgaatctggacctggcggatccggagacaagaagtacagcatcggcctggacatcggcaccaactctgtgggctgggccgtgatcaccgacgagtacaaggtgcccagcaagaaattcaaggtgctgggcaacaccgaccggcacagcatcaagaagaacctgatcggagccctgctgttcgacagcggcgaaacagccgaggccacccggctgaagagaaccgccagaagaagatacaccagacggaagaaccggatctgctatctgcaagagatcttcagcaacgagatggccaaggtggacgacagcttcttccacagactggaagagtccttcctggtggaagaggataagaagcacgagcggcaccccatcttcggcaacatcgtggacgaggtggcctaccacgagaagtaccccaccatctaccacctgagaaagaaactggtggacagcaccgacaaggccgacctgcggctgatctatctggccctggcccacatgatcaagttccggggccacttcctgatcgagggcgacctgaaccccgacaacagcgacgtggacaagctgttcatccagctggtgcagacctacaaccagctgttcgaggaaaaccccatcaacgccagcggcgtggacgccaaggccatcctgtctgccagactgagcaagagcagacggctggaaaatctgatcgcccagctgcccggcgagaagaagaatggcctgttcggcaacctgattgccctgagcctgggcctgacccccaacttcaagagcaacttcgacctggccgaggatgccaaactgcagctgagcaaggacacctacgacgacgacctggacaacctgctggcccagatcggcgaccagtacgccgacctgtttctggccgccaagaacctgtccgacgccatcctgctgagcgacatcctgagagtgaacaccgagatcaccaaggcccccctgagcgcctctatgatcaagagatacgacgagcaccaccaggacctgaccctgctgaaagctctcgtgcggcagcagctgcctgagaagtacaaagagattttcttcgaccagagcaagaacggctacgccggctacattgacggcggagccagccaggaagagttctacaagttcatcaagcccatcctggaaaagatggacggcaccgaggaactgctcgtgaagctgaacagagaggacctgctgcggaagcagcggaccttcgacaacggcagcatcccccaccagatccacctgggagagctgcacgccattctgcggcggcaggaagatttttacccattcctgaaggacaaccgggaaaagatcgagaagatcctgaccttccgcatcccctactacgtgggccctctggccaggggaaacagcagattcgcctggatgaccagaaagagcgaggaaaccatcaccccctggaacttcgaggaagtggtggacaagggcgcttccgcccagagcttcatcgagcggatgaccaacttcgataagaacctgcccaacgagaaggtgctgcccaagcacagcctgctgtacgagtacttcaccgtgtataacgagctgaccaaagtgaaatacgtgaccgagggaatgagaaagcccgccttcctgagcggcgagcagaaaaaggccatcgtggacctgctgttcaagaccaaccggaaagtgaccgtgaagcagctgaaagaggactacttcaagaaaatcgagtgcttcgactccgtggaaatctccggcgtggaagatcggttcaacgcctccctgggcacataccacgatctgctgaaaattatcaaggacaaggacttcctggacaatgaggaaaacgaggacattctggaagatatcgtgctgaccctgacactgtttgaggacagagagatgatcgaggaacggctgaaaacctatgcccacctgttcgacgacaaagtgatgaagcagctgaagcggcggagatacaccggctggggcaggctgagccggaagctgatcaacggcatccgggacaagcagtccggcaagacaatcctggatttcctgaagtccgacggcttcgccaacagaaacttcatgcagctgatccacgacgacagcctgacctttaaagaggacatccagaaagcccaggtgtccggccagggcgatagcctgcacgagcacattgccaatctggccggcagccccgccattaagaagggcatcctgcagacagtgaaggtggtggacgagctcgtgaaagtgatgggccggcacaagcccgagaacatcgtgatcgaaatggccagagagaaccagaccacccagaagggacagaagaacagccgcgagagaatgaagcggatcgaagagggcatcaaagagctgggcagccagatcctgaaagaacaccccgtggaaaacacccagctgcagaacgagaagctgtacctgtactacctgcagaatgggcgggatatgtacgtggaccaggaactggacatcaaccggctgtccgactacgatgtggacgccatcgtgcctcagagctttctgaaggacgactccatcgacaacaaggtgctgaccagaagcgacaagaaccggggcaagagcgacaacgtgccctccgaagaggtcgtgaagaagatgaagaactactggcggcagctgctgaacgccaagctgattacccagagaaagttcgacaatctgaccaaggccgagagaggcggcctgagcgaactggataaggccggcttcatcaagagacagctggtggaaacccggcagatcacaaagcacgtggcacagatcctggactcccggatgaacactaagtacgacgagaatgacaagctgatccgggaagtgaaagtgatcaccctgaagtccaagctggtgtccgatttccggaaggatttccagttttacaaagtgcgcgagatcaacaactaccaccacgcccacgacgcctacctgaacgccgtcgtgggaaccgccctgatcaaaaagtaccctaagctggaaagcgagttcgtgtacggcgactacaaggtgtacgacgtgcggaagatgatcgccaagagcgagcaggaaatcggcaaggctaccgccaagtacttcttctacagcaacatcatgaactttttcaagaccgagattaccctggccaacggcgagatccggaagcggcctctgatcgagacaaacggcgaaaccggggagatcgtgtgggataagggccgggattttgccaccgtgcggaaagtgctgagcatgccccaagtgaatatcgtgaaaaagaccgaggtgcagacaggcggcttcagcaaagagtctatcctgcccaagaggaacagcgataagctgatcgccagaaagaaggactgggaccctaagaagtacggcggcttcgacagccccaccgtggcctattctgtgctggtggtggccaaagtggaaaagggcaagtccaagaaactgaagagtgtgaaagagctgctggggatcaccatcatggaaagaagcagcttcgagaagaatcccatcgactttctggaagccaagggctacaaagaagtgaaaaaggacctgatcatcaagctgcctaagtactccctgttcgagctggaaaacggccggaagagaatgctggcctctgccggcgaactgcagaagggaaacgaactggccctgccctccaaatatgtgaacttcctgtacctggccagccactatgagaagctgaagggctcccccgaggataatgagcagaaacagctgtttgtggaacagcacaagcactacctggacgagatcatcgagcagatcagcgagttctccaagagagtgatcctggccgacgctaatctggacaaagtgctgtccgcctacaacaagcaccgggataagcccatcagagagcaggccgagaatatcatccacctgtttaccctgaccaatctgggagcccctgccgccttcaagtactttgacaccaccatcgaccggaagaggtacaccagcaccaaagaggtgctggacgccaccctgatccaccagagcatcaccggcctgtacgagacacggatcgacctgtctcagctgggaggcgacggatccacaccacctaagaagaaacggaaggtcgaggacggcgagggccctgctgctaagagagtgaaactggactccggagctgctccagccgccaagaagaagaagctcgactacaaggacgacgacgataagtga

SEQ ID NO: 111 - DNA, 5871 bp, Synthetic construct
  source 1..5871: mol_type = other DNA
atgaccctgaacatcgaggacgagtaccggctgcacgagacaagcaaagaacccgatgtgtccctgggcagcacctggcttagtgatttccctcaggcctgggccgagacaggcggaatgggacttgctgttagacaggcccctctgatcatccctctgaaggccacaagcacccctgtgtccatcaagcagtaccccatgagccaagaggcccggctgggaatcaagccccacattcagagactgctggaccagggcatcctggtgccttgtcagagcccttggaatacccctctgctgcccgtgaagaagcccggcaccaacgattacagacccgtgcaggacctgcgggaagtgaacaagagagtggaagatattcaccccaccgtgccgaatccttacaacctgctgtctggcctgcctcctagccaccagtggtacacagtgctggacctgaaggacgccttcttctgtctgcggctgcaccctacaagccagcctctgtttgcctttgagtggcgggaccctgagatgggcattagcggacagctgacctggaccagactgccccagggcttcaagaacagccccacactgttcaacgaggccctgcatagggacctcgccgacttcagaatccagcatcctgacctgatcctgctccagtacgtggacgatctgctgctggccgctacaagcgagctggattgtcagcagggaacaagagccctgctgcaaaccctgggcaacctgggctatagagcctctgccaagaaggcccagatttgccagaaacaagtgaagtatctgggctacctgctgaaagagggccagcgttggctgaccgaggccagaaaagaaaccgtgatgggccagcctacacctaagacacccagacagctgagagagttcctgggcaaagccggattctgtcggctgttcatccctggctttgccgagatggctgcccctctgtacccactgacaaagcccggaactctgttcaactggggcccagatcagcagaaggcctaccaagagatcaagcaggctctgctgacagcccctgctctgggactgcctgatctgaccaagcctttcgagctgttcgtggacgagaagcagggctatgccaaaggcgtgctgacacagaagctcggcccttggagaaggcctgtggcctacctgagcaagaaactggaccctgtggctgccggatggcctccttgtctgagaatggtggccgccattgccgtgctgaccaaggatgccggaaagctgacaatgggacagcctctggtcattctggcccctcatgccgtggaagccctcgtgaaacagcctcctgatcggtggctgagcaacgccaggatgacacactatcaggcactgctgctcgacaccgacagagtgcagtttggacctgtggtggccctgaatcctgccacacttctgcctctgcctgaggaaggcctccagcacaatagcggatccacgccgcccaagaagaagagaaaggttgaggacggcgagggcaccggtggacctggaagcgagcctgctacatctggctctgagacacctggcacctccgagtctgctacacctgaatctggacctggcggatccggagacaagaagtacagcatcggcctggacatcggcaccaactctgtgggctgggccgtgatcaccgacgagtacaaggtgcccagcaagaaattcaaggtgctgggcaacaccgaccggcacagcatcaagaagaacctgatcggagccctgctgttcgacagcggcgaaacagccgaggccacccggctgaagagaaccgccagaagaagatacaccagacggaagaaccggatctgctatctgcaagagatcttcagcaacgagatggccaaggtggacgacagcttcttccacagactggaagagtccttcctggtggaagaggataagaagcacgagcggcaccccatcttcggcaacatcgtggacgaggtggcctaccacgagaagtaccccaccatctaccacctgagaaagaaactggtggacagcaccgacaaggccgacctgcggctgatctatctggccctggcccacatgatcaagttccggggccacttcctgatcgagggcgacctgaaccccgacaacagcgacgtggacaagctgttcatccagctggtgcagacctacaaccagctgttcgaggaaaaccccatcaacgccagcggcgtggacgccaaggccatcctgtctgccagactgagcaagagcagacggctggaaaatctgatcgcccagctgcccggcgagaagaagaatggcctgttcggcaacctgattgccctgagcctgggcctgacccccaacttcaagagcaacttcgacctggccgaggatgccaaactgcagctgagcaaggacacctacgacgacgacctggacaacctgctggcccagatcggcgaccagtacgccgacctgtttctggccgccaagaacctgtccgacgccatcctgctgagcgacatcctgagagtgaacaccgagatcaccaaggcccccctgagcgcctctatgatcaagagatacgacgagcaccaccaggacctgaccctgctgaaagctctcgtgcggcagcagctgcctgagaagtacaaagagattttcttcgaccagagcaagaacggctacgccggctacattgacggcggagccagccaggaagagttctacaagttcatcaagcccatcctggaaaagatggacggcaccgaggaactgctcgtgaagctgaacagagaggacctgctgcggaagcagcggaccttcgacaacggcagcatcccccaccagatccacctgggagagctgcacgccattctgcggcggcaggaagatttttacccattcctgaaggacaaccgggaaaagatcgagaagatcctgaccttccgcatcccctactacgtgggccctctggccaggggaaacagcagattcgcctggatgaccagaaagagcgaggaaaccatcaccccctggaacttcgaggaagtggtggacaagggcgcttccgcccagagcttcatcgagcggatgaccaacttcgataagaacctgcccaacgagaaggtgctgcccaagcacagcctgctgtacgagtacttcaccgtgtataacgagctgaccaaagtgaaatacgtgaccgagggaatgagaaagcccgccttcctgagcggcgagcagaaaaaggccatcgtggacctgctgttcaagaccaaccggaaagtgaccgtgaagcagctgaaagaggactacttcaagaaaatcgagtgcttcgactccgtggaaatctccggcgtggaagatcggttcaacgcctccctgggcacataccacgatctgctgaaaattatcaaggacaaggacttcctggacaatgaggaaaacgaggacattctggaagatatcgtgctgaccctgacactgtttgaggacagagagatgatcgaggaacggctgaaaacctatgcccacctgttcgacgacaaagtgatgaagcagctgaagcggcggagatacaccggctggggcaggctgagccggaagctgatcaacggcatccgggacaagcagtccggcaagacaatcctggatttcctgaagtccgacggcttcgccaacagaaacttcatgcagctgatccacgacgacagcctgacctttaaagaggacatccagaaagcccaggtgtccggccagggcgatagcctgcacgagcacattgccaatctggccggcagccccgccattaagaagggcatcctgcagacagtgaaggtggtggacgagctcgtgaaagtgatgggccggcacaagcccgagaacatcgtgatcgaaatggccagagagaaccagaccacccagaagggacagaagaacagccgcgagagaatgaagcggatcgaagagggcatcaaagagctgggcagccagatcctgaaagaacaccccgtggaaaacacccagctgcagaacgagaagctgtacctgtactacctgcagaatgggcgggatatgtacgtggaccaggaactggacatcaaccggctgtccgactacgatgtggacgccatcgtgcctcagagctttctgaaggacgactccatcgacaacaaggtgctgaccagaagcgacaagaaccggggcaagagcgacaacgtgccctccgaagaggtcgtgaagaagatgaagaactactggcggcagctgctgaacgccaagctgattacccagagaaagttcgacaatctgaccaaggccgagagaggcggcctgagcgaactggataaggccggcttcatcaagagacagctggtggaaacccggcagatcacaaagcacgtggcacagatcctggactcccggatgaacactaagtacgacgagaatgacaagctgatccgggaagtgaaagtgatcaccctgaagtccaagctggtgtccgatttccggaaggatttccagttttacaaagtgcgcgagatcaacaactaccaccacgcccacgacgcctacctgaacgccgtcgtgggaaccgccctgatcaaaaagtaccctaagctggaaagcgagttcgtgtacggcgactacaaggtgtacgacgtgcggaagatgatcgccaagagcgagcaggaaatcggcaaggctaccgccaagtacttcttctacagcaacatcatgaactttttcaagaccgagattaccctggccaacggcgagatccggaagcggcctctgatcgagacaaacggcgaaaccggggagatcgtgtgggataagggccgggattttgccaccgtgcggaaagtgctgagcatgccccaagtgaatatcgtgaaaaagaccgaggtgcagacaggcggcttcagcaaagagtctatcctgcccaagaggaacagcgataagctgatcgccagaaagaaggactgggaccctaagaagtacggcggcttcgacagccccaccgtggcctattctgtgctggtggtggccaaagtggaaaagggcaagtccaagaaactgaagagtgtgaaagagctgctggggatcaccatcatggaaagaagcagcttcgagaagaatcccatcgactttctggaagccaagggctacaaagaagtgaaaaaggacctgatcatcaagctgcctaagtactccctgttcgagctggaaaacggccggaagagaatgctggcctctgccggcgaactgcagaagggaaacgaactggccctgccctccaaatatgtgaacttcctgtacctggccagccactatgagaagctgaagggctcccccgaggataatgagcagaaacagctgtttgtggaacagcacaagcactacctggacgagatcatcgagcagatcagcgagttctccaagagagtgatcctggccgacgctaatctggacaaagtgctgtccgcctacaacaagcaccgggataagcccatcagagagcaggccgagaatatcatccacctgtttaccctgaccaatctgggagcccctgccgccttcaagtactttgacaccaccatcgaccggaagaggtacaccagcaccaaagaggtgctggacgccaccctgatccaccagagcatcaccggcctgtacgagacacggatcgacctgtctcagctgggaggcgacggatccacaccacctaagaagaaacggaaggtcgaggacggcgagggccctgctgctaagagagtgaaactggactccggagctgctccagccgccaagaagaagaagctcgactacaaggacgacgacgataagtga

SEQ ID NO: 112 - DNA, 6621 bp, Synthetic construct
  source 1..6621: mol_type = other DNA
atgaccctgaacatcgaggacgagtaccggctgcacgagacaagcaaagaacccgatgtgtccctgggcagcacctggcttagtgatttccctcaggcctgggccgagacaggcggaatgggacttgctgttagacaggcccctctgatcatccctctgaaggccacaagcacccctgtgtccatcaagcagtaccccatgagccaagaggcccggctgggaatcaagccccacattcagagactgctggaccagggcatcctggtgccttgtcagagcccttggaatacccctctgctgcccgtgaagaagcccggcaccaacgattacagacccgtgcaggacctgcgggaagtgaacaagagagtggaagatattcaccccaccgtgccgaatccttacaacctgctgtctggcctgcctcctagccaccagtggtacacagtgctggacctgaaggacgccttcttctgtctgcggctgcaccctacaagccagcctctgtttgcctttgagtggcgggaccctgagatgggcattagcggacagctgacctggaccagactgccccagggcttcaagaacagccccacactgttcaacgaggccctgcatagggacctcgccgacttcagaatccagcatcctgacctgatcctgctccagtacgtggacgatctgctgctggccgctacaagcgagctggattgtcagcagggaacaagagccctgctgcaaaccctgggcaacctgggctatagagcctctgccaagaaggcccagatttgccagaaacaagtgaagtatctgggctacctgctgaaagagggccagcgttggctgaccgaggccagaaaagaaaccgtgatgggccagcctacacctaagacacccagacagctgagagagttcctgggcaaagccggattctgtcggctgttcatccctggctttgccgagatggctgcccctctgtacccactgacaaagcccggaactctgttcaactggggcccagatcagcagaaggcctaccaagagatcaagcaggctctgctgacagcccctgctctgggactgcctgatctgaccaagcctttcgagctgttcgtggacgagaagcagggctatgccaaaggcgtgctgacacagaagctcggcccttggagaaggcctgtggcctacctgagcaagaaactggaccctgtggctgccggatggcctccttgtctgagaatggtggccgccattgccgtgctgaccaaggatgccggaaagctgacaatgggacagcctctggtcattctggcccctcatgccgtggaagccctcgtgaaacagcctcctgatcggtggctgagcaacgccaggatgacacactatcaggcactgctgctcgacaccgacagagtgcagtttggacctgtggtggccctgaatcctgccacacttctgcctctgcctgaggaaggcctccagcacaattgcctggacatcctggccgaggctcacggcacaagacccgatctgacagatcagccactgcctgacgccgaccacacctggtatacagatggcagctctctgctgcaagaaggacagagaaaagccggggctgccgtgaccaccgagacagaagtgatttgggccaaagctctgcccgctggcacatctgctcagagagccgaactgatcgccctgacacaggccctgaaaatggccgagggcaagaagctgaacgtctacaccgactccagatacgccttcgccaccgctcacatccacggcgaaatctatcggcggagaggatggctgaccagcgagggcaaagagattaagaacaaggacgagattctcgccctgctcaaggccctgttcctgcctaagcggctgagcatcatccactgtccaggccaccagaagggccactctgctgaagctagaggcaacagaatggccgaccaggctgccagaaaggccgccatcacagagacacccgataccagcacactgctgatcgagaacagcagccctggatccacgccgcccaagaagaagagaaaggttgaggacggcgagggcaccggtggacctggaagcgagcctgctacatctggctctgagacacctggcacctccgagtctgctacacctgaatctggacctggcggatccggagacaagaagtacagcatcggcctggacatcggcaccaactctgtgggctgggccgtgatcaccgacgagtacaaggtgcccagcaagaaattcaaggtgctgggcaacaccgaccggcacagcatcaagaagaacctgatcggagccctgctgttcgacagcggcgaaacagccgaggccacccggctgaagagaaccgccagaagaagatacaccagacggaagaaccggatctgctatctgcaagagatcttcagcaacgagatggccaaggtggacgacagcttcttccacagactggaagagtccttcctggtggaagaggataagaagcacgagcggcaccccatcttcggcaacatcgtggacgaggtggcctaccacgagaagtaccccaccatctaccacctgagaaagaaactggtggacagcaccgacaaggccgacctgcggctgatctatctggccctggcccacatgatcaagttccggggccacttcctgatcgagggcgacctgaaccccgacaacagcgacgtggacaagctgttcatccagctggtgcagacctacaaccagctgttcgaggaaaaccccatcaacgccagcggcgtggacgccaaggccatcctgtctgccagactgagcaagagcagacggctggaaaatctgatcgcccagctgcccggcgagaagaagaatggcctgttcggcaacctgattgccctgagcctgggcctgacccccaacttcaagagcaacttcgacctggccgaggatgccaaactgcagctgagcaaggacacctacgacgacgacctggacaacctgctggcccagatcggcgaccagtacgccgacctgtttctggccgccaagaacctgtccgacgccatcctgctgagcgacatcctgagagtgaacaccgagatcaccaaggcccccctgagcgcctctatgatcaagagatacgacgagcaccaccaggacctgaccctgctgaaagctctcgtgcggcagcagctgcctgagaagtacaaagagattttcttcgaccagagcaagaacggctacgccggctacattgacggcggagccagccaggaagagttctacaagttcatcaagcccatcctggaaaagatggacggcaccgaggaactgctcgtgaagctgaacagagaggacctgctgcggaagcagcggaccttcgacaacggcagcatcccccaccagatccacctgggagagctgcacgccattctgcggcggcaggaagatttttacccattcctgaaggacaaccgggaaaagatcgagaagatcctgaccttccgcatcccctactacgtgggccctctggccaggggaaacagcagattcgcctggatgaccagaaagagcgaggaaaccatcaccccctggaacttcgaggaagtggtggacaagggcgcttccgcccagagcttcatcgagcggatgaccaacttcgataagaacctgcccaacgagaaggtgctgcccaagcacagcctgctgtacgagtacttcaccgtgtataacgagctgaccaaagtgaaatacgtgaccgagggaatgagaaagcccgccttcctgagcggcgagcagaaaaaggccatcgtggacctgctgttcaagaccaaccggaaagtgaccgtgaagcagctgaaagaggactacttcaagaaaatcgagtgcttcgactccgtggaaatctccggcgtggaagatcggttcaacgcctccctgggcacataccacgatctgctgaaaattatcaaggacaaggacttcctggacaatgaggaaaacgaggacattctggaagatatcgtgctgaccctgacactgtttgaggacagagagatgatcgaggaacggctgaaaacctatgcccacctgttcgacgacaaagtgatgaagcagctgaagcggcggagatacaccggctggggcaggctgagccggaagctgatcaacggcatccgggacaagcagtccggcaagacaatcctggatttcctgaagtccgacggcttcgccaacagaaacttcatgcagctgatccacgacgacagcctgacctttaaagaggacatccagaaagcccaggtgtccggccagggcgatagcctgcacgagcacattgccaatctggccggcagccccgccattaagaagggcatcctgcagacagtgaaggtggtggacgagctcgtgaaagtgatgggccggcacaagcccgagaacatcgtgatcgaaatggccagagagaaccagaccacccagaagggacagaagaacagccgcgagagaatgaagcggatcgaagagggcatcaaagagctgggcagccagatcctgaaagaacaccccgtggaaaacacccagctgcagaacgagaagctgtacctgtactacctgcagaatgggcgggatatgtacgtggaccaggaactggacatcaaccggctgtccgactacgatgtggacgccatcgtgcctcagagctttctgaaggacgactccatcgacaacaaggtgctgaccagaagcgacaagaaccggggcaagagcgacaacgtgccctccgaagaggtcgtgaagaagatgaagaactactggcggcagctgctgaacgccaagctgattacccagagaaagttcgacaatctgaccaaggccgagagaggcggcctgagcgaactggataaggccggcttcatcaagagacagctggtggaaacccggcagatcacaaagcacgtggcacagatcctggactcccggatgaacactaagtacgacgagaatgacaagctgatccgggaagtgaaagtgatcaccctgaagtccaagctggtgtccgatttccggaaggatttccagttttacaaagtgcgcgagatcaacaactaccaccacgcccacgacgcctacctgaacgccgtcgtgggaaccgccctgatcaaaaagtaccctaagctggaaagcgagttcgtgtacggcgactacaaggtgtacgacgtgcggaagatgatcgccaagagcgagcaggaaatcggcaaggctaccgccaagtacttcttctacagcaacatcatgaactttttcaagaccgagattaccctggccaacggcgagatccggaagcggcctctgatcgagacaaacggcgaaaccggggagatcgtgtgggataagggccgggattttgccaccgtgcggaaagtgctgagcatgccccaagtgaatatcgtgaaaaagaccgaggtgcagacaggcggcttcagcaaagagtctatcctgcccaagaggaacagcgataagctgatcgccagaaagaaggactgggaccctaagaagtacggcggcttcgacagccccaccgtggcctattctgtgctggtggtggccaaagtggaaaagggcaagtccaagaaactgaagagtgtgaaagagctgctggggatcaccatcatggaaagaagcagcttcgagaagaatcccatcgactttctggaagccaagggctacaaagaagtgaaaaaggacctgatcatcaagctgcctaagtactccctgttcgagctggaaaacggccggaagagaatgctggcctctgccggcgaactgcagaagggaaacgaactggccctgccctccaaatatgtgaacttcctgtacctggccagccactatgagaagctgaagggctcccccgaggataatgagcagaaacagctgtttgtggaacagcacaagcactacctggacgagatcatcgagcagatcagcgagttctccaagagagtgatcctggccgacgctaatctggacaaagtgctgtccgcctacaacaagcaccgggataagcccatcagagagcaggccgagaatatcatccacctgtttaccctgaccaatctgggagcccctgccgccttcaagtactttgacaccaccatcgaccggaagaggtacaccagcaccaaagaggtgctggacgccaccctgatccaccagagcatcaccggcctgtacgagacacggatcgacctgtctcagctgggaggcgacggatccacaccacctaagaagaaacggaaggtcgaggacggcgagggccctgctgctaagagagtgaaactggactccggagctgctccagccgccaagaagaagaagctcgactacaaggacgacgacgataagggcggatctggcggagctaccgtgaagttcaagtacaagggcgaagaaaaagaggtggacatcagcaagatcaagaaagtttggcgcgtgggcaagatgatctccttcacctacgatctcggcggaggcaagacaggcaggggagccgtttctgaaaaggacgcccctaaagaactgctccagatgctggaaaagcagaagaagtga

SEQ ID NO: 113 - DNA, 4890 bp, Synthetic construct
  source 1..4890: mol_type = other DNA
atgaaacggacagccgacggaagcgagttcgagtcaccaaagaagaagcggaaagtctctgaggtggagttttcccacgagtactggatgagacatgccctgaccctggccaagagggcacgggatgagagggaggtgcctgtgggagccgtgctggtgctgaacaatagagtgatcggcgagggctggaacagagccatcggcctgcacgacccaacagcccatgccgaaattatggccctgagacagggcggcctggtcatgcagaactacagactgattgacgccaccctgtacgtgacattcgagccttgcgtgatgtgcgccggcgccatgatccactctaggatcggccgcgtggtgtttggcgtgaggaactcaaaaagaggcgccgcaggctccctgatgaacgtgctgaactaccccggcatgaatcaccgcgtcgaaattaccgagggaatcctggcagatgaatgtgccgccctgctgtgcgatttctatcggatgcctagacaggtgttcaatgctcagaagaaggcccagagctccatcaactccggaggatctagcggaggctcctctggctctgagacacctggcacaagcgagagcgcaacacctgaaagcagcgggggcagcagcggggggtcagacaagaagtacagcatcggcctggccatcggcaccaactctgtgggctgggccgtgatcaccgacgagtacaaggtgcccagcaagaaattcaaggtgctgggcaacaccgaccggcacagcatcaagaagaacctgatcggagccctgctgttcgacagcggcgaaacagccgaggccacccggctgaagagaaccgccagaagaagatacaccagacggaagaaccggatctgctatctgcaagagatcttcagcaacgagatggccaaggtggacgacagcttcttccacagactggaagagtccttcctggtggaagaggataagaagcacgagcggcaccccatcttcggcaacatcgtggacgaggtggcctaccacgagaagtaccccaccatctaccacctgagaaagaaactggtggacagcaccgacaaggccgacctgcggctgatctatctggccctggcccacatgatcaagttccggggccacttcctgatcgagggcgacctgaaccccgacaacagcgacgtggacaagctgttcatccagctggtgcagacctacaaccagctgttcgaggaaaaccccatcaacgccagcggcgtggacgccaaggccatcctgtctgccagactgagcaagagcagacggctggaaaatctgatcgcccagctgcccggcgagaagaagaatggcctgttcggcaacctgattgccctgagcctgggcctgacccccaacttcaagagcaacttcgacctggccgaggatgccaaactgcagctgagcaaggacacctacgacgacgacctggacaacctgctggcccagatcggcgaccagtacgccgacctgtttctggccgccaagaacctgtccgacgccatcctgctgagcgacatcctgagagtgaacaccgagatcaccaaggcccccctgagcgcctctatgatcaagagatacgacgagcaccaccaggacctgaccctgctgaaagctctcgtgcggcagcagctgcctgagaagtacaaagagattttcttcgaccagagcaagaacggctacgccggctacattgacggcggagccagccaggaagagttctacaagttcatcaagcccatcctggaaaagatggacggcaccgaggaactgctcgtgaagctgaacagagaggacctgctgcggaagcagcggaccttcgacaacggcagcatcccccaccagatccacctgggagagctgcacgccattctgcggcggcaggaagatttttacccattcctgaaggacaaccgggaaaagatcgagaagatcctgaccttccgcatcccctactacgtgggccctctggccaggggaaacagcagattcgcctggatgaccagaaagagcgaggaaaccatcaccccctggaacttcgaggaagtggtggacaagggcgcttccgcccagagcttcatcgagcggatgaccaacttcgataagaacctgcccaacgagaaggtgctgcccaagcacagcctgctgtacgagtacttcaccgtgtataacgagctgaccaaagtgaaatacgtgaccgagggaatgagaaagcccgccttcctgagcggcgagcagaaaaaggccatcgtggacctgctgttcaagaccaaccggaaagtgaccgtgaagcagctgaaagaggactacttcaagaaaatcgagtgcttcgactccgtggaaatctccggcgtggaagatcggttcaacgcctccctgggcacataccacgatctgctgaaaattatcaaggacaaggacttcctggacaatgaggaaaacgaggacattctggaagatatcgtgctgaccctgacactgtttgaggacagagagatgatcgaggaacggctgaaaacctatgcccacctgttcgacgacaaagtgatgaagcagctgaagcggcggagatacaccggctggggcaggctgagccggaagctgatcaacggcatccgggacaagcagtccggcaagacaatcctggatttcctgaagtccgacggcttcgccaacagaaacttcatgcagctgatccacgacgacagcctgacctttaaagaggacatccagaaagcccaggtgtccggccagggcgatagcctgcacgagcacattgccaatctggccggcagccccgccattaagaagggcatcctgcagacagtgaaggtggtggacgagctcgtgaaagtgatgggccggcacaagcccgagaacatcgtgatcgaaatggccagagagaaccagaccacccagaagggacagaagaacagccgcgagagaatgaagcggatcgaagagggcatcaaagagctgggcagccagatcctgaaagaacaccccgtggaaaacacccagctgcagaacgagaagctgtacctgtactacctgcagaatgggcgggatatgtacgtggaccaggaactggacatcaaccggctgtccgactacgatgtggaccatatcgtgcctcagagctttctgaaggacgactccatcgacaacaaggtgctgaccagaagcgacaagaaccggggcaagagcgacaacgtgccctccgaagaggtcgtgaagaagatgaagaactactggcggcagctgctgaacgccaagctgattacccagagaaagttcgacaatctgaccaaggccgagagaggcggcctgagcgaactggataaggccggcttcatcaagagacagctggtggaaacccggcagatcacaaagcacgtggcacagatcctggactcccggatgaacactaagtacgacgagaatgacaagctgatccgggaagtgaaagtgatcaccctgaagtccaagctggtgtccgatttccggaaggatttccagttttacaaagtgcgcgagatcaacaactaccaccacgcccacgacgcctacctgaacgccgtcgtgggaaccgccctgatcaaaaagtaccctaagctggaaagcgagttcgtgtacggcgactacaaggtgtacgacgtgcggaagatgatcgccaagagcgagcaggaaatcggcaaggctaccgccaagtacttcttctacagcaacatcatgaactttttcaagaccgagattaccctggccaacggcgagatccggaagcggcctctgatcgagacaaacggcgaaaccggggagatcgtgtgggataagggccgggattttgccaccgtgcggaaagtgctgagcatgccccaagtgaatatcgtgaaaaagaccgaggtgcagacaggcggcttcagcaaagagtctatcctgcccaagaggaacagcgataagctgatcgccagaaagaaggactgggaccctaagaagtacggcggcttcgacagccccaccgtggcctattctgtgctggtggtggccaaagtggaaaagggcaagtccaagaaactgaagagtgtgaaagagctgctggggatcaccatcatggaaagaagcagcttcgagaagaatcccatcgactttctggaagccaagggctacaaagaagtgaaaaaggacctgatcatcaagctgcctaagtactccctgttcgagctggaaaacggccggaagagaatgctggcctctgccggcgaactgcagaagggaaacgaactggccctgccctccaaatatgtgaacttcctgtacctggccagccactatgagaagctgaagggctcccccgaggataatgagcagaaacagctgtttgtggaacagcacaagcactacctggacgagatcatcgagcagatcagcgagttctccaagagagtgatcctggccgacgctaatctggacaaagtgctgtccgcctacaacaagcaccgggataagcccatcagagagcaggccgagaatatcatccacctgtttaccctgaccaatctgggagcccctgccgccttcaagtactttgacaccaccatcgaccggaagaggtacaccagcaccaaagaggtgctggacgccaccctgatccaccagagcatcaccggcctgtacgagacacggatcgacctgtctcagctgggaggcgacggatccacaccacctaagaagaaacggaaggtcgaggacggcgagggccctgctgctaagagagtgaaactggactccggagctgctccagccgccaagaagaagaagctcgactacaaggacgacgacgataagtga

SEQ ID NO: 114 - DNA, 4242 bp, Synthetic construct
  source 1..4242: mol_type = other DNA
atggacaagaagtacagcatcggcctggacatcggcaccaactctgtgggctgggccgtgatcaccgacgagtacaaggtgcccagcaagaaattcaaggtgctgggcaacaccgaccggcacagcatcaagaagaacctgatcggagccctgctgttcgacagcggcgaaacagccgaggccacccggctgaagagaaccgccagaagaagatacaccagacggaagaaccggatctgctatctgcaagagatcttcagcaacgagatggccaaggtggacgacagcttcttccacagactggaagagtccttcctggtggaagaggataagaagcacgagcggcaccccatcttcggcaacatcgtggacgaggtggcctaccacgagaagtaccccaccatctaccacctgagaaagaaactggtggacagcaccgacaaggccgacctgcggctgatctatctggccctggcccacatgatcaagttccggggccacttcctgatcgagggcgacctgaaccccgacaacagcgacgtggacaagctgttcatccagctggtgcagacctacaaccagctgttcgaggaaaaccccatcaacgccagcggcgtggacgccaaggccatcctgtctgccagactgagcaagagcagacggctggaaaatctgatcgcccagctgcccggcgagaagaagaatggcctgttcggcaacctgattgccctgagcctgggcctgacccccaacttcaagagcaacttcgacctggccgaggatgccaaactgcagctgagcaaggacacctacgacgacgacctggacaacctgctggcccagatcggcgaccagtacgccgacctgtttctggccgccaagaacctgtccgacgccatcctgctgagcgacatcctgagagtgaacaccgagatcaccaaggcccccctgagcgcctctatgatcaagagatacgacgagcaccaccaggacctgaccctgctgaaagctctcgtgcggcagcagctgcctgagaagtacaaagagattttcttcgaccagagcaagaacggctacgccggctacattgacggcggagccagccaggaagagttctacaagttcatcaagcccatcctggaaaagatggacggcaccgaggaactgctcgtgaagctgaacagagaggacctgctgcggaagcagcggaccttcgacaacggcagcatcccccaccagatccacctgggagagctgcacgccattctgcggcggcaggaagatttttacccattcctgaaggacaaccgggaaaagatcgagaagatcctgaccttccgcatcccctactacgtgggccctctggccaggggaaacagcagattcgcctggatgaccagaaagagcgaggaaaccatcaccccctggaacttcgaggaagtggtggacaagggcgcttccgcccagagcttcatcgagcggatgaccaacttcgataagaacctgcccaacgagaaggtgctgcccaagcacagcctgctgtacgagtacttcaccgtgtataacgagctgaccaaagtgaaatacgtgaccgagggaatgagaaagcccgccttcctgagcggcgagcagaaaaaggccatcgtggacctgctgttcaagaccaaccggaaagtgaccgtgaagcagctgaaagaggactacttcaagaaaatcgagtgcttcgactccgtggaaatctccggcgtggaagatcggttcaacgcctccctgggcacataccacgatctgctgaaaattatcaaggacaaggacttcctggacaatgaggaaaacgaggacattctggaagatatcgtgctgaccctgacactgtttgaggacagagagatgatcgaggaacggctgaaaacctatgcccacctgttcgacgacaaagtgatgaagcagctgaagcggcggagatacaccggctggggcaggctgagccggaagctgatcaacggcatccgggacaagcagtccggcaagacaatcctggatttcctgaagtccgacggcttcgccaacagaaacttcatgcagctgatccacgacgacagcctgacctttaaagaggacatccagaaagcccaggtgtccggccagggcgatagcctgcacgagcacattgccaatctggccggcagccccgccattaagaagggcatcctgcagacagtgaaggtggtggacgagctcgtgaaagtgatgggccggcacaagcccgagaacatcgtgatcgaaatggccagagagaaccagaccacccagaagggacagaagaacagccgcgagagaatgaagcggatcgaagagggcatcaaagagctgggcagccagatcctgaaagaacaccccgtggaaaacacccagctgcagaacgagaagctgtacctgtactacctgcagaatgggcgggatatgtacgtggaccaggaactggacatcaaccggctgtccgactacgatgtggaccatatcgtgcctcagagctttctgaaggacgactccatcgacaacaaggtgctgaccagaagcgacaagaaccggggcaagagcgacaacgtgccctccgaagaggtcgtgaagaagatgaagaactactggcggcagctgctgaacgccaagctgattacccagagaaagttcgacaatctgaccaaggccgagagaggcggcctgagcgaactggataaggccggcttcatcaagagacagctggtggaaacccggcagatcacaaagcacgtggcacagatcctggactcccggatgaacactaagtacgacgagaatgacaagctgatccgggaagtgaaagtgatcaccctgaagtccaagctggtgtccgatttccggaaggatttccagttttacaaagtgcgcgagatcaacaactaccaccacgcccacgacgcctacctgaacgccgtcgtgggaaccgccctgatcaaaaagtaccctaagctggaaagcgagttcgtgtacggcgactacaaggtgtacgacgtgcggaagatgatcgccaagagcgagcaggaaatcggcaaggctaccgccaagtacttcttctacagcaacatcatgaactttttcaagaccgagattaccctggccaacggcgagatccggaagcggcctctgatcgagacaaacggcgaaaccggggagatcgtgtgggataagggccgggattttgccaccgtgcggaaagtgctgagcatgccccaagtgaatatcgtgaaaaagaccgaggtgcagacaggcggcttcagcaaagagtctatcctgcccaagaggaacagcgataagctgatcgccagaaagaaggactgggaccctaagaagtacggcggcttcgacagccccaccgtggcctattctgtgctggtggtggccaaagtggaaaagggcaagtccaagaaactgaagagtgtgaaagagctgctggggatcaccatcatggaaagaagcagcttcgagaagaatcccatcgactttctggaagccaagggctacaaagaagtgaaaaaggacctgatcatcaagctgcctaagtactccctgttcgagctggaaaacggccggaagagaatgctggcctctgccggcgaactgcagaagggaaacgaactggccctgccctccaaatatgtgaacttcctgtacctggccagccactatgagaagctgaagggctcccccgaggataatgagcagaaacagctgtttgtggaacagcacaagcactacctggacgagatcatcgagcagatcagcgagttctccaagagagtgatcctggccgacgctaatctggacaaagtgctgtccgcctacaacaagcaccgggataagcccatcagagagcaggccgagaatatcatccacctgtttaccctgaccaatctgggagcccctgccgccttcaagtactttgacaccaccatcgaccggaagaggtacaccagcaccaaagaggtgctggacgccaccctgatccaccagagcatcaccggcctgtacgagacacggatcgacctgtctcagctgggaggcgacggatccacaccacctaagaagaaacggaaggtcgaggacggcgagggccctgctgctaagagagtgaaactggactccggagctgctccagccgccaagaagaagaagctcgactacaaggacgacgacgataagtga

SEQ ID NO: 115 - DNA, 4206 bp, Synthetic construct
  source 1..4206: mol_type = other DNA
atggacaagaagtacagcatcggcctggacatcggcaccaactctgtgggctgggccgtgatcaccgacgagtacaaggtgcccagcaagaaattcaaggtgctgggcaacaccgaccggcacagcatcaagaagaacctgatcggagccctgctgttcgacagcggcgaaacagccgaggccacccggctgaagagaaccgccagaagaagatacaccagacggaagaaccggatctgctatctgcaagagatcttcagcaacgagatggccaaggtggacgacagcttcttccacagactggaagagtccttcctggtggaagaggataagaagcacgagcggcaccccatcttcggcaacatcgtggacgaggtggcctaccacgagaagtaccccaccatctaccacctgagaaagaaactggtggacagcaccgacaaggccgacctgcggctgatctatctggccctggcccacatgatcaagttccggggccacttcctgatcgagggcgacctgaaccccgacaacagcgacgtggacaagctgttcatccagctggtgcagacctacaaccagctgttcgaggaaaaccccatcaacgccagcggcgtggacgccaaggccatcctgtctgccagactgagcaagagcagacggctggaaaatctgatcgcccagctgcccggcgagaagaagaatggcctgttcggcaacctgattgccctgagcctgggcctgacccccaacttcaagagcaacttcgacctggccgaggatgccaaactgcagctgagcaaggacacctacgacgacgacctggacaacctgctggcccagatcggcgaccagtacgccgacctgtttctggccgccaagaacctgtccgacgccatcctgctgagcgacatcctgagagtgaacaccgagatcaccaaggcccccctgagcgcctctatgatcaagagatacgacgagcaccaccaggacctgaccctgctgaaagctctcgtgcggcagcagctgcctgagaagtacaaagagattttcttcgaccagagcaagaacggctacgccggctacattgacggcggagccagccaggaagagttctacaagttcatcaagcccatcctggaaaagatggacggcaccgaggaactgctcgtgaagctgaacagagaggacctgctgcggaagcagcggaccttcgacaacggcagcatcccccaccagatccacctgggagagctgcacgccattctgcggcggcaggaagatttttacccattcctgaaggacaaccgggaaaagatcgagaagatcctgaccttccgcatcccctactacgtgggccctctggccaggggaaacagcagattcgcctggatgaccagaaagagcgaggaaaccatcaccccctggaacttcgaggaagtggtggacaagggcgcttccgcccagagcttcatcgagcggatgaccaacttcgataagaacctgcccaacgagaaggtgctgcccaagcacagcctgctgtacgagtacttcaccgtgtataacgagctgaccaaagtgaaatacgtgaccgagggaatgagaaagcccgccttcctgagcggcgagcagaaaaaggccatcgtggacctgctgttcaagaccaaccggaaagtgaccgtgaagcagctgaaagaggactacttcaagaaaatcgagtgcttcgactccgtggaaatctccggcgtggaagatcggttcaacgcctccctgggcacataccacgatctgctgaaaattatcaaggacaaggacttcctggacaatgaggaaaacgaggacattctggaagatatcgtgctgaccctgacactgtttgaggacagagagatgatcgaggaacggctgaaaacctatgcccacctgttcgacgacaaagtgatgaagcagctgaagcggcggagatacaccggctggggcaggctgagccggaagctgatcaacggcatccgggacaagcagtccggcaagacaatcctggatttcctgaagtccgacggcttcgccaacagaaacttcatgcagctgatccacgacgacagcctgacctttaaagaggacatccagaaagcccaggtgtccggccagggcgatagcctgcacgagcacattgccaatctggccggcagccccgccattaagaagggcatcctgcagacagtgaaggtggtggacgagctcgtgaaagtgatgggccggcacaagcccgagaacatcgtgatcgaaatggccagagagaaccagaccacccagaagggacagaagaacagccgcgagagaatgaagcggatcgaagagggcatcaaagagctgggcagccagatcctgaaagaacaccccgtggaaaacacccagctgcagaacgagaagctgtacctgtactacctgcagaatgggcgggatatgtacgtggaccaggaactggacatcaaccggctgtccgactacgatgtggaccatatcgtgcctcagagctttctgaaggacgactccatcgacaacaaggtgctgaccagaagcgacaaggcccggggcaagagcgacaacgtgccctccgaagaggtcgtgaagaagatgaagaactactggcggcagctgctgaacgccaagctgattacccagagaaagttcgacaatctgaccaaggccgagagaggcggcctgagcgaactggataaggccggcttcatcaagagacagctggtggaaacccggcagatcacaaagcacgtggcacagatcctggactcccggatgaacactaagtacgacgagaatgacaagctgatccgggaagtgaaagtgatcaccctgaagtccaagctggtgtccgatttccggaaggatttccagttttacaaagtgcgcgagatcaacaactaccaccacgcccacgacgcctacctgaacgccgtcgtgggaaccgccctgatcaaaaagtaccctaagctggaaagcgagttcgtgtacggcgactacaaggtgtacgacgtgcggaagatgatcgccaagagcgagcaggaaatcggcaaggctaccgccaagtacttcttctacagcaacatcatgaactttttcaagaccgagattaccctggccaacggcgagatccggaagcggcctctgatcgagacaaacggcgaaaccggggagatcgtgtgggataagggccgggattttgccaccgtgcggaaagtgctgagcatgccccaagtgaatatcgtgaaaaagaccgaggtgcagacaggcggcttcagcaaagagtctatcctgcccaagaggaacagcgataagctgatcgccagaaagaaggactgggaccctaagaagtacggcggcttcgacagccccaccgtggcctattctgtgctggtggtggccaaagtggaaaagggcaagtccaagaaactgaagagtgtgaaagagctgctggggatcaccatcatggaaagaagcagcttcgagaagaatcccatcgactttctggaagccaagggctacaaagaagtgaaaaaggacctgatcatcaagctgcctaagtactccctgttcgagctggaaaacggccggaagagaatgctggcctctgccggcgaactgcagaagggaaacgaactggccctgccctccaaatatgtgaacttcctgtacctggccagccactatgagaagctgaagggctcccccgaggataatgagcagaaacagctgtttgtggaacagcacaagcactacctggacgagatcatcgagcagatcagcgagttctccaagagagtgatcctggccgacgctaatctggacaaagtgctgtccgcctacaacaagcaccgggataagcccatcagagagcaggccgagaatatcatccacctgtttaccctgaccaatctgggagcccctgccgccttcaagtactttgacaccaccatcgaccggaagaggtacaccagcaccaaagaggtgctggacgccaccctgatccaccagagcatcaccggcctgtacgagacacggatcgacctgtctcagctgggaggcgacgcctatccctatgacgtgcccgattatgccagcctgggcagcggctcccccaagaaaaaacgcaaggtggaagatcctaagaaaaagcggaaagtggactga

SEQ ID NO: 116 - DNA, 2459 bp, Synthetic construct
  source 1..2459: mol_type = other DNA
atggtttctaaaggcgaggccgtgatcaaagagttcatgaggttcaaggtgcacatggaaggcagcatgaacggccacgagttcgagatcgaaggcgaaggcgagggcagaccttacgagggaactcagaccgccaagctgaaagtgaccaaaggcggccctctgcctttcagctgggacatcctgtctccacagtttatgtacggcagcagggccttcatcaagcaccccgctgacatccccgactactacaagcagtctttcccagagggcttcaagtgggagagagtgatgaacttcgaggacggcggagccgtgactgtgacacaggacacatctctggaagatgggaccctgatctacaaagtgaagctgcggggcacaaacttccctccagacggccctgtgatgcagaaaaagacaatgggctgggaagccagcaccgagagactgtaccctgaagatggcgtgctgaagggcgacatcaagatggccctgagactgaaggacggcggcagatacctggccgacttcaagaccacctacaaggccaagaaacctgtgcagatgcctggcgcctacaacgtggacagaaagctggacatcacctcccacaacgaagactgaccgggcgcttccgcctccggttccggcagcggatccgagacacctggcacaagcgagtctgccacaccagagtctggaagcggcgccacaaacttcagcctgctcaaacaggctggcgacgtggaagagaaccctggacctggctctgccgactacaaggacgacgacgacaaaggctctggcagcgaaacccctggcacatccgaaagcgctacaccagaaagcggaggcggcggactgctggaaaagttcgtcggcacctggaagatcgccgactctcacaacttcggcgagtacctcaaggccatcggcgctccaaaagagttgtcagacggaggcgacgccaccacacctacactgtacatcagccagaaagacggcgacaaaatgtccgtcaagatcgagaacggccctcctaccttcctggacacccaagtcaagttcaagctgggcgaggagttcgacgagtttccaagcgacagacggaagggagtcaagtccgtggtcaacctcgtgggagagaagctggtgtacgtgcagaagtgggacggcaaagagacaacctacgtcagagagatcaaggacggcaagctggtggtcaccctcactatgggcgacgtggtggccgtgcggagctacagaagggccacagagtgaaggcagcggcgctaccaacttttcactgctcaagcaggccggggacgtcgaggaaaatcctggaccagcttacccctacgacgtgccagattacgctggctccggcagcgaaacaccaggcaccagcgagtctgctaccccagaatcaggtggcggaggcctgctcgagaagtttgttggaacatggaagattgccgacagtcacaattttggggagtatctcaaggctatcggagccccaaaagaactgtccgacggcggcgacgctacaaccccaactctgtacatctctcaaaaggacggggacaagatgtctgttaagatcgaaaacgggccgccaacattcctggatacgcaagtcaaattcaaactcggcgaagagtttgacgagttcccatccgacagaagaaagggcgtcaagagcgtggtcaatctcgtgggcgaaaaactggtctacgtccaaaagtgggacgggaaagaaaccacatacgtgcgggaaatcaaggacggaaagctcgtggtcacactcacaatgggcgacgtcgtggctgtgcggtcttacagacgcgctaccgaatgacggatctggcgctaccaatttcagccttctcaagcaagcaggcgacgtggaggaaaacccagggcctgctggaaagcccattccaaatcctctgctgggcctcgacagcaccggcagtggttccgaaactcccggaacaagcgagagcgccacaccagaatctggcggtggtggactgctggagaaatttgtcggtacttggaaaatcgccgacagccacaacttcggagaatacctcaaagctattggggcacccaaagagctttccgacggcggggacgcaactactcccacactgtatatttcccaaaaggatggggacaaaatgtccgtcaaaatcgagaatggaccgccgacttttctcgacacacaagtcaagttcaaattgggagaagagttcgatgaatttcccagcgaccgccgcaaaggcgtcaaatctgtggtcaaccttgtcggggaaaagctcgtttacgttcaaaaatgggacggaaaagaaacgacctatgtccgcgaaatcaaagacgggaagcttgttgttactcttacgatgggcgatgtggtcgccgtcaggtcttatcggagagccacagagtga

SEQ ID NO: 117 - DNA, 4101 bp, Synthetic construct
  source 1..4101: mol_type = other DNA
gacaagaagtacagcatcggcctggacatcggcaccaactctgtgggctgggccgtgatcaccgacgagtacaaggtgcccagcaagaaattcaaggtgctgggcaacaccgaccggcacagcatcaagaagaacctgatcggagccctgctgttcgacagcggcgaaacagccgaggccacccggctgaagagaaccgccagaagaagatacaccagacggaagaaccggatctgctatctgcaagagatcttcagcaacgagatggccaaggtggacgacagcttcttccacagactggaagagtccttcctggtggaagaggataagaagcacgagcggcaccccatcttcggcaacatcgtggacgaggtggcctaccacgagaagtaccccaccatctaccacctgagaaagaaactggtggacagcaccgacaaggccgacctgcggctgatctatctggccctggcccacatgatcaagttccggggccacttcctgatcgagggcgacctgaaccccgacaacagcgacgtggacaagctgttcatccagctggtgcagacctacaaccagctgttcgaggaaaaccccatcaacgccagcggcgtggacgccaaggccatcctgtctgccagactgagcaagagcagacggctggaaaatctgatcgcccagctgcccggcgagaagaagaatggcctgttcggcaacctgattgccctgagcctgggcctgacccccaacttcaagagcaacttcgacctggccgaggatgccaaactgcagctgagcaaggacacctacgacgacgacctggacaacctgctggcccagatcggcgaccagtacgccgacctgtttctggccgccaagaacctgtccgacgccatcctgctgagcgacatcctgagagtgaacaccgagatcaccaaggcccccctgagcgcctctatgatcaagagatacgacgagcaccaccaggacctgaccctgctgaaagctctcgtgcggcagcagctgcctgagaagtacaaagagattttcttcgaccagagcaagaacggctacgccggctacattgacggcggagccagccaggaagagttctacaagttcatcaagcccatcctggaaaagatggacggcaccgaggaactgctcgtgaagctgaacagagaggacctgctgcggaagcagcggaccttcgacaacggcagcatcccccaccagatccacctgggagagctgcacgccattctgcggcggcaggaagatttttacccattcctgaaggacaaccgggaaaagatcgagaagatcctgaccttccgcatcccctactacgtgggccctctggccaggggaaacagcagattcgcctggatgaccagaaagagcgaggaaaccatcaccccctggaacttcgaggaagtggtggacaagggcgcttccgcccagagcttcatcgagcggatgaccaacttcgataagaacctgcccaacgagaaggtgctgcccaagcacagcctgctgtacgagtacttcaccgtgtataacgagctgaccaaagtgaaatacgtgaccgagggaatgagaaagcccgccttcctgagcggcgagcagaaaaaggccatcgtggacctgctgttcaagaccaaccggaaagtgaccgtgaagcagctgaaagaggactacttcaagaaaatcgagtgcttcgactccgtggaaatctccggcgtggaagatcggttcaacgcctccctgggcacataccacgatctgctgaaaattatcaaggacaaggacttcctggacaatgaggaaaacgaggacattctggaagatatcgtgctgaccctgacactgtttgaggacagagagatgatcgaggaacggctgaaaacctatgcccacctgttcgacgacaaagtgatgaagcagctgaagcggcggagatacaccggctggggcaggctgagccggaagctgatcaacggcatccgggacaagcagtccggcaagacaatcctggatttcctgaagtccgacggcttcgccaacagaaacttcatgcagctgatccacgacgacagcctgacctttaaagaggacatccagaaagcccaggtgtccggccagggcgatagcctgcacgagcacattgccaatctggccggcagccccgccattaagaagggcatcctgcagacagtgaaggtggtggacgagctcgtgaaagtgatgggccggcacaagcccgagaacatcgtgatcgaaatggccagagagaaccagaccacccagaagggacagaagaacagccgcgagagaatgaagcggatcgaagagggcatcaaagagctgggcagccagatcctgaaagaacaccccgtggaaaacacccagctgcagaacgagaagctgtacctgtactacctgcagaatgggcgggatatgtacgtggaccaggaactggacatcaaccggctgtccgactacgatgtggaccatatcgtgcctcagagctttctgaaggacgactccatcgacaacaaggtgctgaccagaagcgacaagaaccggggcaagagcgacaacgtgccctccgaagaggtcgtgaagaagatgaagaactactggcggcagctgctgaacgccaagctgattacccagagaaagttcgacaatctgaccaaggccgagagaggcggcctgagcgaactggataaggccggcttcatcaagagacagctggtggaaacccggcagatcacaaagcacgtggcacagatcctggactcccggatgaacactaagtacgacgagaatgacaagctgatccgggaagtgaaagtgatcaccctgaagtccaagctggtgtccgatttccggaaggatttccagttttacaaagtgcgcgagatcaacaactaccaccacgcccacgacgcctacctgaacgccgtcgtgggaaccgccctgatcaaaaagtaccctaagctggaaagcgagttcgtgtacggcgactacaaggtgtacgacgtgcggaagatgatcgccaagagcgagcaggaaatcggcaaggctaccgccaagtacttcttctacagcaacatcatgaactttttcaagaccgagattaccctggccaacggcgagatccggaagcggcctctgatcgagacaaacggcgaaaccggggagatcgtgtgggataagggccgggattttgccaccgtgcggaaagtgctgagcatgccccaagtgaatatcgtgaaaaagaccgaggtgcagacaggcggcttcagcaaagagtctatcctgcccaagaggaacagcgataagctgatcgccagaaagaaggactgggaccctaagaagtacggcggcttcgacagccccaccgtggcctattctgtgctggtggtggccaaagtggaaaagggcaagtccaagaaactgaagagtgtgaaagagctgctggggatcaccatcatggaaagaagcagcttcgagaagaatcccatcgactttctggaagccaagggctacaaagaagtgaaaaaggacctgatcatcaagctgcctaagtactccctgttcgagctggaaaacggccggaagagaatgctggcctctgccggcgaactgcagaagggaaacgaactggccctgccctccaaatatgtgaacttcctgtacctggccagccactatgagaagctgaagggctcccccgaggataatgagcagaaacagctgtttgtggaacagcacaagcactacctggacgagatcatcgagcagatcagcgagttctccaagagagtgatcctggccgacgctaatctggacaaagtgctgtccgcctacaacaagcaccgggataagcccatcagagagcaggccgagaatatcatccacctgtttaccctgaccaatctgggagcccctgccgccttcaagtactttgacaccaccatcgaccggaagaggtacaccagcaccaaagaggtgctggacgccaccctgatccaccagagcatcaccggcctgtacgagacacggatcgacctgtctcagctgggaggcgac

SEQ ID NO: 118 - DNA, 4101 bp, Synthetic construct
  source 1..4101: mol_type = other DNA
gacaagaagtacagcatcggcctggacatcggcaccaactctgtgggctgggccgtgatcaccgacgagtacaaggtgcccagcaagaaattcaaggtgctgggcaacaccgaccggcacagcatcaagaagaacctgatcggagccctgctgttcgacagcggcgaaacagccgaggccacccggctgaagagaaccgccagaagaagatacaccagacggaagaaccggatctgctatctgcaagagatcttcagcaacgagatggccaaggtggacgacagcttcttccacagactggaagagtccttcctggtggaagaggataagaagcacgagcggcaccccatcttcggcaacatcgtggacgaggtggcctaccacgagaagtaccccaccatctaccacctgagaaagaaactggtggacagcaccgacaaggccgacctgcggctgatctatctggccctggcccacatgatcaagttccggggccacttcctgatcgagggcgacctgaaccccgacaacagcgacgtggacaagctgttcatccagctggtgcagacctacaaccagctgttcgaggaaaaccccatcaacgccagcggcgtggacgccaaggccatcctgtctgccagactgagcaagagcagacggctggaaaatctgatcgcccagctgcccggcgagaagaagaatggcctgttcggcaacctgattgccctgagcctgggcctgacccccaacttcaagagcaacttcgacctggccgaggatgccaaactgcagctgagcaaggacacctacgacgacgacctggacaacctgctggcccagatcggcgaccagtacgccgacctgtttctggccgccaagaacctgtccgacgccatcctgctgagcgacatcctgagagtgaacaccgagatcaccaaggcccccctgagcgcctctatgatcaagagatacgacgagcaccaccaggacctgaccctgctgaaagctctcgtgcggcagcagctgcctgagaagtacaaagagattttcttcgaccagagcaagaacggctacgccggctacattgacggcggagccagccaggaagagttctacaagttcatcaagcccatcctggaaaagatggacggcaccgaggaactgctcgtgaagctgaacagagaggacctgctgcggaagcagcggaccttcgacaacggcagcatcccccaccagatccacctgggagagctgcacgccattctgcggcggcaggaagatttttacccattcctgaaggacaaccgggaaaagatcgagaagatcctgaccttccgcatcccctactacgtgggccctctggccaggggaaacagcagattcgcctggatgaccagaaagagcgaggaaaccatcaccccctggaacttcgaggaagtggtggacaagggcgcttccgcccagagcttcatcgagcggatgaccaacttcgataagaacctgcccaacgagaaggtgctgcccaagcacagcctgctgtacgagtacttcaccgtgtataacgagctgaccaaagtgaaatacgtgaccgagggaatgagaaagcccgccttcctgagcggcgagcagaaaaaggccatcgtggacctgctgttcaagaccaaccggaaagtgaccgtgaagcagctgaaagaggactacttcaagaaaatcgagtgcttcgactccgtggaaatctccggcgtggaagatcggttcaacgcctccctgggcacataccacgatctgctgaaaattatcaaggacaaggacttcctggacaatgaggaaaacgaggacattctggaagatatcgtgctgaccctgacactgtttgaggacagagagatgatcgaggaacggctgaaaacctatgcccacctgttcgacgacaaagtgatgaagcagctgaagcggcggagatacaccggctggggcaggctgagccggaagctgatcaacggcatccgggacaagcagtccggcaagacaatcctggatttcctgaagtccgacggcttcgccaacagaaacttcatgcagctgatccacgacgacagcctgacctttaaagaggacatccagaaagcccaggtgtccggccagggcgatagcctgcacgagcacattgccaatctggccggcagccccgccattaagaagggcatcctgcagacagtgaaggtggtggacgagctcgtgaaagtgatgggccggcacaagcccgagaacatcgtgatcgaaatggccagagagaaccagaccacccagaagggacagaagaacagccgcgagagaatgaagcggatcgaagagggcatcaaagagctgggcagccagatcctgaaagaacaccccgtggaaaacacccagctgcagaacgagaagctgtacctgtactacctgcagaatgggcgggatatgtacgtggaccaggaactggacatcaaccggctgtccgactacgatgtggacgctatcgtgcctcagagctttctgaaggacgactccatcgacaacaaggtgctgaccagaagcgacaagaaccggggcaagagcgacaacgtgccctccgaagaggtcgtgaagaagatgaagaactactggcggcagctgctgaacgccaagctgattacccagagaaagttcgacaatctgaccaaggccgagagaggcggcctgagcgaactggataaggccggcttcatcaagagacagctggtggaaacccggcagatcacaaagcacgtggcacagatcctggactcccggatgaacactaagtacgacgagaatgacaagctgatccgggaagtgaaagtgatcaccctgaagtccaagctggtgtccgatttccggaaggatttccagttttacaaagtgcgcgagatcaacaactaccaccacgcccacgacgcctacctgaacgccgtcgtgggaaccgccctgatcaaaaagtaccctaagctggaaagcgagttcgtgtacggcgactacaaggtgtacgacgtgcggaagatgatcgccaagagcgagcaggaaatcggcaaggctaccgccaagtacttcttctacagcaacatcatgaactttttcaagaccgagattaccctggccaacggcgagatccggaagcggcctctgatcgagacaaacggcgaaaccggggagatcgtgtgggataagggccgggattttgccaccgtgcggaaagtgctgagcatgccccaagtgaatatcgtgaaaaagaccgaggtgcagacaggcggcttcagcaaagagtctatcctgcccaagaggaacagcgataagctgatcgccagaaagaaggactgggaccctaagaagtacggcggcttcgacagccccaccgtggcctattctgtgctggtggtggccaaagtggaaaagggcaagtccaagaaactgaagagtgtgaaagagctgctggggatcaccatcatggaaagaagcagcttcgagaagaatcccatcgactttctggaagccaagggctacaaagaagtgaaaaaggacctgatcatcaagctgcctaagtactccctgttcgagctggaaaacggccggaagagaatgctggcctctgccggcgaactgcagaagggaaacgaactggccctgccctccaaatatgtgaacttcctgtacctggccagccactatgagaagctgaagggctcccccgaggataatgagcagaaacagctgtttgtggaacagcacaagcactacctggacgagatcatcgagcagatcagcgagttctccaagagagtgatcctggccgacgctaatctggacaaagtgctgtccgcctacaacaagcaccgggataagcccatcagagagcaggccgagaatatcatccacctgtttaccctgaccaatctgggagcccctgccgccttcaagtactttgacaccaccatcgaccggaagaggtacaccagcaccaaagaggtgctggacgccaccctgatccaccagagcatcaccggcctgtacgagacacggatcgacctgtctcagctgggaggcgac

SEQ ID NO: 119 - DNA, 4101 bp, Synthetic construct
  source 1..4101: mol_type = other DNA
gacaagaagtacagcatcggcctggacatcggcaccaactctgtgggctgggccgtgatcaccgacgagtacaaggtgcccagcaagaaattcaaggtgctgggcaacaccgaccggcacagcatcaagaagaacctgatcggagccctgctgttcgacagcggcgaaacagccgaggccacccggctgaagagaaccgccagaagaagatacaccagacggaagaaccggatctgctatctgcaagagatcttcagcaacgagatggccaaggtggacgacagcttcttccacagactggaagagtccttcctggtggaagaggataagaagcacgagcggcaccccatcttcggcaacatcgtggacgaggtggcctaccacgagaagtaccccaccatctaccacctgagaaagaaactggtggacagcaccgacaaggccgacctgcggctgatctatctggccctggcccacatgatcaagttccggggccacttcctgatcgagggcgacctgaaccccgacaacagcgacgtggacaagctgttcatccagctggtgcagacctacaaccagctgttcgaggaaaaccccatcaacgccagcggcgtggacgccaaggccatcctgtctgccagactgagcaagagcagacggctggaaaatctgatcgcccagctgcccggcgagaagaagaatggcctgttcggcaacctgattgccctgagcctgggcctgacccccaacttcaagagcaacttcgacctggccgaggatgccaaactgcagctgagcaaggacacctacgacgacgacctggacaacctgctggcccagatcggcgaccagtacgccgacctgtttctggccgccaagaacctgtccgacgccatcctgctgagcgacatcctgagagtgaacaccgagatcaccaaggcccccctgagcgcctctatgatcaagagatacgacgagcaccaccaggacctgaccctgctgaaagctctcgtgcggcagcagctgcctgagaagtacaaagagattttcttcgaccagagcaagaacggctacgccggctacattgacggcggagccagccaggaagagttctacaagttcatcaagcccatcctggaaaagatggacggcaccgaggaactgctcgtgaagctgaacagagaggacctgctgcggaagcagcggaccttcgacaacggcagcatcccccaccagatccacctgggagagctgcacgccattctgcggcggcaggaagatttttacccattcctgaaggacaaccgggaaaagatcgagaagatcctgaccttccgcatcccctactacgtgggccctctggccaggggaaacagcagattcgcctggatgaccagaaagagcgaggaaaccatcaccccctggaacttcgaggaagtggtggacaagggcgcttccgcccagagcttcatcgagcggatgaccaacttcgataagaacctgcccaacgagaaggtgctgcccaagcacagcctgctgtacgagtacttcaccgtgtataacgagctgaccaaagtgaaatacgtgaccgagggaatgagaaagcccgccttcctgagcggcgagcagaaaaaggccatcgtggacctgctgttcaagaccaaccggaaagtgaccgtgaagcagctgaaagaggactacttcaagaaaatcgagtgcttcgactccgtggaaatctccggcgtggaagatcggttcaacgcctccctgggcacataccacgatctgctgaaaattatcaaggacaaggacttcctggacaatgaggaaaacgaggacattctggaagatatcgtgctgaccctgacactgtttgaggacagagagatgatcgaggaacggctgaaaacctatgcccacctgttcgacgacaaagtgatgaagcagctgaagcggcggagatacaccggctggggcaggctgagccggaagctgatcaacggcatccgggacaagcagtccggcaagacaatcctggatttcctgaagtccgacggcttcgccaacagaaacttcatgcagctgatccacgacgacagcctgacctttaaagaggacatccagaaagcccaggtgtccggccagggcgatagcctgcacgagcacattgccaatctggccggcagccccgccattaagaagggcatcctgcagacagtgaaggtggtggacgagctcgtgaaagtgatgggccggcacaagcccgagaacatcgtgatcgaaatggccagagagaaccagaccacccagaagggacagaagaacagccgcgagagaatgaagcggatcgaagagggcatcaaagagctgggcagccagatcctgaaagaacaccccgtggaaaacacccagctgcagaacgagaagctgtacctgtactacctgcagaatgggcgggatatgtacgtggaccaggaactggacatcaaccggctgtccgactacgatgtggaccatatcgtgcctcagagctttctgaaggacgactccatcgacaacaaggtgctgaccagaagcgacaaggcccggggcaagagcgacaacgtgccctccgaagaggtcgtgaagaagatgaagaactactggcggcagctgctgaacgccaagctgattacccagagaaagttcgacaatctgaccaaggccgagagaggcggcctgagcgaactggataaggccggcttcatcaagagacagctggtggaaacccggcagatcacaaagcacgtggcacagatcctggactcccggatgaacactaagtacgacgagaatgacaagctgatccgggaagtgaaagtgatcaccctgaagtccaagctggtgtccgatttccggaaggatttccagttttacaaagtgcgcgagatcaacaactaccaccacgcccacgacgcctacctgaacgccgtcgtgggaaccgccctgatcaaaaagtaccctaagctggaaagcgagttcgtgtacggcgactacaaggtgtacgacgtgcggaagatgatcgccaagagcgagcaggaaatcggcaaggctaccgccaagtacttcttctacagcaacatcatgaactttttcaagaccgagattaccctggccaacggcgagatccggaagcggcctctgatcgagacaaacggcgaaaccggggagatcgtgtgggataagggccgggattttgccaccgtgcggaaagtgctgagcatgccccaagtgaatatcgtgaaaaagaccgaggtgcagacaggcggcttcagcaaagagtctatcctgcccaagaggaacagcgataagctgatcgccagaaagaaggactgggaccctaagaagtacggcggcttcgacagccccaccgtggcctattctgtgctggtggtggccaaagtggaaaagggcaagtccaagaaactgaagagtgtgaaagagctgctggggatcaccatcatggaaagaagcagcttcgagaagaatcccatcgactttctggaagccaagggctacaaagaagtgaaaaaggacctgatcatcaagctgcctaagtactccctgttcgagctggaaaacggccggaagagaatgctggcctctgccggcgaactgcagaagggaaacgaactggccctgccctccaaatatgtgaacttcctgtacctggccagccactatgagaagctgaagggctcccccgaggataatgagcagaaacagctgtttgtggaacagcacaagcactacctggacgagatcatcgagcagatcagcgagttctccaagagagtgatcctggccgacgctaatctggacaaagtgctgtccgcctacaacaagcaccgggataagcccatcagagagcaggccgagaatatcatccacctgtttaccctgaccaatctgggagcccctgccgccttcaagtactttgacaccaccatcgaccggaagaggtacaccagcaccaaagaggtgctggacgccaccctgatccaccagagcatcaccggcctgtacgagacacggatcgacctgtctcagctgggaggcgac

SEQ ID NO: 120 - DNA, 4101 bp, Synthetic construct
  source 1..4101: mol_type = other DNA
gacaagaagtacagcatcggcctggacatcggcaccaactctgtgggctgggccgtgatcaccgacgagtacaaggtgcccagcaagaaattcaaggtgctgggcaacaccgaccggcacagcatcaagaagaacctgatcggagccctgctgttcgacagcggcgaaacagccgaggccacccggctgaagagaaccgccagaagaagatacaccagacggaagaaccggatctgctatctgcaagagatcttcagcaacgagatggccaaggtggacgacagcttcttccacagactggaagagtccttcctggtggaagaggataagaagcacgagcggcaccccatcttcggcaacatcgtggacgaggtggcctaccacgagaagtaccccaccatctaccacctgagaaagaaactggtggacagcaccgacaaggccgacctgcggctgatctatctggccctggcccacatgatcaagttccggggccacttcctgatcgagggcgacctgaaccccgacaacagcgacgtggacaagctgttcatccagctggtgcagacctacaaccagctgttcgaggaaaaccccatcaacgccagcggcgtggacgccaaggccatcctgtctgccagactgagcaagagcagacggctggaaaatctgatcgcccagctgcccggcgagaagaagaatggcctgttcggcaacctgattgccctgagcctgggcctgacccccaacttcaagagcaacttcgacctggccgaggatgccaaactgcagctgagcaaggacacctacgacgacgacctggacaacctgctggcccagatcggcgaccagtacgccgacctgtttctggccgccaagaacctgtccgacgccatcctgctgagcgacatcctgagagtgaacaccgagatcaccaaggcccccctgagcgcctctatgatcaagagatacgacgagcaccaccaggacctgaccctgctgaaagctctcgtgcggcagcagctgcctgagaagtacaaagagattttcttcgaccagagcaagaacggctacgccggctacattgacggcggagccagccaggaagagttctacaagttcatcaagcccatcctggaaaagatggacggcaccgaggaactgctcgtgaagctgaacagagaggacctgctgcggaagcagcggaccttcgacaacggcagcatcccccaccagatccacctgggagagctgcacgccattctgcggcggcaggaagatttttacccattcctgaaggacaaccgggaaaagatcgagaagatcctgaccttccgcatcccctactacgtgggccctctggccaggggaaacagcagattcgcctggatgaccagaaagagcgaggaaaccatcaccccctggaacttcgaggaagtggtggacaagggcgcttccgcccagagcttcatcgagcggatgaccaacttcgataagaacctgcccaacgagaaggtgctgcccaagcacagcctgctgtacgagtacttcaccgtgtataacgagctgaccaaagtgaaatacgtgaccgagggaatgagaaagcccgccttcctgagcggcgagcagaaaaaggccatcgtggacctgctgttcaagaccaaccggaaagtgaccgtgaagcagctgaaagaggactacttcaagaaaatcgagtgcttcgactccgtggaaatctccggcgtggaagatcggttcaacgcctccctgggcacataccacgatctgctgaaaattatcaaggacaaggacttcctggacaatgaggaaaacgaggacattctggaagatatcgtgctgaccctgacactgtttgaggacagagagatgatcgaggaacggctgaaaacctatgcccacctgttcgacgacaaagtgatgaagcagctgaagcggcggagatacaccggctggggcaggctgagccggaagctgatcaacggcatccgggacaagcagtccggcaagacaatcctggatttcctgaagtccgacggcttcgccaacagaaacttcatgcagctgatccacgacgacagcctgacctttaaagaggacatccagaaagcccaggtgtccggccagggcgatagcctgcacgagcacattgccaatctggccggcagccccgccattaagaagggcatcctgcagacagtgaaggtggtggacgagctcgtgaaagtgatgggccggcacaagcccgagaacatcgtgatcgaaatggccagagagaaccagaccacccagaagggacagaagaacagccgcgagagaatgaagcggatcgaagagggcatcaaagagctgggcagccagatcctgaaagaacaccccgtggaaaacacccagctgcagaacgagaagctgtacctgtactacctgcagaatgggcgggatatgtacgtggaccaggaactggacatcaaccggctgtccgactacgatgtggacgctatcgtgcctcagagctttctgaaggacgactccatcgacaacaaggtgctgaccagaagcgacaaggcccggggcaagagcgacaacgtgccctccgaagaggtcgtgaagaagatgaagaactactggcggcagctgctgaacgccaagctgattacccagagaaagttcgacaatctgaccaaggccgagagaggcggcctgagcgaactggataaggccggcttcatcaagagacagctggtggaaacccggcagatcacaaagcacgtggcacagatcctggactcccggatgaacactaagtacgacgagaatgacaagctgatccgggaagtgaaagtgatcaccctgaagtccaagctggtgtccgatttccggaaggatttccagttttacaaagtgcgcgagatcaacaactaccaccacgcccacgacgcctacctgaacgccgtcgtgggaaccgccctgatcaaaaagtaccctaagctggaaagcgagttcgtgtacggcgactacaaggtgtacgacgtgcggaagatgatcgccaagagcgagcaggaaatcggcaaggctaccgccaagtacttcttctacagcaacatcatgaactttttcaagaccgagattaccctggccaacggcgagatccggaagcggcctctgatcgagacaaacggcgaaaccggggagatcgtgtgggataagggccgggattttgccaccgtgcggaaagtgctgagcatgccccaagtgaatatcgtgaaaaagaccgaggtgcagacaggcggcttcagcaaagagtctatcctgcccaagaggaacagcgataagctgatcgccagaaagaaggactgggaccctaagaagtacggcggcttcgacagccccaccgtggcctattctgtgctggtggtggccaaagtggaaaagggcaagtccaagaaactgaagagtgtgaaagagctgctggggatcaccatcatggaaagaagcagcttcgagaagaatcccatcgactttctggaagccaagggctacaaagaagtgaaaaaggacctgatcatcaagctgcctaagtactccctgttcgagctggaaaacggccggaagagaatgctggcctctgccggcgaactgcagaagggaaacgaactggccctgccctccaaatatgtgaacttcctgtacctggccagccactatgagaagctgaagggctcccccgaggataatgagcagaaacagctgtttgtggaacagcacaagcactacctggacgagatcatcgagcagatcagcgagttctccaagagagtgatcctggccgacgctaatctggacaaagtgctgtccgcctacaacaagcaccgggataagcccatcagagagcaggccgagaatatcatccacctgtttaccctgaccaatctgggagcccctgccgccttcaagtactttgacaccaccatcgaccggaagaggtacaccagcaccaaagaggtgctggacgccaccctgatccaccagagcatcaccggcctgtacgagacacggatcgacctgtctcagctgggaggcgac

SEQ ID NO: 121 - DNA, 189 bp, Synthetic construct
  source 1..189: mol_type = other DNA
gctaccgtgaagttcaagtacaagggcgaagaaaaagaggtggacatcagcaagatcaagaaagtttggcgcgtgggcaagatgatctccttcacctacgatgagggcggaggcaagacaggcaggggagccgtttctgaaaaggacgcccctaaagaactgctccagatgctggaaaagcagaagaag

SEQ ID NO: 122 - DNA, 189 bp, Synthetic construct
  source 1..189: mol_type = other DNA
gctaccgtgaagttcaagtacaagggcgaagaaaaagaggtggacatcagcaagatcaagaaagtttggcgcgtgggcaagatgatctccttcacctacgatctcggcggaggcaagacaggcaggggagccgtttctgaaaaggacgcccctaaagaactgctccagatgctggaaaagcagaagaag

SEQ ID NO: 123 - DNA, 2031 bp, Synthetic construct
  source 1..2031: mol_type = other DNA
accctgaacatcgaggacgagtaccggctgcacgagacaagcaaagaacccgatgtgtccctgggcagcacctggcttagtgatttccctcaggcctgggccgagacaggcggaatgggacttgctgttagacaggcccctctgatcatccctctgaaggccacaagcacccctgtgtccatcaagcagtaccccatgagccaagaggcccggctgggaatcaagccccacattcagagactgctggaccagggcatcctggtgccttgtcagagcccttggaatacccctctgctgcccgtgaagaagcccggcaccaacgattacagacccgtgcaggacctgcgggaagtgaacaagagagtggaagatattcaccccaccgtgccgaatccttacaacctgctgtctggcctgcctcctagccaccagtggtacacagtgctggacctgaaggacgccttcttctgtctgcggctgcaccctacaagccagcctctgtttgcctttgagtggcgggaccctgagatgggcattagcggacagctgacctggaccagactgccccagggcttcaagaacagccccacactgttcaacgaggccctgcatagggacctcgccgacttcagaatccagcatcctgacctgatcctgctccagtacgtggacgatctgctgctggccgctacaagcgagctggattgtcagcagggaacaagagccctgctgcaaaccctgggcaacctgggctatagagcctctgccaagaaggcccagatttgccagaaacaagtgaagtatctgggctacctgctgaaagagggccagcgttggctgaccgaggccagaaaagaaaccgtgatgggccagcctacacctaagacacccagacagctgagagagttcctgggcaaagccggattctgtcggctgttcatccctggctttgccgagatggctgcccctctgtacccactgacaaagcccggaactctgttcaactggggcccagatcagcagaaggcctaccaagagatcaagcaggctctgctgacagcccctgctctgggactgcctgatctgaccaagcctttcgagctgttcgtggacgagaagcagggctatgccaaaggcgtgctgacacagaagctcggcccttggagaaggcctgtggcctacctgagcaagaaactggaccctgtggctgccggatggcctccttgtctgagaatggtggccgccattgccgtgctgaccaaggatgccggaaagctgacaatgggacagcctctggtcattctggcccctcatgccgtggaagccctcgtgaaacagcctcctgatcggtggctgagcaacgccaggatgacacactatcaggcactgctgctcgacaccgacagagtgcagtttggacctgtggtggccctgaatcctgccacacttctgcctctgcctgaggaaggcctccagcacaattgcctggacatcctggccgaggctcacggcacaagacccgatctgacagatcagccactgcctgacgccgaccacacctggtatacagatggcagctctctgctgcaagaaggacagagaaaagccggggctgccgtgaccaccgagacagaagtgatttgggccaaagctctgcccgctggcacatctgctcagagagccgaactgatcgccctgacacaggccctgaaaatggccgagggcaagaagctgaacgtctacaccgactccagatacgccttcgccaccgctcacatccacggcgaaatctatcggcggagaggatggctgaccagcgagggcaaagagattaagaacaaggacgagattctcgccctgctcaaggccctgttcctgcctaagcggctgagcatcatccactgtccaggccaccagaagggccactctgctgaagctagaggcaacagaatggccgaccaggctgccagaaaggccgccatcacagagacacccgataccagcacactgctgatcgagaacagcagccct

SEQ ID NO: 124 - DNA, 1485 bp, Synthetic construct
  source 1..1485: mol_type = other DNA
accctgaacatcgaggacgagtaccggctgcacgagacaagcaaagaacccgatgtgtccctgggcagcacctggcttagtgatttccctcaggcctgggccgagacaggcggaatgggacttgctgttagacaggcccctctgatcatccctctgaaggccacaagcacccctgtgtccatcaagcagtaccccatgagccaagaggcccggctgggaatcaagccccacattcagagactgctggaccagggcatcctggtgccttgtcagagcccttggaatacccctctgctgcccgtgaagaagcccggcaccaacgattacagacccgtgcaggacctgcgggaagtgaacaagagagtggaagatattcaccccaccgtgccgaatccttacaacctgctgtctggcctgcctcctagccaccagtggtacacagtgctggacctgaaggacgccttcttctgtctgcggctgcaccctacaagccagcctctgtttgcctttgagtggcgggaccctgagatgggcattagcggacagctgacctggaccagactgccccagggcttcaagaacagccccacactgttcaacgaggccctgcatagggacctcgccgacttcagaatccagcatcctgacctgatcctgctccagtacgtggacgatctgctgctggccgctacaagcgagctggattgtcagcagggaacaagagccctgctgcaaaccctgggcaacctgggctatagagcctctgccaagaaggcccagatttgccagaaacaagtgaagtatctgggctacctgctgaaagagggccagcgttggctgaccgaggccagaaaagaaaccgtgatgggccagcctacacctaagacacccagacagctgagagagttcctgggcaaagccggattctgtcggctgttcatccctggctttgccgagatggctgcccctctgtacccactgacaaagcccggaactctgttcaactggggcccagatcagcagaaggcctaccaagagatcaagcaggctctgctgacagcccctgctctgggactgcctgatctgaccaagcctttcgagctgttcgtggacgagaagcagggctatgccaaaggcgtgctgacacagaagctcggcccttggagaaggcctgtggcctacctgagcaagaaactggaccctgtggctgccggatggcctccttgtctgagaatggtggccgccattgccgtgctgaccaaggatgccggaaagctgacaatgggacagcctctggtcattctggcccctcatgccgtggaagccctcgtgaaacagcctcctgatcggtggctgagcaacgccaggatgacacactatcaggcactgctgctcgacaccgacagagtgcagtttggacctgtggtggccctgaatcctgccacacttctgcctctgcctgaggaaggcctccagcacaatagc

SEQ ID NO: 125 - DNA, 1278 bp, Synthetic construct
  source 1..1278: mol_type = other DNA
gacacctctaacctgatggaacagattctgagcagcgacaacctgaaccgggcctacctccaggttgtgcggaacaaaggcgctgaaggcgtcgacggcatgaagtacaccgaactgaaagagcacctggctaagaacggggagacaatcaaaggccagctgcggacccggaagtacaagccacaacctgcaagaagagtggaaatccccaagcctgatggcggcgtgcggaatcttggagtgcctaccgtgaccgacagattcattcagcaggccattgctcaggtgctcacccctatctacgaggaacagttccacgaccactcctacggcttcagacccaacagatgtgcacagcaggcaatcctgacagccctgaatatcatgaacgacggcaacgactggatcgtggacatcgatctggaaaagttcttcgacaccgtgaaccacgacaagctcatgaccctgatcggccggaccatcaaggatggcgacgtgatcagcatcgtcagaaagtacctggtgtctggcatcatgatcgacgatgagtacgaggacagcatcgtgggcacaccccaaggcggaaatctgtctcccctgctggctaacatcatgctgaacgaactcgacaaagaaatggaaaagcggggcctgaacttcgtcagatacgccgacgactgcatcatcatggtcggaagcgagatgagcgccaatagagtgatgcggaacatcagccggtttatcgaagagaaactggggctgaaagtgaacatgaccaagagcaaggtcgacagacccagcggcctgaagtatctcggcttcggcttctacttcgaccctcgggctcaccagttcaaggccaagcctcacgctaagtccgtggctaagttcaagaaacggatgaaggaactgacctgccggtcctggggcgtgtccaatagctataaggtggaaaagctgaaccagctcatccgaggctggatcaactactttaagatcggcagcatgaaaaccctgtgcaaagaactggactccagaatccggtacagactgcggatgtgcatctggaagcagtggaaaactccccagaatcaagagaaaaacctggtcaagctgggcatcgacagaaacaccgctcggagagtggcctacaccggcaagagaattgcctacgtgtgcaacaaaggggccgtgaacgtggcaatcagcaacaagagactggcctccttcggcctgatctccatgctggactactacatcgagaagtgcgtgacctgt

SEQ ID NO: 126 - DNA, 66 bp, Synthetic construct
  source 1..66: mol_type = other DNA
cctcctaagaagaagcggaaggtcgaggacggcgaaggacctgccgccaagagagtgaaactggac

SEQ ID NO: 127 - DNA, 105 bp, Synthetic construct
  source 1..105: mol_type = other DNA
ccacctaagaagaaacggaaggtcgaggacggcgagggccctgctgctaagagagtgaaactggactccggagctgctccagccgccaagaagaagaagctcgac

SEQ ID NO: 128 - DNA, 27 bp, Synthetic construct
  source 1..27: mol_type = other DNA
ccagccgccaagaagaagaagctcgac

SEQ ID NO: 129 - DNA, 21 bp, Synthetic construct
  source 1..21: mol_type = other DNA
cctaagaagaaaagaaaggtg

SEQ ID NO: 130 - DNA, 27 bp, Synthetic construct
  source 1..27: mol_type = other DNA
cctgctgctaagagagtgaaactggac

SEQ ID NO: 131 - DNA, 27 bp, Synthetic construct
  source 1..27: mol_type = other DNA
cctgctgccaagaagaaaaagctggac

SEQ ID NO: 132 - DNA, 27 bp, Synthetic construct
  source 1..27: mol_type = other DNA
cctgctgccaagaagaaaaagaacggc

SEQ ID NO: 133 - DNA, 81 bp, Synthetic construct
  source 1..81: mol_type = other DNA
ggacctggaagcgagcctgctacatctggctctgagacacctggcacctccgagtctgctacacctgaatctggacctggc

SEQ ID NO: 134 - DNA, 363 bp, Synthetic construct
  source 1..363: mol_type = other DNA
tctaagacaatcgtgctgtctgtgggcgaagccaccagaacactgaccgagatccagagcacagccgacagacagatcttcgaggaaaaagtgggccctctcgtgggcagactgagactgacagcttccctgagacagaacggcgccaagaccgcctacagagtgaacctgaagctggaccaggccgacgtggtggattctggccttcctaaagtgcggtacacccaagtgtggtcccacgacgtgaccatcgtggccaattctaccgaggccagcagaaagagcctgtacgacctgaccaagagcctggtggccacaagccaggtggaagatctggtcgtgaacctggtgcctctcggacgt

SEQ ID NO: 135 - DNA, 741 bp, Synthetic construct
  source 1..741: mol_type = other DNA
tctaagacaatcgtgctgtctgtgggcgaagccaccagaacactgaccgagatccagagcacagccgacagacagatcttcgaggaaaaagtgggccctctcgtgggcagactgagactgacagcttccctgagacagaacggcgccaagaccgcctacagagtgaacctgaagctggaccaggccgacgtggtggattctggccttcctaaagtgcggtacacccaagtgtggtcccacgacgtgaccatcgtggccaattctaccgaggccagcagaaagagcctgtacgacctgaccaagagcctggtggccacaagccaggtggaagatctggtcgtgaacctggtgcctctcggacgtggtggaagcggcggaagcaaaaccatcgtgctgtctgttggcgaggccacacggaccctgaccgagattcagtctaccgccgatcgccaaatctttgaagagaaagtggggccccttgtcggcaggcttaggctgacagcatctctgcgtcagaatggggccaaaacagcctaccgggtcaacctgaagctcgaccaggctgatgtggtcgattccggcctgccaaaagtccgctatacacaagtttggagccatgatgtgacaatcgtcgccaactccaccgaggcctctcggaagtctctgtatgatctgacaaaaagcctcgtggctaccagccaagtcgaagatctggtcgtgaacctcgtgcctcttggaaga

SEQ ID NO: 136 - DNA, 387 bp, Synthetic construct
  source 1..387: mol_type = other DNA
gctagcaacttcacccagttcgtgctggtggacaacggcggcacaggcgacgtgacagtggccccttctaacttcgctaacggcgtggccgagtggatcagcagcaacagcagatcccaggcctacaaagtgacctgctccgtgcggcagagcagcgcccagaagagaaagtacaccatcaaggtggaagtgcccaaggtggccacacagacagtgggcggcgaagaactgcctgtggctggctggcggagctacctgaacatggaactgaccatccccatcttcgccaccaacagcgactgcgagctgatcgtgaaggccatgcagggcctgctgaaggacggcaaccctatcccttctgctatcgccgccaactccggaatctat

SEQ ID NO: 137 - DNA, 24 bp, Synthetic construct
  source 1..24: mol_type = other DNA
gactacaaggacgacgacgataag

SEQ ID NO: 138 - DNA, 1500 bp, Synthetic construct
  source 1..1500: mol_type = other DNA
atgggcgctagagcctctgttctgtctggcggcgaactggacagatgggagaagatcagactgagacctggcggcaagaagaagtacaagctgaagcacatcgtgtgggccagcagagagctggaaagattcgctgtgaaccccggcctgctggaaacaagcgagggctgtagacagatcctgggccagctccagccatctctccagacaggatctgaggaactgagaagcctgtacaacaccgtggccacactgtactgcgtgcaccagagaatcgagatcaaggacaccaaagaggccctggacaagatcgaggaagaacagaacaagtctaagaagaaggcccagcaggctgccgccgatacaggccactctaatcaggtgtcccagaactaccccatcgtgcagaacatccagggccagatggtgcatcaggctatcagccccagaacactgaacgcctgggtcaaagtggtggaagagaaggctttcagccctgaagtgatccccatgttcagcgccctgtctgagggtgccacacctcaggacctgaacaccatgctgaacacagtcggcggacaccaggccgctatgcagatgctgaaagagacaatcaacgaagaggccgccgagtgggacagagtgcatcctgttcatgctggccctatcgctcccggccagatgagagaacctagaggctctgacattgccggcaccaccagcacactgcaagagcagatcggctggatgacaaacaaccctcctattcctgtgggcgagatctacaagagatggatcatcctgggactgaacaagatcgtgcggatgtacagccccaccagcatcctggacattagacagggccccaaagagcccttcagagactacgtggacagattctacaagaccctgagagccgagcaggccagccaagaagtgaagaactggatgaccgagacactgctggtgcagaacgctaaccccgactgcaagaccatcctgaaggctctgggacctgccgccacactggaagagatgatgacagcctgtcaaggcgtcggaggacctggccataaggctagagttctggccgaggccatgagccaagtgaccaacagcgccacaatcatgatgcagagaggcaacttcagaaaccagcggaagatcgtgaagtgcttcaactgcggcaaagagggccacaccgccagaaactgtagagcccctagaaagaaaggctgctggaagtgtggaaaagaggggcaccagatgaaggactgcaccgagagacaggccaacttcctgggcaagatctggcctagctacaagggcagacccggcaacttcctccagagcagaccagagcctaccgctcctcctgaggaatccttcagatccggcgtggaaaccaccacacctccacagaagcaagagcccatcgacaaagagctgtaccctctgaccagcctgagatccctgttcggcaacgaccctagctctcaa

SEQ ID NO: 139 - DNA, 1500 bp, Synthetic construct
  source 1..1500: mol_type = other DNA
atgggcgctagagcctctgttctgtctggcggcgaactggacagatgggagaagatcagaagcagacctggcggcaagaagaagtacaagctgaagcacatcgtgtgggccagcagagagctggaaagattcgctgtgaaccccggcctgctggaaacaagcgagggctgtagacagatcctgggccagctccagccatctctccagacaggatctgaggaactgagaagcctgtacaacaccgtggccacactgtactgcgtgcaccagagaatcgagatcaaggacaccaaagaggccctggacaagatcgaggaagaacagaacaagtctaagaagaaggcccagcaggctgccgccgatacaggccactctaatcaggtgtcccagaactaccccatcgtgcagaacatccagggccagatggtgcatcaggctatcagccccagaacactgaacgcctgggtcaaagtggtggaagagaaggctttcagccctgaagtgatccccatgttcagcgccctgtctgagggtgccacacctcaggacctgaacaccatgctgaacacagtcggcggacaccaggccgctatgcagatgctgaaagagacaatcaacgaagaggccgccgagtgggacagagtgcatcctgttcatgctggccctatcgctcccggccagatgagagaacctagaggctctgacattgccggcaccaccagcacactgcaagagcagatcggctggatgacaaacaaccctcctattcctgtgggcgagatctacaagagatggatcatcctgggactgaacaagatcgtgcggatgtacagccccaccagcatcctggacattagacagggccccaaagagcccttcagagactacgtggacagattctacaagaccctgagagccgagcaggccagccaagaagtgaagaactggatgaccgagacactgctggtgcagaacgctaaccccgactgcaagaccatcctgaaggctctgggacctgccgccacactggaagagatgatgacagcctgtcaaggcgtcggaggacctggccataaggctagagttctggccgaggccatgagccaagtgaccaacagcgccacaatcatgatgcagagaggcaacttcagaaaccagcggaagatcgtgaagtgcttcaactgcggcaaagagggccacaccgccagaaactgtagagcccctagaaagaaaggctgctggaagtgtggaaaagaggggcaccagatgaaggactgcaccgagagacaggccaacttcctgggcaagatctggcctagctacaagggcagacccggcaacttcctccagagcagaccagagcctaccgctcctcctgaggaatccttcagatccggcgtggaaaccaccacacctccacagaagcaagagcccatcgacaaagagctgtaccctctgaccagcctgagatccctgttcggcaacgaccctagctctcaa

SEQ ID NO: 140 - DNA, 558 bp, Synthetic construct
  source 1..558: mol_type = other DNA
atgcagagaggcaacttcagaaaccagcggaagatcgtgaagtccttcaactccggcaaagagggccacaccgcccgcaattctagagcccctagaaagaaaggtggatccggcggcgtttctggatggcggctgttcaagaagatcagcggcggagctagctctaagacaatcgtgctgtctgtgggcgaagccaccagaacactgaccgagatccagagcacagccgacagacagatcttcgaggaaaaagtgggccctctcgtgggcagactgagactgacagcttccctgagacagaacggcgccaagaccgcctacagagtgaacctgaagctggaccaggccgacgtggtggattctggccttcctaaagtgcggtacacccaagtgtggtcccacgacgtgaccatcgtggccaattctaccgaggccagcagaaagagcctgtacgacctgaccaagagcctggtggccacaagccaggtggaagatctggtcgtgaacctggtgcctctcggacgtggcggatccggtggaaccgagagacaggccaac

SEQ ID NO: 141 - DNA, 603 bp, Synthetic construct
  source 1..603: mol_type = other DNA
atgcagagaggcaacttcagaaaccagcggaagatcgtgaagtgcttcaactgcggcaaagagggccacaccgccagaaactgtagagcccctagaaagaaaggctgctggaagtgtggaaaagaggggcaccagatgaaggactgcggtggatccggcggcgtttctggatggcggctgttcaagaagatcagcggcggagctagctctaagacaatcgtgctgtctgtgggcgaagccaccagaacactgaccgagatccagagcacagccgacagacagatcttcgaggaaaaagtgggccctctcgtgggcagactgagactgacagcttccctgagacagaacggcgccaagaccgcctacagagtgaacctgaagctggaccaggccgacgtggtggattctggccttcctaaagtgcggtacacccaagtgtggtcccacgacgtgaccatcgtggccaattctaccgaggccagcagaaagagcctgtacgacctgaccaagagcctggtggccacaagccaggtggaagatctggtcgtgaacctggtgcctctcggacgtggcggatccggtggaaccgagagacaggccaac

SEQ ID NO: 142 - DNA, 561 bp, Synthetic construct
  source 1..561: mol_type = other DNA
atggaccactacctggacatcagactgcggcccgatcctgagtttcctccagctcagctgatgagcgtgctgttcggcaaactgcaccaggctctggttgcccaaggcggcgatagaatcggagtgtcattccccgacctggacgagagcagaagcagactgggagagagactgagaatccacgccagcgccgatgatctgagagccctgcttgctagaccttggctggaaggcctgagagatcacctccagtttggagagcctgccgtggtgcctcatccaacaccatatagacaggtgtccagagtgcaggccaagagcaaccccgaaagactgcggagaaggctgatgcggagacacgacctgtctgaggaagaggcccggaagagaatccccgacacagtggctagagccctggacctgcctttcgtgacactgagaagccagagcaccggccagcacttccggctgtttatcagacacggccctctgcaagtgaccgccgaagaaggcggctttacctgttacggcctgagcaaaggcggattcgtgccctggttt

SEQ ID NO: 143 - DNA, 33 bp, Synthetic construct
  source 1..33: mol_type = other DNA
ctgcaactgcctccactggaaagactgacactg

SEQ ID NO: 144 - DNA, 369 bp, Synthetic construct
  source 1..369: mol_type = other DNA
caggttcagctggttgaatccggaggcggactggttcaagctggcggatctctgagactgagctgtgccgccagcggctactttagcagctatgctatgggctggttccggcaggcccctggaaaagagagagagtttgtcgccgccatcagctggatcgagagcaccacagattacgccgacagcgtgaagggcagattcaccatcagccgggacaacgccaagaaaaccctgcacctccagatgaacagcctgaagcctgaggacaccgccgtgtactattgtgccgcctgcgacatccctttcggccaggctttttgcgccctgtacgattattggggccagggcacccaagtgaccgtgtcatct

SEQ ID NO: 145 - DNA, 33 bp, Synthetic construct
  source 1..33: mol_type = other DNA
gtttctggatggcggctgttcaagaagatcagc

SEQ ID NO: 146 - DNA, 396 bp, Synthetic construct
  source 1..396: mol_type = other DNA
cacggcctgcaggacgaccctgatctgcaggccctgctgaagggcagccagctgctgaaagtgaagtccagcagctggcggcgggaaagattctacaagctgcaagaggactgcaagaccatctggcaggagtctagaaaggtgatgcgctccccagaaagccaactgttcagcatcgaggacatccaggaggtgcggatgggccacagaacagagggactggaaaagttcgccagagatatccccgaggatagatgttttagcattgtgttcaaggaccagcggaacaccctggacctgatcgcccctagccctgctgatgcccagcattgggtccagggcctcagaaagatcatccaccacagcggctctatggaccagagacagaaactgcag

SEQ ID NO: 147 - DNA, 99 bp, Synthetic construct
  source 1..99: mol_type = other DNA
agaatgaagcagctggaagataaggtggaagaactgctgagcaagaactaccacctggaaaacgaggtggcccggctgaagaagctcgttggagaaaga

SEQ ID NO: 148 - DNA, 99 bp, Synthetic construct
  source 1..99: mol_type = other DNA
aggatgaagcagatcgaggacaagatcgaagagatcctgagcaaaatctaccacatcgagaacgagatcgcccggatcaagaagctgattggcgagaga

SEQ ID NO: 149 - DNA, 717 bp, Synthetic construct
  source 1..717: mol_type = other DNA
gtgagcaagggcgaggagctgttcaccggggtggtgcccatcctggtcgagctggacggcgacgtaaacggccacaagttcagcgtccgcggcgagggcgagggcgatgccaccaacggcaagctgaccctgaagttcatctgcaccaccggcaagctgcccgtgccctggcccaccctcgtgaccaccttaggctacggcgtggcctgcttcgcccgctaccccgaccacatgaagcagcacgacttcttcaagtccgccatgcccgaaggctacgtccaggagcgcaccatctctttcaaggacgacggcacctacaagacccgcgccgaggtgaagttcgagggcgacaccctggtgaaccgcatcgtgctgaagggcatcgacttcaaggaggacggcaacatcctggggcacaagctggagtacaacttcaacagccacaaggtctatatcacggccgacaagcagaagaacggcatcaaggctaacttcaagacccgccacaacgttgaggacggcggcgtgcagctcgccgaccactaccagcagaacacccccatcggcgacggccccgtgctgctgcccgacaaccactacctgagccatcagtccaaactgagcaaagaccccaacgagaagcgcgatcacatggtcctgaaggagagggtgaccgccgccgggattacacatgacatggacgagctgtacaagtag

SEQ ID NO: 150 - DNA, 699 bp, Synthetic construct
  source 1..699: mol_type = other DNA
atggtttctaaaggcgaggccgtgatcaaagagttcatgaggttcaaggtgcacatggaaggcagcatgaacggccacgagttcgagatcgaaggcgaaggcgagggcagaccttacgagggaactcagaccgccaagctgaaagtgaccaaaggcggccctctgcctttcagctgggacatcctgtctccacagtttatgtacggcagcagggccttcatcaagcaccccgctgacatccccgactactacaagcagtctttcccagagggcttcaagtgggagagagtgatgaacttcgaggacggcggagccgtgactgtgacacaggacacatctctggaagatgggaccctgatctacaaagtgaagctgcggggcacaaacttccctccagacggccctgtgatgcagaaaaagacaatgggctgggaagccagcaccgagagactgtaccctgaagatggcgtgctgaagggcgacatcaagatggccctgagactgaaggatggcggcagatacctggccgacttcaagaccacctacaaggccaagaaacctgtgcagatgcctggcgcctacaacgtggacagaaagctggacatcaccagccacaacgaggactacaccgtggtggaacagtacgagagaagcgaggggagacacagcacaggcggaatggacgagctgtacaagtag

SEQ ID NO: 151 - DNA, 387 bp, Synthetic construct
  source 1..387: mol_type = other DNA
atgggagctagagcatctgttctgtctggcggagcacagcaggccgctgctgatacaggccactctaatcaggtgtcccagaactacagccccacctccatcctggacatcagacagggccccaaagagcccttccgggactacgtggacagattctacaagaccctgagagccgagcaggccagccaagaagtgaagaactggatgaccgagacactgctggtgcagaacgccaatcctgactgcaagaccatcctgaaggctctgggacctgccgccacactggaagagatgatgacagcctgtcaaggcgttggcggccctggacacaaagctagagttctggccgaggccatgagccaagtgaccaactccgctaccatcatg

SEQ ID NO: 152 - DNA, 735 bp, Synthetic construct
  source 1..735: mol_type = other DNA
cccatcgtgcagaacatccagggccagatggtgcatcaggctatcagccccagaacactgaacgcctgggtcaaagtggtggaagagaaggctttcagccctgaagtgatccccatgttcagcgccctgtctgagggtgccacacctcaggacctgaacaccatgctgaacacagtcggcggacaccaggccgctatgcagatgctgaaagagacaatcaacgaagaggccgccgagtgggacagagtgcatcctgttcatgctggccctatcgctcccggccagatgagagaacctagaggctctgacattgccggcaccaccagcacactgcaagagcagatcggctggatgacaaacaaccctcctattcctgtgggcgagatctacaagagatggatcatcctgggactgaacaagatcgtgcggatgtacagccccacctccatcctggacatcagacagggccccaaagagcccttccgggactacgtggacagattctacaagaccctgagagccgagcaggccagccaagaagtgaagaactggatgaccgagacactgctggtgcagaacgccaatcctgactgcaagaccatcctgaaggctctgggacctgccgccacactggaagagatgatgacagcctgtcaaggcgttggcggccctggacacaaagctagagttctggccgaggccatgagccaagtgaccaactccgctaccatcatg

SEQ ID NO: 153 - DNA, 156 bp, Synthetic construct
  source 1..156: mol_type = other DNA
ctccagagcagacctgaacctacagctccaccagaggaatccttccgcagcggcgtggaaaccacaacacctccacagaagcaagagcccatcgacaaagagctgtaccctctgaccagcctgagaagcctgttcggcaacgatcccagcagccag

SEQ ID NO: 154 - DNA, 1026 bp, Synthetic construct
  source 1..1026: mol_type = other DNA
agcaacctgctgaccgtgcaccagaacctgcctgctctgcctgtggacgccacatctgatgaagtgcggaagaacctgatggacatgttcagagacagacaggccttcagcgagcacacctggaagatgctgctgagcgtgtgtagaagctgggccgcttggtgcaagctgaacaacagaaagtggttccccgccgagcctgaggacgtgcgagattacctgctgtacctgcaagctagaggcctggccgtgaaaaccatccagcagcacctgggccagctgaacatgctgcacagaagaagcggcctgcctagacctagcgacagcaacgctgtgtccctggtcatgagaaggattcggaaagaaaacgtggacgctggcgagagagctaagcaggctctggccttcgagagaaccgacttcgatcaagtgcgcagcctgatggaaaacagcgacagatgccaggatattcggaacctggccttcctgggaatcgcctacaacaccctgctgagaatcgccgagatcgccagaatcagagtgaaggacatcagcagaaccgacggcggcagaatgctgatccacatcggcagaacaaagaccctggtgtccacagctggcgtcgagaaggctctgagtctgggcgtgacaaagctggtggaaagatggatcagcgtgtccggcgtggccgacgatcctaacaactacctgttctgtcgcgtgcgcaagaacggcgtggcagctccttctgctacaagccagctgagcacaagagccctggaaggcatcttcgaggccacacacagactgatctacggcgccaaggatgacagcggccagagataccttgcttggagcggccacagtgctagagtgggcgctgctagagacatggctagagcaggcgtgtcaatccccgagatcatgcaagctggcggctggaccaacgtgaacatcgtgatgaactacatccgcaacctggacagcgagacaggcgctatggttcgactgcttgaagatggcgac

SEQ ID NO: 155 - DNA, 363 bp, Synthetic construct; identical to SEQ ID NO: 134
  source 1..363: mol_type = other DNA

SEQ ID NO: 156 - DNA, 741 bp, Synthetic construct
  source 1..741: mol_type = other DNA
tctaagacaatcgtgctgtctgtgggcgaagccaccagaacactgaccgagatccagagcacagccgacagacagatcttcgaggaaaaagtgggccctctcgtgggcagactgagactgacagcttccctgagacagaacggcgccaagaccgcctacagagtgaacctgaagctggaccaggccgacgtggtggattctggccttcctaaagtgcggtacacccaagtgtggtcccacgacgtgaccatcgtggccaattctaccgaggccagcagaaagagcctgtacgacctgaccaagagcctggtggccacaagccaggtggaagatctggtcgtgaacctggtgcctctcggacgtggcggctctggcggatctaaaaccattgtgctgagcgtcggcgaggccacaaggaccctgacagagattcagtccaccgccgaccggcagatttttgaagagaaagtggggccactcgtcggaaggcttaggctgactgcaagcctgaggcagaatggggccaaaacagcttaccgggtcaacctgaaactcgatcaggctgatgtggtcgacagcggcctgccaaaagtccgctacacacaagtttggagccatgatgtgacaatcgtcgccaacagcaccgaggcctctaggaagtccctgtacgatctcacaaagtctctggtggcaacctctcaggtcgaggatctggtggtcaatctcgtgcccctgggcaga

SEQ ID NO: 157 - DNA, 741 bp, Synthetic construct
  source 1..741: mol_type = other DNA
tctaagacaatcgtgctgtctgtgggcgaagccaccagaacactgaccgagatccagagcacagccgacagacagatcttcgaggaaaaagtgggccctctcgtgggcagactgagactgacagcttccctgagacagaacggcgccaagaccgcctacagagtgaacctgaagctggaccaggccgacgtggtggattctggccttcctaaagtgcggtacacccaagtgtggtcccacgacgtgaccatcgtggccaattctaccgaggccagcagaaagagcctgtacgacctgaccaagagcctggtggccacaagccaggtggaagatctggtcgtgaatctcgtgcccctgggcagaggcggctctggcggatctaaaaccattgtgctgagcgtcggcgaggccacaaggaccctgacagagattcagtccaccgccgaccggcagatttttgaagagaaagtggggccactcgtcggaaggcttaggctgactgcaagcctgaggcagaatggggccaaaacagcttaccgggtcaacctgaaactcgatcaggctgatgtggtcgacagcggcctgccaaaagtccgctacacacaagtttggagccatgatgtgacaatcgtcgccaacagcaccgaggcctctaggaagtccctgtacgatctcacaaagtctctggtggcaacctctcaggtcgaggatctggtggtcaatctcgtgcctctcggacgt

SEQ ID NO: 158 - DNA, 1998 bp, Synthetic construct
  source 1..1998: mol_type = other DNA
atggcgcgttcaacgctctcaaaaccccttaaaaataaggttaacccgcgaggccccctaatccccttaattcttctgatgctcagaggggtcagtactgcttcgcccggctccagtcctcatcaagtctataatatcacctgggaggtaaccaatggagatcgggagacggtatgggcaacttctggcaaccaccctctgtggacctggtggcctgaccttaccccagatttatgtatgttagcccaccatggaccatcttattgggggctagaatatcaatcccctttttcttctcccccggggcccccttgttgctcagggggcagcagcccaggctgttccagagactgcgaagaacctttaacctccctcacccctcggtgcaacactgcctggaacagactcaagctagaccagacaactcataaatcaaatgagggattttatgtttgccccgggccccaccgcccccgagaatccaagtcatgtgggggtccagactccttctactgtgcctattggggctgtgagacaaccggtagagcttactggaagccctcctcatcatgggatttcatcacagtaaacaacaatctcacctctgaccaggctgtccaggtatgcaaagataataagtggtgcaaccccttagttattcggtttacagacgccgggagacgggttacttcctggaccacaggacattactggggcttacgtttgtatgtctccggacaagatccagggcttacatttgggatccgactcagataccaaaatctaggaccccgcgtcccaatagggccaaaccccgttctggcagaccaacagccactctccaagcccaaacctgttaagtcgccttcagtcaccaaaccacccagtgggactcctctctcccctacccaacttccaccggcgggaacggaaaataggctgctaaacttagtagacggagcctaccaagccctcaacctcaccagtcctgacaaaacccaagagtgctggttgtgtctagtagcgggacccccctactacgaaggggttgccgtcctgggtacctactccaaccatacctctgctccagccaactgctccgtggcctcccaacacaagttgaccctgtccgaagtgaccggacagggactctgcataggagcagttcccaaaacacatcaggccctatgtaataccacccagacaagcagtcgagggtcctattatctagttgcccctacaggtaccatgtgggcttgtagtaccgggcttactccatgcatctccaccaccatactgaaccttaccactgattattgtgttcttgtcgaactctggccaagagtcacctatcattcccccagctatgtttacggcctgtttgagagatccaaccgacacaaaagagaaccggtgtcgttaaccctggccctattattgggtggactaaccatggggggaattgccgctggaataggaacagggactactgctctaatggccactcagcaattccagcagctccaagccgcagtacaggatgatctcagggaggttgaaaaatcaatctctaacctagaaaagtctctcacttccctgtctgaagttgtcctacagaatcgaaggggcctagacttgttatttctaaaagaaggagggctgtgtgctgctctaaaagaagaatgttgcttctatgcggaccacacaggactagtgagagacagcatggccaaattgagagagaggcttaatcagagacagaaactgtttgagtcaactcaaggatggtttgagggactgtttaacagatccccttggtttaccaccttgatatctaccattatgggacccctcattgtactcctaatgattttgctcttcggaccctgcattcttaatcgattagtccaatttgttaaagacaggatatcagtggtccaggctctagttttgactcaacaatatcaccagctgaagcctatagagtacgagccatag

SEQ ID NO: 159 - DNA, 1950 bp, Synthetic construct
  source 1..1950: mol_type = other DNA
atggcgcgttcaacgctctcaaaaccccttaaaaataaggttaacccgcgaggccccctaatccccttaattcttctgatgctcagaggggtcagtactgcttcgcccggctccagtcctcatcaagtctataatatcacctgggaggtaaccaatggagatcgggagacggtatgggcaacttctggcaaccaccctctgtggacctggtggcctgaccttaccccagatttatgtatgttagcccaccatggaccatcttattgggggctagaatatcaatcccctttttcttctcccccggggcccccttgttgctcagggggcagcagcccaggctgttccagagactgcgaagaacctttaacctccctcacccctcggtgcaacactgcctggaacagactcaagctagaccagacaactcataaatcaaatgagggattttatgtttgccccgggccccaccgcccccgagaatccaagtcatgtgggggtccagactccttctactgtgcctattggggctgtgagacaaccggtagagcttactggaagccctcctcatcatgggatttcatcacagtaaacaacaatctcacctctgaccaggctgtccaggtatgcaaagataataagtggtgcaaccccttagttattcggtttacagacgccgggagacgggttacttcctggaccacaggacattactggggcttacgtttgtatgtctccggacaagatccagggcttacatttgggatccgactcagataccaaaatctaggaccccgcgtcccaatagggccaaaccccgttctggcagaccaacagccactctccaagcccaaacctgttaagtcgccttcagtcaccaaaccacccagtgggactcctctctcccctacccaacttccaccggcgggaacggaaaataggctgctaaacttagtagacggagcctaccaagccctcaacctcaccagtcctgacaaaacccaagagtgctggttgtgtctagtagcgggacccccctactacgaaggggttgccgtcctgggtacctactccaaccatacctctgctccagccaactgctccgtggcctcccaacacaagttgaccctgtccgaagtgaccggacagggactctgcataggagcagttcccaaaacacatcaggccctatgtaataccacccagacaagcagtcgagggtcctattatctagttgcccctacaggtaccatgtgggcttgtagtaccgggcttactccatgcatctccaccaccatactgaaccttaccactgattattgtgttcttgtcgaactctggccaagagtcacctatcattcccccagctatgtttacggcctgtttgagagatccaaccgacacaaaagagaaccggtgtcgttaaccctggccctattattgggtggactaaccatggggggaattgccgctggaataggaacagggactactgctctaatggccactcagcaattccagcagctccaagccgcagtacaggatgatctcagggaggttgaaaaatcaatctctaacctagaaaagtctctcacttccctgtctgaagttgtcctacagaatcgaaggggcctagacttgttatttctaaaagaaggagggctgtgtgctgctctaaaagaagaatgttgcttctatgcggaccacacaggactagtgagagacagcatggccaaattgagagagaggcttaatcagagacagaaactgtttgagtcaactcaaggatggtttgagggactgtttaacagatccccttggtttaccaccttgatatctaccattatgggacccctcattgtactcctaatgattttgctcttcggaccctgcattcttaatcgattagtccaatttgttaaagacaggatatcagtggtccaggctctatag

SEQ ID NO: 160 - DNA, 87 bp, Synthetic construct
  source 1..87: mol_type = other DNA
gtttcagagctatgctggaaacagcatagcaagttgaaataaggctagtccgttatcaacttgaaaaagtggcaccgagtcggtgct

SEQ ID NO: 161 - DNA, 87 bp, Synthetic construct
  source 1..87: mol_type = other DNA
gtttaagagctatgctggaaacagcatagcaagtttaaataaggctagtccgttatcaacttgaaaaagtggcaccgagtcggtgct

SEQ ID NO: 162 - DNA, 92 bp, Synthetic construct
  source 1..92: mol_type = other DNA
gtttcagagccaccagaagatatggcttcggtggcaagttgaaataaggctagtccgttatcaacttgaaaaagtggcaccgagtcggtgct

SEQ ID NO: 163 - DNA, 106 bp, Synthetic construct
  source 1..106: mol_type = other DNA
gttttagagctatgctggaccagaagatatggcttcggttcagcatagcaagttaaaataaggctagtccgttatcaacttgaaaaagtggcaccgagtcggtgct

SEQ ID NO: 164 - DNA, 106 bp, Synthetic construct
  source 1..106: mol_type = other DNA
gtttaagagctatgctggaccagaagatatggcttcggttcagcatagcaagtttaaataaggctagtccgttatcaacttgaaaaagtggcaccgagtcggtgct

SEQ ID NO: 165 - RNA, 87 nt, Synthetic construct
  source 1..87: mol_type = other RNA; note = uracil
gtttcagagctatgctggaaacagcatagcaagttgaaataaggctagtccgttatcaacttgaaaaagtggcaccgagtcggtgct

SEQ ID NO: 166 - RNA, 87 nt, Synthetic construct
  source 1..87: mol_type = other RNA; note = uracil
gtttaagagctatgctggaaacagcatagcaagtttaaataaggctagtccgttatcaacttgaaaaagtggcaccgagtcggtgct

SEQ ID NO: 167 - RNA, 92 nt, Synthetic construct
  source 1..92: mol_type = other RNA; note = uracil
gtttcagagccaccagaagatatggcttcggtggcaagttgaaataaggctagtccgttatcaacttgaaaaagtggcaccgagtcggtgct

SEQ ID NO: 168 - RNA, 106 nt, Synthetic construct
  source 1..106: mol_type = other RNA; note = uracil
gttttagagctatgctggaccagaagatatggcttcggttcagcatagcaagttaaaataaggctagtccgttatcaacttgaaaaagtggcaccgagtcggtgct

SEQ ID NO: 169 - RNA, 106 nt, Synthetic construct
  source 1..106: mol_type = other RNA; note = uracil
gtttaagagctatgctggaccagaagatatggcttcggttcagcatagcaagtttaaataaggctagtccgttatcaacttgaaaaagtggcaccgagtcggtgct

SEQ ID NO: 170 - DNA, 37 bp, Synthetic construct
  source 1..37: mol_type = other DNA
cgcggttctatctagttacgcgttaaaccaactagaa

SEQ ID NO: 171 - RNA, 37 nt, Synthetic construct
  source 1..37: mol_type = other RNA; note = uracil
cgcggttctatctagttacgcgttaaaccaactagaa

SEQ ID NO: 172 - DNA, 249 bp, Synthetic construct
  source 1..249: mol_type = other DNA
gagggcctatttcccatgattccttcatatttgcatatacgatacaaggctgttagagagataattggaattaatttgactgtaaacacaaagatattagtacaaaatacgtgacgtagaaagtaataatttcttgggtagtttgcagttttaaaattatgttttaaaatggactatcatatgcttaccgtaacttgaaagtatttcgatttcttggctttatatatcttgtggaaaggacgaaacacc

SEQ ID NO: 173 - DNA, 1671 bp, Synthetic construct
  source 1..1671: mol_type = other DNA
gacattgattattgactagttattaatagtaatcaattacggggtcattagttcatagcccatatatggagttccgcgttacataacttacggtaaatggcccgcctggctgaccgcccaacgacccccgcccattgacgtcaataatgacgtatgttcccatagtaacgccaatagggactttccattgacgtcaatgggtggagtatttacggtaaactgcccacttggcagtacatcaagtgtatcatatgccaagtacgccccctattgacgtcaatgacggtaaatggcccgcctggcattatgcccagtacatgaccttatgggactttcctacttggcagtacatctacgtattagtcatcgctattaccatggtcgaggtgagccccacgttctgcttcactctccccatctcccccccctccccacccccaattttgtatttatttattttttaattattttgtgcagcgatgggggcggggggggggggggggcgcgcgccaggcggggcggggcggggcgaggggcggggcggggcgaggcggagaggtgcggcggcagccaatcagagcggcgcgctccgaaagtttccttttatggcgaggcggcggcggcggcggccctataaaaagcgaagcgcgcggcgggcgggagtcgctgcgtcgcgccttcgccccgtgccccgctccgccgccgcctcgcgccgcccgccccggctctgactgaccgcgttactcccacaggtgagcgggcgggacggcccttctcctccgggctgtaattagcgcttggtttaatgacggctcgtttcttttctgtggctgcgtgaaagccttaaagggctccgggagggccctttgtgcgggggggagcggctcggggggtgcgtgcgtgtgtgtgtgcgtggggagcgccgcgtgcggcccgcgctgcccggcggctgtgagcgctgcgggcgcggcgcggggctttgtgcgctccgcgtgtgcgcgaggggagcgcggccgggggcggtgccccgcggtgcgggggggctgcgaggggaacaaaggctgcgtgcggggtgtgtgcgtgggggggtgagcagggggtgtgggcgcggcggtcgggctgtaacccccccctgcacccccctccccgagttgctgagcacggcccggcttcgggtgcggggctccgtgcggggcgtggcgcggggctcgccgtgccgggcggggggtggcggcaggtgggggtgccgggcggggcggggccgcctcgggccggggagggctcgggggaggggcgcggcggccccggagcgccggcggctgtcgaggcgcggcgagccgcagccattgccttttatggtaatcgtgcgagagggcgcagggacttcctttgtcccaaatctggcggagccgaaatctgggaggcgccgccgcaccccctctagcgggcgcgggcgaagcggtgcggcgccggcaggaaggaaatgggcggggagggccttcgtgcgtcgccgcgccgccgtccccttctccatctccagcctcggggctgccgcagggggacggctgccttcgggggggacggggcagggcggggttcggcttctggcgtgtgaccggcggctctagagcctctgctaaccatgttcatgccttcttctttttcctacag

SEQ ID NO: 174 - DNA, 225 bp, Synthetic construct
  source 1..225: mol_type = other DNA
ctgtgccttctagttgccagccatctgttgtttgcccctcccccgtgccttccttgaccctggaaggtgccactcccactgtcctttcctaataaaatgaggaaattgcatcgcattgtctgagtaggtgtcattctattctggggggtggggtggggcaggacagcaagggggaggattgggaagacaatagcaggcatgctggggatgcggtgggctctatgg

SEQ ID NO: 175-176 - skipped (2 entries)

SEQ ID NO: 177 - DNA, 20 bp, Synthetic construct
  source 1..20: mol_type = other DNA
ctcccacaacgaagactgac

SEQ ID NO: 178 - RNA, 20 nt, Synthetic construct
  source 1..20: mol_type = other RNA; note = uracil
ctcccacaacgaagactgac

SEQ ID NO: 179 - DNA, 21 bp, Synthetic construct
  source 1..21: mol_type = other DNA
gctcccacaacgaagactgac

SEQ ID NO: 180 - RNA, 21 nt, Synthetic construct
  source 1..21: mol_type = other RNA; note = uracil
gctcccacaacgaagactgac

SEQ ID NO: 181 - DNA, 20 bp, Synthetic construct
  source 1..20: mol_type = other DNA
gtcccacaacgaagactgac

SEQ ID NO: 182 - RNA, 20 nt, Synthetic construct
  source 1..20: mol_type = other RNA; note = uracil
gtcccacaacgaagactgac

SEQ ID NO: 183 - DNA, 84 bp, Synthetic construct
  source 1..84: mol_type = other DNA
ggccggcatggtcccagcctcctcgctggcgccggctgggcaacattccgaggggaccgtcccctcggtaatggcgaatgggac

SEQ ID NO: 184 - RNA, 84 nt, Synthetic construct
  source 1..84: mol_type = other RNA; note = uracil
ggccggcatggtcccagcctcctcgctggcgccggctgggcaacattccgaggggaccgtcccctcggtaatggcgaatgggac

SEQ ID NO: 185 - DNA, 50 bp, Synthetic construct
  source 1..50: mol_type = other DNA
gggtcaggagcccccccctgaacccaggataaccctcaaagtcggggggc

SEQ ID NO: 186 - RNA, 50 nt, Synthetic construct
  source 1..50: mol_type = other RNA; note = uracil
gggtcaggagcccccccctgaacccaggataaccctcaaagtcggggggc

SEQ ID NO: 187 - DNA, 33 bp, Synthetic construct
  source 1..33: mol_type = other DNA
ctgaccagctatgaggtcatacatcgtcatagc

SEQ ID NO: 188 - RNA, 33 nt, Synthetic construct
  source 1..33: mol_type = other RNA; note = uracil
ctgaccagctatgaggtcatacatcgtcatagc

SEQ ID NO: 189 - DNA, 26 bp, Synthetic construct
  source 1..26: mol_type = other DNA
cgcggcaccgtccgcggaacaaacgg

SEQ ID NO: 190 - RNA, 26 nt, Synthetic construct
  source 1..26: mol_type = other RNA; note = uracil
cgcggcaccgtccgcggaacaaacgg

SEQ ID NO: 191 - DNA, 27 bp, Synthetic construct
  source 1..27: mol_type = other DNA
tccggtcgactccggagaaacaaagtc

SEQ ID NO: 192 - RNA, 27 nt, Synthetic construct
  source 1..27: mol_type = other RNA; note = uracil
tccggtcgactccggagaaacaaagtc

SEQ ID NO: 193 - DNA, 12 bp, Synthetic construct
  source 1..12: mol_type = other DNA
ggacttcggtcc

SEQ ID NO: 194 - RNA, 12 nt, Synthetic construct
  source 1..12: mol_type = other RNA; note = uracil
ggacttcggtcc

SEQ ID NO: 195 - DNA, 23 bp, Synthetic construct
  source 1..23: mol_type = other DNA
gaccagaagatatggcttcggtt

SEQ ID NO: 196 - RNA, 23 nt, Synthetic construct
  source 1..23: mol_type = other RNA; note = uracil
gaccagaagatatggcttcggtt

SEQ ID NO: 197 - DNA, 23 bp, Synthetic construct
  source 1..23: mol_type = other DNA
caccagaagatatggcttcggtg

SEQ ID NO: 198 - RNA, 23 nt, Synthetic construct
  source 1..23: mol_type = other RNA; note = uracil
caccagaagatatggcttcggtg

SEQ ID NO: 199 - DNA, 23 bp, Synthetic construct
  source 1..23: mol_type = other DNA
gcacagaagatatggcttcgtgc

SEQ ID NO: 200 - RNA, 23 nt, Synthetic construct
  source 1..23: mol_type = other RNA; note = uracil
gcacagaagatatggcttcgtgc

SEQ ID NO: 201 - DNA, 27 bp, Synthetic construct
  source 1..27: mol_type = other DNA
gcgcacagaagatatggcttcgtgcgc

SEQ ID NO: 202 - RNA, 27 nt, Synthetic construct
  source 1..27: mol_type = other RNA; note = uracil
gcgcacagaagatatggcttcgtgcgc

SEQ ID NO: 203 - DNA, 25 bp, Synthetic construct
  source 1..25: mol_type = other DNA
acaggagtttatatggaaaccctgt

SEQ ID NO: 204 - RNA, 25 nt, Synthetic construct
  source 1..25: mol_type = other RNA; note = uracil
acaggagtttatatggaaaccctgt

SEQ ID NO: 205 - DNA, 25 bp, Synthetic construct
  source 1..25: mol_type = other DNA
taaggagtttatatggaaaccctta

SEQ ID NO: 206 - RNA, 25 nt, Synthetic construct
  source 1..25: mol_type = other RNA; note = uracil
taaggagtttatatggaaaccctta

SEQ ID NO: 207 - DNA, 19 bp, Synthetic construct
  source 1..19: mol_type = other DNA
acatgaggattacccatgt

SEQ ID NO: 208 - RNA, 19 nt, Synthetic construct
  source 1..19: mol_type = other RNA; note = uracil
acatgaggattacccatgt

SEQ ID NO: 209 - DNA, 19 bp, Synthetic construct
  source 1..19: mol_type = other DNA
acatgaggatcacccatgt

SEQ ID NO: 210 - RNA, 19 nt, Synthetic construct
  source 1..19: mol_type = other RNA; note = uracil
acatgaggatcacccatgt

SEQ ID NO: 211 - DNA, 19 bp, Synthetic construct
  source 1..19: mol_type = other DNA
acatgaggataacccatgt

SEQ ID NO: 212 - RNA, 19 nt, Synthetic construct
  source 1..19: mol_type = other RNA; note = uracil
acatgaggataacccatgt

SEQ ID NO: 213 - DNA, 14 bp, Synthetic construct
  source 1..14: mol_type = other DNA
ccacagtcactggg

SEQ ID NO: 214 - RNA, 14 nt, Synthetic construct
  source 1..14: mol_type = other RNA; note = uracil
ccacagtcactggg

SEQ ID NO: 215 - DNA, 16 bp, Synthetic construct
  source 1..16: mol_type = other DNA
actgccgtataggcag

SEQ ID NO: 216 - RNA, 16 nt, Synthetic construct
  source 1..16: mol_type = other RNA; note = uracil
actgccgtataggcag

SEQ ID NO: 217 - DNA, 72 bp, Synthetic construct
  source 1..72: mol_type = other DNA
gccagggtagctcaattggtagagcatcaggctagtatcctgtcggttccggttcaagtccgggccctggtt

SEQ ID NO: 218 - RNA, 72 nt, Synthetic construct
  source 1..72: mol_type = other RNA; note = uracil
gccagggtagctcaattggtagagcatcaggctagtatcctgtcggttccggttcaagtccgggccctggtt

SEQ ID NO: 219 - DNA, 72 bp, Synthetic construct
  source 1..72: mol_type = other DNA
ggttccatggtgtaatggttagcactctggactctgaatccagcgatccgagttcaaatctcggtggaacct

SEQ ID NO: 220 - RNA, 72 nt, Synthetic construct
  source 1..72: mol_type = other RNA; note = uracil
ggttccatggtgtaatggttagcactctggactctgaatccagcgatccgagttcaaatctcggtggaacct

SEQ ID NO: 221 - DNA, 836 bp, Synthetic construct
  source 1..836: mol_type = other DNA
atggtgagcaagggcgaggagctgttcaccggggtggtgcccatcctggtcgagctggacggcgacgtaaacggccacaagttcagcgtccgcggcgagggcgagggcgatgccaccaacggcaagctgaccctgaagttcatctgcaccaccggcaagctgcccgtgccctggcccaccctcgtgaccaccttaggctacggcgtggcctgcttcgcccgctaccccgaccacatgaagcagcacgacttcttcaagtccgccatgcccgaaggctacgtccaggagcgcaccatctctttcaaggacgacggcacctacaagacccgcgccgaggtgaagttcgagggcgacaccctggtgaaccgcatcgtgctgaagggcatcgacttcaaggaggacggcaacatcctggggcacaagctggagtacaacttcaacagccacaaggtctatatcacggccgacaagcagaagaacggcatcaaggctaacttcaagacccgccacaacgttgaggacggcggcgtgcagctcgccgaccactaccagcagaacacccccatcggcgacggccccgtgctgctgcccgacaaccactacctgagccatcagtccaaactgagcaaagaccccaacgagaagcgcgatcacatggtcctgaaggagagggtgaccgccgccgggattacacatgacatggacgagctgtacaagtagacgcgtgctcgctttcttgctgtccaatttctattaaaggttcctttgttcgcgttgctggaccagaagatatggcttcggttcagcaaaatgattgcagatccactagttctaga

SEQ ID NO: 222 - DNA, 787 bp, Synthetic construct
  source 1..787: mol_type = other DNA
atggtgagcaagggcgaggagctgttcaccggggtggtgcccatcctggtcgagctggacggcgacgtaaacggccacaagttcagcgtccgcggcgagggcgagggcgatgccaccaacggcaagctgaccctgaagttcatctgcaccaccggcaagctgcccgtgccctggcccaccctcgtgaccaccttaggctacggcgtggcctgcttcgcccgctaccccgaccacatgaagcagcacgacttcttcaagtccgccatgcccgaaggctacgtccaggagcgcaccatctctttcaaggacgacggcacctacaagacccgcgccgaggtgaagttcgagggcgacaccctggtgaaccgcatcgtgctgaagggcatcgacttcaaggaggacggcaacatcctggggcacaagctggagtacaacttcaacagccacaaggtctatatcacggccgacaagcagaagaacggcatcaaggctaacttcaagacccgccacaacgttgaggacggcggcgtgcagctcgccgaccactaccagcagaacacccccatcggcgacggccccgtgctgctgcccgacaaccactacctgagccatcagtccaaactgagcaaagaccccaacgagaagcgcgatcacatggtcctgaaggagagggtgaccgccgccgggattacacatgacatggacgagctgtacaagtagacgcgttgctggaccagaagatatggcttcggttcagcaaaatgattgcagatccactagttctaga

SEQ ID NO: 223 - DNA, 1769 bp, Synthetic construct
  source 1..1769: mol_type = other DNA
atggaagatgccaagaacatcaagaagggccctgctcctagataccctctggaagatggaaccgctggcgagcagctgcacaaggccatgaagagatacgctcaggtgcccggcacaatcgccttcacagatgcccacatcgaagtgaacatcacctacgccgagtacttcgagatgagcgtgcggctggccgaagctatgaagcgatacggcctgaacaccaaccacagaatcgtcgtgtgcagcgagaacagcctccagttcttcatgcctgtgctgggcgctctgttcatcggagtggctgtggctcctgccaacgacatctacaacgagcgcgagctgctgaacagcatgaacatcagccagcctaccgtggtgttcgtgtccaagaagggactgcaaaagatcctgaacgtgcagaagaagctgcccatcatccagaaaatcatcatcatggacagcaagaccgactaccagggcttccagagcatgtataccttcgtgaccagccatctgccaccaggcttcaacgagtacgacttcaagcccgagagcttcgacagagacaagacaatcgccctgatcatgaacagcagcggctctaccggactgcctaaaggcgttgccctgcctcacagaacagcttgcgtcagattcagccacgccagagatcccatcttcggcaaccagatcaagcctgacaccgctatcctgagcgtggtgccttttcaccacggcttcggcatgttcaccacactgggctacctgatctgcggcttcagagtggtgctgatgtatcgctttgaggaagaactgttcctgcggagcctccaggactacaagatccagtctgctctgctggtgcctactctgttcagcttctttgccaagagcaccctgatcgataagtacgacctgagcaacctgcacgagatcgcctctggcggagcccctctgtctaaagaagtgggcgaagccgtcgccaagagatttcatctgcccggcatcagacaaggctacggactgaccgagacaaccagcgccatcctgatcacacctgagggcgacgataagcctggcgctgtgggaaaagtggtgccattcttcgaggctaaggtggtggacctggacaccggcaaaacactgggagtgaatcagaggggcgagctgtgtgtcagaggccctatgatcatgagcggctacgtgaacaaccccgaggccaccaacgctctgatcgacaaggatggctggctgcacagcggcgacattgcctactgggacgaagatgagcacttcttcatcgtggacagactgaagtccctgatcaagtacaagggctaccaggtggcccctgccgagctggaatctatcctgctccagcatcctaacatccgcgacgctggtgttgctggcctgcctgacgatgatgctggcgaacttcctgctgccgtggtggtgctggaacacggcaagaccatgaccgagaaagaaatcgtggactacgtggcctctcaagtgaccaccgccaagaaactgagaggcggcgtggtgtttgtggacgaggtgccaaaaggcctgaccggcaagctggacgccagaaagatcagagagatcctcatcaaggccaagaaaggcggcaagatcgctgtctagacgcgtgctcgctttcttgctgtccaatttctattaaaggttcctttgttcgcgttgctggaccagaagatatggcttcggttcagcaaaatgattgcagatccactagttctaga

SEQ ID NO: 224 - DNA, 815 bp, Synthetic construct
  source 1..815: mol_type = other DNA
atggtttctaaaggcgaggccgtgatcaaagagttcatgaggttcaaggtgcacatggaaggcagcatgaacggccacgagttcgagatcgaaggcgaaggcgagggcagaccttacgagggaactcagaccgccaagctgaaagtgaccaaaggcggccctctgcctttcagctgggacatcctgtctccacagtttatgtacggcagcagggccttcatcaagcaccccgctgacatccccgactactacaagcagtctttcccagagggcttcaagtgggagagagtgatgaacttcgaggacggcggagccgtgactgtgacacaggacacatctctggaagatgggaccctgatctacaaagtgaagctgcggggcacaaacttccctccagacggccctgtgatgcagaaaaagacaatgggctgggaagccagcaccgagagactgtaccctgaagatggcgtgctgaagggcgacatcaagatggccctgagactgaaggatggcggcagatacctggccgacttcaagaccacctacaaggccaagaaacctgtgcagatgcctggcgcctacaacgtggacagaaagctggacatcaccagccacaacgaggactacaccgtggtggaacagtacgagagaagcgaggggagacacagcacaggcggaatggacgagctgtacaagtagacgcgtgctcgctttcttgctgtccaatttctattaaaggttcctttgttcgcgttgctggaccagaagatatggcttcggttcagcaaaatgattgcagatccactagttctaga

SEQ ID NO: 225 - DNA, 1187 bp, Synthetic construct
  source 1..1187: mol_type = other DNA
atgagcaacctgctgaccgtgcaccagaacctgcctgctctgcctgtggacgccacatctgatgaagtgcggaagaacctgatggacatgttcagagacagacaggccttcagcgagcacacctggaagatgctgctgagcgtgtgtagaagctgggccgcttggtgcaagctgaacaacagaaagtggttccccgccgagcctgaggacgtgcgagattacctgctgtacctgcaagctagaggcctggccgtgaaaaccatccagcagcacctgggccagctgaacatgctgcacagaagaagcggcctgcctagacctagcgacagcaacgctgtgtccctggtcatgagaaggattcggaaagaaaacgtggacgctggcgagagagctaagcaggctctggccttcgagagaaccgacttcgatcaagtgcgcagcctgatggaaaacagcgacagatgccaggatattcggaacctggccttcctgggaatcgcctacaacaccctgctgagaatcgccgagatcgccagaatcagagtgaaggacatcagcagaaccgacggcggcagaatgctgatccacatcggcagaacaaagaccctggtgtccacagctggcgtcgagaaggctctgagtctgggcgtgacaaagctggtggaaagatggatcagcgtgtccggcgtggccgacgatcctaacaactacctgttctgtcgcgtgcgcaagaacggcgtggcagctccttctgctacaagccagctgagcacaagagccctggaaggcatcttcgaggccacacacagactgatctacggcgccaaggatgacagcggccagagataccttgcttggagcggccacagtgctagagtgggcgctgctagagacatggctagagcaggcgtgtcaatccccgagatcatgcaagctggcggctggaccaacgtgaacatcgtgatgaactacatccgcaacctggacagcgagacaggcgctatggttcgactgcttgaagatggcgacggtggatccggtcctgccgctaagagagtgaagctggactgaacgcgtgctcgctttcttgctgtccaatttctattaaaggttcctttgttcgcgttgctggaccagaagatatggcttcggttcagcaaaatgattgcagatccactagttctaga

SEQ ID NO: 226 - DNA, 560 bp, Synthetic construct
  source 1..560: mol_type = other DNA
atggctaacctcgacaagatgctgaacaccaccgtgaccgaagtgcggaagttcctccaggccgatagagtgtgcgtgttcaagttcgaggaagattacagcggcaccgtgtctcacgaggccgtggacgatagatggatcagcatcctgaaaacccaggtgcaggatcggtacttcatggaaaccagaggcgaggaatacgtgcacggcagataccaggccattgccgacatctacaccgccaacctggtcgagtgctaccgggatctgctgatcgagttccaagtgcgggccatcctggctgtgcctatcctccagggaaagaagctgtggggactgctggtggctcatcagctggctggacctagagaatggcagacctgggagatcgacttcctgaagcagcaggccgtggtcatgggaatcgccatccagcagagttgaacgcgtgctcgctttcttgctgtccaatttctattaaaggttcctttgttcgcgttgctggaccagaagatatggcttcggttcagcaaaatgattgcagatccactagttctaga

SEQ ID NO: 227 - DNA, 188 bp, Synthetic construct
  source 1..188: mol_type = other DNA
gggcgaagcaggccacgccggtttcagagccaccagaagatatggcttcggtggcaagttgaaataaggctagtccgttatcaacttgaaaaagtggcaccgagtcggtgctgtgaccaccttaggctacggcgtggcctgcttccgcggttctatctagttacgcgttaaaccaactagaatttttt

SEQ ID NO: 228 - DNA, 183 bp, Synthetic construct
  source 1..183: mol_type = other DNA
gggcgaagcaggccacgccggtttaagagctatgctggaaacagcatagcaagtttaaataaggctagtccgttatcaacttgaaaaagtggcaccgagtcggtgctgtgaccaccttaggctacggcgtggcctgcttccgcggttctatctagttacgcgttaaaccaactagaatttttt

SEQ ID NO: 229 - DNA, 118 bp, Synthetic construct
  source 1..118: mol_type = other DNA
gtcccacaacgaagactgacgtttcagagccaccagaagatatggcttcggtggcaagttgaaataaggctagtccgttatcaacttgaaaaagtggcaccgagtcggtgcttttttt

SEQ ID NO: 230 - DNA, 113 bp, Synthetic construct
  source 1..113: mol_type = other DNA
gtcccacaacgaagactgacgtttaagagctatgctggaaacagcatagcaagtttaaataaggctagtccgttatcaacttgaaaaagtggcaccgagtcggtgcttttttt

SEQ ID NO: 231 - DNA, 2378 bp, Synthetic construct
  source 1..2378: mol_type = other DNA
atgagcttcgttgctggagtcatccggagactggacgagacagtggtgaacagaattgccgccggcgaggtgatccagagacctgccaatgcaataaaggagatgatcgagaactgtctggacgccaagtccacaagcattcaggtgatcgtgaaggagggcggactgaagctgatccagatccaagacaacggcacaggcatcagaaaggaagatctggacatcgtgtgtgaacggttcaccacatctaagctgcagtcttttgaggatctggcctctatcagtacctacggcttcagaggcgaggccctggccagcatcagccacgtggcccatgtgaccatcaccaccaaaaccgccgacggcaaatgcgcttatcgcgctagctacagcgacggcaagctgaaagccccgccaaagccttgcgccggcaaccagggtacacagataacagtggaggatctgttctacaacatcgccacccggagaaaggccctgaaaaatcccagcgaggagtacggcaagatcctggaagtcgtcggcagatactccgtgcacaacgccggaatcagctttagcgtaaagaagcagggagaaaccgtggccgatgtgcgcaccctgccaaatgccagcaccgtggataacatcagaagcattttcggaaatgccgtgtccagagaactgatcgagatcggctgcgaagataagaccctggcttttaagatgaacggctacatcagcaacgccaattactctgtgaagaagtgcatctttcttctgttcatcaaccacagactggtggaaagcaccagcctgcggaaagccatcgagacagtgtacgccgcctacctgcctaagaacacccaccccttcctgtacctgagcctcgagatcagccctcagaacgtggacgtcaatgtgcatcctacaaagcacgaggtgcacttcctgcacgaggaaagcatcctggaaagagtgcagcagcacattgagagcaagctgctgggctctaacagcagcagaatgtacttcacacagaccctgctgcctggcctggccggcccctcaggcgaaatggttaagtccacaacctctctgacctcatccagcaccagcggttcttccgataaggtgtacgcccaccagatggtgcggaccgactctcgggagcagaagctggacgcctttctgcaacctctgagcaaacctctgagctctcagcctcaggccatcgtgaccgaggacaagacagatatctcctccggccgtgccagacagcaggacgaagaaatgctcgagctgccagctcctgccgaggtggccgccaagaaccagagcctggagggagataccacaaagggcaccagcgaaatgagcgagaagcggggccctacctccagcaaccccagaaaacggcaccgggaggacagcgacgtggaaatggtggaggacgacagcagaaaggaaatgacagccgcttgtacccctagaagaagaatcatcaacctgacctccgtgctgagcctgcaggaggagatcaacgagcagggccacgaggtgctgagagagatgctgcacaatcacagcttcgtgggctgcgtgaaccctcaatgggccctggctcagcatcaaacaaagctgtacctgctgaacaccaccaagctgagcgaagagctgttctaccagatcctcatctacgacttcgccaacttcggcgtgctacgcctgagcgagcccgcccctctgtttgacctggccatgctggctctggatagcccagaaagcggctggacagaagaggacggacctaaagaggggctggctgaatacatcgtggagttcctgaagaaaaaggccgagatgctggccgactacttttctctggaaatcgacgaggaaggcaacctgatcggcctgcctctgctgatcgataactacgtgcctcccctggaaggcctgcccatcttcatcctgagactggctacagaggtgaactgggacgaggaaaaggaatgcttcgagtctctgagcaaggagtgcgccatgttctatagcatcagaaaacagtacatctctgaagagagcactctgtctggccagcagagtgaagtgcccggaagcatccccaacagctggaagtggaccgtggaacacatcgtgtacaaggccctgcggagccacattctccctcctaagcacttcaccgaggacggcaacatcctgcagctggccaacctgcccgacctttataaggttttctaaacgcgtgctcgctttcttgctgtccaatttctattaaaggttcctttgttcgcgttgctggaccagaagatatggcttcggttcagcaaaatgattgcagatccactagttctaga

SEQ ID NO: 232 - DNA, 225 bp, Synthetic construct
  source 1..225: mol_type = other DNA
gggcgaagcaggccacgccggtttcagagctatgctggaaacagcatagcaagttgaaataaggctagtccgttatcaacttgaaaaagtggcaccgagtcggtgctgtgaccaccttaggctacggcgtggcctgcttccaattccgaccagaagatatggcttcggttggaattgttgacgcggttctatctagttacgcgttaaaccaactagaaatttttt

SEQ ID NO: 233 - DNA, 218 bp, Synthetic construct
  source 1..218: mol_type = other DNA
gggcgaagcaggccacgccggtttcagagccaccagaagatatggcttcggtggcaagttgaaataaggctagtccgttatcaacttgaaaaagtggcaccgagtcggtgctgtgaccaccttaggctacggcgtggcctgcttcaagttcactgccgtataggcagctaagaaacgcggttctatctagttacgcgttaaaccaactagaatttttt

SEQ ID NO: 234 - DNA, 181 bp, Synthetic construct
  source 1..181: mol_type = other DNA
gggcgaagcaggccacgccggtttcagagccaccagaagatatggcttcggtggcaagttgaaataaggctagtccgttatcaacttgaaaaagtggcaccgagtcggtgctgtgaccaccttaggctacggcgtggcctgcttcaagttcactgccgtataggcagctaagaaatttttt

SEQ ID NO: 235 - DNA, 218 bp, Synthetic construct
  source 1..218: mol_type = other DNA
gggcgaagcaggccacgccggtttcagagccaccagaagatatggcttcggtggcaagttgaaataaggctagtccgttatcaacttgaaaaagtggcaccgagtcggtgctgtgaccaccttaggctacggcgtggcctgcttccgcggttctatctagttacgcgttaaaccaactagaaaagttcactgccgtataggcagctaagaaatttttt

SEQ ID NO: 236 - DNA, 250 bp, Synthetic construct
  source 1..250: mol_type = other DNA
gggcgaagcaggccacgccggtttcagagctatgctggaaacagcatagcaagttgaaataaggctagtccgttatcaacttgaaaaagtggcaccgagtcggtgctgtgaccaccttaggctacggcgtggcctgcttccaattccgaccagaagatatggcttcggttggaattgaagttcactgccgtataggcagctaagaaacgcggttctatctagttacgcgttaaaccaactagaatttttt

SEQ ID NO: 237 - DNA, 213 bp, Synthetic construct
  source 1..213: mol_type = other DNA
gggcgaagcaggccacgccggtttcagagctatgctggaaacagcatagcaagttgaaataaggctagtccgttatcaacttgaaaaagtggcaccgagtcggtgctgtgaccaccttaggctacggcgtggcctgcttccaattccgaccagaagatatggcttcggttggaattgaagttcactgccgtataggcagctaagaaatttttt

SEQ ID NO: 238 - DNA, 254 bp, Synthetic construct
  source 1..254: mol_type = other DNA
gggcgaagcaggccacgccggtttcagagctatgctggaaacagcatagcaagttgaaataaggctagtccgttatcaacttgaaaaagtggcaccgagtcggtgctgtgaccaccttaggctacggcgtggcctgcttccaattccgaccagaagatatggcttcggttggaattgttgacgcggttctatctagttacgcgttaaaccaactagaaaagttcactgccgtataggcagctaagaaatttttt

SEQ ID NO: 239 - DNA, 213 bp, Synthetic construct
  source 1..213: mol_type = other DNA
gggcgaagcaggccacgccggtttcagagctatgctggaaacagcatagcaagttgaaataaggctagtccgttatcaacttgaaaaagtggcaccgagtcggtgctgtgaccaccttaggctacggcgtggcctgcttcaagttcactgccgtataggcagctaagaaacgcggttctatctagttacgcgttaaaccaactagaatttttt

SEQ ID NO: 240 - DNA, 176 bp, Synthetic construct
  source 1..176: mol_type = other DNA
gggcgaagcaggccacgccggtttcagagctatgctggaaacagcatagcaagttgaaataaggctagtccgttatcaacttgaaaaagtggcaccgagtcggtgctgtgaccaccttaggctacggcgtggcctgcttcaagttcactgccgtataggcagctaagaaatttttt

SEQ ID NO: 241 - DNA, 213 bp, Synthetic construct
  source 1..213: mol_type = other DNA
gggcgaagcaggccacgccggtttcagagctatgctggaaacagcatagcaagttgaaataaggctagtccgttatcaacttgaaaaagtggcaccgagtcggtgctgtgaccaccttaggctacggcgtggcctgcttccgcggttctatctagttacgcgttaaaccaactagaaaagttcactgccgtataggcagctaagaaatttttt

SEQ ID NO: 242 - DNA, 118 bp, Synthetic construct
  source 1..118: mol_type = other DNA
ggccacgccgtggcttaagggtttcagagccaccagaagatatggcttcggtggcaagttgaaataaggctagtccgttatcaacttgaaaaagtggcaccgagtcggtgcttttttt

SEQ ID NO: 243 - DNA, 5648 bp, Synthetic construct
  source 1..5648: mol_type = other DNA
ggcgcgccggattcgacattgattattgactagttattaatagtaatcaattacggggtcattagttcatagcccatatatggagttccgcgttacataacttacggtaaatggcccgcctggctgaccgcccaacgacccccgcccattgacgtcaataatgacgtatgttcccatagtaacgccaatagggactttccattgacgtcaatgggtggagtatttacggtaaactgcccacttggcagtacatcaagtgtatcatatgccaagtacgccccctattgacgtcaatgacggtaaatggcccgcctggcattatgcccagtacatgaccttatgggactttcctacttggcagtacatctacgtattagtcatcgctattaccatggtcgaggtgagccccacgttctgcttcactctccccatctcccccccctccccacccccaattttgtatttatttattttttaattattttgtgcagcgatgggggcggggggggggggggggcgcgcgccaggcggggcggggcggggcgaggggcggggcggggcgaggcggagaggtgcggcggcagccaatcagagcggcgcgctccgaaagtttccttttatggcgaggcggcggcggcggcggccctataaaaagcgaagcgcgcggcgggcgggagtcgctgcgtcgcgccttcgccccgtgccccgctccgccgccgcctcgcgccgcccgccccggctctgactgaccgcgttactcccacaggtgagcgggcgggacggcccttctcctccgggctgtaattagcgcttggtttaatgacggctcgtttcttttctgtggctgcgtgaaagccttaaagggctccgggagggccctttgtgcgggggggagcggctcggggggtgcgtgcgtgtgtgtgtgcgtggggagcgccgcgtgcggcccgcgctgcccggcggctgtgagcgctgcgggcgcggcgcggggctttgtgcgctccgcgtgtgcgcgaggggagcgcggccgggggcggtgccccgcggtgcgggggggctgcgaggggaacaaaggctgcgtgcggggtgtgtgcgtgggggggtgagcagggggtgtgggcgcggcggtcgggctgtaacccccccctgcacccccctccccgagttgctgagcacggcccggcttcgggtgcggggctccgtgcggggcgtggcgcggggctcgccgtgccgggcggggggtggcggcaggtgggggtgccgggcggggcggggccgcctcgggccggggagggctcgggggaggggcgcggcggccccggagcgccggcggctgtcgaggcgcggcgagccgcagccattgccttttatggtaatcgtgcgagagggcgcagggacttcctttgtcccaaatctggcggagccgaaatctgggaggcgccgccgcaccccctctagcgggcgcgggcgaagcggtgcggcgccggcaggaaggaaatgggcggggagggccttcgtgcgtcgccgcgccgccgtccccttctccatctccagcctcggggctgccgcagggggacggctgccttcgggggggacggggcagggcggggttcggcttctggcgtgtgaccggcggctctagagcctctgctaaccatgttcatgccttcttctttttcctacagatccttaattaataatacgactcactataggggccgccaccatggtgagcaagggcgaggagctgttcaccggggtggtgcccatcctggtcgagctggacggcgacgtaaacggccacaagttcagcgtccgcggcgagggcgagggcgatgccaccaacggcaagctgaccctgaagttcatctgcaccaccggcaagctgcccgtgccctggcccaccctcgtgaccaccttaggctacggcgtggcctgcttcgcccgctaccccgaccacatgaagcagcacgacttcttcaagtccgccatgcccgaaggctacgtccaggagcgcaccatctctttcaaggacgacggcacctacaagacccgcgccgaggtgaagttcgagggcgacaccctggtgaaccgcatcgtgctgaagggcatcgacttcaaggaggacggcaacatcctggggcacaagctggagtacaacttcaacagccacaaggtctatatcacggccgacaagcagaagaacggcatcaaggctaacttcaagacccgccacaacgttgaggacggcggcgtgcagctcgccgaccactaccagcagaacacccccatcggcgacggccccgtgctgctgcccgacaaccactacctgagccatcagtccaaactgagcaaagaccccaacgagaagcgcgatcacatggtcctgaaggagagggtgaccgccgccgggattacacatgacatggacgagctgtacaagtagacgcgtgctcgctttcttgctgtccaatttctattaaaggttcctttgttcgcgttgctggaccagaagatatggcttcggttcagcaaaatgattgcagatccactagttctagagctcgctgatcagcctcgactgtgccttctagttgccagccatctgttgtttgcccctcccccgtgccttccttgaccctggaaggtgccactcccactgtcctttcctaataaaatgaggaaattgcatcgcattgtctgagtaggtgtcattctattctggggggtggggtggggcaggacagcaagggggaggattgggaagacaatagcaggcatgctggggatgcggtgggctctatggcttctgaggcggaaagaaccagctggggctcgagatccactagttctagcctcgaggctagagcggccgccactggccgtcgttttacaacgtcgtgactgggaaaaccctggcgttacccaacttaatcgccttgcagcacatccccctttcgccagctggcgtaatagcgaagaggcccgcaccgatcgcccttcccaacagttgcgcagcctgaatggcgaatgggacgcgccctgtagcggcgcattaagcgcggcgggtgtggtggttacgcgcagcgtgaccgctacacttgccagcgccctagcgcccgctcctttcgctttcttcccttcctttctcgccacgttcgccggctttccccgtcaagctctaaatcgggggctccctttagggttccgatttagtgctttacggcacctcgaccccaaaaaacttgattagggtgatggttcacgtagtgggccatcgccctgatagacggtttttcgccctttgacgttggagtccacgttctttaatagtggactcttgttccaaactggaacaacactcaaccctatctcggtctattcttttgatttataagggattttgccgatttcggcctattggttaaaaaatgagctgatttaacaaaaatttaacgcgaattttaacaaaatattaacgcttacaatttaggtggcacttttcggggaaatgtgcgcggaacccctatttgtttatttttctaaatacattcaaatatgtatccgctcatgagacaataaccctgataaatgcttcaataatattgaaaaaggaagagtatgagtattcaacatttccgtgtcgcccttattcccttttttgcggcattttgccttcctgtttttgctcacccagaaacgctggtgaaagtaaaagatgctgaagatcagttgggtgcacgagtgggttacatcgaactggatctcaacagcggtaagatccttgagagttttcgccccgaagaacgttttccaatgatgagcacttttaaagttctgctatgtggcgcggtattatcccgtattgacgccgggcaagagcaactcggtcgccgcatacactattctcagaatgacttggttgagtactcaccagtcacagaaaagcatcttacggatggcatgacagtaagagaattatgcagtgctgccataaccatgagtgataacactgcggccaacttacttctgacaacgatcggaggaccgaaggagctaaccgcttttttgcacaacatgggggatcatgtaactcgccttgatcgttgggaaccggagctgaatgaagccataccaaacgacgagcgtgacaccacgatgcctgtagcaatggcaacaacgttgcgcaaactattaactggcgaactacttactctagcttcccggcaacaattaatagactggatggaggcggataaagttgcaggaccacttctgcgctcggcccttccggctggctggtttattgctgataaatctggagccggtgagcgtgggtctcgcggtatcattgcagcactggggccagatggtaagccctcccgtatcgtagttatctacacgacggggagtcaggcaactatggatgaacgaaatagacagatcgctgagataggtgcctcactgattaagcattggtaactgtcagaccaagtttactcatatatactttagattgatttaaaacttcatttttaatttaaaaggatctaggtgaagatcctttttgataatctcatgaccaaaatcccttaacgtgagttttcgttccactgagcgtcagaccccgtagaaaagatcaaaggatcttcttgagatcctttttttctgcgcgtaatctgctgcttgcaaacaaaaaaaccaccgctaccagcggtggtttgtttgccggatcaagagctaccaactctttttccgaaggtaactggcttcagcagagcgcagataccaaatactgtccttctagtgtagccgtagttaggccaccacttcaagaactctgtagcaccgcctacatacctcgctctgctaatcctgttaccagtggctgctgccagtggcgataagtcgtgtcttaccgggttggactcaagacgatagttaccggataaggcgcagcggtcgggctgaacggggggttcgtgcacacagcccagcttggagcgaacgacctacaccgaactgagatacctacagcgtgagctatgagaaagcgccacgcttcccgaagggagaaaggcggacaggtatccggtaagcggcagggtcggaacaggagagcgcacgagggagcttccagggggaaacgcctggtatctttatagtcctgtcgggtttcgccacctctgacttgagcgtcgatttttgtgatgctcgtcaggggggcggagcctatggaaaaacgccagcaacgcggcctttttacggttcctggccttttgctggccttttgctcacatgttctttcctgcgttatcccctgattctgtggataaccgtattaccgcctttgagtgagctgataccgctcgccgcagccgaacgaccgagcgcagcgagtcagtgagcgaggaagcggaagagcgcccaatacgcaaaccgcctctccccgcgcgttggccgattcattaatgcagctggcacgacaggtttcccgactggaaagcgggcagtgagcgcaacgcaattaatgtgagttagctcactcattaggcaccccaggctttacactttatgcttccggctcgtatgttgtgtggaattgtgagcggataacaatttcacacaggaaacagctatgaccatga

SEQ ID NO: 244 - DNA, 10644 bp, Synthetic construct
  source 1..10644: mol_type = other DNA
gcatctcaattagtcagcaaccatagtcccgcccctaactccgcccatcccgcccctaactccgcccagttccgcccattctccgccccatggctgactaattttttttatttatgcagaggccgaggccgcctcggcctctgagctattccagaagtagtgaggaggcttttttggaggcctaggcttttgcaaaaagctaacttgtttattgcagcttataatggttacaaataaagcaatagcatcacaaatttcacaaataaagcatttttttcactgcattctagttgtggtttgtccaaactcatcaatgtatcttatcatgtctggatccgctgcattaatgaatcggccaacgcgcggggagaggcggtttgcgtattgggcgctcttccgcttcctcgctcactgactcgctgcgctcggtcgttcggctgcggcgagcggtatcagctcactcaaaggcggtaatacggttatccacagaatcaggggataacgcaggaaagaacatgtgagcaaaaggccagcaaaaggccaggaaccgtaaaaaggccgcgttgctggcgtttttccataggctccgcccccctgacgagcatcacaaaaatcgacgctcaagtcagaggtggcgaaacccgacaggactataaagataccaggcgtttccccctggaagctccctcgtgcgctctcctgttccgaccctgccgcttaccggatacctgtccgcctttctcccttcgggaagcgtggcgctttctcatagctcacgctgtaggtatctcagttcggtgtaggtcgttcgctccaagctgggctgtgtgcacgaaccccccgttcagcccgaccgctgcgccttatccggtaactatcgtcttgagtccaacccggtaagacacgacttatcgccactggcagcagccactggtaacaggattagcagagcgaggtatgtaggcggtgctacagagttcttgaagtggtggcctaactacggctacactagaagaacagtatttggtatctgcgctctgctgaagccagttaccttcggaaaaagagttggtagctcttgatccggcaaacaaaccaccgctggtagcggtggtttttttgtttgcaagcagcagattacgcgcagaaaaaaaggatctcaagaagatcctttgatcttttctacggggtctgacgctcagtggaacgaaaactcacgttaagggattttggtcatgagattatcaaaaaggatcttcacctagatccttttaaattaaaaatgaagttttaaatcaatctaaagtatatatgagtaaacttggtctgacagttaccaatgcttaatcagtgaggcacctatctcagcgatctgtctatttcgttcatccatagttgcctgactccccgtcgtgtagataactacgatacgggagggcttaccatctggccccagtgctgcaatgataccgcgagacccacgctcaccggctccagatttatcagcaataaaccagccagccggaagggccgagcgcagaagtggtcctgcaactttatccgcctccatccagtctattaattgttgccgggaagctagagtaagtagttcgccagttaatagtttgcgcaacgttgttgccattgctacaggcatcgtggtgtcacgctcgtcgtttggtatggcttcattcagctccggttcccaacgatcaaggcgagttacatgatcccccatgttgtgcaaaaaagcggttagctccttcggtcctccgatcgttgtcagaagtaagttggccgcagtgttatcactcatggttatggcagcactgcataattctcttactgtcatgccatccgtaagatgcttttctgtgactggtgagtactcaaccaagtcattctgagaatagtgtatgcggcgaccgagttgctcttgcccggcgtcaatacgggataataccgcgccacatagcagaactttaaaagtgctcatcattggaaaacgttcttcggggcgaaaactctcaaggatcttaccgctgttgagatccagttcgatgtaacccactcgtgcacccaactgatcttcagcatcttttactttcaccagcgtttctgggtgagcaaaaacaggaaggcaaaatgccgcaaaaaagggaataagggcgacacggaaatgttgaatactcatactcttcctttttcaatattattgaagcatttatcagggttattgtctcatgagcggatacatatttgaatgtatttagaaaaataaacaaataggggttccgcgcacatttccccgaaaagtgccacctgggtcgacattgattattgactagttattaatagtaatcaattacggggtcattagttcatagcccatatatggagttccgcgttacataacttacggtaaatggcccgcctggctgaccgcccaacgacccccgcccattgacgtcaataatgacgtatgttcccatagtaacgccaatagggactttccattgacgtcaatgggtggagtatttacggtaaactgcccacttggcagtacatcaagtgtatcatatgccaagtacgccccctattgacgtcaatgacggtaaatggcccgcctggcattatgcccagtacatgaccttatgggactttcctacttggcagtacatctacgtattagtcatcgctattaccatggtcgaggtgagccccacgttctgcttcactctccccatctcccccccctccccacccccaattttgtatttatttattttttaattattttgtgcagggcgaggcggagaggtgcggcggcagccaatcagagcggcgcgctccgaaagtttccttttatggcgaggcggcggcggcggcggccctataaaaagcgaagcgcgcggcgggcgggagtcgctgcgcgctgccttcgccccgtgccccgctccgccgccgcctcgcgccgcccgccccggctctgactgaccgcgttactcccacaggtgagcgggcgggacggcccttctcctccgggctgtaattagcgcttggtttaatgacggcttgtttcttttctgtggctgcgtgaaagccttgaggggctccgggagggccctttgtgcggggggagcggctcggggggtgcgtgcgtgtgtgtgtgcgtggggagcgccgcgtgcggctccgcgctgcccggcggctgtgagcgctgcgggcgcggcgcggggctttgtgcgctccgcagtgtgcgcgaggggagcgcggccgggggcggtgccccgcggtgcggggggggctgcgaggggaacaaaggctgcgtgcggggtgtgtgcgtgggggggtgagcagggggtgtgggcgcgtcggtcgggctgcaaccccccctgcacccccctccccgagttgctgagcacggcccggcttcgggtgcggggctccgtacggggcgtggcgcggggctcgccgtgccgggcggggggtggcggcaggtgggggtgccgggcggggcggggccgcctcgggccggggagggctcgggggaggggcgcggcggcccccggagcgccggcggctgtcgaggcgcggcgagccgcagccattgccttttatggtaatcgtgcgagagggcgcagggacttcctttgtcccaaatctgtgcggagccgaaatctgggaggcgccgccgcaccccctctagcgggcgcggggcgaagcggtgcggcgccggcaggaaggaaatgggcggggagggccttcgtgcgtcgccgcgccgccgtccccttctccctctccagcctcggggctgtccgcggggggacggctgccttcgggggggacggggcagggcggggttcggcttctggcgtgtgaccggcggctctagagcctctgctaaccatgttcatgccttcttctttttcctacagctcctgggcaacgtgctggttattgtgctgtctcatcattttggcaaagaattcgggccgcgttgacgcgcacggcaagaggcgaggggcggcgactggtgagagatgggtgcgagagcgtcagtattaagcgggggagaattagatcgatgggaaaaaattcggttaaggccagggggaaagaaaaaatataaattaaaacatatagtatgggcaagcagggagctagaacgattcgcagttaatcctggcctgttagaaacatcagaaggctgtagacaaatactgggacagctacaaccatcccttcagacaggatcagaagaacttagatcattatataatacagtagcaaccctctattgtgtgcatcaaaggatagagataaaagacaccaaggaagctttagacaagatagaggaagagcaaaacaaaagtaagaaaaaagcacagcaagcagcagctgacacaggacacagcaatcaggtcagccaaaattaccctatagtgcagaacatccaggggcaaatggtacatcaggccatatcacctagaactttaaatgcatgggtaaaagtagtagaagagaaggctttcagcccagaagtgatacccatgttttcagcattatcagaaggagccaccccacaagatttaaacaccatgctaaacacagtggggggacatcaagcagccatgcaaatgttaaaagagaccatcaatgaggaagctgcagaatgggatagagtgcatccagtgcatgcagggcctattgcaccaggccagatgagagaaccaaggggaagtgacatagcaggaactactagtacccttcaggaacaaataggatggatgacacataatccacctatcccagtaggagaaatctataaaagatggataatcctgggattaaataaaatagtaagaatgtatagccctaccagcattctggacataagacaaggaccaaaggaaccctttagagactatgtagaccgattctataaaactctaagagccgagcaagcttcacaagaggtaaaaaattggatgacagaaaccttgttggtccaaaatgcgaacccagattgtaagactattttaaaagcattgggaccaggagcgacactagaagaaatgatgacagcatgtcagggagtggggggacccggccataaagcaagagttttggctgaagcaatgagccaagtaacaaatccagctaccataatgatacagaaaggcaattttaggaaccaaagaaagactgttaagtgtttcaattgtggcaaagaagggcacatagccaaaaattgcagggcccctaggaaaaagggctgttggaaatgtggaaaggaaggacaccaaatgaaagattgtactgagagacaggctaattttttagggaagatctggccttcccacaagggaaggccagggaattttcttcagagcagaccagagccaacagccccaccagaagagagcttcaggtttggggaagagacaacaactccctctcagaagcaggagccgatagacaaggaactgtatcctttagcttccctcagatcactctttggcagcgacccctcgtcacaataaagataggggggcaattaaaggaagctctattagatacaggagcagatgatacagtattagaagaaatgaatttgccaggaagatggaaaccaaaaatgatagggggaattggaggttttatcaaagtaagacagtatgatcagatactcatagaaatctgcggacataaagctataggtacagtattagtaggacctacacctgtcaacataattggaagaaatctgttgactcagattggctgcactttaaattttcccattagtcctattgagactgtaccagtaaaattaaagccaggaatggatggcccaaaagttaaacaatggccattgacagaagaaaaaataaaagcattagtagaaatttgtacagaaatggaaaaggaaggaaaaatttcaaaaattgggcctgaaaatccatacaatactccagtatttgccataaagaaaaaagacagtactaaatggagaaaattagtagatttcagagaacttaataagagaactcaagatttctgggaagttcaattaggaataccacatcctgcagggttaaaacagaaaaaatcagtaacagtactggatgtgggcgatgcatatttttcagttcccttagataaagacttcaggaagtatactgcatttaccatacctagtataaacaatgagacaccagggattagatatcagtacaatgtgcttccacagggatggaaaggatcaccagcaatattccagtgtagcatgacaaaaatcttagagccttttagaaaacaaaatccagacatagtcatctatcaatacatggatgatttgtatgtaggatctgacttagaaatagggcagcatagaacaaaaatagaggaactgagacaacatctgttgaggtggggatttaccacaccagacaaaaaacatcagaaagaacctccattcctttggatgggttatgaactccatcctgataaatggacagtacagcctatagtgctgccagaaaaggacagctggactgtcaatgacatacagaaattagtgggaaaattgaattgggcaagtcagatttatgcagggattaaagtaaggcaattatgtaaacttcttaggggaaccaaagcactaacagaagtagtaccactaacagaagaagcagagctagaactggcagaaaacagggagattctaaaagaaccggtacatggagtgtattatgacccatcaaaagacttaatagcagaaatacagaagcaggggcaaggccaatggacatatcaaatttatcaagagccatttaaaaatctgaaaacaggaaagtatgcaagaatgaagggtgcccacactaatgatgtgaaacaattaacagaggcagtacaaaaaatagccacagaaagcatagtaatatggggaaagactcctaaatttaaattacccatacaaaaggaaacatgggaagcatggtggacagagtattggcaagccacctggattcctgagtgggagtttgtcaatacccctcccttagtgaagttatggtaccagttagagaaagaacccataataggagcagaaactttctatgtagatggggcagccaatagggaaactaaattaggaaaagcaggatatgtaactgacagaggaagacaaaaagttgtccccctaacggacacaacaaatcagaagactgagttacaagcaattcatctagctttgcaggattcgggattagaagtaaacatagtgacagactcacaatatgcattgggaatcattcaagcacaaccagataagagtgaatcagagttagtcagtcaaataatagagcagttaataaaaaaggaaaaagtctacctggcatgggtaccagcacacaaaggaattggaggaaatgaacaagtagataaattggtcagtgctggaatcaggaaagtactatttttagatggaatagataaggcccaagaagaacatgagaaatatcacagtaattggagagcaatggctagtgattttaacctaccacctgtagtagcaaaagaaatagtagccagctgtgataaatgtcagctaaaaggggaagccatgcatggacaagtagactgtagcccaggaatatggcagctagtttgtacacatttagaaggaaaagttatcttggtagcagttcatgtagccagtggatatatagaagcagaagtaattccagcagagacagggcaagaaacagcatacttcctcttaaaattagcaggaagatggccagtaaaaacagtacatacagacaatggcagcaatttcaccagtactacagttaaggccgcctgttggtgggcggggatcaagcaggaatttggcattccctacaatccccaaagtcaaggagtaatagaatctatgaataaagaattaaagaaaattataggacaggtaagagatcaggctgaacatcttaagacagcagtacaaatggcagtattcatccacaattttaaaagaaaaggggggattggggggtacagtgcaggggaaagaatagtagacataatagcaacagacatacaaactaaagaattacaaaaacaaattacaaaaattcaaaattttcgggtttattacagggacagcagagatccagtttggaaaggaccagcaaagctcctctggaaaggtgaaggggcagtagtaatacaagataatagtgacataaaagtagtgccaagaagaaaagcaaagatcatcagggattatggaaaacagatggcaggtgatgattgtgtggcaagtagacaggatgaggattaacacatggaattctgcaacaactgctgtttatccatttcagaattgggtgtcgacatagcagaataggcgttactcgacagaggagagcaagaaatggagccagtagatcctagactagagccctggaagcatccaggaagtcagcctaaaactgcttgtaccaattgctattgtaaaaagtgttgctttcattgccaagtttgtttcatgacaaaagccttaggcatctcctatggcaggaagaagcggagacagcgacgaagagctcatcagaacagtcagactcatcaagcttctctatcaaagcagtaagtagtacatgtaatgcaacctataatagtagcaatagtagcattagtagtagcaataataatagcaatagttgtgtggtccatagtaatcatagaatataggaaaatggccgctgatcttcagacctggaggaggagatatgagggacaattggagaagtgaattatataaatataaagtagtaaaaattgaaccattaggagtagcacccaccaaggcaaagagaagagtggtgcagagagaaaaaagagcagtgggaataggagctttgttccttgggttcttgggagcagcaggaagcactatgggcgcagcgtcaatgacgctgacggtacaggccagacaattattgtctggtatagtgcagcagcagaacaatttgctgagggctattgaggcgcaacagcatctgttgcaactcacagtctggggcatcaagcagctccaggcaagaatcctggctgtggaaagatacctaaaggatcaacagctcctggggatttggggttgctctggaaaactcatttgcaccactgctgtgccttggaatgctagttggagtaataaatctctggaacagatttggaatcacacgacctggatggagtgggacagagaaattaacaattacacaagcttaatacactccttaattgaagaatcgcaaaaccagcaagaaaagaatgaacaagaattattggaattagataaatgggcaagtttgtggaattggtttaacataacaaattggctgtggtatataaaattattcataatgatagtaggaggcttggtaggtttaagaatagtttttgctgtactttctatagtgaatagagttaggcagggatattcaccattatcgtttcagacccacctcccaaccccgaggggacccgacaggcccgaaggaatagaagaagaaggtggagagagagacagagacagatccattcgattagtgaacggatccttggcacttatctgggacgatctgcggagcctgtgcctcttcagctaccaccgcttgagagacttactcttgattgtaacgaggattgtggaacttctgggacgcagggggtgggaagccctcaaatattggtggaatctcctacaatattggagtcaggagctaaagaatagtgctgttagcttgctcaatgccacagccatagcagtagctgaggggacagatagggttatagaagtagtacaaggagcttgtagagctattcgccacatacctagaagaataagacagggcttggaaaggattttgctataagctcgaaacaaccggtacctctagaactatagctagcagatctttttccctctgccaaaaattatggggacatcatgaagccccttgagcatctgacttctggctaataaaggaaatttattttcattgcaatagtgtgttggaattttttgtgtctctcactcggaaggacatatgggagggcaaatcatttaaaacatcagaatgagtatttggtttagagtttggcaacatatgcccatatgctggctgccatgaacaaaggttggctataaagaggtcatcagtatatgaaacagccccctgctgtccattccttattccatagaaaagccttgacttgaggttagattttttttatattttgttttgtgttatttttttctttaacatccctaaaattttccttacatgttttactagccagatttttcctcctctcctgactactcccagtcatagctgtccctcttctcttatggagatccctcgacctgcagcccaagcttggcgtaatcatggtcatagctgtttcctgtgtgaaattgttatccgctcacaattccacacaacatacgagccggaagcataaagtgtaaagcctggggtgcctaatgagtgagctaactcacattaattgcgttgcgctcactgcccgctttccagtcgggaaacctgtcgtgccagcggatcc

SEQ ID NO: 245 - DNA, 5822 bp, Synthetic construct
  source 1..5822: mol_type = other DNA
ggatcccctgagggggcccccatgggctagaggatccggcctcggcctctgcataaataaaaaaaattagtcagccatgagcttggcccattgcatacgttgtatccatatcataatatgtacatttatattggctcatgtccaacattaccgccatgttgacattgattattgactagttattaatagtaatcaattacggggtcattagttcatagcccatatatggagttccgcgttacataacttacggtaaatggcccgcctggctgaccgcccaacgacccccgcccattgacgtcaataatgacgtatgttcccatagtaacgccaatagggactttccattgacgtcaatgggtggagtatttacggtaaactgcccacttggcagtacatcaagtgtatcatatgccaagtacgccccctattgacgtcaatgacggtaaatggcccgcctggcattatgcccagtacatgaccttatgggactttcctacttggcagtacatctacgtattagtcatcgctattaccatggtgatgcggttttggcagtacatcaatgggcgtggatagcggtttgactcacggggatttccaagtctccaccccattgacgtcaatgggagtttgttttggcaccaaaatcaacgggactttccaaaatgtcgtaacaactccgccccattgacgcaaatgggcggtaggcgtgtacggtgggaggtctatataagcagagctcgtttagtgaaccgtcagatcgcctggagacgccatccacgctgttttgacctccatagaagacaccgggaccgatccagcctcccctcgaagcttacatgtggtaccgagctcggatcctgagaacttcagggtgagtctatgggacccttgatgttttctttccccttcttttctatggttaagttcatgtcataggaaggggagaagtaacagggtacacatattgaccaaatcagggtaattttgcatttgtaattttaaaaaatgctttcttcttttaatatacttttttgtttatcttatttctaatactttccctaatctctttctttcagggcaataatgatacaatgtatcatgcctctttgcaccattctaaagaataacagtgataatttctgggttaaggcaatagcaatatttctgcatataaatatttctgcatataaattgtaactgatgtaagaggtttcatattgctaatagcagctacaatccagctaccattctgcttttattttatggttgggataaggctggattattctgagtccaagctaggcccttttgctaatcatgttcatacctcttatcttcctcccacagctcctgggcaacgtgctggtctgtgtgctggcccatcactttggcaaagcacgtgagatctgaattctgacactatgaagtgccttttgtacttagcctttttattcattggggtgaattgcaagttcaccatagtttttccacacaaccaaaaaggaaactggaaaaatgttccttctaattaccattattgcccgtcaagctcagatttaaattggcataatgacttaataggcacagccttacaagtcaaaatgcccaagagtcacaaggctattcaagcagacggttggatgtgtcatgcttccaaatgggtcactacttgtgatttccgctggtatggaccgaagtatataacacattccatccgatccttcactccatctgtagaacaatgcaaggaaagcattgaacaaacgaaacaaggaacttggctgaatccaggcttccctcctcaaagttgtggatatgcaactgtgacggatgccgaagcagtgattgtccaggtgactcctcaccatgtgctggttgatgaatacacaggagaatgggttgattcacagttcatcaacggaaaatgcagcaattacatatgccccactgtccataactctacaacctggcattctgactataaggtcaaagggctatgtgattctaacctcatttccatggacatcaccttcttctcagaggacggagagctatcatccctgggaaaggagggcacagggttcagaagtaactactttgcttatgaaactggaggcaaggcctgcaaaatgcaatactgcaagcattggggagtcagactcccatcaggtgtctggttcgagatggctgataaggatctctttgctgcagccagattccctgaatgcccagaagggtcaagtatctctgctccatctcagacctcagtggatgtaagtctaattcaggacgttgagaggatcttggattattccctctgccaagaaacctggagcaaaatcagagcgggtcttccaatctctccagtggatctcagctatcttgctcctaaaaacccaggaaccggtcctgctttcaccataatcaatggtaccctaaaatactttgagaccagatacatcagagtcgatattgctgctccaatcctctcaagaatggtcggaatgatcagtggaactaccacagaaagggaactgtgggatgactgggcaccatatgaagacgtggaaattggacccaatggagttctgaggaccagttcaggatataagtttcctttatacatgattggacatggtatgttggactccgatcttcatcttagctcaaaggctcaggtgttcgaacatcctcacattcaagacgctgcttcgcaacttcctgatgatgagagtttattttttggtgatactgggctatccaaaaatccaatcgagcttgtagaaggttggttcagtagttggaaaagctctattgcctcttttttctttatcatagggttaatcattggactattcttggttctccgagttggtatccatctttgcattaaattaaagcacaccaagaaaagacagatttatacagacatagagatgaaccgacttggaaagtaactcaaatcctgcacaacagattcttcatgtttggaccaaatcaacttgtgataccatgctcaaagaggcctcaattatatttgagtttttaatttttatgaaaaaaaaaaaaaaaaacggaattcaccccaccagtgcaggctgcctatcagaaagtggtggctggtgtggctaatgccctggcccacaagtatcactaagctcgctttcttgctgtccaatttctattaaaggttcctttgttccctaagtccaactactaaactgggggatattatgaagggccttgagcatctggattctgcctaataaaaaacatttattttcattgcaatgatgtatttaaattatttctgaatattttactaaaaagggaatgtgggaggtcagtgcatttaaaacataaagaaatgaagagctagttcaaaccttgggaaaatacactatatcttaaactccatgaaagaaggtgaggctgcaaacagctaatgcacattggcaacagcccctgatgcctatgccttattcatccctcagaaaaggattcaagtagaggcttgatttggaggttaaagttttgctatgctgtattttacattacttattgttttagctgtcctcatgaatgtcttttcactacccatttgcttatcctgcatctctcagccttgactccactcagttctcttgcttagagataccacctttcccctgaagtgttccttccatgttttacggcgagatggtttctcctcgcctggccactcagccttagttgtctctgttgtcttatagaggtctacttgaagaaggaaaaacagggggcatggtttgactgtcctgtgagcccttcttccctgcctcccccactcacagtgacccggaatccctcgacatggcagtctagcactagtgcggccgcagatctgcttcctcgctcactgactcgctgcgctcggtcgttcggctgcggcgagcggtatcagctcactcaaaggcggtaatacggttatccacagaatcaggggataacgcaggaaagaacatgtgagcaaaaggccagcaaaaggccaggaaccgtaaaaaggccgcgttgctggcgtttttccataggctccgcccccctgacgagcatcacaaaaatcgacgctcaagtcagaggtggcgaaacccgacaggactataaagataccaggcgtttccccctggaagctccctcgtgcgctctcctgttccgaccctgccgcttaccggatacctgtccgcctttctcccttcgggaagcgtggcgctttctcatagctcacgctgtaggtatctcagttcggtgtaggtcgttcgctccaagctgggctgtgtgcacgaaccccccgttcagcccgaccgctgcgccttatccggtaactatcgtcttgagtccaacccggtaagacacgacttatcgccactggcagcagccactggtaacaggattagcagagcgaggtatgtaggcggtgctacagagttcttgaagtggtggcctaactacggctacactagaagaacagtatttggtatctgcgctctgctgaagccagttaccttcggaaaaagagttggtagctcttgatccggcaaacaaaccaccgctggtagcggtggtttttttgtttgcaagcagcagattacgcgcagaaaaaaaggatctcaagaagatcctttgatcttttctacggggtctgacgctcagtggaacgaaaactcacgttaagggattttggtcatgagattatcaaaaaggatcttcacctagatccttttaaattaaaaatgaagttttaaatcaatctaaagtatatatgagtaaacttggtctgacagttaccaatgcttaatcagtgaggcacctatctcagcgatctgtctatttcgttcatccatagttgcctgactccccgtcgtgtagataactacgatacgggagggcttaccatctggccccagtgctgcaatgataccgcgagacccacgctcaccggctccagatttatcagcaataaaccagccagccggaagggccgagcgcagaagtggtcctgcaactttatccgcctccatccagtctattaattgttgccgggaagctagagtaagtagttcgccagttaatagtttgcgcaacgttgttgccattgctacaggcatcgtggtgtcacgctcgtcgtttggtatggcttcattcagctccggttcccaacgatcaaggcgagttacatgatcccccatgttgtgcaaaaaagcggttagctccttcggtcctccgatcgttgtcagaagtaagttggccgcagtgttatcactcatggttatggcagcactgcataattctcttactgtcatgccatccgtaagatgcttttctgtgactggtgagtactcaaccaagtcattctgagaatagtgtatgcggcgaccgagttgctcttgcccggcgtcaatacgggataataccgcgccacatagcagaactttaaaagtgctcatcattggaaaacgttcttcggggcgaaaactctcaaggatcttaccgctgttgagatccagttcgatgtaacccactcgtgcacccaactgatcttcagcatcttttactttcaccagcgtttctgggtgagcaaaaacaggaaggcaaaatgccgcaaaaaagggaataagggcgacacggaaatgttgaatactcatactcttcctttttcaatattattgaagcatttatcagggttattgtctcatgagcggatacatatttgaatgtatttagaaaaataaacaaataggggttccgcgcacatttccccgaaaagtgccacctgacgt

SEQ ID NO: 246 - DNA, 6742 bp, Synthetic construct
  source 1..6742: mol_type = other DNA
ggcgcgccggattcgacattgattattgactagttattaatagtaatcaattacggggtcattagttcatagcccatatatggagttccgcgttacataacttacggtaaatggcccgcctggctgaccgcccaacgacccccgcccattgacgtcaataatgacgtatgttcccatagtaacgccaatagggactttccattgacgtcaatgggtggagtatttacggtaaactgcccacttggcagtacatcaagtgtatcatatgccaagtacgccccctattgacgtcaatgacggtaaatggcccgcctggcattatgcccagtacatgaccttatgggactttcctacttggcagtacatctacgtattagtcatcgctattaccatggtcgaggtgagccccacgttctgcttcactctccccatctcccccccctccccacccccaattttgtatttatttattttttaattattttgtgcagcgatgggggcggggggggggggggggcgcgcgccaggcggggcggggcggggcgaggggcggggcggggcgaggcggagaggtgcggcggcagccaatcagagcggcgcgctccgaaagtttccttttatggcgaggcggcggcggcggcggccctataaaaagcgaagcgcgcggcgggcgggagtcgctgcgtcgcgccttcgccccgtgccccgctccgccgccgcctcgcgccgcccgccccggctctgactgaccgcgttactcccacaggtgagcgggcgggacggcccttctcctccgggctgtaattagcgcttggtttaatgacggctcgtttcttttctgtggctgcgtgaaagccttaaagggctccgggagggccctttgtgcgggggggagcggctcggggggtgcgtgcgtgtgtgtgtgcgtggggagcgccgcgtgcggcccgcgctgcccggcggctgtgagcgctgcgggcgcggcgcggggctttgtgcgctccgcgtgtgcgcgaggggagcgcggccgggggcggtgccccgcggtgcgggggggctgcgaggggaacaaaggctgcgtgcggggtgtgtgcgtgggggggtgagcagggggtgtgggcgcggcggtcgggctgtaacccccccctgcacccccctccccgagttgctgagcacggcccggcttcgggtgcggggctccgtgcggggcgtggcgcggggctcgccgtgccgggcggggggtggcggcaggtgggggtgccgggcggggcggggccgcctcgggccggggagggctcgggggaggggcgcggcggccccggagcgccggcggctgtcgaggcgcggcgagccgcagccattgccttttatggtaatcgtgcgagagggcgcagggacttcctttgtcccaaatctggcggagccgaaatctgggaggcgccgccgcaccccctctagcgggcgcgggcgaagcggtgcggcgccggcaggaaggaaatgggcggggagggccttcgtgcgtcgccgcgccgccgtccccttctccatctccagcctcggggctgccgcagggggacggctgccttcgggggggacggggcagggcggggttcggcttctggcgtgtgaccggcggctctagagcctctgctaaccatgttcatgccttcttctttttcctacagatccttaattaataatacgactcactataggggccgccaccatgggcgctagagcctctgttctgtctggcggcgaactggacagatgggagaagatcagaagcagacctggcggcaagaagaagtacaagctgaagcacatcgtgtgggccagcagagagctggaaagattcgctgtgaaccccggcctgctggaaacaagcgagggctgtagacagatcctgggccagctccagccatctctccagacaggatctgaggaactgagaagcctgtacaacaccgtggccacactgtactgcgtgcaccagagaatcgagatcaaggacaccaaagaggccctggacaagatcgaggaagaacagaacaagtctaagaagaaggcccagcaggctgccgccgatacaggccactctaatcaggtgtcccagaactaccccatcgtgcagaacatccagggccagatggtgcatcaggctatcagccccagaacactgaacgcctgggtcaaagtggtggaagagaaggctttcagccctgaagtgatccccatgttcagcgccctgtctgagggtgccacacctcaggacctgaacaccatgctgaacacagtcggcggacaccaggccgctatgcagatgctgaaagagacaatcaacgaagaggccgccgagtgggacagagtgcatcctgttcatgctggccctatcgctcccggccagatgagagaacctagaggctctgacattgccggcaccaccagcacactgcaagagcagatcggctggatgacaaacaaccctcctattcctgtgggcgagatctacaagagatggatcatcctgggactgaacaagatcgtgcggatgtacagccccaccagcatcctggacattagacagggccccaaagagcccttcagagactacgtggacagattctacaagaccctgagagccgagcaggccagccaagaagtgaagaactggatgaccgagacactgctggtgcagaacgctaaccccgactgcaagaccatcctgaaggctctgggacctgccgccacactggaagagatgatgacagcctgtcaaggcgtcggaggacctggccataaggctagagttctggccgaggccatgagccaagtgaccaacagcgccacaatcatgatgcagagaggcaacttcagaaaccagcggaagatcgtgaagtccttcaactccggcaaagagggccacaccgcccgcaattctagagcccctagaaagaaaggtggatccggcggcgtttctggatggcggctgttcaagaagatcagcggcggagctagctctaagacaatcgtgctgtctgtgggcgaagccaccagaacactgaccgagatccagagcacagccgacagacagatcttcgaggaaaaagtgggccctctcgtgggcagactgagactgacagcttccctgagacagaacggcgccaagaccgcctacagagtgaacctgaagctggaccaggccgacgtggtggattctggccttcctaaagtgcggtacacccaagtgtggtcccacgacgtgaccatcgtggccaattctaccgaggccagcagaaagagcctgtacgacctgaccaagagcctggtggccacaagccaggtggaagatctggtcgtgaacctggtgcctctcggacgtggcggatccggtggaaccgagagacaggccaacttcctgggcaagatctggcctagctacaagggcagacccggcaacttcctccagagcagaccagagcctaccgctcctcctgaggaatccttcagatccggcgtggaaaccaccacacctccacagaagcaagagcccatcgacaaagagctgtaccctctgaccagcctgagatccctgttcggcaacgaccctagctctcaatgaacgcgtaaatgattgcagatccactagttctagagctcgctgatcagcctcgactgtgccttctagttgccagccatctgttgtttgcccctcccccgtgccttccttgaccctggaaggtgccactcccactgtcctttcctaataaaatgaggaaattgcatcgcattgtctgagtaggtgtcattctattctggggggtggggtggggcaggacagcaagggggaggattgggaagacaatagcaggcatgctggggatgcggtgggctctatggcttctgaggcggaaagaaccagctggggctcgagatccactagttctagcctcgaggctagagcggccgccactggccgtcgttttacaacgtcgtgactgggaaaaccctggcgttacccaacttaatcgccttgcagcacatccccctttcgccagctggcgtaatagcgaagaggcccgcaccgatcgcccttcccaacagttgcgcagcctgaatggcgaatgggacgcgccctgtagcggcgcattaagcgcggcgggtgtggtggttacgcgcagcgtgaccgctacacttgccagcgccctagcgcccgctcctttcgctttcttcccttcctttctcgccacgttcgccggctttccccgtcaagctctaaatcgggggctccctttagggttccgatttagtgctttacggcacctcgaccccaaaaaacttgattagggtgatggttcacgtagtgggccatcgccctgatagacggtttttcgccctttgacgttggagtccacgttctttaatagtggactcttgttccaaactggaacaacactcaaccctatctcggtctattcttttgatttataagggattttgccgatttcggcctattggttaaaaaatgagctgatttaacaaaaatttaacgcgaattttaacaaaatattaacgcttacaatttaggtggcacttttcggggaaatgtgcgcggaacccctatttgtttatttttctaaatacattcaaatatgtatccgctcatgagacaataaccctgataaatgcttcaataatattgaaaaaggaagagtatgagtattcaacatttccgtgtcgcccttattcccttttttgcggcattttgccttcctgtttttgctcacccagaaacgctggtgaaagtaaaagatgctgaagatcagttgggtgcacgagtgggttacatcgaactggatctcaacagcggtaagatccttgagagttttcgccccgaagaacgttttccaatgatgagcacttttaaagttctgctatgtggcgcggtattatcccgtattgacgccgggcaagagcaactcggtcgccgcatacactattctcagaatgacttggttgagtactcaccagtcacagaaaagcatcttacggatggcatgacagtaagagaattatgcagtgctgccataaccatgagtgataacactgcggccaacttacttctgacaacgatcggaggaccgaaggagctaaccgcttttttgcacaacatgggggatcatgtaactcgccttgatcgttgggaaccggagctgaatgaagccataccaaacgacgagcgtgacaccacgatgcctgtagcaatggcaacaacgttgcgcaaactattaactggcgaactacttactctagcttcccggcaacaattaatagactggatggaggcggataaagttgcaggaccacttctgcgctcggcccttccggctggctggtttattgctgataaatctggagccggtgagcgtgggtctcgcggtatcattgcagcactggggccagatggtaagccctcccgtatcgtagttatctacacgacggggagtcaggcaactatggatgaacgaaatagacagatcgctgagataggtgcctcactgattaagcattggtaactgtcagaccaagtttactcatatatactttagattgatttaaaacttcatttttaatttaaaaggatctaggtgaagatcctttttgataatctcatgaccaaaatcccttaacgtgagttttcgttccactgagcgtcagaccccgtagaaaagatcaaaggatcttcttgagatcctttttttctgcgcgtaatctgctgcttgcaaacaaaaaaaccaccgctaccagcggtggtttgtttgccggatcaagagctaccaactctttttccgaaggtaactggcttcagcagagcgcagataccaaatactgtccttctagtgtagccgtagttaggccaccacttcaagaactctgtagcaccgcctacatacctcgctctgctaatcctgttaccagtggctgctgccagtggcgataagtcgtgtcttaccgggttggactcaagacgatagttaccggataaggcgcagcggtcgggctgaacggggggttcgtgcacacagcccagcttggagcgaacgacctacaccgaactgagatacctacagcgtgagctatgagaaagcgccacgcttcccgaagggagaaaggcggacaggtatccggtaagcggcagggtcggaacaggagagcgcacgagggagcttccagggggaaacgcctggtatctttatagtcctgtcgggtttcgccacctctgacttgagcgtcgatttttgtgatgctcgtcaggggggcggagcctatggaaaaacgccagcaacgcggcctttttacggttcctggccttttgctggccttttgctcacatgttctttcctgcgttatcccctgattctgtggataaccgtattaccgcctttgagtgagctgataccgctcgccgcagccgaacgaccgagcgcagcgagtcagtgagcgaggaagcggaagagcgcccaatacgcaaaccgcctctccccgcgcgttggccgattcattaatgcagctggcacgacaggtttcccgactggaaagcgggcagtgagcgcaacgcaattaatgtgagttagctcactcattaggcaccccaggctttacactttatgcttccggctcgtatgttgtgtggaattgtgagcggataacaatttcacacaggaaacagctatgaccatga

SEQ ID NO: 247 - DNA, 6742 bp, Synthetic construct
  source 1..6742: mol_type = other DNA
ggcgcgccggattcgacattgattattgactagttattaatagtaatcaattacggggtcattagttcatagcccatatatggagttccgcgttacataacttacggtaaatggcccgcctggctgaccgcccaacgacccccgcccattgacgtcaataatgacgtatgttcccatagtaacgccaatagggactttccattgacgtcaatgggtggagtatttacggtaaactgcccacttggcagtacatcaagtgtatcatatgccaagtacgccccctattgacgtcaatgacggtaaatggcccgcctggcattatgcccagtacatgaccttatgggactttcctacttggcagtacatctacgtattagtcatcgctattaccatggtcgaggtgagccccacgttctgcttcactctccccatctcccccccctccccacccccaattttgtatttatttattttttaattattttgtgcagcgatgggggcggggggggggggggggcgcgcgccaggcggggcggggcggggcgaggggcggggcggggcgaggcggagaggtgcggcggcagccaatcagagcggcgcgctccgaaagtttccttttatggcgaggcggcggcggcggcggccctataaaaagcgaagcgcgcggcgggcgggagtcgctgcgtcgcgccttcgccccgtgccccgctccgccgccgcctcgcgccgcccgccccggctctgactgaccgcgttactcccacaggtgagcgggcgggacggcccttctcctccgggctgtaattagcgcttggtttaatgacggctcgtttcttttctgtggctgcgtgaaagccttaaagggctccgggagggccctttgtgcgggggggagcggctcggggggtgcgtgcgtgtgtgtgtgcgtggggagcgccgcgtgcggcccgcgctgcccggcggctgtgagcgctgcgggcgcggcgcggggctttgtgcgctccgcgtgtgcgcgaggggagcgcggccgggggcggtgccccgcggtgcgggggggctgcgaggggaacaaaggctgcgtgcggggtgtgtgcgtgggggggtgagcagggggtgtgggcgcggcggtcgggctgtaacccccccctgcacccccctccccgagttgctgagcacggcccggcttcgggtgcggggctccgtgcggggcgtggcgcggggctcgccgtgccgggcggggggtggcggcaggtgggggtgccgggcggggcggggccgcctcgggccggggagggctcgggggaggggcgcggcggccccggagcgccggcggctgtcgaggcgcggcgagccgcagccattgccttttatggtaatcgtgcgagagggcgcagggacttcctttgtcccaaatctggcggagccgaaatctgggaggcgccgccgcaccccctctagcgggcgcgggcgaagcggtgcggcgccggcaggaaggaaatgggcggggagggccttcgtgcgtcgccgcgccgccgtccccttctccatctccagcctcggggctgccgcagggggacggctgccttcgggggggacggggcagggcggggttcggcttctggcgtgtgaccggcggctctagagcctctgctaaccatgttcatgccttcttctttttcctacagatccttaattaataatacgactcactataggggccgccaccatgggcgctagagcctctgttctgtctggcggcgaactggacagatgggagaagatcagactgagacctggcggcaagaagaagtacaagctgaagcacatcgtgtgggccagcagagagctggaaagattcgctgtgaaccccggcctgctggaaacaagcgagggctgtagacagatcctgggccagctccagccatctctccagacaggatctgaggaactgagaagcctgtacaacaccgtggccacactgtactgcgtgcaccagagaatcgagatcaaggacaccaaagaggccctggacaagatcgaggaagaacagaacaagtctaagaagaaggcccagcaggctgccgccgatacaggccactctaatcaggtgtcccagaactaccccatcgtgcagaacatccagggccagatggtgcatcaggctatcagccccagaacactgaacgcctgggtcaaagtggtggaagagaaggctttcagccctgaagtgatccccatgttcagcgccctgtctgagggtgccacacctcaggacctgaacaccatgctgaacacagtcggcggacaccaggccgctatgcagatgctgaaagagacaatcaacgaagaggccgccgagtgggacagagtgcatcctgttcatgctggccctatcgctcccggccagatgagagaacctagaggctctgacattgccggcaccaccagcacactgcaagagcagatcggctggatgacaaacaaccctcctattcctgtgggcgagatctacaagagatggatcatcctgggactgaacaagatcgtgcggatgtacagccccaccagcatcctggacattagacagggccccaaagagcccttcagagactacgtggacagattctacaagaccctgagagccgagcaggccagccaagaagtgaagaactggatgaccgagacactgctggtgcagaacgctaaccccgactgcaagaccatcctgaaggctctgggacctgccgccacactggaagagatgatgacagcctgtcaaggcgtcggaggacctggccataaggctagagttctggccgaggccatgagccaagtgaccaacagcgccacaatcatgatgcagagaggcaacttcagaaaccagcggaagatcgtgaagtccttcaactccggcaaagagggccacaccgcccgcaattctagagcccctagaaagaaaggtggatccggcggcgtttctggatggcggctgttcaagaagatcagcggcggagctagctctaagacaatcgtgctgtctgtgggcgaagccaccagaacactgaccgagatccagagcacagccgacagacagatcttcgaggaaaaagtgggccctctcgtgggcagactgagactgacagcttccctgagacagaacggcgccaagaccgcctacagagtgaacctgaagctggaccaggccgacgtggtggattctggccttcctaaagtgcggtacacccaagtgtggtcccacgacgtgaccatcgtggccaattctaccgaggccagcagaaagagcctgtacgacctgaccaagagcctggtggccacaagccaggtggaagatctggtcgtgaacctggtgcctctcggacgtggcggatccggtggaaccgagagacaggccaacttcctgggcaagatctggcctagctacaagggcagacccggcaacttcctccagagcagaccagagcctaccgctcctcctgaggaatccttcagatccggcgtggaaaccaccacacctccacagaagcaagagcccatcgacaaagagctgtaccctctgaccagcctgagatccctgttcggcaacgaccctagctctcaatgaacgcgtaaatgattgcagatccactagttctagagctcgctgatcagcctcgactgtgccttctagttgccagccatctgttgtttgcccctcccccgtgccttccttgaccctggaaggtgccactcccactgtcctttcctaataaaatgaggaaattgcatcgcattgtctgagtaggtgtcattctattctggggggtggggtggggcaggacagcaagggggaggattgggaagacaatagcaggcatgctggggatgcggtgggctctatggcttctgaggcggaaagaaccagctggggctcgagatccactagttctagcctcgaggctagagcggccgccactggccgtcgttttacaacgtcgtgactgggaaaaccctggcgttacccaacttaatcgccttgcagcacatccccctttcgccagctggcgtaatagcgaagaggcccgcaccgatcgcccttcccaacagttgcgcagcctgaatggcgaatgggacgcgccctgtagcggcgcattaagcgcggcgggtgtggtggttacgcgcagcgtgaccgctacacttgccagcgccctagcgcccgctcctttcgctttcttcccttcctttctcgccacgttcgccggctttccccgtcaagctctaaatcgggggctccctttagggttccgatttagtgctttacggcacctcgaccccaaaaaacttgattagggtgatggttcacgtagtgggccatcgccctgatagacggtttttcgccctttgacgttggagtccacgttctttaatagtggactcttgttccaaactggaacaacactcaaccctatctcggtctattcttttgatttataagggattttgccgatttcggcctattggttaaaaaatgagctgatttaacaaaaatttaacgcgaattttaacaaaatattaacgcttacaatttaggtggcacttttcggggaaatgtgcgcggaacccctatttgtttatttttctaaatacattcaaatatgtatccgctcatgagacaataaccctgataaatgcttcaataatattgaaaaaggaagagtatgagtattcaacatttccgtgtcgcccttattcccttttttgcggcattttgccttcctgtttttgctcacccagaaacgctggtgaaagtaaaagatgctgaagatcagttgggtgcacgagtgggttacatcgaactggatctcaacagcggtaagatccttgagagttttcgccccgaagaacgttttccaatgatgagcacttttaaagttctgctatgtggcgcggtattatcccgtattgacgccgggcaagagcaactcggtcgccgcatacactattctcagaatgacttggttgagtactcaccagtcacagaaaagcatcttacggatggcatgacagtaagagaattatgcagtgctgccataaccatgagtgataacactgcggccaacttacttctgacaacgatcggaggaccgaaggagctaaccgcttttttgcacaacatgggggatcatgtaactcgccttgatcgttgggaaccggagctgaatgaagccataccaaacgacgagcgtgacaccacgatgcctgtagcaatggcaacaacgttgcgcaaactattaactggcgaactacttactctagcttcccggcaacaattaatagactggatggaggcggataaagttgcaggaccacttctgcgctcggcccttccggctggctggtttattgctgataaatctggagccggtgagcgtgggtctcgcggtatcattgcagcactggggccagatggtaagccctcccgtatcgtagttatctacacgacggggagtcaggcaactatggatgaacgaaatagacagatcgctgagataggtgcctcactgattaagcattggtaactgtcagaccaagtttactcatatatactttagattgatttaaaacttcatttttaatttaaaaggatctaggtgaagatcctttttgataatctcatgaccaaaatcccttaacgtgagttttcgttccactgagcgtcagaccccgtagaaaagatcaaaggatcttcttgagatcctttttttctgcgcgtaatctgctgcttgcaaacaaaaaaaccaccgctaccagcggtggtttgtttgccggatcaagagctaccaactctttttccgaaggtaactggcttcagcagagcgcagataccaaatactgtccttctagtgtagccgtagttaggccaccacttcaagaactctgtagcaccgcctacatacctcgctctgctaatcctgttaccagtggctgctgccagtggcgataagtcgtgtcttaccgggttggactcaagacgatagttaccggataaggcgcagcggtcgggctgaacggggggttcgtgcacacagcccagcttggagcgaacgacctacaccgaactgagatacctacagcgtgagctatgagaaagcgccacgcttcccgaagggagaaaggcggacaggtatccggtaagcggcagggtcggaacaggagagcgcacgagggagcttccagggggaaacgcctggtatctttatagtcctgtcgggtttcgccacctctgacttgagcgtcgatttttgtgatgctcgtcaggggggcggagcctatggaaaaacgccagcaacgcggcctttttacggttcctggccttttgctggccttttgctcacatgttctttcctgcgttatcccctgattctgtggataaccgtattaccgcctttgagtgagctgataccgctcgccgcagccgaacgaccgagcgcagcgagtcagtgagcgaggaagcggaagagcgcccaatacgcaaaccgcctctccccgcgcgttggccgattcattaatgcagctggcacgacaggtttcccgactggaaagcgggcagtgagcgcaacgcaattaatgtgagttagctcactcattaggcaccccaggctttacactttatgcttccggctcgtatgttgtgtggaattgtgagcggataacaatttcacacaggaaacagctatgaccatga

SEQ ID NO: 248 - DNA, 10644 bp, Synthetic construct
  source 1..10644: mol_type = other DNA
aaccttgttggtccaaaatgcgaacccagattgtaagactattttaaaagcattgggaccaggagcgacactagaagaaatgatgacagcatgtcagggagtggggggacccggccataaagcaagagttttggctgaagcaatgagccaagtaacaaatccagctaccataatgatacagaaaggcaattttaggaaccaaagaaagactgttaagtgtttcaattgtggcaaagaagggcacatagccaaaaattgcagggcccctaggaaaaagggctgttggaaatgtggaaaggaaggacaccaaatgaaagattgtactgagagacaggctaattttttagggaagatctggccttcccacaagggaaggccagggaattttcttcagagcagaccagagccaacagccccaccagaagagagcttcaggtttggggaagagacaacaactccctctcagaagcaggagccgatagacaaggaactgtatcctttagcttccctcagatcactctttggcagcgacccctcgtcacaataaagataggggggcaattaaaggaagctctattagatacaggagcagatgatacagtattagaagaaatgaatttgccaggaagatggaaaccaaaaatgatagggggaattggaggttttatcaaagtaagacagtatgatcagatactcatagaaatctgcggacataaagctataggtacagtattagtaggacctacacctgtcaacataattggaagaaatctgttgactcagattggctgcactttaaattttcccattagtcctattgagactgtaccagtaaaattaaagccaggaatggatggcccaaaagttaaacaatggccattgacagaagaaaaaataaaagcattagtagaaatttgtacagaaatggaaaaggaaggaaaaatttcaaaaattgggcctgaaaatccatacaatactccagtatttgccataaagaaaaaagacagtactaaatggagaaaattagtagatttcagagaacttaataagagaactcaagatttctgggaagttcaattaggaataccacatcctgcagggttaaaacagaaaaaatcagtaacagtactggatgtgggcgatgcatatttttcagttcccttagataaagacttcaggaagtatactgcatttaccatacctagtataaacaatgagacaccagggattagatatcagtacaatgtgcttccacagggatggaaaggatcaccagcaatattccagtgtagcatgacaaaaatcttagagccttttagaaaacaaaatccagacatagtcatctatcaatacatggatgatttgtatgtaggatctgacttagaaatagggcagcatagaacaaaaatagaggaactgagacaacatctgttgaggtggggatttaccacaccagacaaaaaacatcagaaagaacctccattcctttggatgggttatgaactccatcctgataaatggacagtacagcctatagtgctgccagaaaaggacagctggactgtcaatgacatacagaaattagtgggaaaattgaattgggcaagtcagatttatgcagggattaaagtaaggcaattatgtaaacttcttaggggaaccaaagcactaacagaagtagtaccactaacagaagaagcagagctagaactggcagaaaacagggagattctaaaagaaccggtacatggagtgtattatgacccatcaaaagacttaatagcagaaatacagaagcaggggcaaggccaatggacatatcaaatttatcaagagccatttaaaaatctgaaaacaggaaagtatgcaagaatgaagggtgcccacactaatgatgtgaaacaattaacagaggcagtacaaaaaatagccacagaaagcatagtaatatggggaaagactcctaaatttaaattacccatacaaaaggaaacatgggaagcatggtggacagagtattggcaagccacctggattcctgagtgggagtttgtcaatacccctcccttagtgaagttatggtaccagttagagaaagaacccataataggagcagaaactttctatgtagatggggcagccaatagggaaactaaattaggaaaagcaggatatgtaactgacagaggaagacaaaaagttgtccccctaacggacacaacaaatcagaagactgagttacaagcaattcatctagctttgcaggattcgggattagaagtaaacatagtgacagactcacaatatgcattgggaatcattcaagcacaaccagataagagtgaatcagagttagtcagtcaaataatagagcagttaataaaaaaggaaaaagtctacctggcatgggtaccagcacacaaaggaattggaggaaatgaacaagtagataaattggtcagtgctggaatcaggaaagtactatttttagatggaatagataaggcccaagaagaacatgagaaatatcacagtaattggagagcaatggctagtgattttaacctaccacctgtagtagcaaaagaaatagtagccagctgtgataaatgtcagctaaaaggggaagccatgcatggacaagtagactgtagcccaggaatatggcagctagtttgtacacatttagaaggaaaagttatcttggtagcagttcatgtagccagtggatatatagaagcagaagtaattccagcagagacagggcaagaaacagcatacttcctcttaaaattagcaggaagatggccagtaaaaacagtacatacagacaatggcagcaatttcaccagtactacagttaaggccgcctgttggtgggcggggatcaagcaggaatttggcattccctacaatccccaaagtcaaggagtaatagaatctatgaataaagaattaaagaaaattataggacaggtaagagatcaggctgaacatcttaagacagcagtacaaatggcagtattcatccacaattttaaaagaaaaggggggattggggggtacagtgcaggggaaagaatagtagacataatagcaacagacatacaaactaaagaattacaaaaacaaattacaaaaattcaaaattttcgggtttattacagggacagcagagatccagtttggaaaggaccagcaaagctcctctggaaaggtgaaggggcagtagtaatacaagataatagtgacataaaagtagtgccaagaagaaaagcaaagatcatcagggattatggaaaacagatggcaggtgatgattgtgtggcaagtagacaggatgaggattaacacatggaattctgcaacaactgctgtttatccatttcagaattgggtgtcgacatagcagaataggcgttactcgacagaggagagcaagaaatggagccagtagatcctagactagagccctggaagcatccaggaagtcagcctaaaactgcttgtaccaattgctattgtaaaaagtgttgctttcattgccaagtttgtttcatgacaaaagccttaggcatctcctatggcaggaagaagcggagacagcgacgaagagctcatcagaacagtcagactcatcaagcttctctatcaaagcagtaagtagtacatgtaatgcaacctataatagtagcaatagtagcattagtagtagcaataataatagcaatagttgtgtggtccatagtaatcatagaatataggaaaatggccgctgatcttcagacctggaggaggagatatgagggacaattggagaagtgaattatataaatataaagtagtaaaaattgaaccattaggagtagcacccaccaaggcaaagagaagagtggtgcagagagaaaaaagagcagtgggaataggagctttgttccttgggttcttgggagcagcaggaagcactatgggcgcagcgtcaatgacgctgacggtacaggccagacaattattgtctggtatagtgcagcagcagaacaatttgctgagggctattgaggcgcaacagcatctgttgcaactcacagtctggggcatcaagcagctccaggcaagaatcctggctgtggaaagatacctaaaggatcaacagctcctggggatttggggttgctctggaaaactcatttgcaccactgctgtgccttggaatgctagttggagtaataaatctctggaacagatttggaatcacacgacctggatggagtgggacagagaaattaacaattacacaagcttaatacactccttaattgaagaatcgcaaaaccagcaagaaaagaatgaacaagaattattggaattagataaatgggcaagtttgtggaattggtttaacataacaaattggctgtggtatataaaattattcataatgatagtaggaggcttggtaggtttaagaatagtttttgctgtactttctatagtgaatagagttaggcagggatattcaccattatcgtttcagacccacctcccaaccccgaggggacccgacaggcccgaaggaatagaagaagaaggtggagagagagacagagacagatccattcgattagtgaacggatccttggcacttatctgggacgatctgcggagcctgtgcctcttcagctaccaccgcttgagagacttactcttgattgtaacgaggattgtggaacttctgggacgcagggggtgggaagccctcaaatattggtggaatctcctacaatattggagtcaggagctaaagaatagtgctgttagcttgctcaatgccacagccatagcagtagctgaggggacagatagggttatagaagtagtacaaggagcttgtagagctattcgccacatacctagaagaataagacagggcttggaaaggattttgctataagctcgaaacaaccggtacctctagaactatagctagcagatctttttccctctgccaaaaattatggggacatcatgaagccccttgagcatctgacttctggctaataaaggaaatttattttcattgcaatagtgtgttggaattttttgtgtctctcactcggaaggacatatgggagggcaaatcatttaaaacatcagaatgagtatttggtttagagtttggcaacatatgcccatatgctggctgccatgaacaaaggttggctataaagaggtcatcagtatatgaaacagccccctgctgtccattccttattccatagaaaagccttgacttgaggttagattttttttatattttgttttgtgttatttttttctttaacatccctaaaattttccttacatgttttactagccagatttttcctcctctcctgactactcccagtcatagctgtccctcttctcttatggagatccctcgacctgcagcccaagcttggcgtaatcatggtcatagctgtttcctgtgtgaaattgttatccgctcacaattccacacaacatacgagccggaagcataaagtgtaaagcctggggtgcctaatgagtgagctaactcacattaattgcgttgcgctcactgcccgctttccagtcgggaaacctgtcgtgccagcggatccgcatctcaattagtcagcaaccatagtcccgcccctaactccgcccatcccgcccctaactccgcccagttccgcccattctccgccccatggctgactaattttttttatttatgcagaggccgaggccgcctcggcctctgagctattccagaagtagtgaggaggcttttttggaggcctaggcttttgcaaaaagctaacttgtttattgcagcttataatggttacaaataaagcaatagcatcacaaatttcacaaataaagcatttttttcactgcattctagttgtggtttgtccaaactcatcaatgtatcttatcatgtctggatccgctgcattaatgaatcggccaacgcgcggggagaggcggtttgcgtattgggcgctcttccgcttcctcgctcactgactcgctgcgctcggtcgttcggctgcggcgagcggtatcagctcactcaaaggcggtaatacggttatccacagaatcaggggataacgcaggaaagaacatgtgagcaaaaggccagcaaaaggccaggaaccgtaaaaaggccgcgttgctggcgtttttccataggctccgcccccctgacgagcatcacaaaaatcgacgctcaagtcagaggtggcgaaacccgacaggactataaagataccaggcgtttccccctggaagctccctcgtgcgctctcctgttccgaccctgccgcttaccggatacctgtccgcctttctcccttcgggaagcgtggcgctttctcatagctcacgctgtaggtatctcagttcggtgtaggtcgttcgctccaagctgggctgtgtgcacgaaccccccgttcagcccgaccgctgcgccttatccggtaactatcgtcttgagtccaacccggtaagacacgacttatcgccactggcagcagccactggtaacaggattagcagagcgaggtatgtaggcggtgctacagagttcttgaagtggtggcctaactacggctacactagaagaacagtatttggtatctgcgctctgctgaagccagttaccttcggaaaaagagttggtagctcttgatccggcaaacaaaccaccgctggtagcggtggtttttttgtttgcaagcagcagattacgcgcagaaaaaaaggatctcaagaagatcctttgatcttttctacggggtctgacgctcagtggaacgaaaactcacgttaagggattttggtcatgagattatcaaaaaggatcttcacctagatccttttaaattaaaaatgaagttttaaatcaatctaaagtatatatgagtaaacttggtctgacagttaccaatgcttaatcagtgaggcacctatctcagcgatctgtctatttcgttcatccatagttgcctgactccccgtcgtgtagataactacgatacgggagggcttaccatctggccccagtgctgcaatgataccgcgagacccacgctcaccggctccagatttatcagcaataaaccagccagccggaagggccgagcgcagaagtggtcctgcaactttatccgcctccatccagtctattaattgttgccgggaagctagagtaagtagttcgccagttaatagtttgcgcaacgttgttgccattgctacaggcatcgtggtgtcacgctcgtcgtttggtatggcttcattcagctccggttcccaacgatcaaggcgagttacatgatcccccatgttgtgcaaaaaagcggttagctccttcggtcctccgatcgttgtcagaagtaagttggccgcagtgttatcactcatggttatggcagcactgcataattctcttactgtcatgccatccgtaagatgcttttctgtgactggtgagtactcaaccaagtcattctgagaatagtgtatgcggcgaccgagttgctcttgcccggcgtcaatacgggataataccgcgccacatagcagaactttaaaagtgctcatcattggaaaacgttcttcggggcgaaaactctcaaggatcttaccgctgttgagatccagttcgatgtaacccactcgtgcacccaactgatcttcagcatcttttactttcaccagcgtttctgggtgagcaaaaacaggaaggcaaaatgccgcaaaaaagggaataagggcgacacggaaatgttgaatactcatactcttcctttttcaatattattgaagcatttatcagggttattgtctcatgagcggatacatatttgaatgtatttagaaaaataaacaaataggggttccgcgcacatttccccgaaaagtgccacctgggtcgacattgattattgactagttattaatagtaatcaattacggggtcattagttcatagcccatatatggagttccgcgttacataacttacggtaaatggcccgcctggctgaccgcccaacgacccccgcccattgacgtcaataatgacgtatgttcccatagtaacgccaatagggactttccattgacgtcaatgggtggagtatttacggtaaactgcccacttggcagtacatcaagtgtatcatatgccaagtacgccccctattgacgtcaatgacggtaaatggcccgcctggcattatgcccagtacatgaccttatgggactttcctacttggcagtacatctacgtattagtcatcgctattaccatggtcgaggtgagccccacgttctgcttcactctccccatctcccccccctccccacccccaattttgtatttatttattttttaattattttgtgcagggcgaggcggagaggtgcggcggcagccaatcagagcggcgcgctccgaaagtttccttttatggcgaggcggcggcggcggcggccctataaaaagcgaagcgcgcggcgggcgggagtcgctgcgcgctgccttcgccccgtgccccgctccgccgccgcctcgcgccgcccgccccggctctgactgaccgcgttactcccacaggtgagcgggcgggacggcccttctcctccgggctgtaattagcgcttggtttaatgacggcttgtttcttttctgtggctgcgtgaaagccttgaggggctccgggagggccctttgtgcggggggagcggctcggggggtgcgtgcgtgtgtgtgtgcgtggggagcgccgcgtgcggctccgcgctgcccggcggctgtgagcgctgcgggcgcggcgcggggctttgtgcgctccgcagtgtgcgcgaggggagcgcggccgggggcggtgccccgcggtgcggggggggctgcgaggggaacaaaggctgcgtgcggggtgtgtgcgtgggggggtgagcagggggtgtgggcgcgtcggtcgggctgcaaccccccctgcacccccctccccgagttgctgagcacggcccggcttcgggtgcggggctccgtacggggcgtggcgcggggctcgccgtgccgggcggggggtggcggcaggtgggggtgccgggcggggcggggccgcctcgggccggggagggctcgggggaggggcgcggcggcccccggagcgccggcggctgtcgaggcgcggcgagccgcagccattgccttttatggtaatcgtgcgagagggcgcagggacttcctttgtcccaaatctgtgcggagccgaaatctgggaggcgccgccgcaccccctctagcgggcgcggggcgaagcggtgcggcgccggcaggaaggaaatgggcggggagggccttcgtgcgtcgccgcgccgccgtccccttctccctctccagcctcggggctgtccgcggggggacggctgccttcgggggggacggggcagggcggggttcggcttctggcgtgtgaccggcggctctagagcctctgctaaccatgttcatgccttcttctttttcctacagctcctgggcaacgtgctggttattgtgctgtctcatcattttggcaaagaattcgggccgcgttgacgcgcacggcaagaggcgaggggcggcgactggtgagagatgggtgcgagagcgtcagtattaagcgggggagaattagatcgatgggaaaaaattcggagcaggccagggggaaagaaaaaatataaattaaaacatatagtatgggcaagcagggagctagaacgattcgcagttaatcctggcctgttagaaacatcagaaggctgtagacaaatactgggacagctacaaccatcccttcagacaggatcagaagaacttagatcattatataatacagtagcaaccctctattgtgtgcatcaaaggatagagataaaagacaccaaggaagctttagacaagatagaggaagagcaaaacaaaagtaagaaaaaagcacagcaagcagcagctgacacaggacacagcaatcaggtcagccaaaattaccctatagtgcagaacatccaggggcaaatggtacatcaggccatatcacctagaactttaaatgcatgggtaaaagtagtagaagagaaggctttcagcccagaagtgatacccatgttttcagcattatcagaaggagccaccccacaagatttaaacaccatgctaaacacagtggggggacatcaagcagccatgcaaatgttaaaagagaccatcaatgaggaagctgcagaatgggatagagtgcatccagtgcatgcagggcctattgcaccaggccagatgagagaaccaaggggaagtgacatagcaggaactactagtacccttcaggaacaaataggatggatgacacataatccacctatcccagtaggagaaatctataaaagatggataatcctgggattaaataaaatagtaagaatgtatagccctaccagcattctggacataagacaaggaccaaaggaaccctttagagactatgtagaccgattctataaaactctaagagccgagcaagcttcacaagaggtaaaaaattggatgacaga

SEQ ID NO: 249 - DNA, 14749 bp, Synthetic construct
  source 1..14749: mol_type = other DNA
aaccttgttggtccaaaatgcgaacccagattgtaagactattttaaaagcattgggaccaggagcgacactagaagaaatgatgacagcatgtcagggagtggggggacccggccataaagcaagagttttggctgaagcaatgagccaagtaacaaatccagctaccataatgatacagaaaggcaattttaggaaccaaagaaagactgttaagtgtttcaattgtggcaaagaagggcacatagccaaaaattgcagggcccctaggaaaaagggctgttggaaatgtggaaaggaaggacaccaaatgaaagattgtactgagagacaggctaattttttagggaagatctggccttcccacaagggaaggccagggaattttcttcagagcagaccagagccaacagccccaccagaagagagcttcaggtttggggaagagacaacaactccctctcagaagcaggagccgatagacaaggaactgtatcctttagcttccctcagatcactctttggcagcgacccctcgtcacaataaagataggggggcaattaaaggaagctctattagatacaggagcagatgatacagtattagaagaaatgaatttgccaggaagatggaaaccaaaaatgatagggggaattggaggttttatcaaagtaagacagtatgatcagatactcatagaaatctgcggacataaagctataggtacagtattagtaggacctacacctgtcaacataattggaagaaatctgttgactcagattggctgcactttaaattttcccattagtcctattgagactgtaccagtaaaattaaagccaggaatggatggcccaaaagttaaacaatggccattgacagaagaaaaaataaaagcattagtagaaatttgtacagaaatggaaaaggaaggaaaaatttcaaaaattgggcctgaaaatccatacaatactccagtatttgccataaagaaaaaagacagtactaaatggagaaaattagtagatttcagagaacttaataagagaactcaagatttctgggaagttcaattaggaataccacatcctgcagggttaaaacagaaaaaatcagtaacagtactggatgtgggcgatgcatatttttcagttcccttagataaagacttcaggaagtatactgcatttaccatacctagtataaacaatgagacaccagggattagatatcagtacaatgtgcttccacagggatggaaaggatcaccagcaatattccagtgtagcatgacaaaaatcttagagccttttagaaaacaaaatccagacatagtcatctatcaatacatggatgatttgtatgtaggatctgacttagaaatagggcagcatagaacaaaaatagaggaactgagacaacatctgttgaggtggggatttaccacaccagacaaaaaacatcagaaagaacctccattcctttggatgggttatgaactccatcctgataaatggacagtacagcctatagtgctgccagaaaaggacagctggactgtcaatgacatacagaaattagtgggaaaattgaattgggcaagtcagatttatgcagggattaaagtaaggcaattatgtaaacttcttaggggaaccaaagcactaacagaagtagtaccactaacagaagaagcagagctagaactggcagaaaacagggagattctaaaagaaccggtacatggagtgtattatgacccatcaaaagacttaatagcagaaatacagaagcaggggcaaggccaatggacatatcaaatttatcaagagccatttaaaaatctgaaaacaggaaagtatgcaagaatgaagggtgcccacactaatgatgtgaaacaattaacagaggcagtacaaaaaatagccacagaaagcatagtaatatggggaaagactcctaaatttaaattacccatacaaaaggaaacatgggaagcatggtggacagagtattggcaagccacctggattcctgagtgggagtttgtcaatacccctcccttagtgaagttatggtaccagttagagaaagaacccataataggagcagaaactttctatgtagatggggcagccaatagggaaactaaattaggaaaagcaggatatgtaactgacagaggaagacaaaaagttgtccccctaacggacacaacaaatcagaagactgagttacaagcaattcatctagctttgcaggattcgggattagaagtaaacatagtgacagactcacaatatgcattgggaatcattcaagcacaaccagataagagtgaatcagagttagtcagtcaaataatagagcagttaataaaaaaggaaaaagtctacctggcatgggtaccagcacacaaaggaattggaggaaatgaacaagtagataaattggtcagtgctggaatcaggaaagtactatttttagatggaatagataaggcccaagaagaacatgagaaatatcacagtaattggagagcaatggctagtgattttaacctaccacctgtagtagcaaaagaaatagtagccagctgtgataaatgtcagctaaaaggggaagccatgcatggacaagtagactgtagcccaggaatatggcagctagtttgtacacatttagaaggaaaagttatcttggtagcagttcatgtagccagtggatatatagaagcagaagtaattccagcagagacagggcaagaaacagcatacttcctcttaaaattagcaggaagatggccagtaaaaacagtacatacagacaatggcagcaatttcaccagtactacagttaaggccgcctgttggtgggcggggatcaagcaggaatttggcattccctacaatccccaaagtcaaggagtaatagaatctatgaataaagaattaaagaaaattataggacaggtaagagatcaggctgaacatcttaagacagcagtacaaatggcagtattcatccacaattttaaaagaaaaggggggattggggggtacagtgcaggggaaagaatagtagacataatagcaacagacatacaaactaaagaattacaaaaacaaattacaaaaattcaaaattttcgggtttattacagggacagcagagatccagtttggaaaggaccagcaaagctcctctggaaaggtgaaggggcagtagtaatacaagataatagtgacataaaagtagtgccaagaagaaaagcaaagatcatcagggattatggaaaacagatggcaggtgatgattgtgtggcaagtagacaggatgaggattaacacatggaattctgcaacaactgctgtttatccatttcagaattgggtgtcgacatagcagaataggcgttactcgacagaggagagcaagaaatggagccagtagatcctagactagagccctggaagcatccaggaagtcagcctaaaactgcttgtaccaattgctattgtaaaaagtgttgctttcattgccaagtttgtttcatgacaaaagccttaggcatctcctatggcaggaagaagcggagacagcgacgaagagctcatcagaacagtcagactcatcaagcttctctatcaaagcagtaagtagtacatgtaatgcaacctataatagtagcaatagtagcattagtagtagcaataataatagcaatagttgtgtggtccatagtaatcatagaatataggaaaatggccgctgatcttcagacctggaggaggagatatgagggacaattggagaagtgaattatataaatataaagtagtaaaaattgaaccattaggagtagcacccaccaaggcaaagagaagagtggtgcagagagaaaaaagagcagtgggaataggagctttgttccttgggttcttgggagcagcaggaagcactatgggcgcagcgtcaatgacgctgacggtacaggccagacaattattgtctggtatagtgcagcagcagaacaatttgctgagggctattgaggcgcaacagcatctgttgcaactcacagtctggggcatcaagcagctccaggcaagaatcctggctgtggaaagatacctaaaggatcaacagctcctggggatttggggttgctctggaaaactcatttgcaccactgctgtgccttggaatgctagttggagtaataaatctctggaacagatttggaatcacacgacctggatggagtgggacagagaaattaacaattacacaagcttaatacactccttaattgaagaatcgcaaaaccagcaagaaaagaatgaacaagaattattggaattagataaatgggcaagtttgtggaattggtttaacataacaaattggctgtggtatataaaattattcataatgatagtaggaggcttggtaggtttaagaatagtttttgctgtactttctatagtgaatagagttaggcagggatattcaccattatcgtttcagacccacctcccaaccccgaggggacccgacaggcccgaaggaatagaagaagaaggtggagagagagacagagacagatccattcgattagtgaacggatccttggcacttatctgggacgatctgcggagcctgtgcctcttcagctaccaccgcttgagagacttactcttgattgtaacgaggattgtggaacttctgggacgcagggggtgggaagccctcaaatattggtggaatctcctacaatattggagtcaggagctaaagaatagtgctgttagcttgctcaatgccacagccatagcagtagctgaggggacagatagggttatagaagtagtacaaggagcttgtagagctattcgccacatacctagaagaataagacagggcttggaaaggattttgctataagctcgaaacaaccggtacctctagaactatagctagcagatctttttccctctgccaaaaattatggggacatcatgaagccccttgagcatctgacttctggctaataaaggaaatttattttcattgcaatagtgtgttggaattttttgtgtctctcactcggaaggacatatgggagggcaaatcatttaaaacatcagaatgagtatttggtttagagtttggcaacatatgcccatatgctggctgccatgaacaaaggttggctataaagaggtcatcagtatatgaaacagccccctgctgtccattccttattccatagaaaagccttgacttgaggttagattttttttatattttgttttgtgttatttttttctttaacatccctaaaattttccttacatgttttactagccagatttttcctcctctcctgactactcccagtcatagctgtccctcttctcttatggagatccctcgacctgcagcccaagcttggcgtaatcatggtcatagctgtttcctgtgtgaaattgttatccgctcacaattccacacaacatacgagccggaagcataaagtgtaaagcctggggtgcctaatgagtgagctaactcacattaattgcgttgcgctcactgcccgctttccagtcgggaaacctgtcgtgccagcggatccggcgcgccggattcgacattgattattgactagttattaatagtaatcaattacggggtcattagttcatagcccatatatggagttccgcgttacataacttacggtaaatggcccgcctggctgaccgcccaacgacccccgcccattgacgtcaataatgacgtatgttcccatagtaacgccaatagggactttccattgacgtcaatgggtggagtatttacggtaaactgcccacttggcagtacatcaagtgtatcatatgccaagtacgccccctattgacgtcaatgacggtaaatggcccgcctggcattatgcccagtacatgaccttatgggactttcctacttggcagtacatctacgtattagtcatcgctattaccatggtcgaggtgagccccacgttctgcttcactctccccatctcccccccctccccacccccaattttgtatttatttattttttaattattttgtgcagcgatgggggcggggggggggggggggcgcgcgccaggcggggcggggcggggcgaggggcggggcggggcgaggcggagaggtgcggcggcagccaatcagagcggcgcgctccgaaagtttccttttatggcgaggcggcggcggcggcggccctataaaaagcgaagcgcgcggcgggcgggagtcgctgcgtcgcgccttcgccccgtgccccgctccgccgccgcctcgcgccgcccgccccggctctgactgaccgcgttactcccacaggtgagcgggcgggacggcccttctcctccgggctgtaattagcgcttggtttaatgacggctcgtttcttttctgtggctgcgtgaaagccttaaagggctccgggagggccctttgtgcgggggggagcggctcggggggtgcgtgcgtgtgtgtgtgcgtggggagcgccgcgtgcggcccgcgctgcccggcggctgtgagcgctgcgggcgcggcgcggggctttgtgcgctccgcgtgtgcgcgaggggagcgcggccgggggcggtgccccgcggtgcgggggggctgcgaggggaacaaaggctgcgtgcggggtgtgtgcgtgggggggtgagcagggggtgtgggcgcggcggtcgggctgtaacccccccctgcacccccctccccgagttgctgagcacggcccggcttcgggtgcggggctccgtgcggggcgtggcgcggggctcgccgtgccgggcggggggtggcggcaggtgggggtgccgggcggggcggggccgcctcgggccggggagggctcgggggaggggcgcggcggccccggagcgccggcggctgtcgaggcgcggcgagccgcagccattgccttttatggtaatcgtgcgagagggcgcagggacttcctttgtcccaaatctggcggagccgaaatctgggaggcgccgccgcaccccctctagcgggcgcgggcgaagcggtgcggcgccggcaggaaggaaatgggcggggagggccttcgtgcgtcgccgcgccgccgtccccttctccatctccagcctcggggctgccgcagggggacggctgccttcgggggggacggggcagggcggggttcggcttctggcgtgtgaccggcggctctagagcctctgctaaccatgttcatgccttcttctttttcctacagatccttaattaataatacgactcactataggggccgccaccatgggcgctagagcctctgttctgtctggcggcgaactggacagatgggagaagatcagaagcagacctggcggcaagaagaagtacaagctgaagcacatcgtgtgggccagcagagagctggaaagattcgctgtgaaccccggcctgctggaaacaagcgagggctgtagacagatcctgggccagctccagccatctctccagacaggatctgaggaactgagaagcctgtacaacaccgtggccacactgtactgcgtgcaccagagaatcgagatcaaggacaccaaagaggccctggacaagatcgaggaagaacagaacaagtctaagaagaaggcccagcaggctgccgccgatacaggccactctaatcaggtgtcccagaactaccccatcgtgcagaacatccagggccagatggtgcatcaggctatcagccccagaacactgaacgcctgggtcaaagtggtggaagagaaggctttcagccctgaagtgatccccatgttcagcgccctgtctgagggtgccacacctcaggacctgaacaccatgctgaacacagtcggcggacaccaggccgctatgcagatgctgaaagagacaatcaacgaagaggccgccgagtgggacagagtgcatcctgttcatgctggccctatcgctcccggccagatgagagaacctagaggctctgacattgccggcaccaccagcacactgcaagagcagatcggctggatgacaaacaaccctcctattcctgtgggcgagatctacaagagatggatcatcctgggactgaacaagatcgtgcggatgtacagccccaccagcatcctggacattagacagggccccaaagagcccttcagagactacgtggacagattctacaagaccctgagagccgagcaggccagccaagaagtgaagaactggatgaccgagacactgctggtgcagaacgctaaccccgactgcaagaccatcctgaaggctctgggacctgccgccacactggaagagatgatgacagcctgtcaaggcgtcggaggacctggccataaggctagagttctggccgaggccatgagccaagtgaccaacagcgccacaatcatgatgcagagaggcaacttcagaaaccagcggaagatcgtgaagtccttcaactccggcaaagagggccacaccgcccgcaattctagagcccctagaaagaaaggtggatccggcggcgtttctggatggcggctgttcaagaagatcagcggcggttccggacctgctgccaaaagagtgaaactggactccggactgcaactgcctccactggaaagactgacactgggagctgccccagccgccaagaagaaaaagctggactacaaggacgacgacgacaagggcggagctagctctaagacaatcgtgctgtctgtgggcgaagccaccagaacactgaccgagatccagagcacagccgacagacagatcttcgaggaaaaagtgggccctctcgtgggcagactgagactgacagcttccctgagacagaacggcgccaagaccgcctacagagtgaacctgaagctggaccaggccgacgtggtggattctggccttcctaaagtgcggtacacccaagtgtggtcccacgacgtgaccatcgtggccaattctaccgaggccagcagaaagagcctgtacgacctgaccaagagcctggtggccacaagccaggtggaagatctggtcgtgaacctggtgcctctcggacgtggcggatccggtggaaccgagagacaggccaacttcctgggcaagatctggcctagctacaagggcagacccggcaacttcctccagagcagaccagagcctaccgctcctcctgaggaatccttcagatccggcgtggaaaccaccacacctccacagaagcaagagcccatcgacaaagagctgtaccctctgaccagcctgagatccctgttcggcaacgaccctagctctcaatgaacgcgtaaatgattgcagatccactagttctagagctcgctgatcagcctcgactgtgccttctagttgccagccatctgttgtttgcccctcccccgtgccttccttgaccctggaaggtgccactcccactgtcctttcctaataaaatgaggaaattgcatcgcattgtctgagtaggtgtcattctattctggggggtggggtggggcaggacagcaagggggaggattgggaagacaatagcaggcatgctggggatgcggtgggctctatggcttctgaggcggaaagaaccagctggggctcgagatccactagttctagcctcgaggctagagcggccgcgcatctcaattagtcagcaaccatagtcccgcccctaactccgcccatcccgcccctaactccgcccagttccgcccattctccgccccatggctgactaattttttttatttatgcagaggccgaggccgcctcggcctctgagctattccagaagtagtgaggaggcttttttggaggcctaggcttttgcaaaaagctaacttgtttattgcagcttataatggttacaaataaagcaatagcatcacaaatttcacaaataaagcatttttttcactgcattctagttgtggtttgtccaaactcatcaatgtatcttatcatgtctggatccgctgcattaatgaatcggccaacgcgcggggagaggcggtttgcgtattgggcgctcttccgcttcctcgctcactgactcgctgcgctcggtcgttcggctgcggcgagcggtatcagctcactcaaaggcggtaatacggttatccacagaatcaggggataacgcaggaaagaacatgtgagcaaaaggccagcaaaaggccaggaaccgtaaaaaggccgcgttgctggcgtttttccataggctccgcccccctgacgagcatcacaaaaatcgacgctcaagtcagaggtggcgaaacccgacaggactataaagataccaggcgtttccccctggaagctccctcgtgcgctctcctgttccgaccctgccgcttaccggatacctgtccgcctttctcccttcgggaagcgtggcgctttctcatagctcacgctgtaggtatctcagttcggtgtaggtcgttcgctccaagctgggctgtgtgcacgaaccccccgttcagcccgaccgctgcgccttatccggtaactatcgtcttgagtccaacccggtaagacacgacttatcgccactggcagcagccactggtaacaggattagcagagcgaggtatgtaggcggtgctacagagttcttgaagtggtggcctaactacggctacactagaagaacagtatttggtatctgcgctctgctgaagccagttaccttcggaaaaagagttggtagctcttgatccggcaaacaaaccaccgctggtagcggtggtttttttgtttgcaagcagcagattacgcgcagaaaaaaaggatctcaagaagatcctttgatcttttctacggggtctgacgctcagtggaacgaaaactcacgttaagggattttggtcatgagattatcaaaaaggatcttcacctagatccttttaaattaaaaatgaagttttaaatcaatctaaagtatatatgagtaaacttggtctgacagttaccaatgcttaatcagtgaggcacctatctcagcgatctgtctatttcgttcatccatagttgcctgactccccgtcgtgtagataactacgatacgggagggcttaccatctggccccagtgctgcaatgataccgcgagacccacgctcaccggctccagatttatcagcaataaaccagccagccggaagggccgagcgcagaagtggtcctgcaactttatccgcctccatccagtctattaattgttgccgggaagctagagtaagtagttcgccagttaatagtttgcgcaacgttgttgccattgctacaggcatcgtggtgtcacgctcgtcgtttggtatggcttcattcagctccggttcccaacgatcaaggcgagttacatgatcccccatgttgtgcaaaaaagcggttagctccttcggtcctccgatcgttgtcagaagtaagttggccgcagtgttatcactcatggttatggcagcactgcataattctcttactgtcatgccatccgtaagatgcttttctgtgactggtgagtactcaaccaagtcattctgagaatagtgtatgcggcgaccgagttgctcttgcccggcgtcaatacgggataataccgcgccacatagcagaactttaaaagtgctcatcattggaaaacgttcttcggggcgaaaactctcaaggatcttaccgctgttgagatccagttcgatgtaacccactcgtgcacccaactgatcttcagcatcttttactttcaccagcgtttctgggtgagcaaaaacaggaaggcaaaatgccgcaaaaaagggaataagggcgacacggaaatgttgaatactcatactcttcctttttcaatattattgaagcatttatcagggttattgtctcatgagcggatacatatttgaatgtatttagaaaaataaacaaataggggttccgcgcacatttccccgaaaagtgccacctgggtcgacattgattattgactagttattaatagtaatcaattacggggtcattagttcatagcccatatatggagttccgcgttacataacttacggtaaatggcccgcctggctgaccgcccaacgacccccgcccattgacgtcaataatgacgtatgttcccatagtaacgccaatagggactttccattgacgtcaatgggtggagtatttacggtaaactgcccacttggcagtacatcaagtgtatcatatgccaagtacgccccctattgacgtcaatgacggtaaatggcccgcctggcattatgcccagtacatgaccttatgggactttcctacttggcagtacatctacgtattagtcatcgctattaccatggtcgaggtgagccccacgttctgcttcactctccccatctcccccccctccccacccccaattttgtatttatttattttttaattattttgtgcagggcgaggcggagaggtgcggcggcagccaatcagagcggcgcgctccgaaagtttccttttatggcgaggcggcggcggcggcggccctataaaaagcgaagcgcgcggcgggcgggagtcgctgcgcgctgccttcgccccgtgccccgctccgccgccgcctcgcgccgcccgccccggctctgactgaccgcgttactcccacaggtgagcgggcgggacggcccttctcctccgggctgtaattagcgcttggtttaatgacggcttgtttcttttctgtggctgcgtgaaagccttgaggggctccgggagggccctttgtgcggggggagcggctcggggggtgcgtgcgtgtgtgtgtgcgtggggagcgccgcgtgcggctccgcgctgcccggcggctgtgagcgctgcgggcgcggcgcggggctttgtgcgctccgcagtgtgcgcgaggggagcgcggccgggggcggtgccccgcggtgcggggggggctgcgaggggaacaaaggctgcgtgcggggtgtgtgcgtgggggggtgagcagggggtgtgggcgcgtcggtcgggctgcaaccccccctgcacccccctccccgagttgctgagcacggcccggcttcgggtgcggggctccgtacggggcgtggcgcggggctcgccgtgccgggcggggggtggcggcaggtgggggtgccgggcggggcggggccgcctcgggccggggagggctcgggggaggggcgcggcggcccccggagcgccggcggctgtcgaggcgcggcgagccgcagccattgccttttatggtaatcgtgcgagagggcgcagggacttcctttgtcccaaatctgtgcggagccgaaatctgggaggcgccgccgcaccccctctagcgggcgcggggcgaagcggtgcggcgccggcaggaaggaaatgggcggggagggccttcgtgcgtcgccgcgccgccgtccccttctccctctccagcctcggggctgtccgcggggggacggctgccttcgggggggacggggcagggcggggttcggcttctggcgtgtgaccggcggctctagagcctctgctaaccatgttcatgccttcttctttttcctacagctcctgggcaacgtgctggttattgtgctgtctcatcattttggcaaagaattcgggccgcgttgacgcgcacggcaagaggcgaggggcggcgactggtgagagatgggtgcgagagcgtcagtattaagcgggggagaattagatcgatgggaaaaaattcggttaaggccagggggaaagaaaaaatataaattaaaacatatagtatgggcaagcagggagctagaacgattcgcagttaatcctggcctgttagaaacatcagaaggctgtagacaaatactgggacagctacaaccatcccttcagacaggatcagaagaacttagatcattatataatacagtagcaaccctctattgtgtgcatcaaaggatagagataaaagacaccaaggaagctttagacaagatagaggaagagcaaaacaaaagtaagaaaaaagcacagcaagcagcagctgacacaggacacagcaatcaggtcagccaaaattaccctatagtgcagaacatccaggggcaaatggtacatcaggccatatcacctagaactttaaatgcatgggtaaaagtagtagaagagaaggctttcagcccagaagtgatacccatgttttcagcattatcagaaggagccaccccacaagatttaaacaccatgctaaacacagtggggggacatcaagcagccatgcaaatgttaaaagagaccatcaatgaggaagctgcagaatgggatagagtgcatccagtgcatgcagggcctattgcaccaggccagatgagagaaccaaggggaagtgacatagcaggaactactagtacccttcaggaacaaataggatggatgacacataatccacctatcccagtaggagaaatctataaaagatggataatcctgggattaaataaaatagtaagaatgtatagccctaccagcattctggacataagacaaggaccaaaggaaccctttagagactatgtagaccgattctataaaactctaagagccgagcaagcttcacaagaggtaaaaaattggatgacaga

SEQ ID NO: 250 - DNA, 11166 bp, Synthetic construct
  source 1..11166: mol_type = other DNA
agccattgccttttatggtaatcgtgcgagagggcgcagggacttcctttgtcccaaatctgtgcggagccgaaatctgggaggcgccgccgcaccccctctagcgggcgcggggcgaagcggtgcggcgccggcaggaaggaaatgggcggggagggccttcgtgcgtcgccgcgccgccgtccccttctccctctccagcctcggggctgtccgcggggggacggctgccttcgggggggacggggcagggcggggttcggcttctggcgtgtgaccggcggctctagagcctctgctaaccatgttcatgccttcttctttttcctacagctcctgggcaacgtgctggttattgtgctgtctcatcattttggcaaagaattcgggccgcgttgacgcgcacggcaagaggcgaggggcggcgactggtgagagatgggtgcgagagcgtcagtattaagcgggggagaattagatcgatgggaaaaaattcggttaaggccagggggaaagaaaaaatataaattaaaacatatagtatgggcaagcagggagctagaacgattcgcagttaatcctggcctgttagaaacatcagaaggctgtagacaaatactgggacagctacaaccatcccttcagacaggatcagaagaacttagatcattatataatacagtagcaaccctctattgtgtgcatcaaaggatagagataaaagacaccaaggaagctttagacaagatagaggaagagcaaaacaaaagtaagaaaaaagcacagcaagcagcagctgacacaggacacagcaatcaggtcagccaaaattaccctatagtgcagaacatccaggggcaaatggtacatcaggccatatcacctagaactttaaatgcatgggtaaaagtagtagaagagaaggctttcagcccagaagtgatacccatgttttcagcattatcagaaggagccaccccacaagatttaaacaccatgctaaacacagtggggggacatcaagcagccatgcaaatgttaaaagagaccatcaatgaggaagctgcagaatgggatagagtgcatccagtgcatgcagggcctattgcaccaggccagatgagagaaccaaggggaagtgacatagcaggaactactagtacccttcaggaacaaataggatggatgacacataatccacctatcccagtaggagaaatctataaaagatggataatcctgggattaaataaaatagtaagaatgtatagccctaccagcattctggacataagacaaggaccaaaggaaccctttagagactatgtagaccgattctataaaactctaagagccgagcaagcttcacaagaggtaaaaaattggatgacagaaaccttgttggtccaaaatgcgaacccagattgtaagactattttaaaagcattgggaccaggagcgacactagaagaaatgatgacagcatgtcagggagtggggggacccggccataaagcaagagttttggctgaagcaatgagccaagtaacaaatccagctaccataatgatacagaaaggcaattttaggaaccaaagaaagactgttaagggatccggcggcgtttctggatggcggctgttcaagaagatcagcggcggttccggacctgctgccaaaagagtgaaactggactccggactgcaactgcctccactggaaagactgacactgggagctgccccagccgccaagaagaaaaagctggactacaaggacgacgacgacaagggcggagctagctctaagacaatcgtgctgtctgtgggcgaagccaccagaacactgaccgagatccagagcacagccgacagacagatcttcgaggaaaaagtgggccctctcgtgggcagactgagactgacagcttccctgagacagaacggcgccaagaccgcctacagagtgaacctgaagctggaccaggccgacgtggtggattctggccttcctaaagtgcggtacacccaagtgtggtcccacgacgtgaccatcgtggccaattctaccgaggccagcagaaagagcctgtacgacctgaccaagagcctggtggccacaagccaggtggaagatctggtcgtgaacctggtgcctctcggacgtggcggatccagggcccctaggaaaaagggctgttggaaatgtggaaaggaaggacaccaaatgaaagattgtactgagagacaggctaattttttagggaagatctggccttcccacaagggaaggccagggaattttcttcagagcagaccagagccaacagccccaccagaagagagcttcaggtttggggaagagacaacaactccctctcagaagcaggagccgatagacaaggaactgtatcctttagcttccctcagatcactctttggcagcgacccctcgtcacaataaagataggggggcaattaaaggaagctctattagatacaggagcagatgatacagtattagaagaaatgaatttgccaggaagatggaaaccaaaaatgatagggggaattggaggttttatcaaagtaagacagtatgatcagatactcatagaaatctgcggacataaagctataggtacagtattagtaggacctacacctgtcaacataattggaagaaatctgttgactcagattggctgcactttaaattttcccattagtcctattgagactgtaccagtaaaattaaagccaggaatggatggcccaaaagttaaacaatggccattgacagaagaaaaaataaaagcattagtagaaatttgtacagaaatggaaaaggaaggaaaaatttcaaaaattgggcctgaaaatccatacaatactccagtatttgccataaagaaaaaagacagtactaaatggagaaaattagtagatttcagagaacttaataagagaactcaagatttctgggaagttcaattaggaataccacatcctgcagggttaaaacagaaaaaatcagtaacagtactggatgtgggcgatgcatatttttcagttcccttagataaagacttcaggaagtatactgcatttaccatacctagtataaacaatgagacaccagggattagatatcagtacaatgtgcttccacagggatggaaaggatcaccagcaatattccagtgtagcatgacaaaaatcttagagccttttagaaaacaaaatccagacatagtcatctatcaatacatggatgatttgtatgtaggatctgacttagaaatagggcagcatagaacaaaaatagaggaactgagacaacatctgttgaggtggggatttaccacaccagacaaaaaacatcagaaagaacctccattcctttggatgggttatgaactccatcctgataaatggacagtacagcctatagtgctgccagaaaaggacagctggactgtcaatgacatacagaaattagtgggaaaattgaattgggcaagtcagatttatgcagggattaaagtaaggcaattatgtaaacttcttaggggaaccaaagcactaacagaagtagtaccactaacagaagaagcagagctagaactggcagaaaacagggagattctaaaagaaccggtacatggagtgtattatgacccatcaaaagacttaatagcagaaatacagaagcaggggcaaggccaatggacatatcaaatttatcaagagccatttaaaaatctgaaaacaggaaagtatgcaagaatgaagggtgcccacactaatgatgtgaaacaattaacagaggcagtacaaaaaatagccacagaaagcatagtaatatggggaaagactcctaaatttaaattacccatacaaaaggaaacatgggaagcatggtggacagagtattggcaagccacctggattcctgagtgggagtttgtcaatacccctcccttagtgaagttatggtaccagttagagaaagaacccataataggagcagaaactttctatgtagatggggcagccaatagggaaactaaattaggaaaagcaggatatgtaactgacagaggaagacaaaaagttgtccccctaacggacacaacaaatcagaagactgagttacaagcaattcatctagctttgcaggattcgggattagaagtaaacatagtgacagactcacaatatgcattgggaatcattcaagcacaaccagataagagtgaatcagagttagtcagtcaaataatagagcagttaataaaaaaggaaaaagtctacctggcatgggtaccagcacacaaaggaattggaggaaatgaacaagtagataaattggtcagtgctggaatcaggaaagtactatttttagatggaatagataaggcccaagaagaacatgagaaatatcacagtaattggagagcaatggctagtgattttaacctaccacctgtagtagcaaaagaaatagtagccagctgtgataaatgtcagctaaaaggggaagccatgcatggacaagtagactgtagcccaggaatatggcagctagtttgtacacatttagaaggaaaagttatcttggtagcagttcatgtagccagtggatatatagaagcagaagtaattccagcagagacagggcaagaaacagcatacttcctcttaaaattagcaggaagatggccagtaaaaacagtacatacagacaatggcagcaatttcaccagtactacagttaaggccgcctgttggtgggcggggatcaagcaggaatttggcattccctacaatccccaaagtcaaggagtaatagaatctatgaataaagaattaaagaaaattataggacaggtaagagatcaggctgaacatcttaagacagcagtacaaatggcagtattcatccacaattttaaaagaaaaggggggattggggggtacagtgcaggggaaagaatagtagacataatagcaacagacatacaaactaaagaattacaaaaacaaattacaaaaattcaaaattttcgggtttattacagggacagcagagatccagtttggaaaggaccagcaaagctcctctggaaaggtgaaggggcagtagtaatacaagataatagtgacataaaagtagtgccaagaagaaaagcaaagatcatcagggattatggaaaacagatggcaggtgatgattgtgtggcaagtagacaggatgaggattaacacatggaattctgcaacaactgctgtttatccatttcagaattgggtgtcgacatagcagaataggcgttactcgacagaggagagcaagaaatggagccagtagatcctagactagagccctggaagcatccaggaagtcagcctaaaactgcttgtaccaattgctattgtaaaaagtgttgctttcattgccaagtttgtttcatgacaaaagccttaggcatctcctatggcaggaagaagcggagacagcgacgaagagctcatcagaacagtcagactcatcaagcttctctatcaaagcagtaagtagtacatgtaatgcaacctataatagtagcaatagtagcattagtagtagcaataataatagcaatagttgtgtggtccatagtaatcatagaatataggaaaatggccgctgatcttcagacctggaggaggagatatgagggacaattggagaagtgaattatataaatataaagtagtaaaaattgaaccattaggagtagcacccaccaaggcaaagagaagagtggtgcagagagaaaaaagagcagtgggaataggagctttgttccttgggttcttgggagcagcaggaagcactatgggcgcagcgtcaatgacgctgacggtacaggccagacaattattgtctggtatagtgcagcagcagaacaatttgctgagggctattgaggcgcaacagcatctgttgcaactcacagtctggggcatcaagcagctccaggcaagaatcctggctgtggaaagatacctaaaggatcaacagctcctggggatttggggttgctctggaaaactcatttgcaccactgctgtgccttggaatgctagttggagtaataaatctctggaacagatttggaatcacacgacctggatggagtgggacagagaaattaacaattacacaagcttaatacactccttaattgaagaatcgcaaaaccagcaagaaaagaatgaacaagaattattggaattagataaatgggcaagtttgtggaattggtttaacataacaaattggctgtggtatataaaattattcataatgatagtaggaggcttggtaggtttaagaatagtttttgctgtactttctatagtgaatagagttaggcagggatattcaccattatcgtttcagacccacctcccaaccccgaggggacccgacaggcccgaaggaatagaagaagaaggtggagagagagacagagacagatccattcgattagtgaacggatccttggcacttatctgggacgatctgcggagcctgtgcctcttcagctaccaccgcttgagagacttactcttgattgtaacgaggattgtggaacttctgggacgcagggggtgggaagccctcaaatattggtggaatctcctacaatattggagtcaggagctaaagaatagtgctgttagcttgctcaatgccacagccatagcagtagctgaggggacagatagggttatagaagtagtacaaggagcttgtagagctattcgccacatacctagaagaataagacagggcttggaaaggattttgctataagctcgaaacaaccggtacctctagaactatagctagcagatctttttccctctgccaaaaattatggggacatcatgaagccccttgagcatctgacttctggctaataaaggaaatttattttcattgcaatagtgtgttggaattttttgtgtctctcactcggaaggacatatgggagggcaaatcatttaaaacatcagaatgagtatttggtttagagtttggcaacatatgcccatatgctggctgccatgaacaaaggttggctataaagaggtcatcagtatatgaaacagccccctgctgtccattccttattccatagaaaagccttgacttgaggttagattttttttatattttgttttgtgttatttttttctttaacatccctaaaattttccttacatgttttactagccagatttttcctcctctcctgactactcccagtcatagctgtccctcttctcttatggagatccctcgacctgcagcccaagcttggcgtaatcatggtcatagctgtttcctgtgtgaaattgttatccgctcacaattccacacaacatacgagccggaagcataaagtgtaaagcctggggtgcctaatgagtgagctaactcacattaattgcgttgcgctcactgcccgctttccagtcgggaaacctgtcgtgccagcggatccgcatctcaattagtcagcaaccatagtcccgcccctaactccgcccatcccgcccctaactccgcccagttccgcccattctccgccccatggctgactaattttttttatttatgcagaggccgaggccgcctcggcctctgagctattccagaagtagtgaggaggcttttttggaggcctaggcttttgcaaaaagctaacttgtttattgcagcttataatggttacaaataaagcaatagcatcacaaatttcacaaataaagcatttttttcactgcattctagttgtggtttgtccaaactcatcaatgtatcttatcatgtctggatccgctgcattaatgaatcggccaacgcgcggggagaggcggtttgcgtattgggcgctcttccgcttcctcgctcactgactcgctgcgctcggtcgttcggctgcggcgagcggtatcagctcactcaaaggcggtaatacggttatccacagaatcaggggataacgcaggaaagaacatgtgagcaaaaggccagcaaaaggccaggaaccgtaaaaaggccgcgttgctggcgtttttccataggctccgcccccctgacgagcatcacaaaaatcgacgctcaagtcagaggtggcgaaacccgacaggactataaagataccaggcgtttccccctggaagctccctcgtgcgctctcctgttccgaccctgccgcttaccggatacctgtccgcctttctcccttcgggaagcgtggcgctttctcatagctcacgctgtaggtatctcagttcggtgtaggtcgttcgctccaagctgggctgtgtgcacgaaccccccgttcagcccgaccgctgcgccttatccggtaactatcgtcttgagtccaacccggtaagacacgacttatcgccactggcagcagccactggtaacaggattagcagagcgaggtatgtaggcggtgctacagagttcttgaagtggtggcctaactacggctacactagaagaacagtatttggtatctgcgctctgctgaagccagttaccttcggaaaaagagttggtagctcttgatccggcaaacaaaccaccgctggtagcggtggtttttttgtttgcaagcagcagattacgcgcagaaaaaaaggatctcaagaagatcctttgatcttttctacggggtctgacgctcagtggaacgaaaactcacgttaagggattttggtcatgagattatcaaaaaggatcttcacctagatccttttaaattaaaaatgaagttttaaatcaatctaaagtatatatgagtaaacttggtctgacagttaccaatgcttaatcagtgaggcacctatctcagcgatctgtctatttcgttcatccatagttgcctgactccccgtcgtgtagataactacgatacgggagggcttaccatctggccccagtgctgcaatgataccgcgagacccacgctcaccggctccagatttatcagcaataaaccagccagccggaagggccgagcgcagaagtggtcctgcaactttatccgcctccatccagtctattaattgttgccgggaagctagagtaagtagttcgccagttaatagtttgcgcaacgttgttgccattgctacaggcatcgtggtgtcacgctcgtcgtttggtatggcttcattcagctccggttcccaacgatcaaggcgagttacatgatcccccatgttgtgcaaaaaagcggttagctccttcggtcctccgatcgttgtcagaagtaagttggccgcagtgttatcactcatggttatggcagcactgcataattctcttactgtcatgccatccgtaagatgcttttctgtgactggtgagtactcaaccaagtcattctgagaatagtgtatgcggcgaccgagttgctcttgcccggcgtcaatacgggataataccgcgccacatagcagaactttaaaagtgctcatcattggaaaacgttcttcggggcgaaaactctcaaggatcttaccgctgttgagatccagttcgatgtaacccactcgtgcacccaactgatcttcagcatcttttactttcaccagcgtttctgggtgagcaaaaacaggaaggcaaaatgccgcaaaaaagggaataagggcgacacggaaatgttgaatactcatactcttcctttttcaatattattgaagcatttatcagggttattgtctcatgagcggatacatatttgaatgtatttagaaaaataaacaaataggggttccgcgcacatttccccgaaaagtgccacctgggtcgacattgattattgactagttattaatagtaatcaattacggggtcattagttcatagcccatatatggagttccgcgttacataacttacggtaaatggcccgcctggctgaccgcccaacgacccccgcccattgacgtcaataatgacgtatgttcccatagtaacgccaatagggactttccattgacgtcaatgggtggagtatttacggtaaactgcccacttggcagtacatcaagtgtatcatatgccaagtacgccccctattgacgtcaatgacggtaaatggcccgcctggcattatgcccagtacatgaccttatgggactttcctacttggcagtacatctacgtattagtcatcgctattaccatggtcgaggtgagccccacgttctgcttcactctccccatctcccccccctccccacccccaattttgtatttatttattttttaattattttgtgcagggcgaggcggagaggtgcggcggcagccaatcagagcggcgcgctccgaaagtttccttttatggcgaggcggcggcggcggcggccctataaaaagcgaagcgcgcggcgggcgggagtcgctgcgcgctgccttcgccccgtgccccgctccgccgccgcctcgcgccgcccgccccggctctgactgaccgcgttactcccacaggtgagcgggcgggacggcccttctcctccgggctgtaattagcgcttggtttaatgacggcttgtttcttttctgtggctgcgtgaaagccttgaggggctccgggagggccctttgtgcggggggagcggctcggggggtgcgtgcgtgtgtgtgtgcgtggggagcgccgcgtgcggctccgcgctgcccggcggctgtgagcgctgcgggcgcggcgcggggctttgtgcgctccgcagtgtgcgcgaggggagcgcggccgggggcggtgccccgcggtgcggggggggctgcgaggggaacaaaggctgcgtgcggggtgtgtgcgtgggggggtgagcagggggtgtgggcgcgtcggtcgggctgcaaccccccctgcacccccctccccgagttgctgagcacggcccggcttcgggtgcggggctccgtacggggcgtggcgcggggctcgccgtgccgggcggggggtggcggcaggtgggggtgccgggcggggcggggccgcctcgggccggggagggctcgggggaggggcgcggcggcccccggagcgccggcggctgtcgaggcgcggcgagccgc

SEQ ID NO: 251 - DNA, 5639 bp, Synthetic construct
  source 1..5639: mol_type = other DNA
ggcgcgccggattcgacattgattattgactagttattaatagtaatcaattacggggtcattagttcatagcccatatatggagttccgcgttacataacttacggtaaatggcccgcctggctgaccgcccaacgacccccgcccattgacgtcaataatgacgtatgttcccatagtaacgccaatagggactttccattgacgtcaatgggtggagtatttacggtaaactgcccacttggcagtacatcaagtgtatcatatgccaagtacgccccctattgacgtcaatgacggtaaatggcccgcctggcattatgcccagtacatgaccttatgggactttcctacttggcagtacatctacgtattagtcatcgctattaccatggtcgaggtgagccccacgttctgcttcactctccccatctcccccccctccccacccccaattttgtatttatttattttttaattattttgtgcagcgatgggggcggggggggggggggggcgcgcgccaggcggggcggggcggggcgaggggcggggcggggcgaggcggagaggtgcggcggcagccaatcagagcggcgcgctccgaaagtttccttttatggcgaggcggcggcggcggcggccctataaaaagcgaagcgcgcggcgggcgggagtcgctgcgtcgcgccttcgccccgtgccccgctccgccgccgcctcgcgccgcccgccccggctctgactgaccgcgttactcccacaggtgagcgggcgggacggcccttctcctccgggctgtaattagcgcttggtttaatgacggctcgtttcttttctgtggctgcgtgaaagccttaaagggctccgggagggccctttgtgcgggggggagcggctcggggggtgcgtgcgtgtgtgtgtgcgtggggagcgccgcgtgcggcccgcgctgcccggcggctgtgagcgctgcgggcgcggcgcggggctttgtgcgctccgcgtgtgcgcgaggggagcgcggccgggggcggtgccccgcggtgcgggggggctgcgaggggaacaaaggctgcgtgcggggtgtgtgcgtgggggggtgagcagggggtgtgggcgcggcggtcgggctgtaacccccccctgcacccccctccccgagttgctgagcacggcccggcttcgggtgcggggctccgtgcggggcgtggcgcggggctcgccgtgccgggcggggggtggcggcaggtgggggtgccgggcggggcggggccgcctcgggccggggagggctcgggggaggggcgcggcggccccggagcgccggcggctgtcgaggcgcggcgagccgcagccattgccttttatggtaatcgtgcgagagggcgcagggacttcctttgtcccaaatctggcggagccgaaatctgggaggcgccgccgcaccccctctagcgggcgcgggcgaagcggtgcggcgccggcaggaaggaaatgggcggggagggccttcgtgcgtcgccgcgccgccgtccccttctccatctccagcctcggggctgccgcagggggacggctgccttcgggggggacggggcagggcggggttcggcttctggcgtgtgaccggcggctctagagcctctgctaaccatgttcatgccttcttctttttcctacagatccttaattaataatacgactcactataggggccgccaccatggtgagcaagggcgaggagctgttcaccggggtggtgcccatcctggtcgagctggacggcgacgtaaacggccacaagttcagcgtccgcggcgagggcgagggcgatgccaccaacggcaagctgaccctgaagttcatctgcaccaccggcaagctgcccgtgccctggcccaccctcgtgaccaccttaggctacggcgtggcctgcttcgcccgctaccccgaccacatgaagcagcacgacttcttcaagtccgccatgcccgaaggctacgtccaggagcgcaccatctctttcaaggacgacggcacctacaagacccgcgccgaggtgaagttcgagggcgacaccctggtgaaccgcatcgtgctgaagggcatcgacttcaaggaggacggcaacatcctggggcacaagctggagtacaacttcaacagccacaaggtctatatcacggccgacaagcagaagaacggcatcaaggctaacttcaagacccgccacaacgttgaggacggcggcgtgcagctcgccgaccactaccagcagaacacccccatcggcgacggccccgtgctgctgcccgacaaccactacctgagccatcagtccaaactgagcaaagaccccaacgagaagcgcgatcacatggtcctgaaggagagggtgaccgccgccgggattacacatgacatggacgagctgtacaagtagacgcgtgctcgctttcttgctgtccaatttctattaaaggttcctttgttcgcgtggcagagaaaggcgaaagccttgtgaggccatgcagatccactagttctagagctcgctgatcagcctcgactgtgccttctagttgccagccatctgttgtttgcccctcccccgtgccttccttgaccctggaaggtgccactcccactgtcctttcctaataaaatgaggaaattgcatcgcattgtctgagtaggtgtcattctattctggggggtggggtggggcaggacagcaagggggaggattgggaagacaatagcaggcatgctggggatgcggtgggctctatggcttctgaggcggaaagaaccagctggggctcgagatccactagttctagcctcgaggctagagcggccgccactggccgtcgttttacaacgtcgtgactgggaaaaccctggcgttacccaacttaatcgccttgcagcacatccccctttcgccagctggcgtaatagcgaagaggcccgcaccgatcgcccttcccaacagttgcgcagcctgaatggcgaatgggacgcgccctgtagcggcgcattaagcgcggcgggtgtggtggttacgcgcagcgtgaccgctacacttgccagcgccctagcgcccgctcctttcgctttcttcccttcctttctcgccacgttcgccggctttccccgtcaagctctaaatcgggggctccctttagggttccgatttagtgctttacggcacctcgaccccaaaaaacttgattagggtgatggttcacgtagtgggccatcgccctgatagacggtttttcgccctttgacgttggagtccacgttctttaatagtggactcttgttccaaactggaacaacactcaaccctatctcggtctattcttttgatttataagggattttgccgatttcggcctattggttaaaaaatgagctgatttaacaaaaatttaacgcgaattttaacaaaatattaacgcttacaatttaggtggcacttttcggggaaatgtgcgcggaacccctatttgtttatttttctaaatacattcaaatatgtatccgctcatgagacaataaccctgataaatgcttcaataatattgaaaaaggaagagtatgagtattcaacatttccgtgtcgcccttattcccttttttgcggcattttgccttcctgtttttgctcacccagaaacgctggtgaaagtaaaagatgctgaagatcagttgggtgcacgagtgggttacatcgaactggatctcaacagcggtaagatccttgagagttttcgccccgaagaacgttttccaatgatgagcacttttaaagttctgctatgtggcgcggtattatcccgtattgacgccgggcaagagcaactcggtcgccgcatacactattctcagaatgacttggttgagtactcaccagtcacagaaaagcatcttacggatggcatgacagtaagagaattatgcagtgctgccataaccatgagtgataacactgcggccaacttacttctgacaacgatcggaggaccgaaggagctaaccgcttttttgcacaacatgggggatcatgtaactcgccttgatcgttgggaaccggagctgaatgaagccataccaaacgacgagcgtgacaccacgatgcctgtagcaatggcaacaacgttgcgcaaactattaactggcgaactacttactctagcttcccggcaacaattaatagactggatggaggcggataaagttgcaggaccacttctgcgctcggcccttccggctggctggtttattgctgataaatctggagccggtgagcgtgggtctcgcggtatcattgcagcactggggccagatggtaagccctcccgtatcgtagttatctacacgacggggagtcaggcaactatggatgaacgaaatagacagatcgctgagataggtgcctcactgattaagcattggtaactgtcagaccaagtttactcatatatactttagattgatttaaaacttcatttttaatttaaaaggatctaggtgaagatcctttttgataatctcatgaccaaaatcccttaacgtgagttttcgttccactgagcgtcagaccccgtagaaaagatcaaaggatcttcttgagatcctttttttctgcgcgtaatctgctgcttgcaaacaaaaaaaccaccgctaccagcggtggtttgtttgccggatcaagagctaccaactctttttccgaaggtaactggcttcagcagagcgcagataccaaatactgtccttctagtgtagccgtagttaggccaccacttcaagaactctgtagcaccgcctacatacctcgctctgctaatcctgttaccagtggctgctgccagtggcgataagtcgtgtcttaccgggttggactcaagacgatagttaccggataaggcgcagcggtcgggctgaacggggggttcgtgcacacagcccagcttggagcgaacgacctacaccgaactgagatacctacagcgtgagctatgagaaagcgccacgcttcccgaagggagaaaggcggacaggtatccggtaagcggcagggtcggaacaggagagcgcacgagggagcttccagggggaaacgcctggtatctttatagtcctgtcgggtttcgccacctctgacttgagcgtcgatttttgtgatgctcgtcaggggggcggagcctatggaaaaacgccagcaacgcggcctttttacggttcctggccttttgctggccttttgctcacatgttctttcctgcgttatcccctgattctgtggataaccgtattaccgcctttgagtgagctgataccgctcgccgcagccgaacgaccgagcgcagcgagtcagtgagcgaggaagcggaagagcgcccaatacgcaaaccgcctctccccgcgcgttggccgattcattaatgcagctggcacgacaggtttcccgactggaaagcgggcagtgagcgcaacgcaattaatgtgagttagctcactcattaggcaccccaggctttacactttatgcttccggctcgtatgttgtgtggaattgtgagcggataacaatttcacacaggaaacagctatgaccatga

SEQ ID NO: 252 - DNA, 6245 bp, Synthetic construct
  source 1..6245: mol_type = other DNA
ggcgcgccggattcgacattgattattgactagttattaatagtaatcaattacggggtcattagttcatagcccatatatggagttccgcgttacataacttacggtaaatggcccgcctggctgaccgcccaacgacccccgcccattgacgtcaataatgacgtatgttcccatagtaacgccaatagggactttccattgacgtcaatgggtggagtatttacggtaaactgcccacttggcagtacatcaagtgtatcatatgccaagtacgccccctattgacgtcaatgacggtaaatggcccgcctggcattatgcccagtacatgaccttatgggactttcctacttggcagtacatctacgtattagtcatcgctattaccatggtcgaggtgagccccacgttctgcttcactctccccatctcccccccctccccacccccaattttgtatttatttattttttaattattttgtgcagcgatgggggcggggggggggggggggcgcgcgccaggcggggcggggcggggcgaggggcggggcggggcgaggcggagaggtgcggcggcagccaatcagagcggcgcgctccgaaagtttccttttatggcgaggcggcggcggcggcggccctataaaaagcgaagcgcgcggcgggcgggagtcgctgcgtcgcgccttcgccccgtgccccgctccgccgccgcctcgcgccgcccgccccggctctgactgaccgcgttactcccacaggtgagcgggcgggacggcccttctcctccgggctgtaattagcgcttggtttaatgacggctcgtttcttttctgtggctgcgtgaaagccttaaagggctccgggagggccctttgtgcgggggggagcggctcggggggtgcgtgcgtgtgtgtgtgcgtggggagcgccgcgtgcggcccgcgctgcccggcggctgtgagcgctgcgggcgcggcgcggggctttgtgcgctccgcgtgtgcgcgaggggagcgcggccgggggcggtgccccgcggtgcgggggggctgcgaggggaacaaaggctgcgtgcggggtgtgtgcgtgggggggtgagcagggggtgtgggcgcggcggtcgggctgtaacccccccctgcacccccctccccgagttgctgagcacggcccggcttcgggtgcggggctccgtgcggggcgtggcgcggggctcgccgtgccgggcggggggtggcggcaggtgggggtgccgggcggggcggggccgcctcgggccggggagggctcgggggaggggcgcggcggccccggagcgccggcggctgtcgaggcgcggcgagccgcagccattgccttttatggtaatcgtgcgagagggcgcagggacttcctttgtcccaaatctggcggagccgaaatctgggaggcgccgccgcaccccctctagcgggcgcgggcgaagcggtgcggcgccggcaggaaggaaatgggcggggagggccttcgtgcgtcgccgcgccgccgtccccttctccatctccagcctcggggctgccgcagggggacggctgccttcgggggggacggggcagggcggggttcggcttctggcgtgtgaccggcggctctagagcctctgctaaccatgttcatgccttcttctttttcctacagatccttaattaataatacgactcactataggggccgccaccatggccgagggatctgttgctagacagcctgaccttctcacgtgcgacgacgagcccattcatatccctggcgctatccagcctcacggcctgttgcttgctctggccgccgatatgacaatcgtggctggcagcgataacctgcctgagctgacaggactggctatcggcgctctgatcggcaggtaagtatcctttttacagcacaacttaatgagacagatagaaactggtcttgtagaaacagagtagtgtttgaatgaggcttcagtactttacagaatcgttgcctgcacatcttggaaacacttgctgggattacttcgacttcttaacccaacagaaggctcgagaaggtatattgctgttgacagtgagcgttgctgtccaatttctattaaatagtgaagccacagatgtatttaatagaaattggacagcaatgcctactgcctcggacttcaaggggctagaattcgagcaattatcttgtttactaaaactgaataccttgctatctctttgatacatttttacaaagctgaattaaaatggtataaattaaatcacttttcgcctgcttttctgcctggtactaacttctctcccctctcctcttttctttttctgcaggtctgccgccgacgtgttcgacagcgagacacacaacagactgacaatcgccctggctgagcctggtgctgctgtgggagcacctatcacagtgggcttcaccatgagaaaggacgctggcttcatcggcagctggcacagacatgaccagctgatctttctggaactggaacctccacagagagacgtggccgagcctcaggctttcttcagaagaacaaacagcgccatcagaaggctccaggccgccgagacactggaatctgcttgtgctgccgccgctcaagaagtgcggaagatcacaggcttcgaccgcgtgatgatctacagattcgccagcgacttcagcggcagcgtgatcgccgaagatagatgcgccgaggtggaaagcaagctgggcctgcactatcccgccagctttatccctgctcaggccagaaggctgtacacaatcaaccccgtgcggatcatccccgacatcaactacagacccgtgcctgtgacacccgatctgaaccctgttaccggcagacccatcgacctgagcttcgccatcctgagaagcgtgtccccaaaccaccttgagttcatgagaaacatcggcatgcacggcaccatgagcatcagcatcctgaggggcgaaagactgtggggcctgatcgtgtgccaccacagaaccccttactacgtggacctggatggcagacaggcttgcgaactggtggctcaggttctggcttggcagatcggagtgatggaggagtgaacgcgtaaatgattgcagatccactagttctagagctcgctgatcagcctcgactgtgccttctagttgccagccatctgttgtttgcccctcccccgtgccttccttgaccctggaaggtgccactcccactgtcctttcctaataaaatgaggaaattgcatcgcattgtctgagtaggtgtcattctattctggggggtggggtggggcaggacagcaagggggaggattgggaagagaatagcaggcatgctggggatgcggtgggctctatggcttctgaggcggaaagaaccagctggggctcgagatccactagttctagcctcgaggctagagcggccgccactggccgtcgttttacaacgtcgtgactgggaaaaccctggcgttacccaacttaatcgccttgcagcacatccccctttcgccagctggcgtaatagcgaagaggcccgcaccgatcgcccttcccaacagttgcgcagcctgaatggcgaatgggacgcgccctgtagcggcgcattaagcgcggcgggtgtggtggttacgcgcagcgtgaccgctacacttgccagcgccctagcgcccgctcctttcgctttcttcccttcctttctcgccacgttcgccggctttccccgtcaagctctaaatcgggggctccctttagggttccgatttagtgctttacggcacctcgaccccaaaaaacttgattagggtgatggttcacgtagtgggccatcgccctgatagacggtttttcgccctttgacgttggagtccacgttctttaatagtggactcttgttccaaactggaacaacactcaaccctatctcggtctattcttttgatttataagggattttgccgatttcggcctattggttaaaaaatgagctgatttaacaaaaatttaacgcgaattttaacaaaatattaacgcttacaatttaggtggcacttttcggggaaatgtgcgcggaacccctatttgtttatttttctaaatacattcaaatatgtatccgctcatgagacaataaccctgataaatgcttcaataatattgaaaaaggaagagtatgagtattcaacatttccgtgtcgcccttattcccttttttgcggcattttgccttcctgtttttgctcacccagaaacgctggtgaaagtaaaagatgctgaagatcagttgggtgcacgagtgggttacatcgaactggatctcaacagcggtaagatccttgagagttttcgccccgaagaacgttttccaatgatgagcacttttaaagttctgctatgtggcgcggtattatcccgtattgacgccgggcaagagcaactcggtcgccgcatacactattctcagaatgacttggttgagtactcaccagtcacagaaaagcatcttacggatggcatgacagtaagagaattatgcagtgctgccataaccatgagtgataacactgcggccaacttacttctgacaacgatcggaggaccgaaggagctaaccgcttttttgcacaacatgggggatcatgtaactcgccttgatcgttgggaaccggagctgaatgaagccataccaaacgacgagcgtgacaccacgatgcctgtagcaatggcaacaacgttgcgcaaactattaactggcgaactacttactctagcttcccggcaacaattaatagactggatggaggcggataaagttgcaggaccacttctgcgctcggcccttccggctggctggtttattgctgataaatctggagccggtgagcgtgggtctcgcggtatcattgcagcactggggccagatggtaagccctcccgtatcgtagttatctacacgacggggagtcaggcaactatggatgaacgaaatagacagatcgctgagataggtgcctcactgattaagcattggtaactgtcagaccaagtttactcatatatactttagattgatttaaaacttcatttttaatttaaaaggatctaggtgaagatcctttttgataatctcatgaccaaaatcccttaacgtgagttttcgttccactgagcgtcagaccccgtagaaaagatcaaaggatcttcttgagatcctttttttctgcgcgtaatctgctgcttgcaaacaaaaaaaccaccgctaccagcggtggtttgtttgccggatcaagagctaccaactctttttccgaaggtaactggcttcagcagagcgcagataccaaatactgtccttctagtgtagccgtagttaggccaccacttcaagaactctgtagcaccgcctacatacctcgctctgctaatcctgttaccagtggctgctgccagtggcgataagtcgtgtcttaccgggttggactcaagacgatagttaccggataaggcgcagcggtcgggctgaacggggggttcgtgcacacagcccagcttggagcgaacgacctacaccgaactgagatacctacagcgtgagctatgagaaagcgccacgcttcccgaagggagaaaggcggacaggtatccggtaagcggcagggtcggaacaggagagcgcacgagggagcttccagggggaaacgcctggtatctttatagtcctgtcgggtttcgccacctctgacttgagcgtcgatttttgtgatgctcgtcaggggggcggagcctatggaaaaacgccagcaacgcggcctttttacggttcctggccttttgctggccttttgctcacatgttctttcctgcgttatcccctgattctgtggataaccgtattaccgcctttgagtgagctgataccgctcgccgcagccgaacgaccgagcgcagcgagtcagtgagcgaggaagcggaagagcgcccaatacgcaaaccgcctctccccgcgcgttggccgattcattaatgcagctggcacgacaggtttcccgactggaaagcgggcagtgagcgcaacgcaattaatgtgagttagctcactcattaggcaccccaggctttacactttatgcttccggctcgtatgttgtgtggaattgtgagcggataacaatttcacacaggaaacagctatgaccatga

SEQ ID NO: 253 - DNA, 14614 bp, Synthetic construct
  source 1..14614: mol_type = other DNA
atgggtgcgagagcgtcagtattaagcgggggagaattagatcgatgggaaaaaattcggttaaggccagggggaaagaaaaaatataaattaaaacatatagtatgggcaagcagggagctagaacgattcgcagttaatcctggcctgttagaaacatcagaaggctgtagacaaatactgggacagctacaaccatcccttcagacaggatcagaagaacttagatcattatataatacagtagcaaccctctattgtgtgcatcaaaggatagagataaaagacaccaaggaagctttagacaagatagaggaagagcaaaacaaaagtaagaaaaaagcacagcaagcagcagctgacacaggacacagcaatcaggtcagccaaaattaccctatagtgcagaacatccaggggcaaatggtacatcaggccatatcacctagaactttaaatgcatgggtaaaagtagtagaagagaaggctttcagcccagaagtgatacccatgttttcagcattatcagaaggagccaccccacaagatttaaacaccatgctaaacacagtggggggacatcaagcagccatgcaaatgttaaaagagaccatcaatgaggaagctgcagaatgggatagagtgcatccagtgcatgcagggcctattgcaccaggccagatgagagaaccaaggggaagtgacatagcaggaactactagtacccttcaggaacaaataggatggatgacacataatccacctatcccagtaggagaaatctataaaagatggataatcctgggattaaataaaatagtaagaatgtatagccctaccagcattctggacataagacaaggaccaaaggaaccctttagagactatgtagaccgattctataaaactctaagagccgagcaagcttcacaagaggtaaaaaattggatgacagaaaccttgttggtccaaaatgcgaacccagattgtaagactattttaaaagcattgggaccaggagcgacactagaagaaatgatgacagcatgtcagggagtggggggacccggccataaagcaagagttttggctgaagcaatgagccaagtaacaaatccagctaccataatgatacagaaaggcaattttaggaaccaaagaaagactgttaagtgtttcaattgtggcaaagaagggcacatagccaaaaattgcagggcccctaggaaaaagggctgttggaaatgtggaaaggaaggacaccaaatgaaagattgtactgagagacaggctaattttttagggaagatctggccttcccacaagggaaggccagggaattttcttcagagcagaccagagccaacagccccaccagaagagagcttcaggtttggggaagagacaacaactccctctcagaagcaggagccgatagacaaggaactgtatcctttagcttccctcagatcactctttggcagcgacccctcgtcacaataaagataggggggcaattaaaggaagctctattagatacaggagcagatgatacagtattagaagaaatgaatttgccaggaagatggaaaccaaaaatgatagggggaattggaggttttatcaaagtaagacagtatgatcagatactcatagaaatctgcggacataaagctataggtacagtattagtaggacctacacctgtcaacataattggaagaaatctgttgactcagattggctgcactttaaattttcccattagtcctattgagactgtaccagtaaaattaaagccaggaatggatggcccaaaagttaaacaatggccattgacagaagaaaaaataaaagcattagtagaaatttgtacagaaatggaaaaggaaggaaaaatttcaaaaattgggcctgaaaatccatacaatactccagtatttgccataaagaaaaaagacagtactaaatggagaaaattagtagatttcagagaacttaataagagaactcaagatttctgggaagttcaattaggaataccacatcctgcagggttaaaacagaaaaaatcagtaacagtactggatgtgggcgatgcatatttttcagttcccttagataaagacttcaggaagtatactgcatttaccatacctagtataaacaatgagacaccagggattagatatcagtacaatgtgcttccacagggatggaaaggatcaccagcaatattccagtgtagcatgacaaaaatcttagagccttttagaaaacaaaatccagacatagtcatctatcaatacatggatgatttgtatgtaggatctgacttagaaatagggcagcatagaacaaaaatagaggaactgagacaacatctgttgaggtggggatttaccacaccagacaaaaaacatcagaaagaacctccattcctttggatgggttatgaactccatcctgataaatggacagtacagcctatagtgctgccagaaaaggacagctggactgtcaatgacatacagaaattagtgggaaaattgaattgggcaagtcagatttatgcagggattaaagtaaggcaattatgtaaacttcttaggggaaccaaagcactaacagaagtagtaccactaacagaagaagcagagctagaactggcagaaaacagggagattctaaaagaaccggtacatggagtgtattatgacccatcaaaagacttaatagcagaaatacagaagcaggggcaaggccaatggacatatcaaatttatcaagagccatttaaaaatctgaaaacaggaaagtatgcaagaatgaagggtgcccacactaatgatgtgaaacaattaacagaggcagtacaaaaaatagccacagaaagcatagtaatatggggaaagactcctaaatttaaattacccatacaaaaggaaacatgggaagcatggtggacagagtattggcaagccacctggattcctgagtgggagtttgtcaatacccctcccttagtgaagttatggtaccagttagagaaagaacccataataggagcagaaactttctatgtagatggggcagccaatagggaaactaaattaggaaaagcaggatatgtaactgacagaggaagacaaaaagttgtccccctaacggacacaacaaatcagaagactgagttacaagcaattcatctagctttgcaggattcgggattagaagtaaacatagtgacagactcacaatatgcattgggaatcattcaagcacaaccagataagagtgaatcagagttagtcagtcaaataatagagcagttaataaaaaaggaaaaagtctacctggcatgggtaccagcacacaaaggaattggaggaaatgaacaagtagataaattggtcagtgctggaatcaggaaagtactatttttagatggaatagataaggcccaagaagaacatgagaaatatcacagtaattggagagcaatggctagtgattttaacctaccacctgtagtagcaaaagaaatagtagccagctgtgataaatgtcagctaaaaggggaagccatgcatggacaagtagactgtagcccaggaatatggcagctagtttgtacacatttagaaggaaaagttatcttggtagcagttcatgtagccagtggatatatagaagcagaagtaattccagcagagacagggcaagaaacagcatacttcctcttaaaattagcaggaagatggccagtaaaaacagtacatacagacaatggcagcaatttcaccagtactacagttaaggccgcctgttggtgggcggggatcaagcaggaatttggcattccctacaatccccaaagtcaaggagtaatagaatctatgaataaagaattaaagaaaattataggacaggtaagagatcaggctgaacatcttaagacagcagtacaaatggcagtattcatccacaattttaaaagaaaaggggggattggggggtacagtgcaggggaaagaatagtagacataatagcaacagacatacaaactaaagaattacaaaaacaaattacaaaaattcaaaattttcgggtttattacagggacagcagagatccagtttggaaaggaccagcaaagctcctctggaaaggtgaaggggcagtagtaatacaagataatagtgacataaaagtagtgccaagaagaaaagcaaagatcatcagggattatggaaaacagatggcaggtgatgattgtgtggcaagtagacaggatgaggattaacacatggaattctgcaacaactgctgtttatccatttcagaattgggtgtcgacatagcagaataggcgttactcgacagaggagagcaagaaatggagccagtagatcctagactagagccctggaagcatccaggaagtcagcctaaaactgcttgtaccaattgctattgtaaaaagtgttgctttcattgccaagtttgtttcatgacaaaagccttaggcatctcctatggcaggaagaagcggagacagcgacgaagagctcatcagaacagtcagactcatcaagcttctctatcaaagcagtaagtagtacatgtaatgcaacctataatagtagcaatagtagcattagtagtagcaataataatagcaatagttgtgtggtccatagtaatcatagaatataggaaaatggccgctgatcttcagacctggaggaggagatatgagggacaattggagaagtgaattatataaatataaagtagtaaaaattgaaccattaggagtagcacccaccaaggcaaagagaagagtggtgcagagagaaaaaagagcagtgggaataggagctttgttccttgggttcttgggagcagcaggaagcactatgggcgcagcgtcaatgacgctgacggtacaggccagacaattattgtctggtatagtgcagcagcagaacaatttgctgagggctattgaggcgcaacagcatctgttgcaactcacagtctggggcatcaagcagctccaggcaagaatcctggctgtggaaagatacctaaaggatcaacagctcctggggatttggggttgctctggaaaactcatttgcaccactgctgtgccttggaatgctagttggagtaataaatctctggaacagatttggaatcacacgacctggatggagtgggacagagaaattaacaattacacaagcttaatacactccttaattgaagaatcgcaaaaccagcaagaaaagaatgaacaagaattattggaattagataaatgggcaagtttgtggaattggtttaacataacaaattggctgtggtatataaaattattcataatgatagtaggaggcttggtaggtttaagaatagtttttgctgtactttctatagtgaatagagttaggcagggatattcaccattatcgtttcagacccacctcccaaccccgaggggacccgacaggcccgaaggaatagaagaagaaggtggagagagagacagagacagatccattcgattagtgaacggatccttggcacttatctgggacgatctgcggagcctgtgcctcttcagctaccaccgcttgagagacttactcttgattgtaacgaggattgtggaacttctgggacgcagggggtgggaagccctcaaatattggtggaatctcctacaatattggagtcaggagctaaagaatagtgctgttagcttgctcaatgccacagccatagcagtagctgaggggacagatagggttatagaagtagtacaaggagcttgtagagctattcgccacatacctagaagaataagacagggcttggaaaggattttgctataagctcgaaacaaccggtacctctagaactatagctagcagatctttttccctctgccaaaaattatggggacatcatgaagccccttgagcatctgacttctggctaataaaggaaatttattttcattgcaatagtgtgttggaattttttgtgtctctcactcggaaggacatatgggagggcaaatcatttaaaacatcagaatgagtatttggtttagagtttggcaacatatgcccatatgctggctgccatgaacaaaggttggctataaagaggtcatcagtatatgaaacagccccctgctgtccattccttattccatagaaaagccttgacttgaggttagattttttttatattttgttttgtgttatttttttctttaacatccctaaaattttccttacatgttttactagccagatttttcctcctctcctgactactcccagtcatagctgtccctcttctcttatggagatccctcgacctgcagcccaagcttggcgtaatcatggtcatagctgtttcctgtgtgaaattgttatccgctcacaattccacacaacatacgagccggaagcataaagtgtaaagcctggggtgcctaatgagtgagctaactcacattaattgcgttgcgctcactgcccgctttccagtcgggaaacctgtcgtgccagcggatccggcgcgccggattcgacattgattattgactagttattaatagtaatcaattacggggtcattagttcatagcccatatatggagttccgcgttacataacttacggtaaatggcccgcctggctgaccgcccaacgacccccgcccattgacgtcaataatgacgtatgttcccatagtaacgccaatagggactttccattgacgtcaatgggtggagtatttacggtaaactgcccacttggcagtacatcaagtgtatcatatgccaagtacgccccctattgacgtcaatgacggtaaatggcccgcctggcattatgcccagtacatgaccttatgggactttcctacttggcagtacatctacgtattagtcatcgctattaccatggtcgaggtgagccccacgttctgcttcactctccccatctcccccccctccccacccccaattttgtatttatttattttttaattattttgtgcagcgatgggggcggggggggggggggggcgcgcgccaggcggggcggggcggggcgaggggcggggcggggcgaggcggagaggtgcggcggcagccaatcagagcggcgcgctccgaaagtttccttttatggcgaggcggcggcggcggcggccctataaaaagcgaagcgcgcggcgggcgggagtcgctgcgtcgcgccttcgccccgtgccccgctccgccgccgcctcgcgccgcccgccccggctctgactgaccgcgttactcccacaggtgagcgggcgggacggcccttctcctccgggctgtaattagcgcttggtttaatgacggctcgtttcttttctgtggctgcgtgaaagccttaaagggctccgggagggccctttgtgcgggggggagcggctcggggggtgcgtgcgtgtgtgtgtgcgtggggagcgccgcgtgcggcccgcgctgcccggcggctgtgagcgctgcgggcgcggcgcggggctttgtgcgctccgcgtgtgcgcgaggggagcgcggccgggggcggtgccccgcggtgcgggggggctgcgaggggaacaaaggctgcgtgcggggtgtgtgcgtgggggggtgagcagggggtgtgggcgcggcggtcgggctgtaacccccccctgcacccccctccccgagttgctgagcacggcccggcttcgggtgcggggctccgtgcggggcgtggcgcggggctcgccgtgccgggcggggggtggcggcaggtgggggtgccgggcggggcggggccgcctcgggccggggagggctcgggggaggggcgcggcggccccggagcgccggcggctgtcgaggcgcggcgagccgcagccattgccttttatggtaatcgtgcgagagggcgcagggacttcctttgtcccaaatctggcggagccgaaatctgggaggcgccgccgcaccccctctagcgggcgcgggcgaagcggtgcggcgccggcaggaaggaaatgggcggggagggccttcgtgcgtcgccgcgccgccgtccccttctccatctccagcctcggggctgccgcagggggacggctgccttcgggggggacggggcagggcggggttcggcttctggcgtgtgaccggcggctctagagcctctgctaaccatgttcatgccttcttctttttcctacagatccttaattaataatacgactcactataggggccgccaccatgggcgctagagcctctgttctgtctggcggcgaactggacagatgggagaagatcagaagcagacctggcggcaagaagaagtacaagctgaagcacatcgtgtgggccagcagagagctggaaagattcgctgtgaaccccggcctgctggaaacaagcgagggctgtagacagatcctgggccagctccagccatctctccagacaggatctgaggaactgagaagcctgtacaacaccgtggccacactgtactgcgtgcaccagagaatcgagatcaaggacaccaaagaggccctggacaagatcgaggaagaacagaacaagtctaagaagaaggcccagcaggctgccgccgatacaggccactctaatcaggtgtcccagaactaccccatcgtgcagaacatccagggccagatggtgcatcaggctatcagccccagaacactgaacgcctgggtcaaagtggtggaagagaaggctttcagccctgaagtgatccccatgttcagcgccctgtctgagggtgccacacctcaggacctgaacaccatgctgaacacagtcggcggacaccaggccgctatgcagatgctgaaagagacaatcaacgaagaggccgccgagtgggacagagtgcatcctgttcatgctggccctatcgctcccggccagatgagagaacctagaggctctgacattgccggcaccaccagcacactgcaagagcagatcggctggatgacaaacaaccctcctattcctgtgggcgagatctacaagagatggatcatcctgggactgaacaagatcgtgcggatgtacagccccaccagcatcctggacattagacagggccccaaagagcccttcagagactacgtggacagattctacaagaccctgagagccgagcaggccagccaagaagtgaagaactggatgaccgagacactgctggtgcagaacgctaaccccgactgcaagaccatcctgaaggctctgggacctgccgccacactggaagagatgatgacagcctgtcaaggcgtcggaggacctggccataaggctagagttctggccgaggccatgagccaagtgaccaacagcgccacaatcatgatgcagagaggcaacttcagaaaccagcggaagatcgtgaagtccttcaactccggcaaagagggccacaccgcccgcaattctagagcccctagaaagaaaggtggatccggcggcgtttctggatggcggctgttcaagaagatcagcggcggagctagctctaagacaatcgtgctgtctgtgggcgaagccaccagaacactgaccgagatccagagcacagccgacagacagatcttcgaggaaaaagtgggccctctcgtgggcagactgagactgacagcttccctgagacagaacggcgccaagaccgcctacagagtgaacctgaagctggaccaggccgacgtggtggattctggccttcctaaagtgcggtacacccaagtgtggtcccacgacgtgaccatcgtggccaattctaccgaggccagcagaaagagcctgtacgacctgaccaagagcctggtggccacaagccaggtggaagatctggtcgtgaacctggtgcctctcggacgtggcggatccggtggaaccgagagacaggccaacttcctgggcaagatctggcctagctacaagggcagacccggcaacttcctccagagcagaccagagcctaccgctcctcctgaggaatccttcagatccggcgtggaaaccaccacacctccacagaagcaagagcccatcgacaaagagctgtaccctctgaccagcctgagatccctgttcggcaacgaccctagctctcaatgaacgcgtaaatgattgcagatccactagttctagagctcgctgatcagcctcgactgtgccttctagttgccagccatctgttgtttgcccctcccccgtgccttccttgaccctggaaggtgccactcccactgtcctttcctaataaaatgaggaaattgcatcgcattgtctgagtaggtgtcattctattctggggggtggggtggggcaggacagcaagggggaggattgggaagacaatagcaggcatgctggggatgcggtgggctctatggcttctgaggcggaaagaaccagctggggctcgagatccactagttctagcctcgaggctagagcggccgcgcatctcaattagtcagcaaccatagtcccgcccctaactccgcccatcccgcccctaactccgcccagttccgcccattctccgccccatggctgactaattttttttatttatgcagaggccgaggccgcctcggcctctgagctattccagaagtagtgaggaggcttttttggaggcctaggcttttgcaaaaagctaacttgtttattgcagcttataatggttacaaataaagcaatagcatcacaaatttcacaaataaagcatttttttcactgcattctagttgtggtttgtccaaactcatcaatgtatcttatcatgtctggatccgctgcattaatgaatcggccaacgcgcggggagaggcggtttgcgtattgggcgctcttccgcttcctcgctcactgactcgctgcgctcggtcgttcggctgcggcgagcggtatcagctcactcaaaggcggtaatacggttatccacagaatcaggggataacgcaggaaagaacatgtgagcaaaaggccagcaaaaggccaggaaccgtaaaaaggccgcgttgctggcgtttttccataggctccgcccccctgacgagcatcacaaaaatcgacgctcaagtcagaggtggcgaaacccgacaggactataaagataccaggcgtttccccctggaagctccctcgtgcgctctcctgttccgaccctgccgcttaccggatacctgtccgcctttctcccttcgggaagcgtggcgctttctcatagctcacgctgtaggtatctcagttcggtgtaggtcgttcgctccaagctgggctgtgtgcacgaaccccccgttcagcccgaccgctgcgccttatccggtaactatcgtcttgagtccaacccggtaagacacgacttatcgccactggcagcagccactggtaacaggattagcagagcgaggtatgtaggcggtgctacagagttcttgaagtggtggcctaactacggctacactagaagaacagtatttggtatctgcgctctgctgaagccagttaccttcggaaaaagagttggtagctcttgatccggcaaacaaaccaccgctggtagcggtggtttttttgtttgcaagcagcagattacgcgcagaaaaaaaggatctcaagaagatcctttgatcttttctacggggtctgacgctcagtggaacgaaaactcacgttaagggattttggtcatgagattatcaaaaaggatcttcacctagatccttttaaattaaaaatgaagttttaaatcaatctaaagtatatatgagtaaacttggtctgacagttaccaatgcttaatcagtgaggcacctatctcagcgatctgtctatttcgttcatccatagttgcctgactccccgtcgtgtagataactacgatacgggagggcttaccatctggccccagtgctgcaatgataccgcgagacccacgctcaccggctccagatttatcagcaataaaccagccagccggaagggccgagcgcagaagtggtcctgcaactttatccgcctccatccagtctattaattgttgccgggaagctagagtaagtagttcgccagttaatagtttgcgcaacgttgttgccattgctacaggcatcgtggtgtcacgctcgtcgtttggtatggcttcattcagctccggttcccaacgatcaaggcgagttacatgatcccccatgttgtgcaaaaaagcggttagctccttcggtcctccgatcgttgtcagaagtaagttggccgcagtgttatcactcatggttatggcagcactgcataattctcttactgtcatgccatccgtaagatgcttttctgtgactggtgagtactcaaccaagtcattctgagaatagtgtatgcggcgaccgagttgctcttgcccggcgtcaatacgggataataccgcgccacatagcagaactttaaaagtgctcatcattggaaaacgttcttcggggcgaaaactctcaaggatcttaccgctgttgagatccagttcgatgtaacccactcgtgcacccaactgatcttcagcatcttttactttcaccagcgtttctgggtgagcaaaaacaggaaggcaaaatgccgcaaaaaagggaataagggcgacacggaaatgttgaatactcatactcttcctttttcaatattattgaagcatttatcagggttattgtctcatgagcggatacatatttgaatgtatttagaaaaataaacaaataggggttccgcgcacatttccccgaaaagtgccacctgggtcgacattgattattgactagttattaatagtaatcaattacggggtcattagttcatagcccatatatggagttccgcgttacataacttacggtaaatggcccgcctggctgaccgcccaacgacccccgcccattgacgtcaataatgacgtatgttcccatagtaacgccaatagggactttccattgacgtcaatgggtggagtatttacggtaaactgcccacttggcagtacatcaagtgtatcatatgccaagtacgccccctattgacgtcaatgacggtaaatggcccgcctggcattatgcccagtacatgaccttatgggactttcctacttggcagtacatctacgtattagtcatcgctattaccatggtcgaggtgagccccacgttctgcttcactctccccatctcccccccctccccacccccaattttgtatttatttattttttaattattttgtgcagggcgaggcggagaggtgcggcggcagccaatcagagcggcgcgctccgaaagtttccttttatggcgaggcggcggcggcggcggccctataaaaagcgaagcgcgcggcgggcgggagtcgctgcgcgctgccttcgccccgtgccccgctccgccgccgcctcgcgccgcccgccccggctctgactgaccgcgttactcccacaggtgagcgggcgggacggcccttctcctccgggctgtaattagcgcttggtttaatgacggcttgtttcttttctgtggctgcgtgaaagccttgaggggctccgggagggccctttgtgcggggggagcggctcggggggtgcgtgcgtgtgtgtgtgcgtggggagcgccgcgtgcggctccgcgctgcccggcggctgtgagcgctgcgggcgcggcgcggggctttgtgcgctccgcagtgtgcgcgaggggagcgcggccgggggcggtgccccgcggtgcggggggggctgcgaggggaacaaaggctgcgtgcggggtgtgtgcgtgggggggtgagcagggggtgtgggcgcgtcggtcgggctgcaaccccccctgcacccccctccccgagttgctgagcacggcccggcttcgggtgcggggctccgtacggggcgtggcgcggggctcgccgtgccgggcggggggtggcggcaggtgggggtgccgggcggggcggggccgcctcgggccggggagggctcgggggaggggcgcggcggcccccggagcgccggcggctgtcgaggcgcggcgagccgcagccattgccttttatggtaatcgtgcgagagggcgcagggacttcctttgtcccaaatctgtgcggagccgaaatctgggaggcgccgccgcaccccctctagcgggcgcggggcgaagcggtgcggcgccggcaggaaggaaatgggcggggagggccttcgtgcgtcgccgcgccgccgtccccttctccctctccagcctcggggctgtccgcggggggacggctgccttcgggggggacggggcagggcggggttcggcttctggcgtgtgaccggcggctctagagcctctgctaaccatgttcatgccttcttctttttcctacagctcctgggcaacgtgctggttattgtgctgtctcatcattttggcaaagaattcgggccgcgttgacgcgcacggcaagaggcgaggggcggcgactggtgagag

SEQ ID NO: 254 - DNA, 3415 bp, Synthetic construct
  source 1..3415: mol_type = other DNA
ataaaacctgcaggcatgcaagcgatcgcggggccgcccccttcaccgagggcctatttcccatgattccttcatatttgcatatacgatacaaggctgttagagagataattggaattaatttgactgtaaacacaaagatattagtacaaaatacgtgacgtagaaagtaataatttcttgggtagtttgcagttttaaaattatgttttaaaatggactatcatatgcttaccgtaacttgaaagtatttcgatttcttggctttatatatcttgtggaaaggacgaaacaccgggcgaagcaggccacgccggtttcagagccaccagaagatatggcttcggtggcaagttgaaataaggctagtccgttatcaacttgaaaaagtggcaccgagtcggtgctgtgaccaccttaggctacggcgtggcctgcttccgcggttctatctagttacgcgttaaaccaactagaattttttactagttctagagcggccccaattcgccctatagtgagtcgtattacgcgcgctcactggccgtcgttttacaacgtcgtgactgggaaaaccctggcgttacccaacttaatcgccttgcagcacatccccctttcgccagctggcgtaatagcgaagaggcccgcaccgatcgcccttcccaacagttgcgcagcctgaatggcgaatgggacgcgccctgtagcggcgcattaagcgcggcgggtgtggtggttacgcgcagcgtgaccgctacacttgccagcgccctagcgcccgctcctttcgctttcttcccttcctttctcgccacgttcgccggctttccccgtcaagctctaaatcgggggctccctttagggttccgatttagtgctttacggcacctcgaccccaaaaaacttgattagggtgatggttcacgtagtgggccatcgccctgatagacggtttttcgccctttgacgttggagtccacgttctttaatagtggactcttgttccaaactggaacaacactcaaccctatctcggtctattcttttgatttataagggattttgccgatttcggcctattggttaaaaaatgagctgatttaacaaaaatttaacgcgaattttaacaaaatattaacgcttacaatttaggtggcacttttcggggaaatgtgcgcggaacccctatttgtttatttttctaaatacattcaaatatgtatccgctcatgagacaataaccctgataaatgcttcaataatattgaaaaaggaagagtatgagtattcaacatttccgtgtcgcccttattcccttttttgcggcattttgccttcctgtttttgctcacccagaaacgctggtgaaagtaaaagatgctgaagatcagttgggtgcacgagtgggttacatcgaactggatctcaacagcggtaagatccttgagagttttcgccccgaagaacgttttccaatgatgagcacttttaaagttctgctatgtggcgcggtattatcccgtattgacgccgggcaagagcaactcggtcgccgcatacactattctcagaatgacttggttgagtactcaccagtcacagaaaagcatcttacggatggcatgacagtaagagaattatgcagtgctgccataaccatgagtgataacactgcggccaacttacttctgacaacgatcggaggaccgaaggagctaaccgcttttttgcacaacatgggggatcatgtaactcgccttgatcgttgggaaccggagctgaatgaagccataccaaacgacgagcgtgacaccacgatgcctgtagcaatggcaacaacgttgcgcaaactattaactggcgaactacttactctagcttcccggcaacaattaatagactggatggaggcggataaagttgcaggaccacttctgcgctcggcccttccggctggctggtttattgctgataaatctggagccggtgagcgtgggtctcgcggtatcattgcagcactggggccagatggtaagccctcccgtatcgtagttatctacacgacggggagtcaggcaactatggatgaacgaaatagacagatcgctgagataggtgcctcactgattaagcattggtaactgtcagaccaagtttactcatatatactttagattgatttaaaacttcatttttaatttaaaaggatctaggtgaagatcctttttgataatctcatgaccaaaatcccttaacgtgagttttcgttccactgagcgtcagaccccgtagaaaagatcaaaggatcttcttgagatcctttttttctgcgcgtaatctgctgcttgcaaacaaaaaaaccaccgctaccagcggtggtttgtttgccggatcaagagctaccaactctttttccgaaggtaactggcttcagcagagcgcagataccaaatactgtccttctagtgtagccgtagttaggccaccacttcaagaactctgtagcaccgcctacatacctcgctctgctaatcctgttaccagtggctgctgccagtggcgataagtcgtgtcttaccgggttggactcaagacgatagttaccggataaggcgcagcggtcgggctgaacggggggttcgtgcacacagcccagcttggagcgaacgacctacaccgaactgagatacctacagcgtgagctatgagaaagcgccacgcttcccgaagggagaaaggcggacaggtatccggtaagcggcagggtcggaacaggagagcgcacgagggagcttccagggggaaacgcctggtatctttatagtcctgtcgggtttcgccacctctgacttgagcgtcgatttttgtgatgctcgtcaggggggcggagcctatggaaaaacgccagcaacgcggcctttttacggttcctggccttttgctggccttttgctcacatgttctttcctgcgttatcccctgattctgtggataaccgtattaccgcctttgagtgagctgataccgctcgccgcagccgaacgaccgagcgcagcgagtcagtgagcgaggaagcggaagagcgcccaatacgcaaaccgcctctccccgcgcgttggccgattcattaatgcagctggcacgacaggtttcccgactggaaagcgggcagtgagcgcaacgcaattaatgtgagttagctcactcattaggcaccccaggctttacactttatgcttccggctcgtatgttgtgtggaattgtgagcggataacaatttcacacaggaaacagctatgaccatgattacgccaagcgcgcaattaaccctcactaaagggaacaaaagctggaaacatgcatgaagttcctattccgaagttcctattctctagaaagtataggaacttc

SEQ ID NO: 255 - DNA, 11257 bp, Synthetic construct
  source 1..11257: mol_type = other DNA
ggcgcgccggattcgacattgattattgactagttattaatagtaatcaattacggggtcattagttcatagcccatatatggagttccgcgttacataacttacggtaaatggcccgcctggctgaccgcccaacgacccccgcccattgacgtcaataatgacgtatgttcccatagtaacgccaatagggactttccattgacgtcaatgggtggagtatttacggtaaactgcccacttggcagtacatcaagtgtatcatatgccaagtacgccccctattgacgtcaatgacggtaaatggcccgcctggcattatgcccagtacatgaccttatgggactttcctacttggcagtacatctacgtattagtcatcgctattaccatggtcgaggtgagccccacgttctgcttcactctccccatctcccccccctccccacccccaattttgtatttatttattttttaattattttgtgcagcgatgggggcggggggggggggggggcgcgcgccaggcggggcggggcggggcgaggggcggggcggggcgaggcggagaggtgcggcggcagccaatcagagcggcgcgctccgaaagtttccttttatggcgaggcggcggcggcggcggccctataaaaagcgaagcgcgcggcgggcgggagtcgctgcgtcgcgccttcgccccgtgccccgctccgccgccgcctcgcgccgcccgccccggctctgactgaccgcgttactcccacaggtgagcgggcgggacggcccttctcctccgggctgtaattagcgcttggtttaatgacggctcgtttcttttctgtggctgcgtgaaagccttaaagggctccgggagggccctttgtgcgggggggagcggctcggggggtgcgtgcgtgtgtgtgtgcgtggggagcgccgcgtgcggcccgcgctgcccggcggctgtgagcgctgcgggcgcggcgcggggctttgtgcgctccgcgtgtgcgcgaggggagcgcggccgggggcggtgccccgcggtgcgggggggctgcgaggggaacaaaggctgcgtgcggggtgtgtgcgtgggggggtgagcagggggtgtgggcgcggcggtcgggctgtaacccccccctgcacccccctccccgagttgctgagcacggcccggcttcgggtgcggggctccgtgcggggcgtggcgcggggctcgccgtgccgggcggggggtggcggcaggtgggggtgccgggcggggcggggccgcctcgggccggggagggctcgggggaggggcgcggcggccccggagcgccggcggctgtcgaggcgcggcgagccgcagccattgccttttatggtaatcgtgcgagagggcgcagggacttcctttgtcccaaatctggcggagccgaaatctgggaggcgccgccgcaccccctctagcgggcgcgggcgaagcggtgcggcgccggcaggaaggaaatgggcggggagggccttcgtgcgtcgccgcgccgccgtccccttctccatctccagcctcggggctgccgcagggggacggctgccttcgggggggacggggcagggcggggttcggcttctggcgtgtgaccggcggctctagagcctctgctaaccatgttcatgccttcttctttttcctacagatccttaattaataatacgactcactataggggccgccaccatggacaagaagtacagcatcggcctggacatcggcaccaactctgtgggctgggccgtgatcaccgacgagtacaaggtgcccagcaagaaattcaaggtgctgggcaacaccgaccggcacagcatcaagaagaacctgatcggagccctgctgttcgacagcggcgaaacagccgaggccacccggctgaagagaaccgccagaagaagatacaccagacggaagaaccggatctgctatctgcaagagatcttcagcaacgagatggccaaggtggacgacagcttcttccacagactggaagagtccttcctggtggaagaggataagaagcacgagcggcaccccatcttcggcaacatcgtggacgaggtggcctaccacgagaagtaccccaccatctaccacctgagaaagaaactggtggacagcaccgacaaggccgacctgcggctgatctatctggccctggcccacatgatcaagttccggggccacttcctgatcgagggcgacctgaaccccgacaacagcgacgtggacaagctgttcatccagctggtgcagacctacaaccagctgttcgaggaaaaccccatcaacgccagcggcgtggacgccaaggccatcctgtctgccagactgagcaagagcagacggctggaaaatctgatcgcccagctgcccggcgagaagaagaatggcctgttcggcaacctgattgccctgagcctgggcctgacccccaacttcaagagcaacttcgacctggccgaggatgccaaactgcagctgagcaaggacacctacgacgacgacctggacaacctgctggcccagatcggcgaccagtacgccgacctgtttctggccgccaagaacctgtccgacgccatcctgctgagcgacatcctgagagtgaacaccgagatcaccaaggcccccctgagcgcctctatgatcaagagatacgacgagcaccaccaggacctgaccctgctgaaagctctcgtgcggcagcagctgcctgagaagtacaaagagattttcttcgaccagagcaagaacggctacgccggctacattgacggcggagccagccaggaagagttctacaagttcatcaagcccatcctggaaaagatggacggcaccgaggaactgctcgtgaagctgaacagagaggacctgctgcggaagcagcggaccttcgacaacggcagcatcccccaccagatccacctgggagagctgcacgccattctgcggcggcaggaagatttttacccattcctgaaggacaaccgggaaaagatcgagaagatcctgaccttccgcatcccctactacgtgggccctctggccaggggaaacagcagattcgcctggatgaccagaaagagcgaggaaaccatcaccccctggaacttcgaggaagtggtggacaagggcgcttccgcccagagcttcatcgagcggatgaccaacttcgataagaacctgcccaacgagaaggtgctgcccaagcacagcctgctgtacgagtacttcaccgtgtataacgagctgaccaaagtgaaatacgtgaccgagggaatgagaaagcccgccttcctgagcggcgagcagaaaaaggccatcgtggacctgctgttcaagaccaaccggaaagtgaccgtgaagcagctgaaagaggactacttcaagaaaatcgagtgcttcgactccgtggaaatctccggcgtggaagatcggttcaacgcctccctgggcacataccacgatctgctgaaaattatcaaggacaaggacttcctggacaatgaggaaaacgaggacattctggaagatatcgtgctgaccctgacactgtttgaggacagagagatgatcgaggaacggctgaaaacctatgcccacctgttcgacgacaaagtgatgaagcagctgaagcggcggagatacaccggctggggcaggctgagccggaagctgatcaacggcatccgggacaagcagtccggcaagacaatcctggatttcctgaagtccgacggcttcgccaacagaaacttcatgcagctgatccacgacgacagcctgacctttaaagaggacatccagaaagcccaggtgtccggccagggcgatagcctgcacgagcacattgccaatctggccggcagccccgccattaagaagggcatcctgcagacagtgaaggtggtggacgagctcgtgaaagtgatgggccggcacaagcccgagaacatcgtgatcgaaatggccagagagaaccagaccacccagaagggacagaagaacagccgcgagagaatgaagcggatcgaagagggcatcaaagagctgggcagccagatcctgaaagaacaccccgtggaaaacacccagctgcagaacgagaagctgtacctgtactacctgcagaatgggcgggatatgtacgtggaccaggaactggacatcaaccggctgtccgactacgatgtggaccatatcgtgcctcagagctttctgaaggacgactccatcgacaacaaggtgctgaccagaagcgacaaggcccggggcaagagcgacaacgtgccctccgaagaggtcgtgaagaagatgaagaactactggcggcagctgctgaacgccaagctgattacccagagaaagttcgacaatctgaccaaggccgagagaggcggcctgagcgaactggataaggccggcttcatcaagagacagctggtggaaacccggcagatcacaaagcacgtggcacagatcctggactcccggatgaacactaagtacgacgagaatgacaagctgatccgggaagtgaaagtgatcaccctgaagtccaagctggtgtccgatttccggaaggatttccagttttacaaagtgcgcgagatcaacaactaccaccacgcccacgacgcctacctgaacgccgtcgtgggaaccgccctgatcaaaaagtaccctaagctggaaagcgagttcgtgtacggcgactacaaggtgtacgacgtgcggaagatgatcgccaagagcgagcaggaaatcggcaaggctaccgccaagtacttcttctacagcaacatcatgaactttttcaagaccgagattaccctggccaacggcgagatccggaagcggcctctgatcgagacaaacggcgaaaccggggagatcgtgtgggataagggccgggattttgccaccgtgcggaaagtgctgagcatgccccaagtgaatatcgtgaaaaagaccgaggtgcagacaggcggcttcagcaaagagtctatcctgcccaagaggaacagcgataagctgatcgccagaaagaaggactgggaccctaagaagtacggcggcttcgacagccccaccgtggcctattctgtgctggtggtggccaaagtggaaaagggcaagtccaagaaactgaagagtgtgaaagagctgctggggatcaccatcatggaaagaagcagcttcgagaagaatcccatcgactttctggaagccaagggctacaaagaagtgaaaaaggacctgatcatcaagctgcctaagtactccctgttcgagctggaaaacggccggaagagaatgctggcctctgccggcgaactgcagaagggaaacgaactggccctgccctccaaatatgtgaacttcctgtacctggccagccactatgagaagctgaagggctcccccgaggataatgagcagaaacagctgtttgtggaacagcacaagcactacctggacgagatcatcgagcagatcagcgagttctccaagagagtgatcctggccgacgctaatctggacaaagtgctgtccgcctacaacaagcaccgggataagcccatcagagagcaggccgagaatatcatccacctgtttaccctgaccaatctgggagcccctgccgccttcaagtactttgacaccaccatcgaccggaagaggtacaccagcaccaaagaggtgctggacgccaccctgatccaccagagcatcaccggcctgtacgagacacggatcgacctgtctcagctgggaggcgacgcctatccctatgacgtgcccgattatgccagcctgggctccggatcccccaagaagaaacgcaaggtggaagatggcgagggcccagccgctaagagagtgaaactggattccggagctgctcctgccgccaagaagaagaaactcgacaccggtggacctggaagcgagcctgctacatctggctctgagacacctggcacctccgagtctgctacacctgaatctggacctggcgctagcaccctgaacatcgaggacgagtaccggctgcacgagacaagcaaagaacccgatgtgtccctgggcagcacctggcttagtgatttccctcaggcctgggccgagacaggcggaatgggacttgctgttagacaggcccctctgatcatccctctgaaggccacaagcacccctgtgtccatcaagcagtaccccatgagccaagaggcccggctgggaatcaagccccacattcagagactgctggaccagggcatcctggtgccttgtcagagcccttggaatacccctctgctgcccgtgaagaagcccggcaccaacgattacagacccgtgcaggacctgcgggaagtgaacaagagagtggaagatattcaccccaccgtgccgaatccttacaacctgctgtctggcctgcctcctagccaccagtggtacacagtgctggacctgaaggacgccttcttctgtctgcggctgcaccctacaagccagcctctgtttgcctttgagtggcgggaccctgagatgggcattagcggacagctgacctggaccagactgccccagggcttcaagaacagccccacactgttcaacgaggccctgcatagggacctcgccgacttcagaatccagcatcctgacctgatcctgctccagtacgtggacgatctgctgctggccgctacaagcgagctggattgtcagcagggaacaagagccctgctgcaaaccctgggcaacctgggctatagagcctctgccaagaaggcccagatttgccagaaacaagtgaagtatctgggctacctgctgaaagagggccagcgttggctgaccgaggccagaaaagaaaccgtgatgggccagcctacacctaagacacccagacagctgagagagttcctgggcaaagccggattctgtcggctgttcatccctggctttgccgagatggctgcccctctgtacccactgacaaagcccggaactctgttcaactggggcccagatcagcagaaggcctaccaagagatcaagcaggctctgctgacagcccctgctctgggactgcctgatctgaccaagcctttcgagctgttcgtggacgagaagcagggctatgccaaaggcgtgctgacacagaagctcggcccttggagaaggcctgtggcctacctgagcaagaaactggaccctgtggctgccggatggcctccttgtctgagaatggtggccgccattgccgtgctgaccaaggatgccggaaagctgacaatgggacagcctctggtcattctggcccctcatgccgtggaagccctcgtgaaacagcctcctgatcggtggctgagcaacgccaggatgacacactatcaggcactgctgctcgacaccgacagagtgcagtttggacctgtggtggccctgaatcctgccacacttctgcctctgcctgaggaaggcctccagcacaattgcctggacatcctggccgaggctcacggcacaagacccgatctgacagatcagccactgcctgacgccgaccacacctggtatacagatggcagctctctgctgcaagaaggacagagaaaagccggggctgccgtgaccaccgagacagaagtgatttgggccaaagctctgcccgctggcacatctgctcagagagccgaactgatcgccctgacacaggccctgaaaatggccgagggcaagaagctgaacgtctacaccgactccagatacgccttcgccaccgctcacatccacggcgaaatctatcggcggagaggatggctgaccagcgagggcaaagagattaagaacaaggacgagattctcgccctgctcaaggccctgttcctgcctaagcggctgagcatcatccactgtccaggccaccagaagggccactctgctgaagctagaggcaacagaatggccgaccaggctgccagaaaggccgccatcacagagacacccgataccagcacactgctgatcgagaacagcagccctggtacccctaagaagaagcggaaagtggactgaacgcgtaaatgattgcagatccactagttctagagctcgctgatcagcctcgactgtgccttctagttgccagccatctgttgtttgcccctcccccgtgccttccttgaccctggaaggtgccactcccactgtcctttcctaataaaatgaggaaattgcatcgcattgtctgagtaggtgtcattctattctggggggtggggtggggcaggacagcaagggggaggattgggaagacaatagcaggcatgctggggatgcggtgggctctatggcttctgaggcggaaagaaccagctggggctcgagatccactagttctagcctcgaggctagagcggccgccactggccgtcgttttacaacgtcgtgactgggaaaaccctggcgttacccaacttaatcgccttgcagcacatccccctttcgccagctggcgtaatagcgaagaggcccgcaccgatcgcccttcccaacagttgcgcagcctgaatggcgaatgggacgcgccctgtagcggcgcattaagcgcggcgggtgtggtggttacgcgcagcgtgaccgctacacttgccagcgccctagcgcccgctcctttcgctttcttcccttcctttctcgccacgttcgccggctttccccgtcaagctctaaatcgggggctccctttagggttccgatttagtgctttacggcacctcgaccccaaaaaacttgattagggtgatggttcacgtagtgggccatcgccctgatagacggtttttcgccctttgacgttggagtccacgttctttaatagtggactcttgttccaaactggaacaacactcaaccctatctcggtctattcttttgatttataagggattttgccgatttcggcctattggttaaaaaatgagctgatttaacaaaaatttaacgcgaattttaacaaaatattaacgcttacaatttaggtggcacttttcggggaaatgtgcgcggaacccctatttgtttatttttctaaatacattcaaatatgtatccgctcatgagacaataaccctgataaatgcttcaataatattgaaaaaggaagagtatgagtattcaacatttccgtgtcgcccttattcccttttttgcggcattttgccttcctgtttttgctcacccagaaacgctggtgaaagtaaaagatgctgaagatcagttgggtgcacgagtgggttacatcgaactggatctcaacagcggtaagatccttgagagttttcgccccgaagaacgttttccaatgatgagcacttttaaagttctgctatgtggcgcggtattatcccgtattgacgccgggcaagagcaactcggtcgccgcatacactattctcagaatgacttggttgagtactcaccagtcacagaaaagcatcttacggatggcatgacagtaagagaattatgcagtgctgccataaccatgagtgataacactgcggccaacttacttctgacaacgatcggaggaccgaaggagctaaccgcttttttgcacaacatgggggatcatgtaactcgccttgatcgttgggaaccggagctgaatgaagccataccaaacgacgagcgtgacaccacgatgcctgtagcaatggcaacaacgttgcgcaaactattaactggcgaactacttactctagcttcccggcaacaattaatagactggatggaggcggataaagttgcaggaccacttctgcgctcggcccttccggctggctggtttattgctgataaatctggagccggtgagcgtgggtctcgcggtatcattgcagcactggggccagatggtaagccctcccgtatcgtagttatctacacgacggggagtcaggcaactatggatgaacgaaatagacagatcgctgagataggtgcctcactgattaagcattggtaactgtcagaccaagtttactcatatatactttagattgatttaaaacttcatttttaatttaaaaggatctaggtgaagatcctttttgataatctcatgaccaaaatcccttaacgtgagttttcgttccactgagcgtcagaccccgtagaaaagatcaaaggatcttcttgagatcctttttttctgcgcgtaatctgctgcttgcaaacaaaaaaaccaccgctaccagcggtggtttgtttgccggatcaagagctaccaactctttttccgaaggtaactggcttcagcagagcgcagataccaaatactgtccttctagtgtagccgtagttaggccaccacttcaagaactctgtagcaccgcctacatacctcgctctgctaatcctgttaccagtggctgctgccagtggcgataagtcgtgtcttaccgggttggactcaagacgatagttaccggataaggcgcagcggtcgggctgaacggggggttcgtgcacacagcccagcttggagcgaacgacctacaccgaactgagatacctacagcgtgagctatgagaaagcgccacgcttcccgaagggagaaaggcggacaggtatccggtaagcggcagggtcggaacaggagagcgcacgagggagcttccagggggaaacgcctggtatctttatagtcctgtcgggtttcgccacctctgacttgagcgtcgatttttgtgatgctcgtcaggggggcggagcctatggaaaaacgccagcaacgcggcctttttacggttcctggccttttgctggccttttgctcacatgttctttcctgcgttatcccctgattctgtggataaccgtattaccgcctttgagtgagctgataccgctcgccgcagccgaacgaccgagcgcagcgagtcagtgagcgaggaagcggaagagcgcccaatacgcaaaccgcctctccccgcgcgttggccgattcattaatgcagctggcacgacaggtttcccgactggaaagcgggcagtgagcgcaacgcaattaatgtgagttagctcactcattaggcaccccaggctttacactttatgcttccggctcgtatgttgtgtggaattgtgagcggataacaatttcacacaggaaacagctatgaccatga

SEQ ID NO: 256 - DNA, 11339 bp, Synthetic construct
  source 1..11339: mol_type = other DNA
ggcgcgccggattcgacattgattattgactagttattaatagtaatcaattacggggtcattagttcatagcccatatatggagttccgcgttacataacttacggtaaatggcccgcctggctgaccgcccaacgacccccgcccattgacgtcaataatgacgtatgttcccatagtaacgccaatagggactttccattgacgtcaatgggtggagtatttacggtaaactgcccacttggcagtacatcaagtgtatcatatgccaagtacgccccctattgacgtcaatgacggtaaatggcccgcctggcattatgcccagtacatgaccttatgggactttcctacttggcagtacatctacgtattagtcatcgctattaccatggtcgaggtgagccccacgttctgcttcactctccccatctcccccccctccccacccccaattttgtatttatttattttttaattattttgtgcagcgatgggggcggggggggggggggggcgcgcgccaggcggggcggggcggggcgaggggcggggcggggcgaggcggagaggtgcggcggcagccaatcagagcggcgcgctccgaaagtttccttttatggcgaggcggcggcggcggcggccctataaaaagcgaagcgcgcggcgggcgggagtcgctgcgtcgcgccttcgccccgtgccccgctccgccgccgcctcgcgccgcccgccccggctctgactgaccgcgttactcccacaggtgagcgggcgggacggcccttctcctccgggctgtaattagcgcttggtttaatgacggctcgtttcttttctgtggctgcgtgaaagccttaaagggctccgggagggccctttgtgcgggggggagcggctcggggggtgcgtgcgtgtgtgtgtgcgtggggagcgccgcgtgcggcccgcgctgcccggcggctgtgagcgctgcgggcgcggcgcggggctttgtgcgctccgcgtgtgcgcgaggggagcgcggccgggggcggtgccccgcggtgcgggggggctgcgaggggaacaaaggctgcgtgcggggtgtgtgcgtgggggggtgagcagggggtgtgggcgcggcggtcgggctgtaacccccccctgcacccccctccccgagttgctgagcacggcccggcttcgggtgcggggctccgtgcggggcgtggcgcggggctcgccgtgccgggcggggggtggcggcaggtgggggtgccgggcggggcggggccgcctcgggccggggagggctcgggggaggggcgcggcggccccggagcgccggcggctgtcgaggcgcggcgagccgcagccattgccttttatggtaatcgtgcgagagggcgcagggacttcctttgtcccaaatctggcggagccgaaatctgggaggcgccgccgcaccccctctagcgggcgcgggcgaagcggtgcggcgccggcaggaaggaaatgggcggggagggccttcgtgcgtcgccgcgccgccgtccccttctccatctccagcctcggggctgccgcagggggacggctgccttcgggggggacggggcagggcggggttcggcttctggcgtgtgaccggcggctctagagcctctgctaaccatgttcatgccttcttctttttcctacagatccttaattaataatacgactcactataggggccgccaccatggacaagaagtacagcatcggcctggacatcggcaccaactctgtgggctgggccgtgatcaccgacgagtacaaggtgcccagcaagaaattcaaggtgctgggcaacaccgaccggcacagcatcaagaagaacctgatcggagccctgctgttcgacagcggcgaaacagccgaggccacccggctgaagagaaccgccagaagaagatacaccagacggaagaaccggatctgctatctgcaagagatcttcagcaacgagatggccaaggtggacgacagcttcttccacagactggaagagtccttcctggtggaagaggataagaagcacgagcggcaccccatcttcggcaacatcgtggacgaggtggcctaccacgagaagtaccccaccatctaccacctgagaaagaaactggtggacagcaccgacaaggccgacctgcggctgatctatctggccctggcccacatgatcaagttccggggccacttcctgatcgagggcgacctgaaccccgacaacagcgacgtggacaagctgttcatccagctggtgcagacctacaaccagctgttcgaggaaaaccccatcaacgccagcggcgtggacgccaaggccatcctgtctgccagactgagcaagagcagacggctggaaaatctgatcgcccagctgcccggcgagaagaagaatggcctgttcggcaacctgattgccctgagcctgggcctgacccccaacttcaagagcaacttcgacctggccgaggatgccaaactgcagctgagcaaggacacctacgacgacgacctggacaacctgctggcccagatcggcgaccagtacgccgacctgtttctggccgccaagaacctgtccgacgccatcctgctgagcgacatcctgagagtgaacaccgagatcaccaaggcccccctgagcgcctctatgatcaagagatacgacgagcaccaccaggacctgaccctgctgaaagctctcgtgcggcagcagctgcctgagaagtacaaagagattttcttcgaccagagcaagaacggctacgccggctacattgacggcggagccagccaggaagagttctacaagttcatcaagcccatcctggaaaagatggacggcaccgaggaactgctcgtgaagctgaacagagaggacctgctgcggaagcagcggaccttcgacaacggcagcatcccccaccagatccacctgggagagctgcacgccattctgcggcggcaggaagatttttacccattcctgaaggacaaccgggaaaagatcgagaagatcctgaccttccgcatcccctactacgtgggccctctggccaggggaaacagcagattcgcctggatgaccagaaagagcgaggaaaccatcaccccctggaacttcgaggaagtggtggacaagggcgcttccgcccagagcttcatcgagcggatgaccaacttcgataagaacctgcccaacgagaaggtgctgcccaagcacagcctgctgtacgagtacttcaccgtgtataacgagctgaccaaagtgaaatacgtgaccgagggaatgagaaagcccgccttcctgagcggcgagcagaaaaaggccatcgtggacctgctgttcaagaccaaccggaaagtgaccgtgaagcagctgaaagaggactacttcaagaaaatcgagtgcttcgactccgtggaaatctccggcgtggaagatcggttcaacgcctccctgggcacataccacgatctgctgaaaattatcaaggacaaggacttcctggacaatgaggaaaacgaggacattctggaagatatcgtgctgaccctgacactgtttgaggacagagagatgatcgaggaacggctgaaaacctatgcccacctgttcgacgacaaagtgatgaagcagctgaagcggcggagatacaccggctggggcaggctgagccggaagctgatcaacggcatccgggacaagcagtccggcaagacaatcctggatttcctgaagtccgacggcttcgccaacagaaacttcatgcagctgatccacgacgacagcctgacctttaaagaggacatccagaaagcccaggtgtccggccagggcgatagcctgcacgagcacattgccaatctggccggcagccccgccattaagaagggcatcctgcagacagtgaaggtggtggacgagctcgtgaaagtgatgggccggcacaagcccgagaacatcgtgatcgaaatggccagagagaaccagaccacccagaagggacagaagaacagccgcgagagaatgaagcggatcgaagagggcatcaaagagctgggcagccagatcctgaaagaacaccccgtggaaaacacccagctgcagaacgagaagctgtacctgtactacctgcagaatgggcgggatatgtacgtggaccaggaactggacatcaaccggctgtccgactacgatgtggaccatatcgtgcctcagagctttctgaaggacgactccatcgacaacaaggtgctgaccagaagcgacaaggcccggggcaagagcgacaacgtgccctccgaagaggtcgtgaagaagatgaagaactactggcggcagctgctgaacgccaagctgattacccagagaaagttcgacaatctgaccaaggccgagagaggcggcctgagcgaactggataaggccggcttcatcaagagacagctggtggaaacccggcagatcacaaagcacgtggcacagatcctggactcccggatgaacactaagtacgacgagaatgacaagctgatccgggaagtgaaagtgatcaccctgaagtccaagctggtgtccgatttccggaaggatttccagttttacaaagtgcgcgagatcaacaactaccaccacgcccacgacgcctacctgaacgccgtcgtgggaaccgccctgatcaaaaagtaccctaagctggaaagcgagttcgtgtacggcgactacaaggtgtacgacgtgcggaagatgatcgccaagagcgagcaggaaatcggcaaggctaccgccaagtacttcttctacagcaacatcatgaactttttcaagaccgagattaccctggccaacggcgagatccggaagcggcctctgatcgagacaaacggcgaaaccggggagatcgtgtgggataagggccgggattttgccaccgtgcggaaagtgctgagcatgccccaagtgaatatcgtgaaaaagaccgaggtgcagacaggcggcttcagcaaagagtctatcctgcccaagaggaacagcgataagctgatcgccagaaagaaggactgggaccctaagaagtacggcggcttcgacagccccaccgtggcctattctgtgctggtggtggccaaagtggaaaagggcaagtccaagaaactgaagagtgtgaaagagctgctggggatcaccatcatggaaagaagcagcttcgagaagaatcccatcgactttctggaagccaagggctacaaagaagtgaaaaaggacctgatcatcaagctgcctaagtactccctgttcgagctggaaaacggccggaagagaatgctggcctctgccggcgaactgcagaagggaaacgaactggccctgccctccaaatatgtgaacttcctgtacctggccagccactatgagaagctgaagggctcccccgaggataatgagcagaaacagctgtttgtggaacagcacaagcactacctggacgagatcatcgagcagatcagcgagttctccaagagagtgatcctggccgacgctaatctggacaaagtgctgtccgcctacaacaagcaccgggataagcccatcagagagcaggccgagaatatcatccacctgtttaccctgaccaatctgggagcccctgccgccttcaagtactttgacaccaccatcgaccggaagaggtacaccagcaccaaagaggtgctggacgccaccctgatccaccagagcatcaccggcctgtacgagacacggatcgacctgtctcagctgggaggcgacgcctatccctatgacgtgcccgattatgccagcctgggctccggatcccccaagaagaaacgcaaggtggaagatggcgagggcccagccgctaagagagtgaaactggattccggagctgctcctgccgccaagaagaagaaactcgacaccggtggacctggaagcgagcctgctacatctggctctgagacacctggcacctccgagtctgctacacctgaatctggacctggcgctagcaccctgaacatcgaggacgagtaccggctgcacgagacaagcaaagaacccgatgtgtccctgggcagcacctggcttagtgatttccctcaggcctgggccgagacaggcggaatgggacttgctgttagacaggcccctctgatcatccctctgaaggccacaagcacccctgtgtccatcaagcagtaccccatgagccaagaggcccggctgggaatcaagccccacattcagagactgctggaccagggcatcctggtgccttgtcagagcccttggaatacccctctgctgcccgtgaagaagcccggcaccaacgattacagacccgtgcaggacctgcgggaagtgaacaagagagtggaagatattcaccccaccgtgccgaatccttacaacctgctgtctggcctgcctcctagccaccagtggtacacagtgctggacctgaaggacgccttcttctgtctgcggctgcaccctacaagccagcctctgtttgcctttgagtggcgggaccctgagatgggcattagcggacagctgacctggaccagactgccccagggcttcaagaacagccccacactgttcaacgaggccctgcatagggacctcgccgacttcagaatccagcatcctgacctgatcctgctccagtacgtggacgatctgctgctggccgctacaagcgagctggattgtcagcagggaacaagagccctgctgcaaaccctgggcaacctgggctatagagcctctgccaagaaggcccagatttgccagaaacaagtgaagtatctgggctacctgctgaaagagggccagcgttggctgaccgaggccagaaaagaaaccgtgatgggccagcctacacctaagacacccagacagctgagagagttcctgggcaaagccggattctgtcggctgttcatccctggctttgccgagatggctgcccctctgtacccactgacaaagcccggaactctgttcaactggggcccagatcagcagaaggcctaccaagagatcaagcaggctctgctgacagcccctgctctgggactgcctgatctgaccaagcctttcgagctgttcgtggacgagaagcagggctatgccaaaggcgtgctgacacagaagctcggcccttggagaaggcctgtggcctacctgagcaagaaactggaccctgtggctgccggatggcctccttgtctgagaatggtggccgccattgccgtgctgaccaaggatgccggaaagctgacaatgggacagcctctggtcattctggcccctcatgccgtggaagccctcgtgaaacagcctcctgatcggtggctgagcaacgccaggatgacacactatcaggcactgctgctcgacaccgacagagtgcagtttggacctgtggtggccctgaatcctgccacacttctgcctctgcctgaggaaggcctccagcacaattgcctggacatcctggccgaggctcacggcacaagacccgatctgacagatcagccactgcctgacgccgaccacacctggtatacagatggcagctctctgctgcaagaaggacagagaaaagccggggctgccgtgaccaccgagacagaagtgatttgggccaaagctctgcccgctggcacatctgctcagagagccgaactgatcgccctgacacaggccctgaaaatggccgagggcaagaagctgaacgtctacaccgactccagatacgccttcgccaccgctcacatccacggcgaaatctatcggcggagaggatggctgaccagcgagggcaaagagattaagaacaaggacgagattctcgccctgctcaaggccctgttcctgcctaagcggctgagcatcatccactgtccaggccaccagaagggccactctgctgaagctagaggcaacagaatggccgaccaggctgccagaaaggccgccatcacagagacacccgataccagcacactgctgatcgagaacagcagccctggtacccctaagaagaagcggaaagtggactgaacgcgtgctcgctttcttgctgtccaatttctattaaaggttcctttgttcgcgttgctggaccagaagatatggcttcggttcagcaaaatgattgcagatccactagttctagagctcgctgatcagcctcgactgtgccttctagttgccagccatctgttgtttgcccctcccccgtgccttccttgaccctggaaggtgccactcccactgtcctttcctaataaaatgaggaaattgcatcgcattgtctgagtaggtgtcattctattctggggggtggggtggggcaggacagcaagggggaggattgggaagacaatagcaggcatgctggggatgcggtgggctctatggcttctgaggcggaaagaaccagctggggctcgagatccactagttctagcctcgaggctagagcggccgccactggccgtcgttttacaacgtcgtgactgggaaaaccctggcgttacccaacttaatcgccttgcagcacatccccctttcgccagctggcgtaatagcgaagaggcccgcaccgatcgcccttcccaacagttgcgcagcctgaatggcgaatgggacgcgccctgtagcggcgcattaagcgcggcgggtgtggtggttacgcgcagcgtgaccgctacacttgccagcgccctagcgcccgctcctttcgctttcttcccttcctttctcgccacgttcgccggctttccccgtcaagctctaaatcgggggctccctttagggttccgatttagtgctttacggcacctcgaccccaaaaaacttgattagggtgatggttcacgtagtgggccatcgccctgatagacggtttttcgccctttgacgttggagtccacgttctttaatagtggactcttgttccaaactggaacaacactcaaccctatctcggtctattcttttgatttataagggattttgccgatttcggcctattggttaaaaaatgagctgatttaacaaaaatttaacgcgaattttaacaaaatattaacgcttacaatttaggtggcacttttcggggaaatgtgcgcggaacccctatttgtttatttttctaaatacattcaaatatgtatccgctcatgagacaataaccctgataaatgcttcaataatattgaaaaaggaagagtatgagtattcaacatttccgtgtcgcccttattcccttttttgcggcattttgccttcctgtttttgctcacccagaaacgctggtgaaagtaaaagatgctgaagatcagttgggtgcacgagtgggttacatcgaactggatctcaacagcggtaagatccttgagagttttcgccccgaagaacgttttccaatgatgagcacttttaaagttctgctatgtggcgcggtattatcccgtattgacgccgggcaagagcaactcggtcgccgcatacactattctcagaatgacttggttgagtactcaccagtcacagaaaagcatcttacggatggcatgacagtaagagaattatgcagtgctgccataaccatgagtgataacactgcggccaacttacttctgacaacgatcggaggaccgaaggagctaaccgcttttttgcacaacatgggggatcatgtaactcgccttgatcgttgggaaccggagctgaatgaagccataccaaacgacgagcgtgacaccacgatgcctgtagcaatggcaacaacgttgcgcaaactattaactggcgaactacttactctagcttcccggcaacaattaatagactggatggaggcggataaagttgcaggaccacttctgcgctcggcccttccggctggctggtttattgctgataaatctggagccggtgagcgtgggtctcgcggtatcattgcagcactggggccagatggtaagccctcccgtatcgtagttatctacacgacggggagtcaggcaactatggatgaacgaaatagacagatcgctgagataggtgcctcactgattaagcattggtaactgtcagaccaagtttactcatatatactttagattgatttaaaacttcatttttaatttaaaaggatctaggtgaagatcctttttgataatctcatgaccaaaatcccttaacgtgagttttcgttccactgagcgtcagaccccgtagaaaagatcaaaggatcttcttgagatcctttttttctgcgcgtaatctgctgcttgcaaacaaaaaaaccaccgctaccagcggtggtttgtttgccggatcaagagctaccaactctttttccgaaggtaactggcttcagcagagcgcagataccaaatactgtccttctagtgtagccgtagttaggccaccacttcaagaactctgtagcaccgcctacatacctcgctctgctaatcctgttaccagtggctgctgccagtggcgataagtcgtgtcttaccgggttggactcaagacgatagttaccggataaggcgcagcggtcgggctgaacggggggttcgtgcacacagcccagcttggagcgaacgacctacaccgaactgagatacctacagcgtgagctatgagaaagcgccacgcttcccgaagggagaaaggcggacaggtatccggtaagcggcagggtcggaacaggagagcgcacgagggagcttccagggggaaacgcctggtatctttatagtcctgtcgggtttcgccacctctgacttgagcgtcgatttttgtgatgctcgtcaggggggcggagcctatggaaaaacgccagcaacgcggcctttttacggttcctggccttttgctggccttttgctcacatgttctttcctgcgttatcccctgattctgtggataaccgtattaccgcctttgagtgagctgataccgctcgccgcagccgaacgaccgagcgcagcgagtcagtgagcgaggaagcggaagagcgcccaatacgcaaaccgcctctccccgcgcgttggccgattcattaatgcagctggcacgacaggtttcccgactggaaagcgggcagtgagcgcaacgcaattaatgtgagttagctcactcattaggcaccccaggctttacactttatgcttccggctcgtatgttgtgtggaattgtgagcggataacaatttcacacaggaaacagctatgaccatga

SEQ ID NO: 257 - DNA, 14752 bp, Synthetic construct
  source 1..14752: mol_type = other DNA
aaccttgttggtccaaaatgcgaacccagattgtaagactattttaaaagcattgggaccaggagcgacactagaagaaatgatgacagcatgtcagggagtggggggacccggccataaagcaagagttttggctgaagcaatgagccaagtaacaaatccagctaccataatgatacagaaaggcaattttaggaaccaaagaaagactgttaagtgtttcaattgtggcaaagaagggcacatagccaaaaattgcagggcccctaggaaaaagggctgttggaaatgtggaaaggaaggacaccaaatgaaagattgtactgagagacaggctaattttttagggaagatctggccttcccacaagggaaggccagggaattttcttcagagcagaccagagccaacagccccaccagaagagagcttcaggtttggggaagagacaacaactccctctcagaagcaggagccgatagacaaggaactgtatcctttagcttccctcagatcactctttggcagcgacccctcgtcacaataaagataggggggcaattaaaggaagctctattagatacaggagcagatgatacagtattagaagaaatgaatttgccaggaagatggaaaccaaaaatgatagggggaattggaggttttatcaaagtaagacagtatgatcagatactcatagaaatctgcggacataaagctataggtacagtattagtaggacctacacctgtcaacataattggaagaaatctgttgactcagattggctgcactttaaattttcccattagtcctattgagactgtaccagtaaaattaaagccaggaatggatggcccaaaagttaaacaatggccattgacagaagaaaaaataaaagcattagtagaaatttgtacagaaatggaaaaggaaggaaaaatttcaaaaattgggcctgaaaatccatacaatactccagtatttgccataaagaaaaaagacagtactaaatggagaaaattagtagatttcagagaacttaataagagaactcaagatttctgggaagttcaattaggaataccacatcctgcagggttaaaacagaaaaaatcagtaacagtactggatgtgggcgatgcatatttttcagttcccttagataaagacttcaggaagtatactgcatttaccatacctagtataaacaatgagacaccagggattagatatcagtacaatgtgcttccacagggatggaaaggatcaccagcaatattccagtgtagcatgacaaaaatcttagagccttttagaaaacaaaatccagacatagtcatctatcaatacatggatgatttgtatgtaggatctgacttagaaatagggcagcatagaacaaaaatagaggaactgagacaacatctgttgaggtggggatttaccacaccagacaaaaaacatcagaaagaacctccattcctttggatgggttatgaactccatcctgataaatggacagtacagcctatagtgctgccagaaaaggacagctggactgtcaatgacatacagaaattagtgggaaaattgaattgggcaagtcagatttatgcagggattaaagtaaggcaattatgtaaacttcttaggggaaccaaagcactaacagaagtagtaccactaacagaagaagcagagctagaactggcagaaaacagggagattctaaaagaaccggtacatggagtgtattatgacccatcaaaagacttaatagcagaaatacagaagcaggggcaaggccaatggacatatcaaatttatcaagagccatttaaaaatctgaaaacaggaaagtatgcaagaatgaagggtgcccacactaatgatgtgaaacaattaacagaggcagtacaaaaaatagccacagaaagcatagtaatatggggaaagactcctaaatttaaattacccatacaaaaggaaacatgggaagcatggtggacagagtattggcaagccacctggattcctgagtgggagtttgtcaatacccctcccttagtgaagttatggtaccagttagagaaagaacccataataggagcagaaactttctatgtagatggggcagccaatagggaaactaaattaggaaaagcaggatatgtaactgacagaggaagacaaaaagttgtccccctaacggacacaacaaatcagaagactgagttacaagcaattcatctagctttgcaggattcgggattagaagtaaacatagtgacagactcacaatatgcattgggaatcattcaagcacaaccagataagagtgaatcagagttagtcagtcaaataatagagcagttaataaaaaaggaaaaagtctacctggcatgggtaccagcacacaaaggaattggaggaaatgaacaagtagataaattggtcagtgctggaatcaggaaagtactatttttagatggaatagataaggcccaagaagaacatgagaaatatcacagtaattggagagcaatggctagtgattttaacctaccacctgtagtagcaaaagaaatagtagccagctgtgataaatgtcagctaaaaggggaagccatgcatggacaagtagactgtagcccaggaatatggcagctagtttgtacacatttagaaggaaaagttatcttggtagcagttcatgtagccagtggatatatagaagcagaagtaattccagcagagacagggcaagaaacagcatacttcctcttaaaattagcaggaagatggccagtaaaaacagtacatacagacaatggcagcaatttcaccagtactacagttaaggccgcctgttggtgggcggggatcaagcaggaatttggcattccctacaatccccaaagtcaaggagtaatagaatctatgaataaagaattaaagaaaattataggacaggtaagagatcaggctgaacatcttaagacagcagtacaaatggcagtattcatccacaattttaaaagaaaaggggggattggggggtacagtgcaggggaaagaatagtagacataatagcaacagacatacaaactaaagaattacaaaaacaaattacaaaaattcaaaattttcgggtttattacagggacagcagagatccagtttggaaaggaccagcaaagctcctctggaaaggtgaaggggcagtagtaatacaagataatagtgacataaaagtagtgccaagaagaaaagcaaagatcatcagggattatggaaaacagatggcaggtgatgattgtgtggcaagtagacaggatgaggattaacacatggaattctgcaacaactgctgtttatccatttcagaattgggtgtcgacatagcagaataggcgttactcgacagaggagagcaagaaatggagccagtagatcctagactagagccctggaagcatccaggaagtcagcctaaaactgcttgtaccaattgctattgtaaaaagtgttgctttcattgccaagtttgtttcatgacaaaagccttaggcatctcctatggcaggaagaagcggagacagcgacgaagagctcatcagaacagtcagactcatcaagcttctctatcaaagcagtaagtagtacatgtaatgcaacctataatagtagcaatagtagcattagtagtagcaataataatagcaatagttgtgtggtccatagtaatcatagaatataggaaaatggccgctgatcttcagacctggaggaggagatatgagggacaattggagaagtgaattatataaatataaagtagtaaaaattgaaccattaggagtagcacccaccaaggcaaagagaagagtggtgcagagagaaaaaagagcagtgggaataggagctttgttccttgggttcttgggagcagcaggaagcactatgggcgcagcgtcaatgacgctgacggtacaggccagacaattattgtctggtatagtgcagcagcagaacaatttgctgagggctattgaggcgcaacagcatctgttgcaactcacagtctggggcatcaagcagctccaggcaagaatcctggctgtggaaagatacctaaaggatcaacagctcctggggatttggggttgctctggaaaactcatttgcaccactgctgtgccttggaatgctagttggagtaataaatctctggaacagatttggaatcacacgacctggatggagtgggacagagaaattaacaattacacaagcttaatacactccttaattgaagaatcgcaaaaccagcaagaaaagaatgaacaagaattattggaattagataaatgggcaagtttgtggaattggtttaacataacaaattggctgtggtatataaaattattcataatgatagtaggaggcttggtaggtttaagaatagtttttgctgtactttctatagtgaatagagttaggcagggatattcaccattatcgtttcagacccacctcccaaccccgaggggacccgacaggcccgaaggaatagaagaagaaggtggagagagagacagagacagatccattcgattagtgaacggatccttggcacttatctgggacgatctgcggagcctgtgcctcttcagctaccaccgcttgagagacttactcttgattgtaacgaggattgtggaacttctgggacgcagggggtgggaagccctcaaatattggtggaatctcctacaatattggagtcaggagctaaagaatagtgctgttagcttgctcaatgccacagccatagcagtagctgaggggacagatagggttatagaagtagtacaaggagcttgtagagctattcgccacatacctagaagaataagacagggcttggaaaggattttgctataagctcgaaacaaccggtacctctagaactatagctagcagatctttttccctctgccaaaaattatggggacatcatgaagccccttgagcatctgacttctggctaataaaggaaatttattttcattgcaatagtgtgttggaattttttgtgtctctcactcggaaggacatatgggagggcaaatcatttaaaacatcagaatgagtatttggtttagagtttggcaacatatgcccatatgctggctgccatgaacaaaggttggctataaagaggtcatcagtatatgaaacagccccctgctgtccattccttattccatagaaaagccttgacttgaggttagattttttttatattttgttttgtgttatttttttctttaacatccctaaaattttccttacatgttttactagccagatttttcctcctctcctgactactcccagtcatagctgtccctcttctcttatggagatccctcgacctgcagcccaagcttggcgtaatcatggtcatagctgtttcctgtgtgaaattgttatccgctcacaattccacacaacatacgagccggaagcataaagtgtaaagcctggggtgcctaatgagtgagctaactcacattaattgcgttgcgctcactgcccgctttccagtcgggaaacctgtcgtgccagcggatccggcgcgccggattcgacattgattattgactagttattaatagtaatcaattacggggtcattagttcatagcccatatatggagttccgcgttacataacttacggtaaatggcccgcctggctgaccgcccaacgacccccgcccattgacgtcaataatgacgtatgttcccatagtaacgccaatagggactttccattgacgtcaatgggtggagtatttacggtaaactgcccacttggcagtacatcaagtgtatcatatgccaagtacgccccctattgacgtcaatgacggtaaatggcccgcctggcattatgcccagtacatgaccttatgggactttcctacttggcagtacatctacgtattagtcatcgctattaccatggtcgaggtgagccccacgttctgcttcactctccccatctcccccccctccccacccccaattttgtatttatttattttttaattattttgtgcagcgatgggggcggggggggggggggggcgcgcgccaggcggggcggggcggggcgaggggcggggcggggcgaggcggagaggtgcggcggcagccaatcagagcggcgcgctccgaaagtttccttttatggcgaggcggcggcggcggcggccctataaaaagcgaagcgcgcggcgggcgggagtcgctgcgtcgcgccttcgccccgtgccccgctccgccgccgcctcgcgccgcccgccccggctctgactgaccgcgttactcccacaggtgagcgggcgggacggcccttctcctccgggctgtaattagcgcttggtttaatgacggctcgtttcttttctgtggctgcgtgaaagccttaaagggctccgggagggccctttgtgcgggggggagcggctcggggggtgcgtgcgtgtgtgtgtgcgtggggagcgccgcgtgcggcccgcgctgcccggcggctgtgagcgctgcgggcgcggcgcggggctttgtgcgctccgcgtgtgcgcgaggggagcgcggccgggggcggtgccccgcggtgcgggggggctgcgaggggaacaaaggctgcgtgcggggtgtgtgcgtgggggggtgagcagggggtgtgggcgcggcggtcgggctgtaacccccccctgcacccccctccccgagttgctgagcacggcccggcttcgggtgcggggctccgtgcggggcgtggcgcggggctcgccgtgccgggcggggggtggcggcaggtgggggtgccgggcggggcggggccgcctcgggccggggagggctcgggggaggggcgcggcggccccggagcgccggcggctgtcgaggcgcggcgagccgcagccattgccttttatggtaatcgtgcgagagggcgcagggacttcctttgtcccaaatctggcggagccgaaatctgggaggcgccgccgcaccccctctagcgggcgcgggcgaagcggtgcggcgccggcaggaaggaaatgggcggggagggccttcgtgcgtcgccgcgccgccgtccccttctccatctccagcctcggggctgccgcagggggacggctgccttcgggggggacggggcagggcggggttcggcttctggcgtgtgaccggcggctctagagcctctgctaaccatgttcatgccttcttctttttcctacagatccttaattaataatacgactcactataggggccgccaccatgggcgctagagcctctgttctgtctggcggcgaactggacagatgggagaagatcagaagcagacctggcggcaagaagaagtacaagctgaagcacatcgtgtgggccagcagagagctggaaagattcgctgtgaaccccggcctgctggaaacaagcgagggctgtagacagatcctgggccagctccagccatctctccagacaggatctgaggaactgagaagcctgtacaacaccgtggccacactgtactgcgtgcaccagagaatcgagatcaaggacaccaaagaggccctggacaagatcgaggaagaacagaacaagtctaagaagaaggcccagcaggctgccgccgatacaggccactctaatcaggtgtcccagaactaccccatcgtgcagaacatccagggccagatggtgcatcaggctatcagccccagaacactgaacgcctgggtcaaagtggtggaagagaaggctttcagccctgaagtgatccccatgttcagcgccctgtctgagggtgccacacctcaggacctgaacaccatgctgaacacagtcggcggacaccaggccgctatgcagatgctgaaagagacaatcaacgaagaggccgccgagtgggacagagtgcatcctgttcatgctggccctatcgctcccggccagatgagagaacctagaggctctgacattgccggcaccaccagcacactgcaagagcagatcggctggatgacaaacaaccctcctattcctgtgggcgagatctacaagagatggatcatcctgggactgaacaagatcgtgcggatgtacagccccaccagcatcctggacattagacagggccccaaagagcccttcagagactacgtggacagattctacaagaccctgagagccgagcaggccagccaagaagtgaagaactggatgaccgagacactgctggtgcagaacgctaaccccgactgcaagaccatcctgaaggctctgggacctgccgccacactggaagagatgatgacagcctgtcaaggcgtcggaggacctggccataaggctagagttctggccgaggccatgagccaagtgaccaacagcgccacaatcatgatgcagagaggcaacttcagaaaccagcggaagatcgtgaagtccttcaactccggcaaagagggccacaccgcccgcaattctagagcccctagaaagaaaggtggatccggcggcgtttctggatggcggctgttcaagaagatcagcggcggttccggacctgctgccaaaagagtgaaactggactccggagccccagccgccaagaagaaaaagctggactacaaggacgacgacgacaagggcggagctagctctaagacaatcgtgctgtctgtgggcgaagccaccagaacactgaccgagatccagagcacagccgacagacagatcttcgaggaaaaagtgggccctctcgtgggcagactgagactgacagcttccctgagacagaacggcgccaagaccgcctacagagtgaacctgaagctggaccaggccgacgtggtggattctggccttcctaaagtgcggtacacccaagtgtggtcccacgacgtgaccatcgtggccaattctaccgaggccagcagaaagagcctgtacgacctgaccaagagcctggtggccacaagccaggtggaagatctggtcgtgaacctggtgcctctcggacgtggcggatccggtggaaccgagagacaggccaacttcctgggcaagatctggcctagctacaagggcagacccggcaacttcctccagagcagaccagagcctaccgctcctcctgaggaatccttcagatccggcgtggaaaccaccacacctccacagaagcaagagcccatcgacaaagagctgtaccctctgaccagcctgagatccctgttcggcaacgaccctagctctcaaagcggactgcaactgcctccactggaaagactgacactgggatgaacgcgtaaatgattgcagatccactagttctagagctcgctgatcagcctcgactgtgccttctagttgccagccatctgttgtttgcccctcccccgtgccttccttgaccctggaaggtgccactcccactgtcctttcctaataaaatgaggaaattgcatcgcattgtctgagtaggtgtcattctattctggggggtggggtggggcaggacagcaagggggaggattgggaagacaatagcaggcatgctggggatgcggtgggctctatggcttctgaggcggaaagaaccagctggggctcgagatccactagttctagcctcgaggctagagcggccgcgcatctcaattagtcagcaaccatagtcccgcccctaactccgcccatcccgcccctaactccgcccagttccgcccattctccgccccatggctgactaattttttttatttatgcagaggccgaggccgcctcggcctctgagctattccagaagtagtgaggaggcttttttggaggcctaggcttttgcaaaaagctaacttgtttattgcagcttataatggttacaaataaagcaatagcatcacaaatttcacaaataaagcatttttttcactgcattctagttgtggtttgtccaaactcatcaatgtatcttatcatgtctggatccgctgcattaatgaatcggccaacgcgcggggagaggcggtttgcgtattgggcgctcttccgcttcctcgctcactgactcgctgcgctcggtcgttcggctgcggcgagcggtatcagctcactcaaaggcggtaatacggttatccacagaatcaggggataacgcaggaaagaacatgtgagcaaaaggccagcaaaaggccaggaaccgtaaaaaggccgcgttgctggcgtttttccataggctccgcccccctgacgagcatcacaaaaatcgacgctcaagtcagaggtggcgaaacccgacaggactataaagataccaggcgtttccccctggaagctccctcgtgcgctctcctgttccgaccctgccgcttaccggatacctgtccgcctttctcccttcgggaagcgtggcgctttctcatagctcacgctgtaggtatctcagttcggtgtaggtcgttcgctccaagctgggctgtgtgcacgaaccccccgttcagcccgaccgctgcgccttatccggtaactatcgtcttgagtccaacccggtaagacacgacttatcgccactggcagcagccactggtaacaggattagcagagcgaggtatgtaggcggtgctacagagttcttgaagtggtggcctaactacggctacactagaagaacagtatttggtatctgcgctctgctgaagccagttaccttcggaaaaagagttggtagctcttgatccggcaaacaaaccaccgctggtagcggtggtttttttgtttgcaagcagcagattacgcgcagaaaaaaaggatctcaagaagatcctttgatcttttctacggggtctgacgctcagtggaacgaaaactcacgttaagggattttggtcatgagattatcaaaaaggatcttcacctagatccttttaaattaaaaatgaagttttaaatcaatctaaagtatatatgagtaaacttggtctgacagttaccaatgcttaatcagtgaggcacctatctcagcgatctgtctatttcgttcatccatagttgcctgactccccgtcgtgtagataactacgatacgggagggcttaccatctggccccagtgctgcaatgataccgcgagacccacgctcaccggctccagatttatcagcaataaaccagccagccggaagggccgagcgcagaagtggtcctgcaactttatccgcctccatccagtctattaattgttgccgggaagctagagtaagtagttcgccagttaatagtttgcgcaacgttgttgccattgctacaggcatcgtggtgtcacgctcgtcgtttggtatggcttcattcagctccggttcccaacgatcaaggcgagttacatgatcccccatgttgtgcaaaaaagcggttagctccttcggtcctccgatcgttgtcagaagtaagttggccgcagtgttatcactcatggttatggcagcactgcataattctcttactgtcatgccatccgtaagatgcttttctgtgactggtgagtactcaaccaagtcattctgagaatagtgtatgcggcgaccgagttgctcttgcccggcgtcaatacgggataataccgcgccacatagcagaactttaaaagtgctcatcattggaaaacgttcttcggggcgaaaactctcaaggatcttaccgctgttgagatccagttcgatgtaacccactcgtgcacccaactgatcttcagcatcttttactttcaccagcgtttctgggtgagcaaaaacaggaaggcaaaatgccgcaaaaaagggaataagggcgacacggaaatgttgaatactcatactcttcctttttcaatattattgaagcatttatcagggttattgtctcatgagcggatacatatttgaatgtatttagaaaaataaacaaataggggttccgcgcacatttccccgaaaagtgccacctgggtcgacattgattattgactagttattaatagtaatcaattacggggtcattagttcatagcccatatatggagttccgcgttacataacttacggtaaatggcccgcctggctgaccgcccaacgacccccgcccattgacgtcaataatgacgtatgttcccatagtaacgccaatagggactttccattgacgtcaatgggtggagtatttacggtaaactgcccacttggcagtacatcaagtgtatcatatgccaagtacgccccctattgacgtcaatgacggtaaatggcccgcctggcattatgcccagtacatgaccttatgggactttcctacttggcagtacatctacgtattagtcatcgctattaccatggtcgaggtgagccccacgttctgcttcactctccccatctcccccccctccccacccccaattttgtatttatttattttttaattattttgtgcagggcgaggcggagaggtgcggcggcagccaatcagagcggcgcgctccgaaagtttccttttatggcgaggcggcggcggcggcggccctataaaaagcgaagcgcgcggcgggcgggagtcgctgcgcgctgccttcgccccgtgccccgctccgccgccgcctcgcgccgcccgccccggctctgactgaccgcgttactcccacaggtgagcgggcgggacggcccttctcctccgggctgtaattagcgcttggtttaatgacggcttgtttcttttctgtggctgcgtgaaagccttgaggggctccgggagggccctttgtgcggggggagcggctcggggggtgcgtgcgtgtgtgtgtgcgtggggagcgccgcgtgcggctccgcgctgcccggcggctgtgagcgctgcgggcgcggcgcggggctttgtgcgctccgcagtgtgcgcgaggggagcgcggccgggggcggtgccccgcggtgcggggggggctgcgaggggaacaaaggctgcgtgcggggtgtgtgcgtgggggggtgagcagggggtgtgggcgcgtcggtcgggctgcaaccccccctgcacccccctccccgagttgctgagcacggcccggcttcgggtgcggggctccgtacggggcgtggcgcggggctcgccgtgccgggcggggggtggcggcaggtgggggtgccgggcggggcggggccgcctcgggccggggagggctcgggggaggggcgcggcggcccccggagcgccggcggctgtcgaggcgcggcgagccgcagccattgccttttatggtaatcgtgcgagagggcgcagggacttcctttgtcccaaatctgtgcggagccgaaatctgggaggcgccgccgcaccccctctagcgggcgcggggcgaagcggtgcggcgccggcaggaaggaaatgggcggggagggccttcgtgcgtcgccgcgccgccgtccccttctccctctccagcctcggggctgtccgcggggggacggctgccttcgggggggacggggcagggcggggttcggcttctggcgtgtgaccggcggctctagagcctctgctaaccatgttcatgccttcttctttttcctacagctcctgggcaacgtgctggttattgtgctgtctcatcattttggcaaagaattcgggccgcgttgacgcgcacggcaagaggcgaggggcggcgactggtgagagatgggtgcgagagcgtcagtattaagcgggggagaattagatcgatgggaaaaaattcggttaaggccagggggaaagaaaaaatataaattaaaacatatagtatgggcaagcagggagctagaacgattcgcagttaatcctggcctgttagaaacatcagaaggctgtagacaaatactgggacagctacaaccatcccttcagacaggatcagaagaacttagatcattatataatacagtagcaaccctctattgtgtgcatcaaaggatagagataaaagacaccaaggaagctttagacaagatagaggaagagcaaaacaaaagtaagaaaaaagcacagcaagcagcagctgacacaggacacagcaatcaggtcagccaaaattaccctatagtgcagaacatccaggggcaaatggtacatcaggccatatcacctagaactttaaatgcatgggtaaaagtagtagaagagaaggctttcagcccagaagtgatacccatgttttcagcattatcagaaggagccaccccacaagatttaaacaccatgctaaacacagtggggggacatcaagcagccatgcaaatgttaaaagagaccatcaatgaggaagctgcagaatgggatagagtgcatccagtgcatgcagggcctattgcaccaggccagatgagagaaccaaggggaagtgacatagcaggaactactagtacccttcaggaacaaataggatggatgacacataatccacctatcccagtaggagaaatctataaaagatggataatcctgggattaaataaaatagtaagaatgtatagccctaccagcattctggacataagacaaggaccaaaggaaccctttagagactatgtagaccgattctataaaactctaagagccgagcaagcttcacaagaggtaaaaaattggatgacaga

SEQ ID NO: 258 - DNA, 3410 bp, Synthetic construct
  source 1..3410: mol_type = other DNA
ataaaacctgcaggcatgcaagcgatcgcggggccgcccccttcaccgagggcctatttcccatgattccttcatatttgcatatacgatacaaggctgttagagagataattggaattaatttgactgtaaacacaaagatattagtacaaaatacgtgacgtagaaagtaataatttcttgggtagtttgcagttttaaaattatgttttaaaatggactatcatatgcttaccgtaacttgaaagtatttcgatttcttggctttatatatcttgtggaaaggacgaaacaccgggcgaagcaggccacgccggtttaagagctatgctggaaacagcatagcaagtttaaataaggctagtccgttatcaacttgaaaaagtggcaccgagtcggtgctgtgaccaccttaggctacggcgtggcctgcttccgcggttctatctagttacgcgttaaaccaactagaattttttactagttctagagcggccccaattcgccctatagtgagtcgtattacgcgcgctcactggccgtcgttttacaacgtcgtgactgggaaaaccctggcgttacccaacttaatcgccttgcagcacatccccctttcgccagctggcgtaatagcgaagaggcccgcaccgatcgcccttcccaacagttgcgcagcctgaatggcgaatgggacgcgccctgtagcggcgcattaagcgcggcgggtgtggtggttacgcgcagcgtgaccgctacacttgccagcgccctagcgcccgctcctttcgctttcttcccttcctttctcgccacgttcgccggctttccccgtcaagctctaaatcgggggctccctttagggttccgatttagtgctttacggcacctcgaccccaaaaaacttgattagggtgatggttcacgtagtgggccatcgccctgatagacggtttttcgccctttgacgttggagtccacgttctttaatagtggactcttgttccaaactggaacaacactcaaccctatctcggtctattcttttgatttataagggattttgccgatttcggcctattggttaaaaaatgagctgatttaacaaaaatttaacgcgaattttaacaaaatattaacgcttacaatttaggtggcacttttcggggaaatgtgcgcggaacccctatttgtttatttttctaaatacattcaaatatgtatccgctcatgagacaataaccctgataaatgcttcaataatattgaaaaaggaagagtatgagtattcaacatttccgtgtcgcccttattcccttttttgcggcattttgccttcctgtttttgctcacccagaaacgctggtgaaagtaaaagatgctgaagatcagttgggtgcacgagtgggttacatcgaactggatctcaacagcggtaagatccttgagagttttcgccccgaagaacgttttccaatgatgagcacttttaaagttctgctatgtggcgcggtattatcccgtattgacgccgggcaagagcaactcggtcgccgcatacactattctcagaatgacttggttgagtactcaccagtcacagaaaagcatcttacggatggcatgacagtaagagaattatgcagtgctgccataaccatgagtgataacactgcggccaacttacttctgacaacgatcggaggaccgaaggagctaaccgcttttttgcacaacatgggggatcatgtaactcgccttgatcgttgggaaccggagctgaatgaagccataccaaacgacgagcgtgacaccacgatgcctgtagcaatggcaacaacgttgcgcaaactattaactggcgaactacttactctagcttcccggcaacaattaatagactggatggaggcggataaagttgcaggaccacttctgcgctcggcccttccggctggctggtttattgctgataaatctggagccggtgagcgtgggtctcgcggtatcattgcagcactggggccagatggtaagccctcccgtatcgtagttatctacacgacggggagtcaggcaactatggatgaacgaaatagacagatcgctgagataggtgcctcactgattaagcattggtaactgtcagaccaagtttactcatatatactttagattgatttaaaacttcatttttaatttaaaaggatctaggtgaagatcctttttgataatctcatgaccaaaatcccttaacgtgagttttcgttccactgagcgtcagaccccgtagaaaagatcaaaggatcttcttgagatcctttttttctgcgcgtaatctgctgcttgcaaacaaaaaaaccaccgctaccagcggtggtttgtttgccggatcaagagctaccaactctttttccgaaggtaactggcttcagcagagcgcagataccaaatactgtccttctagtgtagccgtagttaggccaccacttcaagaactctgtagcaccgcctacatacctcgctctgctaatcctgttaccagtggctgctgccagtggcgataagtcgtgtcttaccgggttggactcaagacgatagttaccggataaggcgcagcggtcgggctgaacggggggttcgtgcacacagcccagcttggagcgaacgacctacaccgaactgagatacctacagcgtgagctatgagaaagcgccacgcttcccgaagggagaaaggcggacaggtatccggtaagcggcagggtcggaacaggagagcgcacgagggagcttccagggggaaacgcctggtatctttatagtcctgtcgggtttcgccacctctgacttgagcgtcgatttttgtgatgctcgtcaggggggcggagcctatggaaaaacgccagcaacgcggcctttttacggttcctggccttttgctggccttttgctcacatgttctttcctgcgttatcccctgattctgtggataaccgtattaccgcctttgagtgagctgataccgctcgccgcagccgaacgaccgagcgcagcgagtcagtgagcgaggaagcggaagagcgcccaatacgcaaaccgcctctccccgcgcgttggccgattcattaatgcagctggcacgacaggtttcccgactggaaagcgggcagtgagcgcaacgcaattaatgtgagttagctcactcattaggcaccccaggctttacactttatgcttccggctcgtatgttgtgtggaattgtgagcggataacaatttcacacaggaaacagctatgaccatgattacgccaagcgcgcaattaaccctcactaaagggaacaaaagctggaaacatgcatgaagttcctattccgaagttcctattctctagaaagtataggaacttc

SEQ ID NO: 259 - DNA, 5444 bp, Synthetic construct
  source 1..5444: mol_type = other DNA
ggcgcgccggattcgacattgattattgactagttattaatagtaatcaattacggggtcattagttcatagcccatatatggagttccgcgttacataacttacggtaaatggcccgcctggctgaccgcccaacgacccccgcccattgacgtcaataatgacgtatgttcccatagtaacgccaatagggactttccattgacgtcaatgggtggagtatttacggtaaactgcccacttggcagtacatcaagtgtatcatatgccaagtacgccccctattgacgtcaatgacggtaaatggcccgcctggcattatgcccagtacatgaccttatgggactttcctacttggcagtacatctacgtattagtcatcgctattaccatggtcgaggtgagccccacgttctgcttcactctccccatctcccccccctccccacccccaattttgtatttatttattttttaattattttgtgcagcgatgggggcggggggggggggggggcgcgcgccaggcggggcggggcggggcgaggggcggggcggggcgaggcggagaggtgcggcggcagccaatcagagcggcgcgctccgaaagtttccttttatggcgaggcggcggcggcggcggccctataaaaagcgaagcgcgcggcgggcgggagtcgctgcgtcgcgccttcgccccgtgccccgctccgccgccgcctcgcgccgcccgccccggctctgactgaccgcgttactcccacaggtgagcgggcgggacggcccttctcctccgggctgtaattagcgcttggtttaatgacggctcgtttcttttctgtggctgcgtgaaagccttaaagggctccgggagggccctttgtgcgggggggagcggctcggggggtgcgtgcgtgtgtgtgtgcgtggggagcgccgcgtgcggcccgcgctgcccggcggctgtgagcgctgcgggcgcggcgcggggctttgtgcgctccgcgtgtgcgcgaggggagcgcggccgggggcggtgccccgcggtgcgggggggctgcgaggggaacaaaggctgcgtgcggggtgtgtgcgtgggggggtgagcagggggtgtgggcgcggcggtcgggctgtaacccccccctgcacccccctccccgagttgctgagcacggcccggcttcgggtgcggggctccgtgcggggcgtggcgcggggctcgccgtgccgggcggggggtggcggcaggtgggggtgccgggcggggcggggccgcctcgggccggggagggctcgggggaggggcgcggcggccccggagcgccggcggctgtcgaggcgcggcgagccgcagccattgccttttatggtaatcgtgcgagagggcgcagggacttcctttgtcccaaatctggcggagccgaaatctgggaggcgccgccgcaccccctctagcgggcgcgggcgaagcggtgcggcgccggcaggaaggaaatgggcggggagggccttcgtgcgtcgccgcgccgccgtccccttctccatctccagcctcggggctgccgcagggggacggctgccttcgggggggacggggcagggcggggttcggcttctggcgtgtgaccggcggctctagagcctctgctaaccatgttcatgccttcttctttttcctacagatccttaattaataatacgactcactataggggccgccaccatggtctttacactggaagatttcgtcggcgactggcggcagacagctggctacaatctggaccaggtgctggaacaaggcggcgtgtcctctctgtttcaaaacctgggagtgtctgtgacccctatccagagaatcgtgctgagcggcgagaacggcctgaagatcgacatccacgtgatcatcccttacgagggcctgtccggcgatcagatgggacagatcgagaagatctttaaggtggtgtaccccgtggacgaccaccacttcaaagtgatcctgcactacggcaccctggtcatcgatggcgtgaccccaaacatgatcgactacttcggcagaccctacgagggaatcgccgtgttcgacggcaagaaaatcaccgtgaccggcacactgtggaacggcaacaagatcatcgacgagagactgatcaaccccgacggcagcctgctgttcagagtgacaatcaacggcgtgacaggctggcggctgtgcgaaagaatcctggcctagacgcgtgctcgctttcttgctgtccaatttctattaaaggttcctttgttcgcgttgctggaccagaagatatggcttcggttcagcaaaatgattgcagatccactagttctagagctcgctgatcagcctcgactgtgccttctagttgccagccatctgttgtttgcccctcccccgtgccttccttgaccctggaaggtgccactcccactgtcctttcctaataaaatgaggaaattgcatcgcattgtctgagtaggtgtcattctattctggggggtggggtggggcaggacagcaagggggaggattgggaagacaatagcaggcatgctggggatgcggtgggctctatggcttctgaggcggaaagaaccagctggggctcgagatccactagttctagcctcgaggctagagcggccgccactggccgtcgttttacaacgtcgtgactgggaaaaccctggcgttacccaacttaatcgccttgcagcacatccccctttcgccagctggcgtaatagcgaagaggcccgcaccgatcgcccttcccaacagttgcgcagcctgaatggcgaatgggacgcgccctgtagcggcgcattaagcgcggcgggtgtggtggttacgcgcagcgtgaccgctacacttgccagcgccctagcgcccgctcctttcgctttcttcccttcctttctcgccacgttcgccggctttccccgtcaagctctaaatcgggggctccctttagggttccgatttagtgctttacggcacctcgaccccaaaaaacttgattagggtgatggttcacgtagtgggccatcgccctgatagacggtttttcgccctttgacgttggagtccacgttctttaatagtggactcttgttccaaactggaacaacactcaaccctatctcggtctattcttttgatttataagggattttgccgatttcggcctattggttaaaaaatgagctgatttaacaaaaatttaacgcgaattttaacaaaatattaacgcttacaatttaggtggcacttttcggggaaatgtgcgcggaacccctatttgtttatttttctaaatacattcaaatatgtatccgctcatgagacaataaccctgataaatgcttcaataatattgaaaaaggaagagtatgagtattcaacatttccgtgtcgcccttattcccttttttgcggcattttgccttcctgtttttgctcacccagaaacgctggtgaaagtaaaagatgctgaagatcagttgggtgcacgagtgggttacatcgaactggatctcaacagcggtaagatccttgagagttttcgccccgaagaacgttttccaatgatgagcacttttaaagttctgctatgtggcgcggtattatcccgtattgacgccgggcaagagcaactcggtcgccgcatacactattctcagaatgacttggttgagtactcaccagtcacagaaaagcatcttacggatggcatgacagtaagagaattatgcagtgctgccataaccatgagtgataacactgcggccaacttacttctgacaacgatcggaggaccgaaggagctaaccgcttttttgcacaacatgggggatcatgtaactcgccttgatcgttgggaaccggagctgaatgaagccataccaaacgacgagcgtgacaccacgatgcctgtagcaatggcaacaacgttgcgcaaactattaactggcgaactacttactctagcttcccggcaacaattaatagactggatggaggcggataaagttgcaggaccacttctgcgctcggcccttccggctggctggtttattgctgataaatctggagccggtgagcgtgggtctcgcggtatcattgcagcactggggccagatggtaagccctcccgtatcgtagttatctacacgacggggagtcaggcaactatggatgaacgaaatagacagatcgctgagataggtgcctcactgattaagcattggtaactgtcagaccaagtttactcatatatactttagattgatttaaaacttcatttttaatttaaaaggatctaggtgaagatcctttttgataatctcatgaccaaaatcccttaacgtgagttttcgttccactgagcgtcagaccccgtagaaaagatcaaaggatcttcttgagatcctttttttctgcgcgtaatctgctgcttgcaaacaaaaaaaccaccgctaccagcggtggtttgtttgccggatcaagagctaccaactctttttccgaaggtaactggcttcagcagagcgcagataccaaatactgtccttctagtgtagccgtagttaggccaccacttcaagaactctgtagcaccgcctacatacctcgctctgctaatcctgttaccagtggctgctgccagtggcgataagtcgtgtcttaccgggttggactcaagacgatagttaccggataaggcgcagcggtcgggctgaacggggggttcgtgcacacagcccagcttggagcgaacgacctacaccgaactgagatacctacagcgtgagctatgagaaagcgccacgcttcccgaagggagaaaggcggacaggtatccggtaagcggcagggtcggaacaggagagcgcacgagggagcttccagggggaaacgcctggtatctttatagtcctgtcgggtttcgccacctctgacttgagcgtcgatttttgtgatgctcgtcaggggggcggagcctatggaaaaacgccagcaacgcggcctttttacggttcctggccttttgctggccttttgctcacatgttctttcctgcgttatcccctgattctgtggataaccgtattaccgcctttgagtgagctgataccgctcgccgcagccgaacgaccgagcgcagcgagtcagtgagcgaggaagcggaagagcgcccaatacgcaaaccgcctctccccgcgcgttggccgattcattaatgcagctggcacgacaggtttcccgactggaaagcgggcagtgagcgcaacgcaattaatgtgagttagctcactcattaggcaccccaggctttacactttatgcttccggctcgtatgttgtgtggaattgtgagcggataacaatttcacacaggaaacagctatgaccatga

SEQ ID NO: 260 - DNA, 6877 bp, Synthetic construct
  source 1..6877: mol_type = other DNA
ggcgcgccggattcgacattgattattgactagttattaatagtaatcaattacggggtcattagttcatagcccatatatggagttccgcgttacataacttacggtaaatggcccgcctggctgaccgcccaacgacccccgcccattgacgtcaataatgacgtatgttcccatagtaacgccaatagggactttccattgacgtcaatgggtggagtatttacggtaaactgcccacttggcagtacatcaagtgtatcatatgccaagtacgccccctattgacgtcaatgacggtaaatggcccgcctggcattatgcccagtacatgaccttatgggactttcctacttggcagtacatctacgtattagtcatcgctattaccatggtcgaggtgagccccacgttctgcttcactctccccatctcccccccctccccacccccaattttgtatttatttattttttaattattttgtgcagcgatgggggcggggggggggggggggcgcgcgccaggcggggcggggcggggcgaggggcggggcggggcgaggcggagaggtgcggcggcagccaatcagagcggcgcgctccgaaagtttccttttatggcgaggcggcggcggcggcggccctataaaaagcgaagcgcgcggcgggcgggagtcgctgcgtcgcgccttcgccccgtgccccgctccgccgccgcctcgcgccgcccgccccggctctgactgaccgcgttactcccacaggtgagcgggcgggacggcccttctcctccgggctgtaattagcgcttggtttaatgacggctcgtttcttttctgtggctgcgtgaaagccttaaagggctccgggagggccctttgtgcgggggggagcggctcggggggtgcgtgcgtgtgtgtgtgcgtggggagcgccgcgtgcggcccgcgctgcccggcggctgtgagcgctgcgggcgcggcgcggggctttgtgcgctccgcgtgtgcgcgaggggagcgcggccgggggcggtgccccgcggtgcgggggggctgcgaggggaacaaaggctgcgtgcggggtgtgtgcgtgggggggtgagcagggggtgtgggcgcggcggtcgggctgtaacccccccctgcacccccctccccgagttgctgagcacggcccggcttcgggtgcggggctccgtgcggggcgtggcgcggggctcgccgtgccgggcggggggtggcggcaggtgggggtgccgggcggggcggggccgcctcgggccggggagggctcgggggaggggcgcggcggccccggagcgccggcggctgtcgaggcgcggcgagccgcagccattgccttttatggtaatcgtgcgagagggcgcagggacttcctttgtcccaaatctggcggagccgaaatctgggaggcgccgccgcaccccctctagcgggcgcgggcgaagcggtgcggcgccggcaggaaggaaatgggcggggagggccttcgtgcgtcgccgcgccgccgtccccttctccatctccagcctcggggctgccgcagggggacggctgccttcgggggggacggggcagggcggggttcggcttctggcgtgtgaccggcggctctagagcctctgctaaccatgttcatgccttcttctttttcctacagatccttaattaataatacgactcactataggggccgccaccatgggcgctagagcctctgttctgtctggcggcgaactggacagatgggagaagatcagaagcagacctggcggcaagaagaagtacaagctgaagcacatcgtgtgggccagcagagagctggaaagattcgctgtgaaccccggcctgctggaaacaagcgagggctgtagacagatcctgggccagctccagccatctctccagacaggatctgaggaactgagaagcctgtacaacaccgtggccacactgtactgcgtgcaccagagaatcgagatcaaggacaccaaagaggccctggacaagatcgaggaagaacagaacaagtctaagaagaaggcccagcaggctgccgccgatacaggccactctaatcaggtgtcccagaactaccccatcgtgcagaacatccagggccagatggtgcatcaggctatcagccccagaacactgaacgcctgggtcaaagtggtggaagagaaggctttcagccctgaagtgatccccatgttcagcgccctgtctgagggtgccacacctcaggacctgaacaccatgctgaacacagtcggcggacaccaggccgctatgcagatgctgaaagagacaatcaacgaagaggccgccgagtgggacagagtgcatcctgttcatgctggccctatcgctcccggccagatgagagaacctagaggctctgacattgccggcaccaccagcacactgcaagagcagatcggctggatgacaaacaaccctcctattcctgtgggcgagatctacaagagatggatcatcctgggactgaacaagatcgtgcggatgtacagccccaccagcatcctggacattagacagggccccaaagagcccttcagagactacgtggacagattctacaagaccctgagagccgagcaggccagccaagaagtgaagaactggatgaccgagacactgctggtgcagaacgctaaccccgactgcaagaccatcctgaaggctctgggacctgccgccacactggaagagatgatgacagcctgtcaaggcgtcggaggacctggccataaggctagagttctggccgaggccatgagccaagtgaccaacagcgccacaatcatgatgcagagaggcaacttcagaaaccagcggaagatcgtgaagtccttcaactccggcaaagagggccacaccgcccgcaattctagagcccctagaaagaaaggtggatccggcggcgtttctggatggcggctgttcaagaagatcagcggcggttccggacctgctgccaaaagagtgaaactggactccggactgcaactgcctccactggaaagactgacactgggagctgccccagccgccaagaagaaaaagctggactacaaggacgacgacgacaagggcggagctagctctaagacaatcgtgctgtctgtgggcgaagccaccagaacactgaccgagatccagagcacagccgacagacagatcttcgaggaaaaagtgggccctctcgtgggcagactgagactgacagcttccctgagacagaacggcgccaagaccgcctacagagtgaacctgaagctggaccaggccgacgtggtggattctggccttcctaaagtgcggtacacccaagtgtggtcccacgacgtgaccatcgtggccaattctaccgaggccagcagaaagagcctgtacgacctgaccaagagcctggtggccacaagccaggtggaagatctggtcgtgaacctggtgcctctcggacgtggcggatccggtggaaccgagagacaggccaacttcctgggcaagatctggcctagctacaagggcagacccggcaacttcctccagagcagaccagagcctaccgctcctcctgaggaatccttcagatccggcgtggaaaccaccacacctccacagaagcaagagcccatcgacaaagagctgtaccctctgaccagcctgagatccctgttcggcaacgaccctagctctcaatgaacgcgtaaatgattgcagatccactagttctagagctcgctgatcagcctcgactgtgccttctagttgccagccatctgttgtttgcccctcccccgtgccttccttgaccctggaaggtgccactcccactgtcctttcctaataaaatgaggaaattgcatcgcattgtctgagtaggtgtcattctattctggggggtggggtggggcaggacagcaagggggaggattgggaagacaatagcaggcatgctggggatgcggtgggctctatggcttctgaggcggaaagaaccagctggggctcgagatccactagttctagcctcgaggctagagcggccgccactggccgtcgttttacaacgtcgtgactgggaaaaccctggcgttacccaacttaatcgccttgcagcacatccccctttcgccagctggcgtaatagcgaagaggcccgcaccgatcgcccttcccaacagttgcgcagcctgaatggcgaatgggacgcgccctgtagcggcgcattaagcgcggcgggtgtggtggttacgcgcagcgtgaccgctacacttgccagcgccctagcgcccgctcctttcgctttcttcccttcctttctcgccacgttcgccggctttccccgtcaagctctaaatcgggggctccctttagggttccgatttagtgctttacggcacctcgaccccaaaaaacttgattagggtgatggttcacgtagtgggccatcgccctgatagacggtttttcgccctttgacgttggagtccacgttctttaatagtggactcttgttccaaactggaacaacactcaaccctatctcggtctattcttttgatttataagggattttgccgatttcggcctattggttaaaaaatgagctgatttaacaaaaatttaacgcgaattttaacaaaatattaacgcttacaatttaggtggcacttttcggggaaatgtgcgcggaacccctatttgtttatttttctaaatacattcaaatatgtatccgctcatgagacaataaccctgataaatgcttcaataatattgaaaaaggaagagtatgagtattcaacatttccgtgtcgcccttattcccttttttgcggcattttgccttcctgtttttgctcacccagaaacgctggtgaaagtaaaagatgctgaagatcagttgggtgcacgagtgggttacatcgaactggatctcaacagcggtaagatccttgagagttttcgccccgaagaacgttttccaatgatgagcacttttaaagttctgctatgtggcgcggtattatcccgtattgacgccgggcaagagcaactcggtcgccgcatacactattctcagaatgacttggttgagtactcaccagtcacagaaaagcatcttacggatggcatgacagtaagagaattatgcagtgctgccataaccatgagtgataacactgcggccaacttacttctgacaacgatcggaggaccgaaggagctaaccgcttttttgcacaacatgggggatcatgtaactcgccttgatcgttgggaaccggagctgaatgaagccataccaaacgacgagcgtgacaccacgatgcctgtagcaatggcaacaacgttgcgcaaactattaactggcgaactacttactctagcttcccggcaacaattaatagactggatggaggcggataaagttgcaggaccacttctgcgctcggcccttccggctggctggtttattgctgataaatctggagccggtgagcgtgggtctcgcggtatcattgcagcactggggccagatggtaagccctcccgtatcgtagttatctacacgacggggagtcaggcaactatggatgaacgaaatagacagatcgctgagataggtgcctcactgattaagcattggtaactgtcagaccaagtttactcatatatactttagattgatttaaaacttcatttttaatttaaaaggatctaggtgaagatcctttttgataatctcatgaccaaaatcccttaacgtgagttttcgttccactgagcgtcagaccccgtagaaaagatcaaaggatcttcttgagatcctttttttctgcgcgtaatctgctgcttgcaaacaaaaaaaccaccgctaccagcggtggtttgtttgccggatcaagagctaccaactctttttccgaaggtaactggcttcagcagagcgcagataccaaatactgtccttctagtgtagccgtagttaggccaccacttcaagaactctgtagcaccgcctacatacctcgctctgctaatcctgttaccagtggctgctgccagtggcgataagtcgtgtcttaccgggttggactcaagacgatagttaccggataaggcgcagcggtcgggctgaacggggggttcgtgcacacagcccagcttggagcgaacgacctacaccgaactgagatacctacagcgtgagctatgagaaagcgccacgcttcccgaagggagaaaggcggacaggtatccggtaagcggcagggtcggaacaggagagcgcacgagggagcttccagggggaaacgcctggtatctttatagtcctgtcgggtttcgccacctctgacttgagcgtcgatttttgtgatgctcgtcaggggggcggagcctatggaaaaacgccagcaacgcggcctttttacggttcctggccttttgctggccttttgctcacatgttctttcctgcgttatcccctgattctgtggataaccgtattaccgcctttgagtgagctgataccgctcgccgcagccgaacgaccgagcgcagcgagtcagtgagcgaggaagcggaagagcgcccaatacgcaaaccgcctctccccgcgcgttggccgattcattaatgcagctggcacgacaggtttcccgactggaaagcgggcagtgagcgcaacgcaattaatgtgagttagctcactcattaggcaccccaggctttacactttatgcttccggctcgtatgttgtgtggaattgtgagcggataacaatttcacacaggaaacagctatgaccatga

SEQ ID NO: 261 - DNA, 11345 bp, Synthetic construct
  source 1..11345: mol_type = other DNA
ggcgcgccggattcgacattgattattgactagttattaatagtaatcaattacggggtcattagttcatagcccatatatggagttccgcgttacataacttacggtaaatggcccgcctggctgaccgcccaacgacccccgcccattgacgtcaataatgacgtatgttcccatagtaacgccaatagggactttccattgacgtcaatgggtggagtatttacggtaaactgcccacttggcagtacatcaagtgtatcatatgccaagtacgccccctattgacgtcaatgacggtaaatggcccgcctggcattatgcccagtacatgaccttatgggactttcctacttggcagtacatctacgtattagtcatcgctattaccatggtcgaggtgagccccacgttctgcttcactctccccatctcccccccctccccacccccaattttgtatttatttattttttaattattttgtgcagcgatgggggcggggggggggggggggcgcgcgccaggcggggcggggcggggcgaggggcggggcggggcgaggcggagaggtgcggcggcagccaatcagagcggcgcgctccgaaagtttccttttatggcgaggcggcggcggcggcggccctataaaaagcgaagcgcgcggcgggcgggagtcgctgcgtcgcgccttcgccccgtgccccgctccgccgccgcctcgcgccgcccgccccggctctgactgaccgcgttactcccacaggtgagcgggcgggacggcccttctcctccgggctgtaattagcgcttggtttaatgacggctcgtttcttttctgtggctgcgtgaaagccttaaagggctccgggagggccctttgtgcgggggggagcggctcggggggtgcgtgcgtgtgtgtgtgcgtggggagcgccgcgtgcggcccgcgctgcccggcggctgtgagcgctgcgggcgcggcgcggggctttgtgcgctccgcgtgtgcgcgaggggagcgcggccgggggcggtgccccgcggtgcgggggggctgcgaggggaacaaaggctgcgtgcggggtgtgtgcgtgggggggtgagcagggggtgtgggcgcggcggtcgggctgtaacccccccctgcacccccctccccgagttgctgagcacggcccggcttcgggtgcggggctccgtgcggggcgtggcgcggggctcgccgtgccgggcggggggtggcggcaggtgggggtgccgggcggggcggggccgcctcgggccggggagggctcgggggaggggcgcggcggccccggagcgccggcggctgtcgaggcgcggcgagccgcagccattgccttttatggtaatcgtgcgagagggcgcagggacttcctttgtcccaaatctggcggagccgaaatctgggaggcgccgccgcaccccctctagcgggcgcgggcgaagcggtgcggcgccggcaggaaggaaatgggcggggagggccttcgtgcgtcgccgcgccgccgtccccttctccatctccagcctcggggctgccgcagggggacggctgccttcgggggggacggggcagggcggggttcggcttctggcgtgtgaccggcggctctagagcctctgctaaccatgttcatgccttcttctttttcctacagatccttaattaataatacgactcactataggggccgccaccatgaccctgaacatcgaggacgagtaccggctgcacgagacaagcaaagaacccgatgtgtccctgggcagcacctggcttagtgatttccctcaggcctgggccgagacaggcggaatgggacttgctgttagacaggcccctctgatcatccctctgaaggccacaagcacccctgtgtccatcaagcagtaccccatgagccaagaggcccggctgggaatcaagccccacattcagagactgctggaccagggcatcctggtgccttgtcagagcccttggaatacccctctgctgcccgtgaagaagcccggcaccaacgattacagacccgtgcaggacctgcgggaagtgaacaagagagtggaagatattcaccccaccgtgccgaatccttacaacctgctgtctggcctgcctcctagccaccagtggtacacagtgctggacctgaaggacgccttcttctgtctgcggctgcaccctacaagccagcctctgtttgcctttgagtggcgggaccctgagatgggcattagcggacagctgacctggaccagactgccccagggcttcaagaacagccccacactgttcaacgaggccctgcatagggacctcgccgacttcagaatccagcatcctgacctgatcctgctccagtacgtggacgatctgctgctggccgctacaagcgagctggattgtcagcagggaacaagagccctgctgcaaaccctgggcaacctgggctatagagcctctgccaagaaggcccagatttgccagaaacaagtgaagtatctgggctacctgctgaaagagggccagcgttggctgaccgaggccagaaaagaaaccgtgatgggccagcctacacctaagacacccagacagctgagagagttcctgggcaaagccggattctgtcggctgttcatccctggctttgccgagatggctgcccctctgtacccactgacaaagcccggaactctgttcaactggggcccagatcagcagaaggcctaccaagagatcaagcaggctctgctgacagcccctgctctgggactgcctgatctgaccaagcctttcgagctgttcgtggacgagaagcagggctatgccaaaggcgtgctgacacagaagctcggcccttggagaaggcctgtggcctacctgagcaagaaactggaccctgtggctgccggatggcctccttgtctgagaatggtggccgccattgccgtgctgaccaaggatgccggaaagctgacaatgggacagcctctggtcattctggcccctcatgccgtggaagccctcgtgaaacagcctcctgatcggtggctgagcaacgccaggatgacacactatcaggcactgctgctcgacaccgacagagtgcagtttggacctgtggtggccctgaatcctgccacacttctgcctctgcctgaggaaggcctccagcacaattgcctggacatcctggccgaggctcacggcacaagacccgatctgacagatcagccactgcctgacgccgaccacacctggtatacagatggcagctctctgctgcaagaaggacagagaaaagccggggctgccgtgaccaccgagacagaagtgatttgggccaaagctctgcccgctggcacatctgctcagagagccgaactgatcgccctgacacaggccctgaaaatggccgagggcaagaagctgaacgtctacaccgactccagatacgccttcgccaccgctcacatccacggcgaaatctatcggcggagaggatggctgaccagcgagggcaaagagattaagaacaaggacgagattctcgccctgctcaaggccctgttcctgcctaagcggctgagcatcatccactgtccaggccaccagaagggccactctgctgaagctagaggcaacagaatggccgaccaggctgccagaaaggccgccatcacagagacacccgataccagcacactgctgatcgagaacagcagccctggatccacgccgcccaagaagaagagaaaggttgaggacggcgagggcaccggtggacctggaagcgagcctgctacatctggctctgagacacctggcacctccgagtctgctacacctgaatctggacctggcggatccggagacaagaagtacagcatcggcctggacatcggcaccaactctgtgggctgggccgtgatcaccgacgagtacaaggtgcccagcaagaaattcaaggtgctgggcaacaccgaccggcacagcatcaagaagaacctgatcggagccctgctgttcgacagcggcgaaacagccgaggccacccggctgaagagaaccgccagaagaagatacaccagacggaagaaccggatctgctatctgcaagagatcttcagcaacgagatggccaaggtggacgacagcttcttccacagactggaagagtccttcctggtggaagaggataagaagcacgagcggcaccccatcttcggcaacatcgtggacgaggtggcctaccacgagaagtaccccaccatctaccacctgagaaagaaactggtggacagcaccgacaaggccgacctgcggctgatctatctggccctggcccacatgatcaagttccggggccacttcctgatcgagggcgacctgaaccccgacaacagcgacgtggacaagctgttcatccagctggtgcagacctacaaccagctgttcgaggaaaaccccatcaacgccagcggcgtggacgccaaggccatcctgtctgccagactgagcaagagcagacggctggaaaatctgatcgcccagctgcccggcgagaagaagaatggcctgttcggcaacctgattgccctgagcctgggcctgacccccaacttcaagagcaacttcgacctggccgaggatgccaaactgcagctgagcaaggacacctacgacgacgacctggacaacctgctggcccagatcggcgaccagtacgccgacctgtttctggccgccaagaacctgtccgacgccatcctgctgagcgacatcctgagagtgaacaccgagatcaccaaggcccccctgagcgcctctatgatcaagagatacgacgagcaccaccaggacctgaccctgctgaaagctctcgtgcggcagcagctgcctgagaagtacaaagagattttcttcgaccagagcaagaacggctacgccggctacattgacggcggagccagccaggaagagttctacaagttcatcaagcccatcctggaaaagatggacggcaccgaggaactgctcgtgaagctgaacagagaggacctgctgcggaagcagcggaccttcgacaacggcagcatcccccaccagatccacctgggagagctgcacgccattctgcggcggcaggaagatttttacccattcctgaaggacaaccgggaaaagatcgagaagatcctgaccttccgcatcccctactacgtgggccctctggccaggggaaacagcagattcgcctggatgaccagaaagagcgaggaaaccatcaccccctggaacttcgaggaagtggtggacaagggcgcttccgcccagagcttcatcgagcggatgaccaacttcgataagaacctgcccaacgagaaggtgctgcccaagcacagcctgctgtacgagtacttcaccgtgtataacgagctgaccaaagtgaaatacgtgaccgagggaatgagaaagcccgccttcctgagcggcgagcagaaaaaggccatcgtggacctgctgttcaagaccaaccggaaagtgaccgtgaagcagctgaaagaggactacttcaagaaaatcgagtgcttcgactccgtggaaatctccggcgtggaagatcggttcaacgcctccctgggcacataccacgatctgctgaaaattatcaaggacaaggacttcctggacaatgaggaaaacgaggacattctggaagatatcgtgctgaccctgacactgtttgaggacagagagatgatcgaggaacggctgaaaacctatgcccacctgttcgacgacaaagtgatgaagcagctgaagcggcggagatacaccggctggggcaggctgagccggaagctgatcaacggcatccgggacaagcagtccggcaagacaatcctggatttcctgaagtccgacggcttcgccaacagaaacttcatgcagctgatccacgacgacagcctgacctttaaagaggacatccagaaagcccaggtgtccggccagggcgatagcctgcacgagcacattgccaatctggccggcagccccgccattaagaagggcatcctgcagacagtgaaggtggtggacgagctcgtgaaagtgatgggccggcacaagcccgagaacatcgtgatcgaaatggccagagagaaccagaccacccagaagggacagaagaacagccgcgagagaatgaagcggatcgaagagggcatcaaagagctgggcagccagatcctgaaagaacaccccgtggaaaacacccagctgcagaacgagaagctgtacctgtactacctgcagaatgggcgggatatgtacgtggaccaggaactggacatcaaccggctgtccgactacgatgtggacgccatcgtgcctcagagctttctgaaggacgactccatcgacaacaaggtgctgaccagaagcgacaagaaccggggcaagagcgacaacgtgccctccgaagaggtcgtgaagaagatgaagaactactggcggcagctgctgaacgccaagctgattacccagagaaagttcgacaatctgaccaaggccgagagaggcggcctgagcgaactggataaggccggcttcatcaagagacagctggtggaaacccggcagatcacaaagcacgtggcacagatcctggactcccggatgaacactaagtacgacgagaatgacaagctgatccgggaagtgaaagtgatcaccctgaagtccaagctggtgtccgatttccggaaggatttccagttttacaaagtgcgcgagatcaacaactaccaccacgcccacgacgcctacctgaacgccgtcgtgggaaccgccctgatcaaaaagtaccctaagctggaaagcgagttcgtgtacggcgactacaaggtgtacgacgtgcggaagatgatcgccaagagcgagcaggaaatcggcaaggctaccgccaagtacttcttctacagcaacatcatgaactttttcaagaccgagattaccctggccaacggcgagatccggaagcggcctctgatcgagacaaacggcgaaaccggggagatcgtgtgggataagggccgggattttgccaccgtgcggaaagtgctgagcatgccccaagtgaatatcgtgaaaaagaccgaggtgcagacaggcggcttcagcaaagagtctatcctgcccaagaggaacagcgataagctgatcgccagaaagaaggactgggaccctaagaagtacggcggcttcgacagccccaccgtggcctattctgtgctggtggtggccaaagtggaaaagggcaagtccaagaaactgaagagtgtgaaagagctgctggggatcaccatcatggaaagaagcagcttcgagaagaatcccatcgactttctggaagccaagggctacaaagaagtgaaaaaggacctgatcatcaagctgcctaagtactccctgttcgagctggaaaacggccggaagagaatgctggcctctgccggcgaactgcagaagggaaacgaactggccctgccctccaaatatgtgaacttcctgtacctggccagccactatgagaagctgaagggctcccccgaggataatgagcagaaacagctgtttgtggaacagcacaagcactacctggacgagatcatcgagcagatcagcgagttctccaagagagtgatcctggccgacgctaatctggacaaagtgctgtccgcctacaacaagcaccgggataagcccatcagagagcaggccgagaatatcatccacctgtttaccctgaccaatctgggagcccctgccgccttcaagtactttgacaccaccatcgaccggaagaggtacaccagcaccaaagaggtgctggacgccaccctgatccaccagagcatcaccggcctgtacgagacacggatcgacctgtctcagctgggaggcgacggatccacaccacctaagaagaaacggaaggtcgaggacggcgagggccctgctgctaagagagtgaaactggactccggagctgctccagccgccaagaagaagaagctcgactacaaggacgacgacgataagtgaacgcgtgctcgctttcttgctgtccaatttctattaaaggttcctttgttcgcgttgctggaccagaagatatggcttcggttcagcaaaatgattgcagatccactagttctagagctcgctgatcagcctcgactgtgccttctagttgccagccatctgttgtttgcccctcccccgtgccttccttgaccctggaaggtgccactcccactgtcctttcctaataaaatgaggaaattgcatcgcattgtctgagtaggtgtcattctattctggggggtggggtggggcaggacagcaagggggaggattgggaagacaatagcaggcatgctggggatgcggtgggctctatggcttctgaggcggaaagaaccagctggggctcgagatccactagttctagcctcgaggctagagcggccgccactggccgtcgttttacaacgtcgtgactgggaaaaccctggcgttacccaacttaatcgccttgcagcacatccccctttcgccagctggcgtaatagcgaagaggcccgcaccgatcgcccttcccaacagttgcgcagcctgaatggcgaatgggacgcgccctgtagcggcgcattaagcgcggcgggtgtggtggttacgcgcagcgtgaccgctacacttgccagcgccctagcgcccgctcctttcgctttcttcccttcctttctcgccacgttcgccggctttccccgtcaagctctaaatcgggggctccctttagggttccgatttagtgctttacggcacctcgaccccaaaaaacttgattagggtgatggttcacgtagtgggccatcgccctgatagacggtttttcgccctttgacgttggagtccacgttctttaatagtggactcttgttccaaactggaacaacactcaaccctatctcggtctattcttttgatttataagggattttgccgatttcggcctattggttaaaaaatgagctgatttaacaaaaatttaacgcgaattttaacaaaatattaacgcttacaatttaggtggcacttttcggggaaatgtgcgcggaacccctatttgtttatttttctaaatacattcaaatatgtatccgctcatgagacaataaccctgataaatgcttcaataatattgaaaaaggaagagtatgagtattcaacatttccgtgtcgcccttattcccttttttgcggcattttgccttcctgtttttgctcacccagaaacgctggtgaaagtaaaagatgctgaagatcagttgggtgcacgagtgggttacatcgaactggatctcaacagcggtaagatccttgagagttttcgccccgaagaacgttttccaatgatgagcacttttaaagttctgctatgtggcgcggtattatcccgtattgacgccgggcaagagcaactcggtcgccgcatacactattctcagaatgacttggttgagtactcaccagtcacagaaaagcatcttacggatggcatgacagtaagagaattatgcagtgctgccataaccatgagtgataacactgcggccaacttacttctgacaacgatcggaggaccgaaggagctaaccgcttttttgcacaacatgggggatcatgtaactcgccttgatcgttgggaaccggagctgaatgaagccataccaaacgacgagcgtgacaccacgatgcctgtagcaatggcaacaacgttgcgcaaactattaactggcgaactacttactctagcttcccggcaacaattaatagactggatggaggcggataaagttgcaggaccacttctgcgctcggcccttccggctggctggtttattgctgataaatctggagccggtgagcgtgggtctcgcggtatcattgcagcactggggccagatggtaagccctcccgtatcgtagttatctacacgacggggagtcaggcaactatggatgaacgaaatagacagatcgctgagataggtgcctcactgattaagcattggtaactgtcagaccaagtttactcatatatactttagattgatttaaaacttcatttttaatttaaaaggatctaggtgaagatcctttttgataatctcatgaccaaaatcccttaacgtgagttttcgttccactgagcgtcagaccccgtagaaaagatcaaaggatcttcttgagatcctttttttctgcgcgtaatctgctgcttgcaaacaaaaaaaccaccgctaccagcggtggtttgtttgccggatcaagagctaccaactctttttccgaaggtaactggcttcagcagagcgcagataccaaatactgtccttctagtgtagccgtagttaggccaccacttcaagaactctgtagcaccgcctacatacctcgctctgctaatcctgttaccagtggctgctgccagtggcgataagtcgtgtcttaccgggttggactcaagacgatagttaccggataaggcgcagcggtcgggctgaacggggggttcgtgcacacagcccagcttggagcgaacgacctacaccgaactgagatacctacagcgtgagctatgagaaagcgccacgcttcccgaagggagaaaggcggacaggtatccggtaagcggcagggtcggaacaggagagcgcacgagggagcttccagggggaaacgcctggtatctttatagtcctgtcgggtttcgccacctctgacttgagcgtcgatttttgtgatgctcgtcaggggggcggagcctatggaaaaacgccagcaacgcggcctttttacggttcctggccttttgctggccttttgctcacatgttctttcctgcgttatcccctgattctgtggataaccgtattaccgcctttgagtgagctgataccgctcgccgcagccgaacgaccgagcgcagcgagtcagtgagcgaggaagcggaagagcgcccaatacgcaaaccgcctctccccgcgcgttggccgattcattaatgcagctggcacgacaggtttcccgactggaaagcgggcagtgagcgcaacgcaattaatgtgagttagctcactcattaggcaccccaggctttacactttatgcttccggctcgtatgttgtgtggaattgtgagcggataacaatttcacacaggaaacagctatgaccatga

SEQ ID NO: 262 - DNA, 3477 bp, Synthetic construct
  source 1..3477: mol_type = other DNA
ataaaacctgcaggcatgcaagcgatcgcggggccgcccccttcaccgagggcctatttcccatgattccttcatatttgcatatacgatacaaggctgttagagagataattggaattaatttgactgtaaacacaaagatattagtacaaaatacgtgacgtagaaagtaataatttcttgggtagtttgcagttttaaaattatgttttaaaatggactatcatatgcttaccgtaacttgaaagtatttcgatttcttggctttatatatcttgtggaaaggacgaaacaccgctcccacaacgaagactgacgtttcagagccaccagaagatatggcttcggtggcaagttgaaataaggctagtccgttatcaacttgaaaaagtggcaccgagtcggtgctcggaaccggaggcggaagcgcccggtcatccgcctgtgctgtgtctcccctcgcttctctcgtactgttccaccacggtgtagtcttcgttgtgcgcggttctatctagttacgcgttaaaccaactagaattttttactagttctagagcggccccaattcgccctatagtgagtcgtattacgcgcgctcactggccgtcgttttacaacgtcgtgactgggaaaaccctggcgttacccaacttaatcgccttgcagcacatccccctttcgccagctggcgtaatagcgaagaggcccgcaccgatcgcccttcccaacagttgcgcagcctgaatggcgaatgggacgcgccctgtagcggcgcattaagcgcggcgggtgtggtggttacgcgcagcgtgaccgctacacttgccagcgccctagcgcccgctcctttcgctttcttcccttcctttctcgccacgttcgccggctttccccgtcaagctctaaatcgggggctccctttagggttccgatttagtgctttacggcacctcgaccccaaaaaacttgattagggtgatggttcacgtagtgggccatcgccctgatagacggtttttcgccctttgacgttggagtccacgttctttaatagtggactcttgttccaaactggaacaacactcaaccctatctcggtctattcttttgatttataagggattttgccgatttcggcctattggttaaaaaatgagctgatttaacaaaaatttaacgcgaattttaacaaaatattaacgcttacaatttaggtggcacttttcggggaaatgtgcgcggaacccctatttgtttatttttctaaatacattcaaatatgtatccgctcatgagacaataaccctgataaatgcttcaataatattgaaaaaggaagagtatgagtattcaacatttccgtgtcgcccttattcccttttttgcggcattttgccttcctgtttttgctcacccagaaacgctggtgaaagtaaaagatgctgaagatcagttgggtgcacgagtgggttacatcgaactggatctcaacagcggtaagatccttgagagttttcgccccgaagaacgttttccaatgatgagcacttttaaagttctgctatgtggcgcggtattatcccgtattgacgccgggcaagagcaactcggtcgccgcatacactattctcagaatgacttggttgagtactcaccagtcacagaaaagcatcttacggatggcatgacagtaagagaattatgcagtgctgccataaccatgagtgataacactgcggccaacttacttctgacaacgatcggaggaccgaaggagctaaccgcttttttgcacaacatgggggatcatgtaactcgccttgatcgttgggaaccggagctgaatgaagccataccaaacgacgagcgtgacaccacgatgcctgtagcaatggcaacaacgttgcgcaaactattaactggcgaactacttactctagcttcccggcaacaattaatagactggatggaggcggataaagttgcaggaccacttctgcgctcggcccttccggctggctggtttattgctgataaatctggagccggtgagcgtgggtctcgcggtatcattgcagcactggggccagatggtaagccctcccgtatcgtagttatctacacgacggggagtcaggcaactatggatgaacgaaatagacagatcgctgagataggtgcctcactgattaagcattggtaactgtcagaccaagtttactcatatatactttagattgatttaaaacttcatttttaatttaaaaggatctaggtgaagatcctttttgataatctcatgaccaaaatcccttaacgtgagttttcgttccactgagcgtcagaccccgtagaaaagatcaaaggatcttcttgagatcctttttttctgcgcgtaatctgctgcttgcaaacaaaaaaaccaccgctaccagcggtggtttgtttgccggatcaagagctaccaactctttttccgaaggtaactggcttcagcagagcgcagataccaaatactgtccttctagtgtagccgtagttaggccaccacttcaagaactctgtagcaccgcctacatacctcgctctgctaatcctgttaccagtggctgctgccagtggcgataagtcgtgtcttaccgggttggactcaagacgatagttaccggataaggcgcagcggtcgggctgaacggggggttcgtgcacacagcccagcttggagcgaacgacctacaccgaactgagatacctacagcgtgagctatgagaaagcgccacgcttcccgaagggagaaaggcggacaggtatccggtaagcggcagggtcggaacaggagagcgcacgagggagcttccagggggaaacgcctggtatctttatagtcctgtcgggtttcgccacctctgacttgagcgtcgatttttgtgatgctcgtcaggggggcggagcctatggaaaaacgccagcaacgcggcctttttacggttcctggccttttgctggccttttgctcacatgttctttcctgcgttatcccctgattctgtggataaccgtattaccgcctttgagtgagctgataccgctcgccgcagccgaacgaccgagcgcagcgagtcagtgagcgaggaagcggaagagcgcccaatacgcaaaccgcctctccccgcgcgttggccgattcattaatgcagctggcacgacaggtttcccgactggaaagcgggcagtgagcgcaacgcaattaatgtgagttagctcactcattaggcaccccaggctttacactttatgcttccggctcgtatgttgtgtggaattgtgagcggataacaatttcacacaggaaacagctatgaccatgattacgccaagcgcgcaattaaccctcactaaagggaacaaaagctggaaacatgcatgaagttcctattccgaagttcctattctctagaaagtataggaacttc

SEQ ID NO: 263 - DNA, 5797 bp, Synthetic construct
  source 1..5797: mol_type = other DNA
ggcgcgccggattcgacattgattattgactagttattaatagtaatcaattacggggtcattagttcatagcccatatatggagttccgcgttacataacttacggtaaatggcccgcctggctgaccgcccaacgacccccgcccattgacgtcaataatgacgtatgttcccatagtaacgccaatagggactttccattgacgtcaatgggtggagtatttacggtaaactgcccacttggcagtacatcaagtgtatcatatgccaagtacgccccctattgacgtcaatgacggtaaatggcccgcctggcattatgcccagtacatgaccttatgggactttcctacttggcagtacatctacgtattagtcatcgctattaccatggtcgaggtgagccccacgttctgcttcactctccccatctcccccccctccccacccccaattttgtatttatttattttttaattattttgtgcagcgatgggggcggggggggggggggggcgcgcgccaggcggggcggggcggggcgaggggcggggcggggcgaggcggagaggtgcggcggcagccaatcagagcggcgcgctccgaaagtttccttttatggcgaggcggcggcggcggcggccctataaaaagcgaagcgcgcggcgggcgggagtcgctgcgtcgcgccttcgccccgtgccccgctccgccgccgcctcgcgccgcccgccccggctctgactgaccgcgttactcccacaggtgagcgggcgggacggcccttctcctccgggctgtaattagcgcttggtttaatgacggctcgtttcttttctgtggctgcgtgaaagccttaaagggctccgggagggccctttgtgcgggggggagcggctcggggggtgcgtgcgtgtgtgtgtgcgtggggagcgccgcgtgcggcccgcgctgcccggcggctgtgagcgctgcgggcgcggcgcggggctttgtgcgctccgcgtgtgcgcgaggggagcgcggccgggggcggtgccccgcggtgcgggggggctgcgaggggaacaaaggctgcgtgcggggtgtgtgcgtgggggggtgagcagggggtgtgggcgcggcggtcgggctgtaacccccccctgcacccccctccccgagttgctgagcacggcccggcttcgggtgcggggctccgtgcggggcgtggcgcggggctcgccgtgccgggcggggggtggcggcaggtgggggtgccgggcggggcggggccgcctcgggccggggagggctcgggggaggggcgcggcggccccggagcgccggcggctgtcgaggcgcggcgagccgcagccattgccttttatggtaatcgtgcgagagggcgcagggacttcctttgtcccaaatctggcggagccgaaatctgggaggcgccgccgcaccccctctagcgggcgcgggcgaagcggtgcggcgccggcaggaaggaaatgggcggggagggccttcgtgcgtcgccgcgccgccgtccccttctccatctccagcctcggggctgccgcagggggacggctgccttcgggggggacggggcagggcggggttcggcttctggcgtgtgaccggcggctctagagcctctgctaaccatgttcatgccttcttctttttcctacagatccttaattaataatacgactcactataggggccgccaccatggccgagggatctgttgctagacagcctgaccttctcacgtgcgacgacgagcccattcatatccctggcgctatccagcctcacggcctgttgcttgctctggccgccgatatgacaatcgtggctggcagcgataacctgcctgagctgacaggactggctatcggcgctctgatcggaagatctgccgccgacgtgttcgacagcgagacacacaacagactgacaatcgccctggctgagcctggtgctgctgtgggagcacctatcacagtgggcttcaccatgagaaaggacgctggcttcatcggcagctggcacagacatgaccagctgatctttctggaactggaacctccacagagagacgtggccgagcctcaggctttcttcagaagaacaaacagcgccatcagaaggctccaggccgccgagacactggaatctgcttgtgctgccgccgctcaagaagtgcggaagatcacaggcttcgaccgcgtgatgatctacagattcgccagcgacttcagcggcagcgtgatcgccgaagatagatgcgccgaggtggaaagcaagctgggcctgcactatcccgccagctttatccctgctcaggccagaaggctgtacacaatcaaccccgtgcggatcatccccgacatcaactacagacccgtgcctgtgacacccgatctgaaccctgttaccggcagacccatcgacctgagcttcgccatcctgagaagcgtgtccccaaaccaccttgagttcatgagaaacatcggcatgcacggcaccatgagcatcagcatcctgaggggcgaaagactgtggggcctgatcgtgtgccaccacagaaccccttactacgtggacctggatggcagacaggcttgcgaactggtggctcaggttctggcttggcagatcggagtgatggaggagtgaacgcgtaaatgattgcagatccactagttctagagctcgctgatcagcctcgactgtgccttctagttgccagccatctgttgtttgcccctcccccgtgccttccttgaccctggaaggtgccactcccactgtcctttcctaataaaatgaggaaattgcatcgcattgtctgagtaggtgtcattctattctggggggtggggtggggcaggacagcaagggggaggattgggaagacaatagcaggcatgctggggatgcggtgggctctatggcttctgaggcggaaagaaccagctggggctcgagatccactagttctagcctcgaggctagagcggccgccactggccgtcgttttacaacgtcgtgactgggaaaaccctggcgttacccaacttaatcgccttgcagcacatccccctttcgccagctggcgtaatagcgaagaggcccgcaccgatcgcccttcccaacagttgcgcagcctgaatggcgaatgggacgcgccctgtagcggcgcattaagcgcggcgggtgtggtggttacgcgcagcgtgaccgctacacttgccagcgccctagcgcccgctcctttcgctttcttcccttcctttctcgccacgttcgccggctttccccgtcaagctctaaatcgggggctccctttagggttccgatttagtgctttacggcacctcgaccccaaaaaacttgattagggtgatggttcacgtagtgggccatcgccctgatagacggtttttcgccctttgacgttggagtccacgttctttaatagtggactcttgttccaaactggaacaacactcaaccctatctcggtctattcttttgatttataagggattttgccgatttcggcctattggttaaaaaatgagctgatttaacaaaaatttaacgcgaattttaacaaaatattaacgcttacaatttaggtggcacttttcggggaaatgtgcgcggaacccctatttgtttatttttctaaatacattcaaatatgtatccgctcatgagacaataaccctgataaatgcttcaataatattgaaaaaggaagagtatgagtattcaacatttccgtgtcgcccttattcccttttttgcggcattttgccttcctgtttttgctcacccagaaacgctggtgaaagtaaaagatgctgaagatcagttgggtgcacgagtgggttacatcgaactggatctcaacagcggtaagatccttgagagttttcgccccgaagaacgttttccaatgatgagcacttttaaagttctgctatgtggcgcggtattatcccgtattgacgccgggcaagagcaactcggtcgccgcatacactattctcagaatgacttggttgagtactcaccagtcacagaaaagcatcttacggatggcatgacagtaagagaattatgcagtgctgccataaccatgagtgataacactgcggccaacttacttctgacaacgatcggaggaccgaaggagctaaccgcttttttgcacaacatgggggatcatgtaactcgccttgatcgttgggaaccggagctgaatgaagccataccaaacgacgagcgtgacaccacgatgcctgtagcaatggcaacaacgttgcgcaaactattaactggcgaactacttactctagcttcccggcaacaattaatagactggatggaggcggataaagttgcaggaccacttctgcgctcggcccttccggctggctggtttattgctgataaatctggagccggtgagcgtgggtctcgcggtatcattgcagcactggggccagatggtaagccctcccgtatcgtagttatctacacgacggggagtcaggcaactatggatgaacgaaatagacagatcgctgagataggtgcctcactgattaagcattggtaactgtcagaccaagtttactcatatatactttagattgatttaaaacttcatttttaatttaaaaggatctaggtgaagatcctttttgataatctcatgaccaaaatcccttaacgtgagttttcgttccactgagcgtcagaccccgtagaaaagatcaaaggatcttcttgagatcctttttttctgcgcgtaatctgctgcttgcaaacaaaaaaaccaccgctaccagcggtggtttgtttgccggatcaagagctaccaactctttttccgaaggtaactggcttcagcagagcgcagataccaaatactgtccttctagtgtagccgtagttaggccaccacttcaagaactctgtagcaccgcctacatacctcgctctgctaatcctgttaccagtggctgctgccagtggcgataagtcgtgtcttaccgggttggactcaagacgatagttaccggataaggcgcagcggtcgggctgaacggggggttcgtgcacacagcccagcttggagcgaacgacctacaccgaactgagatacctacagcgtgagctatgagaaagcgccacgcttcccgaagggagaaaggcggacaggtatccggtaagcggcagggtcggaacaggagagcgcacgagggagcttccagggggaaacgcctggtatctttatagtcctgtcgggtttcgccacctctgacttgagcgtcgatttttgtgatgctcgtcaggggggcggagcctatggaaaaacgccagcaacgcggcctttttacggttcctggccttttgctggccttttgctcacatgttctttcctgcgttatcccctgattctgtggataaccgtattaccgcctttgagtgagctgataccgctcgccgcagccgaacgaccgagcgcagcgagtcagtgagcgaggaagcggaagagcgcccaatacgcaaaccgcctctccccgcgcgttggccgattcattaatgcagctggcacgacaggtttcccgactggaaagcgggcagtgagcgcaacgcaattaatgtgagttagctcactcattaggcaccccaggctttacactttatgcttccggctcgtatgttgtgtggaattgtgagcggataacaatttcacacaggaaacagctatgaccatga

SEQ ID NO: 264 - DNA, 6245 bp, Synthetic construct; identical to SEQ ID NO: 252
  source 1..6245: mol_type = other DNA

SEQ ID NO: 265 - DNA, 6364 bp, Synthetic construct
  source 1..6364: mol_type = other DNA
ggcgcgccggattcgacattgattattgactagttattaatagtaatcaattacggggtcattagttcatagcccatatatggagttccgcgttacataacttacggtaaatggcccgcctggctgaccgcccaacgacccccgcccattgacgtcaataatgacgtatgttcccatagtaacgccaatagggactttccattgacgtcaatgggtggagtatttacggtaaactgcccacttggcagtacatcaagtgtatcatatgccaagtacgccccctattgacgtcaatgacggtaaatggcccgcctggcattatgcccagtacatgaccttatgggactttcctacttggcagtacatctacgtattagtcatcgctattaccatggtcgaggtgagccccacgttctgcttcactctccccatctcccccccctccccacccccaattttgtatttatttattttttaattattttgtgcagcgatgggggcggggggggggggggggcgcgcgccaggcggggcggggcggggcgaggggcggggcggggcgaggcggagaggtgcggcggcagccaatcagagcggcgcgctccgaaagtttccttttatggcgaggcggcggcggcggcggccctataaaaagcgaagcgcgcggcgggcgggagtcgctgcgtcgcgccttcgccccgtgccccgctccgccgccgcctcgcgccgcccgccccggctctgactgaccgcgttactcccacaggtgagcgggcgggacggcccttctcctccgggctgtaattagcgcttggtttaatgacggctcgtttcttttctgtggctgcgtgaaagccttaaagggctccgggagggccctttgtgcgggggggagcggctcggggggtgcgtgcgtgtgtgtgtgcgtggggagcgccgcgtgcggcccgcgctgcccggcggctgtgagcgctgcgggcgcggcgcggggctttgtgcgctccgcgtgtgcgcgaggggagcgcggccgggggcggtgccccgcggtgcgggggggctgcgaggggaacaaaggctgcgtgcggggtgtgtgcgtgggggggtgagcagggggtgtgggcgcggcggtcgggctgtaacccccccctgcacccccctccccgagttgctgagcacggcccggcttcgggtgcggggctccgtgcggggcgtggcgcggggctcgccgtgccgggcggggggtggcggcaggtgggggtgccgggcggggcggggccgcctcgggccggggagggctcgggggaggggcgcggcggccccggagcgccggcggctgtcgaggcgcggcgagccgcagccattgccttttatggtaatcgtgcgagagggcgcagggacttcctttgtcccaaatctggcggagccgaaatctgggaggcgccgccgcaccccctctagcgggcgcgggcgaagcggtgcggcgccggcaggaaggaaatgggcggggagggccttcgtgcgtcgccgcgccgccgtccccttctccatctccagcctcggggctgccgcagggggacggctgccttcgggggggacggggcagggcggggttcggcttctggcgtgtgaccggcggctctagagcctctgctaaccatgttcatgccttcttctttttcctacagatccttaattaataatacgactcactataggggccgccaccatgggcgctagagcctctgttctgtctggcggcgaactggacagatgggagaagatcagaagcagacctggcggcaagaagaagtacaagctgaagcacatcgtgtgggccagcagagagctggaaagattcgctgtgaaccccggcctgctggaaacaagcgagggctgtagacagatcctgggccagctccagccatctctccagacaggatctgaggaactgagaagcctgtacaacaccgtggccacactgtactgcgtgcaccagagaatcgagatcaaggacaccaaagaggccctggacaagatcgaggaagaacagaacaagtctaagaagaaggcccagcaggctgccgccgatacaggccactctaatcaggtgtcccagaactaccccatcgtgcagaacatccagggccagatggtgcatcaggctatcagccccagaacactgaacgcctgggtcaaagtggtggaagagaaggctttcagccctgaagtgatccccatgttcagcgccctgtctgagggtgccacacctcaggacctgaacaccatgctgaacacagtcggcggacaccaggccgctatgcagatgctgaaagagacaatcaacgaagaggccgccgagtgggacagagtgcatcctgttcatgctggccctatcgctcccggccagatgagagaacctagaggctctgacattgccggcaccaccagcacactgcaagagcagatcggctggatgacaaacaaccctcctattcctgtgggcgagatctacaagagatggatcatcctgggactgaacaagatcgtgcggatgtacagccccaccagcatcctggacattagacagggccccaaagagcccttcagagactacgtggacagattctacaagaccctgagagccgagcaggccagccaagaagtgaagaactggatgaccgagacactgctggtgcagaacgctaaccccgactgcaagaccatcctgaaggctctgggacctgccgccacactggaagagatgatgacagcctgtcaaggcgtcggaggacctggccataaggctagagttctggccgaggccatgagccaagtgaccaacagcgccacaatcatgatgcagagaggcaacttcagaaaccagcggaagatcgtgaagtccttcaactccggcaaagagggccacaccgcccgcaattctagagcccctagaaagaaaggtggatccggcggcgtttctggatggcggctgttcaagaagatcagcgctagcggtggaaccgagagacaggccaacttcctgggcaagatctggcctagctacaagggcagacccggcaacttcctccagagcagaccagagcctaccgctcctcctgaggaatccttcagatccggcgtggaaaccaccacacctccacagaagcaagagcccatcgacaaagagctgtaccctctgaccagcctgagatccctgttcggcaacgaccctagctctcaatgaacgcgtaaatgattgcagatccactagttctagagctcgctgatcagcctcgactgtgccttctagttgccagccatctgttgtttgcccctcccccgtgccttccttgaccctggaaggtgccactcccactgtcctttcctaataaaatgaggaaattgcatcgcattgtctgagtaggtgtcattctattctggggggtggggtggggcaggacagcaagggggaggattgggaagacaatagcaggcatgctggggatgcggtgggctctatggcttctgaggcggaaagaaccagctggggctcgagatccactagttctagcctcgaggctagagcggccgccactggccgtcgttttacaacgtcgtgactgggaaaaccctggcgttacccaacttaatcgccttgcagcacatccccctttcgccagctggcgtaatagcgaagaggcccgcaccgatcgcccttcccaacagttgcgcagcctgaatggcgaatgggacgcgccctgtagcggcgcattaagcgcggcgggtgtggtggttacgcgcagcgtgaccgctacacttgccagcgccctagcgcccgctcctttcgctttcttcccttcctttctcgccacgttcgccggctttccccgtcaagctctaaatcgggggctccctttagggttccgatttagtgctttacggcacctcgaccccaaaaaacttgattagggtgatggttcacgtagtgggccatcgccctgatagacggtttttcgccctttgacgttggagtccacgttctttaatagtggactcttgttccaaactggaacaacactcaaccctatctcggtctattcttttgatttataagggattttgccgatttcggcctattggttaaaaaatgagctgatttaacaaaaatttaacgcgaattttaacaaaatattaacgcttacaatttaggtggcacttttcggggaaatgtgcgcggaacccctatttgtttatttttctaaatacattcaaatatgtatccgctcatgagacaataaccctgataaatgcttcaataatattgaaaaaggaagagtatgagtattcaacatttccgtgtcgcccttattcccttttttgcggcattttgccttcctgtttttgctcacccagaaacgctggtgaaagtaaaagatgctgaagatcagttgggtgcacgagtgggttacatcgaactggatctcaacagcggtaagatccttgagagttttcgccccgaagaacgttttccaatgatgagcacttttaaagttctgctatgtggcgcggtattatcccgtattgacgccgggcaagagcaactcggtcgccgcatacactattctcagaatgacttggttgagtactcaccagtcacagaaaagcatcttacggatggcatgacagtaagagaattatgcagtgctgccataaccatgagtgataacactgcggccaacttacttctgacaacgatcggaggaccgaaggagctaaccgcttttttgcacaacatgggggatcatgtaactcgccttgatcgttgggaaccggagctgaatgaagccataccaaacgacgagcgtgacaccacgatgcctgtagcaatggcaacaacgttgcgcaaactattaactggcgaactacttactctagcttcccggcaacaattaatagactggatggaggcggataaagttgcaggaccacttctgcgctcggcccttccggctggctggtttattgctgataaatctggagccggtgagcgtgggtctcgcggtatcattgcagcactggggccagatggtaagccctcccgtatcgtagttatctacacgacggggagtcaggcaactatggatgaacgaaatagacagatcgctgagataggtgcctcactgattaagcattggtaactgtcagaccaagtttactcatatatactttagattgatttaaaacttcatttttaatttaaaaggatctaggtgaagatcctttttgataatctcatgaccaaaatcccttaacgtgagttttcgttccactgagcgtcagaccccgtagaaaagatcaaaggatcttcttgagatcctttttttctgcgcgtaatctgctgcttgcaaacaaaaaaaccaccgctaccagcggtggtttgtttgccggatcaagagctaccaactctttttccgaaggtaactggcttcagcagagcgcagataccaaatactgtccttctagtgtagccgtagttaggccaccacttcaagaactctgtagcaccgcctacatacctcgctctgctaatcctgttaccagtggctgctgccagtggcgataagtcgtgtcttaccgggttggactcaagacgatagttaccggataaggcgcagcggtcgggctgaacggggggttcgtgcacacagcccagcttggagcgaacgacctacaccgaactgagatacctacagcgtgagctatgagaaagcgccacgcttcccgaagggagaaaggcggacaggtatccggtaagcggcagggtcggaacaggagagcgcacgagggagcttccagggggaaacgcctggtatctttatagtcctgtcgggtttcgccacctctgacttgagcgtcgatttttgtgatgctcgtcaggggggcggagcctatggaaaaacgccagcaacgcggcctttttacggttcctggccttttgctggccttttgctcacatgttctttcctgcgttatcccctgattctgtggataaccgtattaccgcctttgagtgagctgataccgctcgccgcagccgaacgaccgagcgcagcgagtcagtgagcgaggaagcggaagagcgcccaatacgcaaaccgcctctccccgcgcgttggccgattcattaatgcagctggcacgacaggtttcccgactggaaagcgggcagtgagcgcaacgcaattaatgtgagttagctcactcattaggcaccccaggctttacactttatgcttccggctcgtatgttgtgtggaattgtgagcggataacaatttcacacaggaaacagctatgaccatga

SEQ ID NO: 266 - DNA, 6877 bp, Synthetic construct
  source 1..6877: mol_type = other DNA
ggcgcgccggattcgacattgattattgactagttattaatagtaatcaattacggggtcattagttcatagcccatatatggagttccgcgttacataacttacggtaaatggcccgcctggctgaccgcccaacgacccccgcccattgacgtcaataatgacgtatgttcccatagtaacgccaatagggactttccattgacgtcaatgggtggagtatttacggtaaactgcccacttggcagtacatcaagtgtatcatatgccaagtacgccccctattgacgtcaatgacggtaaatggcccgcctggcattatgcccagtacatgaccttatgggactttcctacttggcagtacatctacgtattagtcatcgctattaccatggtcgaggtgagccccacgttctgcttcactctccccatctcccccccctccccacccccaattttgtatttatttattttttaattattttgtgcagcgatgggggcggggggggggggggggcgcgcgccaggcggggcggggcggggcgaggggcggggcggggcgaggcggagaggtgcggcggcagccaatcagagcggcgcgctccgaaagtttccttttatggcgaggcggcggcggcggcggccctataaaaagcgaagcgcgcggcgggcgggagtcgctgcgtcgcgccttcgccccgtgccccgctccgccgccgcctcgcgccgcccgccccggctctgactgaccgcgttactcccacaggtgagcgggcgggacggcccttctcctccgggctgtaattagcgcttggtttaatgacggctcgtttcttttctgtggctgcgtgaaagccttaaagggctccgggagggccctttgtgcgggggggagcggctcggggggtgcgtgcgtgtgtgtgtgcgtggggagcgccgcgtgcggcccgcgctgcccggcggctgtgagcgctgcgggcgcggcgcggggctttgtgcgctccgcgtgtgcgcgaggggagcgcggccgggggcggtgccccgcggtgcgggggggctgcgaggggaacaaaggctgcgtgcggggtgtgtgcgtgggggggtgagcagggggtgtgggcgcggcggtcgggctgtaacccccccctgcacccccctccccgagttgctgagcacggcccggcttcgggtgcggggctccgtgcggggcgtggcgcggggctcgccgtgccgggcggggggtggcggcaggtgggggtgccgggcggggcggggccgcctcgggccggggagggctcgggggaggggcgcggcggccccggagcgccggcggctgtcgaggcgcggcgagccgcagccattgccttttatggtaatcgtgcgagagggcgcagggacttcctttgtcccaaatctggcggagccgaaatctgggaggcgccgccgcaccccctctagcgggcgcgggcgaagcggtgcggcgccggcaggaaggaaatgggcggggagggccttcgtgcgtcgccgcgccgccgtccccttctccatctccagcctcggggctgccgcagggggacggctgccttcgggggggacggggcagggcggggttcggcttctggcgtgtgaccggcggctctagagcctctgctaaccatgttcatgccttcttctttttcctacagatccttaattaataatacgactcactataggggccgccaccatgggcgctagagcctctgttctgtctggcggcgaactggacagatgggagaagatcagactgagacctggcggcaagaagaagtacaagctgaagcacatcgtgtgggccagcagagagctggaaagattcgctgtgaaccccggcctgctggaaacaagcgagggctgtagacagatcctgggccagctccagccatctctccagacaggatctgaggaactgagaagcctgtacaacaccgtggccacactgtactgcgtgcaccagagaatcgagatcaaggacaccaaagaggccctggacaagatcgaggaagaacagaacaagtctaagaagaaggcccagcaggctgccgccgatacaggccactctaatcaggtgtcccagaactaccccatcgtgcagaacatccagggccagatggtgcatcaggctatcagccccagaacactgaacgcctgggtcaaagtggtggaagagaaggctttcagccctgaagtgatccccatgttcagcgccctgtctgagggtgccacacctcaggacctgaacaccatgctgaacacagtcggcggacaccaggccgctatgcagatgctgaaagagacaatcaacgaagaggccgccgagtgggacagagtgcatcctgttcatgctggccctatcgctcccggccagatgagagaacctagaggctctgacattgccggcaccaccagcacactgcaagagcagatcggctggatgacaaacaaccctcctattcctgtgggcgagatctacaagagatggatcatcctgggactgaacaagatcgtgcggatgtacagccccaccagcatcctggacattagacagggccccaaagagcccttcagagactacgtggacagattctacaagaccctgagagccgagcaggccagccaagaagtgaagaactggatgaccgagacactgctggtgcagaacgctaaccccgactgcaagaccatcctgaaggctctgggacctgccgccacactggaagagatgatgacagcctgtcaaggcgtcggaggacctggccataaggctagagttctggccgaggccatgagccaagtgaccaacagcgccacaatcatgatgcagagaggcaacttcagaaaccagcggaagatcgtgaagtccttcaactccggcaaagagggccacaccgcccgcaattctagagcccctagaaagaaaggtggatccggcggcgtttctggatggcggctgttcaagaagatcagcggcggttccggacctgctgccaaaagagtgaaactggactccggactgcaactgcctccactggaaagactgacactgggagctgccccagccgccaagaagaaaaagctggactacaaggacgacgacgacaagggcggagctagctctaagacaatcgtgctgtctgtgggcgaagccaccagaacactgaccgagatccagagcacagccgacagacagatcttcgaggaaaaagtgggccctctcgtgggcagactgagactgacagcttccctgagacagaacggcgccaagaccgcctacagagtgaacctgaagctggaccaggccgacgtggtggattctggccttcctaaagtgcggtacacccaagtgtggtcccacgacgtgaccatcgtggccaattctaccgaggccagcagaaagagcctgtacgacctgaccaagagcctggtggccacaagccaggtggaagatctggtcgtgaacctggtgcctctcggacgtggcggatccggtggaaccgagagacaggccaacttcctgggcaagatctggcctagctacaagggcagacccggcaacttcctccagagcagaccagagcctaccgctcctcctgaggaatccttcagatccggcgtggaaaccaccacacctccacagaagcaagagcccatcgacaaagagctgtaccctctgaccagcctgagatccctgttcggcaacgaccctagctctcaatgaacgcgtaaatgattgcagatccactagttctagagctcgctgatcagcctcgactgtgccttctagttgccagccatctgttgtttgcccctcccccgtgccttccttgaccctggaaggtgccactcccactgtcctttcctaataaaatgaggaaattgcatcgcattgtctgagtaggtgtcattctattctggggggtggggtggggcaggacagcaagggggaggattgggaagacaatagcaggcatgctggggatgcggtgggctctatggcttctgaggcggaaagaaccagctggggctcgagatccactagttctagcctcgaggctagagcggccgccactggccgtcgttttacaacgtcgtgactgggaaaaccctggcgttacccaacttaatcgccttgcagcacatccccctttcgccagctggcgtaatagcgaagaggcccgcaccgatcgcccttcccaacagttgcgcagcctgaatggcgaatgggacgcgccctgtagcggcgcattaagcgcggcgggtgtggtggttacgcgcagcgtgaccgctacacttgccagcgccctagcgcccgctcctttcgctttcttcccttcctttctcgccacgttcgccggctttccccgtcaagctctaaatcgggggctccctttagggttccgatttagtgctttacggcacctcgaccccaaaaaacttgattagggtgatggttcacgtagtgggccatcgccctgatagacggtttttcgccctttgacgttggagtccacgttctttaatagtggactcttgttccaaactggaacaacactcaaccctatctcggtctattcttttgatttataagggattttgccgatttcggcctattggttaaaaaatgagctgatttaacaaaaatttaacgcgaattttaacaaaatattaacgcttacaatttaggtggcacttttcggggaaatgtgcgcggaacccctatttgtttatttttctaaatacattcaaatatgtatccgctcatgagacaataaccctgataaatgcttcaataatattgaaaaaggaagagtatgagtattcaacatttccgtgtcgcccttattcccttttttgcggcattttgccttcctgtttttgctcacccagaaacgctggtgaaagtaaaagatgctgaagatcagttgggtgcacgagtgggttacatcgaactggatctcaacagcggtaagatccttgagagttttcgccccgaagaacgttttccaatgatgagcacttttaaagttctgctatgtggcgcggtattatcccgtattgacgccgggcaagagcaactcggtcgccgcatacactattctcagaatgacttggttgagtactcaccagtcacagaaaagcatcttacggatggcatgacagtaagagaattatgcagtgctgccataaccatgagtgataacactgcggccaacttacttctgacaacgatcggaggaccgaaggagctaaccgcttttttgcacaacatgggggatcatgtaactcgccttgatcgttgggaaccggagctgaatgaagccataccaaacgacgagcgtgacaccacgatgcctgtagcaatggcaacaacgttgcgcaaactattaactggcgaactacttactctagcttcccggcaacaattaatagactggatggaggcggataaagttgcaggaccacttctgcgctcggcccttccggctggctggtttattgctgataaatctggagccggtgagcgtgggtctcgcggtatcattgcagcactggggccagatggtaagccctcccgtatcgtagttatctacacgacggggagtcaggcaactatggatgaacgaaatagacagatcgctgagataggtgcctcactgattaagcattggtaactgtcagaccaagtttactcatatatactttagattgatttaaaacttcatttttaatttaaaaggatctaggtgaagatcctttttgataatctcatgaccaaaatcccttaacgtgagttttcgttccactgagcgtcagaccccgtagaaaagatcaaaggatcttcttgagatcctttttttctgcgcgtaatctgctgcttgcaaacaaaaaaaccaccgctaccagcggtggtttgtttgccggatcaagagctaccaactctttttccgaaggtaactggcttcagcagagcgcagataccaaatactgtccttctagtgtagccgtagttaggccaccacttcaagaactctgtagcaccgcctacatacctcgctctgctaatcctgttaccagtggctgctgccagtggcgataagtcgtgtcttaccgggttggactcaagacgatagttaccggataaggcgcagcggtcgggctgaacggggggttcgtgcacacagcccagcttggagcgaacgacctacaccgaactgagatacctacagcgtgagctatgagaaagcgccacgcttcccgaagggagaaaggcggacaggtatccggtaagcggcagggtcggaacaggagagcgcacgagggagcttccagggggaaacgcctggtatctttatagtcctgtcgggtttcgccacctctgacttgagcgtcgatttttgtgatgctcgtcaggggggcggagcctatggaaaaacgccagcaacgcggcctttttacggttcctggccttttgctggccttttgctcacatgttctttcctgcgttatcccctgattctgtggataaccgtattaccgcctttgagtgagctgataccgctcgccgcagccgaacgaccgagcgcagcgagtcagtgagcgaggaagcggaagagcgcccaatacgcaaaccgcctctccccgcgcgttggccgattcattaatgcagctggcacgacaggtttcccgactggaaagcgggcagtgagcgcaacgcaattaatgtgagttagctcactcattaggcaccccaggctttacactttatgcttccggctcgtatgttgtgtggaattgtgagcggataacaatttcacacaggaaacagctatgaccatga

SEQ ID NO: 267 - DNA, 10644 bp, Synthetic construct
  source 1..10644: mol_type = other DNA
aaccttgttggtccaaaatgcgaacccagattgtaagactattttaaaagcattgggaccaggagcgacactagaagaaatgatgacagcatgtcagggagtggggggacccggccataaagcaagagttttggctgaagcaatgagccaagtaacaaatccagctaccataatgatacagaaaggcaattttaggaaccaaagaaagactgttaagtgtttcaattgtggcaaagaagggcacatagccaaaaattgcagggcccctaggaaaaagggctgttggaaatgtggaaaggaaggacaccaaatgaaagattgtactgagagacaggctaattttttagggaagatctggccttcccacaagggaaggccagggaattttcttcagagcagaccagagccaacagccccaccagaagagagcttcaggtttggggaagagacaacaactccctctcagaagcaggagccgatagacaaggaactgtatcctttagcttccctcagatcactctttggcagcgacccctcgtcacaataaagataggggggcaattaaaggaagctctattagatacaggagcagatgatacagtattagaagaaatgaatttgccaggaagatggaaaccaaaaatgatagggggaattggaggttttatcaaagtaagacagtatgatcagatactcatagaaatctgcggacataaagctataggtacagtattagtaggacctacacctgtcaacataattggaagaaatctgttgactcagattggctgcactttaaattttcccattagtcctattgagactgtaccagtaaaattaaagccaggaatggatggcccaaaagttaaacaatggccattgacagaagaaaaaataaaagcattagtagaaatttgtacagaaatggaaaaggaaggaaaaatttcaaaaattgggcctgaaaatccatacaatactccagtatttgccataaagaaaaaagacagtactaaatggagaaaattagtagatttcagagaacttaataagagaactcaagatttctgggaagttcaattaggaataccacatcctgcagggttaaaacagaaaaaatcagtaacagtactggatgtgggcgatgcatatttttcagttcccttagataaagacttcaggaagtatactgcatttaccatacctagtataaacaatgagacaccagggattagatatcagtacaatgtgcttccacagggatggaaaggatcaccagcaatattccagtgtagcatgacaaaaatcttagagccttttagaaaacaaaatccagacatagtcatctatcaatacatggccgctttgtatgtaggatctgacttagaaatagggcagcatagaacaaaaatagaggaactgagacaacatctgttgaggtggggatttaccacaccagacaaaaaacatcagaaagaacctccattcctttggatgggttatgaactccatcctgataaatggacagtacagcctatagtgctgccagaaaaggacagctggactgtcaatgacatacagaaattagtgggaaaattgaattgggcaagtcagatttatgcagggattaaagtaaggcaattatgtaaacttcttaggggaaccaaagcactaacagaagtagtaccactaacagaagaagcagagctagaactggcagaaaacagggagattctaaaagaaccggtacatggagtgtattatgacccatcaaaagacttaatagcagaaatacagaagcaggggcaaggccaatggacatatcaaatttatcaagagccatttaaaaatctgaaaacaggaaagtatgcaagaatgaagggtgcccacactaatgatgtgaaacaattaacagaggcagtacaaaaaatagccacagaaagcatagtaatatggggaaagactcctaaatttaaattacccatacaaaaggaaacatgggaagcatggtggacagagtattggcaagccacctggattcctgagtgggagtttgtcaatacccctcccttagtgaagttatggtaccagttagagaaagaacccataataggagcagaaactttctatgtagatggggcagccaatagggaaactaaattaggaaaagcaggatatgtaactgacagaggaagacaaaaagttgtccccctaacggacacaacaaatcagaagactgagttacaagcaattcatctagctttgcaggattcgggattagaagtaaacatagtgacagactcacaatatgcattgggaatcattcaagcacaaccagataagagtgaatcagagttagtcagtcaaataatagagcagttaataaaaaaggaaaaagtctacctggcatgggtaccagcacacaaaggaattggaggaaatgaacaagtagataaattggtcagtgctggaatcaggaaagtactatttttagatggaatagataaggcccaagaagaacatgagaaatatcacagtaattggagagcaatggctagtgattttaacctaccacctgtagtagcaaaagaaatagtagccagctgtgataaatgtcagctaaaaggggaagccatgcatggacaagtagactgtagcccaggaatatggcagctagtttgtacacatttagaaggaaaagttatcttggtagcagttcatgtagccagtggatatatagaagcagaagtaattccagcagagacagggcaagaaacagcatacttcctcttaaaattagcaggaagatggccagtaaaaacagtacatacagacaatggcagcaatttcaccagtactacagttaaggccgcctgttggtgggcggggatcaagcaggaatttggcattccctacaatccccaaagtcaaggagtaatagaatctatgaataaagaattaaagaaaattataggacaggtaagagatcaggctgaacatcttaagacagcagtacaaatggcagtattcatccacaattttaaaagaaaaggggggattggggggtacagtgcaggggaaagaatagtagacataatagcaacagacatacaaactaaagaattacaaaaacaaattacaaaaattcaaaattttcgggtttattacagggacagcagagatccagtttggaaaggaccagcaaagctcctctggaaaggtgaaggggcagtagtaatacaagataatagtgacataaaagtagtgccaagaagaaaagcaaagatcatcagggattatggaaaacagatggcaggtgatgattgtgtggcaagtagacaggatgaggattaacacatggaattctgcaacaactgctgtttatccatttcagaattgggtgtcgacatagcagaataggcgttactcgacagaggagagcaagaaatggagccagtagatcctagactagagccctggaagcatccaggaagtcagcctaaaactgcttgtaccaattgctattgtaaaaagtgttgctttcattgccaagtttgtttcatgacaaaagccttaggcatctcctatggcaggaagaagcggagacagcgacgaagagctcatcagaacagtcagactcatcaagcttctctatcaaagcagtaagtagtacatgtaatgcaacctataatagtagcaatagtagcattagtagtagcaataataatagcaatagttgtgtggtccatagtaatcatagaatataggaaaatggccgctgatcttcagacctggaggaggagatatgagggacaattggagaagtgaattatataaatataaagtagtaaaaattgaaccattaggagtagcacccaccaaggcaaagagaagagtggtgcagagagaaaaaagagcagtgggaataggagctttgttccttgggttcttgggagcagcaggaagcactatgggcgcagcgtcaatgacgctgacggtacaggccagacaattattgtctggtatagtgcagcagcagaacaatttgctgagggctattgaggcgcaacagcatctgttgcaactcacagtctggggcatcaagcagctccaggcaagaatcctggctgtggaaagatacctaaaggatcaacagctcctggggatttggggttgctctggaaaactcatttgcaccactgctgtgccttggaatgctagttggagtaataaatctctggaacagatttggaatcacacgacctggatggagtgggacagagaaattaacaattacacaagcttaatacactccttaattgaagaatcgcaaaaccagcaagaaaagaatgaacaagaattattggaattagataaatgggcaagtttgtggaattggtttaacataacaaattggctgtggtatataaaattattcataatgatagtaggaggcttggtaggtttaagaatagtttttgctgtactttctatagtgaatagagttaggcagggatattcaccattatcgtttcagacccacctcccaaccccgaggggacccgacaggcccgaaggaatagaagaagaaggtggagagagagacagagacagatccattcgattagtgaacggatccttggcacttatctgggacgatctgcggagcctgtgcctcttcagctaccaccgcttgagagacttactcttgattgtaacgaggattgtggaacttctgggacgcagggggtgggaagccctcaaatattggtggaatctcctacaatattggagtcaggagctaaagaatagtgctgttagcttgctcaatgccacagccatagcagtagctgaggggacagatagggttatagaagtagtacaaggagcttgtagagctattcgccacatacctagaagaataagacagggcttggaaaggattttgctataagctcgaaacaaccggtacctctagaactatagctagcagatctttttccctctgccaaaaattatggggacatcatgaagccccttgagcatctgacttctggctaataaaggaaatttattttcattgcaatagtgtgttggaattttttgtgtctctcactcggaaggacatatgggagggcaaatcatttaaaacatcagaatgagtatttggtttagagtttggcaacatatgcccatatgctggctgccatgaacaaaggttggctataaagaggtcatcagtatatgaaacagccccctgctgtccattccttattccatagaaaagccttgacttgaggttagattttttttatattttgttttgtgttatttttttctttaacatccctaaaattttccttacatgttttactagccagatttttcctcctctcctgactactcccagtcatagctgtccctcttctcttatggagatccctcgacctgcagcccaagcttggcgtaatcatggtcatagctgtttcctgtgtgaaattgttatccgctcacaattccacacaacatacgagccggaagcataaagtgtaaagcctggggtgcctaatgagtgagctaactcacattaattgcgttgcgctcactgcccgctttccagtcgggaaacctgtcgtgccagcggatccgcatctcaattagtcagcaaccatagtcccgcccctaactccgcccatcccgcccctaactccgcccagttccgcccattctccgccccatggctgactaattttttttatttatgcagaggccgaggccgcctcggcctctgagctattccagaagtagtgaggaggcttttttggaggcctaggcttttgcaaaaagctaacttgtttattgcagcttataatggttacaaataaagcaatagcatcacaaatttcacaaataaagcatttttttcactgcattctagttgtggtttgtccaaactcatcaatgtatcttatcatgtctggatccgctgcattaatgaatcggccaacgcgcggggagaggcggtttgcgtattgggcgctcttccgcttcctcgctcactgactcgctgcgctcggtcgttcggctgcggcgagcggtatcagctcactcaaaggcggtaatacggttatccacagaatcaggggataacgcaggaaagaacatgtgagcaaaaggccagcaaaaggccaggaaccgtaaaaaggccgcgttgctggcgtttttccataggctccgcccccctgacgagcatcacaaaaatcgacgctcaagtcagaggtggcgaaacccgacaggactataaagataccaggcgtttccccctggaagctccctcgtgcgctctcctgttccgaccctgccgcttaccggatacctgtccgcctttctcccttcgggaagcgtggcgctttctcatagctcacgctgtaggtatctcagttcggtgtaggtcgttcgctccaagctgggctgtgtgcacgaaccccccgttcagcccgaccgctgcgccttatccggtaactatcgtcttgagtccaacccggtaagacacgacttatcgccactggcagcagccactggtaacaggattagcagagcgaggtatgtaggcggtgctacagagttcttgaagtggtggcctaactacggctacactagaagaacagtatttggtatctgcgctctgctgaagccagttaccttcggaaaaagagttggtagctcttgatccggcaaacaaaccaccgctggtagcggtggtttttttgtttgcaagcagcagattacgcgcagaaaaaaaggatctcaagaagatcctttgatcttttctacggggtctgacgctcagtggaacgaaaactcacgttaagggattttggtcatgagattatcaaaaaggatcttcacctagatccttttaaattaaaaatgaagttttaaatcaatctaaagtatatatgagtaaacttggtctgacagttaccaatgcttaatcagtgaggcacctatctcagcgatctgtctatttcgttcatccatagttgcctgactccccgtcgtgtagataactacgatacgggagggcttaccatctggccccagtgctgcaatgataccgcgagacccacgctcaccggctccagatttatcagcaataaaccagccagccggaagggccgagcgcagaagtggtcctgcaactttatccgcctccatccagtctattaattgttgccgggaagctagagtaagtagttcgccagttaatagtttgcgcaacgttgttgccattgctacaggcatcgtggtgtcacgctcgtcgtttggtatggcttcattcagctccggttcccaacgatcaaggcgagttacatgatcccccatgttgtgcaaaaaagcggttagctccttcggtcctccgatcgttgtcagaagtaagttggccgcagtgttatcactcatggttatggcagcactgcataattctcttactgtcatgccatccgtaagatgcttttctgtgactggtgagtactcaaccaagtcattctgagaatagtgtatgcggcgaccgagttgctcttgcccggcgtcaatacgggataataccgcgccacatagcagaactttaaaagtgctcatcattggaaaacgttcttcggggcgaaaactctcaaggatcttaccgctgttgagatccagttcgatgtaacccactcgtgcacccaactgatcttcagcatcttttactttcaccagcgtttctgggtgagcaaaaacaggaaggcaaaatgccgcaaaaaagggaataagggcgacacggaaatgttgaatactcatactcttcctttttcaatattattgaagcatttatcagggttattgtctcatgagcggatacatatttgaatgtatttagaaaaataaacaaataggggttccgcgcacatttccccgaaaagtgccacctgggtcgacattgattattgactagttattaatagtaatcaattacggggtcattagttcatagcccatatatggagttccgcgttacataacttacggtaaatggcccgcctggctgaccgcccaacgacccccgcccattgacgtcaataatgacgtatgttcccatagtaacgccaatagggactttccattgacgtcaatgggtggagtatttacggtaaactgcccacttggcagtacatcaagtgtatcatatgccaagtacgccccctattgacgtcaatgacggtaaatggcccgcctggcattatgcccagtacatgaccttatgggactttcctacttggcagtacatctacgtattagtcatcgctattaccatggtcgaggtgagccccacgttctgcttcactctccccatctcccccccctccccacccccaattttgtatttatttattttttaattattttgtgcagggcgaggcggagaggtgcggcggcagccaatcagagcggcgcgctccgaaagtttccttttatggcgaggcggcggcggcggcggccctataaaaagcgaagcgcgcggcgggcgggagtcgctgcgcgctgccttcgccccgtgccccgctccgccgccgcctcgcgccgcccgccccggctctgactgaccgcgttactcccacaggtgagcgggcgggacggcccttctcctccgggctgtaattagcgcttggtttaatgacggcttgtttcttttctgtggctgcgtgaaagccttgaggggctccgggagggccctttgtgcggggggagcggctcggggggtgcgtgcgtgtgtgtgtgcgtggggagcgccgcgtgcggctccgcgctgcccggcggctgtgagcgctgcgggcgcggcgcggggctttgtgcgctccgcagtgtgcgcgaggggagcgcggccgggggcggtgccccgcggtgcggggggggctgcgaggggaacaaaggctgcgtgcggggtgtgtgcgtgggggggtgagcagggggtgtgggcgcgtcggtcgggctgcaaccccccctgcacccccctccccgagttgctgagcacggcccggcttcgggtgcggggctccgtacggggcgtggcgcggggctcgccgtgccgggcggggggtggcggcaggtgggggtgccgggcggggcggggccgcctcgggccggggagggctcgggggaggggcgcggcggcccccggagcgccggcggctgtcgaggcgcggcgagccgcagccattgccttttatggtaatcgtgcgagagggcgcagggacttcctttgtcccaaatctgtgcggagccgaaatctgggaggcgccgccgcaccccctctagcgggcgcggggcgaagcggtgcggcgccggcaggaaggaaatgggcggggagggccttcgtgcgtcgccgcgccgccgtccccttctccctctccagcctcggggctgtccgcggggggacggctgccttcgggggggacggggcagggcggggttcggcttctggcgtgtgaccggcggctctagagcctctgctaaccatgttcatgccttcttctttttcctacagctcctgggcaacgtgctggttattgtgctgtctcatcattttggcaaagaattcgggccgcgttgacgcgcacggcaagaggcgaggggcggcgactggtgagagatgggtgcgagagcgtcagtattaagcgggggagaattagatcgatgggaaaaaattcggttaaggccagggggaaagaaaaaatataaattaaaacatatagtatgggcaagcagggagctagaacgattcgcagttaatcctggcctgttagaaacatcagaaggctgtagacaaatactgggacagctacaaccatcccttcagacaggatcagaagaacttagatcattatataatacagtagcaaccctctattgtgtgcatcaaaggatagagataaaagacaccaaggaagctttagacaagatagaggaagagcaaaacaaaagtaagaaaaaagcacagcaagcagcagctgacacaggacacagcaatcaggtcagccaaaattaccctatagtgcagaacatccaggggcaaatggtacatcaggccatatcacctagaactttaaatgcatgggtaaaagtagtagaagagaaggctttcagcccagaagtgatacccatgttttcagcattatcagaaggagccaccccacaagatttaaacaccatgctaaacacagtggggggacatcaagcagccatgcaaatgttaaaagagaccatcaatgaggaagctgcagaatgggatagagtgcatccagtgcatgcagggcctattgcaccaggccagatgagagaaccaaggggaagtgacatagcaggaactactagtacccttcaggaacaaataggatggatgacacataatccacctatcccagtaggagaaatctataaaagatggataatcctgggattaaataaaatagtaagaatgtatagccctaccagcattctggacataagacaaggaccaaaggaaccctttagagactatgtagaccgattctataaaactctaagagccgagcaagcttcacaagaggtaaaaaattggatgacaga

SEQ ID NO: 268 - DNA, 10644 bp, Synthetic construct
  source 1..10644: mol_type = other DNA
aaccttgttggtccaaaatgcgaacccagattgtaagactattttaaaagcattgggaccaggagcgacactagaagaaatgatgacagcatgtcagggagtggggggacccggccataaagcaagagttttggctgaagcaatgagccaagtaacaaatccagctaccataatgatacagaaaggcaattttaggaaccaaagaaagactgttaagtgtttcaattgtggcaaagaagggcacatagccaaaaattgcagggcccctaggaaaaagggctgttggaaatgtggaaaggaaggacaccaaatgaaagattgtactgagagacaggctaattttttagggaagatctggccttcccacaagggaaggccagggaattttcttcagagcagaccagagccaacagccccaccagaagagagcttcaggtttggggaagagacaacaactccctctcagaagcaggagccgatagacaaggaactgtatcctttagcttccctcagatcactctttggcagcgacccctcgtcacaataaagataggggggcaattaaaggaagctctattagatacaggagcagatgatacagtattagaagaaatgaatttgccaggaagatggaaaccaaaaatgatagggggaattggaggttttatcaaagtaagacagtatgatcagatactcatagaaatctgcggacataaagctataggtacagtattagtaggacctacacctgtcaacataattggaagaaatctgttgactcagattggctgcactttaaattttcccattagtcctattgagactgtaccagtaaaattaaagccaggaatggatggcccaaaagttaaacaatggccattgacagaagaaaaaataaaagcattagtagaaatttgtacagaaatggaaaaggaaggaaaaatttcaaaaattgggcctgaaaatccatacaatactccagtatttgccataaagaaaaaagacagtactaaatggagaaaattagtagatttcagagaacttaataagagaactcaagatttctgggaagttcaattaggaataccacatcctgcagggttaaaacagaaaaaatcagtaacagtactggatgtgggcgatgcatatttttcagttcccttagataaagacttcaggaagtatactgcatttaccatacctagtataaacaatgagacaccagggattagatatcagtacaatgtgcttccacagggatggaaaggatcaccagcaatattccagtgtagcatgacaaaaatcttagagccttttagaaaacaaaatccagacatagtcatctatcaatacatggatgatttgtatgtaggatctgacttagaaatagggcagcatagaacaaaaatagaggaactgagacaacatctgttgaggtggggatttaccacaccagacaaaaaacatcagaaagaacctccattcctttggatgggttatgaactccatcctgataaatggacagtacagcctatagtgctgccagaaaaggacagctggactgtcaatgacatacagaaattagtgggaaaattgaattgggcaagtcagatttatgcagggattaaagtaaggcaattatgtaaacttcttaggggaaccaaagcactaacagaagtagtaccactaacagaagaagcagagctagaactggcagaaaacagggagattctaaaagaaccggtacatggagtgtattatgacccatcaaaagacttaatagcagaaatacagaagcaggggcaaggccaatggacatatcaaatttatcaagagccatttaaaaatctgaaaacaggaaagtatgcaagaatgaagggtgcccacactaatgatgtgaaacaattaacagaggcagtacaaaaaatagccacagaaagcatagtaatatggggaaagactcctaaatttaaattacccatacaaaaggaaacatgggaagcatggtggacagagtattggcaagccacctggattcctgagtgggagtttgtcaatacccctcccttagtgaagttatggtaccagttagagaaagaacccataataggagcagaaactttctatgtagatggggcagccaatagggaaactaaattaggaaaagcaggatatgtaactgacagaggaagacaaaaagttgtccccctaacggacacaacaaatcagaagactgagttacaagcaattcatctagctttgcaggattcgggattagaagtaaacatagtgacagactcacaatatgcattgggaatcattcaagcacaaccagataagagtgaatcagagttagtcagtcaaataatagagcagttaataaaaaaggaaaaagtctacctggcatgggtaccagcacacaaaggaattggaggaaatgaacaagtagataaattggtcagtgctggaatcaggaaagtactatttttagatggaatagataaggcccaagaagaacatgagaaatatcacagtaattggagagcaatggctagtgattttaacctaccacctgtagtagcaaaagaaatagtagccagctgtgataaatgtcagctaaaaggggaagccatgcatggacaagtagactgtagcccaggaatatggcagctagtttgtacacatttagaaggaaaagttatcttggtagcagttcatgtagccagtggatatatagaagcagaagtaattccagcagagacagggcaagaaacagcatacttcctcttaaaattagcaggaagatggccagtaaaaacagtacatacagacaatggcagcaatttcaccagtactacagttaaggccgcctgttggtgggcggggatcaagcaggaatttggcattccctacaatccccaaagtcaaggagtaatagaatctatgaataaagaattaaagaaaattataggacaggtaagagatcaggctgaacatcttaagacagcagtacaaatggcagtattcatccacaattttaaaagaaaaggggggattggggggtacagtgcaggggaaagaatagtagacataatagcaacagacatacaaactaaagaattacaaaaacaaattacaaaaattcaaaattttcgggtttattacagggacagcagagatccagtttggaaaggaccagcaaagctcctctggaaaggtgaaggggcagtagtaatacaagataatagtgacataaaagtagtgccaagaagaaaagcaaagatcatcagggattatggaaaacagatggcaggtgatgattgtgtggcaagtagacaggatgaggattaacacatggaattctgcaacaactgctgtttatccatttcagaattgggtgtcgacatagcagaataggcgttactcgacagaggagagcaagaaatggagccagtagatcctagactagagccctggaagcatccaggaagtcagcctaaaactgcttgtaccaattgctattgtaaaaagtgttgctttcattgccaagtttgtttctgaacaaaagccttaggcatctcctatggcaggaagaagcggagacagcgacgaagagctcatcagaacagtcagactcatcaagcttctctatcaaagcagtaagtagtacatgtaatgcaacctataatagtagcaatagtagcattagtagtagcaataataatagcaatagttgtgtggtccatagtaatcatagaatataggaaaatggccgctgatcttcagacctggaggaggagatatgagggacaattggagaagtgaattatataaatataaagtagtaaaaattgaaccattaggagtagcacccaccaaggcaaagagaagagtggtgcagagagaaaaaagagcagtgggaataggagctttgttccttgggttcttgggagcagcaggaagcactatgggcgcagcgtcaatgacgctgacggtacaggccagacaattattgtctggtatagtgcagcagcagaacaatttgctgagggctattgaggcgcaacagcatctgttgcaactcacagtctggggcatcaagcagctccaggcaagaatcctggctgtggaaagatacctaaaggatcaacagctcctggggatttggggttgctctggaaaactcatttgcaccactgctgtgccttggaatgctagttggagtaataaatctctggaacagatttggaatcacacgacctggatggagtgggacagagaaattaacaattacacaagcttaatacactccttaattgaagaatcgcaaaaccagcaagaaaagaatgaacaagaattattggaattagataaatgggcaagtttgtggaattggtttaacataacaaattggctgtggtatataaaattattcataatgatagtaggaggcttggtaggtttaagaatagtttttgctgtactttctatagtgaatagagttaggcagggatattcaccattatcgtttcagacccacctcccaaccccgaggggacccgacaggcccgaaggaatagaagaagaaggtggagagagagacagagacagatccattcgattagtgaacggatccttggcacttatctgggacgatctgcggagcctgtgcctcttcagctaccaccgcttgagagacttactcttgattgtaacgaggattgtggaacttctgggacgcagggggtgggaagccctcaaatattggtggaatctcctacaatattggagtcaggagctaaagaatagtgctgttagcttgctcaatgccacagccatagcagtagctgaggggacagatagggttatagaagtagtacaaggagcttgtagagctattcgccacatacctagaagaataagacagggcttggaaaggattttgctataagctcgaaacaaccggtacctctagaactatagctagcagatctttttccctctgccaaaaattatggggacatcatgaagccccttgagcatctgacttctggctaataaaggaaatttattttcattgcaatagtgtgttggaattttttgtgtctctcactcggaaggacatatgggagggcaaatcatttaaaacatcagaatgagtatttggtttagagtttggcaacatatgcccatatgctggctgccatgaacaaaggttggctataaagaggtcatcagtatatgaaacagccccctgctgtccattccttattccatagaaaagccttgacttgaggttagattttttttatattttgttttgtgttatttttttctttaacatccctaaaattttccttacatgttttactagccagatttttcctcctctcctgactactcccagtcatagctgtccctcttctcttatggagatccctcgacctgcagcccaagcttggcgtaatcatggtcatagctgtttcctgtgtgaaattgttatccgctcacaattccacacaacatacgagccggaagcataaagtgtaaagcctggggtgcctaatgagtgagctaactcacattaattgcgttgcgctcactgcccgctttccagtcgggaaacctgtcgtgccagcggatccgcatctcaattagtcagcaaccatagtcccgcccctaactccgcccatcccgcccctaactccgcccagttccgcccattctccgccccatggctgactaattttttttatttatgcagaggccgaggccgcctcggcctctgagctattccagaagtagtgaggaggcttttttggaggcctaggcttttgcaaaaagctaacttgtttattgcagcttataatggttacaaataaagcaatagcatcacaaatttcacaaataaagcatttttttcactgcattctagttgtggtttgtccaaactcatcaatgtatcttatcatgtctggatccgctgcattaatgaatcggccaacgcgcggggagaggcggtttgcgtattgggcgctcttccgcttcctcgctcactgactcgctgcgctcggtcgttcggctgcggcgagcggtatcagctcactcaaaggcggtaatacggttatccacagaatcaggggataacgcaggaaagaacatgtgagcaaaaggccagcaaaaggccaggaaccgtaaaaaggccgcgttgctggcgtttttccataggctccgcccccctgacgagcatcacaaaaatcgacgctcaagtcagaggtggcgaaacccgacaggactataaagataccaggcgtttccccctggaagctccctcgtgcgctctcctgttccgaccctgccgcttaccggatacctgtccgcctttctcccttcgggaagcgtggcgctttctcatagctcacgctgtaggtatctcagttcggtgtaggtcgttcgctccaagctgggctgtgtgcacgaaccccccgttcagcccgaccgctgcgccttatccggtaactatcgtcttgagtccaacccggtaagacacgacttatcgccactggcagcagccactggtaacaggattagcagagcgaggtatgtaggcggtgctacagagttcttgaagtggtggcctaactacggctacactagaagaacagtatttggtatctgcgctctgctgaagccagttaccttcggaaaaagagttggtagctcttgatccggcaaacaaaccaccgctggtagcggtggtttttttgtttgcaagcagcagattacgcgcagaaaaaaaggatctcaagaagatcctttgatcttttctacggggtctgacgctcagtggaacgaaaactcacgttaagggattttggtcatgagattatcaaaaaggatcttcacctagatccttttaaattaaaaatgaagttttaaatcaatctaaagtatatatgagtaaacttggtctgacagttaccaatgcttaatcagtgaggcacctatctcagcgatctgtctatttcgttcatccatagttgcctgactccccgtcgtgtagataactacgatacgggagggcttaccatctggccccagtgctgcaatgataccgcgagacccacgctcaccggctccagatttatcagcaataaaccagccagccggaagggccgagcgcagaagtggtcctgcaactttatccgcctccatccagtctattaattgttgccgggaagctagagtaagtagttcgccagttaatagtttgcgcaacgttgttgccattgctacaggcatcgtggtgtcacgctcgtcgtttggtatggcttcattcagctccggttcccaacgatcaaggcgagttacatgatcccccatgttgtgcaaaaaagcggttagctccttcggtcctccgatcgttgtcagaagtaagttggccgcagtgttatcactcatggttatggcagcactgcataattctcttactgtcatgccatccgtaagatgcttttctgtgactggtgagtactcaaccaagtcattctgagaatagtgtatgcggcgaccgagttgctcttgcccggcgtcaatacgggataataccgcgccacatagcagaactttaaaagtgctcatcattggaaaacgttcttcggggcgaaaactctcaaggatcttaccgctgttgagatccagttcgatgtaacccactcgtgcacccaactgatcttcagcatcttttactttcaccagcgtttctgggtgagcaaaaacaggaaggcaaaatgccgcaaaaaagggaataagggcgacacggaaatgttgaatactcatactcttcctttttcaatattattgaagcatttatcagggttattgtctcatgagcggatacatatttgaatgtatttagaaaaataaacaaataggggttccgcgcacatttccccgaaaagtgccacctgggtcgacattgattattgactagttattaatagtaatcaattacggggtcattagttcatagcccatatatggagttccgcgttacataacttacggtaaatggcccgcctggctgaccgcccaacgacccccgcccattgacgtcaataatgacgtatgttcccatagtaacgccaatagggactttccattgacgtcaatgggtggagtatttacggtaaactgcccacttggcagtacatcaagtgtatcatatgccaagtacgccccctattgacgtcaatgacggtaaatggcccgcctggcattatgcccagtacatgaccttatgggactttcctacttggcagtacatctacgtattagtcatcgctattaccatggtcgaggtgagccccacgttctgcttcactctccccatctcccccccctccccacccccaattttgtatttatttattttttaattattttgtgcagggcgaggcggagaggtgcggcggcagccaatcagagcggcgcgctccgaaagtttccttttatggcgaggcggcggcggcggcggccctataaaaagcgaagcgcgcggcgggcgggagtcgctgcgcgctgccttcgccccgtgccccgctccgccgccgcctcgcgccgcccgccccggctctgactgaccgcgttactcccacaggtgagcgggcgggacggcccttctcctccgggctgtaattagcgcttggtttaatgacggcttgtttcttttctgtggctgcgtgaaagccttgaggggctccgggagggccctttgtgcggggggagcggctcggggggtgcgtgcgtgtgtgtgtgcgtggggagcgccgcgtgcggctccgcgctgcccggcggctgtgagcgctgcgggcgcggcgcggggctttgtgcgctccgcagtgtgcgcgaggggagcgcggccgggggcggtgccccgcggtgcggggggggctgcgaggggaacaaaggctgcgtgcggggtgtgtgcgtgggggggtgagcagggggtgtgggcgcgtcggtcgggctgcaaccccccctgcacccccctccccgagttgctgagcacggcccggcttcgggtgcggggctccgtacggggcgtggcgcggggctcgccgtgccgggcggggggtggcggcaggtgggggtgccgggcggggcggggccgcctcgggccggggagggctcgggggaggggcgcggcggcccccggagcgccggcggctgtcgaggcgcggcgagccgcagccattgccttttatggtaatcgtgcgagagggcgcagggacttcctttgtcccaaatctgtgcggagccgaaatctgggaggcgccgccgcaccccctctagcgggcgcggggcgaagcggtgcggcgccggcaggaaggaaatgggcggggagggccttcgtgcgtcgccgcgccgccgtccccttctccctctccagcctcggggctgtccgcggggggacggctgccttcgggggggacggggcagggcggggttcggcttctggcgtgtgaccggcggctctagagcctctgctaaccatgttcatgccttcttctttttcctacagctcctgggcaacgtgctggttattgtgctgtctcatcattttggcaaagaattcgggccgcgttgacgcgcacggcaagaggcgaggggcggcgactggtgagagatgggtgcgagagcgtcagtattaagcgggggagaattagatcgatgggaaaaaattcggttaaggccagggggaaagaaaaaatataaattaaaacatatagtatgggcaagcagggagctagaacgattcgcagttaatcctggcctgttagaaacatcagaaggctgtagacaaatactgggacagctacaaccatcccttcagacaggatcagaagaacttagatcattatataatacagtagcaaccctctattgtgtgcatcaaaggatagagataaaagacaccaaggaagctttagacaagatagaggaagagcaaaacaaaagtaagaaaaaagcacagcaagcagcagctgacacaggacacagcaatcaggtcagccaaaattaccctatagtgcagaacatccaggggcaaatggtacatcaggccatatcacctagaactttaaatgcatgggtaaaagtagtagaagagaaggctttcagcccagaagtgatacccatgttttcagcattatcagaaggagccaccccacaagatttaaacaccatgctaaacacagtggggggacatcaagcagccatgcaaatgttaaaagagaccatcaatgaggaagctgcagaatgggatagagtgcatccagtgcatgcagggcctattgcaccaggccagatgagagaaccaaggggaagtgacatagcaggaactactagtacccttcaggaacaaataggatggatgacacataatccacctatcccagtaggagaaatctataaaagatggataatcctgggattaaataaaatagtaagaatgtatagccctaccagcattctggacataagacaaggaccaaaggaaccctttagagactatgtagaccgattctataaaactctaagagccgagcaagcttcacaagaggtaaaaaattggatgacaga

SEQ ID NO: 269 - DNA, 10644 bp, Synthetic construct
  source 1..10644: mol_type = other DNA
aaccttgttggtccaaaatgcgaacccagattgtaagactattttaaaagcattgggaccaggagcgacactagaagaaatgatgacagcatgtcagggagtggggggacccggccataaagcaagagttttggctgaagcaatgagccaagtaacaaatccagctaccataatgatacagaaaggcaattttaggaaccaaagaaagactgttaagtgtttcaattgtggcaaagaagggcacatagccaaaaattgcagggcccctaggaaaaagggctgttggaaatgtggaaaggaaggacaccaaatgaaagattgtactgagagacaggctaattttttagggaagatctggccttcccacaagggaaggccagggaattttcttcagagcagaccagagccaacagccccaccagaagagagcttcaggtttggggaagagacaacaactccctctcagaagcaggagccgatagacaaggaactgtatcctttagcttccctcagatcactctttggcagcgacccctcgtcacaataaagataggggggcaattaaaggaagctctattagatacaggagcagatgatacagtattagaagaaatgaatttgccaggaagatggaaaccaaaaatgatagggggaattggaggttttatcaaagtaagacagtatgatcagatactcatagaaatctgcggacataaagctataggtacagtattagtaggacctacacctgtcaacataattggaagaaatctgttgactcagattggctgcactttaaattttcccattagtcctattgagactgtaccagtaaaattaaagccaggaatggatggcccaaaagttaaacaatggccattgacagaagaaaaaataaaagcattagtagaaatttgtacagaaatggaaaaggaaggaaaaatttcaaaaattgggcctgaaaatccatacaatactccagtatttgccataaagaaaaaagacagtactaaatggagaaaattagtagatttcagagaacttaataagagaactcaagatttctgggaagttcaattaggaataccacatcctgcagggttaaaacagaaaaaatcagtaacagtactggatgtgggcgatgcatatttttcagttcccttagataaagacttcaggaagtatactgcatttaccatacctagtataaacaatgagacaccagggattagatatcagtacaatgtgcttccacagggatggaaaggatcaccagcaatattccagtgtagcatgacaaaaatcttagagccttttagaaaacaaaatccagacatagtcatctatcaatacatggatgatttgtatgtaggatctgacttagaaatagggcagcatagaacaaaaatagaggaactgagacaacatctgttgaggtggggatttaccacaccagacaaaaaacatcagaaagaacctccattcctttggatgggttatgaactccatcctgataaatggacagtacagcctatagtgctgccagaaaaggacagctggactgtcaatgacatacagaaattagtgggaaaattgaattgggcaagtcagatttatgcagggattaaagtaaggcaattatgtaaacttcttaggggaaccaaagcactaacagaagtagtaccactaacagaagaagcagagctagaactggcagaaaacagggagattctaaaagaaccggtacatggagtgtattatgacccatcaaaagacttaatagcagaaatacagaagcaggggcaaggccaatggacatatcaaatttatcaagagccatttaaaaatctgaaaacaggaaagtatgcaagaatgaagggtgcccacactaatgatgtgaaacaattaacagaggcagtacaaaaaatagccacagaaagcatagtaatatggggaaagactcctaaatttaaattacccatacaaaaggaaacatgggaagcatggtggacagagtattggcaagccacctggattcctgagtgggagtttgtcaatacccctcccttagtgaagttatggtaccagttagagaaagaacccataataggagcagaaactttctatgtagatggggcagccaatagggaaactaaattaggaaaagcaggatatgtaactgacagaggaagacaaaaagttgtccccctaacggacacaacaaatcagaagactgagttacaagcaattcatctagctttgcaggattcgggattagaagtaaacatagtgacagactcacaatatgcattgggaatcattcaagcacaaccagataagagtgaatcagagttagtcagtcaaataatagagcagttaataaaaaaggaaaaagtctacctggcatgggtaccagcacacaaaggaattggaggaaatgaacaagtagataaattggtcagtgctggaatcaggaaagtactatttttagatggaatagataaggcccaagaagaacatgagaaatatcacagtaattggagagcaatggctagtgattttaacctaccacctgtagtagcaaaagaaatagtagccagctgtgataaatgtcagctaaaaggggaagccatgcatggacaagtagactgtagcccaggaatatggcagctagtttgtacacatttagaaggaaaagttatcttggtagcagttcatgtagccagtggatatatagaagcagaagtaattccagcagagacagggcaagaaacagcatacttcctcttaaaattagcaggaagatggccagtaaaaacagtacatacagacaatggcagcaatttcaccagtactacagttaaggccgcctgttggtgggcggggatcaagcaggaatttggcattccctacaatccccaaagtcaaggagtaatagaatctatgaataaagaattaaagaaaattataggacaggtaagagatcaggctgaacatcttaagacagcagtacaaatggcagtattcatccacaattttaaaagaaaaggggggattggggggtacagtgcaggggaaagaatagtagacataatagcaacagacatacaaactaaagaattacaaaaacaaattacaaaaattcaaaattttcgggtttattacagggacagcagagatccagtttggaaaggaccagcaaagctcctctggaaaggtgaaggggcagtagtaatacaagataatagtgacataaaagtagtgccaagaagaaaagcaaagatcatcagggattatggaaaacagatggcaggtgatgattgtgtggcaagtagacaggatgaggattaacacatggaattctgcaacaactgctgtttatccatttcagaattgggtgtcgacatagcagaataggcgttactcgacagaggagagcaagaaatggagccagtagatcctagactagagccctggaagcatccaggaagtcagcctaaaactgcttgtaccaattgctattgtaaaaagtgttgctttcattgccaagtttgtttcatgacaaaagccttaggcatctcctatggcaggaagaagcggagacagcgacgaagagctcatcagaacagtcagactcatcaagcttctctatcaaagcagtaagtagtacatgtaatgcaacctataatagtagcaatagtagcattagtagtagcaataataatagcaatagttgtgtggtccatagtaatcatagaatataggaaaatggccgctgatcttcagacctggaggaggagatatgagggacaattggagaagtgaattatataaatataaagtagtaaaaattgaaccattaggagtagcacccaccaaggcaaagagaagagtggtgcagagagaaaaaagagcagtgggaataggagctttgttccttgggttcttgggagcagcaggaagcactatgggcgcagcgtcaatgacgctgacggtacaggccagacaattattgtctggtatagtgcagcagcagaacaatttgctgagggctattgaggcgcaacagcatctgttgcaactcacagtctggggcatcaagcagctccaggcaagaatcctggctgtggaaagatacctaaaggatcaacagctcctggggatttggggttgctctggaaaactcatttgcaccactgctgtgccttggaatgctagttggagtaataaatctctggaacagatttggaatcacacgacctggatggagtgggacagagaaattaacaattacacaagcttaatacactccttaattgaagaatcgcaaaaccagcaagaaaagaatgaacaagaattattggaattagataaatgggcaagtttgtggaattggtttaacataacaaattggctgtggtatataaaattattcataatgatagtaggaggcttggtaggtttaagaatagtttttgctgtactttctatagtgaatagagttaggcagggatattcaccattatcgtttcagacccacctcccaaccccgaggggacccgacaggcccgaaggaatagatgaagaaggtggagagagagacagagacagatccattcgattagtgaacggatccttggcacttatctgggacgatctgcggagcctgtgcctcttcagctaccaccgcttgagagacttactcttgattgtaacgaggattgtggaacttctgggacgcagggggtgggaagccctcaaatattggtggaatctcctacaatattggagtcaggagctaaagaatagtgctgttagcttgctcaatgccacagccatagcagtagctgaggggacagatagggttatagaagtagtacaaggagcttgtagagctattcgccacatacctagaagaataagacagggcttggaaaggattttgctataagctcgaaacaaccggtacctctagaactatagctagcagatctttttccctctgccaaaaattatggggacatcatgaagccccttgagcatctgacttctggctaataaaggaaatttattttcattgcaatagtgtgttggaattttttgtgtctctcactcggaaggacatatgggagggcaaatcatttaaaacatcagaatgagtatttggtttagagtttggcaacatatgcccatatgctggctgccatgaacaaaggttggctataaagaggtcatcagtatatgaaacagccccctgctgtccattccttattccatagaaaagccttgacttgaggttagattttttttatattttgttttgtgttatttttttctttaacatccctaaaattttccttacatgttttactagccagatttttcctcctctcctgactactcccagtcatagctgtccctcttctcttatggagatccctcgacctgcagcccaagcttggcgtaatcatggtcatagctgtttcctgtgtgaaattgttatccgctcacaattccacacaacatacgagccggaagcataaagtgtaaagcctggggtgcctaatgagtgagctaactcacattaattgcgttgcgctcactgcccgctttccagtcgggaaacctgtcgtgccagcggatccgcatctcaattagtcagcaaccatagtcccgcccctaactccgcccatcccgcccctaactccgcccagttccgcccattctccgccccatggctgactaattttttttatttatgcagaggccgaggccgcctcggcctctgagctattccagaagtagtgaggaggcttttttggaggcctaggcttttgcaaaaagctaacttgtttattgcagcttataatggttacaaataaagcaatagcatcacaaatttcacaaataaagcatttttttcactgcattctagttgtggtttgtccaaactcatcaatgtatcttatcatgtctggatccgctgcattaatgaatcggccaacgcgcggggagaggcggtttgcgtattgggcgctcttccgcttcctcgctcactgactcgctgcgctcggtcgttcggctgcggcgagcggtatcagctcactcaaaggcggtaatacggttatccacagaatcaggggataacgcaggaaagaacatgtgagcaaaaggccagcaaaaggccaggaaccgtaaaaaggccgcgttgctggcgtttttccataggctccgcccccctgacgagcatcacaaaaatcgacgctcaagtcagaggtggcgaaacccgacaggactataaagataccaggcgtttccccctggaagctccctcgtgcgctctcctgttccgaccctgccgcttaccggatacctgtccgcctttctcccttcgggaagcgtggcgctttctcatagctcacgctgtaggtatctcagttcggtgtaggtcgttcgctccaagctgggctgtgtgcacgaaccccccgttcagcccgaccgctgcgccttatccggtaactatcgtcttgagtccaacccggtaagacacgacttatcgccactggcagcagccactggtaacaggattagcagagcgaggtatgtaggcggtgctacagagttcttgaagtggtggcctaactacggctacactagaagaacagtatttggtatctgcgctctgctgaagccagttaccttcggaaaaagagttggtagctcttgatccggcaaacaaaccaccgctggtagcggtggtttttttgtttgcaagcagcagattacgcgcagaaaaaaaggatctcaagaagatcctttgatcttttctacggggtctgacgctcagtggaacgaaaactcacgttaagggattttggtcatgagattatcaaaaaggatcttcacctagatccttttaaattaaaaatgaagttttaaatcaatctaaagtatatatgagtaaacttggtctgacagttaccaatgcttaatcagtgaggcacctatctcagcgatctgtctatttcgttcatccatagttgcctgactccccgtcgtgtagataactacgatacgggagggcttaccatctggccccagtgctgcaatgataccgcgagacccacgctcaccggctccagatttatcagcaataaaccagccagccggaagggccgagcgcagaagtggtcctgcaactttatccgcctccatccagtctattaattgttgccgggaagctagagtaagtagttcgccagttaatagtttgcgcaacgttgttgccattgctacaggcatcgtggtgtcacgctcgtcgtttggtatggcttcattcagctccggttcccaacgatcaaggcgagttacatgatcccccatgttgtgcaaaaaagcggttagctccttcggtcctccgatcgttgtcagaagtaagttggccgcagtgttatcactcatggttatggcagcactgcataattctcttactgtcatgccatccgtaagatgcttttctgtgactggtgagtactcaaccaagtcattctgagaatagtgtatgcggcgaccgagttgctcttgcccggcgtcaatacgggataataccgcgccacatagcagaactttaaaagtgctcatcattggaaaacgttcttcggggcgaaaactctcaaggatcttaccgctgttgagatccagttcgatgtaacccactcgtgcacccaactgatcttcagcatcttttactttcaccagcgtttctgggtgagcaaaaacaggaaggcaaaatgccgcaaaaaagggaataagggcgacacggaaatgttgaatactcatactcttcctttttcaatattattgaagcatttatcagggttattgtctcatgagcggatacatatttgaatgtatttagaaaaataaacaaataggggttccgcgcacatttccccgaaaagtgccacctgggtcgacattgattattgactagttattaatagtaatcaattacggggtcattagttcatagcccatatatggagttccgcgttacataacttacggtaaatggcccgcctggctgaccgcccaacgacccccgcccattgacgtcaataatgacgtatgttcccatagtaacgccaatagggactttccattgacgtcaatgggtggagtatttacggtaaactgcccacttggcagtacatcaagtgtatcatatgccaagtacgccccctattgacgtcaatgacggtaaatggcccgcctggcattatgcccagtacatgaccttatgggactttcctacttggcagtacatctacgtattagtcatcgctattaccatggtcgaggtgagccccacgttctgcttcactctccccatctcccccccctccccacccccaattttgtatttatttattttttaattattttgtgcagggcgaggcggagaggtgcggcggcagccaatcagagcggcgcgctccgaaagtttccttttatggcgaggcggcggcggcggcggccctataaaaagcgaagcgcgcggcgggcgggagtcgctgcgcgctgccttcgccccgtgccccgctccgccgccgcctcgcgccgcccgccccggctctgactgaccgcgttactcccacaggtgagcgggcgggacggcccttctcctccgggctgtaattagcgcttggtttaatgacggcttgtttcttttctgtggctgcgtgaaagccttgaggggctccgggagggccctttgtgcggggggagcggctcggggggtgcgtgcgtgtgtgtgtgcgtggggagcgccgcgtgcggctccgcgctgcccggcggctgtgagcgctgcgggcgcggcgcggggctttgtgcgctccgcagtgtgcgcgaggggagcgcggccgggggcggtgccccgcggtgcggggggggctgcgaggggaacaaaggctgcgtgcggggtgtgtgcgtgggggggtgagcagggggtgtgggcgcgtcggtcgggctgcaaccccccctgcacccccctccccgagttgctgagcacggcccggcttcgggtgcggggctccgtacggggcgtggcgcggggctcgccgtgccgggcggggggtggcggcaggtgggggtgccgggcggggcggggccgcctcgggccggggagggctcgggggaggggcgcggcggcccccggagcgccggcggctgtcgaggcgcggcgagccgcagccattgccttttatggtaatcgtgcgagagggcgcagggacttcctttgtcccaaatctgtgcggagccgaaatctgggaggcgccgccgcaccccctctagcgggcgcggggcgaagcggtgcggcgccggcaggaaggaaatgggcggggagggccttcgtgcgtcgccgcgccgccgtccccttctccctctccagcctcggggctgtccgcggggggacggctgccttcgggggggacggggcagggcggggttcggcttctggcgtgtgaccggcggctctagagcctctgctaaccatgttcatgccttcttctttttcctacagctcctgggcaacgtgctggttattgtgctgtctcatcattttggcaaagaattcgggccgcgttgacgcgcacggcaagaggcgaggggcggcgactggtgagagatgggtgcgagagcgtcagtattaagcgggggagaattagatcgatgggaaaaaattcggttaaggccagggggaaagaaaaaatataaattaaaacatatagtatgggcaagcagggagctagaacgattcgcagttaatcctggcctgttagaaacatcagaaggctgtagacaaatactgggacagctacaaccatcccttcagacaggatcagaagaacttagatcattatataatacagtagcaaccctctattgtgtgcatcaaaggatagagataaaagacaccaaggaagctttagacaagatagaggaagagcaaaacaaaagtaagaaaaaagcacagcaagcagcagctgacacaggacacagcaatcaggtcagccaaaattaccctatagtgcagaacatccaggggcaaatggtacatcaggccatatcacctagaactttaaatgcatgggtaaaagtagtagaagagaaggctttcagcccagaagtgatacccatgttttcagcattatcagaaggagccaccccacaagatttaaacaccatgctaaacacagtggggggacatcaagcagccatgcaaatgttaaaagagaccatcaatgaggaagctgcagaatgggatagagtgcatccagtgcatgcagggcctattgcaccaggccagatgagagaaccaaggggaagtgacatagcaggaactactagtacccttcaggaacaaataggatggatgacacataatccacctatcccagtaggagaaatctataaaagatggataatcctgggattaaataaaatagtaagaatgtatagccctaccagcattctggacataagacaaggaccaaaggaaccctttagagactatgtagaccgattctataaaactctaagagccgagcaagcttcacaagaggtaaaaaattggatgacaga

SEQ ID NO: 270 - DNA, 10644 bp, Synthetic construct
  source 1..10644: mol_type = other DNA
ccgaaaagtgccacctgggtcgacattgattattgactagttattaatagtaatcaattacggggtcattagttcatagcccatatatggagttccgcgttacataacttacggtaaatggcccgcctggctgaccgcccaacgacccccgcccattgacgtcaataatgacgtatgttcccatagtaacgccaatagggactttccattgacgtcaatgggtggagtatttacggtaaactgcccacttggcagtacatcaagtgtatcatatgccaagtacgccccctattgacgtcaatgacggtaaatggcccgcctggcattatgcccagtacatgaccttatgggactttcctacttggcagtacatctacgtattagtcatcgctattaccatggtcgaggtgagccccacgttctgcttcactctccccatctcccccccctccccacccccaattttgtatttatttattttttaattattttgtgcagggcgaggcggagaggtgcggcggcagccaatcagagcggcgcgctccgaaagtttccttttatggcgaggcggcggcggcggcggccctataaaaagcgaagcgcgcggcgggcgggagtcgctgcgcgctgccttcgccccgtgccccgctccgccgccgcctcgcgccgcccgccccggctctgactgaccgcgttactcccacaggtgagcgggcgggacggcccttctcctccgggctgtaattagcgcttggtttaatgacggcttgtttcttttctgtggctgcgtgaaagccttgaggggctccgggagggccctttgtgcggggggagcggctcggggggtgcgtgcgtgtgtgtgtgcgtggggagcgccgcgtgcggctccgcgctgcccggcggctgtgagcgctgcgggcgcggcgcggggctttgtgcgctccgcagtgtgcgcgaggggagcgcggccgggggcggtgccccgcggtgcggggggggctgcgaggggaacaaaggctgcgtgcggggtgtgtgcgtgggggggtgagcagggggtgtgggcgcgtcggtcgggctgcaaccccccctgcacccccctccccgagttgctgagcacggcccggcttcgggtgcggggctccgtacggggcgtggcgcggggctcgccgtgccgggcggggggtggcggcaggtgggggtgccgggcggggcggggccgcctcgggccggggagggctcgggggaggggcgcggcggcccccggagcgccggcggctgtcgaggcgcggcgagccgcagccattgccttttatggtaatcgtgcgagagggcgcagggacttcctttgtcccaaatctgtgcggagccgaaatctgggaggcgccgccgcaccccctctagcgggcgcggggcgaagcggtgcggcgccggcaggaaggaaatgggcggggagggccttcgtgcgtcgccgcgccgccgtccccttctccctctccagcctcggggctgtccgcggggggacggctgccttcgggggggacggggcagggcggggttcggcttctggcgtgtgaccggcggctctagagcctctgctaaccatgttcatgccttcttctttttcctacagctcctgggcaacgtgctggttattgtgctgtctcatcattttggcaaagaattcgggccgcgttgacgcgcacggcaagaggcgaggggcggcgactggtgagagatgggtgcgagagcgtcagtattaagcgggggagaattagatcgatgggaaaaaattcggttaaggccagggggaaagaaaaaatataaattaaaacatatagtatgggcaagcagggagctagaacgattcgcagttaatcctggcctgttagaaacatcagaaggctgtagacaaatactgggacagctacaaccatcccttcagacaggatcagaagaacttagatcattatataatacagtagcaaccctctattgtgtgcatcaaaggatagagataaaagacaccaaggaagctttagacaagatagaggaagagcaaaacaaaagtaagaaaaaagcacagcaagcagcagctgacacaggacacagcaatcaggtcagccaaaattaccctatagtgcagaacatccaggggcaaatggtacatcaggccatatcacctagaactttaaatgcatgggtaaaagtagtagaagagaaggctttcagcccagaagtgatacccatgttttcagcattatcagaaggagccaccccacaagatttaaacaccatgctaaacacagtggggggacatcaagcagccatgcaaatgttaaaagagaccatcaatgaggaagctgcagaatgggatagagtgcatccagtgcatgcagggcctattgcaccaggccagatgagagaaccaaggggaagtgacatagcaggaactactagtacccttcaggaacaaataggatggatgacacataatccacctatcccagtaggagaaatctataaaagatggataatcctgggattaaataaaatagtaagaatgtatagccctaccagcattctggacataagacaaggaccaaaggaaccctttagagactatgtagaccgattctataaaactctaagagccgagcaagcttcacaagaggtaaaaaattggatgacagaaaccttgttggtccaaaatgcgaacccagattgtaagactattttaaaagcattgggaccaggagcgacactagaagaaatgatgacagcatgtcagggagtggggggacccggccataaagcaagagttttggctgaagcaatgagccaagtaacaaatccagctaccataatgatacagaaaggcaattttaggaaccaaagaaagactgttaagtgtttcaattgtggcaaagaagggcacatagccaaaaattgcagggcccctaggaaaaagggctgttggaaatgtggaaaggaaggacaccaaatgaaagattgtactgagagacaggctaattttttagggaagatctggccttcccacaagggaaggccagggaattttcttcagagcagaccagagccaacagccccaccagaagagagcttcaggtttggggaagagacaacaactccctctcagaagcaggagccgatagacaaggaactgtatcctttagcttccctcagatcactctttggcagcgacccctcgtcacaataaagataggggggcaattaaaggaagctctattagcgacaggagcagatgatacagtattagaagaaatgaatttgccaggaagatggaaaccaaaaatgatagggggaattggaggttttatcaaagtaagacagtatgatcagatactcatagaaatctgcggacataaagctataggtacagtattagtaggacctacacctgtcaacataattggaagaaatctgttgactcagattggctgcactttaaattttcccattagtcctattgagactgtaccagtaaaattaaagccaggaatggatggcccaaaagttaaacaatggccattgacagaagaaaaaataaaagcattagtagaaatttgtacagaaatggaaaaggaaggaaaaatttcaaaaattgggcctgaaaatccatacaatactccagtatttgccataaagaaaaaagacagtactaaatggagaaaattagtagatttcagagaacttaataagagaactcaagatttctgggaagttcaattaggaataccacatcctgcagggttaaaacagaaaaaatcagtaacagtactggatgtgggcgatgcatatttttcagttcccttagataaagacttcaggaagtatactgcatttaccatacctagtataaacaatgagacaccagggattagatatcagtacaatgtgcttccacagggatggaaaggatcaccagcaatattccagtgtagcatgacaaaaatcttagagccttttagaaaacaaaatccagacatagtcatctatcaatacatggatgatttgtatgtaggatctgacttagaaatagggcagcatagaacaaaaatagaggaactgagacaacatctgttgaggtggggatttaccacaccagacaaaaaacatcagaaagaacctccattcctttggatgggttatgaactccatcctgataaatggacagtacagcctatagtgctgccagaaaaggacagctggactgtcaatgacatacagaaattagtgggaaaattgaattgggcaagtcagatttatgcagggattaaagtaaggcaattatgtaaacttcttaggggaaccaaagcactaacagaagtagtaccactaacagaagaagcagagctagaactggcagaaaacagggagattctaaaagaaccggtacatggagtgtattatgacccatcaaaagacttaatagcagaaatacagaagcaggggcaaggccaatggacatatcaaatttatcaagagccatttaaaaatctgaaaacaggaaagtatgcaagaatgaagggtgcccacactaatgatgtgaaacaattaacagaggcagtacaaaaaatagccacagaaagcatagtaatatggggaaagactcctaaatttaaattacccatacaaaaggaaacatgggaagcatggtggacagagtattggcaagccacctggattcctgagtgggagtttgtcaatacccctcccttagtgaagttatggtaccagttagagaaagaacccataataggagcagaaactttctatgtagatggggcagccaatagggaaactaaattaggaaaagcaggatatgtaactgacagaggaagacaaaaagttgtccccctaacggacacaacaaatcagaagactgagttacaagcaattcatctagctttgcaggattcgggattagaagtaaacatagtgacagactcacaatatgcattgggaatcattcaagcacaaccagataagagtgaatcagagttagtcagtcaaataatagagcagttaataaaaaaggaaaaagtctacctggcatgggtaccagcacacaaaggaattggaggaaatgaacaagtagataaattggtcagtgctggaatcaggaaagtactatttttagatggaatagataaggcccaagaagaacatgagaaatatcacagtaattggagagcaatggctagtgattttaacctaccacctgtagtagcaaaagaaatagtagccagctgtgataaatgtcagctaaaaggggaagccatgcatggacaagtagactgtagcccaggaatatggcagctagtttgtacacatttagaaggaaaagttatcttggtagcagttcatgtagccagtggatatatagaagcagaagtaattccagcagagacagggcaagaaacagcatacttcctcttaaaattagcaggaagatggccagtaaaaacagtacatacagacaatggcagcaatttcaccagtactacagttaaggccgcctgttggtgggcggggatcaagcaggaatttggcattccctacaatccccaaagtcaaggagtaatagaatctatgaataaagaattaaagaaaattataggacaggtaagagatcaggctgaacatcttaagacagcagtacaaatggcagtattcatccacaattttaaaagaaaaggggggattggggggtacagtgcaggggaaagaatagtagacataatagcaacagacatacaaactaaagaattacaaaaacaaattacaaaaattcaaaattttcgggtttattacagggacagcagagatccagtttggaaaggaccagcaaagctcctctggaaaggtgaaggggcagtagtaatacaagataatagtgacataaaagtagtgccaagaagaaaagcaaagatcatcagggattatggaaaacagatggcaggtgatgattgtgtggcaagtagacaggatgaggattaacacatggaattctgcaacaactgctgtttatccatttcagaattgggtgtcgacatagcagaataggcgttactcgacagaggagagcaagaaatggagccagtagatcctagactagagccctggaagcatccaggaagtcagcctaaaactgcttgtaccaattgctattgtaaaaagtgttgctttcattgccaagtttgtttcatgacaaaagccttaggcatctcctatggcaggaagaagcggagacagcgacgaagagctcatcagaacagtcagactcatcaagcttctctatcaaagcagtaagtagtacatgtaatgcaacctataatagtagcaatagtagcattagtagtagcaataataatagcaatagttgtgtggtccatagtaatcatagaatataggaaaatggccgctgatcttcagacctggaggaggagatatgagggacaattggagaagtgaattatataaatataaagtagtaaaaattgaaccattaggagtagcacccaccaaggcaaagagaagagtggtgcagagagaaaaaagagcagtgggaataggagctttgttccttgggttcttgggagcagcaggaagcactatgggcgcagcgtcaatgacgctgacggtacaggccagacaattattgtctggtatagtgcagcagcagaacaatttgctgagggctattgaggcgcaacagcatctgttgcaactcacagtctggggcatcaagcagctccaggcaagaatcctggctgtggaaagatacctaaaggatcaacagctcctggggatttggggttgctctggaaaactcatttgcaccactgctgtgccttggaatgctagttggagtaataaatctctggaacagatttggaatcacacgacctggatggagtgggacagagaaattaacaattacacaagcttaatacactccttaattgaagaatcgcaaaaccagcaagaaaagaatgaacaagaattattggaattagataaatgggcaagtttgtggaattggtttaacataacaaattggctgtggtatataaaattattcataatgatagtaggaggcttggtaggtttaagaatagtttttgctgtactttctatagtgaatagagttaggcagggatattcaccattatcgtttcagacccacctcccaaccccgaggggacccgacaggcccgaaggaatagaagaagaaggtggagagagagacagagacagatccattcgattagtgaacggatccttggcacttatctgggacgatctgcggagcctgtgcctcttcagctaccaccgcttgagagacttactcttgattgtaacgaggattgtggaacttctgggacgcagggggtgggaagccctcaaatattggtggaatctcctacaatattggagtcaggagctaaagaatagtgctgttagcttgctcaatgccacagccatagcagtagctgaggggacagatagggttatagaagtagtacaaggagcttgtagagctattcgccacatacctagaagaataagacagggcttggaaaggattttgctataagctcgaaacaaccggtacctctagaactatagctagcagatctttttccctctgccaaaaattatggggacatcatgaagccccttgagcatctgacttctggctaataaaggaaatttattttcattgcaatagtgtgttggaattttttgtgtctctcactcggaaggacatatgggagggcaaatcatttaaaacatcagaatgagtatttggtttagagtttggcaacatatgcccatatgctggctgccatgaacaaaggttggctataaagaggtcatcagtatatgaaacagccccctgctgtccattccttattccatagaaaagccttgacttgaggttagattttttttatattttgttttgtgttatttttttctttaacatccctaaaattttccttacatgttttactagccagatttttcctcctctcctgactactcccagtcatagctgtccctcttctcttatggagatccctcgacctgcagcccaagcttggcgtaatcatggtcatagctgtttcctgtgtgaaattgttatccgctcacaattccacacaacatacgagccggaagcataaagtgtaaagcctggggtgcctaatgagtgagctaactcacattaattgcgttgcgctcactgcccgctttccagtcgggaaacctgtcgtgccagcggatccgcatctcaattagtcagcaaccatagtcccgcccctaactccgcccatcccgcccctaactccgcccagttccgcccattctccgccccatggctgactaattttttttatttatgcagaggccgaggccgcctcggcctctgagctattccagaagtagtgaggaggcttttttggaggcctaggcttttgcaaaaagctaacttgtttattgcagcttataatggttacaaataaagcaatagcatcacaaatttcacaaataaagcatttttttcactgcattctagttgtggtttgtccaaactcatcaatgtatcttatcatgtctggatccgctgcattaatgaatcggccaacgcgcggggagaggcggtttgcgtattgggcgctcttccgcttcctcgctcactgactcgctgcgctcggtcgttcggctgcggcgagcggtatcagctcactcaaaggcggtaatacggttatccacagaatcaggggataacgcaggaaagaacatgtgagcaaaaggccagcaaaaggccaggaaccgtaaaaaggccgcgttgctggcgtttttccataggctccgcccccctgacgagcatcacaaaaatcgacgctcaagtcagaggtggcgaaacccgacaggactataaagataccaggcgtttccccctggaagctccctcgtgcgctctcctgttccgaccctgccgcttaccggatacctgtccgcctttctcccttcgggaagcgtggcgctttctcatagctcacgctgtaggtatctcagttcggtgtaggtcgttcgctccaagctgggctgtgtgcacgaaccccccgttcagcccgaccgctgcgccttatccggtaactatcgtcttgagtccaacccggtaagacacgacttatcgccactggcagcagccactggtaacaggattagcagagcgaggtatgtaggcggtgctacagagttcttgaagtggtggcctaactacggctacactagaagaacagtatttggtatctgcgctctgctgaagccagttaccttcggaaaaagagttggtagctcttgatccggcaaacaaaccaccgctggtagcggtggtttttttgtttgcaagcagcagattacgcgcagaaaaaaaggatctcaagaagatcctttgatcttttctacggggtctgacgctcagtggaacgaaaactcacgttaagggattttggtcatgagattatcaaaaaggatcttcacctagatccttttaaattaaaaatgaagttttaaatcaatctaaagtatatatgagtaaacttggtctgacagttaccaatgcttaatcagtgaggcacctatctcagcgatctgtctatttcgttcatccatagttgcctgactccccgtcgtgtagataactacgatacgggagggcttaccatctggccccagtgctgcaatgataccgcgagacccacgctcaccggctccagatttatcagcaataaaccagccagccggaagggccgagcgcagaagtggtcctgcaactttatccgcctccatccagtctattaattgttgccgggaagctagagtaagtagttcgccagttaatagtttgcgcaacgttgttgccattgctacaggcatcgtggtgtcacgctcgtcgtttggtatggcttcattcagctccggttcccaacgatcaaggcgagttacatgatcccccatgttgtgcaaaaaagcggttagctccttcggtcctccgatcgttgtcagaagtaagttggccgcagtgttatcactcatggttatggcagcactgcataattctcttactgtcatgccatccgtaagatgcttttctgtgactggtgagtactcaaccaagtcattctgagaatagtgtatgcggcgaccgagttgctcttgcccggcgtcaatacgggataataccgcgccacatagcagaactttaaaagtgctcatcattggaaaacgttcttcggggcgaaaactctcaaggatcttaccgctgttgagatccagttcgatgtaacccactcgtgcacccaactgatcttcagcatcttttactttcaccagcgtttctgggtgagcaaaaacaggaaggcaaaatgccgcaaaaaagggaataagggcgacacggaaatgttgaatactcatactcttcctttttcaatattattgaagcatttatcagggttattgtctcatgagcggatacatatttgaatgtatttagaaaaataaacaaataggggttccgcgcacatttcc

SEQ ID NO: 271 - DNA, 3452 bp, Synthetic construct
  source 1..3452: mol_type = other DNA
ataaaacctgcaggcatgcaagcgatcgcggggccgcccccttcaccgagggcctatttcccatgattccttcatatttgcatatacgatacaaggctgttagagagataattggaattaatttgactgtaaacacaaagatattagtacaaaatacgtgacgtagaaagtaataatttcttgggtagtttgcagttttaaaattatgttttaaaatggactatcatatgcttaccgtaacttgaaagtatttcgatttcttggctttatatatcttgtggaaaggacgaaacaccgggcgaagcaggccacgccggtttcagagctatgctggaaacagcatagcaagttgaaataaggctagtccgttatcaacttgaaaaagtggcaccgagtcggtgctgtgaccaccttaggctacggcgtggcctgcttccaattccgaccagaagatatggcttcggttggaattgttgacgcggttctatctagttacgcgttaaaccaactagaaattttttactagttctagagcggccccaattcgccctatagtgagtcgtattacgcgcgctcactggccgtcgttttacaacgtcgtgactgggaaaaccctggcgttacccaacttaatcgccttgcagcacatccccctttcgccagctggcgtaatagcgaagaggcccgcaccgatcgcccttcccaacagttgcgcagcctgaatggcgaatgggacgcgccctgtagcggcgcattaagcgcggcgggtgtggtggttacgcgcagcgtgaccgctacacttgccagcgccctagcgcccgctcctttcgctttcttcccttcctttctcgccacgttcgccggctttccccgtcaagctctaaatcgggggctccctttagggttccgatttagtgctttacggcacctcgaccccaaaaaacttgattagggtgatggttcacgtagtgggccatcgccctgatagacggtttttcgccctttgacgttggagtccacgttctttaatagtggactcttgttccaaactggaacaacactcaaccctatctcggtctattcttttgatttataagggattttgccgatttcggcctattggttaaaaaatgagctgatttaacaaaaatttaacgcgaattttaacaaaatattaacgcttacaatttaggtggcacttttcggggaaatgtgcgcggaacccctatttgtttatttttctaaatacattcaaatatgtatccgctcatgagacaataaccctgataaatgcttcaataatattgaaaaaggaagagtatgagtattcaacatttccgtgtcgcccttattcccttttttgcggcattttgccttcctgtttttgctcacccagaaacgctggtgaaagtaaaagatgctgaagatcagttgggtgcacgagtgggttacatcgaactggatctcaacagcggtaagatccttgagagttttcgccccgaagaacgttttccaatgatgagcacttttaaagttctgctatgtggcgcggtattatcccgtattgacgccgggcaagagcaactcggtcgccgcatacactattctcagaatgacttggttgagtactcaccagtcacagaaaagcatcttacggatggcatgacagtaagagaattatgcagtgctgccataaccatgagtgataacactgcggccaacttacttctgacaacgatcggaggaccgaaggagctaaccgcttttttgcacaacatgggggatcatgtaactcgccttgatcgttgggaaccggagctgaatgaagccataccaaacgacgagcgtgacaccacgatgcctgtagcaatggcaacaacgttgcgcaaactattaactggcgaactacttactctagcttcccggcaacaattaatagactggatggaggcggataaagttgcaggaccacttctgcgctcggcccttccggctggctggtttattgctgataaatctggagccggtgagcgtgggtctcgcggtatcattgcagcactggggccagatggtaagccctcccgtatcgtagttatctacacgacggggagtcaggcaactatggatgaacgaaatagacagatcgctgagataggtgcctcactgattaagcattggtaactgtcagaccaagtttactcatatatactttagattgatttaaaacttcatttttaatttaaaaggatctaggtgaagatcctttttgataatctcatgaccaaaatcccttaacgtgagttttcgttccactgagcgtcagaccccgtagaaaagatcaaaggatcttcttgagatcctttttttctgcgcgtaatctgctgcttgcaaacaaaaaaaccaccgctaccagcggtggtttgtttgccggatcaagagctaccaactctttttccgaaggtaactggcttcagcagagcgcagataccaaatactgtccttctagtgtagccgtagttaggccaccacttcaagaactctgtagcaccgcctacatacctcgctctgctaatcctgttaccagtggctgctgccagtggcgataagtcgtgtcttaccgggttggactcaagacgatagttaccggataaggcgcagcggtcgggctgaacggggggttcgtgcacacagcccagcttggagcgaacgacctacaccgaactgagatacctacagcgtgagctatgagaaagcgccacgcttcccgaagggagaaaggcggacaggtatccggtaagcggcagggtcggaacaggagagcgcacgagggagcttccagggggaaacgcctggtatctttatagtcctgtcgggtttcgccacctctgacttgagcgtcgatttttgtgatgctcgtcaggggggcggagcctatggaaaaacgccagcaacgcggcctttttacggttcctggccttttgctggccttttgctcacatgttctttcctgcgttatcccctgattctgtggataaccgtattaccgcctttgagtgagctgataccgctcgccgcagccgaacgaccgagcgcagcgagtcagtgagcgaggaagcggaagagcgcccaatacgcaaaccgcctctccccgcgcgttggccgattcattaatgcagctggcacgacaggtttcccgactggaaagcgggcagtgagcgcaacgcaattaatgtgagttagctcactcattaggcaccccaggctttacactttatgcttccggctcgtatgttgtgtggaattgtgagcggataacaatttcacacaggaaacagctatgaccatgattacgccaagcgcgcaattaaccctcactaaagggaacaaaagctggaaacatgcatgaagttcctattccgaagttcctattctctagaaagtataggaacttc

SEQ ID NO: 272 - DNA, 3345 bp, Synthetic construct
  source 1..3345: mol_type = other DNA
ataaaacctgcaggcatgcaagcgatcgcggggccgcccccttcaccgagggcctatttcccatgattccttcatatttgcatatacgatacaaggctgttagagagataattggaattaatttgactgtaaacacaaagatattagtacaaaatacgtgacgtagaaagtaataatttcttgggtagtttgcagttttaaaattatgttttaaaatggactatcatatgcttaccgtaacttgaaagtatttcgatttcttggctttatatatcttgtggaaaggacgaaacaccgttaaagaaaatatcatcttgtttcagagccaccagaagatatggcttcggtggcaagttgaaataaggctagtccgttatcaacttgaaaaagtggcaccgagtcggtgctttttttactagttctagagcggccccaattcgccctatagtgagtcgtattacgcgcgctcactggccgtcgttttacaacgtcgtgactgggaaaaccctggcgttacccaacttaatcgccttgcagcacatccccctttcgccagctggcgtaatagcgaagaggcccgcaccgatcgcccttcccaacagttgcgcagcctgaatggcgaatgggacgcgccctgtagcggcgcattaagcgcggcgggtgtggtggttacgcgcagcgtgaccgctacacttgccagcgccctagcgcccgctcctttcgctttcttcccttcctttctcgccacgttcgccggctttccccgtcaagctctaaatcgggggctccctttagggttccgatttagtgctttacggcacctcgaccccaaaaaacttgattagggtgatggttcacgtagtgggccatcgccctgatagacggtttttcgccctttgacgttggagtccacgttctttaatagtggactcttgttccaaactggaacaacactcaaccctatctcggtctattcttttgatttataagggattttgccgatttcggcctattggttaaaaaatgagctgatttaacaaaaatttaacgcgaattttaacaaaatattaacgcttacaatttaggtggcacttttcggggaaatgtgcgcggaacccctatttgtttatttttctaaatacattcaaatatgtatccgctcatgagacaataaccctgataaatgcttcaataatattgaaaaaggaagagtatgagtattcaacatttccgtgtcgcccttattcccttttttgcggcattttgccttcctgtttttgctcacccagaaacgctggtgaaagtaaaagatgctgaagatcagttgggtgcacgagtgggttacatcgaactggatctcaacagcggtaagatccttgagagttttcgccccgaagaacgttttccaatgatgagcacttttaaagttctgctatgtggcgcggtattatcccgtattgacgccgggcaagagcaactcggtcgccgcatacactattctcagaatgacttggttgagtactcaccagtcacagaaaagcatcttacggatggcatgacagtaagagaattatgcagtgctgccataaccatgagtgataacactgcggccaacttacttctgacaacgatcggaggaccgaaggagctaaccgcttttttgcacaacatgggggatcatgtaactcgccttgatcgttgggaaccggagctgaatgaagccataccaaacgacgagcgtgacaccacgatgcctgtagcaatggcaacaacgttgcgcaaactattaactggcgaactacttactctagcttcccggcaacaattaatagactggatggaggcggataaagttgcaggaccacttctgcgctcggcccttccggctggctggtttattgctgataaatctggagccggtgagcgtgggtctcgcggtatcattgcagcactggggccagatggtaagccctcccgtatcgtagttatctacacgacggggagtcaggcaactatggatgaacgaaatagacagatcgctgagataggtgcctcactgattaagcattggtaactgtcagaccaagtttactcatatatactttagattgatttaaaacttcatttttaatttaaaaggatctaggtgaagatcctttttgataatctcatgaccaaaatcccttaacgtgagttttcgttccactgagcgtcagaccccgtagaaaagatcaaaggatcttcttgagatcctttttttctgcgcgtaatctgctgcttgcaaacaaaaaaaccaccgctaccagcggtggtttgtttgccggatcaagagctaccaactctttttccgaaggtaactggcttcagcagagcgcagataccaaatactgtccttctagtgtagccgtagttaggccaccacttcaagaactctgtagcaccgcctacatacctcgctctgctaatcctgttaccagtggctgctgccagtggcgataagtcgtgtcttaccgggttggactcaagacgatagttaccggataaggcgcagcggtcgggctgaacggggggttcgtgcacacagcccagcttggagcgaacgacctacaccgaactgagatacctacagcgtgagctatgagaaagcgccacgcttcccgaagggagaaaggcggacaggtatccggtaagcggcagggtcggaacaggagagcgcacgagggagcttccagggggaaacgcctggtatctttatagtcctgtcgggtttcgccacctctgacttgagcgtcgatttttgtgatgctcgtcaggggggcggagcctatggaaaaacgccagcaacgcggcctttttacggttcctggccttttgctggccttttgctcacatgttctttcctgcgttatcccctgattctgtggataaccgtattaccgcctttgagtgagctgataccgctcgccgcagccgaacgaccgagcgcagcgagtcagtgagcgaggaagcggaagagcgcccaatacgcaaaccgcctctccccgcgcgttggccgattcattaatgcagctggcacgacaggtttcccgactggaaagcgggcagtgagcgcaacgcaattaatgtgagttagctcactcattaggcaccccaggctttacactttatgcttccggctcgtatgttgtgtggaattgtgagcggataacaatttcacacaggaaacagctatgaccatgattacgccaagcgcgcaattaaccctcactaaagggaacaaaagctggaaacatgcatgaagttcctattccgaagttcctattctctagaaagtataggaacttc

SEQ ID NO: 273 - DNA, 9170 bp, Synthetic construct
  source 1..9170: mol_type = other DNA
ggcgcgccggattcgacattgattattgactagttattaatagtaatcaattacggggtcattagttcatagcccatatatggagttccgcgttacataacttacggtaaatggcccgcctggctgaccgcccaacgacccccgcccattgacgtcaataatgacgtatgttcccatagtaacgccaatagggactttccattgacgtcaatgggtggagtatttacggtaaactgcccacttggcagtacatcaagtgtatcatatgccaagtacgccccctattgacgtcaatgacggtaaatggcccgcctggcattatgcccagtacatgaccttatgggactttcctacttggcagtacatctacgtattagtcatcgctattaccatggtcgaggtgagccccacgttctgcttcactctccccatctcccccccctccccacccccaattttgtatttatttattttttaattattttgtgcagcgatgggggcggggggggggggggggcgcgcgccaggcggggcggggcggggcgaggggcggggcggggcgaggcggagaggtgcggcggcagccaatcagagcggcgcgctccgaaagtttccttttatggcgaggcggcggcggcggcggccctataaaaagcgaagcgcgcggcgggcgggagtcgctgcgtcgcgccttcgccccgtgccccgctccgccgccgcctcgcgccgcccgccccggctctgactgaccgcgttactcccacaggtgagcgggcgggacggcccttctcctccgggctgtaattagcgcttggtttaatgacggctcgtttcttttctgtggctgcgtgaaagccttaaagggctccgggagggccctttgtgcgggggggagcggctcggggggtgcgtgcgtgtgtgtgtgcgtggggagcgccgcgtgcggcccgcgctgcccggcggctgtgagcgctgcgggcgcggcgcggggctttgtgcgctccgcgtgtgcgcgaggggagcgcggccgggggcggtgccccgcggtgcgggggggctgcgaggggaacaaaggctgcgtgcggggtgtgtgcgtgggggggtgagcagggggtgtgggcgcggcggtcgggctgtaacccccccctgcacccccctccccgagttgctgagcacggcccggcttcgggtgcggggctccgtgcggggcgtggcgcggggctcgccgtgccgggcggggggtggcggcaggtgggggtgccgggcggggcggggccgcctcgggccggggagggctcgggggaggggcgcggcggccccggagcgccggcggctgtcgaggcgcggcgagccgcagccattgccttttatggtaatcgtgcgagagggcgcagggacttcctttgtcccaaatctggcggagccgaaatctgggaggcgccgccgcaccccctctagcgggcgcgggcgaagcggtgcggcgccggcaggaaggaaatgggcggggagggccttcgtgcgtcgccgcgccgccgtccccttctccatctccagcctcggggctgccgcagggggacggctgccttcgggggggacggggcagggcggggttcggcttctggcgtgtgaccggcggctctagagcctctgctaaccatgttcatgccttcttctttttcctacagatccttaattaataatacgactcactataggggccgccaccatggacaagaagtacagcatcggcctggacatcggcaccaactctgtgggctgggccgtgatcaccgacgagtacaaggtgcccagcaagaaattcaaggtgctgggcaacaccgaccggcacagcatcaagaagaacctgatcggagccctgctgttcgacagcggcgaaacagccgaggccacccggctgaagagaaccgccagaagaagatacaccagacggaagaaccggatctgctatctgcaagagatcttcagcaacgagatggccaaggtggacgacagcttcttccacagactggaagagtccttcctggtggaagaggataagaagcacgagcggcaccccatcttcggcaacatcgtggacgaggtggcctaccacgagaagtaccccaccatctaccacctgagaaagaaactggtggacagcaccgacaaggccgacctgcggctgatctatctggccctggcccacatgatcaagttccggggccacttcctgatcgagggcgacctgaaccccgacaacagcgacgtggacaagctgttcatccagctggtgcagacctacaaccagctgttcgaggaaaaccccatcaacgccagcggcgtggacgccaaggccatcctgtctgccagactgagcaagagcagacggctggaaaatctgatcgcccagctgcccggcgagaagaagaatggcctgttcggcaacctgattgccctgagcctgggcctgacccccaacttcaagagcaacttcgacctggccgaggatgccaaactgcagctgagcaaggacacctacgacgacgacctggacaacctgctggcccagatcggcgaccagtacgccgacctgtttctggccgccaagaacctgtccgacgccatcctgctgagcgacatcctgagagtgaacaccgagatcaccaaggcccccctgagcgcctctatgatcaagagatacgacgagcaccaccaggacctgaccctgctgaaagctctcgtgcggcagcagctgcctgagaagtacaaagagattttcttcgaccagagcaagaacggctacgccggctacattgacggcggagccagccaggaagagttctacaagttcatcaagcccatcctggaaaagatggacggcaccgaggaactgctcgtgaagctgaacagagaggacctgctgcggaagcagcggaccttcgacaacggcagcatcccccaccagatccacctgggagagctgcacgccattctgcggcggcaggaagatttttacccattcctgaaggacaaccgggaaaagatcgagaagatcctgaccttccgcatcccctactacgtgggccctctggccaggggaaacagcagattcgcctggatgaccagaaagagcgaggaaaccatcaccccctggaacttcgaggaagtggtggacaagggcgcttccgcccagagcttcatcgagcggatgaccaacttcgataagaacctgcccaacgagaaggtgctgcccaagcacagcctgctgtacgagtacttcaccgtgtataacgagctgaccaaagtgaaatacgtgaccgagggaatgagaaagcccgccttcctgagcggcgagcagaaaaaggccatcgtggacctgctgttcaagaccaaccggaaagtgaccgtgaagcagctgaaagaggactacttcaagaaaatcgagtgcttcgactccgtggaaatctccggcgtggaagatcggttcaacgcctccctgggcacataccacgatctgctgaaaattatcaaggacaaggacttcctggacaatgaggaaaacgaggacattctggaagatatcgtgctgaccctgacactgtttgaggacagagagatgatcgaggaacggctgaaaacctatgcccacctgttcgacgacaaagtgatgaagcagctgaagcggcggagatacaccggctggggcaggctgagccggaagctgatcaacggcatccgggacaagcagtccggcaagacaatcctggatttcctgaagtccgacggcttcgccaacagaaacttcatgcagctgatccacgacgacagcctgacctttaaagaggacatccagaaagcccaggtgtccggccagggcgatagcctgcacgagcacattgccaatctggccggcagccccgccattaagaagggcatcctgcagacagtgaaggtggtggacgagctcgtgaaagtgatgggccggcacaagcccgagaacatcgtgatcgaaatggccagagagaaccagaccacccagaagggacagaagaacagccgcgagagaatgaagcggatcgaagagggcatcaaagagctgggcagccagatcctgaaagaacaccccgtggaaaacacccagctgcagaacgagaagctgtacctgtactacctgcagaatgggcgggatatgtacgtggaccaggaactggacatcaaccggctgtccgactacgatgtggaccatatcgtgcctcagagctttctgaaggacgactccatcgacaacaaggtgctgaccagaagcgacaagaaccggggcaagagcgacaacgtgccctccgaagaggtcgtgaagaagatgaagaactactggcggcagctgctgaacgccaagctgattacccagagaaagttcgacaatctgaccaaggccgagagaggcggcctgagcgaactggataaggccggcttcatcaagagacagctggtggaaacccggcagatcacaaagcacgtggcacagatcctggactcccggatgaacactaagtacgacgagaatgacaagctgatccgggaagtgaaagtgatcaccctgaagtccaagctggtgtccgatttccggaaggatttccagttttacaaagtgcgcgagatcaacaactaccaccacgcccacgacgcctacctgaacgccgtcgtgggaaccgccctgatcaaaaagtaccctaagctggaaagcgagttcgtgtacggcgactacaaggtgtacgacgtgcggaagatgatcgccaagagcgagcaggaaatcggcaaggctaccgccaagtacttcttctacagcaacatcatgaactttttcaagaccgagattaccctggccaacggcgagatccggaagcggcctctgatcgagacaaacggcgaaaccggggagatcgtgtgggataagggccgggattttgccaccgtgcggaaagtgctgagcatgccccaagtgaatatcgtgaaaaagaccgaggtgcagacaggcggcttcagcaaagagtctatcctgcccaagaggaacagcgataagctgatcgccagaaagaaggactgggaccctaagaagtacggcggcttcgacagccccaccgtggcctattctgtgctggtggtggccaaagtggaaaagggcaagtccaagaaactgaagagtgtgaaagagctgctggggatcaccatcatggaaagaagcagcttcgagaagaatcccatcgactttctggaagccaagggctacaaagaagtgaaaaaggacctgatcatcaagctgcctaagtactccctgttcgagctggaaaacggccggaagagaatgctggcctctgccggcgaactgcagaagggaaacgaactggccctgccctccaaatatgtgaacttcctgtacctggccagccactatgagaagctgaagggctcccccgaggataatgagcagaaacagctgtttgtggaacagcacaagcactacctggacgagatcatcgagcagatcagcgagttctccaagagagtgatcctggccgacgctaatctggacaaagtgctgtccgcctacaacaagcaccgggataagcccatcagagagcaggccgagaatatcatccacctgtttaccctgaccaatctgggagcccctgccgccttcaagtactttgacaccaccatcgaccggaagaggtacaccagcaccaaagaggtgctggacgccaccctgatccaccagagcatcaccggcctgtacgagacacggatcgacctgtctcagctgggaggcgacggatccacaccacctaagaagaaacggaaggtcgaggacggcgagggccctgctgctaagagagtgaaactggactccggagctgctccagccgccaagaagaagaagctcgactacaaggacgacgacgataagtgaacgcgtgctcgctttcttgctgtccaatttctattaaaggttcctttgttcgcgttgctggaccagaagatatggcttcggttcagcaaaatgattgcagatccactagttctagagctcgctgatcagcctcgactgtgccttctagttgccagccatctgttgtttgcccctcccccgtgccttccttgaccctggaaggtgccactcccactgtcctttcctaataaaatgaggaaattgcatcgcattgtctgagtaggtgtcattctattctggggggtggggtggggcaggacagcaagggggaggattgggaagacaatagcaggcatgctggggatgcggtgggctctatggcttctgaggcggaaagaaccagctggggctcgagatccactagttctagcctcgaggctagagcggccgccactggccgtcgttttacaacgtcgtgactgggaaaaccctggcgttacccaacttaatcgccttgcagcacatccccctttcgccagctggcgtaatagcgaagaggcccgcaccgatcgcccttcccaacagttgcgcagcctgaatggcgaatgggacgcgccctgtagcggcgcattaagcgcggcgggtgtggtggttacgcgcagcgtgaccgctacacttgccagcgccctagcgcccgctcctttcgctttcttcccttcctttctcgccacgttcgccggctttccccgtcaagctctaaatcgggggctccctttagggttccgatttagtgctttacggcacctcgaccccaaaaaacttgattagggtgatggttcacgtagtgggccatcgccctgatagacggtttttcgccctttgacgttggagtccacgttctttaatagtggactcttgttccaaactggaacaacactcaaccctatctcggtctattcttttgatttataagggattttgccgatttcggcctattggttaaaaaatgagctgatttaacaaaaatttaacgcgaattttaacaaaatattaacgcttacaatttaggtggcacttttcggggaaatgtgcgcggaacccctatttgtttatttttctaaatacattcaaatatgtatccgctcatgagacaataaccctgataaatgcttcaataatattgaaaaaggaagagtatgagtattcaacatttccgtgtcgcccttattcccttttttgcggcattttgccttcctgtttttgctcacccagaaacgctggtgaaagtaaaagatgctgaagatcagttgggtgcacgagtgggttacatcgaactggatctcaacagcggtaagatccttgagagttttcgccccgaagaacgttttccaatgatgagcacttttaaagttctgctatgtggcgcggtattatcccgtattgacgccgggcaagagcaactcggtcgccgcatacactattctcagaatgacttggttgagtactcaccagtcacagaaaagcatcttacggatggcatgacagtaagagaattatgcagtgctgccataaccatgagtgataacactgcggccaacttacttctgacaacgatcggaggaccgaaggagctaaccgcttttttgcacaacatgggggatcatgtaactcgccttgatcgttgggaaccggagctgaatgaagccataccaaacgacgagcgtgacaccacgatgcctgtagcaatggcaacaacgttgcgcaaactattaactggcgaactacttactctagcttcccggcaacaattaatagactggatggaggcggataaagttgcaggaccacttctgcgctcggcccttccggctggctggtttattgctgataaatctggagccggtgagcgtgggtctcgcggtatcattgcagcactggggccagatggtaagccctcccgtatcgtagttatctacacgacggggagtcaggcaactatggatgaacgaaatagacagatcgctgagataggtgcctcactgattaagcattggtaactgtcagaccaagtttactcatatatactttagattgatttaaaacttcatttttaatttaaaaggatctaggtgaagatcctttttgataatctcatgaccaaaatcccttaacgtgagttttcgttccactgagcgtcagaccccgtagaaaagatcaaaggatcttcttgagatcctttttttctgcgcgtaatctgctgcttgcaaacaaaaaaaccaccgctaccagcggtggtttgtttgccggatcaagagctaccaactctttttccgaaggtaactggcttcagcagagcgcagataccaaatactgtccttctagtgtagccgtagttaggccaccacttcaagaactctgtagcaccgcctacatacctcgctctgctaatcctgttaccagtggctgctgccagtggcgataagtcgtgtcttaccgggttggactcaagacgatagttaccggataaggcgcagcggtcgggctgaacggggggttcgtgcacacagcccagcttggagcgaacgacctacaccgaactgagatacctacagcgtgagctatgagaaagcgccacgcttcccgaagggagaaaggcggacaggtatccggtaagcggcagggtcggaacaggagagcgcacgagggagcttccagggggaaacgcctggtatctttatagtcctgtcgggtttcgccacctctgacttgagcgtcgatttttgtgatgctcgtcaggggggcggagcctatggaaaaacgccagcaacgcggcctttttacggttcctggccttttgctggccttttgctcacatgttctttcctgcgttatcccctgattctgtggataaccgtattaccgcctttgagtgagctgataccgctcgccgcagccgaacgaccgagcgcagcgagtcagtgagcgaggaagcggaagagcgcccaatacgcaaaccgcctctccccgcgcgttggccgattcattaatgcagctggcacgacaggtttcccgactggaaagcgggcagtgagcgcaacgcaattaatgtgagttagctcactcattaggcaccccaggctttacactttatgcttccggctcgtatgttgtgtggaattgtgagcggataacaatttcacacaggaaacagctatgaccatga

SEQ ID NO: 274 - DNA, 3345 bp, Synthetic construct
  source 1..3345: mol_type = other DNA
ataaaacctgcaggcatgcaagcgatcgcggggccgcccccttcaccgagggcctatttcccatgattccttcatatttgcatatacgatacaaggctgttagagagataattggaattaatttgactgtaaacacaaagatattagtacaaaatacgtgacgtagaaagtaataatttcttgggtagtttgcagttttaaaattatgttttaaaatggactatcatatgcttaccgtaacttgaaagtatttcgatttcttggctttatatatcttgtggaaaggacgaaacaccgtcccacaacgaagactgacgtttcagagccaccagaagatatggcttcggtggcaagttgaaataaggctagtccgttatcaacttgaaaaagtggcaccgagtcggtgctttttttactagttctagagcggccccaattcgccctatagtgagtcgtattacgcgcgctcactggccgtcgttttacaacgtcgtgactgggaaaaccctggcgttacccaacttaatcgccttgcagcacatccccctttcgccagctggcgtaatagcgaagaggcccgcaccgatcgcccttcccaacagttgcgcagcctgaatggcgaatgggacgcgccctgtagcggcgcattaagcgcggcgggtgtggtggttacgcgcagcgtgaccgctacacttgccagcgccctagcgcccgctcctttcgctttcttcccttcctttctcgccacgttcgccggctttccccgtcaagctctaaatcgggggctccctttagggttccgatttagtgctttacggcacctcgaccccaaaaaacttgattagggtgatggttcacgtagtgggccatcgccctgatagacggtttttcgccctttgacgttggagtccacgttctttaatagtggactcttgttccaaactggaacaacactcaaccctatctcggtctattcttttgatttataagggattttgccgatttcggcctattggttaaaaaatgagctgatttaacaaaaatttaacgcgaattttaacaaaatattaacgcttacaatttaggtggcacttttcggggaaatgtgcgcggaacccctatttgtttatttttctaaatacattcaaatatgtatccgctcatgagacaataaccctgataaatgcttcaataatattgaaaaaggaagagtatgagtattcaacatttccgtgtcgcccttattcccttttttgcggcattttgccttcctgtttttgctcacccagaaacgctggtgaaagtaaaagatgctgaagatcagttgggtgcacgagtgggttacatcgaactggatctcaacagcggtaagatccttgagagttttcgccccgaagaacgttttccaatgatgagcacttttaaagttctgctatgtggcgcggtattatcccgtattgacgccgggcaagagcaactcggtcgccgcatacactattctcagaatgacttggttgagtactcaccagtcacagaaaagcatcttacggatggcatgacagtaagagaattatgcagtgctgccataaccatgagtgataacactgcggccaacttacttctgacaacgatcggaggaccgaaggagctaaccgcttttttgcacaacatgggggatcatgtaactcgccttgatcgttgggaaccggagctgaatgaagccataccaaacgacgagcgtgacaccacgatgcctgtagcaatggcaacaacgttgcgcaaactattaactggcgaactacttactctagcttcccggcaacaattaatagactggatggaggcggataaagttgcaggaccacttctgcgctcggcccttccggctggctggtttattgctgataaatctggagccggtgagcgtgggtctcgcggtatcattgcagcactggggccagatggtaagccctcccgtatcgtagttatctacacgacggggagtcaggcaactatggatgaacgaaatagacagatcgctgagataggtgcctcactgattaagcattggtaactgtcagaccaagtttactcatatatactttagattgatttaaaacttcatttttaatttaaaaggatctaggtgaagatcctttttgataatctcatgaccaaaatcccttaacgtgagttttcgttccactgagcgtcagaccccgtagaaaagatcaaaggatcttcttgagatcctttttttctgcgcgtaatctgctgcttgcaaacaaaaaaaccaccgctaccagcggtggtttgtttgccggatcaagagctaccaactctttttccgaaggtaactggcttcagcagagcgcagataccaaatactgtccttctagtgtagccgtagttaggccaccacttcaagaactctgtagcaccgcctacatacctcgctctgctaatcctgttaccagtggctgctgccagtggcgataagtcgtgtcttaccgggttggactcaagacgatagttaccggataaggcgcagcggtcgggctgaacggggggttcgtgcacacagcccagcttggagcgaacgacctacaccgaactgagatacctacagcgtgagctatgagaaagcgccacgcttcccgaagggagaaaggcggacaggtatccggtaagcggcagggtcggaacaggagagcgcacgagggagcttccagggggaaacgcctggtatctttatagtcctgtcgggtttcgccacctctgacttgagcgtcgatttttgtgatgctcgtcaggggggcggagcctatggaaaaacgccagcaacgcggcctttttacggttcctggccttttgctggccttttgctcacatgttctttcctgcgttatcccctgattctgtggataaccgtattaccgcctttgagtgagctgataccgctcgccgcagccgaacgaccgagcgcagcgagtcagtgagcgaggaagcggaagagcgcccaatacgcaaaccgcctctccccgcgcgttggccgattcattaatgcagctggcacgacaggtttcccgactggaaagcgggcagtgagcgcaacgcaattaatgtgagttagctcactcattaggcaccccaggctttacactttatgcttccggctcgtatgttgtgtggaattgtgagcggataacaatttcacacaggaaacagctatgaccatgattacgccaagcgcgcaattaaccctcactaaagggaacaaaagctggaaacatgcatgaagttcctattccgaagttcctattctctagaaagtataggaacttc

SEQ ID NO: 275 - DNA, 9088 bp, Synthetic construct
  source 1..9088: mol_type = other DNA
ggcgcgccggattcgacattgattattgactagttattaatagtaatcaattacggggtcattagttcatagcccatatatggagttccgcgttacataacttacggtaaatggcccgcctggctgaccgcccaacgacccccgcccattgacgtcaataatgacgtatgttcccatagtaacgccaatagggactttccattgacgtcaatgggtggagtatttacggtaaactgcccacttggcagtacatcaagtgtatcatatgccaagtacgccccctattgacgtcaatgacggtaaatggcccgcctggcattatgcccagtacatgaccttatgggactttcctacttggcagtacatctacgtattagtcatcgctattaccatggtcgaggtgagccccacgttctgcttcactctccccatctcccccccctccccacccccaattttgtatttatttattttttaattattttgtgcagcgatgggggcggggggggggggggggcgcgcgccaggcggggcggggcggggcgaggggcggggcggggcgaggcggagaggtgcggcggcagccaatcagagcggcgcgctccgaaagtttccttttatggcgaggcggcggcggcggcggccctataaaaagcgaagcgcgcggcgggcgggagtcgctgcgtcgcgccttcgccccgtgccccgctccgccgccgcctcgcgccgcccgccccggctctgactgaccgcgttactcccacaggtgagcgggcgggacggcccttctcctccgggctgtaattagcgcttggtttaatgacggctcgtttcttttctgtggctgcgtgaaagccttaaagggctccgggagggccctttgtgcgggggggagcggctcggggggtgcgtgcgtgtgtgtgtgcgtggggagcgccgcgtgcggcccgcgctgcccggcggctgtgagcgctgcgggcgcggcgcggggctttgtgcgctccgcgtgtgcgcgaggggagcgcggccgggggcggtgccccgcggtgcgggggggctgcgaggggaacaaaggctgcgtgcggggtgtgtgcgtgggggggtgagcagggggtgtgggcgcggcggtcgggctgtaacccccccctgcacccccctccccgagttgctgagcacggcccggcttcgggtgcggggctccgtgcggggcgtggcgcggggctcgccgtgccgggcggggggtggcggcaggtgggggtgccgggcggggcggggccgcctcgggccggggagggctcgggggaggggcgcggcggccccggagcgccggcggctgtcgaggcgcggcgagccgcagccattgccttttatggtaatcgtgcgagagggcgcagggacttcctttgtcccaaatctggcggagccgaaatctgggaggcgccgccgcaccccctctagcgggcgcgggcgaagcggtgcggcgccggcaggaaggaaatgggcggggagggccttcgtgcgtcgccgcgccgccgtccccttctccatctccagcctcggggctgccgcagggggacggctgccttcgggggggacggggcagggcggggttcggcttctggcgtgtgaccggcggctctagagcctctgctaaccatgttcatgccttcttctttttcctacagatccttaattaataatacgactcactataggggccgccaccatggacaagaagtacagcatcggcctggacatcggcaccaactctgtgggctgggccgtgatcaccgacgagtacaaggtgcccagcaagaaattcaaggtgctgggcaacaccgaccggcacagcatcaagaagaacctgatcggagccctgctgttcgacagcggcgaaacagccgaggccacccggctgaagagaaccgccagaagaagatacaccagacggaagaaccggatctgctatctgcaagagatcttcagcaacgagatggccaaggtggacgacagcttcttccacagactggaagagtccttcctggtggaagaggataagaagcacgagcggcaccccatcttcggcaacatcgtggacgaggtggcctaccacgagaagtaccccaccatctaccacctgagaaagaaactggtggacagcaccgacaaggccgacctgcggctgatctatctggccctggcccacatgatcaagttccggggccacttcctgatcgagggcgacctgaaccccgacaacagcgacgtggacaagctgttcatccagctggtgcagacctacaaccagctgttcgaggaaaaccccatcaacgccagcggcgtggacgccaaggccatcctgtctgccagactgagcaagagcagacggctggaaaatctgatcgcccagctgcccggcgagaagaagaatggcctgttcggcaacctgattgccctgagcctgggcctgacccccaacttcaagagcaacttcgacctggccgaggatgccaaactgcagctgagcaaggacacctacgacgacgacctggacaacctgctggcccagatcggcgaccagtacgccgacctgtttctggccgccaagaacctgtccgacgccatcctgctgagcgacatcctgagagtgaacaccgagatcaccaaggcccccctgagcgcctctatgatcaagagatacgacgagcaccaccaggacctgaccctgctgaaagctctcgtgcggcagcagctgcctgagaagtacaaagagattttcttcgaccagagcaagaacggctacgccggctacattgacggcggagccagccaggaagagttctacaagttcatcaagcccatcctggaaaagatggacggcaccgaggaactgctcgtgaagctgaacagagaggacctgctgcggaagcagcggaccttcgacaacggcagcatcccccaccagatccacctgggagagctgcacgccattctgcggcggcaggaagatttttacccattcctgaaggacaaccgggaaaagatcgagaagatcctgaccttccgcatcccctactacgtgggccctctggccaggggaaacagcagattcgcctggatgaccagaaagagcgaggaaaccatcaccccctggaacttcgaggaagtggtggacaagggcgcttccgcccagagcttcatcgagcggatgaccaacttcgataagaacctgcccaacgagaaggtgctgcccaagcacagcctgctgtacgagtacttcaccgtgtataacgagctgaccaaagtgaaatacgtgaccgagggaatgagaaagcccgccttcctgagcggcgagcagaaaaaggccatcgtggacctgctgttcaagaccaaccggaaagtgaccgtgaagcagctgaaagaggactacttcaagaaaatcgagtgcttcgactccgtggaaatctccggcgtggaagatcggttcaacgcctccctgggcacataccacgatctgctgaaaattatcaaggacaaggacttcctggacaatgaggaaaacgaggacattctggaagatatcgtgctgaccctgacactgtttgaggacagagagatgatcgaggaacggctgaaaacctatgcccacctgttcgacgacaaagtgatgaagcagctgaagcggcggagatacaccggctggggcaggctgagccggaagctgatcaacggcatccgggacaagcagtccggcaagacaatcctggatttcctgaagtccgacggcttcgccaacagaaacttcatgcagctgatccacgacgacagcctgacctttaaagaggacatccagaaagcccaggtgtccggccagggcgatagcctgcacgagcacattgccaatctggccggcagccccgccattaagaagggcatcctgcagacagtgaaggtggtggacgagctcgtgaaagtgatgggccggcacaagcccgagaacatcgtgatcgaaatggccagagagaaccagaccacccagaagggacagaagaacagccgcgagagaatgaagcggatcgaagagggcatcaaagagctgggcagccagatcctgaaagaacaccccgtggaaaacacccagctgcagaacgagaagctgtacctgtactacctgcagaatgggcgggatatgtacgtggaccaggaactggacatcaaccggctgtccgactacgatgtggaccatatcgtgcctcagagctttctgaaggacgactccatcgacaacaaggtgctgaccagaagcgacaagaaccggggcaagagcgacaacgtgccctccgaagaggtcgtgaagaagatgaagaactactggcggcagctgctgaacgccaagctgattacccagagaaagttcgacaatctgaccaaggccgagagaggcggcctgagcgaactggataaggccggcttcatcaagagacagctggtggaaacccggcagatcacaaagcacgtggcacagatcctggactcccggatgaacactaagtacgacgagaatgacaagctgatccgggaagtgaaagtgatcaccctgaagtccaagctggtgtccgatttccggaaggatttccagttttacaaagtgcgcgagatcaacaactaccaccacgcccacgacgcctacctgaacgccgtcgtgggaaccgccctgatcaaaaagtaccctaagctggaaagcgagttcgtgtacggcgactacaaggtgtacgacgtgcggaagatgatcgccaagagcgagcaggaaatcggcaaggctaccgccaagtacttcttctacagcaacatcatgaactttttcaagaccgagattaccctggccaacggcgagatccggaagcggcctctgatcgagacaaacggcgaaaccggggagatcgtgtgggataagggccgggattttgccaccgtgcggaaagtgctgagcatgccccaagtgaatatcgtgaaaaagaccgaggtgcagacaggcggcttcagcaaagagtctatcctgcccaagaggaacagcgataagctgatcgccagaaagaaggactgggaccctaagaagtacggcggcttcgacagccccaccgtggcctattctgtgctggtggtggccaaagtggaaaagggcaagtccaagaaactgaagagtgtgaaagagctgctggggatcaccatcatggaaagaagcagcttcgagaagaatcccatcgactttctggaagccaagggctacaaagaagtgaaaaaggacctgatcatcaagctgcctaagtactccctgttcgagctggaaaacggccggaagagaatgctggcctctgccggcgaactgcagaagggaaacgaactggccctgccctccaaatatgtgaacttcctgtacctggccagccactatgagaagctgaagggctcccccgaggataatgagcagaaacagctgtttgtggaacagcacaagcactacctggacgagatcatcgagcagatcagcgagttctccaagagagtgatcctggccgacgctaatctggacaaagtgctgtccgcctacaacaagcaccgggataagcccatcagagagcaggccgagaatatcatccacctgtttaccctgaccaatctgggagcccctgccgccttcaagtactttgacaccaccatcgaccggaagaggtacaccagcaccaaagaggtgctggacgccaccctgatccaccagagcatcaccggcctgtacgagacacggatcgacctgtctcagctgggaggcgacggatccacaccacctaagaagaaacggaaggtcgaggacggcgagggccctgctgctaagagagtgaaactggactccggagctgctccagccgccaagaagaagaagctcgactacaaggacgacgacgataagtgaacgcgtaaatgattgcagatccactagttctagagctcgctgatcagcctcgactgtgccttctagttgccagccatctgttgtttgcccctcccccgtgccttccttgaccctggaaggtgccactcccactgtcctttcctaataaaatgaggaaattgcatcgcattgtctgagtaggtgtcattctattctggggggtggggtggggcaggacagcaagggggaggattgggaagacaatagcaggcatgctggggatgcggtgggctctatggcttctgaggcggaaagaaccagctggggctcgagatccactagttctagcctcgaggctagagcggccgccactggccgtcgttttacaacgtcgtgactgggaaaaccctggcgttacccaacttaatcgccttgcagcacatccccctttcgccagctggcgtaatagcgaagaggcccgcaccgatcgcccttcccaacagttgcgcagcctgaatggcgaatgggacgcgccctgtagcggcgcattaagcgcggcgggtgtggtggttacgcgcagcgtgaccgctacacttgccagcgccctagcgcccgctcctttcgctttcttcccttcctttctcgccacgttcgccggctttccccgtcaagctctaaatcgggggctccctttagggttccgatttagtgctttacggcacctcgaccccaaaaaacttgattagggtgatggttcacgtagtgggccatcgccctgatagacggtttttcgccctttgacgttggagtccacgttctttaatagtggactcttgttccaaactggaacaacactcaaccctatctcggtctattcttttgatttataagggattttgccgatttcggcctattggttaaaaaatgagctgatttaacaaaaatttaacgcgaattttaacaaaatattaacgcttacaatttaggtggcacttttcggggaaatgtgcgcggaacccctatttgtttatttttctaaatacattcaaatatgtatccgctcatgagacaataaccctgataaatgcttcaataatattgaaaaaggaagagtatgagtattcaacatttccgtgtcgcccttattcccttttttgcggcattttgccttcctgtttttgctcacccagaaacgctggtgaaagtaaaagatgctgaagatcagttgggtgcacgagtgggttacatcgaactggatctcaacagcggtaagatccttgagagttttcgccccgaagaacgttttccaatgatgagcacttttaaagttctgctatgtggcgcggtattatcccgtattgacgccgggcaagagcaactcggtcgccgcatacactattctcagaatgacttggttgagtactcaccagtcacagaaaagcatcttacggatggcatgacagtaagagaattatgcagtgctgccataaccatgagtgataacactgcggccaacttacttctgacaacgatcggaggaccgaaggagctaaccgcttttttgcacaacatgggggatcatgtaactcgccttgatcgttgggaaccggagctgaatgaagccataccaaacgacgagcgtgacaccacgatgcctgtagcaatggcaacaacgttgcgcaaactattaactggcgaactacttactctagcttcccggcaacaattaatagactggatggaggcggataaagttgcaggaccacttctgcgctcggcccttccggctggctggtttattgctgataaatctggagccggtgagcgtgggtctcgcggtatcattgcagcactggggccagatggtaagccctcccgtatcgtagttatctacacgacggggagtcaggcaactatggatgaacgaaatagacagatcgctgagataggtgcctcactgattaagcattggtaactgtcagaccaagtttactcatatatactttagattgatttaaaacttcatttttaatttaaaaggatctaggtgaagatcctttttgataatctcatgaccaaaatcccttaacgtgagttttcgttccactgagcgtcagaccccgtagaaaagatcaaaggatcttcttgagatcctttttttctgcgcgtaatctgctgcttgcaaacaaaaaaaccaccgctaccagcggtggtttgtttgccggatcaagagctaccaactctttttccgaaggtaactggcttcagcagagcgcagataccaaatactgtccttctagtgtagccgtagttaggccaccacttcaagaactctgtagcaccgcctacatacctcgctctgctaatcctgttaccagtggctgctgccagtggcgataagtcgtgtcttaccgggttggactcaagacgatagttaccggataaggcgcagcggtcgggctgaacggggggttcgtgcacacagcccagcttggagcgaacgacctacaccgaactgagatacctacagcgtgagctatgagaaagcgccacgcttcccgaagggagaaaggcggacaggtatccggtaagcggcagggtcggaacaggagagcgcacgagggagcttccagggggaaacgcctggtatctttatagtcctgtcgggtttcgccacctctgacttgagcgtcgatttttgtgatgctcgtcaggggggcggagcctatggaaaaacgccagcaacgcggcctttttacggttcctggccttttgctggccttttgctcacatgttctttcctgcgttatcccctgattctgtggataaccgtattaccgcctttgagtgagctgataccgctcgccgcagccgaacgaccgagcgcagcgagtcagtgagcgaggaagcggaagagcgcccaatacgcaaaccgcctctccccgcgcgttggccgattcattaatgcagctggcacgacaggtttcccgactggaaagcgggcagtgagcgcaacgcaattaatgtgagttagctcactcattaggcaccccaggctttacactttatgcttccggctcgtatgttgtgtggaattgtgagcggataacaatttcacacaggaaacagctatgaccatga

SEQ ID NO: 276 - DNA, 3375 bp, Synthetic construct
  source 1..3375: mol_type = other DNA
ataaaacctgcaggcatgcaagcgatcgcggggccgcccccttcaccgagggcctatttcccatgattccttcatatttgcatatacgatacaaggctgttagagagataattggaattaatttgactgtaaacacaaagatattagtacaaaatacgtgacgtagaaagtaataatttcttgggtagtttgcagttttaaaattatgttttaaaatggactatcatatgcttaccgtaacttgaaagtatttcgatttcttggctttatatatcttgtggaaaggacgaaacaccgtcccacaacgaagactgacgtttaagagctatgctggaaacagcatagcaagtttaaataaggctagtccgttatcaacttgaaaaagtggcaccgagtcggtgctttttttgatccaagggtgggcgcgccaaggcccgcggggccactagttctagagcggccccaattcgccctatagtgagtcgtattacgcgcgctcactggccgtcgttttacaacgtcgtgactgggaaaaccctggcgttacccaacttaatcgccttgcagcacatccccctttcgccagctggcgtaatagcgaagaggcccgcaccgatcgcccttcccaacagttgcgcagcctgaatggcgaatgggacgcgccctgtagcggcgcattaagcgcggcgggtgtggtggttacgcgcagcgtgaccgctacacttgccagcgccctagcgcccgctcctttcgctttcttcccttcctttctcgccacgttcgccggctttccccgtcaagctctaaatcgggggctccctttagggttccgatttagtgctttacggcacctcgaccccaaaaaacttgattagggtgatggttcacgtagtgggccatcgccctgatagacggtttttcgccctttgacgttggagtccacgttctttaatagtggactcttgttccaaactggaacaacactcaaccctatctcggtctattcttttgatttataagggattttgccgatttcggcctattggttaaaaaatgagctgatttaacaaaaatttaacgcgaattttaacaaaatattaacgcttacaatttaggtggcacttttcggggaaatgtgcgcggaacccctatttgtttatttttctaaatacattcaaatatgtatccgctcatgagacaataaccctgataaatgcttcaataatattgaaaaaggaagagtatgagtattcaacatttccgtgtcgcccttattcccttttttgcggcattttgccttcctgtttttgctcacccagaaacgctggtgaaagtaaaagatgctgaagatcagttgggtgcacgagtgggttacatcgaactggatctcaacagcggtaagatccttgagagttttcgccccgaagaacgttttccaatgatgagcacttttaaagttctgctatgtggcgcggtattatcccgtattgacgccgggcaagagcaactcggtcgccgcatacactattctcagaatgacttggttgagtactcaccagtcacagaaaagcatcttacggatggcatgacagtaagagaattatgcagtgctgccataaccatgagtgataacactgcggccaacttacttctgacaacgatcggaggaccgaaggagctaaccgcttttttgcacaacatgggggatcatgtaactcgccttgatcgttgggaaccggagctgaatgaagccataccaaacgacgagcgtgacaccacgatgcctgtagcaatggcaacaacgttgcgcaaactattaactggcgaactacttactctagcttcccggcaacaattaatagactggatggaggcggataaagttgcaggaccacttctgcgctcggcccttccggctggctggtttattgctgataaatctggagccggtgagcgtgggtctcgcggtatcattgcagcactggggccagatggtaagccctcccgtatcgtagttatctacacgacggggagtcaggcaactatggatgaacgaaatagacagatcgctgagataggtgcctcactgattaagcattggtaactgtcagaccaagtttactcatatatactttagattgatttaaaacttcatttttaatttaaaaggatctaggtgaagatcctttttgataatctcatgaccaaaatcccttaacgtgagttttcgttccactgagcgtcagaccccgtagaaaagatcaaaggatcttcttgagatcctttttttctgcgcgtaatctgctgcttgcaaacaaaaaaaccaccgctaccagcggtggtttgtttgccggatcaagagctaccaactctttttccgaaggtaactggcttcagcagagcgcagataccaaatactgtccttctagtgtagccgtagttaggccaccacttcaagaactctgtagcaccgcctacatacctcgctctgctaatcctgttaccagtggctgctgccagtggcgataagtcgtgtcttaccgggttggactcaagacgatagttaccggataaggcgcagcggtcgggctgaacggggggttcgtgcacacagcccagcttggagcgaacgacctacaccgaactgagatacctacagcgtgagctatgagaaagcgccacgcttcccgaagggagaaaggcggacaggtatccggtaagcggcagggtcggaacaggagagcgcacgagggagcttccagggggaaacgcctggtatctttatagtcctgtcgggtttcgccacctctgacttgagcgtcgatttttgtgatgctcgtcaggggggcggagcctatggaaaaacgccagcaacgcggcctttttacggttcctggccttttgctggccttttgctcacatgttctttcctgcgttatcccctgattctgtggataaccgtattaccgcctttgagtgagctgataccgctcgccgcagccgaacgaccgagcgcagcgagtcagtgagcgaggaagcggaagagcgcccaatacgcaaaccgcctctccccgcgcgttggccgattcattaatgcagctggcacgacaggtttcccgactggaaagcgggcagtgagcgcaacgcaattaatgtgagttagctcactcattaggcaccccaggctttacactttatgcttccggctcgtatgttgtgtggaattgtgagcggataacaatttcacacaggaaacagctatgaccatgattacgccaagcgcgcaattaaccctcactaaagggaacaaaagctggaaacatgcatgaagttcctattccgaagttcctattctctagaaagtataggaacttc

SEQ ID NO: 277 - DNA, 3345 bp, Synthetic construct
  source 1..3345: mol_type = other DNA
ataaaacctgcaggcatgcaagcgatcgcggggccgcccccttcaccgagggcctatttcccatgattccttcatatttgcatatacgatacaaggctgttagagagataattggaattaatttgactgtaaacacaaagatattagtacaaaatacgtgacgtagaaagtaataatttcttgggtagtttgcagttttaaaattatgttttaaaatggactatcatatgcttaccgtaacttgaaagtatttcgatttcttggctttatatatcttgtggaaaggacgaaacaccgctcacgctggatagcctccgtttcagagccaccagaagatatggcttcggtggcaagttgaaataaggctagtccgttatcaacttgaaaaagtggcaccgagtcggtgctttttttactagttctagagcggccccaattcgccctatagtgagtcgtattacgcgcgctcactggccgtcgttttacaacgtcgtgactgggaaaaccctggcgttacccaacttaatcgccttgcagcacatccccctttcgccagctggcgtaatagcgaagaggcccgcaccgatcgcccttcccaacagttgcgcagcctgaatggcgaatgggacgcgccctgtagcggcgcattaagcgcggcgggtgtggtggttacgcgcagcgtgaccgctacacttgccagcgccctagcgcccgctcctttcgctttcttcccttcctttctcgccacgttcgccggctttccccgtcaagctctaaatcgggggctccctttagggttccgatttagtgctttacggcacctcgaccccaaaaaacttgattagggtgatggttcacgtagtgggccatcgccctgatagacggtttttcgccctttgacgttggagtccacgttctttaatagtggactcttgttccaaactggaacaacactcaaccctatctcggtctattcttttgatttataagggattttgccgatttcggcctattggttaaaaaatgagctgatttaacaaaaatttaacgcgaattttaacaaaatattaacgcttacaatttaggtggcacttttcggggaaatgtgcgcggaacccctatttgtttatttttctaaatacattcaaatatgtatccgctcatgagacaataaccctgataaatgcttcaataatattgaaaaaggaagagtatgagtattcaacatttccgtgtcgcccttattcccttttttgcggcattttgccttcctgtttttgctcacccagaaacgctggtgaaagtaaaagatgctgaagatcagttgggtgcacgagtgggttacatcgaactggatctcaacagcggtaagatccttgagagttttcgccccgaagaacgttttccaatgatgagcacttttaaagttctgctatgtggcgcggtattatcccgtattgacgccgggcaagagcaactcggtcgccgcatacactattctcagaatgacttggttgagtactcaccagtcacagaaaagcatcttacggatggcatgacagtaagagaattatgcagtgctgccataaccatgagtgataacactgcggccaacttacttctgacaacgatcggaggaccgaaggagctaaccgcttttttgcacaacatgggggatcatgtaactcgccttgatcgttgggaaccggagctgaatgaagccataccaaacgacgagcgtgacaccacgatgcctgtagcaatggcaacaacgttgcgcaaactattaactggcgaactacttactctagcttcccggcaacaattaatagactggatggaggcggataaagttgcaggaccacttctgcgctcggcccttccggctggctggtttattgctgataaatctggagccggtgagcgtgggtctcgcggtatcattgcagcactggggccagatggtaagccctcccgtatcgtagttatctacacgacggggagtcaggcaactatggatgaacgaaatagacagatcgctgagataggtgcctcactgattaagcattggtaactgtcagaccaagtttactcatatatactttagattgatttaaaacttcatttttaatttaaaaggatctaggtgaagatcctttttgataatctcatgaccaaaatcccttaacgtgagttttcgttccactgagcgtcagaccccgtagaaaagatcaaaggatcttcttgagatcctttttttctgcgcgtaatctgctgcttgcaaacaaaaaaaccaccgctaccagcggtggtttgtttgccggatcaagagctaccaactctttttccgaaggtaactggcttcagcagagcgcagataccaaatactgtccttctagtgtagccgtagttaggccaccacttcaagaactctgtagcaccgcctacatacctcgctctgctaatcctgttaccagtggctgctgccagtggcgataagtcgtgtcttaccgggttggactcaagacgatagttaccggataaggcgcagcggtcgggctgaacggggggttcgtgcacacagcccagcttggagcgaacgacctacaccgaactgagatacctacagcgtgagctatgagaaagcgccacgcttcccgaagggagaaaggcggacaggtatccggtaagcggcagggtcggaacaggagagcgcacgagggagcttccagggggaaacgcctggtatctttatagtcctgtcgggtttcgccacctctgacttgagcgtcgatttttgtgatgctcgtcaggggggcggagcctatggaaaaacgccagcaacgcggcctttttacggttcctggccttttgctggccttttgctcacatgttctttcctgcgttatcccctgattctgtggataaccgtattaccgcctttgagtgagctgataccgctcgccgcagccgaacgaccgagcgcagcgagtcagtgagcgaggaagcggaagagcgcccaatacgcaaaccgcctctccccgcgcgttggccgattcattaatgcagctggcacgacaggtttcccgactggaaagcgggcagtgagcgcaacgcaattaatgtgagttagctcactcattaggcaccccaggctttacactttatgcttccggctcgtatgttgtgtggaattgtgagcggataacaatttcacacaggaaacagctatgaccatgattacgccaagcgcgcaattaaccctcactaaagggaacaaaagctggaaacatgcatgaagttcctattccgaagttcctattctctagaaagtataggaacttc

SEQ ID NO: 278 - DNA, 9736 bp, Synthetic construct
  source 1..9736: mol_type = other DNA
ggcgcgccggattcgacattgattattgactagttattaatagtaatcaattacggggtcattagttcatagcccatatatggagttccgcgttacataacttacggtaaatggcccgcctggctgaccgcccaacgacccccgcccattgacgtcaataatgacgtatgttcccatagtaacgccaatagggactttccattgacgtcaatgggtggagtatttacggtaaactgcccacttggcagtacatcaagtgtatcatatgccaagtacgccccctattgacgtcaatgacggtaaatggcccgcctggcattatgcccagtacatgaccttatgggactttcctacttggcagtacatctacgtattagtcatcgctattaccatggtcgaggtgagccccacgttctgcttcactctccccatctcccccccctccccacccccaattttgtatttatttattttttaattattttgtgcagcgatgggggcggggggggggggggggcgcgcgccaggcggggcggggcggggcgaggggcggggcggggcgaggcggagaggtgcggcggcagccaatcagagcggcgcgctccgaaagtttccttttatggcgaggcggcggcggcggcggccctataaaaagcgaagcgcgcggcgggcgggagtcgctgcgtcgcgccttcgccccgtgccccgctccgccgccgcctcgcgccgcccgccccggctctgactgaccgcgttactcccacaggtgagcgggcgggacggcccttctcctccgggctgtaattagcgcttggtttaatgacggctcgtttcttttctgtggctgcgtgaaagccttaaagggctccgggagggccctttgtgcgggggggagcggctcggggggtgcgtgcgtgtgtgtgtgcgtggggagcgccgcgtgcggcccgcgctgcccggcggctgtgagcgctgcgggcgcggcgcggggctttgtgcgctccgcgtgtgcgcgaggggagcgcggccgggggcggtgccccgcggtgcgggggggctgcgaggggaacaaaggctgcgtgcggggtgtgtgcgtgggggggtgagcagggggtgtgggcgcggcggtcgggctgtaacccccccctgcacccccctccccgagttgctgagcacggcccggcttcgggtgcggggctccgtgcggggcgtggcgcggggctcgccgtgccgggcggggggtggcggcaggtgggggtgccgggcggggcggggccgcctcgggccggggagggctcgggggaggggcgcggcggccccggagcgccggcggctgtcgaggcgcggcgagccgcagccattgccttttatggtaatcgtgcgagagggcgcagggacttcctttgtcccaaatctggcggagccgaaatctgggaggcgccgccgcaccccctctagcgggcgcgggcgaagcggtgcggcgccggcaggaaggaaatgggcggggagggccttcgtgcgtcgccgcgccgccgtccccttctccatctccagcctcggggctgccgcagggggacggctgccttcgggggggacggggcagggcggggttcggcttctggcgtgtgaccggcggctctagagcctctgctaaccatgttcatgccttcttctttttcctacagatccttaattaataatacgactcactataggggccgccaccatgaaacggacagccgacggaagcgagttcgagtcaccaaagaagaagcggaaagtctctgaggtggagttttcccacgagtactggatgagacatgccctgaccctggccaagagggcacgggatgagagggaggtgcctgtgggagccgtgctggtgctgaacaatagagtgatcggcgagggctggaacagagccatcggcctgcacgacccaacagcccatgccgaaattatggccctgagacagggcggcctggtcatgcagaactacagactgattgacgccaccctgtacgtgacattcgagccttgcgtgatgtgcgccggcgccatgatccactctaggatcggccgcgtggtgtttggcgtgaggaactcaaaaagaggcgccgcaggctccctgatgaacgtgctgaactaccccggcatgaatcaccgcgtcgaaattaccgagggaatcctggcagatgaatgtgccgccctgctgtgcgatttctatcggatgcctagacaggtgttcaatgctcagaagaaggcccagagctccatcaactccggaggatctagcggaggctcctctggctctgagacacctggcacaagcgagagcgcaacacctgaaagcagcgggggcagcagcggggggtcagacaagaagtacagcatcggcctggccatcggcaccaactctgtgggctgggccgtgatcaccgacgagtacaaggtgcccagcaagaaattcaaggtgctgggcaacaccgaccggcacagcatcaagaagaacctgatcggagccctgctgttcgacagcggcgaaacagccgaggccacccggctgaagagaaccgccagaagaagatacaccagacggaagaaccggatctgctatctgcaagagatcttcagcaacgagatggccaaggtggacgacagcttcttccacagactggaagagtccttcctggtggaagaggataagaagcacgagcggcaccccatcttcggcaacatcgtggacgaggtggcctaccacgagaagtaccccaccatctaccacctgagaaagaaactggtggacagcaccgacaaggccgacctgcggctgatctatctggccctggcccacatgatcaagttccggggccacttcctgatcgagggcgacctgaaccccgacaacagcgacgtggacaagctgttcatccagctggtgcagacctacaaccagctgttcgaggaaaaccccatcaacgccagcggcgtggacgccaaggccatcctgtctgccagactgagcaagagcagacggctggaaaatctgatcgcccagctgcccggcgagaagaagaatggcctgttcggcaacctgattgccctgagcctgggcctgacccccaacttcaagagcaacttcgacctggccgaggatgccaaactgcagctgagcaaggacacctacgacgacgacctggacaacctgctggcccagatcggcgaccagtacgccgacctgtttctggccgccaagaacctgtccgacgccatcctgctgagcgacatcctgagagtgaacaccgagatcaccaaggcccccctgagcgcctctatgatcaagagatacgacgagcaccaccaggacctgaccctgctgaaagctctcgtgcggcagcagctgcctgagaagtacaaagagattttcttcgaccagagcaagaacggctacgccggctacattgacggcggagccagccaggaagagttctacaagttcatcaagcccatcctggaaaagatggacggcaccgaggaactgctcgtgaagctgaacagagaggacctgctgcggaagcagcggaccttcgacaacggcagcatcccccaccagatccacctgggagagctgcacgccattctgcggcggcaggaagatttttacccattcctgaaggacaaccgggaaaagatcgagaagatcctgaccttccgcatcccctactacgtgggccctctggccaggggaaacagcagattcgcctggatgaccagaaagagcgaggaaaccatcaccccctggaacttcgaggaagtggtggacaagggcgcttccgcccagagcttcatcgagcggatgaccaacttcgataagaacctgcccaacgagaaggtgctgcccaagcacagcctgctgtacgagtacttcaccgtgtataacgagctgaccaaagtgaaatacgtgaccgagggaatgagaaagcccgccttcctgagcggcgagcagaaaaaggccatcgtggacctgctgttcaagaccaaccggaaagtgaccgtgaagcagctgaaagaggactacttcaagaaaatcgagtgcttcgactccgtggaaatctccggcgtggaagatcggttcaacgcctccctgggcacataccacgatctgctgaaaattatcaaggacaaggacttcctggacaatgaggaaaacgaggacattctggaagatatcgtgctgaccctgacactgtttgaggacagagagatgatcgaggaacggctgaaaacctatgcccacctgttcgacgacaaagtgatgaagcagctgaagcggcggagatacaccggctggggcaggctgagccggaagctgatcaacggcatccgggacaagcagtccggcaagacaatcctggatttcctgaagtccgacggcttcgccaacagaaacttcatgcagctgatccacgacgacagcctgacctttaaagaggacatccagaaagcccaggtgtccggccagggcgatagcctgcacgagcacattgccaatctggccggcagccccgccattaagaagggcatcctgcagacagtgaaggtggtggacgagctcgtgaaagtgatgggccggcacaagcccgagaacatcgtgatcgaaatggccagagagaaccagaccacccagaagggacagaagaacagccgcgagagaatgaagcggatcgaagagggcatcaaagagctgggcagccagatcctgaaagaacaccccgtggaaaacacccagctgcagaacgagaagctgtacctgtactacctgcagaatgggcgggatatgtacgtggaccaggaactggacatcaaccggctgtccgactacgatgtggaccatatcgtgcctcagagctttctgaaggacgactccatcgacaacaaggtgctgaccagaagcgacaagaaccggggcaagagcgacaacgtgccctccgaagaggtcgtgaagaagatgaagaactactggcggcagctgctgaacgccaagctgattacccagagaaagttcgacaatctgaccaaggccgagagaggcggcctgagcgaactggataaggccggcttcatcaagagacagctggtggaaacccggcagatcacaaagcacgtggcacagatcctggactcccggatgaacactaagtacgacgagaatgacaagctgatccgggaagtgaaagtgatcaccctgaagtccaagctggtgtccgatttccggaaggatttccagttttacaaagtgcgcgagatcaacaactaccaccacgcccacgacgcctacctgaacgccgtcgtgggaaccgccctgatcaaaaagtaccctaagctggaaagcgagttcgtgtacggcgactacaaggtgtacgacgtgcggaagatgatcgccaagagcgagcaggaaatcggcaaggctaccgccaagtacttcttctacagcaacatcatgaactttttcaagaccgagattaccctggccaacggcgagatccggaagcggcctctgatcgagacaaacggcgaaaccggggagatcgtgtgggataagggccgggattttgccaccgtgcggaaagtgctgagcatgccccaagtgaatatcgtgaaaaagaccgaggtgcagacaggcggcttcagcaaagagtctatcctgcccaagaggaacagcgataagctgatcgccagaaagaaggactgggaccctaagaagtacggcggcttcgacagccccaccgtggcctattctgtgctggtggtggccaaagtggaaaagggcaagtccaagaaactgaagagtgtgaaagagctgctggggatcaccatcatggaaagaagcagcttcgagaagaatcccatcgactttctggaagccaagggctacaaagaagtgaaaaaggacctgatcatcaagctgcctaagtactccctgttcgagctggaaaacggccggaagagaatgctggcctctgccggcgaactgcagaagggaaacgaactggccctgccctccaaatatgtgaacttcctgtacctggccagccactatgagaagctgaagggctcccccgaggataatgagcagaaacagctgtttgtggaacagcacaagcactacctggacgagatcatcgagcagatcagcgagttctccaagagagtgatcctggccgacgctaatctggacaaagtgctgtccgcctacaacaagcaccgggataagcccatcagagagcaggccgagaatatcatccacctgtttaccctgaccaatctgggagcccctgccgccttcaagtactttgacaccaccatcgaccggaagaggtacaccagcaccaaagaggtgctggacgccaccctgatccaccagagcatcaccggcctgtacgagacacggatcgacctgtctcagctgggaggcgacggatccacaccacctaagaagaaacggaaggtcgaggacggcgagggccctgctgctaagagagtgaaactggactccggagctgctccagccgccaagaagaagaagctcgactacaaggacgacgacgataagtgaacgcgtaaatgattgcagatccactagttctagagctcgctgatcagcctcgactgtgccttctagttgccagccatctgttgtttgcccctcccccgtgccttccttgaccctggaaggtgccactcccactgtcctttcctaataaaatgaggaaattgcatcgcattgtctgagtaggtgtcattctattctggggggtggggtggggcaggacagcaagggggaggattgggaagacaatagcaggcatgctggggatgcggtgggctctatggcttctgaggcggaaagaaccagctggggctcgagatccactagttctagcctcgaggctagagcggccgccactggccgtcgttttacaacgtcgtgactgggaaaaccctggcgttacccaacttaatcgccttgcagcacatccccctttcgccagctggcgtaatagcgaagaggcccgcaccgatcgcccttcccaacagttgcgcagcctgaatggcgaatgggacgcgccctgtagcggcgcattaagcgcggcgggtgtggtggttacgcgcagcgtgaccgctacacttgccagcgccctagcgcccgctcctttcgctttcttcccttcctttctcgccacgttcgccggctttccccgtcaagctctaaatcgggggctccctttagggttccgatttagtgctttacggcacctcgaccccaaaaaacttgattagggtgatggttcacgtagtgggccatcgccctgatagacggtttttcgccctttgacgttggagtccacgttctttaatagtggactcttgttccaaactggaacaacactcaaccctatctcggtctattcttttgatttataagggattttgccgatttcggcctattggttaaaaaatgagctgatttaacaaaaatttaacgcgaattttaacaaaatattaacgcttacaatttaggtggcacttttcggggaaatgtgcgcggaacccctatttgtttatttttctaaatacattcaaatatgtatccgctcatgagacaataaccctgataaatgcttcaataatattgaaaaaggaagagtatgagtattcaacatttccgtgtcgcccttattcccttttttgcggcattttgccttcctgtttttgctcacccagaaacgctggtgaaagtaaaagatgctgaagatcagttgggtgcacgagtgggttacatcgaactggatctcaacagcggtaagatccttgagagttttcgccccgaagaacgttttccaatgatgagcacttttaaagttctgctatgtggcgcggtattatcccgtattgacgccgggcaagagcaactcggtcgccgcatacactattctcagaatgacttggttgagtactcaccagtcacagaaaagcatcttacggatggcatgacagtaagagaattatgcagtgctgccataaccatgagtgataacactgcggccaacttacttctgacaacgatcggaggaccgaaggagctaaccgcttttttgcacaacatgggggatcatgtaactcgccttgatcgttgggaaccggagctgaatgaagccataccaaacgacgagcgtgacaccacgatgcctgtagcaatggcaacaacgttgcgcaaactattaactggcgaactacttactctagcttcccggcaacaattaatagactggatggaggcggataaagttgcaggaccacttctgcgctcggcccttccggctggctggtttattgctgataaatctggagccggtgagcgtgggtctcgcggtatcattgcagcactggggccagatggtaagccctcccgtatcgtagttatctacacgacggggagtcaggcaactatggatgaacgaaatagacagatcgctgagataggtgcctcactgattaagcattggtaactgtcagaccaagtttactcatatatactttagattgatttaaaacttcatttttaatttaaaaggatctaggtgaagatcctttttgataatctcatgaccaaaatcccttaacgtgagttttcgttccactgagcgtcagaccccgtagaaaagatcaaaggatcttcttgagatcctttttttctgcgcgtaatctgctgcttgcaaacaaaaaaaccaccgctaccagcggtggtttgtttgccggatcaagagctaccaactctttttccgaaggtaactggcttcagcagagcgcagataccaaatactgtccttctagtgtagccgtagttaggccaccacttcaagaactctgtagcaccgcctacatacctcgctctgctaatcctgttaccagtggctgctgccagtggcgataagtcgtgtcttaccgggttggactcaagacgatagttaccggataaggcgcagcggtcgggctgaacggggggttcgtgcacacagcccagcttggagcgaacgacctacaccgaactgagatacctacagcgtgagctatgagaaagcgccacgcttcccgaagggagaaaggcggacaggtatccggtaagcggcagggtcggaacaggagagcgcacgagggagcttccagggggaaacgcctggtatctttatagtcctgtcgggtttcgccacctctgacttgagcgtcgatttttgtgatgctcgtcaggggggcggagcctatggaaaaacgccagcaacgcggcctttttacggttcctggccttttgctggccttttgctcacatgttctttcctgcgttatcccctgattctgtggataaccgtattaccgcctttgagtgagctgataccgctcgccgcagccgaacgaccgagcgcagcgagtcagtgagcgaggaagcggaagagcgcccaatacgcaaaccgcctctccccgcgcgttggccgattcattaatgcagctggcacgacaggtttcccgactggaaagcgggcagtgagcgcaacgcaattaatgtgagttagctcactcattaggcaccccaggctttacactttatgcttccggctcgtatgttgtgtggaattgtgagcggataacaatttcacacaggaaacagctatgaccatga

SEQ ID NO: 279 - DNA, 3345 bp, Synthetic construct
  source 1..3345: mol_type = other DNA
ataaaacctgcaggcatgcaagcgatcgcggggccgcccccttcaccgagggcctatttcccatgattccttcatatttgcatatacgatacaaggctgttagagagataattggaattaatttgactgtaaacacaaagatattagtacaaaatacgtgacgtagaaagtaataatttcttgggtagtttgcagttttaaaattatgttttaaaatggactatcatatgcttaccgtaacttgaaagtatttcgatttcttggctttatatatcttgtggaaaggacgaaacaccggcgaaagggcagcgccgaggtttcagagccaccagaagatatggcttcggtggcaagttgaaataaggctagtccgttatcaacttgaaaaagtggcaccgagtcggtgctttttttactagttctagagcggccccaattcgccctatagtgagtcgtattacgcgcgctcactggccgtcgttttacaacgtcgtgactgggaaaaccctggcgttacccaacttaatcgccttgcagcacatccccctttcgccagctggcgtaatagcgaagaggcccgcaccgatcgcccttcccaacagttgcgcagcctgaatggcgaatgggacgcgccctgtagcggcgcattaagcgcggcgggtgtggtggttacgcgcagcgtgaccgctacacttgccagcgccctagcgcccgctcctttcgctttcttcccttcctttctcgccacgttcgccggctttccccgtcaagctctaaatcgggggctccctttagggttccgatttagtgctttacggcacctcgaccccaaaaaacttgattagggtgatggttcacgtagtgggccatcgccctgatagacggtttttcgccctttgacgttggagtccacgttctttaatagtggactcttgttccaaactggaacaacactcaaccctatctcggtctattcttttgatttataagggattttgccgatttcggcctattggttaaaaaatgagctgatttaacaaaaatttaacgcgaattttaacaaaatattaacgcttacaatttaggtggcacttttcggggaaatgtgcgcggaacccctatttgtttatttttctaaatacattcaaatatgtatccgctcatgagacaataaccctgataaatgcttcaataatattgaaaaaggaagagtatgagtattcaacatttccgtgtcgcccttattcccttttttgcggcattttgccttcctgtttttgctcacccagaaacgctggtgaaagtaaaagatgctgaagatcagttgggtgcacgagtgggttacatcgaactggatctcaacagcggtaagatccttgagagttttcgccccgaagaacgttttccaatgatgagcacttttaaagttctgctatgtggcgcggtattatcccgtattgacgccgggcaagagcaactcggtcgccgcatacactattctcagaatgacttggttgagtactcaccagtcacagaaaagcatcttacggatggcatgacagtaagagaattatgcagtgctgccataaccatgagtgataacactgcggccaacttacttctgacaacgatcggaggaccgaaggagctaaccgcttttttgcacaacatgggggatcatgtaactcgccttgatcgttgggaaccggagctgaatgaagccataccaaacgacgagcgtgacaccacgatgcctgtagcaatggcaacaacgttgcgcaaactattaactggcgaactacttactctagcttcccggcaacaattaatagactggatggaggcggataaagttgcaggaccacttctgcgctcggcccttccggctggctggtttattgctgataaatctggagccggtgagcgtgggtctcgcggtatcattgcagcactggggccagatggtaagccctcccgtatcgtagttatctacacgacggggagtcaggcaactatggatgaacgaaatagacagatcgctgagataggtgcctcactgattaagcattggtaactgtcagaccaagtttactcatatatactttagattgatttaaaacttcatttttaatttaaaaggatctaggtgaagatcctttttgataatctcatgaccaaaatcccttaacgtgagttttcgttccactgagcgtcagaccccgtagaaaagatcaaaggatcttcttgagatcctttttttctgcgcgtaatctgctgcttgcaaacaaaaaaaccaccgctaccagcggtggtttgtttgccggatcaagagctaccaactctttttccgaaggtaactggcttcagcagagcgcagataccaaatactgtccttctagtgtagccgtagttaggccaccacttcaagaactctgtagcaccgcctacatacctcgctctgctaatcctgttaccagtggctgctgccagtggcgataagtcgtgtcttaccgggttggactcaagacgatagttaccggataaggcgcagcggtcgggctgaacggggggttcgtgcacacagcccagcttggagcgaacgacctacaccgaactgagatacctacagcgtgagctatgagaaagcgccacgcttcccgaagggagaaaggcggacaggtatccggtaagcggcagggtcggaacaggagagcgcacgagggagcttccagggggaaacgcctggtatctttatagtcctgtcgggtttcgccacctctgacttgagcgtcgatttttgtgatgctcgtcaggggggcggagcctatggaaaaacgccagcaacgcggcctttttacggttcctggccttttgctggccttttgctcacatgttctttcctgcgttatcccctgattctgtggataaccgtattaccgcctttgagtgagctgataccgctcgccgcagccgaacgaccgagcgcagcgagtcagtgagcgaggaagcggaagagcgcccaatacgcaaaccgcctctccccgcgcgttggccgattcattaatgcagctggcacgacaggtttcccgactggaaagcgggcagtgagcgcaacgcaattaatgtgagttagctcactcattaggcaccccaggctttacactttatgcttccggctcgtatgttgtgtggaattgtgagcggataacaatttcacacaggaaacagctatgaccatgattacgccaagcgcgcaattaaccctcactaaagggaacaaaagctggaaacatgcatgaagttcctattccgaagttcctattctctagaaagtataggaacttc

SEQ ID NO: 280 - DNA, 3345 bp, Synthetic construct
  source 1..3345: mol_type = other DNA
ataaaacctgcaggcatgcaagcgatcgcggggccgcccccttcaccgagggcctatttcccatgattccttcatatttgcatatacgatacaaggctgttagagagataattggaattaatttgactgtaaacacaaagatattagtacaaaatacgtgacgtagaaagtaataatttcttgggtagtttgcagttttaaaattatgttttaaaatggactatcatatgcttaccgtaacttgaaagtatttcgatttcttggctttatatatcttgtggaaaggacgaaacaccgccggaggagaaggctcccggtttcagagccaccagaagatatggcttcggtggcaagttgaaataaggctagtccgttatcaacttgaaaaagtggcaccgagtcggtgctttttttactagttctagagcggccccaattcgccctatagtgagtcgtattacgcgcgctcactggccgtcgttttacaacgtcgtgactgggaaaaccctggcgttacccaacttaatcgccttgcagcacatccccctttcgccagctggcgtaatagcgaagaggcccgcaccgatcgcccttcccaacagttgcgcagcctgaatggcgaatgggacgcgccctgtagcggcgcattaagcgcggcgggtgtggtggttacgcgcagcgtgaccgctacacttgccagcgccctagcgcccgctcctttcgctttcttcccttcctttctcgccacgttcgccggctttccccgtcaagctctaaatcgggggctccctttagggttccgatttagtgctttacggcacctcgaccccaaaaaacttgattagggtgatggttcacgtagtgggccatcgccctgatagacggtttttcgccctttgacgttggagtccacgttctttaatagtggactcttgttccaaactggaacaacactcaaccctatctcggtctattcttttgatttataagggattttgccgatttcggcctattggttaaaaaatgagctgatttaacaaaaatttaacgcgaattttaacaaaatattaacgcttacaatttaggtggcacttttcggggaaatgtgcgcggaacccctatttgtttatttttctaaatacattcaaatatgtatccgctcatgagacaataaccctgataaatgcttcaataatattgaaaaaggaagagtatgagtattcaacatttccgtgtcgcccttattcccttttttgcggcattttgccttcctgtttttgctcacccagaaacgctggtgaaagtaaaagatgctgaagatcagttgggtgcacgagtgggttacatcgaactggatctcaacagcggtaagatccttgagagttttcgccccgaagaacgttttccaatgatgagcacttttaaagttctgctatgtggcgcggtattatcccgtattgacgccgggcaagagcaactcggtcgccgcatacactattctcagaatgacttggttgagtactcaccagtcacagaaaagcatcttacggatggcatgacagtaagagaattatgcagtgctgccataaccatgagtgataacactgcggccaacttacttctgacaacgatcggaggaccgaaggagctaaccgcttttttgcacaacatgggggatcatgtaactcgccttgatcgttgggaaccggagctgaatgaagccataccaaacgacgagcgtgacaccacgatgcctgtagcaatggcaacaacgttgcgcaaactattaactggcgaactacttactctagcttcccggcaacaattaatagactggatggaggcggataaagttgcaggaccacttctgcgctcggcccttccggctggctggtttattgctgataaatctggagccggtgagcgtgggtctcgcggtatcattgcagcactggggccagatggtaagccctcccgtatcgtagttatctacacgacggggagtcaggcaactatggatgaacgaaatagacagatcgctgagataggtgcctcactgattaagcattggtaactgtcagaccaagtttactcatatatactttagattgatttaaaacttcatttttaatttaaaaggatctaggtgaagatcctttttgataatctcatgaccaaaatcccttaacgtgagttttcgttccactgagcgtcagaccccgtagaaaagatcaaaggatcttcttgagatcctttttttctgcgcgtaatctgctgcttgcaaacaaaaaaaccaccgctaccagcggtggtttgtttgccggatcaagagctaccaactctttttccgaaggtaactggcttcagcagagcgcagataccaaatactgtccttctagtgtagccgtagttaggccaccacttcaagaactctgtagcaccgcctacatacctcgctctgctaatcctgttaccagtggctgctgccagtggcgataagtcgtgtcttaccgggttggactcaagacgatagttaccggataaggcgcagcggtcgggctgaacggggggttcgtgcacacagcccagcttggagcgaacgacctacaccgaactgagatacctacagcgtgagctatgagaaagcgccacgcttcccgaagggagaaaggcggacaggtatccggtaagcggcagggtcggaacaggagagcgcacgagggagcttccagggggaaacgcctggtatctttatagtcctgtcgggtttcgccacctctgacttgagcgtcgatttttgtgatgctcgtcaggggggcggagcctatggaaaaacgccagcaacgcggcctttttacggttcctggccttttgctggccttttgctcacatgttctttcctgcgttatcccctgattctgtggataaccgtattaccgcctttgagtgagctgataccgctcgccgcagccgaacgaccgagcgcagcgagtcagtgagcgaggaagcggaagagcgcccaatacgcaaaccgcctctccccgcgcgttggccgattcattaatgcagctggcacgacaggtttcccgactggaaagcgggcagtgagcgcaacgcaattaatgtgagttagctcactcattaggcaccccaggctttacactttatgcttccggctcgtatgttgtgtggaattgtgagcggataacaatttcacacaggaaacagctatgaccatgattacgccaagcgcgcaattaaccctcactaaagggaacaaaagctggaaacatgcatgaagttcctattccgaagttcctattctctagaaagtataggaacttc

SEQ ID NO: 281 - DNA, 3345 bp, Synthetic construct
  source 1..3345: mol_type = other DNA
ataaaacctgcaggcatgcaagcgatcgcggggccgcccccttcaccgagggcctatttcccatgattccttcatatttgcatatacgatacaaggctgttagagagataattggaattaatttgactgtaaacacaaagatattagtacaaaatacgtgacgtagaaagtaataatttcttgggtagtttgcagttttaaaattatgttttaaaatggactatcatatgcttaccgtaacttgaaagtatttcgatttcttggctttatatatcttgtggaaaggacgaaacaccgggaacgcgagcctccccaggtttcagagccaccagaagatatggcttcggtggcaagttgaaataaggctagtccgttatcaacttgaaaaagtggcaccgagtcggtgctttttttactagttctagagcggccccaattcgccctatagtgagtcgtattacgcgcgctcactggccgtcgttttacaacgtcgtgactgggaaaaccctggcgttacccaacttaatcgccttgcagcacatccccctttcgccagctggcgtaatagcgaagaggcccgcaccgatcgcccttcccaacagttgcgcagcctgaatggcgaatgggacgcgccctgtagcggcgcattaagcgcggcgggtgtggtggttacgcgcagcgtgaccgctacacttgccagcgccctagcgcccgctcctttcgctttcttcccttcctttctcgccacgttcgccggctttccccgtcaagctctaaatcgggggctccctttagggttccgatttagtgctttacggcacctcgaccccaaaaaacttgattagggtgatggttcacgtagtgggccatcgccctgatagacggtttttcgccctttgacgttggagtccacgttctttaatagtggactcttgttccaaactggaacaacactcaaccctatctcggtctattcttttgatttataagggattttgccgatttcggcctattggttaaaaaatgagctgatttaacaaaaatttaacgcgaattttaacaaaatattaacgcttacaatttaggtggcacttttcggggaaatgtgcgcggaacccctatttgtttatttttctaaatacattcaaatatgtatccgctcatgagacaataaccctgataaatgcttcaataatattgaaaaaggaagagtatgagtattcaacatttccgtgtcgcccttattcccttttttgcggcattttgccttcctgtttttgctcacccagaaacgctggtgaaagtaaaagatgctgaagatcagttgggtgcacgagtgggttacatcgaactggatctcaacagcggtaagatccttgagagttttcgccccgaagaacgttttccaatgatgagcacttttaaagttctgctatgtggcgcggtattatcccgtattgacgccgggcaagagcaactcggtcgccgcatacactattctcagaatgacttggttgagtactcaccagtcacagaaaagcatcttacggatggcatgacagtaagagaattatgcagtgctgccataaccatgagtgataacactgcggccaacttacttctgacaacgatcggaggaccgaaggagctaaccgcttttttgcacaacatgggggatcatgtaactcgccttgatcgttgggaaccggagctgaatgaagccataccaaacgacgagcgtgacaccacgatgcctgtagcaatggcaacaacgttgcgcaaactattaactggcgaactacttactctagcttcccggcaacaattaatagactggatggaggcggataaagttgcaggaccacttctgcgctcggcccttccggctggctggtttattgctgataaatctggagccggtgagcgtgggtctcgcggtatcattgcagcactggggccagatggtaagccctcccgtatcgtagttatctacacgacggggagtcaggcaactatggatgaacgaaatagacagatcgctgagataggtgcctcactgattaagcattggtaactgtcagaccaagtttactcatatatactttagattgatttaaaacttcatttttaatttaaaaggatctaggtgaagatcctttttgataatctcatgaccaaaatcccttaacgtgagttttcgttccactgagcgtcagaccccgtagaaaagatcaaaggatcttcttgagatcctttttttctgcgcgtaatctgctgcttgcaaacaaaaaaaccaccgctaccagcggtggtttgtttgccggatcaagagctaccaactctttttccgaaggtaactggcttcagcagagcgcagataccaaatactgtccttctagtgtagccgtagttaggccaccacttcaagaactctgtagcaccgcctacatacctcgctctgctaatcctgttaccagtggctgctgccagtggcgataagtcgtgtcttaccgggttggactcaagacgatagttaccggataaggcgcagcggtcgggctgaacggggggttcgtgcacacagcccagcttggagcgaacgacctacaccgaactgagatacctacagcgtgagctatgagaaagcgccacgcttcccgaagggagaaaggcggacaggtatccggtaagcggcagggtcggaacaggagagcgcacgagggagcttccagggggaaacgcctggtatctttatagtcctgtcgggtttcgccacctctgacttgagcgtcgatttttgtgatgctcgtcaggggggcggagcctatggaaaaacgccagcaacgcggcctttttacggttcctggccttttgctggccttttgctcacatgttctttcctgcgttatcccctgattctgtggataaccgtattaccgcctttgagtgagctgataccgctcgccgcagccgaacgaccgagcgcagcgagtcagtgagcgaggaagcggaagagcgcccaatacgcaaaccgcctctccccgcgcgttggccgattcattaatgcagctggcacgacaggtttcccgactggaaagcgggcagtgagcgcaacgcaattaatgtgagttagctcactcattaggcaccccaggctttacactttatgcttccggctcgtatgttgtgtggaattgtgagcggataacaatttcacacaggaaacagctatgaccatgattacgccaagcgcgcaattaaccctcactaaagggaacaaaagctggaaacatgcatgaagttcctattccgaagttcctattctctagaaagtataggaacttc

SEQ ID NO: 282 - DNA, 3345 bp, Synthetic construct
  source 1..3345: mol_type = other DNA
ataaaacctgcaggcatgcaagcgatcgcggggccgcccccttcaccgagggcctatttcccatgattccttcatatttgcatatacgatacaaggctgttagagagataattggaattaatttgactgtaaacacaaagatattagtacaaaatacgtgacgtagaaagtaataatttcttgggtagtttgcagttttaaaattatgttttaaaatggactatcatatgcttaccgtaacttgaaagtatttcgatttcttggctttatatatcttgtggaaaggacgaaacaccgggtcagtcttcgttgtggggtttcagagccaccagaagatatggcttcggtggcaagttgaaataaggctagtccgttatcaacttgaaaaagtggcaccgagtcggtgctttttttactagttctagagcggccccaattcgccctatagtgagtcgtattacgcgcgctcactggccgtcgttttacaacgtcgtgactgggaaaaccctggcgttacccaacttaatcgccttgcagcacatccccctttcgccagctggcgtaatagcgaagaggcccgcaccgatcgcccttcccaacagttgcgcagcctgaatggcgaatgggacgcgccctgtagcggcgcattaagcgcggcgggtgtggtggttacgcgcagcgtgaccgctacacttgccagcgccctagcgcccgctcctttcgctttcttcccttcctttctcgccacgttcgccggctttccccgtcaagctctaaatcgggggctccctttagggttccgatttagtgctttacggcacctcgaccccaaaaaacttgattagggtgatggttcacgtagtgggccatcgccctgatagacggtttttcgccctttgacgttggagtccacgttctttaatagtggactcttgttccaaactggaacaacactcaaccctatctcggtctattcttttgatttataagggattttgccgatttcggcctattggttaaaaaatgagctgatttaacaaaaatttaacgcgaattttaacaaaatattaacgcttacaatttaggtggcacttttcggggaaatgtgcgcggaacccctatttgtttatttttctaaatacattcaaatatgtatccgctcatgagacaataaccctgataaatgcttcaataatattgaaaaaggaagagtatgagtattcaacatttccgtgtcgcccttattcccttttttgcggcattttgccttcctgtttttgctcacccagaaacgctggtgaaagtaaaagatgctgaagatcagttgggtgcacgagtgggttacatcgaactggatctcaacagcggtaagatccttgagagttttcgccccgaagaacgttttccaatgatgagcacttttaaagttctgctatgtggcgcggtattatcccgtattgacgccgggcaagagcaactcggtcgccgcatacactattctcagaatgacttggttgagtactcaccagtcacagaaaagcatcttacggatggcatgacagtaagagaattatgcagtgctgccataaccatgagtgataacactgcggccaacttacttctgacaacgatcggaggaccgaaggagctaaccgcttttttgcacaacatgggggatcatgtaactcgccttgatcgttgggaaccggagctgaatgaagccataccaaacgacgagcgtgacaccacgatgcctgtagcaatggcaacaacgttgcgcaaactattaactggcgaactacttactctagcttcccggcaacaattaatagactggatggaggcggataaagttgcaggaccacttctgcgctcggcccttccggctggctggtttattgctgataaatctggagccggtgagcgtgggtctcgcggtatcattgcagcactggggccagatggtaagccctcccgtatcgtagttatctacacgacggggagtcaggcaactatggatgaacgaaatagacagatcgctgagataggtgcctcactgattaagcattggtaactgtcagaccaagtttactcatatatactttagattgatttaaaacttcatttttaatttaaaaggatctaggtgaagatcctttttgataatctcatgaccaaaatcccttaacgtgagttttcgttccactgagcgtcagaccccgtagaaaagatcaaaggatcttcttgagatcctttttttctgcgcgtaatctgctgcttgcaaacaaaaaaaccaccgctaccagcggtggtttgtttgccggatcaagagctaccaactctttttccgaaggtaactggcttcagcagagcgcagataccaaatactgtccttctagtgtagccgtagttaggccaccacttcaagaactctgtagcaccgcctacatacctcgctctgctaatcctgttaccagtggctgctgccagtggcgataagtcgtgtcttaccgggttggactcaagacgatagttaccggataaggcgcagcggtcgggctgaacggggggttcgtgcacacagcccagcttggagcgaacgacctacaccgaactgagatacctacagcgtgagctatgagaaagcgccacgcttcccgaagggagaaaggcggacaggtatccggtaagcggcagggtcggaacaggagagcgcacgagggagcttccagggggaaacgcctggtatctttatagtcctgtcgggtttcgccacctctgacttgagcgtcgatttttgtgatgctcgtcaggggggcggagcctatggaaaaacgccagcaacgcggcctttttacggttcctggccttttgctggccttttgctcacatgttctttcctgcgttatcccctgattctgtggataaccgtattaccgcctttgagtgagctgataccgctcgccgcagccgaacgaccgagcgcagcgagtcagtgagcgaggaagcggaagagcgcccaatacgcaaaccgcctctccccgcgcgttggccgattcattaatgcagctggcacgacaggtttcccgactggaaagcgggcagtgagcgcaacgcaattaatgtgagttagctcactcattaggcaccccaggctttacactttatgcttccggctcgtatgttgtgtggaattgtgagcggataacaatttcacacaggaaacagctatgaccatgattacgccaagcgcgcaattaaccctcactaaagggaacaaaagctggaaacatgcatgaagttcctattccgaagttcctattctctagaaagtataggaacttc

SEQ ID NO: 283 - DNA, 3375 bp, Synthetic construct
  source 1..3375: mol_type = other DNA
ataaaacctgcaggcatgcaagcgatcgcggggccgcccccttcaccgagggcctatttcccatgattccttcatatttgcatatacgatacaaggctgttagagagataattggaattaatttgactgtaaacacaaagatattagtacaaaatacgtgacgtagaaagtaataatttcttgggtagtttgcagttttaaaattatgttttaaaatggactatcatatgcttaccgtaacttgaaagtatttcgatttcttggctttatatatcttgtggaaaggacgaaacaccgggtcagtcttcgttgtggggtttaagagctatgctggaaacagcatagcaagtttaaataaggctagtccgttatcaacttgaaaaagtggcaccgagtcggtgctttttttgatccaagggtgggcgcgccaaggcccgcggggccactagttctagagcggccccaattcgccctatagtgagtcgtattacgcgcgctcactggccgtcgttttacaacgtcgtgactgggaaaaccctggcgttacccaacttaatcgccttgcagcacatccccctttcgccagctggcgtaatagcgaagaggcccgcaccgatcgcccttcccaacagttgcgcagcctgaatggcgaatgggacgcgccctgtagcggcgcattaagcgcggcgggtgtggtggttacgcgcagcgtgaccgctacacttgccagcgccctagcgcccgctcctttcgctttcttcccttcctttctcgccacgttcgccggctttccccgtcaagctctaaatcgggggctccctttagggttccgatttagtgctttacggcacctcgaccccaaaaaacttgattagggtgatggttcacgtagtgggccatcgccctgatagacggtttttcgccctttgacgttggagtccacgttctttaatagtggactcttgttccaaactggaacaacactcaaccctatctcggtctattcttttgatttataagggattttgccgatttcggcctattggttaaaaaatgagctgatttaacaaaaatttaacgcgaattttaacaaaatattaacgcttacaatttaggtggcacttttcggggaaatgtgcgcggaacccctatttgtttatttttctaaatacattcaaatatgtatccgctcatgagacaataaccctgataaatgcttcaataatattgaaaaaggaagagtatgagtattcaacatttccgtgtcgcccttattcccttttttgcggcattttgccttcctgtttttgctcacccagaaacgctggtgaaagtaaaagatgctgaagatcagttgggtgcacgagtgggttacatcgaactggatctcaacagcggtaagatccttgagagttttcgccccgaagaacgttttccaatgatgagcacttttaaagttctgctatgtggcgcggtattatcccgtattgacgccgggcaagagcaactcggtcgccgcatacactattctcagaatgacttggttgagtactcaccagtcacagaaaagcatcttacggatggcatgacagtaagagaattatgcagtgctgccataaccatgagtgataacactgcggccaacttacttctgacaacgatcggaggaccgaaggagctaaccgcttttttgcacaacatgggggatcatgtaactcgccttgatcgttgggaaccggagctgaatgaagccataccaaacgacgagcgtgacaccacgatgcctgtagcaatggcaacaacgttgcgcaaactattaactggcgaactacttactctagcttcccggcaacaattaatagactggatggaggcggataaagttgcaggaccacttctgcgctcggcccttccggctggctggtttattgctgataaatctggagccggtgagcgtgggtctcgcggtatcattgcagcactggggccagatggtaagccctcccgtatcgtagttatctacacgacggggagtcaggcaactatggatgaacgaaatagacagatcgctgagataggtgcctcactgattaagcattggtaactgtcagaccaagtttactcatatatactttagattgatttaaaacttcatttttaatttaaaaggatctaggtgaagatcctttttgataatctcatgaccaaaatcccttaacgtgagttttcgttccactgagcgtcagaccccgtagaaaagatcaaaggatcttcttgagatcctttttttctgcgcgtaatctgctgcttgcaaacaaaaaaaccaccgctaccagcggtggtttgtttgccggatcaagagctaccaactctttttccgaaggtaactggcttcagcagagcgcagataccaaatactgtccttctagtgtagccgtagttaggccaccacttcaagaactctgtagcaccgcctacatacctcgctctgctaatcctgttaccagtggctgctgccagtggcgataagtcgtgtcttaccgggttggactcaagacgatagttaccggataaggcgcagcggtcgggctgaacggggggttcgtgcacacagcccagcttggagcgaacgacctacaccgaactgagatacctacagcgtgagctatgagaaagcgccacgcttcccgaagggagaaaggcggacaggtatccggtaagcggcagggtcggaacaggagagcgcacgagggagcttccagggggaaacgcctggtatctttatagtcctgtcgggtttcgccacctctgacttgagcgtcgatttttgtgatgctcgtcaggggggcggagcctatggaaaaacgccagcaacgcggcctttttacggttcctggccttttgctggccttttgctcacatgttctttcctgcgttatcccctgattctgtggataaccgtattaccgcctttgagtgagctgataccgctcgccgcagccgaacgaccgagcgcagcgagtcagtgagcgaggaagcggaagagcgcccaatacgcaaaccgcctctccccgcgcgttggccgattcattaatgcagctggcacgacaggtttcccgactggaaagcgggcagtgagcgcaacgcaattaatgtgagttagctcactcattaggcaccccaggctttacactttatgcttccggctcgtatgttgtgtggaattgtgagcggataacaatttcacacaggaaacagctatgaccatgattacgccaagcgcgcaattaaccctcactaaagggaacaaaagctggaaacatgcatgaagttcctattccgaagttcctattctctagaaagtataggaacttc

SEQ ID NO: 284 - DNA, 9326 bp, Synthetic construct
  source 1..9326: mol_type = other DNA
ataaatcaatattggctattggccattgcatacgttgtatccatatcataatatgtacatttatattggctcatgtccaacattaccgccatgttgacattgattattgactagttattaatagtaatcaattacggggtcattagttcatagcccatatatggagttccgcgttacataacttacggtaaatggcccgcctggctgaccgcccaacgacccccgcccattgacgtcaataatgacgtatgttcccatagtaacgccaatagggactttccattgacgtcaatgggtggagtatttacggtaaactgcccacttggcagtacatcaagtgtatcatatgccaagtacgccccctattgacgtcaatgacggtaaatggcccgcctggcattatgcccagtacatgaccttatgggactttcctacttggcagtacatctacgtattagtcatcgctattaccatggtgatgcggttttggcagtacatcaatgggcgtggatagcggtttgactcacggggatttccaagtctccaccccattgacgtcaatgggagtttgttttggcaccaaaatcaacgggactttccaaaatgtcgtaacaactccgccccattgacgcaaatgggcggtaggcgtgtacggtgggaggtctatataagcagagctcgtttagtgaaccgtcagatcgcctggagacgccatccacgctgttttgacctccatagaagacaccgggaccgatccagcctccgcggccccaagcttgggcatcgttctgtgttgtctctgtctgactgtgtttctgtatttgtctgaaaatatgggccagactgttaccactcccttaagtttgaccttaggtcactggaaagatgtcgagcggatcgctcacaaccagtcggtagatgtcaagaagagacgttgggttaccttctgctctgcagaatggccaacctttaacgtcggatggccgcgagacggcacctttaaccgagacctcatcacccaggttaagatcaaggtcttttcacctggcccgcatggacacccagaccaggtcccctacatcgtgacctgggaagccttggcttttgacccccctccctgggtcaagccctttgtacaccctaagcctccgcctcctcttcctccatccgccccgtctctcccccttgaacctcctcgttcgaccccgcctcgatcctccctttatccagccctcactccttctctaggcgccaaacctaaacctcaagttctttctgacagtggggggccgctcatcgacctacttacagaagaccccccgccttatagggacccaagaccacccccttccgacagggacggaaatggtggagaagcgacccctgcgggagaggcaccggacccctccccaatggcatctcgcctacgtgggagacgggagccccctgtggccgactccactacctcgcaggcattccccctccgcgcaggaggaaacggacagcttcaatactggccgttctcctcttctgacctttacaactggaaaaataataacccttctttttctgaagatccaggtaaactgacagctctgatcgagtctgtcctcatcacccatcagcccacctgggacgactgtcagcagctgttggggactctgctgaccggagaagaaaaacaacgggtgctcttagaggctagaaaggcggtgcggggcgatgatgggcgccccactcaactgcccaatgaagtcgatgccgcttttcccctcgagcgcccagactgggattacaccacccaggcaggtaggaaccacctagtccactatcgccagttgctcctagcgggtctccaaaacgcgggcagaagccccaccaatttggccaaggtaaaaggaataacacaagggcccaatgagtctccctcggccttcctagagagacttaaggaagcctatcgcaggtacactccttatgaccctgaggacccagggcaagaaactaatgtgtctatgtctttcatttggcagtctgccccagacattgggagaaagttagagaggttagaagatttaaaaaacaagacgcttggagatttggttagagaggcagaaaagatctttaataaacgagaaaccccggaagaaagagaggaacgtatcaggagagaaacagaggaaaaagaagaacgccgtaggacagaggatgagcagaaagagaaagaaagagatcgtaggagacatagagagatgagcaagctattggccactgtcgttagtggacagaaacaggatagacagggaggagaacgaaggaggtcccaactcgatcgcgaccagtgtgcctactgcaaagaaaaggggcactgggctaaagattgtcccaagaaaccacgaggacctcggggaccaagaccccagacctccctcctgaccctagatgactagggaggtcagggtcaggagcccccccctgaacccaggataaccctcaaagtcggggggcaacccgtcaccttcctggtagatactggggcccaacactccgtgctgacccaaaatcctggacccctaagtgataagtctgcctgggtccaaggggctactggaggaaagcggtatcgctggaccacggatcgcaaagtacatctagctaccggtaaggtcacccactctttcctccatgtaccagactgtccctatcctctgttaggaagagatttgctgactaaactaaaagcccaaatccactttgagggatcaggagctcaggttatgggaccaatggggcagcccctgcaagtgttgaccctaaatatagaagatgagtatcggctacatgagacctcaaaagagccagatgtttctctagggtccacatggctgtctgattttcctcaggcctgggcggaaaccgggggcatgggactggcagttcgccaagctcctctgatcatacctctgaaagcaacctctacccccgtgtccataaaacaataccccatgtcacaagaagccagactggggatcaagccccacatacagagactgttggaccagggaatactggtaccctgccagtccccctggaacacgcccctgctacccgttaagaaaccagggactaatgattataggcctgtccaggatctgagagaagtcaacaagcgggtggaagacatccaccccaccgtgcccaacccttacaacctcttgagcgggctcccaccgtcccaccagtggtacactgtgcttgatttaaaggatgcctttttctgcctgagactccaccccaccagtcagcctctcttcgcctttgagtggagagatccagagatgggaatctcaggacaattgacctggaccagactcccacagggtttcaaaaacagtcccaccctgtttgatgaggcactgcacagagacctagcagacttccggatccagcacccagacttgatcctgctacagtacgtggatgacttactgctggccgccacttctgagctagactgccaacaaggtactcgggccctgttacaaaccctagggaacctcgggtatcgggcctcggccaagaaagcccaaatttgccagaaacaggtcaagtatctggggtatcttctaaaagagggtcagagatggctgactgaggccagaaaagagactgtgatggggcagcctactccgaagacccctcgacaactaagggagttcctagggacggcaggcttctgtcgcctctggatccctgggtttgcagaaatggcagcccccttgtaccctctcaccaaaacggggactctgtttaattggggcccagaccaacaaaaggcctatcaagaaatcaagcaagctcttctaactgccccagccctggggttgccagatttgactaagccctttgaactctttgtcgacgagaagcagggctacgccaaaggtgtcctaacgcaaaaactgggaccttggcgtcggccggtggcctacctgtccaaaaagctagacccagtagcagctgggtggcccccttgcctacggatggtagcagccattgccgtactgacaaaggatgcaggcaagctaaccatgggacagccactagtcattctggccccccatgcagtagaggcactagtcaaacaaccccccgaccgctggctttccaacgcccggatgactcactatcaggccttgcttttggacacggaccgggtccagttcggaccggtggtagccctgaacccggctacgctgctcccactgcctgaggaagggctgcaacacaactgccttgatatcctggccgaagcccacggaacccgacccgacctaacggaccagccgctcccagacgccgaccacacctggtacacggatggaagcagtctcttacaagagggacagcgtaaggcgggagctgcggtgaccaccgagaccgaggtaatctgggctaaagccctgccagccgggacatccgctcagcgggctgaactgatagcactcacccaggccctaaagatggcagaaggtaagaagctaaatgtttatactgatagccgttatgcttttgctactgcccatatccatggagaaatatacagaaggcgtgggttgctcacatcagaaggcaaagagatcaaaaataaagacgagatcttggccctactaaaagccctctttctgcccaaaagacttagcataatccattgtccaggacatcaaaagggacacagcgccgaggctagaggcaaccggatggctgaccaagcggcccgaaaggcagccatcacagagactccagacacctctaccctcctcatagaaaattcatcaccctacacctcagaacattttcattacacagtgactgatataaaggacctaaccaagttgggggccatttatgataaaacaaagaagtattgggtctaccaaggaaaacctgtgatgcctgaccagtttacttttgaattattagactttcttcatcagctgactcacctcagcttctcaaaaatgaaggctctcctagagagaagccacagtccctactacatgctgaaccgggatcgaacactcaaaaatatcactgagacctgcaaagcttgtgcacaagtcaacgccagcaagtctgccgttaaacagggaactagggtccgcgggcatcggcccggcactcattgggagatcgatttcaccgagataaagcccggattgtatggctataaatatcttctagtttttatagataccttttctggctggatagaagccttcccaaccaagaaagaaaccgccaaggtcgtaaccaagaagctactagaggagatcttccccaggttcggcatgcctcaggtattgggaactgacaatgggcctgccttcgtctccaaggtgagtcagacagtggccgatctgttggggattgattggaaattacattgtgcatacagaccccaaagctcaggccaggtagaaagaatgaatagaaccatcaaggagactttaactaaattaacgcttgcaactggctctagagactgggtgctcctactccccttagccctgtaccgagcccgcaacacgccgggcccccatggcctcaccccatatgagatcttatatggggcacccccgccccttgtaaacttccctgaccctgacatgacaagagttactaacagcccctctctccaagctcacttacaggctctctacttagtccagcacgaagtctggagacctctggcggcagcctaccaagaacaactggaccgaccggtggtacctcacccttaccgagtcggcgacacagtgtgggtccgccgacaccagactaagaacctagaacctcgctggaaaggaccttacacagtcctgctgaccacccccaccgccctcaaagtagacggcatcgcagcttggatacacgccgcccacgtgaaggctgccgaccccgggggtggaccatcctctagactgacatggcgcgttcaacgctctcaaaaccccttaaaaataaggttgacgcgtcaacccgcgaggccccctaatccccttaattcttctgatgctcagaggggtcagtatcgaattcctgcagccccgctgatcagcctcgactgtgccttctagttgccagccatctgttgtttgcccctcccccgtgccttccttgaccctggaaggtgccactcccactgtcctttcctaataaaatgaggaaattgcatcgcattgtctgagtaggtgtcattctattctggggggtggggtggggcaggacagcaagggggaggattgggaagacaatagcaggcatgctggggatgcggtgggctctatggcttctgaggcggaaagaaccagctggggctcgatcctctagagcggccgccaccgcggtggagctccaattcgccctatagtgagtcgtattacaattcactggccgtcgttttacaacgtcgtgactgggaaaaccctggcgttacccaacttaatcgccttgcagcacatccccctttcgccagctggcgtaatagcgaagaggcccgcaccgatcgcccttcccaacagttgcgcagcctgaatggcgaatgggacgcgccctgtagcggcgcattaagcgcggcgggtgtggtggttacgcgcagcgtgaccgctacacttgccagcgccctagcgcccgctcctttcgctttcttcccttcctttctcgccacgttcgccggctttccccgtcaagctctaaatcgggggctccctttagggttccgatttagtgctttacggcacctcgaccccaaaaaacttgattagggtgatggttcacgtagtgggccatcgccctgatagacggtttttcgccctttgacgttggagtccacgttctttaatagtggactcttgttccaaactggaacaacactcaaccctatctcggtctattcttttgatttataagggattttgccgatttcggcctattggttaaaaaatgagctgatttaacaaaaatttaacgcgaattttaacaaaatattaacgcttacaatttaggtggcacttttcggggaaatgtgcgcggaacccctatttgtttatttttctaaatacattcaaatatgtatccgctcatgagacaataaccctgataaatgcttcaataatattgaaaaaggaagagtatgagtattcaacatttccgtgtcgcccttattcccttttttgcggcattttgccttcctgtttttgctcacccagaaacgctggtgaaagtaaaagatgctgaagatcagttgggtgcacgagtgggttacatcgaactggatctcaacagcggtaagatccttgagagttttcgccccgaagaacgttttccaatgatgagcacttttaaagttctgctatgtggcgcggtattatcccgtattgacgccgggcaagagcaactcggtcgccgcatacactattctcagaatgacttggttgagtactcaccagtcacagaaaagcatcttacggatggcatgacagtaagagaattatgcagtgctgccataaccatgagtgataacactgcggccaacttacttctgacaacgatcggaggaccgaaggagctaaccgcttttttgcacaacatgggggatcatgtaactcgccttgatcgttgggaaccggagctgaatgaagccataccaaacgacgagcgtgacaccacgatgcctgtagcaatggcaacaacgttgcgcaaactattaactggcgaactacttactctagcttcccggcaacaattaatagactggatggaggcggataaagttgcaggaccacttctgcgctcggcccttccggctggctggtttattgctgataaatctggagccggtgagcgtgggtctcgcggtatcattgcagcactggggccagatggtaagccctcccgtatcgtagttatctacacgacggggagtcaggcaactatggatgaacgaaatagacagatcgctgagataggtgcctcactgattaagcattggtaactgtcagaccaagtttactcatatatactttagattgatttaaaacttcatttttaatttaaaaggatctaggtgaagatcctttttgataatctcatgaccaaaatcccttaacgtgagttttcgttccactgagcgtcagaccccgtagaaaagatcaaaggatcttcttgagatcctttttttctgcgcgtaatctgctgcttgcaaacaaaaaaaccaccgctaccagcggtggtttgtttgccggatcaagagctaccaactctttttccgaaggtaactggcttcagcagagcgcagataccaaatactgttcttctagtgtagccgtagttaggccaccacttcaagaactctgtagcaccgcctacatacctcgctctgctaatcctgttaccagtggctgctgccagtggcgataagtcgtgtcttaccgggttggactcaagacgatagttaccggataaggcgcagcggtcgggctgaacggggggttcgtgcacacagcccagcttggagcgaacgacctacaccgaactgagatacctacagcgtgagctatgagaaagcgccacgcttcccgaagggagaaaggcggacaggtatccggtaagcggcagggtcggaacaggagagcgcacgagggagcttccagggggaaacgcctggtatctttatagtcctgtcgggtttcgccacctctgacttgagcgtcgatttttgtgatgctcgtcaggggggcggagcctatggaaaaacgccagcaacgcggcctttttacggttcctggccttttgctggccttttgctcacatgttctttcctgcgttatcccctgattctgtggataaccgtattaccgcctttgagtgagctgataccgctcgccgcagccgaacgaccgagcgcagcgagtcagtgagcgaggaagcggaagagcgcccaatacgcaaaccgcctctccccgcgcgttggccgattcattaatgcagctggcacgacaggtttcccgactggaaagcgggcagtgagcgcaacgcaattaatgtgagttagctcactcattaggcaccccaggctttacactttatgcttccggctcgtatgttgtgtggaattgtgagcggataacaatttcacacaggaaacagctatgaccatgattacgccaagctcgaaattaaccctcactaaagggaacaaaagctggtaccgggccccccctcgagatccggccattagccatattattcattggttatatagc

SEQ ID NO: 285 - DNA, 11365 bp, Synthetic construct
  source 1..11365: mol_type = other DNA
atgggccagactgttaccactcccttaagtttgaccttaggtcactggaaagatgtcgagcggatcgctcacaaccagtcggtagatgtcaagaagagacgttgggttaccttctgctctgcagaatggccaacctttaacgtcggatggccgcgagacggcacctttaaccgagacctcatcacccaggttaagatcaaggtcttttcacctggcccgcatggacacccagaccaggtcccctacatcgtgacctgggaagccttggcttttgacccccctccctgggtcaagccctttgtacaccctaagcctccgcctcctcttcctccatccgccccgtctctcccccttgaacctcctcgttcgaccccgcctcgatcctccctttatccagccctcactccttctctaggcgccaaacctaaacctcaagttctttctgacagtggggggccgctcatcgacctacttacagaagaccccccgccttatagggacccaagaccacccccttccgacagggacggaaatggtggagaagcgacccctgcgggagaggcaccggacccctccccaatggcatctcgcctacgtgggagacgggagccccctgtggccgactccactacctcgcaggcattccccctccgcgcaggaggaaacggacagcttcaatactggccgttctcctcttctgacctttacaactggaaaaataataacccttctttttctgaagatccaggtaaactgacagctctgatcgagtctgtcctcatcacccatcagcccacctgggacgactgtcagcagctgttggggactctgctgaccggagaagaaaaacaacgggtgctcttagaggctagaaaggcggtgcggggcgatgatgggcgccccactcaactgcccaatgaagtcgatgccgcttttcccctcgagcgcccagactgggattacaccacccaggcaggtaggaaccacctagtccactatcgccagttgctcctagcgggtctccaaaacgcgggcagaagccccaccaatttggccaaggtaaaaggaataacacaagggcccaatgagtctccctcggccttcctagagagacttaaggaagcctatcgcaggtacactccttatgaccctgaggacccagggcaagaaactaatgtgtctatgtctttcatttggcagtctgccccagacattgggagaaagttagagaggttagaagatttaaaaaacaagacgcttggagatttggttagagaggcagaaaagatctttaataaacgagaaaccccggaagaaagagaggaacgtatcaggagagaaacagaggaaaaagaagaacgccgtaggacagaggatgagcagaaagagaaagaaagagatcgtaggagacatagagagatgagcaagctattggccactgtcgttagtggacagaaacaggatagacagggaggagaacgaaggaggtcccaactcgatcgcgaccagtgtgcctactgcaaagaaaaggggcactgggctaaagattgtcccaagaaaccacgaggacctcggggaccaagaccccagacctccctcctgaccctagatgactctggcggctcacttcaactgcctccacttgaaagactgacactgggatcattacaattacctcctttagaacgattaacactcggttcactacagcttccgcctcttgagagattgacattaacgtccacgctgctaatggagaactcgtctggagattacaaagacgatgacgataagaaacggacagccgacggaagcgagttcgagtcaccaaagaagaagcggaaagtctctgaggtggagttttcccacgagtactggatgagacatgccctgaccctggccaagagggcacgggatgagagggaggtgcctgtgggagccgtgctggtgctgaacaatagagtgatcggcgagggctggaacagagccatcggcctgcacgacccaacagcccatgccgaaattatggccctgagacagggcggcctggtcatgcagaactacagactgattgacgccaccctgtacgtgacattcgagccttgcgtgatgtgcgccggcgccatgatccactctaggatcggccgcgtggtgtttggcgtgaggaactcaaaaagaggcgccgcaggctccctgatgaacgtgctgaactaccccggcatgaatcaccgcgtcgaaattaccgagggaatcctggcagatgaatgtgccgccctgctgtgcgatttctatcggatgcctagacaggtgttcaatgctcagaagaaggcccagagctccatcaactccggaggatctagcggaggctcctctggctctgagacacctggcacaagcgagagcgcaacacctgaaagcagcgggggcagcagcggggggtcagacaagaagtacagcatcggcctggccatcggcaccaactctgtgggctgggccgtgatcaccgacgagtacaaggtgcccagcaagaaattcaaggtgctgggcaacaccgaccggcacagcatcaagaagaacctgatcggagccctgctgttcgacagcggcgaaacagccgaggccacccggctgaagagaaccgccagaagaagatacaccagacggaagaaccggatctgctatctgcaagagatcttcagcaacgagatggccaaggtggacgacagcttcttccacagactggaagagtccttcctggtggaagaggataagaagcacgagcggcaccccatcttcggcaacatcgtggacgaggtggcctaccacgagaagtaccccaccatctaccacctgagaaagaaactggtggacagcaccgacaaggccgacctgcggctgatctatctggccctggcccacatgatcaagttccggggccacttcctgatcgagggcgacctgaaccccgacaacagcgacgtggacaagctgttcatccagctggtgcagacctacaaccagctgttcgaggaaaaccccatcaacgccagcggcgtggacgccaaggccatcctgtctgccagactgagcaagagcagacggctggaaaatctgatcgcccagctgcccggcgagaagaagaatggcctgttcggaaacctgattgccctgagcctgggcctgacccccaacttcaagagcaacttcgacctggccgaggatgccaaactgcagctgagcaaggacacctacgacgacgacctggacaacctgctggcccagatcggcgaccagtacgccgacctgtttctggccgccaagaacctgtccgacgccatcctgctgagcgacatcctgagagtgaacaccgagatcaccaaggcccccctgagcgcctctatgatcaagagatacgacgagcaccaccaggacctgaccctgctgaaagctctcgtgcggcagcagctgcctgagaagtacaaagagattttcttcgaccagagcaagaacggctacgccggctacattgacggcggagccagccaggaagagttctacaagttcatcaagcccatcctggaaaagatggacggcaccgaggaactgctcgtgaagctgaacagagaggacctgctgcggaagcagcggaccttcgacaacggcagcatcccccaccagatccacctgggagagctgcacgccattctgcggcggcaggaagatttttacccattcctgaaggacaaccgggaaaagatcgagaagatcctgaccttccgcatcccctactacgtgggccctctggccaggggaaacagcagattcgcctggatgaccagaaagagcgaggaaaccatcaccccctggaacttcgaggaagtggtggacaagggcgcttccgcccagagcttcatcgagcggatgaccaacttcgataagaacctgcccaacgagaaggtgctgcccaagcacagcctgctgtacgagtacttcaccgtgtataacgagctgaccaaagtgaaatacgtgaccgagggaatgagaaagcccgccttcctgagcggcgagcagaaaaaggccatcgtggacctgctgttcaagaccaaccggaaagtgaccgtgaagcagctgaaagaggactacttcaagaaaatcgagtgcttcgactccgtggaaatctccggcgtggaagatcggttcaacgcctccctgggcacataccacgatctgctgaaaattatcaaggacaaggacttcctggacaatgaggaaaacgaggacattctggaagatatcgtgctgaccctgacactgtttgaggacagagagatgatcgaggaacggctgaaaacctatgcccacctgttcgacgacaaagtgatgaagcagctgaagcggcggagatacaccggctggggcaggctgagccggaagctgatcaacggcatccgggacaagcagtccggcaagacaatcctggatttcctgaagtccgacggcttcgccaacagaaacttcatgcagctgatccacgacgacagcctgacctttaaagaggacatccagaaagcccaggtgtccggccagggcgatagcctgcacgagcacattgccaatctggccggcagccccgccattaagaagggcatcctgcagacagtgaaggtggtggacgagctcgtgaaagtgatgggccggcacaagcccgagaacatcgtgatcgaaatggccagagagaaccagaccacccagaagggacagaagaacagccgcgagagaatgaagcggatcgaagagggcatcaaagagctgggcagccagatcctgaaagaacaccccgtggaaaacacccagctgcagaacgagaagctgtacctgtactacctgcagaatgggcgggatatgtacgtggaccaggaactggacatcaaccggctgtccgactacgatgtggaccatatcgtgcctcagagctttctgaaggacgactccatcgacaacaaggtgctgaccagaagcgacaagaaccggggcaagagcgacaacgtgccctccgaagaggtcgtgaagaagatgaagaactactggcggcagctgctgaacgccaagctgattacccagagaaagttcgacaatctgaccaaggccgagagaggcggcctgagcgaactggataaggccggcttcatcaagagacagctggtggaaacccggcagatcacaaagcacgtggcacagatcctggactcccggatgaacactaagtacgacgagaatgacaagctgatccgggaagtgaaagtgatcaccctgaagtccaagctggtgtccgatttccggaaggatttccagttttacaaagtgcgcgagatcaacaactaccaccacgcccacgacgcctacctgaacgccgtcgtgggaaccgccctgatcaaaaagtaccctaagctggaaagcgagtttgtgtacggcgactacaaggtgtacgacgtgcggaagatgatcgccaagagcgagcaggaaatcggcaaggctaccgccaagtacttcttctacagcaacatcatgaactttttcaagaccgagattaccctggccaacggcgagatccggaagcggcctctgatcgagacaaacggcgaaaccggggagatcgtgtgggataagggccgggattttgccaccgtgcggaaagtgctgagcatgccccaagtgaatatcgtgaaaaagaccgaggtgcagacaggcggcttcagcaaagagtctatcctgcccaagaggaacagcgataagctgatcgccagaaagaaggactgggaccctaagaagtacggcggcttcgacagccccaccgtggcctattctgtgctggtggtggccaaagtggaaaagggcaagtccaagaaactgaagagtgtgaaagagctgctggggatcaccatcatggaaagaagcagcttcgagaagaatcccatcgactttctggaagccaagggctacaaagaagtgaaaaaggacctgatcatcaagctgcctaagtactccctgttcgagctggaaaacggccggaagagaatgctggcctctgccggcgaactgcagaagggaaacgaactggccctgccctccaaatatgtgaacttcctgtacctggccagccactatgagaagctgaagggctcccccgaggataatgagcagaaacagctgtttgtggaacagcacaagcactacctggacgagatcatcgagcagatcagcgagttctccaagagagtgatcctggccgacgctaatctggacaaagtgctgtccgcctacaacaagcaccgggataagcccatcagagagcaggccgagaatatcatccacctgtttaccctgaccaatctgggagcccctgccgccttcaagtactttgacaccaccatcgaccggaagaggtacaccagcaccaaagaggtgctggacgccaccctgatccaccagagcatcaccggcctgtacgagacacggatcgacctgtctcagctgggaggtgactctggcggctcaaaaagaaccgccgacggcagcgaattcgagcccaagaagaagaggaaagtctgagatctttttccctctgccaaaaattatggggacatcatgaagccccttgagcatctgacttctggctaataaaggaaatttattttcattgcaatagtgtgttggaattttttgtgtctctcactcggaaggacatatgggagggcaaatcatttaaaacatcagaatgagtatttggtttagagtttggcaacatatgcccatatgctggctgccatgaacaaaggttggctataaagaggtcatcagtatatgaaacagccccctgctgtccattccttattccatagaaaagccttgacttgaggttagattttttttatattttgttttgtgttatttttttctttaacatccctaaaattttccttacatgttttactagccagatttttcctcctctcctgactactcccagtcatagctgtccctcttctcttatggagatccctcgacggatcggccgcaattcgtaaccatgtcatagctgtttcctgtgtgaaattgttatccgctcacaattccacacaacatacgagccggaagcataaagtgtaaagcctggggtgcctaatgagtgagctaactcacattaattgcgttgcgctcactgcccgctttccagtcgggaaacctgtcgtgccagctgcattaatgaatcggccaacgcgcggggagaggcggtttgcgtattgggcgctcttccgcttcctcgctcactgactcgctgcgctcggtcgttcggctgcggcgagcggtatcagctcactcaaaggcggtaatacggttatccacagaatcaggggataacgcaggaaagaacatgtgagcaaaaggccagcaaaaggccaggaaccgtaaaaaggccgcgttgctggcgtttttccataggctccgcccccctgacgagcatcacaaaaatcgacgctcaagtcagaggtggcgaaacccgacaggactataaagataccaggcgtttccccctggaagctccctcgtgcgctctcctgttccgaccctgccgcttaccggatacctgtccgcctttctcccttcgggaagcgtggcgctttctcatagctcacgctgtaggtatctcagttcggtgtaggtcgttcgctccaagctgggctgtgtgcacgaaccccccgttcagcccgaccgctgcgccttatccggtaactatcgtcttgagtccaacccggtaagacacgacttatcgccactggcagcagccactggtaacaggattagcagagcgaggtatgtaggcggtgctacagagttcttgaagtggtggcctaactacggctacactagaagaacagtatttggtatctgcgctctgctgaagccagttaccttcggaaaaagagttggtagctcttgatccggcaaacaaaccaccgctggtagcggtggtttttttgtttgcaagcagcagattacgcgcagaaaaaaaggatctcaagaagatcctttgatcttttctacggggtctgacgctcagtggaacgaaaactcacgttaagggattttggtcatgagattatcaaaaaggatcttcacctagatccttttaaattaaaaatgaagttttaaatcaatctaaagtatatatgagtaaacttggtctgacagttaccaatgcttaatcagtgaggcacctatctcagcgatctgtctatttcgttcatccatagttgcctgactccccgtcgtgtagataactacgatacgggagggcttaccatctggccccagtgctgcaatgataccgcgagacccacgctcaccggctccagatttatcagcaataaaccagccagccggaagggccgagcgcagaagtggtcctgcaactttatccgcctccatccagtctattaattgttgccgggaagctagagtaagtagttcgccagttaatagtttgcgcaacgttgttgccattgctacaggcatcgtggtgtcacgctcgtcgtttggtatggcttcattcagctccggttcccaacgatcaaggcgagttacatgatcccccatgttgtgcaaaaaagcggttagctccttcggtcctccgatcgttgtcagaagtaagttggccgcagtgttatcactcatggttatggcagcactgcataattctcttactgtcatgccatccgtaagatgcttttctgtgactggtgagtactcaaccaagtcattctgagaatagtgtatgcggcgaccgagttgctcttgcccggcgtcaatacgggataataccgcgccacatagcagaactttaaaagtgctcatcattggaaaacgttcttcggggcgaaaactctcaaggatcttaccgctgttgagatccagttcgatgtaacccactcgtgcacccaactgatcttcagcatcttttactttcaccagcgtttctgggtgagcaaaaacaggaaggcaaaatgccgcaaaaaagggaataagggcgacacggaaatgttgaatactcatactcttcctttttcaatattattgaagcatttatcagggttattgtctcatgagcggatacatatttgaatgtatttagaaaaataaacaaataggggttccgcgcacatttccccgaaaagtgccacctaaattgtaagcgttaatattttgttaaaattcgcgttaaatttttgttaaatcagctcattttttaaccaataggccgaaatcggcaaaatcccttataaatcaaaagaatagaccgagatagggttgagtgttgttccagtttggaacaagagtccactattaaagaacgtggactccaacgtcaaagggcgaaaaaccgtctatcagggcgatggcccactacgtgaaccatcaccctaatcaagttttttggggtcgaggtgccgtaaagcactaaatcggaaccctaaagggagcccccgatttagagcttgacggggaaagccggcgaacgtggcgagaaaggaagggaagaaagcgaaaggagcgggcgctagggcgctggcaagtgtagcggtcacgctgcgcgtaaccaccacacccgccgcgcttaatgcgccgctacagggcgcgtcccattcgccattcaggctgcgcaactgttgggaagggcgatcggtgcgggcctcttcgctattacgccagctggcgaaagggggatgtgctgcaaggcgattaagttgggtaacgccagggttttcccagtcacgacgttgtaaaacgacggccagtgagcgcgcgtaatacgactcactatagggcgaattggagctccaccgcggtggcggccgctctagagagcttggcccattgcatacgttgtatccatatcataatatgtacatttatattggctcatgtccaacattaccgccatgttgacattgattattgactagttattaatagtaatcaattacggggtcattagttcatagcccatatatggagttccgcgttacataacttacggtaaatggcccgcctggctgaccgcccaacgacccccgcccattgacgtcaataatgacgtatgttcccatagtaacgccaatagggactttccattgacgtcaatgggtggagtatttacggtaaactgcccacttggcagtacatcaagtgtatcatatgccaagtacgccccctattgacgtcaatgacggtaaatggcccgcctggcattatgcccagtacatgaccttatgggactttcctacttggcagtacatctacgtattagtcatcgctattaccatggtgatgcggttttggcagtacatcaatgggcgtggatagcggtttgactcacggggatttccaagtctccaccccattgacgtcaatgggagtttgttttggcaccaaaatcaacgggactttccaaaatgtcgtaacaactccgccccattgacgcaaatgggcggtaggcgtgtacggtgggaggtctatataagcagagctcgtttagtgaaccgtcagatcgcctggagacgccatccacgctgttttgacctccatagaagacaccgggaccgatccagcctccggtcgaccgatcctgagaacttcagggtgagtttggggacccttgattgttctttctttttcgctattgtaaaattcatgttatatggagggggcaaagttttcagggtgttgtttagaatgggaagatgtcccttgtatcaccatggaccctcatgataattttgtttctttcactttctactctgttgacaaccattgtctcctcttattttcttttcattttctgtaactttttcgttaaactttagcttgcatttgtaacgaatttttaaattcacttttgtttatttgtcagattgtaagtactttctctaatcacttttttttcaaggcaatcagggtatattatattgtacttcagcacagttttagagaacaattgttataattaaatgataaggtagaatatttctgcatataaattctggctggcgtggaaatattcttattggtagaaacaactacaccctggtcatcatcctgcctttctctttatggttacaatgatatacactgtttgagatgaggataaaatactctgagtccaaaccgggcccctctgctaaccatgttcatgccttcttctctttcctacagctcctgggcaacgtgctggttgttgtgctgtctcatcattttggcaaagaattcctcgagggccggatccgaattcctgtatttgtctgaaaac

SEQ ID NO: 286 - DNA, 3375 bp, Synthetic construct
  source 1..3375: mol_type = other DNA
ataaaacctgcaggcatgcaagcgatcgcggggccgcccccttcaccgagggcctatttcccatgattccttcatatttgcatatacgatacaaggctgttagagagataattggaattaatttgactgtaaacacaaagatattagtacaaaatacgtgacgtagaaagtaataatttcttgggtagtttgcagttttaaaattatgttttaaaatggactatcatatgcttaccgtaacttgaaagtatttcgatttcttggctttatatatcttgtggaaaggacgaaacaccgctcacgctggatagcctccgtttaagagctatgctggaaacagcatagcaagtttaaataaggctagtccgttatcaacttgaaaaagtggcaccgagtcggtgctttttttgatccaagggtgggcgcgccaaggcccgcggggccactagttctagagcggccccaattcgccctatagtgagtcgtattacgcgcgctcactggccgtcgttttacaacgtcgtgactgggaaaaccctggcgttacccaacttaatcgccttgcagcacatccccctttcgccagctggcgtaatagcgaagaggcccgcaccgatcgcccttcccaacagttgcgcagcctgaatggcgaatgggacgcgccctgtagcggcgcattaagcgcggcgggtgtggtggttacgcgcagcgtgaccgctacacttgccagcgccctagcgcccgctcctttcgctttcttcccttcctttctcgccacgttcgccggctttccccgtcaagctctaaatcgggggctccctttagggttccgatttagtgctttacggcacctcgaccccaaaaaacttgattagggtgatggttcacgtagtgggccatcgccctgatagacggtttttcgccctttgacgttggagtccacgttctttaatagtggactcttgttccaaactggaacaacactcaaccctatctcggtctattcttttgatttataagggattttgccgatttcggcctattggttaaaaaatgagctgatttaacaaaaatttaacgcgaattttaacaaaatattaacgcttacaatttaggtggcacttttcggggaaatgtgcgcggaacccctatttgtttatttttctaaatacattcaaatatgtatccgctcatgagacaataaccctgataaatgcttcaataatattgaaaaaggaagagtatgagtattcaacatttccgtgtcgcccttattcccttttttgcggcattttgccttcctgtttttgctcacccagaaacgctggtgaaagtaaaagatgctgaagatcagttgggtgcacgagtgggttacatcgaactggatctcaacagcggtaagatccttgagagttttcgccccgaagaacgttttccaatgatgagcacttttaaagttctgctatgtggcgcggtattatcccgtattgacgccgggcaagagcaactcggtcgccgcatacactattctcagaatgacttggttgagtactcaccagtcacagaaaagcatcttacggatggcatgacagtaagagaattatgcagtgctgccataaccatgagtgataacactgcggccaacttacttctgacaacgatcggaggaccgaaggagctaaccgcttttttgcacaacatgggggatcatgtaactcgccttgatcgttgggaaccggagctgaatgaagccataccaaacgacgagcgtgacaccacgatgcctgtagcaatggcaacaacgttgcgcaaactattaactggcgaactacttactctagcttcccggcaacaattaatagactggatggaggcggataaagttgcaggaccacttctgcgctcggcccttccggctggctggtttattgctgataaatctggagccggtgagcgtgggtctcgcggtatcattgcagcactggggccagatggtaagccctcccgtatcgtagttatctacacgacggggagtcaggcaactatggatgaacgaaatagacagatcgctgagataggtgcctcactgattaagcattggtaactgtcagaccaagtttactcatatatactttagattgatttaaaacttcatttttaatttaaaaggatctaggtgaagatcctttttgataatctcatgaccaaaatcccttaacgtgagttttcgttccactgagcgtcagaccccgtagaaaagatcaaaggatcttcttgagatcctttttttctgcgcgtaatctgctgcttgcaaacaaaaaaaccaccgctaccagcggtggtttgtttgccggatcaagagctaccaactctttttccgaaggtaactggcttcagcagagcgcagataccaaatactgtccttctagtgtagccgtagttaggccaccacttcaagaactctgtagcaccgcctacatacctcgctctgctaatcctgttaccagtggctgctgccagtggcgataagtcgtgtcttaccgggttggactcaagacgatagttaccggataaggcgcagcggtcgggctgaacggggggttcgtgcacacagcccagcttggagcgaacgacctacaccgaactgagatacctacagcgtgagctatgagaaagcgccacgcttcccgaagggagaaaggcggacaggtatccggtaagcggcagggtcggaacaggagagcgcacgagggagcttccagggggaaacgcctggtatctttatagtcctgtcgggtttcgccacctctgacttgagcgtcgatttttgtgatgctcgtcaggggggcggagcctatggaaaaacgccagcaacgcggcctttttacggttcctggccttttgctggccttttgctcacatgttctttcctgcgttatcccctgattctgtggataaccgtattaccgcctttgagtgagctgataccgctcgccgcagccgaacgaccgagcgcagcgagtcagtgagcgaggaagcggaagagcgcccaatacgcaaaccgcctctccccgcgcgttggccgattcattaatgcagctggcacgacaggtttcccgactggaaagcgggcagtgagcgcaacgcaattaatgtgagttagctcactcattaggcaccccaggctttacactttatgcttccggctcgtatgttgtgtggaattgtgagcggataacaatttcacacaggaaacagctatgaccatgattacgccaagcgcgcaattaaccctcactaaagggaacaaaagctggaaacatgcatgaagttcctattccgaagttcctattctctagaaagtataggaacttc

SEQ ID NO: 287 - DNA, 10783 bp, Synthetic construct
  source 1..10783: mol_type = other DNA
atgggccagactgttaccactcccttaagtttgaccttaggtcactggaaagatgtcgagcggatcgctcacaaccagtcggtagatgtcaagaagagacgttgggttaccttctgctctgcagaatggccaacctttaacgtcggatggccgcgagacggcacctttaaccgagacctcatcacccaggttaagatcaaggtcttttcacctggcccgcatggacacccagaccaggtcccctacatcgtgacctgggaagccttggcttttgacccccctccctgggtcaagccctttgtacaccctaagcctccgcctcctcttcctccatccgccccgtctctcccccttgaacctcctcgttcgaccccgcctcgatcctccctttatccagccctcactccttctctaggcgccaaacctaaacctcaagttctttctgacagtggggggccgctcatcgacctacttacagaagaccccccgccttatagggacccaagaccacccccttccgacagggacggaaatggtggagaagcgacccctgcgggagaggcaccggacccctccccaatggcatctcgcctacgtgggagacgggagccccctgtggccgactccactacctcgcaggcattccccctccgcgcaggaggaaacggacagcttcaatactggccgttctcctcttctgacctttacaactggaaaaataataacccttctttttctgaagatccaggtaaactgacagctctgatcgagtctgtcctcatcacccatcagcccacctgggacgactgtcagcagctgttggggactctgctgaccggagaagaaaaacaacgggtgctcttagaggctagaaaggcggtgcggggcgatgatgggcgccccactcaactgcccaatgaagtcgatgccgcttttcccctcgagcgcccagactgggattacaccacccaggcaggtaggaaccacctagtccactatcgccagttgctcctagcgggtctccaaaacgcgggcagaagccccaccaatttggccaaggtaaaaggaataacacaagggcccaatgagtctccctcggccttcctagagagacttaaggaagcctatcgcaggtacactccttatgaccctgaggacccagggcaagaaactaatgtgtctatgtctttcatttggcagtctgccccagacattgggagaaagttagagaggttagaagatttaaaaaacaagacgcttggagatttggttagagaggcagaaaagatctttaataaacgagaaaccccggaagaaagagaggaacgtatcaggagagaaacagaggaaaaagaagaacgccgtaggacagaggatgagcagaaagagaaagaaagagatcgtaggagacatagagagatgagcaagctattggccactgtcgttagtggacagaaacaggatagacagggaggagaacgaaggaggtcccaactcgatcgcgaccagtgtgcctactgcaaagaaaaggggcactgggctaaagattgtcccaagaaaccacgaggacctcggggaccaagaccccagacctccctcctgaccctagatgactctggcggctcacttcaactgcctccacttgaaagactgacactgggatcattacaattacctcctttagaacgattaacactcggttcactacagcttccgcctcttgagagattgacattaacgtccacgctgctaatggagaactcgtctggagattacaaagacgatgacgataagaaacggacagccgacggaagcgagttcgagtcaccaaagaagaagcggaaagtcagcggggggtcagacaagaagtacagcatcggcctggacatcggcaccaactctgtgggctgggccgtgatcaccgacgagtacaaggtgcccagcaagaaattcaaggtgctgggcaacaccgaccggcacagcatcaagaagaacctgatcggagccctgctgttcgacagcggcgaaacagccgaggccacccggctgaagagaaccgccagaagaagatacaccagacggaagaaccggatctgctatctgcaagagatcttcagcaacgagatggccaaggtggacgacagcttcttccacagactggaagagtccttcctggtggaagaggataagaagcacgagcggcaccccatcttcggcaacatcgtggacgaggtggcctaccacgagaagtaccccaccatctaccacctgagaaagaaactggtggacagcaccgacaaggccgacctgcggctgatctatctggccctggcccacatgatcaagttccggggccacttcctgatcgagggcgacctgaaccccgacaacagcgacgtggacaagctgttcatccagctggtgcagacctacaaccagctgttcgaggaaaaccccatcaacgccagcggcgtggacgccaaggccatcctgtctgccagactgagcaagagcagacggctggaaaatctgatcgcccagctgcccggcgagaagaagaatggcctgttcggaaacctgattgccctgagcctgggcctgacccccaacttcaagagcaacttcgacctggccgaggatgccaaactgcagctgagcaaggacacctacgacgacgacctggacaacctgctggcccagatcggcgaccagtacgccgacctgtttctggccgccaagaacctgtccgacgccatcctgctgagcgacatcctgagagtgaacaccgagatcaccaaggcccccctgagcgcctctatgatcaagagatacgacgagcaccaccaggacctgaccctgctgaaagctctcgtgcggcagcagctgcctgagaagtacaaagagattttcttcgaccagagcaagaacggctacgccggctacattgacggcggagccagccaggaagagttctacaagttcatcaagcccatcctggaaaagatggacggcaccgaggaactgctcgtgaagctgaacagagaggacctgctgcggaagcagcggaccttcgacaacggcagcatcccccaccagatccacctgggagagctgcacgccattctgcggcggcaggaagatttttacccattcctgaaggacaaccgggaaaagatcgagaagatcctgaccttccgcatcccctactacgtgggccctctggccaggggaaacagcagattcgcctggatgaccagaaagagcgaggaaaccatcaccccctggaacttcgaggaagtggtggacaagggcgcttccgcccagagcttcatcgagcggatgaccaacttcgataagaacctgcccaacgagaaggtgctgcccaagcacagcctgctgtacgagtacttcaccgtgtataacgagctgaccaaagtgaaatacgtgaccgagggaatgagaaagcccgccttcctgagcggcgagcagaaaaaggccatcgtggacctgctgttcaagaccaaccggaaagtgaccgtgaagcagctgaaagaggactacttcaagaaaatcgagtgcttcgactccgtggaaatctccggcgtggaagatcggttcaacgcctccctgggcacataccacgatctgctgaaaattatcaaggacaaggacttcctggacaatgaggaaaacgaggacattctggaagatatcgtgctgaccctgacactgtttgaggacagagagatgatcgaggaacggctgaaaacctatgcccacctgttcgacgacaaagtgatgaagcagctgaagcggcggagatacaccggctggggcaggctgagccggaagctgatcaacggcatccgggacaagcagtccggcaagacaatcctggatttcctgaagtccgacggcttcgccaacagaaacttcatgcagctgatccacgacgacagcctgacctttaaagaggacatccagaaagcccaggtgtccggccagggcgatagcctgcacgagcacattgccaatctggccggcagccccgccattaagaagggcatcctgcagacagtgaaggtggtggacgagctcgtgaaagtgatgggccggcacaagcccgagaacatcgtgatcgaaatggccagagagaaccagaccacccagaagggacagaagaacagccgcgagagaatgaagcggatcgaagagggcatcaaagagctgggcagccagatcctgaaagaacaccccgtggaaaacacccagctgcagaacgagaagctgtacctgtactacctgcagaatgggcgggatatgtacgtggaccaggaactggacatcaaccggctgtccgactacgatgtggaccatatcgtgcctcagagctttctgaaggacgactccatcgacaacaaggtgctgaccagaagcgacaagaaccggggcaagagcgacaacgtgccctccgaagaggtcgtgaagaagatgaagaactactggcggcagctgctgaacgccaagctgattacccagagaaagttcgacaatctgaccaaggccgagagaggcggcctgagcgaactggataaggccggcttcatcaagagacagctggtggaaacccggcagatcacaaagcacgtggcacagatcctggactcccggatgaacactaagtacgacgagaatgacaagctgatccgggaagtgaaagtgatcaccctgaagtccaagctggtgtccgatttccggaaggatttccagttttacaaagtgcgcgagatcaacaactaccaccacgcccacgacgcctacctgaacgccgtcgtgggaaccgccctgatcaaaaagtaccctaagctggaaagcgagttcgtgtacggcgactacaaggtgtacgacgtgcggaagatgatcgccaagagcgagcaggaaatcggcaaggctaccgccaagtacttcttctacagcaacatcatgaactttttcaagaccgagattaccctggccaacggcgagatccggaagcggcctctgatcgagacaaacggcgaaaccggggagatcgtgtgggataagggccgggattttgccaccgtgcggaaagtgctgagcatgccccaagtgaatatcgtgaaaaagaccgaggtgcagacaggcggcttcagcaaagagtctatcctgcccaagaggaacagcgataagctgatcgccagaaagaaggactgggaccctaagaagtacggcggcttcgacagccccaccgtggcctattctgtgctggtggtggccaaagtggaaaagggcaagtccaagaaactgaagagtgtgaaagagctgctggggatcaccatcatggaaagaagcagcttcgagaagaatcccatcgactttctggaagccaagggctacaaagaagtgaaaaaggacctgatcatcaagctgcctaagtactccctgttcgagctggaaaacggccggaagagaatgctggcctctgccggcgaactgcagaagggaaacgaactggccctgccctccaaatatgtgaacttcctgtacctggccagccactatgagaagctgaagggctcccccgaggataatgagcagaaacagctgtttgtggaacagcacaagcactacctggacgagatcatcgagcagatcagcgagttctccaagagagtgatcctggccgacgctaatctggacaaagtgctgtccgcctacaacaagcaccgggataagcccatcagagagcaggccgagaatatcatccacctgtttaccctgaccaatctgggagcccctgccgccttcaagtactttgacaccaccatcgaccggaagaggtacaccagcaccaaagaggtgctggacgccaccctgatccaccagagcatcaccggcctgtacgagacacggatcgacctgtctcagctgggaggtgactctggcggctcaaaaagaaccgccgacggcagcgaattcgagcccaagaagaagaggaaagtctgagatctttttccctctgccaaaaattatggggacatcatgaagccccttgagcatctgacttctggctaataaaggaaatttattttcattgcaatagtgtgttggaattttttgtgtctctcactcggaaggacatatgggagggcaaatcatttaaaacatcagaatgagtatttggtttagagtttggcaacatatgcccatatgctggctgccatgaacaaaggttggctataaagaggtcatcagtatatgaaacagccccctgctgtccattccttattccatagaaaagccttgacttgaggttagattttttttatattttgttttgtgttatttttttctttaacatccctaaaattttccttacatgttttactagccagatttttcctcctctcctgactactcccagtcatagctgtccctcttctcttatggagatccctcgacggatcggccgcaattcgtaaccatgtcatagctgtttcctgtgtgaaattgttatccgctcacaattccacacaacatacgagccggaagcataaagtgtaaagcctggggtgcctaatgagtgagctaactcacattaattgcgttgcgctcactgcccgctttccagtcgggaaacctgtcgtgccagctgcattaatgaatcggccaacgcgcggggagaggcggtttgcgtattgggcgctcttccgcttcctcgctcactgactcgctgcgctcggtcgttcggctgcggcgagcggtatcagctcactcaaaggcggtaatacggttatccacagaatcaggggataacgcaggaaagaacatgtgagcaaaaggccagcaaaaggccaggaaccgtaaaaaggccgcgttgctggcgtttttccataggctccgcccccctgacgagcatcacaaaaatcgacgctcaagtcagaggtggcgaaacccgacaggactataaagataccaggcgtttccccctggaagctccctcgtgcgctctcctgttccgaccctgccgcttaccggatacctgtccgcctttctcccttcgggaagcgtggcgctttctcatagctcacgctgtaggtatctcagttcggtgtaggtcgttcgctccaagctgggctgtgtgcacgaaccccccgttcagcccgaccgctgcgccttatccggtaactatcgtcttgagtccaacccggtaagacacgacttatcgccactggcagcagccactggtaacaggattagcagagcgaggtatgtaggcggtgctacagagttcttgaagtggtggcctaactacggctacactagaagaacagtatttggtatctgcgctctgctgaagccagttaccttcggaaaaagagttggtagctcttgatccggcaaacaaaccaccgctggtagcggtggtttttttgtttgcaagcagcagattacgcgcagaaaaaaaggatctcaagaagatcctttgatcttttctacggggtctgacgctcagtggaacgaaaactcacgttaagggattttggtcatgagattatcaaaaaggatcttcacctagatccttttaaattaaaaatgaagttttaaatcaatctaaagtatatatgagtaaacttggtctgacagttaccaatgcttaatcagtgaggcacctatctcagcgatctgtctatttcgttcatccatagttgcctgactccccgtcgtgtagataactacgatacgggagggcttaccatctggccccagtgctgcaatgataccgcgagacccacgctcaccggctccagatttatcagcaataaaccagccagccggaagggccgagcgcagaagtggtcctgcaactttatccgcctccatccagtctattaattgttgccgggaagctagagtaagtagttcgccagttaatagtttgcgcaacgttgttgccattgctacaggcatcgtggtgtcacgctcgtcgtttggtatggcttcattcagctccggttcccaacgatcaaggcgagttacatgatcccccatgttgtgcaaaaaagcggttagctccttcggtcctccgatcgttgtcagaagtaagttggccgcagtgttatcactcatggttatggcagcactgcataattctcttactgtcatgccatccgtaagatgcttttctgtgactggtgagtactcaaccaagtcattctgagaatagtgtatgcggcgaccgagttgctcttgcccggcgtcaatacgggataataccgcgccacatagcagaactttaaaagtgctcatcattggaaaacgttcttcggggcgaaaactctcaaggatcttaccgctgttgagatccagttcgatgtaacccactcgtgcacccaactgatcttcagcatcttttactttcaccagcgtttctgggtgagcaaaaacaggaaggcaaaatgccgcaaaaaagggaataagggcgacacggaaatgttgaatactcatactcttcctttttcaatattattgaagcatttatcagggttattgtctcatgagcggatacatatttgaatgtatttagaaaaataaacaaataggggttccgcgcacatttccccgaaaagtgccacctaaattgtaagcgttaatattttgttaaaattcgcgttaaatttttgttaaatcagctcattttttaaccaataggccgaaatcggcaaaatcccttataaatcaaaagaatagaccgagatagggttgagtgttgttccagtttggaacaagagtccactattaaagaacgtggactccaacgtcaaagggcgaaaaaccgtctatcagggcgatggcccactacgtgaaccatcaccctaatcaagttttttggggtcgaggtgccgtaaagcactaaatcggaaccctaaagggagcccccgatttagagcttgacggggaaagccggcgaacgtggcgagaaaggaagggaagaaagcgaaaggagcgggcgctagggcgctggcaagtgtagcggtcacgctgcgcgtaaccaccacacccgccgcgcttaatgcgccgctacagggcgcgtcccattcgccattcaggctgcgcaactgttgggaagggcgatcggtgcgggcctcttcgctattacgccagctggcgaaagggggatgtgctgcaaggcgattaagttgggtaacgccagggttttcccagtcacgacgttgtaaaacgacggccagtgagcgcgcgtaatacgactcactatagggcgaattggagctccaccgcggtggcggccgctctagagagcttggcccattgcatacgttgtatccatatcataatatgtacatttatattggctcatgtccaacattaccgccatgttgacattgattattgactagttattaatagtaatcaattacggggtcattagttcatagcccatatatggagttccgcgttacataacttacggtaaatggcccgcctggctgaccgcccaacgacccccgcccattgacgtcaataatgacgtatgttcccatagtaacgccaatagggactttccattgacgtcaatgggtggagtatttacggtaaactgcccacttggcagtacatcaagtgtatcatatgccaagtacgccccctattgacgtcaatgacggtaaatggcccgcctggcattatgcccagtacatgaccttatgggactttcctacttggcagtacatctacgtattagtcatcgctattaccatggtgatgcggttttggcagtacatcaatgggcgtggatagcggtttgactcacggggatttccaagtctccaccccattgacgtcaatgggagtttgttttggcaccaaaatcaacgggactttccaaaatgtcgtaacaactccgccccattgacgcaaatgggcggtaggcgtgtacggtgggaggtctatataagcagagctcgtttagtgaaccgtcagatcgcctggagacgccatccacgctgttttgacctccatagaagacaccgggaccgatccagcctccggtcgaccgatcctgagaacttcagggtgagtttggggacccttgattgttctttctttttcgctattgtaaaattcatgttatatggagggggcaaagttttcagggtgttgtttagaatgggaagatgtcccttgtatcaccatggaccctcatgataattttgtttctttcactttctactctgttgacaaccattgtctcctcttattttcttttcattttctgtaactttttcgttaaactttagcttgcatttgtaacgaatttttaaattcacttttgtttatttgtcagattgtaagtactttctctaatcacttttttttcaaggcaatcagggtatattatattgtacttcagcacagttttagagaacaattgttataattaaatgataaggtagaatatttctgcatataaattctggctggcgtggaaatattcttattggtagaaacaactacaccctggtcatcatcctgcctttctctttatggttacaatgatatacactgtttgagatgaggataaaatactctgagtccaaaccgggcccctctgctaaccatgttcatgccttcttctctttcctacagctcctgggcaacgtgctggttgttgtgctgtctcatcattttggcaaagaattcctcgagggccggatccgaattcctgtatttgtctgaaaac

SEQ ID NO: 288 - DNA, 9052 bp, Synthetic construct
  source 1..9052: mol_type = other DNA
ggcgcgccggattcgacattgattattgactagttattaatagtaatcaattacggggtcattagttcatagcccatatatggagttccgcgttacataacttacggtaaatggcccgcctggctgaccgcccaacgacccccgcccattgacgtcaataatgacgtatgttcccatagtaacgccaatagggactttccattgacgtcaatgggtggagtatttacggtaaactgcccacttggcagtacatcaagtgtatcatatgccaagtacgccccctattgacgtcaatgacggtaaatggcccgcctggcattatgcccagtacatgaccttatgggactttcctacttggcagtacatctacgtattagtcatcgctattaccatggtcgaggtgagccccacgttctgcttcactctccccatctcccccccctccccacccccaattttgtatttatttattttttaattattttgtgcagcgatgggggcggggggggggggggggcgcgcgccaggcggggcggggcggggcgaggggcggggcggggcgaggcggagaggtgcggcggcagccaatcagagcggcgcgctccgaaagtttccttttatggcgaggcggcggcggcggcggccctataaaaagcgaagcgcgcggcgggcgggagtcgctgcgtcgcgccttcgccccgtgccccgctccgccgccgcctcgcgccgcccgccccggctctgactgaccgcgttactcccacaggtgagcgggcgggacggcccttctcctccgggctgtaattagcgcttggtttaatgacggctcgtttcttttctgtggctgcgtgaaagccttaaagggctccgggagggccctttgtgcgggggggagcggctcggggggtgcgtgcgtgtgtgtgtgcgtggggagcgccgcgtgcggcccgcgctgcccggcggctgtgagcgctgcgggcgcggcgcggggctttgtgcgctccgcgtgtgcgcgaggggagcgcggccgggggcggtgccccgcggtgcgggggggctgcgaggggaacaaaggctgcgtgcggggtgtgtgcgtgggggggtgagcagggggtgtgggcgcggcggtcgggctgtaacccccccctgcacccccctccccgagttgctgagcacggcccggcttcgggtgcggggctccgtgcggggcgtggcgcggggctcgccgtgccgggcggggggtggcggcaggtgggggtgccgggcggggcggggccgcctcgggccggggagggctcgggggaggggcgcggcggccccggagcgccggcggctgtcgaggcgcggcgagccgcagccattgccttttatggtaatcgtgcgagagggcgcagggacttcctttgtcccaaatctggcggagccgaaatctgggaggcgccgccgcaccccctctagcgggcgcgggcgaagcggtgcggcgccggcaggaaggaaatgggcggggagggccttcgtgcgtcgccgcgccgccgtccccttctccatctccagcctcggggctgccgcagggggacggctgccttcgggggggacggggcagggcggggttcggcttctggcgtgtgaccggcggctctagagcctctgctaaccatgttcatgccttcttctttttcctacagatccttaattaataatacgactcactataggggccgccaccatggacaagaagtacagcatcggcctggacatcggcaccaactctgtgggctgggccgtgatcaccgacgagtacaaggtgcccagcaagaaattcaaggtgctgggcaacaccgaccggcacagcatcaagaagaacctgatcggagccctgctgttcgacagcggcgaaacagccgaggccacccggctgaagagaaccgccagaagaagatacaccagacggaagaaccggatctgctatctgcaagagatcttcagcaacgagatggccaaggtggacgacagcttcttccacagactggaagagtccttcctggtggaagaggataagaagcacgagcggcaccccatcttcggcaacatcgtggacgaggtggcctaccacgagaagtaccccaccatctaccacctgagaaagaaactggtggacagcaccgacaaggccgacctgcggctgatctatctggccctggcccacatgatcaagttccggggccacttcctgatcgagggcgacctgaaccccgacaacagcgacgtggacaagctgttcatccagctggtgcagacctacaaccagctgttcgaggaaaaccccatcaacgccagcggcgtggacgccaaggccatcctgtctgccagactgagcaagagcagacggctggaaaatctgatcgcccagctgcccggcgagaagaagaatggcctgttcggcaacctgattgccctgagcctgggcctgacccccaacttcaagagcaacttcgacctggccgaggatgccaaactgcagctgagcaaggacacctacgacgacgacctggacaacctgctggcccagatcggcgaccagtacgccgacctgtttctggccgccaagaacctgtccgacgccatcctgctgagcgacatcctgagagtgaacaccgagatcaccaaggcccccctgagcgcctctatgatcaagagatacgacgagcaccaccaggacctgaccctgctgaaagctctcgtgcggcagcagctgcctgagaagtacaaagagattttcttcgaccagagcaagaacggctacgccggctacattgacggcggagccagccaggaagagttctacaagttcatcaagcccatcctggaaaagatggacggcaccgaggaactgctcgtgaagctgaacagagaggacctgctgcggaagcagcggaccttcgacaacggcagcatcccccaccagatccacctgggagagctgcacgccattctgcggcggcaggaagatttttacccattcctgaaggacaaccgggaaaagatcgagaagatcctgaccttccgcatcccctactacgtgggccctctggccaggggaaacagcagattcgcctggatgaccagaaagagcgaggaaaccatcaccccctggaacttcgaggaagtggtggacaagggcgcttccgcccagagcttcatcgagcggatgaccaacttcgataagaacctgcccaacgagaaggtgctgcccaagcacagcctgctgtacgagtacttcaccgtgtataacgagctgaccaaagtgaaatacgtgaccgagggaatgagaaagcccgccttcctgagcggcgagcagaaaaaggccatcgtggacctgctgttcaagaccaaccggaaagtgaccgtgaagcagctgaaagaggactacttcaagaaaatcgagtgcttcgactccgtggaaatctccggcgtggaagatcggttcaacgcctccctgggcacataccacgatctgctgaaaattatcaaggacaaggacttcctggacaatgaggaaaacgaggacattctggaagatatcgtgctgaccctgacactgtttgaggacagagagatgatcgaggaacggctgaaaacctatgcccacctgttcgacgacaaagtgatgaagcagctgaagcggcggagatacaccggctggggcaggctgagccggaagctgatcaacggcatccgggacaagcagtccggcaagacaatcctggatttcctgaagtccgacggcttcgccaacagaaacttcatgcagctgatccacgacgacagcctgacctttaaagaggacatccagaaagcccaggtgtccggccagggcgatagcctgcacgagcacattgccaatctggccggcagccccgccattaagaagggcatcctgcagacagtgaaggtggtggacgagctcgtgaaagtgatgggccggcacaagcccgagaacatcgtgatcgaaatggccagagagaaccagaccacccagaagggacagaagaacagccgcgagagaatgaagcggatcgaagagggcatcaaagagctgggcagccagatcctgaaagaacaccccgtggaaaacacccagctgcagaacgagaagctgtacctgtactacctgcagaatgggcgggatatgtacgtggaccaggaactggacatcaaccggctgtccgactacgatgtggaccatatcgtgcctcagagctttctgaaggacgactccatcgacaacaaggtgctgaccagaagcgacaagaaccggggcaagagcgacaacgtgccctccgaagaggtcgtgaagaagatgaagaactactggcggcagctgctgaacgccaagctgattacccagagaaagttcgacaatctgaccaaggccgagagaggcggcctgagcgaactggataaggccggcttcatcaagagacagctggtggaaacccggcagatcacaaagcacgtggcacagatcctggactcccggatgaacactaagtacgacgagaatgacaagctgatccgggaagtgaaagtgatcaccctgaagtccaagctggtgtccgatttccggaaggatttccagttttacaaagtgcgcgagatcaacaactaccaccacgcccacgacgcctacctgaacgccgtcgtgggaaccgccctgatcaaaaagtaccctaagctggaaagcgagttcgtgtacggcgactacaaggtgtacgacgtgcggaagatgatcgccaagagcgagcaggaaatcggcaaggctaccgccaagtacttcttctacagcaacatcatgaactttttcaagaccgagattaccctggccaacggcgagatccggaagcggcctctgatcgagacaaacggcgaaaccggggagatcgtgtgggataagggccgggattttgccaccgtgcggaaagtgctgagcatgccccaagtgaatatcgtgaaaaagaccgaggtgcagacaggcggcttcagcaaagagtctatcctgcccaagaggaacagcgataagctgatcgccagaaagaaggactgggaccctaagaagtacggcggcttcgacagccccaccgtggcctattctgtgctggtggtggccaaagtggaaaagggcaagtccaagaaactgaagagtgtgaaagagctgctggggatcaccatcatggaaagaagcagcttcgagaagaatcccatcgactttctggaagccaagggctacaaagaagtgaaaaaggacctgatcatcaagctgcctaagtactccctgttcgagctggaaaacggccggaagagaatgctggcctctgccggcgaactgcagaagggaaacgaactggccctgccctccaaatatgtgaacttcctgtacctggccagccactatgagaagctgaagggctcccccgaggataatgagcagaaacagctgtttgtggaacagcacaagcactacctggacgagatcatcgagcagatcagcgagttctccaagagagtgatcctggccgacgctaatctggacaaagtgctgtccgcctacaacaagcaccgggataagcccatcagagagcaggccgagaatatcatccacctgtttaccctgaccaatctgggagcccctgccgccttcaagtactttgacaccaccatcgaccggaagaggtacaccagcaccaaagaggtgctggacgccaccctgatccaccagagcatcaccggcctgtacgagacacggatcgacctgtctcagctgggaggcgacgcctatccctatgacgtgcccgattatgccagcctgggcagcggctcccccaagaaaaaacgcaaggtggaagatcctaagaaaaagcggaaagtggactgaacgcgtaaatgattgcagatccactagttctagagctcgctgatcagcctcgactgtgccttctagttgccagccatctgttgtttgcccctcccccgtgccttccttgaccctggaaggtgccactcccactgtcctttcctaataaaatgaggaaattgcatcgcattgtctgagtaggtgtcattctattctggggggtggggtggggcaggacagcaagggggaggattgggaagacaatagcaggcatgctggggatgcggtgggctctatggcttctgaggcggaaagaaccagctggggctcgagatccactagttctagcctcgaggctagagcggccgccactggccgtcgttttacaacgtcgtgactgggaaaaccctggcgttacccaacttaatcgccttgcagcacatccccctttcgccagctggcgtaatagcgaagaggcccgcaccgatcgcccttcccaacagttgcgcagcctgaatggcgaatgggacgcgccctgtagcggcgcattaagcgcggcgggtgtggtggttacgcgcagcgtgaccgctacacttgccagcgccctagcgcccgctcctttcgctttcttcccttcctttctcgccacgttcgccggctttccccgtcaagctctaaatcgggggctccctttagggttccgatttagtgctttacggcacctcgaccccaaaaaacttgattagggtgatggttcacgtagtgggccatcgccctgatagacggtttttcgccctttgacgttggagtccacgttctttaatagtggactcttgttccaaactggaacaacactcaaccctatctcggtctattcttttgatttataagggattttgccgatttcggcctattggttaaaaaatgagctgatttaacaaaaatttaacgcgaattttaacaaaatattaacgcttacaatttaggtggcacttttcggggaaatgtgcgcggaacccctatttgtttatttttctaaatacattcaaatatgtatccgctcatgagacaataaccctgataaatgcttcaataatattgaaaaaggaagagtatgagtattcaacatttccgtgtcgcccttattcccttttttgcggcattttgccttcctgtttttgctcacccagaaacgctggtgaaagtaaaagatgctgaagatcagttgggtgcacgagtgggttacatcgaactggatctcaacagcggtaagatccttgagagttttcgccccgaagaacgttttccaatgatgagcacttttaaagttctgctatgtggcgcggtattatcccgtattgacgccgggcaagagcaactcggtcgccgcatacactattctcagaatgacttggttgagtactcaccagtcacagaaaagcatcttacggatggcatgacagtaagagaattatgcagtgctgccataaccatgagtgataacactgcggccaacttacttctgacaacgatcggaggaccgaaggagctaaccgcttttttgcacaacatgggggatcatgtaactcgccttgatcgttgggaaccggagctgaatgaagccataccaaacgacgagcgtgacaccacgatgcctgtagcaatggcaacaacgttgcgcaaactattaactggcgaactacttactctagcttcccggcaacaattaatagactggatggaggcggataaagttgcaggaccacttctgcgctcggcccttccggctggctggtttattgctgataaatctggagccggtgagcgtgggtctcgcggtatcattgcagcactggggccagatggtaagccctcccgtatcgtagttatctacacgacggggagtcaggcaactatggatgaacgaaatagacagatcgctgagataggtgcctcactgattaagcattggtaactgtcagaccaagtttactcatatatactttagattgatttaaaacttcatttttaatttaaaaggatctaggtgaagatcctttttgataatctcatgaccaaaatcccttaacgtgagttttcgttccactgagcgtcagaccccgtagaaaagatcaaaggatcttcttgagatcctttttttctgcgcgtaatctgctgcttgcaaacaaaaaaaccaccgctaccagcggtggtttgtttgccggatcaagagctaccaactctttttccgaaggtaactggcttcagcagagcgcagataccaaatactgtccttctagtgtagccgtagttaggccaccacttcaagaactctgtagcaccgcctacatacctcgctctgctaatcctgttaccagtggctgctgccagtggcgataagtcgtgtcttaccgggttggactcaagacgatagttaccggataaggcgcagcggtcgggctgaacggggggttcgtgcacacagcccagcttggagcgaacgacctacaccgaactgagatacctacagcgtgagctatgagaaagcgccacgcttcccgaagggagaaaggcggacaggtatccggtaagcggcagggtcggaacaggagagcgcacgagggagcttccagggggaaacgcctggtatctttatagtcctgtcgggtttcgccacctctgacttgagcgtcgatttttgtgatgctcgtcaggggggcggagcctatggaaaaacgccagcaacgcggcctttttacggttcctggccttttgctggccttttgctcacatgttctttcctgcgttatcccctgattctgtggataaccgtattaccgcctttgagtgagctgataccgctcgccgcagccgaacgaccgagcgcagcgagtcagtgagcgaggaagcggaagagcgcccaatacgcaaaccgcctctccccgcgcgttggccgattcattaatgcagctggcacgacaggtttcccgactggaaagcgggcagtgagcgcaacgcaattaatgtgagttagctcactcattaggcaccccaggctttacactttatgcttccggctcgtatgttgtgtggaattgtgagcggataacaatttcacacaggaaacagctatgaccatga

SEQ ID NO: 289 - DNA, 13024 bp, Synthetic construct
  source 1..13024: mol_type = other DNA
atgggccagactgttaccactcccttaagtttgaccttaggtcactggaaagatgtcgagcggatcgctcacaaccagtcggtagatgtcaagaagagacgttgggttaccttctgctctgcagaatggccaacctttaacgtcggatggccgcgagacggcacctttaaccgagacctcatcacccaggttaagatcaaggtcttttcacctggcccgcatggacacccagaccaggtcccctacatcgtgacctgggaagccttggcttttgacccccctccctgggtcaagccctttgtacaccctaagcctccgcctcctcttcctccatccgccccgtctctcccccttgaacctcctcgttcgaccccgcctcgatcctccctttatccagccctcactccttctctaggcgccaaacctaaacctcaagttctttctgacagtggggggccgctcatcgacctacttacagaagaccccccgccttatagggacccaagaccacccccttccgacagggacggaaatggtggagaagcgacccctgcgggagaggcaccggacccctccccaatggcatctcgcctacgtgggagacgggagccccctgtggccgactccactacctcgcaggcattccccctccgcgcaggaggaaacggacagcttcaatactggccgttctcctcttctgacctttacaactggaaaaataataacccttctttttctgaagatccaggtaaactgacagctctgatcgagtctgtcctcatcacccatcagcccacctgggacgactgtcagcagctgttggggactctgctgaccggagaagaaaaacaacgggtgctcttagaggctagaaaggcggtgcggggcgatgatgggcgccccactcaactgcccaatgaagtcgatgccgcttttcccctcgagcgcccagactgggattacaccacccaggcaggtaggaaccacctagtccactatcgccagttgctcctagcgggtctccaaaacgcgggcagaagccccaccaatttggccaaggtaaaaggaataacacaagggcccaatgagtctccctcggccttcctagagagacttaaggaagcctatcgcaggtacactccttatgaccctgaggacccagggcaagaaactaatgtgtctatgtctttcatttggcagtctgccccagacattgggagaaagttagagaggttagaagatttaaaaaacaagacgcttggagatttggttagagaggcagaaaagatctttaataaacgagaaaccccggaagaaagagaggaacgtatcaggagagaaacagaggaaaaagaagaacgccgtaggacagaggatgagcagaaagagaaagaaagagatcgtaggagacatagagagatgagcaagctattggccactgtcgttagtggacagaaacaggatagacagggaggagaacgaaggaggtcccaactcgatcgcgaccagtgtgcctactgcaaagaaaaggggcactgggctaaagattgtcccaagaaaccacgaggacctcggggaccaagaccccagacctccctcctgaccctagatgactctggcggctcacttcaactgcctccacttgaaagactgacactgggatcattacaattacctcctttagaacgattaacactcggttcactacagcttccgcctcttgagagattgacattaacgtccacgctgctaatggagaactcgtctggagattacaaagacgatgacgataagaaacggacagccgacggaagcgagttcgagtcaccaaagaagaagcggaaagtctccggagggtcagacaagaagtacagcatcggcctggacatcggcaccaactctgtgggctgggccgtgatcaccgacgagtacaaggtgcccagcaagaaattcaaggtgctgggcaacaccgaccggcacagcatcaagaagaacctgatcggagccctgctgttcgacagcggcgaaacagccgaggccacccggctgaagagaaccgccagaagaagatacaccagacggaagaaccggatctgctatctgcaagagatcttcagcaacgagatggccaaggtggacgacagcttcttccacagactggaagagtccttcctggtggaagaggataagaagcacgagcggcaccccatcttcggcaacatcgtggacgaggtggcctaccacgagaagtaccccaccatctaccacctgagaaagaaactggtggacagcaccgacaaggccgacctgcggctgatctatctggccctggcccacatgatcaagttccggggccacttcctgatcgagggcgacctgaaccccgacaacagcgacgtggacaagctgttcatccagctggtgcagacctacaaccagctgttcgaggaaaaccccatcaacgccagcggcgtggacgccaaggccatcctgtctgccagactgagcaagagcagacggctggaaaatctgatcgcccagctgcccggcgagaagaagaatggcctgttcggcaacctgattgccctgagcctgggcctgacccccaacttcaagagcaacttcgacctggccgaggatgccaaactgcagctgagcaaggacacctacgacgacgacctggacaacctgctggcccagatcggcgaccagtacgccgacctgtttctggccgccaagaacctgtccgacgccatcctgctgagcgacatcctgagagtgaacaccgagatcaccaaggcccccctgagcgcctctatgatcaagagatacgacgagcaccaccaggacctgaccctgctgaaagctctcgtgcggcagcagctgcctgagaagtacaaagagattttcttcgaccagagcaagaacggctacgccggctacattgacggcggagccagccaggaagagttctacaagttcatcaagcccatcctggaaaagatggacggcaccgaggaactgctcgtgaagctgaacagagaggacctgctgcggaagcagcggaccttcgacaacggcagcatcccccaccagatccacctgggagagctgcacgccattctgcggcggcaggaagatttttacccattcctgaaggacaaccgggaaaagatcgagaagatcctgaccttccgcatcccctactacgtgggccctctggccaggggaaacagcagattcgcctggatgaccagaaagagcgaggaaaccatcaccccctggaacttcgaggaagtggtggacaagggcgcttccgcccagagcttcatcgagcggatgaccaacttcgataagaacctgcccaacgagaaggtgctgcccaagcacagcctgctgtacgagtacttcaccgtgtataacgagctgaccaaagtgaaatacgtgaccgagggaatgagaaagcccgccttcctgagcggcgagcagaaaaaggccatcgtggacctgctgttcaagaccaaccggaaagtgaccgtgaagcagctgaaagaggactacttcaagaaaatcgagtgcttcgactccgtggaaatctccggcgtggaagatcggttcaacgcctccctgggcacataccacgatctgctgaaaattatcaaggacaaggacttcctggacaatgaggaaaacgaggacattctggaagatatcgtgctgaccctgacactgtttgaggacagagagatgatcgaggaacggctgaaaacctatgcccacctgttcgacgacaaagtgatgaagcagctgaagcggcggagatacaccggctggggcaggctgagccggaagctgatcaacggcatccgggacaagcagtccggcaagacaatcctggatttcctgaagtccgacggcttcgccaacagaaacttcatgcagctgatccacgacgacagcctgacctttaaagaggacatccagaaagcccaggtgtccggccagggcgatagcctgcacgagcacattgccaatctggccggcagccccgccattaagaagggcatcctgcagacagtgaaggtggtggacgagctcgtgaaagtgatgggccggcacaagcccgagaacatcgtgatcgaaatggccagagagaaccagaccacccagaagggacagaagaacagccgcgagagaatgaagcggatcgaagagggcatcaaagagctgggcagccagatcctgaaagaacaccccgtggaaaacacccagctgcagaacgagaagctgtacctgtactacctgcagaatgggcgggatatgtacgtggaccaggaactggacatcaaccggctgtccgactacgatgtggaccatatcgtgcctcagagctttctgaaggacgactccatcgacaacaaggtgctgaccagaagcgacaaggcccggggcaagagcgacaacgtgccctccgaagaggtcgtgaagaagatgaagaactactggcggcagctgctgaacgccaagctgattacccagagaaagttcgacaatctgaccaaggccgagagaggcggcctgagcgaactggataaggccggcttcatcaagagacagctggtggaaacccggcagatcacaaagcacgtggcacagatcctggactcccggatgaacactaagtacgacgagaatgacaagctgatccgggaagtgaaagtgatcaccctgaagtccaagctggtgtccgatttccggaaggatttccagttttacaaagtgcgcgagatcaacaactaccaccacgcccacgacgcctacctgaacgccgtcgtgggaaccgccctgatcaaaaagtaccctaagctggaaagcgagttcgtgtacggcgactacaaggtgtacgacgtgcggaagatgatcgccaagagcgagcaggaaatcggcaaggctaccgccaagtacttcttctacagcaacatcatgaactttttcaagaccgagattaccctggccaacggcgagatccggaagcggcctctgatcgagacaaacggcgaaaccggggagatcgtgtgggataagggccgggattttgccaccgtgcggaaagtgctgagcatgccccaagtgaatatcgtgaaaaagaccgaggtgcagacaggcggcttcagcaaagagtctatcctgcccaagaggaacagcgataagctgatcgccagaaagaaggactgggaccctaagaagtacggcggcttcgacagccccaccgtggcctattctgtgctggtggtggccaaagtggaaaagggcaagtccaagaaactgaagagtgtgaaagagctgctggggatcaccatcatggaaagaagcagcttcgagaagaatcccatcgactttctggaagccaagggctacaaagaagtgaaaaaggacctgatcatcaagctgcctaagtactccctgttcgagctggaaaacggccggaagagaatgctggcctctgccggcgaactgcagaagggaaacgaactggccctgccctccaaatatgtgaacttcctgtacctggccagccactatgagaagctgaagggctcccccgaggataatgagcagaaacagctgtttgtggaacagcacaagcactacctggacgagatcatcgagcagatcagcgagttctccaagagagtgatcctggccgacgctaatctggacaaagtgctgtccgcctacaacaagcaccgggataagcccatcagagagcaggccgagaatatcatccacctgtttaccctgaccaatctgggagcccctgccgccttcaagtactttgacaccaccatcgaccggaagaggtacaccagcaccaaagaggtgctggacgccaccctgatccaccagagcatcaccggcctgtacgagacacggatcgacctgtctcagctgggaggcgacgcctatccctatgacgtgcccgattatgccagcctgggctccggatcccccaagaagaaacgcaaggtggaagatggcgagggcccagccgctaagagagtgaaactggattccggagctgctcctgccgccaagaagaagaaactcgacaccggtggacctggaagcgagcctgctacatctggctctgagacacctggcacctccgagtctgctacacctgaatctggacctggcgctagcaccctgaacatcgaggacgagtaccggctgcacgagacaagcaaagaacccgatgtgtccctgggcagcacctggcttagtgatttccctcaggcctgggccgagacaggcggaatgggacttgctgttagacaggcccctctgatcatccctctgaaggccacaagcacccctgtgtccatcaagcagtaccccatgagccaagaggcccggctgggaatcaagccccacattcagagactgctggaccagggcatcctggtgccttgtcagagcccttggaatacccctctgctgcccgtgaagaagcccggcaccaacgattacagacccgtgcaggacctgcgggaagtgaacaagagagtggaagatattcaccccaccgtgccgaatccttacaacctgctgtctggcctgcctcctagccaccagtggtacacagtgctggacctgaaggacgccttcttctgtctgcggctgcaccctacaagccagcctctgtttgcctttgagtggcgggaccctgagatgggcattagcggacagctgacctggaccagactgccccagggcttcaagaacagccccacactgttcaacgaggccctgcatagggacctcgccgacttcagaatccagcatcctgacctgatcctgctccagtacgtggacgatctgctgctggccgctacaagcgagctggattgtcagcagggaacaagagccctgctgcaaaccctgggcaacctgggctatagagcctctgccaagaaggcccagatttgccagaaacaagtgaagtatctgggctacctgctgaaagagggccagcgttggctgaccgaggccagaaaagaaaccgtgatgggccagcctacacctaagacacccagacagctgagagagttcctgggcaaagccggattctgtcggctgttcatccctggctttgccgagatggctgcccctctgtacccactgacaaagcccggaactctgttcaactggggcccagatcagcagaaggcctaccaagagatcaagcaggctctgctgacagcccctgctctgggactgcctgatctgaccaagcctttcgagctgttcgtggacgagaagcagggctatgccaaaggcgtgctgacacagaagctcggcccttggagaaggcctgtggcctacctgagcaagaaactggaccctgtggctgccggatggcctccttgtctgagaatggtggccgccattgccgtgctgaccaaggatgccggaaagctgacaatgggacagcctctggtcattctggcccctcatgccgtggaagccctcgtgaaacagcctcctgatcggtggctgagcaacgccaggatgacacactatcaggcactgctgctcgacaccgacagagtgcagtttggacctgtggtggccctgaatcctgccacacttctgcctctgcctgaggaaggcctccagcacaattgcctggacatcctggccgaggctcacggcacaagacccgatctgacagatcagccactgcctgacgccgaccacacctggtatacagatggcagctctctgctgcaagaaggacagagaaaagccggggctgccgtgaccaccgagacagaagtgatttgggccaaagctctgcccgctggcacatctgctcagagagccgaactgatcgccctgacacaggccctgaaaatggccgagggcaagaagctgaacgtctacaccgactccagatacgccttcgccaccgctcacatccacggcgaaatctatcggcggagaggatggctgaccagcgagggcaaagagattaagaacaaggacgagattctcgccctgctcaaggccctgttcctgcctaagcggctgagcatcatccactgtccaggccaccagaagggccactctgctgaagctagaggcaacagaatggccgaccaggctgccagaaaggccgccatcacagagacacccgataccagcacactgctgatcgagaacagcagccctggtacccctaagaagaagcggaaagtggactgagatctttttccctctgccaaaaattatggggacatcatgaagccccttgagcatctgacttctggctaataaaggaaatttattttcattgcaatagtgtgttggaattttttgtgtctctcactcggaaggacatatgggagggcaaatcatttaaaacatcagaatgagtatttggtttagagtttggcaacatatgcccatatgctggctgccatgaacaaaggttggctataaagaggtcatcagtatatgaaacagccccctgctgtccattccttattccatagaaaagccttgacttgaggttagattttttttatattttgttttgtgttatttttttctttaacatccctaaaattttccttacatgttttactagccagatttttcctcctctcctgactactcccagtcatagctgtccctcttctcttatggagatccctcgacggatcggccgcaattcgtaaccatgtcatagctgtttcctgtgtgaaattgttatccgctcacaattccacacaacatacgagccggaagcataaagtgtaaagcctggggtgcctaatgagtgagctaactcacattaattgcgttgcgctcactgcccgctttccagtcgggaaacctgtcgtgccagctgcattaatgaatcggccaacgcgcggggagaggcggtttgcgtattgggcgctcttccgcttcctcgctcactgactcgctgcgctcggtcgttcggctgcggcgagcggtatcagctcactcaaaggcggtaatacggttatccacagaatcaggggataacgcaggaaagaacatgtgagcaaaaggccagcaaaaggccaggaaccgtaaaaaggccgcgttgctggcgtttttccataggctccgcccccctgacgagcatcacaaaaatcgacgctcaagtcagaggtggcgaaacccgacaggactataaagataccaggcgtttccccctggaagctccctcgtgcgctctcctgttccgaccctgccgcttaccggatacctgtccgcctttctcccttcgggaagcgtggcgctttctcatagctcacgctgtaggtatctcagttcggtgtaggtcgttcgctccaagctgggctgtgtgcacgaaccccccgttcagcccgaccgctgcgccttatccggtaactatcgtcttgagtccaacccggtaagacacgacttatcgccactggcagcagccactggtaacaggattagcagagcgaggtatgtaggcggtgctacagagttcttgaagtggtggcctaactacggctacactagaagaacagtatttggtatctgcgctctgctgaagccagttaccttcggaaaaagagttggtagctcttgatccggcaaacaaaccaccgctggtagcggtggtttttttgtttgcaagcagcagattacgcgcagaaaaaaaggatctcaagaagatcctttgatcttttctacggggtctgacgctcagtggaacgaaaactcacgttaagggattttggtcatgagattatcaaaaaggatcttcacctagatccttttaaattaaaaatgaagttttaaatcaatctaaagtatatatgagtaaacttggtctgacagttaccaatgcttaatcagtgaggcacctatctcagcgatctgtctatttcgttcatccatagttgcctgactccccgtcgtgtagataactacgatacgggagggcttaccatctggccccagtgctgcaatgataccgcgagacccacgctcaccggctccagatttatcagcaataaaccagccagccggaagggccgagcgcagaagtggtcctgcaactttatccgcctccatccagtctattaattgttgccgggaagctagagtaagtagttcgccagttaatagtttgcgcaacgttgttgccattgctacaggcatcgtggtgtcacgctcgtcgtttggtatggcttcattcagctccggttcccaacgatcaaggcgagttacatgatcccccatgttgtgcaaaaaagcggttagctccttcggtcctccgatcgttgtcagaagtaagttggccgcagtgttatcactcatggttatggcagcactgcataattctcttactgtcatgccatccgtaagatgcttttctgtgactggtgagtactcaaccaagtcattctgagaatagtgtatgcggcgaccgagttgctcttgcccggcgtcaatacgggataataccgcgccacatagcagaactttaaaagtgctcatcattggaaaacgttcttcggggcgaaaactctcaaggatcttaccgctgttgagatccagttcgatgtaacccactcgtgcacccaactgatcttcagcatcttttactttcaccagcgtttctgggtgagcaaaaacaggaaggcaaaatgccgcaaaaaagggaataagggcgacacggaaatgttgaatactcatactcttcctttttcaatattattgaagcatttatcagggttattgtctcatgagcggatacatatttgaatgtatttagaaaaataaacaaataggggttccgcgcacatttccccgaaaagtgccacctaaattgtaagcgttaatattttgttaaaattcgcgttaaatttttgttaaatcagctcattttttaaccaataggccgaaatcggcaaaatcccttataaatcaaaagaatagaccgagatagggttgagtgttgttccagtttggaacaagagtccactattaaagaacgtggactccaacgtcaaagggcgaaaaaccgtctatcagggcgatggcccactacgtgaaccatcaccctaatcaagttttttggggtcgaggtgccgtaaagcactaaatcggaaccctaaagggagcccccgatttagagcttgacggggaaagccggcgaacgtggcgagaaaggaagggaagaaagcgaaaggagcgggcgctagggcgctggcaagtgtagcggtcacgctgcgcgtaaccaccacacccgccgcgcttaatgcgccgctacagggcgcgtcccattcgccattcaggctgcgcaactgttgggaagggcgatcggtgcgggcctcttcgctattacgccagctggcgaaagggggatgtgctgcaaggcgattaagttgggtaacgccagggttttcccagtcacgacgttgtaaaacgacggccagtgagcgcgcgtaatacgactcactatagggcgaattggagctccaccgcggtggcggccgctctagagagcttggcccattgcatacgttgtatccatatcataatatgtacatttatattggctcatgtccaacattaccgccatgttgacattgattattgactagttattaatagtaatcaattacggggtcattagttcatagcccatatatggagttccgcgttacataacttacggtaaatggcccgcctggctgaccgcccaacgacccccgcccattgacgtcaataatgacgtatgttcccatagtaacgccaatagggactttccattgacgtcaatgggtggagtatttacggtaaactgcccacttggcagtacatcaagtgtatcatatgccaagtacgccccctattgacgtcaatgacggtaaatggcccgcctggcattatgcccagtacatgaccttatgggactttcctacttggcagtacatctacgtattagtcatcgctattaccatggtgatgcggttttggcagtacatcaatgggcgtggatagcggtttgactcacggggatttccaagtctccaccccattgacgtcaatgggagtttgttttggcaccaaaatcaacgggactttccaaaatgtcgtaacaactccgccccattgacgcaaatgggcggtaggcgtgtacggtgggaggtctatataagcagagctcgtttagtgaaccgtcagatcgcctggagacgccatccacgctgttttgacctccatagaagacaccgggaccgatccagcctccggtcgaccgatcctgagaacttcagggtgagtttggggacccttgattgttctttctttttcgctattgtaaaattcatgttatatggagggggcaaagttttcagggtgttgtttagaatgggaagatgtcccttgtatcaccatggaccctcatgataattttgtttctttcactttctactctgttgacaaccattgtctcctcttattttcttttcattttctgtaactttttcgttaaactttagcttgcatttgtaacgaatttttaaattcacttttgtttatttgtcagattgtaagtactttctctaatcacttttttttcaaggcaatcagggtatattatattgtacttcagcacagttttagagaacaattgttataattaaatgataaggtagaatatttctgcatataaattctggctggcgtggaaatattcttattggtagaaacaactacaccctggtcatcatcctgcctttctctttatggttacaatgatatacactgtttgagatgaggataaaatactctgagtccaaaccgggcccctctgctaaccatgttcatgccttcttctctttcctacagctcctgggcaacgtgctggttgttgtgctgtctcatcattttggcaaagaattcctcgagggccggatccgaattcctgtatttgtctgaaaac

SEQ ID NO: 290 - DNA, 7281 bp, Synthetic construct
  source 1..7281: mol_type = other DNA
ggcgcgccggattcgacattgattattgactagttattaatagtaatcaattacggggtcattagttcatagcccatatatggagttccgcgttacataacttacggtaaatggcccgcctggctgaccgcccaacgacccccgcccattgacgtcaataatgacgtatgttcccatagtaacgccaatagggactttccattgacgtcaatgggtggagtatttacggtaaactgcccacttggcagtacatcaagtgtatcatatgccaagtacgccccctattgacgtcaatgacggtaaatggcccgcctggcattatgcccagtacatgaccttatgggactttcctacttggcagtacatctacgtattagtcatcgctattaccatggtcgaggtgagccccacgttctgcttcactctccccatctcccccccctccccacccccaattttgtatttatttattttttaattattttgtgcagcgatgggggcggggggggggggggggcgcgcgccaggcggggcggggcggggcgaggggcggggcggggcgaggcggagaggtgcggcggcagccaatcagagcggcgcgctccgaaagtttccttttatggcgaggcggcggcggcggcggccctataaaaagcgaagcgcgcggcgggcgggagtcgctgcgcgctgccttcgccccgtgccccgctccgccgccgcctcgcgccgcccgccccggctctgactgaccgcgttactcccacaggtgagcgggcgggacggcccttctcctccgggctgtaattagcgcttggtttaatgacggcttgtttcttttctgtggctgcgtgaaagccttgaggggctccgggagggccctttgtgcggggggagcggctcggggggtgcgtgcgtgtgtgtgtgcgtggggagcgccgcgtgcggctccgcgctgcccggcggctgtgagcgctgcgggcgcggcgcggggctttgtgcgctccgcagtgtgcgcgaggggagcgcggccgggggcggtgccccgcggtgcggggggggctgcgaggggaacaaaggctgcgtgcggggtgtgtgcgtgggggggtgagcagggggtgtgggcgcgtcggtcgggctgcaaccccccctgcacccccctccccgagttgctgagcacggcccggcttcgggtgcggggctccgtacggggcgtggcgcggggctcgccgtgccgggcggggggtggcggcaggtgggggtgccgggcggggcggggccgcctcgggccggggagggctcgggggaggggcgcggcggcccccggagcgccggcggctgtcgaggcgcggcgagccgcagccattgccttttatggtaatcgtgcgagagggcgcagggacttcctttgtcccaaatctgtgcggagccgaaatctgggaggcgccgccgcaccccctctagcgggcgcggggcgaagcggtgcggcgccggcaggaaggaaatgggcggggagggccttcgtgcgtcgccgcgccgccgtccccttctccctctccagcctcggggctgtccgcggggggacggctgccttcgggggggacggggcagggcggggttcggcttctggcgtgtgaccggcggctctagagcctctgctaaccatgttcatgccttcttctttttcctacagatccttaattaataatacgactcactataggggccgccaccatgcacggcctgcaggacgaccctgatctgcaggccctgctgaagggcagccagctgctgaaagtgaagtccagcagctggcggcgggaaagattctacaagctgcaagaggactgcaagaccatctggcaggagtctagaaaggtgatgcgctccccagaaagccaactgttcagcatcgaggacatccaggaggtgcggatgggccacagaacagagggactggaaaagttcgccagagatatccccgaggatagatgttttagcattgtgttcaaggaccagcggaacaccctggacctgatcgcccctagccctgctgatgcccagcattgggtccagggcctcagaaagatcatccaccacagcggctctatggaccagagacagaaactgcagaccggtgctagagcctctgttctgtctggcggcgaactggacagatgggagaagatcagaagcagacctggcggcaagaagaagtacaagctgaagcacatcgtgtgggccagcagagagctggaaagattcgctgtgaaccccggcctgctggaaacaagcgagggctgtagacagatcctgggccagctccagccatctctccagacaggatctgaggaactgagaagcctgtacaacaccgtggccacactgtactgcgtgcaccagagaatcgagatcaaggacaccaaagaggccctggacaagatcgaggaagaacagaacaagtctaagaagaaggcccagcaggctgccgccgatacaggccactctaatcaggtgtcccagaactaccccatcgtgcagaacatccagggccagatggtgcatcaggctatcagccccagaacactgaacgcctgggtcaaagtggtggaagagaaggctttcagccctgaagtgatccccatgttcagcgccctgtctgagggtgccacacctcaggacctgaacaccatgctgaacacagtcggcggacaccaggccgctatgcagatgctgaaagagacaatcaacgaagaggccgccgagtgggacagagtgcatcctgttcatgctggccctatcgctcccggccagatgagagaacctagaggctctgacattgccggcaccaccagcacactgcaagagcagatcggctggatgacaaacaaccctcctattcctgtgggcgagatctacaagagatggatcatcctgggactgaacaagatcgtgcggatgtacagccccaccagcatcctggacattagacagggccccaaagagcccttcagagactacgtggacagattctacaagaccctgagagccgagcaggccagccaagaagtgaagaactggatgaccgagacactgctggtgcagaacgctaaccccgactgcaagaccatcctgaaggctctgggacctgccgccacactggaagagatgatgacagcctgtcaaggcgtcggaggacctggccataaggctagagttctggccgaggccatgagccaagtgaccaacagcgccacaatcatgatgcagagaggcaacttcagaaaccagcggaagatcgtgaagtccttcaactccggcaaagagggccacaccgcccgcaattctagagcccctagaaagaaaggtggatccggcggcgtttctggatggcggctgttcaagaagatcagcggcggttccggacctgctgccaaaagagtgaaactggactccggactgcaactgcctccactggaaagactgacactgggagctgccccagccgccaagaagaaaaagctggactacaaggacgacgacgacaagggcggagctagctctaagacaatcgtgctgtctgtgggcgaagccaccagaacactgaccgagatccagagcacagccgacagacagatcttcgaggaaaaagtgggccctctcgtgggcagactgagactgacagcttccctgagacagaacggcgccaagaccgcctacagagtgaacctgaagctggaccaggccgacgtggtggattctggccttcctaaagtgcggtacacccaagtgtggtcccacgacgtgaccatcgtggccaattctaccgaggccagcagaaagagcctgtacgacctgaccaagagcctggtggccacaagccaggtggaagatctggtcgtgaacctggtgcctctcggacgtggcggatccggtggaaccgagagacaggccaacttcctgggcaagatctggcctagctacaagggcagacccggcaacttcctccagagcagaccagagcctaccgctcctcctgaggaatccttcagatccggcgtggaaaccaccacacctccacagaagcaagagcccatcgacaaagagctgtaccctctgaccagcctgagatccctgttcggcaacgaccctagctctcaatgaacgcgtaaatgattgcagatccactagttctagagctcgctgatcagcctcgactgtgccttctagttgccagccatctgttgtttgcccctcccccgtgccttccttgaccctggaaggtgccactcccactgtcctttcctaataaaatgaggaaattgcatcgcattgtctgagtaggtgtcattctattctggggggtggggtggggcaggacagcaagggggaggattgggaagacaatagcaggcatgctggggatgcggtgggctctatggcttctgaggcggaaagaaccagctggggctcgagatccactagttctagcctcgaggctagagcggccgccactggccgtcgttttacaacgtcgtgactgggaaaaccctggcgttacccaacttaatcgccttgcagcacatccccctttcgccagctggcgtaatagcgaagaggcccgcaccgatcgcccttcccaacagttgcgcagcctgaatggcgaatgggacgcgccctgtagcggcgcattaagcgcggcgggtgtggtggttacgcgcagcgtgaccgctacacttgccagcgccctagcgcccgctcctttcgctttcttcccttcctttctcgccacgttcgccggctttccccgtcaagctctaaatcgggggctccctttagggttccgatttagtgctttacggcacctcgaccccaaaaaacttgattagggtgatggttcacgtagtgggccatcgccctgatagacggtttttcgccctttgacgttggagtccacgttctttaatagtggactcttgttccaaactggaacaacactcaaccctatctcggtctattcttttgatttataagggattttgccgatttcggcctattggttaaaaaatgagctgatttaacaaaaatttaacgcgaattttaacaaaatattaacgcttacaatttaggtggcacttttcggggaaatgtgcgcggaacccctatttgtttatttttctaaatacattcaaatatgtatccgctcatgagacaataaccctgataaatgcttcaataatattgaaaaaggaagagtatgagtattcaacatttccgtgtcgcccttattcccttttttgcggcattttgccttcctgtttttgctcacccagaaacgctggtgaaagtaaaagatgctgaagatcagttgggtgcacgagtgggttacatcgaactggatctcaacagcggtaagatccttgagagttttcgccccgaagaacgttttccaatgatgagcacttttaaagttctgctatgtggcgcggtattatcccgtattgacgccgggcaagagcaactcggtcgccgcatacactattctcagaatgacttggttgagtactcaccagtcacagaaaagcatcttacggatggcatgacagtaagagaattatgcagtgctgccataaccatgagtgataacactgcggccaacttacttctgacaacgatcggaggaccgaaggagctaaccgcttttttgcacaacatgggggatcatgtaactcgccttgatcgttgggaaccggagctgaatgaagccataccaaacgacgagcgtgacaccacgatgcctgtagcaatggcaacaacgttgcgcaaactattaactggcgaactacttactctagcttcccggcaacaattaatagactggatggaggcggataaagttgcaggaccacttctgcgctcggcccttccggctggctggtttattgctgataaatctggagccggtgagcgtgggtctcgcggtatcattgcagcactggggccagatggtaagccctcccgtatcgtagttatctacacgacggggagtcaggcaactatggatgaacgaaatagacagatcgctgagataggtgcctcactgattaagcattggtaactgtcagaccaagtttactcatatatactttagattgatttaaaacttcatttttaatttaaaaggatctaggtgaagatcctttttgataatctcatgaccaaaatcccttaacgtgagttttcgttccactgagcgtcagaccccgtagaaaagatcaaaggatcttcttgagatcctttttttctgcgcgtaatctgctgcttgcaaacaaaaaaaccaccgctaccagcggtggtttgtttgccggatcaagagctaccaactctttttccgaaggtaactggcttcagcagagcgcagataccaaatactgtccttctagtgtagccgtagttaggccaccacttcaagaactctgtagcaccgcctacatacctcgctctgctaatcctgttaccagtggctgctgccagtggcgataagtcgtgtcttaccgggttggactcaagacgatagttaccggataaggcgcagcggtcgggctgaacggggggttcgtgcacacagcccagcttggagcgaacgacctacaccgaactgagatacctacagcgtgagctatgagaaagcgccacgcttcccgaagggagaaaggcggacaggtatccggtaagcggcagggtcggaacaggagagcgcacgagggagcttccagggggaaacgcctggtatctttatagtcctgtcgggtttcgccacctctgacttgagcgtcgatttttgtgatgctcgtcaggggggcggagcctatggaaaaacgccagcaacgcggcctttttacggttcctggccttttgctggccttttgctcacatgttctttcctgcgttatcccctgattctgtggataaccgtattaccgcctttgagtgagctgataccgctcgccgcagccgaacgaccgagcgcagcgagtcagtgagcgaggaagcggaagagcgcccaatacgcaaaccgcctctccccgcgcgttggccgattcattaatgcagctggcacgacaggtttcccgactggaaagcgggcagtgagcgcaacgcaattaatgtgagttagctcactcattaggcaccccaggctttacactttatgcttccggctcgtatgttgtgtggaattgtgagcggataacaatttcacacaggaaacagctatgaccatga

SEQ ID NO: 291 - DNA, 6083 bp, Synthetic construct
  source 1..6083: mol_type = other DNA
ggcgcgccggattcgacattgattattgactagttattaatagtaatcaattacggggtcattagttcatagcccatatatggagttccgcgttacataacttacggtaaatggcccgcctggctgaccgcccaacgacccccgcccattgacgtcaataatgacgtatgttcccatagtaacgccaatagggactttccattgacgtcaatgggtggagtatttacggtaaactgcccacttggcagtacatcaagtgtatcatatgccaagtacgccccctattgacgtcaatgacggtaaatggcccgcctggcattatgcccagtacatgaccttatgggactttcctacttggcagtacatctacgtattagtcatcgctattaccatggtcgaggtgagccccacgttctgcttcactctccccatctcccccccctccccacccccaattttgtatttatttattttttaattattttgtgcagcgatgggggcggggggggggggggggcgcgcgccaggcggggcggggcggggcgaggggcggggcggggcgaggcggagaggtgcggcggcagccaatcagagcggcgcgctccgaaagtttccttttatggcgaggcggcggcggcggcggccctataaaaagcgaagcgcgcggcgggcgggagtcgctgcgtcgcgccttcgccccgtgccccgctccgccgccgcctcgcgccgcccgccccggctctgactgaccgcgttactcccacaggtgagcgggcgggacggcccttctcctccgggctgtaattagcgcttggtttaatgacggctcgtttcttttctgtggctgcgtgaaagccttaaagggctccgggagggccctttgtgcgggggggagcggctcggggggtgcgtgcgtgtgtgtgtgcgtggggagcgccgcgtgcggcccgcgctgcccggcggctgtgagcgctgcgggcgcggcgcggggctttgtgcgctccgcgtgtgcgcgaggggagcgcggccgggggcggtgccccgcggtgcgggggggctgcgaggggaacaaaggctgcgtgcggggtgtgtgcgtgggggggtgagcagggggtgtgggcgcggcggtcgggctgtaacccccccctgcacccccctccccgagttgctgagcacggcccggcttcgggtgcggggctccgtgcggggcgtggcgcggggctcgccgtgccgggcggggggtggcggcaggtgggggtgccgggcggggcggggccgcctcgggccggggagggctcgggggaggggcgcggcggccccggagcgccggcggctgtcgaggcgcggcgagccgcagccattgccttttatggtaatcgtgcgagagggcgcagggacttcctttgtcccaaatctggcggagccgaaatctgggaggcgccgccgcaccccctctagcgggcgcgggcgaagcggtgcggcgccggcaggaaggaaatgggcggggagggccttcgtgcgtcgccgcgccgccgtccccttctccatctccagcctcggggctgccgcagggggacggctgccttcgggggggacggggcagggcggggttcggcttctggcgtgtgaccggcggctctagagcctctgctaaccatgttcatgccttcttctttttcctacagatccttaattaataatacgactcactataggggccgccaccatgggagctagagcatctgttctgtctggcggagcacagcaggccgctgctgatacaggccactctaatcaggtgtcccagaactacagccccacctccatcctggacatcagacagggccccaaagagcccttccgggactacgtggacagattctacaagaccctgagagccgagcaggccagccaagaagtgaagaactggatgaccgagacactgctggtgcagaacgccaatcctgactgcaagaccatcctgaaggctctgggacctgccgccacactggaagagatgatgacagcctgtcaaggcgttggcggccctggacacaaagctagagttctggccgaggccatgagccaagtgaccaactccgctaccatcatgggaggatccggcggcagaatgaagcagctggaagataaggtggaagaactgctgagcaagaactaccacctggaaaacgaggtggcccggctgaagaagctcgttggagaaagaggtggcagcggcggagtttctggatggcggctgttcaagaagatcagcggcggttccggacctgctgccaaaagagtgaaactggactccggactgcaactgcctccactggaaagactgacactgggagctgccccagccgccaagaagaaaaagctggactacaaggacgacgacgacaagggcggagctagctctaagacaatcgtgctgtctgtgggcgaagccaccagaacactgaccgagatccagagcacagccgacagacagatcttcgaggaaaaagtgggccctctcgtgggcagactgagactgacagcttccctgagacagaacggcgccaagaccgcctacagagtgaacctgaagctggaccaggccgacgtggtggattctggccttcctaaagtgcggtacacccaagtgtggtcccacgacgtgaccatcgtggccaattctaccgaggccagcagaaagagcctgtacgacctgaccaagagcctggtggccacaagccaggtggaagatctggtcgtgaacctggtgcctctcggacgtggcggcagcgctggcggactccagagcagacctgaacctacagctccaccagaggaatccttccgcagcggcgtggaaaccacaacacctccacagaagcaagagcccatcgacaaagagctgtaccctctgaccagcctgagaagcctgttcggcaacgatcccagcagccagtaaaacgcgtaaatgattgcagatccactagttctagagctcgctgatcagcctcgactgtgccttctagttgccagccatctgttgtttgcccctcccccgtgccttccttgaccctggaaggtgccactcccactgtcctttcctaataaaatgaggaaattgcatcgcattgtctgagtaggtgtcattctattctggggggtggggtggggcaggacagcaagggggaggattgggaagacaatagcaggcatgctggggatgcggtgggctctatggcttctgaggcggaaagaaccagctggggctcgagatccactagttctagcctcgaggctagagcggccgccactggccgtcgttttacaacgtcgtgactgggaaaaccctggcgttacccaacttaatcgccttgcagcacatccccctttcgccagctggcgtaatagcgaagaggcccgcaccgatcgcccttcccaacagttgcgcagcctgaatggcgaatgggacgcgccctgtagcggcgcattaagcgcggcgggtgtggtggttacgcgcagcgtgaccgctacacttgccagcgccctagcgcccgctcctttcgctttcttcccttcctttctcgccacgttcgccggctttccccgtcaagctctaaatcgggggctccctttagggttccgatttagtgctttacggcacctcgaccccaaaaaacttgattagggtgatggttcacgtagtgggccatcgccctgatagacggtttttcgccctttgacgttggagtccacgttctttaatagtggactcttgttccaaactggaacaacactcaaccctatctcggtctattcttttgatttataagggattttgccgatttcggcctattggttaaaaaatgagctgatttaacaaaaatttaacgcgaattttaacaaaatattaacgcttacaatttaggtggcacttttcggggaaatgtgcgcggaacccctatttgtttatttttctaaatacattcaaatatgtatccgctcatgagacaataaccctgataaatgcttcaataatattgaaaaaggaagagtatgagtattcaacatttccgtgtcgcccttattcccttttttgcggcattttgccttcctgtttttgctcacccagaaacgctggtgaaagtaaaagatgctgaagatcagttgggtgcacgagtgggttacatcgaactggatctcaacagcggtaagatccttgagagttttcgccccgaagaacgttttccaatgatgagcacttttaaagttctgctatgtggcgcggtattatcccgtattgacgccgggcaagagcaactcggtcgccgcatacactattctcagaatgacttggttgagtactcaccagtcacagaaaagcatcttacggatggcatgacagtaagagaattatgcagtgctgccataaccatgagtgataacactgcggccaacttacttctgacaacgatcggaggaccgaaggagctaaccgcttttttgcacaacatgggggatcatgtaactcgccttgatcgttgggaaccggagctgaatgaagccataccaaacgacgagcgtgacaccacgatgcctgtagcaatggcaacaacgttgcgcaaactattaactggcgaactacttactctagcttcccggcaacaattaatagactggatggaggcggataaagttgcaggaccacttctgcgctcggcccttccggctggctggtttattgctgataaatctggagccggtgagcgtgggtctcgcggtatcattgcagcactggggccagatggtaagccctcccgtatcgtagttatctacacgacggggagtcaggcaactatggatgaacgaaatagacagatcgctgagataggtgcctcactgattaagcattggtaactgtcagaccaagtttactcatatatactttagattgatttaaaacttcatttttaatttaaaaggatctaggtgaagatcctttttgataatctcatgaccaaaatcccttaacgtgagttttcgttccactgagcgtcagaccccgtagaaaagatcaaaggatcttcttgagatcctttttttctgcgcgtaatctgctgcttgcaaacaaaaaaaccaccgctaccagcggtggtttgtttgccggatcaagagctaccaactctttttccgaaggtaactggcttcagcagagcgcagataccaaatactgtccttctagtgtagccgtagttaggccaccacttcaagaactctgtagcaccgcctacatacctcgctctgctaatcctgttaccagtggctgctgccagtggcgataagtcgtgtcttaccgggttggactcaagacgatagttaccggataaggcgcagcggtcgggctgaacggggggttcgtgcacacagcccagcttggagcgaacgacctacaccgaactgagatacctacagcgtgagctatgagaaagcgccacgcttcccgaagggagaaaggcggacaggtatccggtaagcggcagggtcggaacaggagagcgcacgagggagcttccagggggaaacgcctggtatctttatagtcctgtcgggtttcgccacctctgacttgagcgtcgatttttgtgatgctcgtcaggggggcggagcctatggaaaaacgccagcaacgcggcctttttacggttcctggccttttgctggccttttgctcacatgttctttcctgcgttatcccctgattctgtggataaccgtattaccgcctttgagtgagctgataccgctcgccgcagccgaacgaccgagcgcagcgagtcagtgagcgaggaagcggaagagcgcccaatacgcaaaccgcctctccccgcgcgttggccgattcattaatgcagctggcacgacaggtttcccgactggaaagcgggcagtgagcgcaacgcaattaatgtgagttagctcactcattaggcaccccaggctttacactttatgcttccggctcgtatgttgtgtggaattgtgagcggataacaatttcacacaggaaacagctatgaccatga

SEQ ID NO: 292 - DNA, 5948 bp, Synthetic construct
  source 1..5948: mol_type = other DNA
ggcgcgccggattcgacattgattattgactagttattaatagtaatcaattacggggtcattagttcatagcccatatatggagttccgcgttacataacttacggtaaatggcccgcctggctgaccgcccaacgacccccgcccattgacgtcaataatgacgtatgttcccatagtaacgccaatagggactttccattgacgtcaatgggtggagtatttacggtaaactgcccacttggcagtacatcaagtgtatcatatgccaagtacgccccctattgacgtcaatgacggtaaatggcccgcctggcattatgcccagtacatgaccttatgggactttcctacttggcagtacatctacgtattagtcatcgctattaccatggtcgaggtgagccccacgttctgcttcactctccccatctcccccccctccccacccccaattttgtatttatttattttttaattattttgtgcagcgatgggggcggggggggggggggggcgcgcgccaggcggggcggggcggggcgaggggcggggcggggcgaggcggagaggtgcggcggcagccaatcagagcggcgcgctccgaaagtttccttttatggcgaggcggcggcggcggcggccctataaaaagcgaagcgcgcggcgggcgggagtcgctgcgtcgcgccttcgccccgtgccccgctccgccgccgcctcgcgccgcccgccccggctctgactgaccgcgttactcccacaggtgagcgggcgggacggcccttctcctccgggctgtaattagcgcttggtttaatgacggctcgtttcttttctgtggctgcgtgaaagccttaaagggctccgggagggccctttgtgcgggggggagcggctcggggggtgcgtgcgtgtgtgtgtgcgtggggagcgccgcgtgcggcccgcgctgcccggcggctgtgagcgctgcgggcgcggcgcggggctttgtgcgctccgcgtgtgcgcgaggggagcgcggccgggggcggtgccccgcggtgcgggggggctgcgaggggaacaaaggctgcgtgcggggtgtgtgcgtgggggggtgagcagggggtgtgggcgcggcggtcgggctgtaacccccccctgcacccccctccccgagttgctgagcacggcccggcttcgggtgcggggctccgtgcggggcgtggcgcggggctcgccgtgccgggcggggggtggcggcaggtgggggtgccgggcggggcggggccgcctcgggccggggagggctcgggggaggggcgcggcggccccggagcgccggcggctgtcgaggcgcggcgagccgcagccattgccttttatggtaatcgtgcgagagggcgcagggacttcctttgtcccaaatctggcggagccgaaatctgggaggcgccgccgcaccccctctagcgggcgcgggcgaagcggtgcggcgccggcaggaaggaaatgggcggggagggccttcgtgcgtcgccgcgccgccgtccccttctccatctccagcctcggggctgccgcagggggacggctgccttcgggggggacggggcagggcggggttcggcttctggcgtgtgaccggcggctctagagcctctgctaaccatgttcatgccttcttctttttcctacagatccttaattaataatacgactcactataggggccgccaccatgggagctagagcatctgttctgtctggcggagcacagcaggccgctgctgatacaggccactctaatcaggtgtcccagaactacagccccacctccatcctggacatcagacagggccccaaagagcccttccgggactacgtggacagattctacaagaccctgagagccgagcaggccagccaagaagtgaagaactggatgaccgagacactgctggtgcagaacgccaatcctgactgcaagaccatcctgaaggctctgggacctgccgccacactggaagagatgatgacagcctgtcaaggcgttggcggccctggacacaaagctagagttctggccgaggccatgagccaagtgaccaactccgctaccatcatgggaggatccggcggcagaatgaagcagctggaagataaggtggaagaactgctgagcaagaactaccacctggaaaacgaggtggcccggctgaagaagctcgttggagaaagaggtggcagcggcggagtttctggatggcggctgttcaagaagatcagcggcggagctagctctaagacaatcgtgctgtctgtgggcgaagccaccagaacactgaccgagatccagagcacagccgacagacagatcttcgaggaaaaagtgggccctctcgtgggcagactgagactgacagcttccctgagacagaacggcgccaagaccgcctacagagtgaacctgaagctggaccaggccgacgtggtggattctggccttcctaaagtgcggtacacccaagtgtggtcccacgacgtgaccatcgtggccaattctaccgaggccagcagaaagagcctgtacgacctgaccaagagcctggtggccacaagccaggtggaagatctggtcgtgaacctggtgcctctcggacgtggcggcagcgctggcggactccagagcagacctgaacctacagctccaccagaggaatccttccgcagcggcgtggaaaccacaacacctccacagaagcaagagcccatcgacaaagagctgtaccctctgaccagcctgagaagcctgttcggcaacgatcccagcagccagtaaaacgcgtaaatgattgcagatccactagttctagagctcgctgatcagcctcgactgtgccttctagttgccagccatctgttgtttgcccctcccccgtgccttccttgaccctggaaggtgccactcccactgtcctttcctaataaaatgaggaaattgcatcgcattgtctgagtaggtgtcattctattctggggggtggggtggggcaggacagcaagggggaggattgggaagacaatagcaggcatgctggggatgcggtgggctctatggcttctgaggcggaaagaaccagctggggctcgagatccactagttctagcctcgaggctagagcggccgccactggccgtcgttttacaacgtcgtgactgggaaaaccctggcgttacccaacttaatcgccttgcagcacatccccctttcgccagctggcgtaatagcgaagaggcccgcaccgatcgcccttcccaacagttgcgcagcctgaatggcgaatgggacgcgccctgtagcggcgcattaagcgcggcgggtgtggtggttacgcgcagcgtgaccgctacacttgccagcgccctagcgcccgctcctttcgctttcttcccttcctttctcgccacgttcgccggctttccccgtcaagctctaaatcgggggctccctttagggttccgatttagtgctttacggcacctcgaccccaaaaaacttgattagggtgatggttcacgtagtgggccatcgccctgatagacggtttttcgccctttgacgttggagtccacgttctttaatagtggactcttgttccaaactggaacaacactcaaccctatctcggtctattcttttgatttataagggattttgccgatttcggcctattggttaaaaaatgagctgatttaacaaaaatttaacgcgaattttaacaaaatattaacgcttacaatttaggtggcacttttcggggaaatgtgcgcggaacccctatttgtttatttttctaaatacattcaaatatgtatccgctcatgagacaataaccctgataaatgcttcaataatattgaaaaaggaagagtatgagtattcaacatttccgtgtcgcccttattcccttttttgcggcattttgccttcctgtttttgctcacccagaaacgctggtgaaagtaaaagatgctgaagatcagttgggtgcacgagtgggttacatcgaactggatctcaacagcggtaagatccttgagagttttcgccccgaagaacgttttccaatgatgagcacttttaaagttctgctatgtggcgcggtattatcccgtattgacgccgggcaagagcaactcggtcgccgcatacactattctcagaatgacttggttgagtactcaccagtcacagaaaagcatcttacggatggcatgacagtaagagaattatgcagtgctgccataaccatgagtgataacactgcggccaacttacttctgacaacgatcggaggaccgaaggagctaaccgcttttttgcacaacatgggggatcatgtaactcgccttgatcgttgggaaccggagctgaatgaagccataccaaacgacgagcgtgacaccacgatgcctgtagcaatggcaacaacgttgcgcaaactattaactggcgaactacttactctagcttcccggcaacaattaatagactggatggaggcggataaagttgcaggaccacttctgcgctcggcccttccggctggctggtttattgctgataaatctggagccggtgagcgtgggtctcgcggtatcattgcagcactggggccagatggtaagccctcccgtatcgtagttatctacacgacggggagtcaggcaactatggatgaacgaaatagacagatcgctgagataggtgcctcactgattaagcattggtaactgtcagaccaagtttactcatatatactttagattgatttaaaacttcatttttaatttaaaaggatctaggtgaagatcctttttgataatctcatgaccaaaatcccttaacgtgagttttcgttccactgagcgtcagaccccgtagaaaagatcaaaggatcttcttgagatcctttttttctgcgcgtaatctgctgcttgcaaacaaaaaaaccaccgctaccagcggtggtttgtttgccggatcaagagctaccaactctttttccgaaggtaactggcttcagcagagcgcagataccaaatactgtccttctagtgtagccgtagttaggccaccacttcaagaactctgtagcaccgcctacatacctcgctctgctaatcctgttaccagtggctgctgccagtggcgataagtcgtgtcttaccgggttggactcaagacgatagttaccggataaggcgcagcggtcgggctgaacggggggttcgtgcacacagcccagcttggagcgaacgacctacaccgaactgagatacctacagcgtgagctatgagaaagcgccacgcttcccgaagggagaaaggcggacaggtatccggtaagcggcagggtcggaacaggagagcgcacgagggagcttccagggggaaacgcctggtatctttatagtcctgtcgggtttcgccacctctgacttgagcgtcgatttttgtgatgctcgtcaggggggcggagcctatggaaaaacgccagcaacgcggcctttttacggttcctggccttttgctggccttttgctcacatgttctttcctgcgttatcccctgattctgtggataaccgtattaccgcctttgagtgagctgataccgctcgccgcagccgaacgaccgagcgcagcgagtcagtgagcgaggaagcggaagagcgcccaatacgcaaaccgcctctccccgcgcgttggccgattcattaatgcagctggcacgacaggtttcccgactggaaagcgggcagtgagcgcaacgcaattaatgtgagttagctcactcattaggcaccccaggctttacactttatgcttccggctcgtatgttgtgtggaattgtgagcggataacaatttcacacaggaaacagctatgaccatga

SEQ ID NO: 293 - DNA, 6487 bp, Synthetic construct
  source 1..6487: mol_type = other DNA
ggcgcgccggattcgacattgattattgactagttattaatagtaatcaattacggggtcattagttcatagcccatatatggagttccgcgttacataacttacggtaaatggcccgcctggctgaccgcccaacgacccccgcccattgacgtcaataatgacgtatgttcccatagtaacgccaatagggactttccattgacgtcaatgggtggagtatttacggtaaactgcccacttggcagtacatcaagtgtatcatatgccaagtacgccccctattgacgtcaatgacggtaaatggcccgcctggcattatgcccagtacatgaccttatgggactttcctacttggcagtacatctacgtattagtcatcgctattaccatggtcgaggtgagccccacgttctgcttcactctccccatctcccccccctccccacccccaattttgtatttatttattttttaattattttgtgcagcgatgggggcggggggggggggggggcgcgcgccaggcggggcggggcggggcgaggggcggggcggggcgaggcggagaggtgcggcggcagccaatcagagcggcgcgctccgaaagtttccttttatggcgaggcggcggcggcggcggccctataaaaagcgaagcgcgcggcgggcgggagtcgctgcgcgctgccttcgccccgtgccccgctccgccgccgcctcgcgccgcccgccccggctctgactgaccgcgttactcccacaggtgagcgggcgggacggcccttctcctccgggctgtaattagcgcttggtttaatgacggcttgtttcttttctgtggctgcgtgaaagccttgaggggctccgggagggccctttgtgcggggggagcggctcggggggtgcgtgcgtgtgtgtgtgcgtggggagcgccgcgtgcggctccgcgctgcccggcggctgtgagcgctgcgggcgcggcgcggggctttgtgcgctccgcagtgtgcgcgaggggagcgcggccgggggcggtgccccgcggtgcggggggggctgcgaggggaacaaaggctgcgtgcggggtgtgtgcgtgggggggtgagcagggggtgtgggcgcgtcggtcgggctgcaaccccccctgcacccccctccccgagttgctgagcacggcccggcttcgggtgcggggctccgtacggggcgtggcgcggggctcgccgtgccgggcggggggtggcggcaggtgggggtgccgggcggggcggggccgcctcgggccggggagggctcgggggaggggcgcggcggcccccggagcgccggcggctgtcgaggcgcggcgagccgcagccattgccttttatggtaatcgtgcgagagggcgcagggacttcctttgtcccaaatctgtgcggagccgaaatctgggaggcgccgccgcaccccctctagcgggcgcggggcgaagcggtgcggcgccggcaggaaggaaatgggcggggagggccttcgtgcgtcgccgcgccgccgtccccttctccctctccagcctcggggctgtccgcggggggacggctgccttcgggggggacggggcagggcggggttcggcttctggcgtgtgaccggcggctctagagcctctgctaaccatgttcatgccttcttctttttcctacagatccttaattaataatacgactcactataggggccgccaccatgcacggcctgcaggacgaccctgatctgcaggccctgctgaagggcagccagctgctgaaagtgaagtccagcagctggcggcgggaaagattctacaagctgcaagaggactgcaagaccatctggcaggagtctagaaaggtgatgcgctccccagaaagccaactgttcagcatcgaggacatccaggaggtgcggatgggccacagaacagagggactggaaaagttcgccagagatatccccgaggatagatgttttagcattgtgttcaaggaccagcggaacaccctggacctgatcgcccctagccctgctgatgcccagcattgggtccagggcctcagaaagatcatccaccacagcggctctatggaccagagacagaaactgcagaccggtgctagagcatctgttctgtctggcggagcacagcaggccgctgctgatacaggccactctaatcaggtgtcccagaactacagccccacctccatcctggacatcagacagggccccaaagagcccttccgggactacgtggacagattctacaagaccctgagagccgagcaggccagccaagaagtgaagaactggatgaccgagacactgctggtgcagaacgccaatcctgactgcaagaccatcctgaaggctctgggacctgccgccacactggaagagatgatgacagcctgtcaaggcgttggcggccctggacacaaagctagagttctggccgaggccatgagccaagtgaccaactccgctaccatcatgggaggatccggcggcagaatgaagcagctggaagataaggtggaagaactgctgagcaagaactaccacctggaaaacgaggtggcccggctgaagaagctcgttggagaaagaggtggcagcggcggagtttctggatggcggctgttcaagaagatcagcggcggttccggacctgctgccaaaagagtgaaactggactccggactgcaactgcctccactggaaagactgacactgggagctgccccagccgccaagaagaaaaagctggactacaaggacgacgacgacaagggcggagctagctctaagacaatcgtgctgtctgtgggcgaagccaccagaacactgaccgagatccagagcacagccgacagacagatcttcgaggaaaaagtgggccctctcgtgggcagactgagactgacagcttccctgagacagaacggcgccaagaccgcctacagagtgaacctgaagctggaccaggccgacgtggtggattctggccttcctaaagtgcggtacacccaagtgtggtcccacgacgtgaccatcgtggccaattctaccgaggccagcagaaagagcctgtacgacctgaccaagagcctggtggccacaagccaggtggaagatctggtcgtgaacctggtgcctctcggacgtggcggcagcgctggcggactccagagcagacctgaacctacagctccaccagaggaatccttccgcagcggcgtggaaaccacaacacctccacagaagcaagagcccatcgacaaagagctgtaccctctgaccagcctgagaagcctgttcggcaacgatcccagcagccagtaaaacgcgtaaatgattgcagatccactagttctagagctcgctgatcagcctcgactgtgccttctagttgccagccatctgttgtttgcccctcccccgtgccttccttgaccctggaaggtgccactcccactgtcctttcctaataaaatgaggaaattgcatcgcattgtctgagtaggtgtcattctattctggggggtggggtggggcaggacagcaagggggaggattgggaagacaatagcaggcatgctggggatgcggtgggctctatggcttctgaggcggaaagaaccagctggggctcgagatccactagttctagcctcgaggctagagcggccgccactggccgtcgttttacaacgtcgtgactgggaaaaccctggcgttacccaacttaatcgccttgcagcacatccccctttcgccagctggcgtaatagcgaagaggcccgcaccgatcgcccttcccaacagttgcgcagcctgaatggcgaatgggacgcgccctgtagcggcgcattaagcgcggcgggtgtggtggttacgcgcagcgtgaccgctacacttgccagcgccctagcgcccgctcctttcgctttcttcccttcctttctcgccacgttcgccggctttccccgtcaagctctaaatcgggggctccctttagggttccgatttagtgctttacggcacctcgaccccaaaaaacttgattagggtgatggttcacgtagtgggccatcgccctgatagacggtttttcgccctttgacgttggagtccacgttctttaatagtggactcttgttccaaactggaacaacactcaaccctatctcggtctattcttttgatttataagggattttgccgatttcggcctattggttaaaaaatgagctgatttaacaaaaatttaacgcgaattttaacaaaatattaacgcttacaatttaggtggcacttttcggggaaatgtgcgcggaacccctatttgtttatttttctaaatacattcaaatatgtatccgctcatgagacaataaccctgataaatgcttcaataatattgaaaaaggaagagtatgagtattcaacatttccgtgtcgcccttattcccttttttgcggcattttgccttcctgtttttgctcacccagaaacgctggtgaaagtaaaagatgctgaagatcagttgggtgcacgagtgggttacatcgaactggatctcaacagcggtaagatccttgagagttttcgccccgaagaacgttttccaatgatgagcacttttaaagttctgctatgtggcgcggtattatcccgtattgacgccgggcaagagcaactcggtcgccgcatacactattctcagaatgacttggttgagtactcaccagtcacagaaaagcatcttacggatggcatgacagtaagagaattatgcagtgctgccataaccatgagtgataacactgcggccaacttacttctgacaacgatcggaggaccgaaggagctaaccgcttttttgcacaacatgggggatcatgtaactcgccttgatcgttgggaaccggagctgaatgaagccataccaaacgacgagcgtgacaccacgatgcctgtagcaatggcaacaacgttgcgcaaactattaactggcgaactacttactctagcttcccggcaacaattaatagactggatggaggcggataaagttgcaggaccacttctgcgctcggcccttccggctggctggtttattgctgataaatctggagccggtgagcgtgggtctcgcggtatcattgcagcactggggccagatggtaagccctcccgtatcgtagttatctacacgacggggagtcaggcaactatggatgaacgaaatagacagatcgctgagataggtgcctcactgattaagcattggtaactgtcagaccaagtttactcatatatactttagattgatttaaaacttcatttttaatttaaaaggatctaggtgaagatcctttttgataatctcatgaccaaaatcccttaacgtgagttttcgttccactgagcgtcagaccccgtagaaaagatcaaaggatcttcttgagatcctttttttctgcgcgtaatctgctgcttgcaaacaaaaaaaccaccgctaccagcggtggtttgtttgccggatcaagagctaccaactctttttccgaaggtaactggcttcagcagagcgcagataccaaatactgtccttctagtgtagccgtagttaggccaccacttcaagaactctgtagcaccgcctacatacctcgctctgctaatcctgttaccagtggctgctgccagtggcgataagtcgtgtcttaccgggttggactcaagacgatagttaccggataaggcgcagcggtcgggctgaacggggggttcgtgcacacagcccagcttggagcgaacgacctacaccgaactgagatacctacagcgtgagctatgagaaagcgccacgcttcccgaagggagaaaggcggacaggtatccggtaagcggcagggtcggaacaggagagcgcacgagggagcttccagggggaaacgcctggtatctttatagtcctgtcgggtttcgccacctctgacttgagcgtcgatttttgtgatgctcgtcaggggggcggagcctatggaaaaacgccagcaacgcggcctttttacggttcctggccttttgctggccttttgctcacatgttctttcctgcgttatcccctgattctgtggataaccgtattaccgcctttgagtgagctgataccgctcgccgcagccgaacgaccgagcgcagcgagtcagtgagcgaggaagcggaagagcgcccaatacgcaaaccgcctctccccgcgcgttggccgattcattaatgcagctggcacgacaggtttcccgactggaaagcgggcagtgagcgcaacgcaattaatgtgagttagctcactcattaggcaccccaggctttacactttatgcttccggctcgtatgttgtgtggaattgtgagcggataacaatttcacacaggaaacagctatgaccatga

SEQ ID NO: 294 - DNA, 6059 bp, Synthetic construct
  source 1..6059: mol_type = other DNA
ggcgcgccggattcgacattgattattgactagttattaatagtaatcaattacggggtcattagttcatagcccatatatggagttccgcgttacataacttacggtaaatggcccgcctggctgaccgcccaacgacccccgcccattgacgtcaataatgacgtatgttcccatagtaacgccaatagggactttccattgacgtcaatgggtggagtatttacggtaaactgcccacttggcagtacatcaagtgtatcatatgccaagtacgccccctattgacgtcaatgacggtaaatggcccgcctggcattatgcccagtacatgaccttatgggactttcctacttggcagtacatctacgtattagtcatcgctattaccatggtcgaggtgagccccacgttctgcttcactctccccatctcccccccctccccacccccaattttgtatttatttattttttaattattttgtgcagcgatgggggcggggggggggggggggcgcgcgccaggcggggcggggcggggcgaggggcggggcggggcgaggcggagaggtgcggcggcagccaatcagagcggcgcgctccgaaagtttccttttatggcgaggcggcggcggcggcggccctataaaaagcgaagcgcgcggcgggcgggagtcgctgcgtcgcgccttcgccccgtgccccgctccgccgccgcctcgcgccgcccgccccggctctgactgaccgcgttactcccacaggtgagcgggcgggacggcccttctcctccgggctgtaattagcgcttggtttaatgacggctcgtttcttttctgtggctgcgtgaaagccttaaagggctccgggagggccctttgtgcgggggggagcggctcggggggtgcgtgcgtgtgtgtgtgcgtggggagcgccgcgtgcggcccgcgctgcccggcggctgtgagcgctgcgggcgcggcgcggggctttgtgcgctccgcgtgtgcgcgaggggagcgcggccgggggcggtgccccgcggtgcgggggggctgcgaggggaacaaaggctgcgtgcggggtgtgtgcgtgggggggtgagcagggggtgtgggcgcggcggtcgggctgtaacccccccctgcacccccctccccgagttgctgagcacggcccggcttcgggtgcggggctccgtgcggggcgtggcgcggggctcgccgtgccgggcggggggtggcggcaggtgggggtgccgggcggggcggggccgcctcgggccggggagggctcgggggaggggcgcggcggccccggagcgccggcggctgtcgaggcgcggcgagccgcagccattgccttttatggtaatcgtgcgagagggcgcagggacttcctttgtcccaaatctggcggagccgaaatctgggaggcgccgccgcaccccctctagcgggcgcgggcgaagcggtgcggcgccggcaggaaggaaatgggcggggagggccttcgtgcgtcgccgcgccgccgtccccttctccatctccagcctcggggctgccgcagggggacggctgccttcgggggggacggggcagggcggggttcggcttctggcgtgtgaccggcggctctagagcctctgctaaccatgttcatgccttcttctttttcctacagatccttaattaataatacgactcactataggggccgccaccatgggagctagagcatctgttctgtctggcggagcacagcaggccgctgctgatacaggccactctaatcaggtgtcccagaactacagccccacctccatcctggacatcagacagggccccaaagagcccttccgggactacgtggacagattctacaagaccctgagagccgagcaggccagccaagaagtgaagaactggatgaccgagacactgctggtgcagaacgccaatcctgactgcaagaccatcctgaaggctctgggacctgccgccacactggaagagatgatgacagcctgtcaaggcgttggcggccctggacacaaagctagagttctggccgaggccatgagccaagtgaccaactccgctaccatcatgggaggatccggcggcagaatgaagcagctggaagataaggtggaagaactgctgagcaagaactaccacctggaaaacgaggtggcccggctgaagaagctcgttggagaaagaggtggcagcggcggagtttctggatggcggctgttcaagaagatcagcggcggttccggacctgctgccaagaagaaaaagaacggctccggactgcaactgcctccactggaaagactgacactgggagctgccgactacaaggacgacgacgacaagggcggagctagctctaagacaatcgtgctgtctgtgggcgaagccaccagaacactgaccgagatccagagcacagccgacagacagatcttcgaggaaaaagtgggccctctcgtgggcagactgagactgacagcttccctgagacagaacggcgccaagaccgcctacagagtgaacctgaagctggaccaggccgacgtggtggattctggccttcctaaagtgcggtacacccaagtgtggtcccacgacgtgaccatcgtggccaattctaccgaggccagcagaaagagcctgtacgacctgaccaagagcctggtggccacaagccaggtggaagatctggtcgtgaacctggtgcctctcggacgtggcggcagcgctggcggactccagagcagacctgaacctacagctccaccagaggaatccttccgcagcggcgtggaaaccacaacacctccacagaagcaagagcccatcgacaaagagctgtaccctctgaccagcctgagaagcctgttcggcaacgatcccagcagccagtaaaacgcgtaaatgattgcagatccactagttctagagctcgctgatcagcctcgactgtgccttctagttgccagccatctgttgtttgcccctcccccgtgccttccttgaccctggaaggtgccactcccactgtcctttcctaataaaatgaggaaattgcatcgcattgtctgagtaggtgtcattctattctggggggtggggtggggcaggacagcaagggggaggattgggaagacaatagcaggcatgctggggatgcggtgggctctatggcttctgaggcggaaagaaccagctggggctcgagatccactagttctagcctcgaggctagagcggccgccactggccgtcgttttacaacgtcgtgactgggaaaaccctggcgttacccaacttaatcgccttgcagcacatccccctttcgccagctggcgtaatagcgaagaggcccgcaccgatcgcccttcccaacagttgcgcagcctgaatggcgaatgggacgcgccctgtagcggcgcattaagcgcggcgggtgtggtggttacgcgcagcgtgaccgctacacttgccagcgccctagcgcccgctcctttcgctttcttcccttcctttctcgccacgttcgccggctttccccgtcaagctctaaatcgggggctccctttagggttccgatttagtgctttacggcacctcgaccccaaaaaacttgattagggtgatggttcacgtagtgggccatcgccctgatagacggtttttcgccctttgacgttggagtccacgttctttaatagtggactcttgttccaaactggaacaacactcaaccctatctcggtctattcttttgatttataagggattttgccgatttcggcctattggttaaaaaatgagctgatttaacaaaaatttaacgcgaattttaacaaaatattaacgcttacaatttaggtggcacttttcggggaaatgtgcgcggaacccctatttgtttatttttctaaatacattcaaatatgtatccgctcatgagacaataaccctgataaatgcttcaataatattgaaaaaggaagagtatgagtattcaacatttccgtgtcgcccttattcccttttttgcggcattttgccttcctgtttttgctcacccagaaacgctggtgaaagtaaaagatgctgaagatcagttgggtgcacgagtgggttacatcgaactggatctcaacagcggtaagatccttgagagttttcgccccgaagaacgttttccaatgatgagcacttttaaagttctgctatgtggcgcggtattatcccgtattgacgccgggcaagagcaactcggtcgccgcatacactattctcagaatgacttggttgagtactcaccagtcacagaaaagcatcttacggatggcatgacagtaagagaattatgcagtgctgccataaccatgagtgataacactgcggccaacttacttctgacaacgatcggaggaccgaaggagctaaccgcttttttgcacaacatgggggatcatgtaactcgccttgatcgttgggaaccggagctgaatgaagccataccaaacgacgagcgtgacaccacgatgcctgtagcaatggcaacaacgttgcgcaaactattaactggcgaactacttactctagcttcccggcaacaattaatagactggatggaggcggataaagttgcaggaccacttctgcgctcggcccttccggctggctggtttattgctgataaatctggagccggtgagcgtgggtctcgcggtatcattgcagcactggggccagatggtaagccctcccgtatcgtagttatctacacgacggggagtcaggcaactatggatgaacgaaatagacagatcgctgagataggtgcctcactgattaagcattggtaactgtcagaccaagtttactcatatatactttagattgatttaaaacttcatttttaatttaaaaggatctaggtgaagatcctttttgataatctcatgaccaaaatcccttaacgtgagttttcgttccactgagcgtcagaccccgtagaaaagatcaaaggatcttcttgagatcctttttttctgcgcgtaatctgctgcttgcaaacaaaaaaaccaccgctaccagcggtggtttgtttgccggatcaagagctaccaactctttttccgaaggtaactggcttcagcagagcgcagataccaaatactgtccttctagtgtagccgtagttaggccaccacttcaagaactctgtagcaccgcctacatacctcgctctgctaatcctgttaccagtggctgctgccagtggcgataagtcgtgtcttaccgggttggactcaagacgatagttaccggataaggcgcagcggtcgggctgaacggggggttcgtgcacacagcccagcttggagcgaacgacctacaccgaactgagatacctacagcgtgagctatgagaaagcgccacgcttcccgaagggagaaaggcggacaggtatccggtaagcggcagggtcggaacaggagagcgcacgagggagcttccagggggaaacgcctggtatctttatagtcctgtcgggtttcgccacctctgacttgagcgtcgatttttgtgatgctcgtcaggggggcggagcctatggaaaaacgccagcaacgcggcctttttacggttcctggccttttgctggccttttgctcacatgttctttcctgcgttatcccctgattctgtggataaccgtattaccgcctttgagtgagctgataccgctcgccgcagccgaacgaccgagcgcagcgagtcagtgagcgaggaagcggaagagcgcccaatacgcaaaccgcctctccccgcgcgttggccgattcattaatgcagctggcacgacaggtttcccgactggaaagcgggcagtgagcgcaacgcaattaatgtgagttagctcactcattaggcaccccaggctttacactttatgcttccggctcgtatgttgtgtggaattgtgagcggataacaatttcacacaggaaacagctatgaccatga

SEQ ID NO: 295 - DNA, 6053 bp, Synthetic construct
  source 1..6053: mol_type = other DNA
ggcgcgccggattcgacattgattattgactagttattaatagtaatcaattacggggtcattagttcatagcccatatatggagttccgcgttacataacttacggtaaatggcccgcctggctgaccgcccaacgacccccgcccattgacgtcaataatgacgtatgttcccatagtaacgccaatagggactttccattgacgtcaatgggtggagtatttacggtaaactgcccacttggcagtacatcaagtgtatcatatgccaagtacgccccctattgacgtcaatgacggtaaatggcccgcctggcattatgcccagtacatgaccttatgggactttcctacttggcagtacatctacgtattagtcatcgctattaccatggtcgaggtgagccccacgttctgcttcactctccccatctcccccccctccccacccccaattttgtatttatttattttttaattattttgtgcagcgatgggggcggggggggggggggggcgcgcgccaggcggggcggggcggggcgaggggcggggcggggcgaggcggagaggtgcggcggcagccaatcagagcggcgcgctccgaaagtttccttttatggcgaggcggcggcggcggcggccctataaaaagcgaagcgcgcggcgggcgggagtcgctgcgtcgcgccttcgccccgtgccccgctccgccgccgcctcgcgccgcccgccccggctctgactgaccgcgttactcccacaggtgagcgggcgggacggcccttctcctccgggctgtaattagcgcttggtttaatgacggctcgtttcttttctgtggctgcgtgaaagccttaaagggctccgggagggccctttgtgcgggggggagcggctcggggggtgcgtgcgtgtgtgtgtgcgtggggagcgccgcgtgcggcccgcgctgcccggcggctgtgagcgctgcgggcgcggcgcggggctttgtgcgctccgcgtgtgcgcgaggggagcgcggccgggggcggtgccccgcggtgcgggggggctgcgaggggaacaaaggctgcgtgcggggtgtgtgcgtgggggggtgagcagggggtgtgggcgcggcggtcgggctgtaacccccccctgcacccccctccccgagttgctgagcacggcccggcttcgggtgcggggctccgtgcggggcgtggcgcggggctcgccgtgccgggcggggggtggcggcaggtgggggtgccgggcggggcggggccgcctcgggccggggagggctcgggggaggggcgcggcggccccggagcgccggcggctgtcgaggcgcggcgagccgcagccattgccttttatggtaatcgtgcgagagggcgcagggacttcctttgtcccaaatctggcggagccgaaatctgggaggcgccgccgcaccccctctagcgggcgcgggcgaagcggtgcggcgccggcaggaaggaaatgggcggggagggccttcgtgcgtcgccgcgccgccgtccccttctccatctccagcctcggggctgccgcagggggacggctgccttcgggggggacggggcagggcggggttcggcttctggcgtgtgaccggcggctctagagcctctgctaaccatgttcatgccttcttctttttcctacagatccttaattaataatacgactcactataggggccgccaccatgggagctagagcatctgttctgtctggcggagcacagcaggccgctgctgatacaggccactctaatcaggtgtcccagaactacagccccacctccatcctggacatcagacagggccccaaagagcccttccgggactacgtggacagattctacaagaccctgagagccgagcaggccagccaagaagtgaagaactggatgaccgagacactgctggtgcagaacgccaatcctgactgcaagaccatcctgaaggctctgggacctgccgccacactggaagagatgatgacagcctgtcaaggcgttggcggccctggacacaaagctagagttctggccgaggccatgagccaagtgaccaactccgctaccatcatgggaggatccggcggcagaatgaagcagctggaagataaggtggaagaactgctgagcaagaactaccacctggaaaacgaggtggcccggctgaagaagctcgttggagaaagaggtggcagcggcggagtttctggatggcggctgttcaagaagatcagcggcggttccggacctaagaagaaaagaaaggtgtccggactgcaactgcctccactggaaagactgacactgggagctgccgactacaaggacgacgacgacaagggcggagctagctctaagacaatcgtgctgtctgtgggcgaagccaccagaacactgaccgagatccagagcacagccgacagacagatcttcgaggaaaaagtgggccctctcgtgggcagactgagactgacagcttccctgagacagaacggcgccaagaccgcctacagagtgaacctgaagctggaccaggccgacgtggtggattctggccttcctaaagtgcggtacacccaagtgtggtcccacgacgtgaccatcgtggccaattctaccgaggccagcagaaagagcctgtacgacctgaccaagagcctggtggccacaagccaggtggaagatctggtcgtgaacctggtgcctctcggacgtggcggcagcgctggcggactccagagcagacctgaacctacagctccaccagaggaatccttccgcagcggcgtggaaaccacaacacctccacagaagcaagagcccatcgacaaagagctgtaccctctgaccagcctgagaagcctgttcggcaacgatcccagcagccagtaaaacgcgtaaatgattgcagatccactagttctagagctcgctgatcagcctcgactgtgccttctagttgccagccatctgttgtttgcccctcccccgtgccttccttgaccctggaaggtgccactcccactgtcctttcctaataaaatgaggaaattgcatcgcattgtctgagtaggtgtcattctattctggggggtggggtggggcaggacagcaagggggaggattgggaagacaatagcaggcatgctggggatgcggtgggctctatggcttctgaggcggaaagaaccagctggggctcgagatccactagttctagcctcgaggctagagcggccgccactggccgtcgttttacaacgtcgtgactgggaaaaccctggcgttacccaacttaatcgccttgcagcacatccccctttcgccagctggcgtaatagcgaagaggcccgcaccgatcgcccttcccaacagttgcgcagcctgaatggcgaatgggacgcgccctgtagcggcgcattaagcgcggcgggtgtggtggttacgcgcagcgtgaccgctacacttgccagcgccctagcgcccgctcctttcgctttcttcccttcctttctcgccacgttcgccggctttccccgtcaagctctaaatcgggggctccctttagggttccgatttagtgctttacggcacctcgaccccaaaaaacttgattagggtgatggttcacgtagtgggccatcgccctgatagacggtttttcgccctttgacgttggagtccacgttctttaatagtggactcttgttccaaactggaacaacactcaaccctatctcggtctattcttttgatttataagggattttgccgatttcggcctattggttaaaaaatgagctgatttaacaaaaatttaacgcgaattttaacaaaatattaacgcttacaatttaggtggcacttttcggggaaatgtgcgcggaacccctatttgtttatttttctaaatacattcaaatatgtatccgctcatgagacaataaccctgataaatgcttcaataatattgaaaaaggaagagtatgagtattcaacatttccgtgtcgcccttattcccttttttgcggcattttgccttcctgtttttgctcacccagaaacgctggtgaaagtaaaagatgctgaagatcagttgggtgcacgagtgggttacatcgaactggatctcaacagcggtaagatccttgagagttttcgccccgaagaacgttttccaatgatgagcacttttaaagttctgctatgtggcgcggtattatcccgtattgacgccgggcaagagcaactcggtcgccgcatacactattctcagaatgacttggttgagtactcaccagtcacagaaaagcatcttacggatggcatgacagtaagagaattatgcagtgctgccataaccatgagtgataacactgcggccaacttacttctgacaacgatcggaggaccgaaggagctaaccgcttttttgcacaacatgggggatcatgtaactcgccttgatcgttgggaaccggagctgaatgaagccataccaaacgacgagcgtgacaccacgatgcctgtagcaatggcaacaacgttgcgcaaactattaactggcgaactacttactctagcttcccggcaacaattaatagactggatggaggcggataaagttgcaggaccacttctgcgctcggcccttccggctggctggtttattgctgataaatctggagccggtgagcgtgggtctcgcggtatcattgcagcactggggccagatggtaagccctcccgtatcgtagttatctacacgacggggagtcaggcaactatggatgaacgaaatagacagatcgctgagataggtgcctcactgattaagcattggtaactgtcagaccaagtttactcatatatactttagattgatttaaaacttcatttttaatttaaaaggatctaggtgaagatcctttttgataatctcatgaccaaaatcccttaacgtgagttttcgttccactgagcgtcagaccccgtagaaaagatcaaaggatcttcttgagatcctttttttctgcgcgtaatctgctgcttgcaaacaaaaaaaccaccgctaccagcggtggtttgtttgccggatcaagagctaccaactctttttccgaaggtaactggcttcagcagagcgcagataccaaatactgtccttctagtgtagccgtagttaggccaccacttcaagaactctgtagcaccgcctacatacctcgctctgctaatcctgttaccagtggctgctgccagtggcgataagtcgtgtcttaccgggttggactcaagacgatagttaccggataaggcgcagcggtcgggctgaacggggggttcgtgcacacagcccagcttggagcgaacgacctacaccgaactgagatacctacagcgtgagctatgagaaagcgccacgcttcccgaagggagaaaggcggacaggtatccggtaagcggcagggtcggaacaggagagcgcacgagggagcttccagggggaaacgcctggtatctttatagtcctgtcgggtttcgccacctctgacttgagcgtcgatttttgtgatgctcgtcaggggggcggagcctatggaaaaacgccagcaacgcggcctttttacggttcctggccttttgctggccttttgctcacatgttctttcctgcgttatcccctgattctgtggataaccgtattaccgcctttgagtgagctgataccgctcgccgcagccgaacgaccgagcgcagcgagtcagtgagcgaggaagcggaagagcgcccaatacgcaaaccgcctctccccgcgcgttggccgattcattaatgcagctggcacgacaggtttcccgactggaaagcgggcagtgagcgcaacgcaattaatgtgagttagctcactcattaggcaccccaggctttacactttatgcttccggctcgtatgttgtgtggaattgtgagcggataacaatttcacacaggaaacagctatgaccatga

SEQ ID NO: 296 - DNA, 6518 bp, Synthetic construct
  source 1..6518: mol_type = other DNA
ggcgcgccggattcgacattgattattgactagttattaatagtaatcaattacggggtcattagttcatagcccatatatggagttccgcgttacataacttacggtaaatggcccgcctggctgaccgcccaacgacccccgcccattgacgtcaataatgacgtatgttcccatagtaacgccaatagggactttccattgacgtcaatgggtggagtatttacggtaaactgcccacttggcagtacatcaagtgtatcatatgccaagtacgccccctattgacgtcaatgacggtaaatggcccgcctggcattatgcccagtacatgaccttatgggactttcctacttggcagtacatctacgtattagtcatcgctattaccatggtcgaggtgagccccacgttctgcttcactctccccatctcccccccctccccacccccaattttgtatttatttattttttaattattttgtgcagcgatgggggcggggggggggggggggcgcgcgccaggcggggcggggcggggcgaggggcggggcggggcgaggcggagaggtgcggcggcagccaatcagagcggcgcgctccgaaagtttccttttatggcgaggcggcggcggcggcggccctataaaaagcgaagcgcgcggcgggcgggagtcgctgcgtcgcgccttcgccccgtgccccgctccgccgccgcctcgcgccgcccgccccggctctgactgaccgcgttactcccacaggtgagcgggcgggacggcccttctcctccgggctgtaattagcgcttggtttaatgacggctcgtttcttttctgtggctgcgtgaaagccttaaagggctccgggagggccctttgtgcgggggggagcggctcggggggtgcgtgcgtgtgtgtgtgcgtggggagcgccgcgtgcggcccgcgctgcccggcggctgtgagcgctgcgggcgcggcgcggggctttgtgcgctccgcgtgtgcgcgaggggagcgcggccgggggcggtgccccgcggtgcgggggggctgcgaggggaacaaaggctgcgtgcggggtgtgtgcgtgggggggtgagcagggggtgtgggcgcggcggtcgggctgtaacccccccctgcacccccctccccgagttgctgagcacggcccggcttcgggtgcggggctccgtgcggggcgtggcgcggggctcgccgtgccgggcggggggtggcggcaggtgggggtgccgggcggggcggggccgcctcgggccggggagggctcgggggaggggcgcggcggccccggagcgccggcggctgtcgaggcgcggcgagccgcagccattgccttttatggtaatcgtgcgagagggcgcagggacttcctttgtcccaaatctggcggagccgaaatctgggaggcgccgccgcaccccctctagcgggcgcgggcgaagcggtgcggcgccggcaggaaggaaatgggcggggagggccttcgtgcgtcgccgcgccgccgtccccttctccatctccagcctcggggctgccgcagggggacggctgccttcgggggggacggggcagggcggggttcggcttctggcgtgtgaccggcggctctagagcctctgctaaccatgttcatgccttcttctttttcctacagatccttaattaataatacgactcactataggggccgccaccatgggagctagagcatctgttctgtctggcggagcacagcaggccgctgctgatacaggccactctaatcaggtgtcccagaactaccccatcgtgcagaacatccagggccagatggtgcatcaggctatcagccccagaacactgaacgcctgggtcaaagtggtggaagagaaggctttcagccctgaagtgatccccatgttcagcgccctgtctgagggtgccacacctcaggacctgaacaccatgctgaacacagtcggcggacaccaggccgctatgcagatgctgaaagagacaatcaacgaagaggccgccgagtgggacagagtgcatcctgttcatgctggccctatcgctcccggccagatgagagaacctagaggctctgacattgccggcaccaccagcacactgcaagagcagatcggctggatgacaaacaaccctcctattcctgtgggcgagatctacaagagatggatcatcctgggactgaacaagatcgtgcggatgtacagccccacctccatcctggacatcagacagggccccaaagagcccttccgggactacgtggacagattctacaagaccctgagagccgagcaggccagccaagaagtgaagaactggatgaccgagacactgctggtgcagaacgccaatcctgactgcaagaccatcctgaaggctctgggacctgccgccacactggaagagatgatgacagcctgtcaaggcgttggcggccctggacacaaagctagagttctggccgaggccatgagccaagtgaccaactccgctaccatcatgggaggatccggcggcagaatgaagcagctggaagataaggtggaagaactgctgagcaagaactaccacctggaaaacgaggtggcccggctgaagaagctcgttggagaaagaggtggcagcggcggagtttctggatggcggctgttcaagaagatcagcggcggttccggacctgctgccaaaagagtgaaactggactccggactgcaactgcctccactggaaagactgacactgggagctgccccagccgccaagaagaaaaagctggactacaaggacgacgacgacaagggcggagctagctctaagacaatcgtgctgtctgtgggcgaagccaccagaacactgaccgagatccagagcacagccgacagacagatcttcgaggaaaaagtgggccctctcgtgggcagactgagactgacagcttccctgagacagaacggcgccaagaccgcctacagagtgaacctgaagctggaccaggccgacgtggtggattctggccttcctaaagtgcggtacacccaagtgtggtcccacgacgtgaccatcgtggccaattctaccgaggccagcagaaagagcctgtacgacctgaccaagagcctggtggccacaagccaggtggaagatctggtcgtgaacctggtgcctctcggacgtggcggcagcgctggcggactccagagcagacctgaacctacagctccaccagaggaatccttccgcagcggcgtggaaaccacaacacctccacagaagcaagagcccatcgacaaagagctgtaccctctgaccagcctgagaagcctgttcggcaacgatcccagcagccagtaaaacgcgtaaatgattgcagatccactagttctagagctcgctgatcagcctcgactgtgccttctagttgccagccatctgttgtttgcccctcccccgtgccttccttgaccctggaaggtgccactcccactgtcctttcctaataaaatgaggaaattgcatcgcattgtctgagtaggtgtcattctattctggggggtggggtggggcaggacagcaagggggaggattgggaagacaatagcaggcatgctggggatgcggtgggctctatggcttctgaggcggaaagaaccagctggggctcgagatccactagttctagcctcgaggctagagcggccgccactggccgtcgttttacaacgtcgtgactgggaaaaccctggcgttacccaacttaatcgccttgcagcacatccccctttcgccagctggcgtaatagcgaagaggcccgcaccgatcgcccttcccaacagttgcgcagcctgaatggcgaatgggacgcgccctgtagcggcgcattaagcgcggcgggtgtggtggttacgcgcagcgtgaccgctacacttgccagcgccctagcgcccgctcctttcgctttcttcccttcctttctcgccacgttcgccggctttccccgtcaagctctaaatcgggggctccctttagggttccgatttagtgctttacggcacctcgaccccaaaaaacttgattagggtgatggttcacgtagtgggccatcgccctgatagacggtttttcgccctttgacgttggagtccacgttctttaatagtggactcttgttccaaactggaacaacactcaaccctatctcggtctattcttttgatttataagggattttgccgatttcggcctattggttaaaaaatgagctgatttaacaaaaatttaacgcgaattttaacaaaatattaacgcttacaatttaggtggcacttttcggggaaatgtgcgcggaacccctatttgtttatttttctaaatacattcaaatatgtatccgctcatgagacaataaccctgataaatgcttcaataatattgaaaaaggaagagtatgagtattcaacatttccgtgtcgcccttattcccttttttgcggcattttgccttcctgtttttgctcacccagaaacgctggtgaaagtaaaagatgctgaagatcagttgggtgcacgagtgggttacatcgaactggatctcaacagcggtaagatccttgagagttttcgccccgaagaacgttttccaatgatgagcacttttaaagttctgctatgtggcgcggtattatcccgtattgacgccgggcaagagcaactcggtcgccgcatacactattctcagaatgacttggttgagtactcaccagtcacagaaaagcatcttacggatggcatgacagtaagagaattatgcagtgctgccataaccatgagtgataacactgcggccaacttacttctgacaacgatcggaggaccgaaggagctaaccgcttttttgcacaacatgggggatcatgtaactcgccttgatcgttgggaaccggagctgaatgaagccataccaaacgacgagcgtgacaccacgatgcctgtagcaatggcaacaacgttgcgcaaactattaactggcgaactacttactctagcttcccggcaacaattaatagactggatggaggcggataaagttgcaggaccacttctgcgctcggcccttccggctggctggtttattgctgataaatctggagccggtgagcgtgggtctcgcggtatcattgcagcactggggccagatggtaagccctcccgtatcgtagttatctacacgacggggagtcaggcaactatggatgaacgaaatagacagatcgctgagataggtgcctcactgattaagcattggtaactgtcagaccaagtttactcatatatactttagattgatttaaaacttcatttttaatttaaaaggatctaggtgaagatcctttttgataatctcatgaccaaaatcccttaacgtgagttttcgttccactgagcgtcagaccccgtagaaaagatcaaaggatcttcttgagatcctttttttctgcgcgtaatctgctgcttgcaaacaaaaaaaccaccgctaccagcggtggtttgtttgccggatcaagagctaccaactctttttccgaaggtaactggcttcagcagagcgcagataccaaatactgtccttctagtgtagccgtagttaggccaccacttcaagaactctgtagcaccgcctacatacctcgctctgctaatcctgttaccagtggctgctgccagtggcgataagtcgtgtcttaccgggttggactcaagacgatagttaccggataaggcgcagcggtcgggctgaacggggggttcgtgcacacagcccagcttggagcgaacgacctacaccgaactgagatacctacagcgtgagctatgagaaagcgccacgcttcccgaagggagaaaggcggacaggtatccggtaagcggcagggtcggaacaggagagcgcacgagggagcttccagggggaaacgcctggtatctttatagtcctgtcgggtttcgccacctctgacttgagcgtcgatttttgtgatgctcgtcaggggggcggagcctatggaaaaacgccagcaacgcggcctttttacggttcctggccttttgctggccttttgctcacatgttctttcctgcgttatcccctgattctgtggataaccgtattaccgcctttgagtgagctgataccgctcgccgcagccgaacgaccgagcgcagcgagtcagtgagcgaggaagcggaagagcgcccaatacgcaaaccgcctctccccgcgcgttggccgattcattaatgcagctggcacgacaggtttcccgactggaaagcgggcagtgagcgcaacgcaattaatgtgagttagctcactcattaggcaccccaggctttacactttatgcttccggctcgtatgttgtgtggaattgtgagcggataacaatttcacacaggaaacagctatgaccatga

SEQ ID NO: 297 - DNA, 6463 bp, Synthetic construct
  source 1..6463: mol_type = other DNA
ggcgcgccggattcgacattgattattgactagttattaatagtaatcaattacggggtcattagttcatagcccatatatggagttccgcgttacataacttacggtaaatggcccgcctggctgaccgcccaacgacccccgcccattgacgtcaataatgacgtatgttcccatagtaacgccaatagggactttccattgacgtcaatgggtggagtatttacggtaaactgcccacttggcagtacatcaagtgtatcatatgccaagtacgccccctattgacgtcaatgacggtaaatggcccgcctggcattatgcccagtacatgaccttatgggactttcctacttggcagtacatctacgtattagtcatcgctattaccatggtcgaggtgagccccacgttctgcttcactctccccatctcccccccctccccacccccaattttgtatttatttattttttaattattttgtgcagcgatgggggcggggggggggggggggcgcgcgccaggcggggcggggcggggcgaggggcggggcggggcgaggcggagaggtgcggcggcagccaatcagagcggcgcgctccgaaagtttccttttatggcgaggcggcggcggcggcggccctataaaaagcgaagcgcgcggcgggcgggagtcgctgcgcgctgccttcgccccgtgccccgctccgccgccgcctcgcgccgcccgccccggctctgactgaccgcgttactcccacaggtgagcgggcgggacggcccttctcctccgggctgtaattagcgcttggtttaatgacggcttgtttcttttctgtggctgcgtgaaagccttgaggggctccgggagggccctttgtgcggggggagcggctcggggggtgcgtgcgtgtgtgtgtgcgtggggagcgccgcgtgcggctccgcgctgcccggcggctgtgagcgctgcgggcgcggcgcggggctttgtgcgctccgcagtgtgcgcgaggggagcgcggccgggggcggtgccccgcggtgcggggggggctgcgaggggaacaaaggctgcgtgcggggtgtgtgcgtgggggggtgagcagggggtgtgggcgcgtcggtcgggctgcaaccccccctgcacccccctccccgagttgctgagcacggcccggcttcgggtgcggggctccgtacggggcgtggcgcggggctcgccgtgccgggcggggggtggcggcaggtgggggtgccgggcggggcggggccgcctcgggccggggagggctcgggggaggggcgcggcggcccccggagcgccggcggctgtcgaggcgcggcgagccgcagccattgccttttatggtaatcgtgcgagagggcgcagggacttcctttgtcccaaatctgtgcggagccgaaatctgggaggcgccgccgcaccccctctagcgggcgcggggcgaagcggtgcggcgccggcaggaaggaaatgggcggggagggccttcgtgcgtcgccgcgccgccgtccccttctccctctccagcctcggggctgtccgcggggggacggctgccttcgggggggacggggcagggcggggttcggcttctggcgtgtgaccggcggctctagagcctctgctaaccatgttcatgccttcttctttttcctacagatccttaattaataatacgactcactataggggccgccaccatgcacggcctgcaggacgaccctgatctgcaggccctgctgaagggcagccagctgctgaaagtgaagtccagcagctggcggcgggaaagattctacaagctgcaagaggactgcaagaccatctggcaggagtctagaaaggtgatgcgctccccagaaagccaactgttcagcatcgaggacatccaggaggtgcggatgggccacagaacagagggactggaaaagttcgccagagatatccccgaggatagatgttttagcattgtgttcaaggaccagcggaacaccctggacctgatcgcccctagccctgctgatgcccagcattgggtccagggcctcagaaagatcatccaccacagcggctctatggaccagagacagaaactgcagaccggtgctagagcatctgttctgtctggcggagcacagcaggccgctgctgatacaggccactctaatcaggtgtcccagaactacagccccacctccatcctggacatcagacagggccccaaagagcccttccgggactacgtggacagattctacaagaccctgagagccgagcaggccagccaagaagtgaagaactggatgaccgagacactgctggtgcagaacgccaatcctgactgcaagaccatcctgaaggctctgggacctgccgccacactggaagagatgatgacagcctgtcaaggcgttggcggccctggacacaaagctagagttctggccgaggccatgagccaagtgaccaactccgctaccatcatgggaggatccggcggcagaatgaagcagctggaagataaggtggaagaactgctgagcaagaactaccacctggaaaacgaggtggcccggctgaagaagctcgttggagaaagaggtggcagcggcggagtttctggatggcggctgttcaagaagatcagcggcggttccggacctgctgccaagaagaaaaagctggactccggactgcaactgcctccactggaaagactgacactgggagctgccgactacaaggacgacgacgacaagggcggagctagctctaagacaatcgtgctgtctgtgggcgaagccaccagaacactgaccgagatccagagcacagccgacagacagatcttcgaggaaaaagtgggccctctcgtgggcagactgagactgacagcttccctgagacagaacggcgccaagaccgcctacagagtgaacctgaagctggaccaggccgacgtggtggattctggccttcctaaagtgcggtacacccaagtgtggtcccacgacgtgaccatcgtggccaattctaccgaggccagcagaaagagcctgtacgacctgaccaagagcctggtggccacaagccaggtggaagatctggtcgtgaacctggtgcctctcggacgtggcggcagcgctggcggactccagagcagacctgaacctacagctccaccagaggaatccttccgcagcggcgtggaaaccacaacacctccacagaagcaagagcccatcgacaaagagctgtaccctctgaccagcctgagaagcctgttcggcaacgatcccagcagccagtaaaacgcgtaaatgattgcagatccactagttctagagctcgctgatcagcctcgactgtgccttctagttgccagccatctgttgtttgcccctcccccgtgccttccttgaccctggaaggtgccactcccactgtcctttcctaataaaatgaggaaattgcatcgcattgtctgagtaggtgtcattctattctggggggtggggtggggcaggacagcaagggggaggattgggaagacaatagcaggcatgctggggatgcggtgggctctatggcttctgaggcggaaagaaccagctggggctcgagatccactagttctagcctcgaggctagagcggccgccactggccgtcgttttacaacgtcgtgactgggaaaaccctggcgttacccaacttaatcgccttgcagcacatccccctttcgccagctggcgtaatagcgaagaggcccgcaccgatcgcccttcccaacagttgcgcagcctgaatggcgaatgggacgcgccctgtagcggcgcattaagcgcggcgggtgtggtggttacgcgcagcgtgaccgctacacttgccagcgccctagcgcccgctcctttcgctttcttcccttcctttctcgccacgttcgccggctttccccgtcaagctctaaatcgggggctccctttagggttccgatttagtgctttacggcacctcgaccccaaaaaacttgattagggtgatggttcacgtagtgggccatcgccctgatagacggtttttcgccctttgacgttggagtccacgttctttaatagtggactcttgttccaaactggaacaacactcaaccctatctcggtctattcttttgatttataagggattttgccgatttcggcctattggttaaaaaatgagctgatttaacaaaaatttaacgcgaattttaacaaaatattaacgcttacaatttaggtggcacttttcggggaaatgtgcgcggaacccctatttgtttatttttctaaatacattcaaatatgtatccgctcatgagacaataaccctgataaatgcttcaataatattgaaaaaggaagagtatgagtattcaacatttccgtgtcgcccttattcccttttttgcggcattttgccttcctgtttttgctcacccagaaacgctggtgaaagtaaaagatgctgaagatcagttgggtgcacgagtgggttacatcgaactggatctcaacagcggtaagatccttgagagttttcgccccgaagaacgttttccaatgatgagcacttttaaagttctgctatgtggcgcggtattatcccgtattgacgccgggcaagagcaactcggtcgccgcatacactattctcagaatgacttggttgagtactcaccagtcacagaaaagcatcttacggatggcatgacagtaagagaattatgcagtgctgccataaccatgagtgataacactgcggccaacttacttctgacaacgatcggaggaccgaaggagctaaccgcttttttgcacaacatgggggatcatgtaactcgccttgatcgttgggaaccggagctgaatgaagccataccaaacgacgagcgtgacaccacgatgcctgtagcaatggcaacaacgttgcgcaaactattaactggcgaactacttactctagcttcccggcaacaattaatagactggatggaggcggataaagttgcaggaccacttctgcgctcggcccttccggctggctggtttattgctgataaatctggagccggtgagcgtgggtctcgcggtatcattgcagcactggggccagatggtaagccctcccgtatcgtagttatctacacgacggggagtcaggcaactatggatgaacgaaatagacagatcgctgagataggtgcctcactgattaagcattggtaactgtcagaccaagtttactcatatatactttagattgatttaaaacttcatttttaatttaaaaggatctaggtgaagatcctttttgataatctcatgaccaaaatcccttaacgtgagttttcgttccactgagcgtcagaccccgtagaaaagatcaaaggatcttcttgagatcctttttttctgcgcgtaatctgctgcttgcaaacaaaaaaaccaccgctaccagcggtggtttgtttgccggatcaagagctaccaactctttttccgaaggtaactggcttcagcagagcgcagataccaaatactgtccttctagtgtagccgtagttaggccaccacttcaagaactctgtagcaccgcctacatacctcgctctgctaatcctgttaccagtggctgctgccagtggcgataagtcgtgtcttaccgggttggactcaagacgatagttaccggataaggcgcagcggtcgggctgaacggggggttcgtgcacacagcccagcttggagcgaacgacctacaccgaactgagatacctacagcgtgagctatgagaaagcgccacgcttcccgaagggagaaaggcggacaggtatccggtaagcggcagggtcggaacaggagagcgcacgagggagcttccagggggaaacgcctggtatctttatagtcctgtcgggtttcgccacctctgacttgagcgtcgatttttgtgatgctcgtcaggggggcggagcctatggaaaaacgccagcaacgcggcctttttacggttcctggccttttgctggccttttgctcacatgttctttcctgcgttatcccctgattctgtggataaccgtattaccgcctttgagtgagctgataccgctcgccgcagccgaacgaccgagcgcagcgagtcagtgagcgaggaagcggaagagcgcccaatacgcaaaccgcctctccccgcgcgttggccgattcattaatgcagctggcacgacaggtttcccgactggaaagcgggcagtgagcgcaacgcaattaatgtgagttagctcactcattaggcaccccaggctttacactttatgcttccggctcgtatgttgtgtggaattgtgagcggataacaatttcacacaggaaacagctatgaccatga

SEQ ID NO: 298 - DNA, 6463 bp, Synthetic construct
  source 1..6463: mol_type = other DNA
ggcgcgccggattcgacattgattattgactagttattaatagtaatcaattacggggtcattagttcatagcccatatatggagttccgcgttacataacttacggtaaatggcccgcctggctgaccgcccaacgacccccgcccattgacgtcaataatgacgtatgttcccatagtaacgccaatagggactttccattgacgtcaatgggtggagtatttacggtaaactgcccacttggcagtacatcaagtgtatcatatgccaagtacgccccctattgacgtcaatgacggtaaatggcccgcctggcattatgcccagtacatgaccttatgggactttcctacttggcagtacatctacgtattagtcatcgctattaccatggtcgaggtgagccccacgttctgcttcactctccccatctcccccccctccccacccccaattttgtatttatttattttttaattattttgtgcagcgatgggggcggggggggggggggggcgcgcgccaggcggggcggggcggggcgaggggcggggcggggcgaggcggagaggtgcggcggcagccaatcagagcggcgcgctccgaaagtttccttttatggcgaggcggcggcggcggcggccctataaaaagcgaagcgcgcggcgggcgggagtcgctgcgcgctgccttcgccccgtgccccgctccgccgccgcctcgcgccgcccgccccggctctgactgaccgcgttactcccacaggtgagcgggcgggacggcccttctcctccgggctgtaattagcgcttggtttaatgacggcttgtttcttttctgtggctgcgtgaaagccttgaggggctccgggagggccctttgtgcggggggagcggctcggggggtgcgtgcgtgtgtgtgtgcgtggggagcgccgcgtgcggctccgcgctgcccggcggctgtgagcgctgcgggcgcggcgcggggctttgtgcgctccgcagtgtgcgcgaggggagcgcggccgggggcggtgccccgcggtgcggggggggctgcgaggggaacaaaggctgcgtgcggggtgtgtgcgtgggggggtgagcagggggtgtgggcgcgtcggtcgggctgcaaccccccctgcacccccctccccgagttgctgagcacggcccggcttcgggtgcggggctccgtacggggcgtggcgcggggctcgccgtgccgggcggggggtggcggcaggtgggggtgccgggcggggcggggccgcctcgggccggggagggctcgggggaggggcgcggcggcccccggagcgccggcggctgtcgaggcgcggcgagccgcagccattgccttttatggtaatcgtgcgagagggcgcagggacttcctttgtcccaaatctgtgcggagccgaaatctgggaggcgccgccgcaccccctctagcgggcgcggggcgaagcggtgcggcgccggcaggaaggaaatgggcggggagggccttcgtgcgtcgccgcgccgccgtccccttctccctctccagcctcggggctgtccgcggggggacggctgccttcgggggggacggggcagggcggggttcggcttctggcgtgtgaccggcggctctagagcctctgctaaccatgttcatgccttcttctttttcctacagatccttaattaataatacgactcactataggggccgccaccatgcacggcctgcaggacgaccctgatctgcaggccctgctgaagggcagccagctgctgaaagtgaagtccagcagctggcggcgggaaagattctacaagctgcaagaggactgcaagaccatctggcaggagtctagaaaggtgatgcgctccccagaaagccaactgttcagcatcgaggacatccaggaggtgcggatgggccacagaacagagggactggaaaagttcgccagagatatccccgaggatagatgttttagcattgtgttcaaggaccagcggaacaccctggacctgatcgcccctagccctgctgatgcccagcattgggtccagggcctcagaaagatcatccaccacagcggctctatggaccagagacagaaactgcagaccggtgctagagcatctgttctgtctggcggagcacagcaggccgctgctgatacaggccactctaatcaggtgtcccagaactacagccccacctccatcctggacatcagacagggccccaaagagcccttccgggactacgtggacagattctacaagaccctgagagccgagcaggccagccaagaagtgaagaactggatgaccgagacactgctggtgcagaacgccaatcctgactgcaagaccatcctgaaggctctgggacctgccgccacactggaagagatgatgacagcctgtcaaggcgttggcggccctggacacaaagctagagttctggccgaggccatgagccaagtgaccaactccgctaccatcatgggaggatccggcggcagaatgaagcagctggaagataaggtggaagaactgctgagcaagaactaccacctggaaaacgaggtggcccggctgaagaagctcgttggagaaagaggtggcagcggcggagtttctggatggcggctgttcaagaagatcagcggcggttccggacctgctgccaaaagagtgaaactggactccggactgcaactgcctccactggaaagactgacactgggagctgccgactacaaggacgacgacgacaagggcggagctagctctaagacaatcgtgctgtctgtgggcgaagccaccagaacactgaccgagatccagagcacagccgacagacagatcttcgaggaaaaagtgggccctctcgtgggcagactgagactgacagcttccctgagacagaacggcgccaagaccgcctacagagtgaacctgaagctggaccaggccgacgtggtggattctggccttcctaaagtgcggtacacccaagtgtggtcccacgacgtgaccatcgtggccaattctaccgaggccagcagaaagagcctgtacgacctgaccaagagcctggtggccacaagccaggtggaagatctggtcgtgaacctggtgcctctcggacgtggcggcagcgctggcggactccagagcagacctgaacctacagctccaccagaggaatccttccgcagcggcgtggaaaccacaacacctccacagaagcaagagcccatcgacaaagagctgtaccctctgaccagcctgagaagcctgttcggcaacgatcccagcagccagtaaaacgcgtaaatgattgcagatccactagttctagagctcgctgatcagcctcgactgtgccttctagttgccagccatctgttgtttgcccctcccccgtgccttccttgaccctggaaggtgccactcccactgtcctttcctaataaaatgaggaaattgcatcgcattgtctgagtaggtgtcattctattctggggggtggggtggggcaggacagcaagggggaggattgggaagacaatagcaggcatgctggggatgcggtgggctctatggcttctgaggcggaaagaaccagctggggctcgagatccactagttctagcctcgaggctagagcggccgccactggccgtcgttttacaacgtcgtgactgggaaaaccctggcgttacccaacttaatcgccttgcagcacatccccctttcgccagctggcgtaatagcgaagaggcccgcaccgatcgcccttcccaacagttgcgcagcctgaatggcgaatgggacgcgccctgtagcggcgcattaagcgcggcgggtgtggtggttacgcgcagcgtgaccgctacacttgccagcgccctagcgcccgctcctttcgctttcttcccttcctttctcgccacgttcgccggctttccccgtcaagctctaaatcgggggctccctttagggttccgatttagtgctttacggcacctcgaccccaaaaaacttgattagggtgatggttcacgtagtgggccatcgccctgatagacggtttttcgccctttgacgttggagtccacgttctttaatagtggactcttgttccaaactggaacaacactcaaccctatctcggtctattcttttgatttataagggattttgccgatttcggcctattggttaaaaaatgagctgatttaacaaaaatttaacgcgaattttaacaaaatattaacgcttacaatttaggtggcacttttcggggaaatgtgcgcggaacccctatttgtttatttttctaaatacattcaaatatgtatccgctcatgagacaataaccctgataaatgcttcaataatattgaaaaaggaagagtatgagtattcaacatttccgtgtcgcccttattcccttttttgcggcattttgccttcctgtttttgctcacccagaaacgctggtgaaagtaaaagatgctgaagatcagttgggtgcacgagtgggttacatcgaactggatctcaacagcggtaagatccttgagagttttcgccccgaagaacgttttccaatgatgagcacttttaaagttctgctatgtggcgcggtattatcccgtattgacgccgggcaagagcaactcggtcgccgcatacactattctcagaatgacttggttgagtactcaccagtcacagaaaagcatcttacggatggcatgacagtaagagaattatgcagtgctgccataaccatgagtgataacactgcggccaacttacttctgacaacgatcggaggaccgaaggagctaaccgcttttttgcacaacatgggggatcatgtaactcgccttgatcgttgggaaccggagctgaatgaagccataccaaacgacgagcgtgacaccacgatgcctgtagcaatggcaacaacgttgcgcaaactattaactggcgaactacttactctagcttcccggcaacaattaatagactggatggaggcggataaagttgcaggaccacttctgcgctcggcccttccggctggctggtttattgctgataaatctggagccggtgagcgtgggtctcgcggtatcattgcagcactggggccagatggtaagccctcccgtatcgtagttatctacacgacggggagtcaggcaactatggatgaacgaaatagacagatcgctgagataggtgcctcactgattaagcattggtaactgtcagaccaagtttactcatatatactttagattgatttaaaacttcatttttaatttaaaaggatctaggtgaagatcctttttgataatctcatgaccaaaatcccttaacgtgagttttcgttccactgagcgtcagaccccgtagaaaagatcaaaggatcttcttgagatcctttttttctgcgcgtaatctgctgcttgcaaacaaaaaaaccaccgctaccagcggtggtttgtttgccggatcaagagctaccaactctttttccgaaggtaactggcttcagcagagcgcagataccaaatactgtccttctagtgtagccgtagttaggccaccacttcaagaactctgtagcaccgcctacatacctcgctctgctaatcctgttaccagtggctgctgccagtggcgataagtcgtgtcttaccgggttggactcaagacgatagttaccggataaggcgcagcggtcgggctgaacggggggttcgtgcacacagcccagcttggagcgaacgacctacaccgaactgagatacctacagcgtgagctatgagaaagcgccacgcttcccgaagggagaaaggcggacaggtatccggtaagcggcagggtcggaacaggagagcgcacgagggagcttccagggggaaacgcctggtatctttatagtcctgtcgggtttcgccacctctgacttgagcgtcgatttttgtgatgctcgtcaggggggcggagcctatggaaaaacgccagcaacgcggcctttttacggttcctggccttttgctggccttttgctcacatgttctttcctgcgttatcccctgattctgtggataaccgtattaccgcctttgagtgagctgataccgctcgccgcagccgaacgaccgagcgcagcgagtcagtgagcgaggaagcggaagagcgcccaatacgcaaaccgcctctccccgcgcgttggccgattcattaatgcagctggcacgacaggtttcccgactggaaagcgggcagtgagcgcaacgcaattaatgtgagttagctcactcattaggcaccccaggctttacactttatgcttccggctcgtatgttgtgtggaattgtgagcggataacaatttcacacaggaaacagctatgaccatga

SEQ ID NO: 299 - DNA, 6463 bp, Synthetic construct
  source 1..6463: mol_type = other DNA
ggcgcgccggattcgacattgattattgactagttattaatagtaatcaattacggggtcattagttcatagcccatatatggagttccgcgttacataacttacggtaaatggcccgcctggctgaccgcccaacgacccccgcccattgacgtcaataatgacgtatgttcccatagtaacgccaatagggactttccattgacgtcaatgggtggagtatttacggtaaactgcccacttggcagtacatcaagtgtatcatatgccaagtacgccccctattgacgtcaatgacggtaaatggcccgcctggcattatgcccagtacatgaccttatgggactttcctacttggcagtacatctacgtattagtcatcgctattaccatggtcgaggtgagccccacgttctgcttcactctccccatctcccccccctccccacccccaattttgtatttatttattttttaattattttgtgcagcgatgggggcggggggggggggggggcgcgcgccaggcggggcggggcggggcgaggggcggggcggggcgaggcggagaggtgcggcggcagccaatcagagcggcgcgctccgaaagtttccttttatggcgaggcggcggcggcggcggccctataaaaagcgaagcgcgcggcgggcgggagtcgctgcgcgctgccttcgccccgtgccccgctccgccgccgcctcgcgccgcccgccccggctctgactgaccgcgttactcccacaggtgagcgggcgggacggcccttctcctccgggctgtaattagcgcttggtttaatgacggcttgtttcttttctgtggctgcgtgaaagccttgaggggctccgggagggccctttgtgcggggggagcggctcggggggtgcgtgcgtgtgtgtgtgcgtggggagcgccgcgtgcggctccgcgctgcccggcggctgtgagcgctgcgggcgcggcgcggggctttgtgcgctccgcagtgtgcgcgaggggagcgcggccgggggcggtgccccgcggtgcggggggggctgcgaggggaacaaaggctgcgtgcggggtgtgtgcgtgggggggtgagcagggggtgtgggcgcgtcggtcgggctgcaaccccccctgcacccccctccccgagttgctgagcacggcccggcttcgggtgcggggctccgtacggggcgtggcgcggggctcgccgtgccgggcggggggtggcggcaggtgggggtgccgggcggggcggggccgcctcgggccggggagggctcgggggaggggcgcggcggcccccggagcgccggcggctgtcgaggcgcggcgagccgcagccattgccttttatggtaatcgtgcgagagggcgcagggacttcctttgtcccaaatctgtgcggagccgaaatctgggaggcgccgccgcaccccctctagcgggcgcggggcgaagcggtgcggcgccggcaggaaggaaatgggcggggagggccttcgtgcgtcgccgcgccgccgtccccttctccctctccagcctcggggctgtccgcggggggacggctgccttcgggggggacggggcagggcggggttcggcttctggcgtgtgaccggcggctctagagcctctgctaaccatgttcatgccttcttctttttcctacagatccttaattaataatacgactcactataggggccgccaccatgcacggcctgcaggacgaccctgatctgcaggccctgctgaagggcagccagctgctgaaagtgaagtccagcagctggcggcgggaaagattctacaagctgcaagaggactgcaagaccatctggcaggagtctagaaaggtgatgcgctccccagaaagccaactgttcagcatcgaggacatccaggaggtgcggatgggccacagaacagagggactggaaaagttcgccagagatatccccgaggatagatgttttagcattgtgttcaaggaccagcggaacaccctggacctgatcgcccctagccctgctgatgcccagcattgggtccagggcctcagaaagatcatccaccacagcggctctatggaccagagacagaaactgcagaccggtgctagagcatctgttctgtctggcggagcacagcaggccgctgctgatacaggccactctaatcaggtgtcccagaactacagccccacctccatcctggacatcagacagggccccaaagagcccttccgggactacgtggacagattctacaagaccctgagagccgagcaggccagccaagaagtgaagaactggatgaccgagacactgctggtgcagaacgccaatcctgactgcaagaccatcctgaaggctctgggacctgccgccacactggaagagatgatgacagcctgtcaaggcgttggcggccctggacacaaagctagagttctggccgaggccatgagccaagtgaccaactccgctaccatcatgggaggatccggcggcagaatgaagcagctggaagataaggtggaagaactgctgagcaagaactaccacctggaaaacgaggtggcccggctgaagaagctcgttggagaaagaggtggcagcggcggagtttctggatggcggctgttcaagaagatcagcggcggttccggacctgctgccaagaagaaaaagaacggctccggactgcaactgcctccactggaaagactgacactgggagctgccgactacaaggacgacgacgacaagggcggagctagctctaagacaatcgtgctgtctgtgggcgaagccaccagaacactgaccgagatccagagcacagccgacagacagatcttcgaggaaaaagtgggccctctcgtgggcagactgagactgacagcttccctgagacagaacggcgccaagaccgcctacagagtgaacctgaagctggaccaggccgacgtggtggattctggccttcctaaagtgcggtacacccaagtgtggtcccacgacgtgaccatcgtggccaattctaccgaggccagcagaaagagcctgtacgacctgaccaagagcctggtggccacaagccaggtggaagatctggtcgtgaacctggtgcctctcggacgtggcggcagcgctggcggactccagagcagacctgaacctacagctccaccagaggaatccttccgcagcggcgtggaaaccacaacacctccacagaagcaagagcccatcgacaaagagctgtaccctctgaccagcctgagaagcctgttcggcaacgatcccagcagccagtaaaacgcgtaaatgattgcagatccactagttctagagctcgctgatcagcctcgactgtgccttctagttgccagccatctgttgtttgcccctcccccgtgccttccttgaccctggaaggtgccactcccactgtcctttcctaataaaatgaggaaattgcatcgcattgtctgagtaggtgtcattctattctggggggtggggtggggcaggacagcaagggggaggattgggaagacaatagcaggcatgctggggatgcggtgggctctatggcttctgaggcggaaagaaccagctggggctcgagatccactagttctagcctcgaggctagagcggccgccactggccgtcgttttacaacgtcgtgactgggaaaaccctggcgttacccaacttaatcgccttgcagcacatccccctttcgccagctggcgtaatagcgaagaggcccgcaccgatcgcccttcccaacagttgcgcagcctgaatggcgaatgggacgcgccctgtagcggcgcattaagcgcggcgggtgtggtggttacgcgcagcgtgaccgctacacttgccagcgccctagcgcccgctcctttcgctttcttcccttcctttctcgccacgttcgccggctttccccgtcaagctctaaatcgggggctccctttagggttccgatttagtgctttacggcacctcgaccccaaaaaacttgattagggtgatggttcacgtagtgggccatcgccctgatagacggtttttcgccctttgacgttggagtccacgttctttaatagtggactcttgttccaaactggaacaacactcaaccctatctcggtctattcttttgatttataagggattttgccgatttcggcctattggttaaaaaatgagctgatttaacaaaaatttaacgcgaattttaacaaaatattaacgcttacaatttaggtggcacttttcggggaaatgtgcgcggaacccctatttgtttatttttctaaatacattcaaatatgtatccgctcatgagacaataaccctgataaatgcttcaataatattgaaaaaggaagagtatgagtattcaacatttccgtgtcgcccttattcccttttttgcggcattttgccttcctgtttttgctcacccagaaacgctggtgaaagtaaaagatgctgaagatcagttgggtgcacgagtgggttacatcgaactggatctcaacagcggtaagatccttgagagttttcgccccgaagaacgttttccaatgatgagcacttttaaagttctgctatgtggcgcggtattatcccgtattgacgccgggcaagagcaactcggtcgccgcatacactattctcagaatgacttggttgagtactcaccagtcacagaaaagcatcttacggatggcatgacagtaagagaattatgcagtgctgccataaccatgagtgataacactgcggccaacttacttctgacaacgatcggaggaccgaaggagctaaccgcttttttgcacaacatgggggatcatgtaactcgccttgatcgttgggaaccggagctgaatgaagccataccaaacgacgagcgtgacaccacgatgcctgtagcaatggcaacaacgttgcgcaaactattaactggcgaactacttactctagcttcccggcaacaattaatagactggatggaggcggataaagttgcaggaccacttctgcgctcggcccttccggctggctggtttattgctgataaatctggagccggtgagcgtgggtctcgcggtatcattgcagcactggggccagatggtaagccctcccgtatcgtagttatctacacgacggggagtcaggcaactatggatgaacgaaatagacagatcgctgagataggtgcctcactgattaagcattggtaactgtcagaccaagtttactcatatatactttagattgatttaaaacttcatttttaatttaaaaggatctaggtgaagatcctttttgataatctcatgaccaaaatcccttaacgtgagttttcgttccactgagcgtcagaccccgtagaaaagatcaaaggatcttcttgagatcctttttttctgcgcgtaatctgctgcttgcaaacaaaaaaaccaccgctaccagcggtggtttgtttgccggatcaagagctaccaactctttttccgaaggtaactggcttcagcagagcgcagataccaaatactgtccttctagtgtagccgtagttaggccaccacttcaagaactctgtagcaccgcctacatacctcgctctgctaatcctgttaccagtggctgctgccagtggcgataagtcgtgtcttaccgggttggactcaagacgatagttaccggataaggcgcagcggtcgggctgaacggggggttcgtgcacacagcccagcttggagcgaacgacctacaccgaactgagatacctacagcgtgagctatgagaaagcgccacgcttcccgaagggagaaaggcggacaggtatccggtaagcggcagggtcggaacaggagagcgcacgagggagcttccagggggaaacgcctggtatctttatagtcctgtcgggtttcgccacctctgacttgagcgtcgatttttgtgatgctcgtcaggggggcggagcctatggaaaaacgccagcaacgcggcctttttacggttcctggccttttgctggccttttgctcacatgttctttcctgcgttatcccctgattctgtggataaccgtattaccgcctttgagtgagctgataccgctcgccgcagccgaacgaccgagcgcagcgagtcagtgagcgaggaagcggaagagcgcccaatacgcaaaccgcctctccccgcgcgttggccgattcattaatgcagctggcacgacaggtttcccgactggaaagcgggcagtgagcgcaacgcaattaatgtgagttagctcactcattaggcaccccaggctttacactttatgcttccggctcgtatgttgtgtggaattgtgagcggataacaatttcacacaggaaacagctatgaccatga

SEQ ID NO: 300 - DNA, 6457 bp, Synthetic construct
  source 1..6457: mol_type = other DNA
ggcgcgccggattcgacattgattattgactagttattaatagtaatcaattacggggtcattagttcatagcccatatatggagttccgcgttacataacttacggtaaatggcccgcctggctgaccgcccaacgacccccgcccattgacgtcaataatgacgtatgttcccatagtaacgccaatagggactttccattgacgtcaatgggtggagtatttacggtaaactgcccacttggcagtacatcaagtgtatcatatgccaagtacgccccctattgacgtcaatgacggtaaatggcccgcctggcattatgcccagtacatgaccttatgggactttcctacttggcagtacatctacgtattagtcatcgctattaccatggtcgaggtgagccccacgttctgcttcactctccccatctcccccccctccccacccccaattttgtatttatttattttttaattattttgtgcagcgatgggggcggggggggggggggggcgcgcgccaggcggggcggggcggggcgaggggcggggcggggcgaggcggagaggtgcggcggcagccaatcagagcggcgcgctccgaaagtttccttttatggcgaggcggcggcggcggcggccctataaaaagcgaagcgcgcggcgggcgggagtcgctgcgcgctgccttcgccccgtgccccgctccgccgccgcctcgcgccgcccgccccggctctgactgaccgcgttactcccacaggtgagcgggcgggacggcccttctcctccgggctgtaattagcgcttggtttaatgacggcttgtttcttttctgtggctgcgtgaaagccttgaggggctccgggagggccctttgtgcggggggagcggctcggggggtgcgtgcgtgtgtgtgtgcgtggggagcgccgcgtgcggctccgcgctgcccggcggctgtgagcgctgcgggcgcggcgcggggctttgtgcgctccgcagtgtgcgcgaggggagcgcggccgggggcggtgccccgcggtgcggggggggctgcgaggggaacaaaggctgcgtgcggggtgtgtgcgtgggggggtgagcagggggtgtgggcgcgtcggtcgggctgcaaccccccctgcacccccctccccgagttgctgagcacggcccggcttcgggtgcggggctccgtacggggcgtggcgcggggctcgccgtgccgggcggggggtggcggcaggtgggggtgccgggcggggcggggccgcctcgggccggggagggctcgggggaggggcgcggcggcccccggagcgccggcggctgtcgaggcgcggcgagccgcagccattgccttttatggtaatcgtgcgagagggcgcagggacttcctttgtcccaaatctgtgcggagccgaaatctgggaggcgccgccgcaccccctctagcgggcgcggggcgaagcggtgcggcgccggcaggaaggaaatgggcggggagggccttcgtgcgtcgccgcgccgccgtccccttctccctctccagcctcggggctgtccgcggggggacggctgccttcgggggggacggggcagggcggggttcggcttctggcgtgtgaccggcggctctagagcctctgctaaccatgttcatgccttcttctttttcctacagatccttaattaataatacgactcactataggggccgccaccatgcacggcctgcaggacgaccctgatctgcaggccctgctgaagggcagccagctgctgaaagtgaagtccagcagctggcggcgggaaagattctacaagctgcaagaggactgcaagaccatctggcaggagtctagaaaggtgatgcgctccccagaaagccaactgttcagcatcgaggacatccaggaggtgcggatgggccacagaacagagggactggaaaagttcgccagagatatccccgaggatagatgttttagcattgtgttcaaggaccagcggaacaccctggacctgatcgcccctagccctgctgatgcccagcattgggtccagggcctcagaaagatcatccaccacagcggctctatggaccagagacagaaactgcagaccggtgctagagcatctgttctgtctggcggagcacagcaggccgctgctgatacaggccactctaatcaggtgtcccagaactacagccccacctccatcctggacatcagacagggccccaaagagcccttccgggactacgtggacagattctacaagaccctgagagccgagcaggccagccaagaagtgaagaactggatgaccgagacactgctggtgcagaacgccaatcctgactgcaagaccatcctgaaggctctgggacctgccgccacactggaagagatgatgacagcctgtcaaggcgttggcggccctggacacaaagctagagttctggccgaggccatgagccaagtgaccaactccgctaccatcatgggaggatccggcggcagaatgaagcagctggaagataaggtggaagaactgctgagcaagaactaccacctggaaaacgaggtggcccggctgaagaagctcgttggagaaagaggtggcagcggcggagtttctggatggcggctgttcaagaagatcagcggcggttccggacctaagaagaaaagaaaggtgtccggactgcaactgcctccactggaaagactgacactgggagctgccgactacaaggacgacgacgacaagggcggagctagctctaagacaatcgtgctgtctgtgggcgaagccaccagaacactgaccgagatccagagcacagccgacagacagatcttcgaggaaaaagtgggccctctcgtgggcagactgagactgacagcttccctgagacagaacggcgccaagaccgcctacagagtgaacctgaagctggaccaggccgacgtggtggattctggccttcctaaagtgcggtacacccaagtgtggtcccacgacgtgaccatcgtggccaattctaccgaggccagcagaaagagcctgtacgacctgaccaagagcctggtggccacaagccaggtggaagatctggtcgtgaacctggtgcctctcggacgtggcggcagcgctggcggactccagagcagacctgaacctacagctccaccagaggaatccttccgcagcggcgtggaaaccacaacacctccacagaagcaagagcccatcgacaaagagctgtaccctctgaccagcctgagaagcctgttcggcaacgatcccagcagccagtaaaacgcgtaaatgattgcagatccactagttctagagctcgctgatcagcctcgactgtgccttctagttgccagccatctgttgtttgcccctcccccgtgccttccttgaccctggaaggtgccactcccactgtcctttcctaataaaatgaggaaattgcatcgcattgtctgagtaggtgtcattctattctggggggtggggtggggcaggacagcaagggggaggattgggaagacaatagcaggcatgctggggatgcggtgggctctatggcttctgaggcggaaagaaccagctggggctcgagatccactagttctagcctcgaggctagagcggccgccactggccgtcgttttacaacgtcgtgactgggaaaaccctggcgttacccaacttaatcgccttgcagcacatccccctttcgccagctggcgtaatagcgaagaggcccgcaccgatcgcccttcccaacagttgcgcagcctgaatggcgaatgggacgcgccctgtagcggcgcattaagcgcggcgggtgtggtggttacgcgcagcgtgaccgctacacttgccagcgccctagcgcccgctcctttcgctttcttcccttcctttctcgccacgttcgccggctttccccgtcaagctctaaatcgggggctccctttagggttccgatttagtgctttacggcacctcgaccccaaaaaacttgattagggtgatggttcacgtagtgggccatcgccctgatagacggtttttcgccctttgacgttggagtccacgttctttaatagtggactcttgttccaaactggaacaacactcaaccctatctcggtctattcttttgatttataagggattttgccgatttcggcctattggttaaaaaatgagctgatttaacaaaaatttaacgcgaattttaacaaaatattaacgcttacaatttaggtggcacttttcggggaaatgtgcgcggaacccctatttgtttatttttctaaatacattcaaatatgtatccgctcatgagacaataaccctgataaatgcttcaataatattgaaaaaggaagagtatgagtattcaacatttccgtgtcgcccttattcccttttttgcggcattttgccttcctgtttttgctcacccagaaacgctggtgaaagtaaaagatgctgaagatcagttgggtgcacgagtgggttacatcgaactggatctcaacagcggtaagatccttgagagttttcgccccgaagaacgttttccaatgatgagcacttttaaagttctgctatgtggcgcggtattatcccgtattgacgccgggcaagagcaactcggtcgccgcatacactattctcagaatgacttggttgagtactcaccagtcacagaaaagcatcttacggatggcatgacagtaagagaattatgcagtgctgccataaccatgagtgataacactgcggccaacttacttctgacaacgatcggaggaccgaaggagctaaccgcttttttgcacaacatgggggatcatgtaactcgccttgatcgttgggaaccggagctgaatgaagccataccaaacgacgagcgtgacaccacgatgcctgtagcaatggcaacaacgttgcgcaaactattaactggcgaactacttactctagcttcccggcaacaattaatagactggatggaggcggataaagttgcaggaccacttctgcgctcggcccttccggctggctggtttattgctgataaatctggagccggtgagcgtgggtctcgcggtatcattgcagcactggggccagatggtaagccctcccgtatcgtagttatctacacgacggggagtcaggcaactatggatgaacgaaatagacagatcgctgagataggtgcctcactgattaagcattggtaactgtcagaccaagtttactcatatatactttagattgatttaaaacttcatttttaatttaaaaggatctaggtgaagatcctttttgataatctcatgaccaaaatcccttaacgtgagttttcgttccactgagcgtcagaccccgtagaaaagatcaaaggatcttcttgagatcctttttttctgcgcgtaatctgctgcttgcaaacaaaaaaaccaccgctaccagcggtggtttgtttgccggatcaagagctaccaactctttttccgaaggtaactggcttcagcagagcgcagataccaaatactgtccttctagtgtagccgtagttaggccaccacttcaagaactctgtagcaccgcctacatacctcgctctgctaatcctgttaccagtggctgctgccagtggcgataagtcgtgtcttaccgggttggactcaagacgatagttaccggataaggcgcagcggtcgggctgaacggggggttcgtgcacacagcccagcttggagcgaacgacctacaccgaactgagatacctacagcgtgagctatgagaaagcgccacgcttcccgaagggagaaaggcggacaggtatccggtaagcggcagggtcggaacaggagagcgcacgagggagcttccagggggaaacgcctggtatctttatagtcctgtcgggtttcgccacctctgacttgagcgtcgatttttgtgatgctcgtcaggggggcggagcctatggaaaaacgccagcaacgcggcctttttacggttcctggccttttgctggccttttgctcacatgttctttcctgcgttatcccctgattctgtggataaccgtattaccgcctttgagtgagctgataccgctcgccgcagccgaacgaccgagcgcagcgagtcagtgagcgaggaagcggaagagcgcccaatacgcaaaccgcctctccccgcgcgttggccgattcattaatgcagctggcacgacaggtttcccgactggaaagcgggcagtgagcgcaacgcaattaatgtgagttagctcactcattaggcaccccaggctttacactttatgcttccggctcgtatgttgtgtggaattgtgagcggataacaatttcacacaggaaacagctatgaccatga

SEQ ID NO: 301 - DNA, 11966 bp, Synthetic construct
  source 1..11966: mol_type = other DNA
ggcgcgccggattcgacattgattattgactagttattaatagtaatcaattacggggtcattagttcatagcccatatatggagttccgcgttacataacttacggtaaatggcccgcctggctgaccgcccaacgacccccgcccattgacgtcaataatgacgtatgttcccatagtaacgccaatagggactttccattgacgtcaatgggtggagtatttacggtaaactgcccacttggcagtacatcaagtgtatcatatgccaagtacgccccctattgacgtcaatgacggtaaatggcccgcctggcattatgcccagtacatgaccttatgggactttcctacttggcagtacatctacgtattagtcatcgctattaccatggtcgaggtgagccccacgttctgcttcactctccccatctcccccccctccccacccccaattttgtatttatttattttttaattattttgtgcagcgatgggggcggggggggggggggggcgcgcgccaggcggggcggggcggggcgaggggcggggcggggcgaggcggagaggtgcggcggcagccaatcagagcggcgcgctccgaaagtttccttttatggcgaggcggcggcggcggcggccctataaaaagcgaagcgcgcggcgggcgggagtcgctgcgtcgcgccttcgccccgtgccccgctccgccgccgcctcgcgccgcccgccccggctctgactgaccgcgttactcccacaggtgagcgggcgggacggcccttctcctccgggctgtaattagcgcttggtttaatgacggctcgtttcttttctgtggctgcgtgaaagccttaaagggctccgggagggccctttgtgcgggggggagcggctcggggggtgcgtgcgtgtgtgtgtgcgtggggagcgccgcgtgcggcccgcgctgcccggcggctgtgagcgctgcgggcgcggcgcggggctttgtgcgctccgcgtgtgcgcgaggggagcgcggccgggggcggtgccccgcggtgcgggggggctgcgaggggaacaaaggctgcgtgcggggtgtgtgcgtgggggggtgagcagggggtgtgggcgcggcggtcgggctgtaacccccccctgcacccccctccccgagttgctgagcacggcccggcttcgggtgcggggctccgtgcggggcgtggcgcggggctcgccgtgccgggcggggggtggcggcaggtgggggtgccgggcggggcggggccgcctcgggccggggagggctcgggggaggggcgcggcggccccggagcgccggcggctgtcgaggcgcggcgagccgcagccattgccttttatggtaatcgtgcgagagggcgcagggacttcctttgtcccaaatctggcggagccgaaatctgggaggcgccgccgcaccccctctagcgggcgcgggcgaagcggtgcggcgccggcaggaaggaaatgggcggggagggccttcgtgcgtcgccgcgccgccgtccccttctccatctccagcctcggggctgccgcagggggacggctgccttcgggggggacggggcagggcggggttcggcttctggcgtgtgaccggcggctctagagcctctgctaaccatgttcatgccttcttctttttcctacagatccttaattaataatacgactcactataggggccgccaccatggacaagaagtacagcatcggcctggacatcggcaccaactctgtgggctgggccgtgatcaccgacgagtacaaggtgcccagcaagaaattcaaggtgctgggcaacaccgaccggcacagcatcaagaagaacctgatcggagccctgctgttcgacagcggcgaaacagccgaggccacccggctgaagagaaccgccagaagaagatacaccagacggaagaaccggatctgctatctgcaagagatcttcagcaacgagatggccaaggtggacgacagcttcttccacagactggaagagtccttcctggtggaagaggataagaagcacgagcggcaccccatcttcggcaacatcgtggacgaggtggcctaccacgagaagtaccccaccatctaccacctgagaaagaaactggtggacagcaccgacaaggccgacctgcggctgatctatctggccctggcccacatgatcaagttccggggccacttcctgatcgagggcgacctgaaccccgacaacagcgacgtggacaagctgttcatccagctggtgcagacctacaaccagctgttcgaggaaaaccccatcaacgccagcggcgtggacgccaaggccatcctgtctgccagactgagcaagagcagacggctggaaaatctgatcgcccagctgcccggcgagaagaagaatggcctgttcggcaacctgattgccctgagcctgggcctgacccccaacttcaagagcaacttcgacctggccgaggatgccaaactgcagctgagcaaggacacctacgacgacgacctggacaacctgctggcccagatcggcgaccagtacgccgacctgtttctggccgccaagaacctgtccgacgccatcctgctgagcgacatcctgagagtgaacaccgagatcaccaaggcccccctgagcgcctctatgatcaagagatacgacgagcaccaccaggacctgaccctgctgaaagctctcgtgcggcagcagctgcctgagaagtacaaagagattttcttcgaccagagcaagaacggctacgccggctacattgacggcggagccagccaggaagagttctacaagttcatcaagcccatcctggaaaagatggacggcaccgaggaactgctcgtgaagctgaacagagaggacctgctgcggaagcagcggaccttcgacaacggcagcatcccccaccagatccacctgggagagctgcacgccattctgcggcggcaggaagatttttacccattcctgaaggacaaccgggaaaagatcgagaagatcctgaccttccgcatcccctactacgtgggccctctggccaggggaaacagcagattcgcctggatgaccagaaagagcgaggaaaccatcaccccctggaacttcgaggaagtggtggacaagggcgcttccgcccagagcttcatcgagcggatgaccaacttcgataagaacctgcccaacgagaaggtgctgcccaagcacagcctgctgtacgagtacttcaccgtgtataacgagctgaccaaagtgaaatacgtgaccgagggaatgagaaagcccgccttcctgagcggcgagcagaaaaaggccatcgtggacctgctgttcaagaccaaccggaaagtgaccgtgaagcagctgaaagaggactacttcaagaaaatcgagtgcttcgactccgtggaaatctccggcgtggaagatcggttcaacgcctccctgggcacataccacgatctgctgaaaattatcaaggacaaggacttcctggacaatgaggaaaacgaggacattctggaagatatcgtgctgaccctgacactgtttgaggacagagagatgatcgaggaacggctgaaaacctatgcccacctgttcgacgacaaagtgatgaagcagctgaagcggcggagatacaccggctggggcaggctgagccggaagctgatcaacggcatccgggacaagcagtccggcaagacaatcctggatttcctgaagtccgacggcttcgccaacagaaacttcatgcagctgatccacgacgacagcctgacctttaaagaggacatccagaaagcccaggtgtccggccagggcgatagcctgcacgagcacattgccaatctggccggcagccccgccattaagaagggcatcctgcagacagtgaaggtggtggacgagctcgtgaaagtgatgggccggcacaagcccgagaacatcgtgatcgaaatggccagagagaaccagaccacccagaagggacagaagaacagccgcgagagaatgaagcggatcgaagagggcatcaaagagctgggcagccagatcctgaaagaacaccccgtggaaaacacccagctgcagaacgagaagctgtacctgtactacctgcagaatgggcgggatatgtacgtggaccaggaactggacatcaaccggctgtccgactacgatgtggaccatatcgtgcctcagagctttctgaaggacgactccatcgacaacaaggtgctgaccagaagcgacaaggcccggggcaagagcgacaacgtgccctccgaagaggtcgtgaagaagatgaagaactactggcggcagctgctgaacgccaagctgattacccagagaaagttcgacaatctgaccaaggccgagagaggcggcctgagcgaactggataaggccggcttcatcaagagacagctggtggaaacccggcagatcacaaagcacgtggcacagatcctggactcccggatgaacactaagtacgacgagaatgacaagctgatccgggaagtgaaagtgatcaccctgaagtccaagctggtgtccgatttccggaaggatttccagttttacaaagtgcgcgagatcaacaactaccaccacgcccacgacgcctacctgaacgccgtcgtgggaaccgccctgatcaaaaagtaccctaagctggaaagcgagttcgtgtacggcgactacaaggtgtacgacgtgcggaagatgatcgccaagagcgagcaggaaatcggcaaggctaccgccaagtacttcttctacagcaacatcatgaactttttcaagaccgagattaccctggccaacggcgagatccggaagcggcctctgatcgagacaaacggcgaaaccggggagatcgtgtgggataagggccgggattttgccaccgtgcggaaagtgctgagcatgccccaagtgaatatcgtgaaaaagaccgaggtgcagacaggcggcttcagcaaagagtctatcctgcccaagaggaacagcgataagctgatcgccagaaagaaggactgggaccctaagaagtacggcggcttcgacagccccaccgtggcctattctgtgctggtggtggccaaagtggaaaagggcaagtccaagaaactgaagagtgtgaaagagctgctggggatcaccatcatggaaagaagcagcttcgagaagaatcccatcgactttctggaagccaagggctacaaagaagtgaaaaaggacctgatcatcaagctgcctaagtactccctgttcgagctggaaaacggccggaagagaatgctggcctctgccggcgaactgcagaagggaaacgaactggccctgccctccaaatatgtgaacttcctgtacctggccagccactatgagaagctgaagggctcccccgaggataatgagcagaaacagctgtttgtggaacagcacaagcactacctggacgagatcatcgagcagatcagcgagttctccaagagagtgatcctggccgacgctaatctggacaaagtgctgtccgcctacaacaagcaccgggataagcccatcagagagcaggccgagaatatcatccacctgtttaccctgaccaatctgggagcccctgccgccttcaagtactttgacaccaccatcgaccggaagaggtacaccagcaccaaagaggtgctggacgccaccctgatccaccagagcatcaccggcctgtacgagacacggatcgacctgtctcagctgggaggcgacgcctatccctatgacgtgcccgattatgccagcctgggctccggatcccccaagaagaaacgcaaggtggaagatggcgagggcccagccgctaagagagtgaaactggattccggagctgctcctgccgccaagaagaagaaactcgacaccggtggacctggaagcgagcctgctacatctggctctgagacacctggcacctccgagtctgctacacctgaatctggacctggcgctagcaccctgaacatcgaggacgagtaccggctgcacgagacaagcaaagaacccgatgtgtccctgggcagcacctggcttagtgatttccctcaggcctgggccgagacaggcggaatgggacttgctgttagacaggcccctctgatcatccctctgaaggccacaagcacccctgtgtccatcaagcagtaccccatgagccaagaggcccggctgggaatcaagccccacattcagagactgctggaccagggcatcctggtgccttgtcagagcccttggaatacccctctgctgcccgtgaagaagcccggcaccaacgattacagacccgtgcaggacctgcgggaagtgaacaagagagtggaagatattcaccccaccgtgccgaatccttacaacctgctgtctggcctgcctcctagccaccagtggtacacagtgctggacctgaaggacgccttcttctgtctgcggctgcaccctacaagccagcctctgtttgcctttgagtggcgggaccctgagatgggcattagcggacagctgacctggaccagactgccccagggcttcaagaacagccccacactgttcaacgaggccctgcatagggacctcgccgacttcagaatccagcatcctgacctgatcctgctccagtacgtggacgatctgctgctggccgctacaagcgagctggattgtcagcagggaacaagagccctgctgcaaaccctgggcaacctgggctatagagcctctgccaagaaggcccagatttgccagaaacaagtgaagtatctgggctacctgctgaaagagggccagcgttggctgaccgaggccagaaaagaaaccgtgatgggccagcctacacctaagacacccagacagctgagagagttcctgggcaaagccggattctgtcggctgttcatccctggctttgccgagatggctgcccctctgtacccactgacaaagcccggaactctgttcaactggggcccagatcagcagaaggcctaccaagagatcaagcaggctctgctgacagcccctgctctgggactgcctgatctgaccaagcctttcgagctgttcgtggacgagaagcagggctatgccaaaggcgtgctgacacagaagctcggcccttggagaaggcctgtggcctacctgagcaagaaactggaccctgtggctgccggatggcctccttgtctgagaatggtggccgccattgccgtgctgaccaaggatgccggaaagctgacaatgggacagcctctggtcattctggcccctcatgccgtggaagccctcgtgaaacagcctcctgatcggtggctgagcaacgccaggatgacacactatcaggcactgctgctcgacaccgacagagtgcagtttggacctgtggtggccctgaatcctgccacacttctgcctctgcctgaggaaggcctccagcacaattgcctggacatcctggccgaggctcacggcacaagacccgatctgacagatcagccactgcctgacgccgaccacacctggtatacagatggcagctctctgctgcaagaaggacagagaaaagccggggctgccgtgaccaccgagacagaagtgatttgggccaaagctctgcccgctggcacatctgctcagagagccgaactgatcgccctgacacaggccctgaaaatggccgagggcaagaagctgaacgtctacaccgactccagatacgccttcgccaccgctcacatccacggcgaaatctatcggcggagaggatggctgaccagcgagggcaaagagattaagaacaaggacgagattctcgccctgctcaaggccctgttcctgcctaagcggctgagcatcatccactgtccaggccaccagaagggccactctgctgaagctagaggcaacagaatggccgaccaggctgccagaaaggccgccatcacagagacacccgataccagcacactgctgatcgagaacagcagccctggtacccctaagaagaagcggaaagtggacggatccggcgccaccaatttcagcctgctgaaacaggctggcgacgtggaagaaaatcccgggcctatggaccactacctggacatcagactgcggcccgatcctgagtttcctccagctcagctgatgagcgtgctgttcggcaaactgcaccaggctctggttgcccaaggcggcgatagaatcggagtgtcattccccgacctggacgagagcagaagcagactgggagagagactgagaatccacgccagcgccgatgatctgagagccctgcttgctagaccttggctggaaggcctgagagatcacctccagtttggagagcctgccgtggtgcctcatccaacaccatatagacaggtgtccagagtgcaggccaagagcaaccccgaaagactgcggagaaggctgatgcggagacacgacctgtctgaggaagaggcccggaagagaatccccgacacagtggctagagccctggacctgcctttcgtgacactgagaagccagagcaccggccagcacttccggctgtttatcagacacggccctctgcaagtgaccgccgaagaaggcggctttacctgttacggcctgagcaaaggcggattcgtgccctggttttgaacgcgtgctcgctttcttgctgtccaatttctattaaaggttcctttgttcgcgttgctggaccagaagatatggcttcggttcagcaaaatgattgcagatccactagttctagagctcgctgatcagcctcgactgtgccttctagttgccagccatctgttgtttgcccctcccccgtgccttccttgaccctggaaggtgccactcccactgtcctttcctaataaaatgaggaaattgcatcgcattgtctgagtaggtgtcattctattctggggggtggggtggggcaggacagcaagggggaggattgggaagacaatagcaggcatgctggggatgcggtgggctctatggcttctgaggcggaaagaaccagctggggctcgagatccactagttctagcctcgaggctagagcggccgccactggccgtcgttttacaacgtcgtgactgggaaaaccctggcgttacccaacttaatcgccttgcagcacatccccctttcgccagctggcgtaatagcgaagaggcccgcaccgatcgcccttcccaacagttgcgcagcctgaatggcgaatgggacgcgccctgtagcggcgcattaagcgcggcgggtgtggtggttacgcgcagcgtgaccgctacacttgccagcgccctagcgcccgctcctttcgctttcttcccttcctttctcgccacgttcgccggctttccccgtcaagctctaaatcgggggctccctttagggttccgatttagtgctttacggcacctcgaccccaaaaaacttgattagggtgatggttcacgtagtgggccatcgccctgatagacggtttttcgccctttgacgttggagtccacgttctttaatagtggactcttgttccaaactggaacaacactcaaccctatctcggtctattcttttgatttataagggattttgccgatttcggcctattggttaaaaaatgagctgatttaacaaaaatttaacgcgaattttaacaaaatattaacgcttacaatttaggtggcacttttcggggaaatgtgcgcggaacccctatttgtttatttttctaaatacattcaaatatgtatccgctcatgagacaataaccctgataaatgcttcaataatattgaaaaaggaagagtatgagtattcaacatttccgtgtcgcccttattcccttttttgcggcattttgccttcctgtttttgctcacccagaaacgctggtgaaagtaaaagatgctgaagatcagttgggtgcacgagtgggttacatcgaactggatctcaacagcggtaagatccttgagagttttcgccccgaagaacgttttccaatgatgagcacttttaaagttctgctatgtggcgcggtattatcccgtattgacgccgggcaagagcaactcggtcgccgcatacactattctcagaatgacttggttgagtactcaccagtcacagaaaagcatcttacggatggcatgacagtaagagaattatgcagtgctgccataaccatgagtgataacactgcggccaacttacttctgacaacgatcggaggaccgaaggagctaaccgcttttttgcacaacatgggggatcatgtaactcgccttgatcgttgggaaccggagctgaatgaagccataccaaacgacgagcgtgacaccacgatgcctgtagcaatggcaacaacgttgcgcaaactattaactggcgaactacttactctagcttcccggcaacaattaatagactggatggaggcggataaagttgcaggaccacttctgcgctcggcccttccggctggctggtttattgctgataaatctggagccggtgagcgtgggtctcgcggtatcattgcagcactggggccagatggtaagccctcccgtatcgtagttatctacacgacggggagtcaggcaactatggatgaacgaaatagacagatcgctgagataggtgcctcactgattaagcattggtaactgtcagaccaagtttactcatatatactttagattgatttaaaacttcatttttaatttaaaaggatctaggtgaagatcctttttgataatctcatgaccaaaatcccttaacgtgagttttcgttccactgagcgtcagaccccgtagaaaagatcaaaggatcttcttgagatcctttttttctgcgcgtaatctgctgcttgcaaacaaaaaaaccaccgctaccagcggtggtttgtttgccggatcaagagctaccaactctttttccgaaggtaactggcttcagcagagcgcagataccaaatactgtccttctagtgtagccgtagttaggccaccacttcaagaactctgtagcaccgcctacatacctcgctctgctaatcctgttaccagtggctgctgccagtggcgataagtcgtgtcttaccgggttggactcaagacgatagttaccggataaggcgcagcggtcgggctgaacggggggttcgtgcacacagcccagcttggagcgaacgacctacaccgaactgagatacctacagcgtgagctatgagaaagcgccacgcttcccgaagggagaaaggcggacaggtatccggtaagcggcagggtcggaacaggagagcgcacgagggagcttccagggggaaacgcctggtatctttatagtcctgtcgggtttcgccacctctgacttgagcgtcgatttttgtgatgctcgtcaggggggcggagcctatggaaaaacgccagcaacgcggcctttttacggttcctggccttttgctggccttttgctcacatgttctttcctgcgttatcccctgattctgtggataaccgtattaccgcctttgagtgagctgataccgctcgccgcagccgaacgaccgagcgcagcgagtcagtgagcgaggaagcggaagagcgcccaatacgcaaaccgcctctccccgcgcgttggccgattcattaatgcagctggcacgacaggtttcccgactggaaagcgggcagtgagcgcaacgcaattaatgtgagttagctcactcattaggcaccccaggctttacactttatgcttccggctcgtatgttgtgtggaattgtgagcggataacaatttcacacaggaaacagctatgaccatga

SEQ ID NO: 302 - DNA, 3445 bp, Synthetic construct
  source 1..3445: mol_type = other DNA
ataaaacctgcaggcatgcaagcgatcgcggggccgcccccttcaccgagggcctatttcccatgattccttcatatttgcatatacgatacaaggctgttagagagataattggaattaatttgactgtaaacacaaagatattagtacaaaatacgtgacgtagaaagtaataatttcttgggtagtttgcagttttaaaattatgttttaaaatggactatcatatgcttaccgtaacttgaaagtatttcgatttcttggctttatatatcttgtggaaaggacgaaacaccgggcgaagcaggccacgccggtttcagagccaccagaagatatggcttcggtggcaagttgaaataaggctagtccgttatcaacttgaaaaagtggcaccgagtcggtgctgtgaccaccttaggctacggcgtggcctgcttcaagttcactgccgtataggcagctaagaaacgcggttctatctagttacgcgttaaaccaactagaattttttactagttctagagcggccccaattcgccctatagtgagtcgtattacgcgcgctcactggccgtcgttttacaacgtcgtgactgggaaaaccctggcgttacccaacttaatcgccttgcagcacatccccctttcgccagctggcgtaatagcgaagaggcccgcaccgatcgcccttcccaacagttgcgcagcctgaatggcgaatgggacgcgccctgtagcggcgcattaagcgcggcgggtgtggtggttacgcgcagcgtgaccgctacacttgccagcgccctagcgcccgctcctttcgctttcttcccttcctttctcgccacgttcgccggctttccccgtcaagctctaaatcgggggctccctttagggttccgatttagtgctttacggcacctcgaccccaaaaaacttgattagggtgatggttcacgtagtgggccatcgccctgatagacggtttttcgccctttgacgttggagtccacgttctttaatagtggactcttgttccaaactggaacaacactcaaccctatctcggtctattcttttgatttataagggattttgccgatttcggcctattggttaaaaaatgagctgatttaacaaaaatttaacgcgaattttaacaaaatattaacgcttacaatttaggtggcacttttcggggaaatgtgcgcggaacccctatttgtttatttttctaaatacattcaaatatgtatccgctcatgagacaataaccctgataaatgcttcaataatattgaaaaaggaagagtatgagtattcaacatttccgtgtcgcccttattcccttttttgcggcattttgccttcctgtttttgctcacccagaaacgctggtgaaagtaaaagatgctgaagatcagttgggtgcacgagtgggttacatcgaactggatctcaacagcggtaagatccttgagagttttcgccccgaagaacgttttccaatgatgagcacttttaaagttctgctatgtggcgcggtattatcccgtattgacgccgggcaagagcaactcggtcgccgcatacactattctcagaatgacttggttgagtactcaccagtcacagaaaagcatcttacggatggcatgacagtaagagaattatgcagtgctgccataaccatgagtgataacactgcggccaacttacttctgacaacgatcggaggaccgaaggagctaaccgcttttttgcacaacatgggggatcatgtaactcgccttgatcgttgggaaccggagctgaatgaagccataccaaacgacgagcgtgacaccacgatgcctgtagcaatggcaacaacgttgcgcaaactattaactggcgaactacttactctagcttcccggcaacaattaatagactggatggaggcggataaagttgcaggaccacttctgcgctcggcccttccggctggctggtttattgctgataaatctggagccggtgagcgtgggtctcgcggtatcattgcagcactggggccagatggtaagccctcccgtatcgtagttatctacacgacggggagtcaggcaactatggatgaacgaaatagacagatcgctgagataggtgcctcactgattaagcattggtaactgtcagaccaagtttactcatatatactttagattgatttaaaacttcatttttaatttaaaaggatctaggtgaagatcctttttgataatctcatgaccaaaatcccttaacgtgagttttcgttccactgagcgtcagaccccgtagaaaagatcaaaggatcttcttgagatcctttttttctgcgcgtaatctgctgcttgcaaacaaaaaaaccaccgctaccagcggtggtttgtttgccggatcaagagctaccaactctttttccgaaggtaactggcttcagcagagcgcagataccaaatactgtccttctagtgtagccgtagttaggccaccacttcaagaactctgtagcaccgcctacatacctcgctctgctaatcctgttaccagtggctgctgccagtggcgataagtcgtgtcttaccgggttggactcaagacgatagttaccggataaggcgcagcggtcgggctgaacggggggttcgtgcacacagcccagcttggagcgaacgacctacaccgaactgagatacctacagcgtgagctatgagaaagcgccacgcttcccgaagggagaaaggcggacaggtatccggtaagcggcagggtcggaacaggagagcgcacgagggagcttccagggggaaacgcctggtatctttatagtcctgtcgggtttcgccacctctgacttgagcgtcgatttttgtgatgctcgtcaggggggcggagcctatggaaaaacgccagcaacgcggcctttttacggttcctggccttttgctggccttttgctcacatgttctttcctgcgttatcccctgattctgtggataaccgtattaccgcctttgagtgagctgataccgctcgccgcagccgaacgaccgagcgcagcgagtcagtgagcgaggaagcggaagagcgcccaatacgcaaaccgcctctccccgcgcgttggccgattcattaatgcagctggcacgacaggtttcccgactggaaagcgggcagtgagcgcaacgcaattaatgtgagttagctcactcattaggcaccccaggctttacactttatgcttccggctcgtatgttgtgtggaattgtgagcggataacaatttcacacaggaaacagctatgaccatgattacgccaagcgcgcaattaaccctcactaaagggaacaaaagctggaaacatgcatgaagttcctattccgaagttcctattctctagaaagtataggaacttc

SEQ ID NO: 303 - DNA, 3408 bp, Synthetic construct
  source 1..3408: mol_type = other DNA
ataaaacctgcaggcatgcaagcgatcgcggggccgcccccttcaccgagggcctatttcccatgattccttcatatttgcatatacgatacaaggctgttagagagataattggaattaatttgactgtaaacacaaagatattagtacaaaatacgtgacgtagaaagtaataatttcttgggtagtttgcagttttaaaattatgttttaaaatggactatcatatgcttaccgtaacttgaaagtatttcgatttcttggctttatatatcttgtggaaaggacgaaacaccgggcgaagcaggccacgccggtttcagagccaccagaagatatggcttcggtggcaagttgaaataaggctagtccgttatcaacttgaaaaagtggcaccgagtcggtgctgtgaccaccttaggctacggcgtggcctgcttcaagttcactgccgtataggcagctaagaaattttttactagttctagagcggccccaattcgccctatagtgagtcgtattacgcgcgctcactggccgtcgttttacaacgtcgtgactgggaaaaccctggcgttacccaacttaatcgccttgcagcacatccccctttcgccagctggcgtaatagcgaagaggcccgcaccgatcgcccttcccaacagttgcgcagcctgaatggcgaatgggacgcgccctgtagcggcgcattaagcgcggcgggtgtggtggttacgcgcagcgtgaccgctacacttgccagcgccctagcgcccgctcctttcgctttcttcccttcctttctcgccacgttcgccggctttccccgtcaagctctaaatcgggggctccctttagggttccgatttagtgctttacggcacctcgaccccaaaaaacttgattagggtgatggttcacgtagtgggccatcgccctgatagacggtttttcgccctttgacgttggagtccacgttctttaatagtggactcttgttccaaactggaacaacactcaaccctatctcggtctattcttttgatttataagggattttgccgatttcggcctattggttaaaaaatgagctgatttaacaaaaatttaacgcgaattttaacaaaatattaacgcttacaatttaggtggcacttttcggggaaatgtgcgcggaacccctatttgtttatttttctaaatacattcaaatatgtatccgctcatgagacaataaccctgataaatgcttcaataatattgaaaaaggaagagtatgagtattcaacatttccgtgtcgcccttattcccttttttgcggcattttgccttcctgtttttgctcacccagaaacgctggtgaaagtaaaagatgctgaagatcagttgggtgcacgagtgggttacatcgaactggatctcaacagcggtaagatccttgagagttttcgccccgaagaacgttttccaatgatgagcacttttaaagttctgctatgtggcgcggtattatcccgtattgacgccgggcaagagcaactcggtcgccgcatacactattctcagaatgacttggttgagtactcaccagtcacagaaaagcatcttacggatggcatgacagtaagagaattatgcagtgctgccataaccatgagtgataacactgcggccaacttacttctgacaacgatcggaggaccgaaggagctaaccgcttttttgcacaacatgggggatcatgtaactcgccttgatcgttgggaaccggagctgaatgaagccataccaaacgacgagcgtgacaccacgatgcctgtagcaatggcaacaacgttgcgcaaactattaactggcgaactacttactctagcttcccggcaacaattaatagactggatggaggcggataaagttgcaggaccacttctgcgctcggcccttccggctggctggtttattgctgataaatctggagccggtgagcgtgggtctcgcggtatcattgcagcactggggccagatggtaagccctcccgtatcgtagttatctacacgacggggagtcaggcaactatggatgaacgaaatagacagatcgctgagataggtgcctcactgattaagcattggtaactgtcagaccaagtttactcatatatactttagattgatttaaaacttcatttttaatttaaaaggatctaggtgaagatcctttttgataatctcatgaccaaaatcccttaacgtgagttttcgttccactgagcgtcagaccccgtagaaaagatcaaaggatcttcttgagatcctttttttctgcgcgtaatctgctgcttgcaaacaaaaaaaccaccgctaccagcggtggtttgtttgccggatcaagagctaccaactctttttccgaaggtaactggcttcagcagagcgcagataccaaatactgtccttctagtgtagccgtagttaggccaccacttcaagaactctgtagcaccgcctacatacctcgctctgctaatcctgttaccagtggctgctgccagtggcgataagtcgtgtcttaccgggttggactcaagacgatagttaccggataaggcgcagcggtcgggctgaacggggggttcgtgcacacagcccagcttggagcgaacgacctacaccgaactgagatacctacagcgtgagctatgagaaagcgccacgcttcccgaagggagaaaggcggacaggtatccggtaagcggcagggtcggaacaggagagcgcacgagggagcttccagggggaaacgcctggtatctttatagtcctgtcgggtttcgccacctctgacttgagcgtcgatttttgtgatgctcgtcaggggggcggagcctatggaaaaacgccagcaacgcggcctttttacggttcctggccttttgctggccttttgctcacatgttctttcctgcgttatcccctgattctgtggataaccgtattaccgcctttgagtgagctgataccgctcgccgcagccgaacgaccgagcgcagcgagtcagtgagcgaggaagcggaagagcgcccaatacgcaaaccgcctctccccgcgcgttggccgattcattaatgcagctggcacgacaggtttcccgactggaaagcgggcagtgagcgcaacgcaattaatgtgagttagctcactcattaggcaccccaggctttacactttatgcttccggctcgtatgttgtgtggaattgtgagcggataacaatttcacacaggaaacagctatgaccatgattacgccaagcgcgcaattaaccctcactaaagggaacaaaagctggaaacatgcatgaagttcctattccgaagttcctattctctagaaagtataggaacttc

SEQ ID NO: 304 - DNA, 3445 bp, Synthetic construct
  source 1..3445: mol_type = other DNA
ataaaacctgcaggcatgcaagcgatcgcggggccgcccccttcaccgagggcctatttcccatgattccttcatatttgcatatacgatacaaggctgttagagagataattggaattaatttgactgtaaacacaaagatattagtacaaaatacgtgacgtagaaagtaataatttcttgggtagtttgcagttttaaaattatgttttaaaatggactatcatatgcttaccgtaacttgaaagtatttcgatttcttggctttatatatcttgtggaaaggacgaaacaccgggcgaagcaggccacgccggtttcagagccaccagaagatatggcttcggtggcaagttgaaataaggctagtccgttatcaacttgaaaaagtggcaccgagtcggtgctgtgaccaccttaggctacggcgtggcctgcttccgcggttctatctagttacgcgttaaaccaactagaaaagttcactgccgtataggcagctaagaaattttttactagttctagagcggccccaattcgccctatagtgagtcgtattacgcgcgctcactggccgtcgttttacaacgtcgtgactgggaaaaccctggcgttacccaacttaatcgccttgcagcacatccccctttcgccagctggcgtaatagcgaagaggcccgcaccgatcgcccttcccaacagttgcgcagcctgaatggcgaatgggacgcgccctgtagcggcgcattaagcgcggcgggtgtggtggttacgcgcagcgtgaccgctacacttgccagcgccctagcgcccgctcctttcgctttcttcccttcctttctcgccacgttcgccggctttccccgtcaagctctaaatcgggggctccctttagggttccgatttagtgctttacggcacctcgaccccaaaaaacttgattagggtgatggttcacgtagtgggccatcgccctgatagacggtttttcgccctttgacgttggagtccacgttctttaatagtggactcttgttccaaactggaacaacactcaaccctatctcggtctattcttttgatttataagggattttgccgatttcggcctattggttaaaaaatgagctgatttaacaaaaatttaacgcgaattttaacaaaatattaacgcttacaatttaggtggcacttttcggggaaatgtgcgcggaacccctatttgtttatttttctaaatacattcaaatatgtatccgctcatgagacaataaccctgataaatgcttcaataatattgaaaaaggaagagtatgagtattcaacatttccgtgtcgcccttattcccttttttgcggcattttgccttcctgtttttgctcacccagaaacgctggtgaaagtaaaagatgctgaagatcagttgggtgcacgagtgggttacatcgaactggatctcaacagcggtaagatccttgagagttttcgccccgaagaacgttttccaatgatgagcacttttaaagttctgctatgtggcgcggtattatcccgtattgacgccgggcaagagcaactcggtcgccgcatacactattctcagaatgacttggttgagtactcaccagtcacagaaaagcatcttacggatggcatgacagtaagagaattatgcagtgctgccataaccatgagtgataacactgcggccaacttacttctgacaacgatcggaggaccgaaggagctaaccgcttttttgcacaacatgggggatcatgtaactcgccttgatcgttgggaaccggagctgaatgaagccataccaaacgacgagcgtgacaccacgatgcctgtagcaatggcaacaacgttgcgcaaactattaactggcgaactacttactctagcttcccggcaacaattaatagactggatggaggcggataaagttgcaggaccacttctgcgctcggcccttccggctggctggtttattgctgataaatctggagccggtgagcgtgggtctcgcggtatcattgcagcactggggccagatggtaagccctcccgtatcgtagttatctacacgacggggagtcaggcaactatggatgaacgaaatagacagatcgctgagataggtgcctcactgattaagcattggtaactgtcagaccaagtttactcatatatactttagattgatttaaaacttcatttttaatttaaaaggatctaggtgaagatcctttttgataatctcatgaccaaaatcccttaacgtgagttttcgttccactgagcgtcagaccccgtagaaaagatcaaaggatcttcttgagatcctttttttctgcgcgtaatctgctgcttgcaaacaaaaaaaccaccgctaccagcggtggtttgtttgccggatcaagagctaccaactctttttccgaaggtaactggcttcagcagagcgcagataccaaatactgtccttctagtgtagccgtagttaggccaccacttcaagaactctgtagcaccgcctacatacctcgctctgctaatcctgttaccagtggctgctgccagtggcgataagtcgtgtcttaccgggttggactcaagacgatagttaccggataaggcgcagcggtcgggctgaacggggggttcgtgcacacagcccagcttggagcgaacgacctacaccgaactgagatacctacagcgtgagctatgagaaagcgccacgcttcccgaagggagaaaggcggacaggtatccggtaagcggcagggtcggaacaggagagcgcacgagggagcttccagggggaaacgcctggtatctttatagtcctgtcgggtttcgccacctctgacttgagcgtcgatttttgtgatgctcgtcaggggggcggagcctatggaaaaacgccagcaacgcggcctttttacggttcctggccttttgctggccttttgctcacatgttctttcctgcgttatcccctgattctgtggataaccgtattaccgcctttgagtgagctgataccgctcgccgcagccgaacgaccgagcgcagcgagtcagtgagcgaggaagcggaagagcgcccaatacgcaaaccgcctctccccgcgcgttggccgattcattaatgcagctggcacgacaggtttcccgactggaaagcgggcagtgagcgcaacgcaattaatgtgagttagctcactcattaggcaccccaggctttacactttatgcttccggctcgtatgttgtgtggaattgtgagcggataacaatttcacacaggaaacagctatgaccatgattacgccaagcgcgcaattaaccctcactaaagggaacaaaagctggaaacatgcatgaagttcctattccgaagttcctattctctagaaagtataggaacttc

SEQ ID NO: 305 - DNA, 3477 bp, Synthetic construct
  source 1..3477: mol_type = other DNA
ataaaacctgcaggcatgcaagcgatcgcggggccgcccccttcaccgagggcctatttcccatgattccttcatatttgcatatacgatacaaggctgttagagagataattggaattaatttgactgtaaacacaaagatattagtacaaaatacgtgacgtagaaagtaataatttcttgggtagtttgcagttttaaaattatgttttaaaatggactatcatatgcttaccgtaacttgaaagtatttcgatttcttggctttatatatcttgtggaaaggacgaaacaccgggcgaagcaggccacgccggtttcagagctatgctggaaacagcatagcaagttgaaataaggctagtccgttatcaacttgaaaaagtggcaccgagtcggtgctgtgaccaccttaggctacggcgtggcctgcttccaattccgaccagaagatatggcttcggttggaattgaagttcactgccgtataggcagctaagaaacgcggttctatctagttacgcgttaaaccaactagaattttttactagttctagagcggccccaattcgccctatagtgagtcgtattacgcgcgctcactggccgtcgttttacaacgtcgtgactgggaaaaccctggcgttacccaacttaatcgccttgcagcacatccccctttcgccagctggcgtaatagcgaagaggcccgcaccgatcgcccttcccaacagttgcgcagcctgaatggcgaatgggacgcgccctgtagcggcgcattaagcgcggcgggtgtggtggttacgcgcagcgtgaccgctacacttgccagcgccctagcgcccgctcctttcgctttcttcccttcctttctcgccacgttcgccggctttccccgtcaagctctaaatcgggggctccctttagggttccgatttagtgctttacggcacctcgaccccaaaaaacttgattagggtgatggttcacgtagtgggccatcgccctgatagacggtttttcgccctttgacgttggagtccacgttctttaatagtggactcttgttccaaactggaacaacactcaaccctatctcggtctattcttttgatttataagggattttgccgatttcggcctattggttaaaaaatgagctgatttaacaaaaatttaacgcgaattttaacaaaatattaacgcttacaatttaggtggcacttttcggggaaatgtgcgcggaacccctatttgtttatttttctaaatacattcaaatatgtatccgctcatgagacaataaccctgataaatgcttcaataatattgaaaaaggaagagtatgagtattcaacatttccgtgtcgcccttattcccttttttgcggcattttgccttcctgtttttgctcacccagaaacgctggtgaaagtaaaagatgctgaagatcagttgggtgcacgagtgggttacatcgaactggatctcaacagcggtaagatccttgagagttttcgccccgaagaacgttttccaatgatgagcacttttaaagttctgctatgtggcgcggtattatcccgtattgacgccgggcaagagcaactcggtcgccgcatacactattctcagaatgacttggttgagtactcaccagtcacagaaaagcatcttacggatggcatgacagtaagagaattatgcagtgctgccataaccatgagtgataacactgcggccaacttacttctgacaacgatcggaggaccgaaggagctaaccgcttttttgcacaacatgggggatcatgtaactcgccttgatcgttgggaaccggagctgaatgaagccataccaaacgacgagcgtgacaccacgatgcctgtagcaatggcaacaacgttgcgcaaactattaactggcgaactacttactctagcttcccggcaacaattaatagactggatggaggcggataaagttgcaggaccacttctgcgctcggcccttccggctggctggtttattgctgataaatctggagccggtgagcgtgggtctcgcggtatcattgcagcactggggccagatggtaagccctcccgtatcgtagttatctacacgacggggagtcaggcaactatggatgaacgaaatagacagatcgctgagataggtgcctcactgattaagcattggtaactgtcagaccaagtttactcatatatactttagattgatttaaaacttcatttttaatttaaaaggatctaggtgaagatcctttttgataatctcatgaccaaaatcccttaacgtgagttttcgttccactgagcgtcagaccccgtagaaaagatcaaaggatcttcttgagatcctttttttctgcgcgtaatctgctgcttgcaaacaaaaaaaccaccgctaccagcggtggtttgtttgccggatcaagagctaccaactctttttccgaaggtaactggcttcagcagagcgcagataccaaatactgtccttctagtgtagccgtagttaggccaccacttcaagaactctgtagcaccgcctacatacctcgctctgctaatcctgttaccagtggctgctgccagtggcgataagtcgtgtcttaccgggttggactcaagacgatagttaccggataaggcgcagcggtcgggctgaacggggggttcgtgcacacagcccagcttggagcgaacgacctacaccgaactgagatacctacagcgtgagctatgagaaagcgccacgcttcccgaagggagaaaggcggacaggtatccggtaagcggcagggtcggaacaggagagcgcacgagggagcttccagggggaaacgcctggtatctttatagtcctgtcgggtttcgccacctctgacttgagcgtcgatttttgtgatgctcgtcaggggggcggagcctatggaaaaacgccagcaacgcggcctttttacggttcctggccttttgctggccttttgctcacatgttctttcctgcgttatcccctgattctgtggataaccgtattaccgcctttgagtgagctgataccgctcgccgcagccgaacgaccgagcgcagcgagtcagtgagcgaggaagcggaagagcgcccaatacgcaaaccgcctctccccgcgcgttggccgattcattaatgcagctggcacgacaggtttcccgactggaaagcgggcagtgagcgcaacgcaattaatgtgagttagctcactcattaggcaccccaggctttacactttatgcttccggctcgtatgttgtgtggaattgtgagcggataacaatttcacacaggaaacagctatgaccatgattacgccaagcgcgcaattaaccctcactaaagggaacaaaagctggaaacatgcatgaagttcctattccgaagttcctattctctagaaagtataggaacttc

SEQ ID NO: 306 - DNA, 3440 bp, Synthetic construct
  source 1..3440: mol_type = other DNA
ataaaacctgcaggcatgcaagcgatcgcggggccgcccccttcaccgagggcctatttcccatgattccttcatatttgcatatacgatacaaggctgttagagagataattggaattaatttgactgtaaacacaaagatattagtacaaaatacgtgacgtagaaagtaataatttcttgggtagtttgcagttttaaaattatgttttaaaatggactatcatatgcttaccgtaacttgaaagtatttcgatttcttggctttatatatcttgtggaaaggacgaaacaccgggcgaagcaggccacgccggtttcagagctatgctggaaacagcatagcaagttgaaataaggctagtccgttatcaacttgaaaaagtggcaccgagtcggtgctgtgaccaccttaggctacggcgtggcctgcttccaattccgaccagaagatatggcttcggttggaattgaagttcactgccgtataggcagctaagaaattttttactagttctagagcggccccaattcgccctatagtgagtcgtattacgcgcgctcactggccgtcgttttacaacgtcgtgactgggaaaaccctggcgttacccaacttaatcgccttgcagcacatccccctttcgccagctggcgtaatagcgaagaggcccgcaccgatcgcccttcccaacagttgcgcagcctgaatggcgaatgggacgcgccctgtagcggcgcattaagcgcggcgggtgtggtggttacgcgcagcgtgaccgctacacttgccagcgccctagcgcccgctcctttcgctttcttcccttcctttctcgccacgttcgccggctttccccgtcaagctctaaatcgggggctccctttagggttccgatttagtgctttacggcacctcgaccccaaaaaacttgattagggtgatggttcacgtagtgggccatcgccctgatagacggtttttcgccctttgacgttggagtccacgttctttaatagtggactcttgttccaaactggaacaacactcaaccctatctcggtctattcttttgatttataagggattttgccgatttcggcctattggttaaaaaatgagctgatttaacaaaaatttaacgcgaattttaacaaaatattaacgcttacaatttaggtggcacttttcggggaaatgtgcgcggaacccctatttgtttatttttctaaatacattcaaatatgtatccgctcatgagacaataaccctgataaatgcttcaataatattgaaaaaggaagagtatgagtattcaacatttccgtgtcgcccttattcccttttttgcggcattttgccttcctgtttttgctcacccagaaacgctggtgaaagtaaaagatgctgaagatcagttgggtgcacgagtgggttacatcgaactggatctcaacagcggtaagatccttgagagttttcgccccgaagaacgttttccaatgatgagcacttttaaagttctgctatgtggcgcggtattatcccgtattgacgccgggcaagagcaactcggtcgccgcatacactattctcagaatgacttggttgagtactcaccagtcacagaaaagcatcttacggatggcatgacagtaagagaattatgcagtgctgccataaccatgagtgataacactgcggccaacttacttctgacaacgatcggaggaccgaaggagctaaccgcttttttgcacaacatgggggatcatgtaactcgccttgatcgttgggaaccggagctgaatgaagccataccaaacgacgagcgtgacaccacgatgcctgtagcaatggcaacaacgttgcgcaaactattaactggcgaactacttactctagcttcccggcaacaattaatagactggatggaggcggataaagttgcaggaccacttctgcgctcggcccttccggctggctggtttattgctgataaatctggagccggtgagcgtgggtctcgcggtatcattgcagcactggggccagatggtaagccctcccgtatcgtagttatctacacgacggggagtcaggcaactatggatgaacgaaatagacagatcgctgagataggtgcctcactgattaagcattggtaactgtcagaccaagtttactcatatatactttagattgatttaaaacttcatttttaatttaaaaggatctaggtgaagatcctttttgataatctcatgaccaaaatcccttaacgtgagttttcgttccactgagcgtcagaccccgtagaaaagatcaaaggatcttcttgagatcctttttttctgcgcgtaatctgctgcttgcaaacaaaaaaaccaccgctaccagcggtggtttgtttgccggatcaagagctaccaactctttttccgaaggtaactggcttcagcagagcgcagataccaaatactgtccttctagtgtagccgtagttaggccaccacttcaagaactctgtagcaccgcctacatacctcgctctgctaatcctgttaccagtggctgctgccagtggcgataagtcgtgtcttaccgggttggactcaagacgatagttaccggataaggcgcagcggtcgggctgaacggggggttcgtgcacacagcccagcttggagcgaacgacctacaccgaactgagatacctacagcgtgagctatgagaaagcgccacgcttcccgaagggagaaaggcggacaggtatccggtaagcggcagggtcggaacaggagagcgcacgagggagcttccagggggaaacgcctggtatctttatagtcctgtcgggtttcgccacctctgacttgagcgtcgatttttgtgatgctcgtcaggggggcggagcctatggaaaaacgccagcaacgcggcctttttacggttcctggccttttgctggccttttgctcacatgttctttcctgcgttatcccctgattctgtggataaccgtattaccgcctttgagtgagctgataccgctcgccgcagccgaacgaccgagcgcagcgagtcagtgagcgaggaagcggaagagcgcccaatacgcaaaccgcctctccccgcgcgttggccgattcattaatgcagctggcacgacaggtttcccgactggaaagcgggcagtgagcgcaacgcaattaatgtgagttagctcactcattaggcaccccaggctttacactttatgcttccggctcgtatgttgtgtggaattgtgagcggataacaatttcacacaggaaacagctatgaccatgattacgccaagcgcgcaattaaccctcactaaagggaacaaaagctggaaacatgcatgaagttcctattccgaagttcctattctctagaaagtataggaacttc

SEQ ID NO: 307 - DNA, 3481 bp, Synthetic construct
  source 1..3481: mol_type = other DNA
ataaaacctgcaggcatgcaagcgatcgcggggccgcccccttcaccgagggcctatttcccatgattccttcatatttgcatatacgatacaaggctgttagagagataattggaattaatttgactgtaaacacaaagatattagtacaaaatacgtgacgtagaaagtaataatttcttgggtagtttgcagttttaaaattatgttttaaaatggactatcatatgcttaccgtaacttgaaagtatttcgatttcttggctttatatatcttgtggaaaggacgaaacaccgggcgaagcaggccacgccggtttcagagctatgctggaaacagcatagcaagttgaaataaggctagtccgttatcaacttgaaaaagtggcaccgagtcggtgctgtgaccaccttaggctacggcgtggcctgcttccaattccgaccagaagatatggcttcggttggaattgttgacgcggttctatctagttacgcgttaaaccaactagaaaagttcactgccgtataggcagctaagaaattttttactagttctagagcggccccaattcgccctatagtgagtcgtattacgcgcgctcactggccgtcgttttacaacgtcgtgactgggaaaaccctggcgttacccaacttaatcgccttgcagcacatccccctttcgccagctggcgtaatagcgaagaggcccgcaccgatcgcccttcccaacagttgcgcagcctgaatggcgaatgggacgcgccctgtagcggcgcattaagcgcggcgggtgtggtggttacgcgcagcgtgaccgctacacttgccagcgccctagcgcccgctcctttcgctttcttcccttcctttctcgccacgttcgccggctttccccgtcaagctctaaatcgggggctccctttagggttccgatttagtgctttacggcacctcgaccccaaaaaacttgattagggtgatggttcacgtagtgggccatcgccctgatagacggtttttcgccctttgacgttggagtccacgttctttaatagtggactcttgttccaaactggaacaacactcaaccctatctcggtctattcttttgatttataagggattttgccgatttcggcctattggttaaaaaatgagctgatttaacaaaaatttaacgcgaattttaacaaaatattaacgcttacaatttaggtggcacttttcggggaaatgtgcgcggaacccctatttgtttatttttctaaatacattcaaatatgtatccgctcatgagacaataaccctgataaatgcttcaataatattgaaaaaggaagagtatgagtattcaacatttccgtgtcgcccttattcccttttttgcggcattttgccttcctgtttttgctcacccagaaacgctggtgaaagtaaaagatgctgaagatcagttgggtgcacgagtgggttacatcgaactggatctcaacagcggtaagatccttgagagttttcgccccgaagaacgttttccaatgatgagcacttttaaagttctgctatgtggcgcggtattatcccgtattgacgccgggcaagagcaactcggtcgccgcatacactattctcagaatgacttggttgagtactcaccagtcacagaaaagcatcttacggatggcatgacagtaagagaattatgcagtgctgccataaccatgagtgataacactgcggccaacttacttctgacaacgatcggaggaccgaaggagctaaccgcttttttgcacaacatgggggatcatgtaactcgccttgatcgttgggaaccggagctgaatgaagccataccaaacgacgagcgtgacaccacgatgcctgtagcaatggcaacaacgttgcgcaaactattaactggcgaactacttactctagcttcccggcaacaattaatagactggatggaggcggataaagttgcaggaccacttctgcgctcggcccttccggctggctggtttattgctgataaatctggagccggtgagcgtgggtctcgcggtatcattgcagcactggggccagatggtaagccctcccgtatcgtagttatctacacgacggggagtcaggcaactatggatgaacgaaatagacagatcgctgagataggtgcctcactgattaagcattggtaactgtcagaccaagtttactcatatatactttagattgatttaaaacttcatttttaatttaaaaggatctaggtgaagatcctttttgataatctcatgaccaaaatcccttaacgtgagttttcgttccactgagcgtcagaccccgtagaaaagatcaaaggatcttcttgagatcctttttttctgcgcgtaatctgctgcttgcaaacaaaaaaaccaccgctaccagcggtggtttgtttgccggatcaagagctaccaactctttttccgaaggtaactggcttcagcagagcgcagataccaaatactgtccttctagtgtagccgtagttaggccaccacttcaagaactctgtagcaccgcctacatacctcgctctgctaatcctgttaccagtggctgctgccagtggcgataagtcgtgtcttaccgggttggactcaagacgatagttaccggataaggcgcagcggtcgggctgaacggggggttcgtgcacacagcccagcttggagcgaacgacctacaccgaactgagatacctacagcgtgagctatgagaaagcgccacgcttcccgaagggagaaaggcggacaggtatccggtaagcggcagggtcggaacaggagagcgcacgagggagcttccagggggaaacgcctggtatctttatagtcctgtcgggtttcgccacctctgacttgagcgtcgatttttgtgatgctcgtcaggggggcggagcctatggaaaaacgccagcaacgcggcctttttacggttcctggccttttgctggccttttgctcacatgttctttcctgcgttatcccctgattctgtggataaccgtattaccgcctttgagtgagctgataccgctcgccgcagccgaacgaccgagcgcagcgagtcagtgagcgaggaagcggaagagcgcccaatacgcaaaccgcctctccccgcgcgttggccgattcattaatgcagctggcacgacaggtttcccgactggaaagcgggcagtgagcgcaacgcaattaatgtgagttagctcactcattaggcaccccaggctttacactttatgcttccggctcgtatgttgtgtggaattgtgagcggataacaatttcacacaggaaacagctatgaccatgattacgccaagcgcgcaattaaccctcactaaagggaacaaaagctggaaacatgcatgaagttcctattccgaagttcctattctctagaaagtataggaacttc

SEQ ID NO: 308 - DNA, 3440 bp, Synthetic construct
  source 1..3440: mol_type = other DNA
ataaaacctgcaggcatgcaagcgatcgcggggccgcccccttcaccgagggcctatttcccatgattccttcatatttgcatatacgatacaaggctgttagagagataattggaattaatttgactgtaaacacaaagatattagtacaaaatacgtgacgtagaaagtaataatttcttgggtagtttgcagttttaaaattatgttttaaaatggactatcatatgcttaccgtaacttgaaagtatttcgatttcttggctttatatatcttgtggaaaggacgaaacaccgggcgaagcaggccacgccggtttcagagctatgctggaaacagcatagcaagttgaaataaggctagtccgttatcaacttgaaaaagtggcaccgagtcggtgctgtgaccaccttaggctacggcgtggcctgcttcaagttcactgccgtataggcagctaagaaacgcggttctatctagttacgcgttaaaccaactagaattttttactagttctagagcggccccaattcgccctatagtgagtcgtattacgcgcgctcactggccgtcgttttacaacgtcgtgactgggaaaaccctggcgttacccaacttaatcgccttgcagcacatccccctttcgccagctggcgtaatagcgaagaggcccgcaccgatcgcccttcccaacagttgcgcagcctgaatggcgaatgggacgcgccctgtagcggcgcattaagcgcggcgggtgtggtggttacgcgcagcgtgaccgctacacttgccagcgccctagcgcccgctcctttcgctttcttcccttcctttctcgccacgttcgccggctttccccgtcaagctctaaatcgggggctccctttagggttccgatttagtgctttacggcacctcgaccccaaaaaacttgattagggtgatggttcacgtagtgggccatcgccctgatagacggtttttcgccctttgacgttggagtccacgttctttaatagtggactcttgttccaaactggaacaacactcaaccctatctcggtctattcttttgatttataagggattttgccgatttcggcctattggttaaaaaatgagctgatttaacaaaaatttaacgcgaattttaacaaaatattaacgcttacaatttaggtggcacttttcggggaaatgtgcgcggaacccctatttgtttatttttctaaatacattcaaatatgtatccgctcatgagacaataaccctgataaatgcttcaataatattgaaaaaggaagagtatgagtattcaacatttccgtgtcgcccttattcccttttttgcggcattttgccttcctgtttttgctcacccagaaacgctggtgaaagtaaaagatgctgaagatcagttgggtgcacgagtgggttacatcgaactggatctcaacagcggtaagatccttgagagttttcgccccgaagaacgttttccaatgatgagcacttttaaagttctgctatgtggcgcggtattatcccgtattgacgccgggcaagagcaactcggtcgccgcatacactattctcagaatgacttggttgagtactcaccagtcacagaaaagcatcttacggatggcatgacagtaagagaattatgcagtgctgccataaccatgagtgataacactgcggccaacttacttctgacaacgatcggaggaccgaaggagctaaccgcttttttgcacaacatgggggatcatgtaactcgccttgatcgttgggaaccggagctgaatgaagccataccaaacgacgagcgtgacaccacgatgcctgtagcaatggcaacaacgttgcgcaaactattaactggcgaactacttactctagcttcccggcaacaattaatagactggatggaggcggataaagttgcaggaccacttctgcgctcggcccttccggctggctggtttattgctgataaatctggagccggtgagcgtgggtctcgcggtatcattgcagcactggggccagatggtaagccctcccgtatcgtagttatctacacgacggggagtcaggcaactatggatgaacgaaatagacagatcgctgagataggtgcctcactgattaagcattggtaactgtcagaccaagtttactcatatatactttagattgatttaaaacttcatttttaatttaaaaggatctaggtgaagatcctttttgataatctcatgaccaaaatcccttaacgtgagttttcgttccactgagcgtcagaccccgtagaaaagatcaaaggatcttcttgagatcctttttttctgcgcgtaatctgctgcttgcaaacaaaaaaaccaccgctaccagcggtggtttgtttgccggatcaagagctaccaactctttttccgaaggtaactggcttcagcagagcgcagataccaaatactgtccttctagtgtagccgtagttaggccaccacttcaagaactctgtagcaccgcctacatacctcgctctgctaatcctgttaccagtggctgctgccagtggcgataagtcgtgtcttaccgggttggactcaagacgatagttaccggataaggcgcagcggtcgggctgaacggggggttcgtgcacacagcccagcttggagcgaacgacctacaccgaactgagatacctacagcgtgagctatgagaaagcgccacgcttcccgaagggagaaaggcggacaggtatccggtaagcggcagggtcggaacaggagagcgcacgagggagcttccagggggaaacgcctggtatctttatagtcctgtcgggtttcgccacctctgacttgagcgtcgatttttgtgatgctcgtcaggggggcggagcctatggaaaaacgccagcaacgcggcctttttacggttcctggccttttgctggccttttgctcacatgttctttcctgcgttatcccctgattctgtggataaccgtattaccgcctttgagtgagctgataccgctcgccgcagccgaacgaccgagcgcagcgagtcagtgagcgaggaagcggaagagcgcccaatacgcaaaccgcctctccccgcgcgttggccgattcattaatgcagctggcacgacaggtttcccgactggaaagcgggcagtgagcgcaacgcaattaatgtgagttagctcactcattaggcaccccaggctttacactttatgcttccggctcgtatgttgtgtggaattgtgagcggataacaatttcacacaggaaacagctatgaccatgattacgccaagcgcgcaattaaccctcactaaagggaacaaaagctggaaacatgcatgaagttcctattccgaagttcctattctctagaaagtataggaacttc

SEQ ID NO: 309 - DNA, 3403 bp, Synthetic construct
  source 1..3403: mol_type = other DNA
ataaaacctgcaggcatgcaagcgatcgcggggccgcccccttcaccgagggcctatttcccatgattccttcatatttgcatatacgatacaaggctgttagagagataattggaattaatttgactgtaaacacaaagatattagtacaaaatacgtgacgtagaaagtaataatttcttgggtagtttgcagttttaaaattatgttttaaaatggactatcatatgcttaccgtaacttgaaagtatttcgatttcttggctttatatatcttgtggaaaggacgaaacaccgggcgaagcaggccacgccggtttcagagctatgctggaaacagcatagcaagttgaaataaggctagtccgttatcaacttgaaaaagtggcaccgagtcggtgctgtgaccaccttaggctacggcgtggcctgcttcaagttcactgccgtataggcagctaagaaattttttactagttctagagcggccccaattcgccctatagtgagtcgtattacgcgcgctcactggccgtcgttttacaacgtcgtgactgggaaaaccctggcgttacccaacttaatcgccttgcagcacatccccctttcgccagctggcgtaatagcgaagaggcccgcaccgatcgcccttcccaacagttgcgcagcctgaatggcgaatgggacgcgccctgtagcggcgcattaagcgcggcgggtgtggtggttacgcgcagcgtgaccgctacacttgccagcgccctagcgcccgctcctttcgctttcttcccttcctttctcgccacgttcgccggctttccccgtcaagctctaaatcgggggctccctttagggttccgatttagtgctttacggcacctcgaccccaaaaaacttgattagggtgatggttcacgtagtgggccatcgccctgatagacggtttttcgccctttgacgttggagtccacgttctttaatagtggactcttgttccaaactggaacaacactcaaccctatctcggtctattcttttgatttataagggattttgccgatttcggcctattggttaaaaaatgagctgatttaacaaaaatttaacgcgaattttaacaaaatattaacgcttacaatttaggtggcacttttcggggaaatgtgcgcggaacccctatttgtttatttttctaaatacattcaaatatgtatccgctcatgagacaataaccctgataaatgcttcaataatattgaaaaaggaagagtatgagtattcaacatttccgtgtcgcccttattcccttttttgcggcattttgccttcctgtttttgctcacccagaaacgctggtgaaagtaaaagatgctgaagatcagttgggtgcacgagtgggttacatcgaactggatctcaacagcggtaagatccttgagagttttcgccccgaagaacgttttccaatgatgagcacttttaaagttctgctatgtggcgcggtattatcccgtattgacgccgggcaagagcaactcggtcgccgcatacactattctcagaatgacttggttgagtactcaccagtcacagaaaagcatcttacggatggcatgacagtaagagaattatgcagtgctgccataaccatgagtgataacactgcggccaacttacttctgacaacgatcggaggaccgaaggagctaaccgcttttttgcacaacatgggggatcatgtaactcgccttgatcgttgggaaccggagctgaatgaagccataccaaacgacgagcgtgacaccacgatgcctgtagcaatggcaacaacgttgcgcaaactattaactggcgaactacttactctagcttcccggcaacaattaatagactggatggaggcggataaagttgcaggaccacttctgcgctcggcccttccggctggctggtttattgctgataaatctggagccggtgagcgtgggtctcgcggtatcattgcagcactggggccagatggtaagccctcccgtatcgtagttatctacacgacggggagtcaggcaactatggatgaacgaaatagacagatcgctgagataggtgcctcactgattaagcattggtaactgtcagaccaagtttactcatatatactttagattgatttaaaacttcatttttaatttaaaaggatctaggtgaagatcctttttgataatctcatgaccaaaatcccttaacgtgagttttcgttccactgagcgtcagaccccgtagaaaagatcaaaggatcttcttgagatcctttttttctgcgcgtaatctgctgcttgcaaacaaaaaaaccaccgctaccagcggtggtttgtttgccggatcaagagctaccaactctttttccgaaggtaactggcttcagcagagcgcagataccaaatactgtccttctagtgtagccgtagttaggccaccacttcaagaactctgtagcaccgcctacatacctcgctctgctaatcctgttaccagtggctgctgccagtggcgataagtcgtgtcttaccgggttggactcaagacgatagttaccggataaggcgcagcggtcgggctgaacggggggttcgtgcacacagcccagcttggagcgaacgacctacaccgaactgagatacctacagcgtgagctatgagaaagcgccacgcttcccgaagggagaaaggcggacaggtatccggtaagcggcagggtcggaacaggagagcgcacgagggagcttccagggggaaacgcctggtatctttatagtcctgtcgggtttcgccacctctgacttgagcgtcgatttttgtgatgctcgtcaggggggcggagcctatggaaaaacgccagcaacgcggcctttttacggttcctggccttttgctggccttttgctcacatgttctttcctgcgttatcccctgattctgtggataaccgtattaccgcctttgagtgagctgataccgctcgccgcagccgaacgaccgagcgcagcgagtcagtgagcgaggaagcggaagagcgcccaatacgcaaaccgcctctccccgcgcgttggccgattcattaatgcagctggcacgacaggtttcccgactggaaagcgggcagtgagcgcaacgcaattaatgtgagttagctcactcattaggcaccccaggctttacactttatgcttccggctcgtatgttgtgtggaattgtgagcggataacaatttcacacaggaaacagctatgaccatgattacgccaagcgcgcaattaaccctcactaaagggaacaaaagctggaaacatgcatgaagttcctattccgaagttcctattctctagaaagtataggaacttc

SEQ ID NO: 310 - DNA, 3440 bp, Synthetic construct
  source 1..3440: mol_type = other DNA
ataaaacctgcaggcatgcaagcgatcgcggggccgcccccttcaccgagggcctatttcccatgattccttcatatttgcatatacgatacaaggctgttagagagataattggaattaatttgactgtaaacacaaagatattagtacaaaatacgtgacgtagaaagtaataatttcttgggtagtttgcagttttaaaattatgttttaaaatggactatcatatgcttaccgtaacttgaaagtatttcgatttcttggctttatatatcttgtggaaaggacgaaacaccgggcgaagcaggccacgccggtttcagagctatgctggaaacagcatagcaagttgaaataaggctagtccgttatcaacttgaaaaagtggcaccgagtcggtgctgtgaccaccttaggctacggcgtggcctgcttccgcggttctatctagttacgcgttaaaccaactagaaaagttcactgccgtataggcagctaagaaattttttactagttctagagcggccccaattcgccctatagtgagtcgtattacgcgcgctcactggccgtcgttttacaacgtcgtgactgggaaaaccctggcgttacccaacttaatcgccttgcagcacatccccctttcgccagctggcgtaatagcgaagaggcccgcaccgatcgcccttcccaacagttgcgcagcctgaatggcgaatgggacgcgccctgtagcggcgcattaagcgcggcgggtgtggtggttacgcgcagcgtgaccgctacacttgccagcgccctagcgcccgctcctttcgctttcttcccttcctttctcgccacgttcgccggctttccccgtcaagctctaaatcgggggctccctttagggttccgatttagtgctttacggcacctcgaccccaaaaaacttgattagggtgatggttcacgtagtgggccatcgccctgatagacggtttttcgccctttgacgttggagtccacgttctttaatagtggactcttgttccaaactggaacaacactcaaccctatctcggtctattcttttgatttataagggattttgccgatttcggcctattggttaaaaaatgagctgatttaacaaaaatttaacgcgaattttaacaaaatattaacgcttacaatttaggtggcacttttcggggaaatgtgcgcggaacccctatttgtttatttttctaaatacattcaaatatgtatccgctcatgagacaataaccctgataaatgcttcaataatattgaaaaaggaagagtatgagtattcaacatttccgtgtcgcccttattcccttttttgcggcattttgccttcctgtttttgctcacccagaaacgctggtgaaagtaaaagatgctgaagatcagttgggtgcacgagtgggttacatcgaactggatctcaacagcggtaagatccttgagagttttcgccccgaagaacgttttccaatgatgagcacttttaaagttctgctatgtggcgcggtattatcccgtattgacgccgggcaagagcaactcggtcgccgcatacactattctcagaatgacttggttgagtactcaccagtcacagaaaagcatcttacggatggcatgacagtaagagaattatgcagtgctgccataaccatgagtgataacactgcggccaacttacttctgacaacgatcggaggaccgaaggagctaaccgcttttttgcacaacatgggggatcatgtaactcgccttgatcgttgggaaccggagctgaatgaagccataccaaacgacgagcgtgacaccacgatgcctgtagcaatggcaacaacgttgcgcaaactattaactggcgaactacttactctagcttcccggcaacaattaatagactggatggaggcggataaagttgcaggaccacttctgcgctcggcccttccggctggctggtttattgctgataaatctggagccggtgagcgtgggtctcgcggtatcattgcagcactggggccagatggtaagccctcccgtatcgtagttatctacacgacggggagtcaggcaactatggatgaacgaaatagacagatcgctgagataggtgcctcactgattaagcattggtaactgtcagaccaagtttactcatatatactttagattgatttaaaacttcatttttaatttaaaaggatctaggtgaagatcctttttgataatctcatgaccaaaatcccttaacgtgagttttcgttccactgagcgtcagaccccgtagaaaagatcaaaggatcttcttgagatcctttttttctgcgcgtaatctgctgcttgcaaacaaaaaaaccaccgctaccagcggtggtttgtttgccggatcaagagctaccaactctttttccgaaggtaactggcttcagcagagcgcagataccaaatactgtccttctagtgtagccgtagttaggccaccacttcaagaactctgtagcaccgcctacatacctcgctctgctaatcctgttaccagtggctgctgccagtggcgataagtcgtgtcttaccgggttggactcaagacgatagttaccggataaggcgcagcggtcgggctgaacggggggttcgtgcacacagcccagcttggagcgaacgacctacaccgaactgagatacctacagcgtgagctatgagaaagcgccacgcttcccgaagggagaaaggcggacaggtatccggtaagcggcagggtcggaacaggagagcgcacgagggagcttccagggggaaacgcctggtatctttatagtcctgtcgggtttcgccacctctgacttgagcgtcgatttttgtgatgctcgtcaggggggcggagcctatggaaaaacgccagcaacgcggcctttttacggttcctggccttttgctggccttttgctcacatgttctttcctgcgttatcccctgattctgtggataaccgtattaccgcctttgagtgagctgataccgctcgccgcagccgaacgaccgagcgcagcgagtcagtgagcgaggaagcggaagagcgcccaatacgcaaaccgcctctccccgcgcgttggccgattcattaatgcagctggcacgacaggtttcccgactggaaagcgggcagtgagcgcaacgcaattaatgtgagttagctcactcattaggcaccccaggctttacactttatgcttccggctcgtatgttgtgtggaattgtgagcggataacaatttcacacaggaaacagctatgaccatgattacgccaagcgcgcaattaaccctcactaaagggaacaaaagctggaaacatgcatgaagttcctattccgaagttcctattctctagaaagtataggaacttc

SEQ ID NO: 311 - DNA, 15127 bp, Synthetic construct
  source 1..15127: mol_type = other DNA
aaccttgttggtccaaaatgcgaacccagattgtaagactattttaaaagcattgggaccaggagcgacactagaagaaatgatgacagcatgtcagggagtggggggacccggccataaagcaagagttttggctgaagcaatgagccaagtaacaaatccagctaccataatgatacagaaaggcaattttaggaaccaaagaaagactgttaagtgtttcaattgtggcaaagaagggcacatagccaaaaattgcagggcccctaggaaaaagggctgttggaaatgtggaaaggaaggacaccaaatgaaagattgtactgagagacaggctaattttttagggaagatctggccttcccacaagggaaggccagggaattttcttcagagcagaccagagccaacagccccaccagaagagagcttcaggtttggggaagagacaacaactccctctcagaagcaggagccgatagacaaggaactgtatcctttagcttccctcagatcactctttggcagcgacccctcgtcacaataaagataggggggcaattaaaggaagctctattagatacaggagcagatgatacagtattagaagaaatgaatttgccaggaagatggaaaccaaaaatgatagggggaattggaggttttatcaaagtaagacagtatgatcagatactcatagaaatctgcggacataaagctataggtacagtattagtaggacctacacctgtcaacataattggaagaaatctgttgactcagattggctgcactttaaattttcccattagtcctattgagactgtaccagtaaaattaaagccaggaatggatggcccaaaagttaaacaatggccattgacagaagaaaaaataaaagcattagtagaaatttgtacagaaatggaaaaggaaggaaaaatttcaaaaattgggcctgaaaatccatacaatactccagtatttgccataaagaaaaaagacagtactaaatggagaaaattagtagatttcagagaacttaataagagaactcaagatttctgggaagttcaattaggaataccacatcctgcagggttaaaacagaaaaaatcagtaacagtactggatgtgggcgatgcatatttttcagttcccttagataaagacttcaggaagtatactgcatttaccatacctagtataaacaatgagacaccagggattagatatcagtacaatgtgcttccacagggatggaaaggatcaccagcaatattccagtgtagcatgacaaaaatcttagagccttttagaaaacaaaatccagacatagtcatctatcaatacatggatgatttgtatgtaggatctgacttagaaatagggcagcatagaacaaaaatagaggaactgagacaacatctgttgaggtggggatttaccacaccagacaaaaaacatcagaaagaacctccattcctttggatgggttatgaactccatcctgataaatggacagtacagcctatagtgctgccagaaaaggacagctggactgtcaatgacatacagaaattagtgggaaaattgaattgggcaagtcagatttatgcagggattaaagtaaggcaattatgtaaacttcttaggggaaccaaagcactaacagaagtagtaccactaacagaagaagcagagctagaactggcagaaaacagggagattctaaaagaaccggtacatggagtgtattatgacccatcaaaagacttaatagcagaaatacagaagcaggggcaaggccaatggacatatcaaatttatcaagagccatttaaaaatctgaaaacaggaaagtatgcaagaatgaagggtgcccacactaatgatgtgaaacaattaacagaggcagtacaaaaaatagccacagaaagcatagtaatatggggaaagactcctaaatttaaattacccatacaaaaggaaacatgggaagcatggtggacagagtattggcaagccacctggattcctgagtgggagtttgtcaatacccctcccttagtgaagttatggtaccagttagagaaagaacccataataggagcagaaactttctatgtagatggggcagccaatagggaaactaaattaggaaaagcaggatatgtaactgacagaggaagacaaaaagttgtccccctaacggacacaacaaatcagaagactgagttacaagcaattcatctagctttgcaggattcgggattagaagtaaacatagtgacagactcacaatatgcattgggaatcattcaagcacaaccagataagagtgaatcagagttagtcagtcaaataatagagcagttaataaaaaaggaaaaagtctacctggcatgggtaccagcacacaaaggaattggaggaaatgaacaagtagataaattggtcagtgctggaatcaggaaagtactatttttagatggaatagataaggcccaagaagaacatgagaaatatcacagtaattggagagcaatggctagtgattttaacctaccacctgtagtagcaaaagaaatagtagccagctgtgataaatgtcagctaaaaggggaagccatgcatggacaagtagactgtagcccaggaatatggcagctagtttgtacacatttagaaggaaaagttatcttggtagcagttcatgtagccagtggatatatagaagcagaagtaattccagcagagacagggcaagaaacagcatacttcctcttaaaattagcaggaagatggccagtaaaaacagtacatacagacaatggcagcaatttcaccagtactacagttaaggccgcctgttggtgggcggggatcaagcaggaatttggcattccctacaatccccaaagtcaaggagtaatagaatctatgaataaagaattaaagaaaattataggacaggtaagagatcaggctgaacatcttaagacagcagtacaaatggcagtattcatccacaattttaaaagaaaaggggggattggggggtacagtgcaggggaaagaatagtagacataatagcaacagacatacaaactaaagaattacaaaaacaaattacaaaaattcaaaattttcgggtttattacagggacagcagagatccagtttggaaaggaccagcaaagctcctctggaaaggtgaaggggcagtagtaatacaagataatagtgacataaaagtagtgccaagaagaaaagcaaagatcatcagggattatggaaaacagatggcaggtgatgattgtgtggcaagtagacaggatgaggattaacacatggaattctgcaacaactgctgtttatccatttcagaattgggtgtcgacatagcagaataggcgttactcgacagaggagagcaagaaatggagccagtagatcctagactagagccctggaagcatccaggaagtcagcctaaaactgcttgtaccaattgctattgtaaaaagtgttgctttcattgccaagtttgtttcatgacaaaagccttaggcatctcctatggcaggaagaagcggagacagcgacgaagagctcatcagaacagtcagactcatcaagcttctctatcaaagcagtaagtagtacatgtaatgcaacctataatagtagcaatagtagcattagtagtagcaataataatagcaatagttgtgtggtccatagtaatcatagaatataggaaaatggccgctgatcttcagacctggaggaggagatatgagggacaattggagaagtgaattatataaatataaagtagtaaaaattgaaccattaggagtagcacccaccaaggcaaagagaagagtggtgcagagagaaaaaagagcagtgggaataggagctttgttccttgggttcttgggagcagcaggaagcactatgggcgcagcgtcaatgacgctgacggtacaggccagacaattattgtctggtatagtgcagcagcagaacaatttgctgagggctattgaggcgcaacagcatctgttgcaactcacagtctggggcatcaagcagctccaggcaagaatcctggctgtggaaagatacctaaaggatcaacagctcctggggatttggggttgctctggaaaactcatttgcaccactgctgtgccttggaatgctagttggagtaataaatctctggaacagatttggaatcacacgacctggatggagtgggacagagaaattaacaattacacaagcttaatacactccttaattgaagaatcgcaaaaccagcaagaaaagaatgaacaagaattattggaattagataaatgggcaagtttgtggaattggtttaacataacaaattggctgtggtatataaaattattcataatgatagtaggaggcttggtaggtttaagaatagtttttgctgtactttctatagtgaatagagttaggcagggatattcaccattatcgtttcagacccacctcccaaccccgaggggacccgacaggcccgaaggaatagaagaagaaggtggagagagagacagagacagatccattcgattagtgaacggatccttggcacttatctgggacgatctgcggagcctgtgcctcttcagctaccaccgcttgagagacttactcttgattgtaacgaggattgtggaacttctgggacgcagggggtgggaagccctcaaatattggtggaatctcctacaatattggagtcaggagctaaagaatagtgctgttagcttgctcaatgccacagccatagcagtagctgaggggacagatagggttatagaagtagtacaaggagcttgtagagctattcgccacatacctagaagaataagacagggcttggaaaggattttgctataagctcgaaacaaccggtacctctagaactatagctagcagatctttttccctctgccaaaaattatggggacatcatgaagccccttgagcatctgacttctggctaataaaggaaatttattttcattgcaatagtgtgttggaattttttgtgtctctcactcggaaggacatatgggagggcaaatcatttaaaacatcagaatgagtatttggtttagagtttggcaacatatgcccatatgctggctgccatgaacaaaggttggctataaagaggtcatcagtatatgaaacagccccctgctgtccattccttattccatagaaaagccttgacttgaggttagattttttttatattttgttttgtgttatttttttctttaacatccctaaaattttccttacatgttttactagccagatttttcctcctctcctgactactcccagtcatagctgtccctcttctcttatggagatccctcgacctgcagcccaagcttggcgtaatcatggtcatagctgtttcctgtgtgaaattgttatccgctcacaattccacacaacatacgagccggaagcataaagtgtaaagcctggggtgcctaatgagtgagctaactcacattaattgcgttgcgctcactgcccgctttccagtcgggaaacctgtcgtgccagcggatccggcgcgccggattcgacattgattattgactagttattaatagtaatcaattacggggtcattagttcatagcccatatatggagttccgcgttacataacttacggtaaatggcccgcctggctgaccgcccaacgacccccgcccattgacgtcaataatgacgtatgttcccatagtaacgccaatagggactttccattgacgtcaatgggtggagtatttacggtaaactgcccacttggcagtacatcaagtgtatcatatgccaagtacgccccctattgacgtcaatgacggtaaatggcccgcctggcattatgcccagtacatgaccttatgggactttcctacttggcagtacatctacgtattagtcatcgctattaccatggtcgaggtgagccccacgttctgcttcactctccccatctcccccccctccccacccccaattttgtatttatttattttttaattattttgtgcagcgatgggggcggggggggggggggggcgcgcgccaggcggggcggggcggggcgaggggcggggcggggcgaggcggagaggtgcggcggcagccaatcagagcggcgcgctccgaaagtttccttttatggcgaggcggcggcggcggcggccctataaaaagcgaagcgcgcggcgggcgggagtcgctgcgtcgcgccttcgccccgtgccccgctccgccgccgcctcgcgccgcccgccccggctctgactgaccgcgttactcccacaggtgagcgggcgggacggcccttctcctccgggctgtaattagcgcttggtttaatgacggctcgtttcttttctgtggctgcgtgaaagccttaaagggctccgggagggccctttgtgcgggggggagcggctcggggggtgcgtgcgtgtgtgtgtgcgtggggagcgccgcgtgcggcccgcgctgcccggcggctgtgagcgctgcgggcgcggcgcggggctttgtgcgctccgcgtgtgcgcgaggggagcgcggccgggggcggtgccccgcggtgcgggggggctgcgaggggaacaaaggctgcgtgcggggtgtgtgcgtgggggggtgagcagggggtgtgggcgcggcggtcgggctgtaacccccccctgcacccccctccccgagttgctgagcacggcccggcttcgggtgcggggctccgtgcggggcgtggcgcggggctcgccgtgccgggcggggggtggcggcaggtgggggtgccgggcggggcggggccgcctcgggccggggagggctcgggggaggggcgcggcggccccggagcgccggcggctgtcgaggcgcggcgagccgcagccattgccttttatggtaatcgtgcgagagggcgcagggacttcctttgtcccaaatctggcggagccgaaatctgggaggcgccgccgcaccccctctagcgggcgcgggcgaagcggtgcggcgccggcaggaaggaaatgggcggggagggccttcgtgcgtcgccgcgccgccgtccccttctccatctccagcctcggggctgccgcagggggacggctgccttcgggggggacggggcagggcggggttcggcttctggcgtgtgaccggcggctctagagcctctgctaaccatgttcatgccttcttctttttcctacagatccttaattaataatacgactcactataggggccgccaccatgggcgctagagcctctgttctgtctggcggcgaactggacagatgggagaagatcagaagcagacctggcggcaagaagaagtacaagctgaagcacatcgtgtgggccagcagagagctggaaagattcgctgtgaaccccggcctgctggaaacaagcgagggctgtagacagatcctgggccagctccagccatctctccagacaggatctgaggaactgagaagcctgtacaacaccgtggccacactgtactgcgtgcaccagagaatcgagatcaaggacaccaaagaggccctggacaagatcgaggaagaacagaacaagtctaagaagaaggcccagcaggctgccgccgatacaggccactctaatcaggtgtcccagaactaccccatcgtgcagaacatccagggccagatggtgcatcaggctatcagccccagaacactgaacgcctgggtcaaagtggtggaagagaaggctttcagccctgaagtgatccccatgttcagcgccctgtctgagggtgccacacctcaggacctgaacaccatgctgaacacagtcggcggacaccaggccgctatgcagatgctgaaagagacaatcaacgaagaggccgccgagtgggacagagtgcatcctgttcatgctggccctatcgctcccggccagatgagagaacctagaggctctgacattgccggcaccaccagcacactgcaagagcagatcggctggatgacaaacaaccctcctattcctgtgggcgagatctacaagagatggatcatcctgggactgaacaagatcgtgcggatgtacagccccaccagcatcctggacattagacagggccccaaagagcccttcagagactacgtggacagattctacaagaccctgagagccgagcaggccagccaagaagtgaagaactggatgaccgagacactgctggtgcagaacgctaaccccgactgcaagaccatcctgaaggctctgggacctgccgccacactggaagagatgatgacagcctgtcaaggcgtcggaggacctggccataaggctagagttctggccgaggccatgagccaagtgaccaacagcgccacaatcatgatgcagagaggcaacttcagaaaccagcggaagatcgtgaagtccttcaactccggcaaagagggccacaccgcccgcaattctagagcccctagaaagaaaggtggatccggcggcgtttctggatggcggctgttcaagaagatcagcggcggttccggacctgctgccaaaagagtgaaactggactccggactgcaactgcctccactggaaagactgacactgggagctgccccagccgccaagaagaaaaagctggactacaaggacgacgacgacaagggcggagctagctctaagacaatcgtgctgtctgtgggcgaagccaccagaacactgaccgagatccagagcacagccgacagacagatcttcgaggaaaaagtgggccctctcgtgggcagactgagactgacagcttccctgagacagaacggcgccaagaccgcctacagagtgaacctgaagctggaccaggccgacgtggtggattctggccttcctaaagtgcggtacacccaagtgtggtcccacgacgtgaccatcgtggccaattctaccgaggccagcagaaagagcctgtacgacctgaccaagagcctggtggccacaagccaggtggaagatctggtcgtgaatctcgtgcccctgggcagaggcggctctggcggatctaaaaccattgtgctgagcgtcggcgaggccacaaggaccctgacagagattcagtccaccgccgaccggcagatttttgaagagaaagtggggccactcgtcggaaggcttaggctgactgcaagcctgaggcagaatggggccaaaacagcttaccgggtcaacctgaaactcgatcaggctgatgtggtcgacagcggcctgccaaaagtccgctacacacaagtttggagccatgatgtgacaatcgtcgccaacagcaccgaggcctctaggaagtccctgtacgatctcacaaagtctctggtggcaacctctcaggtcgaggatctggtggtcaatctcgtgcctctcggacgtggcggatccggtggaaccgagagacaggccaacttcctgggcaagatctggcctagctacaagggcagacccggcaacttcctccagagcagaccagagcctaccgctcctcctgaggaatccttcagatccggcgtggaaaccaccacacctccacagaagcaagagcccatcgacaaagagctgtaccctctgaccagcctgagatccctgttcggcaacgaccctagctctcaatgaacgcgtaaatgattgcagatccactagttctagagctcgctgatcagcctcgactgtgccttctagttgccagccatctgttgtttgcccctcccccgtgccttccttgaccctggaaggtgccactcccactgtcctttcctaataaaatgaggaaattgcatcgcattgtctgagtaggtgtcattctattctggggggtggggtggggcaggacagcaagggggaggattgggaagacaatagcaggcatgctggggatgcggtgggctctatggcttctgaggcggaaagaaccagctggggctcgagatccactagttctagcctcgaggctagagcggccgcgcatctcaattagtcagcaaccatagtcccgcccctaactccgcccatcccgcccctaactccgcccagttccgcccattctccgccccatggctgactaattttttttatttatgcagaggccgaggccgcctcggcctctgagctattccagaagtagtgaggaggcttttttggaggcctaggcttttgcaaaaagctaacttgtttattgcagcttataatggttacaaataaagcaatagcatcacaaatttcacaaataaagcatttttttcactgcattctagttgtggtttgtccaaactcatcaatgtatcttatcatgtctggatccgctgcattaatgaatcggccaacgcgcggggagaggcggtttgcgtattgggcgctcttccgcttcctcgctcactgactcgctgcgctcggtcgttcggctgcggcgagcggtatcagctcactcaaaggcggtaatacggttatccacagaatcaggggataacgcaggaaagaacatgtgagcaaaaggccagcaaaaggccaggaaccgtaaaaaggccgcgttgctggcgtttttccataggctccgcccccctgacgagcatcacaaaaatcgacgctcaagtcagaggtggcgaaacccgacaggactataaagataccaggcgtttccccctggaagctccctcgtgcgctctcctgttccgaccctgccgcttaccggatacctgtccgcctttctcccttcgggaagcgtggcgctttctcatagctcacgctgtaggtatctcagttcggtgtaggtcgttcgctccaagctgggctgtgtgcacgaaccccccgttcagcccgaccgctgcgccttatccggtaactatcgtcttgagtccaacccggtaagacacgacttatcgccactggcagcagccactggtaacaggattagcagagcgaggtatgtaggcggtgctacagagttcttgaagtggtggcctaactacggctacactagaagaacagtatttggtatctgcgctctgctgaagccagttaccttcggaaaaagagttggtagctcttgatccggcaaacaaaccaccgctggtagcggtggtttttttgtttgcaagcagcagattacgcgcagaaaaaaaggatctcaagaagatcctttgatcttttctacggggtctgacgctcagtggaacgaaaactcacgttaagggattttggtcatgagattatcaaaaaggatcttcacctagatccttttaaattaaaaatgaagttttaaatcaatctaaagtatatatgagtaaacttggtctgacagttaccaatgcttaatcagtgaggcacctatctcagcgatctgtctatttcgttcatccatagttgcctgactccccgtcgtgtagataactacgatacgggagggcttaccatctggccccagtgctgcaatgataccgcgagacccacgctcaccggctccagatttatcagcaataaaccagccagccggaagggccgagcgcagaagtggtcctgcaactttatccgcctccatccagtctattaattgttgccgggaagctagagtaagtagttcgccagttaatagtttgcgcaacgttgttgccattgctacaggcatcgtggtgtcacgctcgtcgtttggtatggcttcattcagctccggttcccaacgatcaaggcgagttacatgatcccccatgttgtgcaaaaaagcggttagctccttcggtcctccgatcgttgtcagaagtaagttggccgcagtgttatcactcatggttatggcagcactgcataattctcttactgtcatgccatccgtaagatgcttttctgtgactggtgagtactcaaccaagtcattctgagaatagtgtatgcggcgaccgagttgctcttgcccggcgtcaatacgggataataccgcgccacatagcagaactttaaaagtgctcatcattggaaaacgttcttcggggcgaaaactctcaaggatcttaccgctgttgagatccagttcgatgtaacccactcgtgcacccaactgatcttcagcatcttttactttcaccagcgtttctgggtgagcaaaaacaggaaggcaaaatgccgcaaaaaagggaataagggcgacacggaaatgttgaatactcatactcttcctttttcaatattattgaagcatttatcagggttattgtctcatgagcggatacatatttgaatgtatttagaaaaataaacaaataggggttccgcgcacatttccccgaaaagtgccacctgggtcgacattgattattgactagttattaatagtaatcaattacggggtcattagttcatagcccatatatggagttccgcgttacataacttacggtaaatggcccgcctggctgaccgcccaacgacccccgcccattgacgtcaataatgacgtatgttcccatagtaacgccaatagggactttccattgacgtcaatgggtggagtatttacggtaaactgcccacttggcagtacatcaagtgtatcatatgccaagtacgccccctattgacgtcaatgacggtaaatggcccgcctggcattatgcccagtacatgaccttatgggactttcctacttggcagtacatctacgtattagtcatcgctattaccatggtcgaggtgagccccacgttctgcttcactctccccatctcccccccctccccacccccaattttgtatttatttattttttaattattttgtgcagggcgaggcggagaggtgcggcggcagccaatcagagcggcgcgctccgaaagtttccttttatggcgaggcggcggcggcggcggccctataaaaagcgaagcgcgcggcgggcgggagtcgctgcgcgctgccttcgccccgtgccccgctccgccgccgcctcgcgccgcccgccccggctctgactgaccgcgttactcccacaggtgagcgggcgggacggcccttctcctccgggctgtaattagcgcttggtttaatgacggcttgtttcttttctgtggctgcgtgaaagccttgaggggctccgggagggccctttgtgcggggggagcggctcggggggtgcgtgcgtgtgtgtgtgcgtggggagcgccgcgtgcggctccgcgctgcccggcggctgtgagcgctgcgggcgcggcgcggggctttgtgcgctccgcagtgtgcgcgaggggagcgcggccgggggcggtgccccgcggtgcggggggggctgcgaggggaacaaaggctgcgtgcggggtgtgtgcgtgggggggtgagcagggggtgtgggcgcgtcggtcgggctgcaaccccccctgcacccccctccccgagttgctgagcacggcccggcttcgggtgcggggctccgtacggggcgtggcgcggggctcgccgtgccgggcggggggtggcggcaggtgggggtgccgggcggggcggggccgcctcgggccggggagggctcgggggaggggcgcggcggcccccggagcgccggcggctgtcgaggcgcggcgagccgcagccattgccttttatggtaatcgtgcgagagggcgcagggacttcctttgtcccaaatctgtgcggagccgaaatctgggaggcgccgccgcaccccctctagcgggcgcggggcgaagcggtgcggcgccggcaggaaggaaatgggcggggagggccttcgtgcgtcgccgcgccgccgtccccttctccctctccagcctcggggctgtccgcggggggacggctgccttcgggggggacggggcagggcggggttcggcttctggcgtgtgaccggcggctctagagcctctgctaaccatgttcatgccttcttctttttcctacagctcctgggcaacgtgctggttattgtgctgtctcatcattttggcaaagaattcgggccgcgttgacgcgcacggcaagaggcgaggggcggcgactggtgagagatgggtgcgagagcgtcagtattaagcgggggagaattagatcgatgggaaaaaattcggttaaggccagggggaaagaaaaaatataaattaaaacatatagtatgggcaagcagggagctagaacgattcgcagttaatcctggcctgttagaaacatcagaaggctgtagacaaatactgggacagctacaaccatcccttcagacaggatcagaagaacttagatcattatataatacagtagcaaccctctattgtgtgcatcaaaggatagagataaaagacaccaaggaagctttagacaagatagaggaagagcaaaacaaaagtaagaaaaaagcacagcaagcagcagctgacacaggacacagcaatcaggtcagccaaaattaccctatagtgcagaacatccaggggcaaatggtacatcaggccatatcacctagaactttaaatgcatgggtaaaagtagtagaagagaaggctttcagcccagaagtgatacccatgttttcagcattatcagaaggagccaccccacaagatttaaacaccatgctaaacacagtggggggacatcaagcagccatgcaaatgttaaaagagaccatcaatgaggaagctgcagaatgggatagagtgcatccagtgcatgcagggcctattgcaccaggccagatgagagaaccaaggggaagtgacatagcaggaactactagtacccttcaggaacaaataggatggatgacacataatccacctatcccagtaggagaaatctataaaagatggataatcctgggattaaataaaatagtaagaatgtatagccctaccagcattctggacataagacaaggaccaaaggaaccctttagagactatgtagaccgattctataaaactctaagagccgagcaagcttcacaagaggtaaaaaattggatgacaga

SEQ ID NO: 312 - DNA, 15160 bp, Synthetic construct
  source 1..15160: mol_type = other DNA
aaccttgttggtccaaaatgcgaacccagattgtaagactattttaaaagcattgggaccaggagcgacactagaagaaatgatgacagcatgtcagggagtggggggacccggccataaagcaagagttttggctgaagcaatgagccaagtaacaaatccagctaccataatgatacagaaaggcaattttaggaaccaaagaaagactgttaagtgtttcaattgtggcaaagaagggcacatagccaaaaattgcagggcccctaggaaaaagggctgttggaaatgtggaaaggaaggacaccaaatgaaagattgtactgagagacaggctaattttttagggaagatctggccttcccacaagggaaggccagggaattttcttcagagcagaccagagccaacagccccaccagaagagagcttcaggtttggggaagagacaacaactccctctcagaagcaggagccgatagacaaggaactgtatcctttagcttccctcagatcactctttggcagcgacccctcgtcacaataaagataggggggcaattaaaggaagctctattagatacaggagcagatgatacagtattagaagaaatgaatttgccaggaagatggaaaccaaaaatgatagggggaattggaggttttatcaaagtaagacagtatgatcagatactcatagaaatctgcggacataaagctataggtacagtattagtaggacctacacctgtcaacataattggaagaaatctgttgactcagattggctgcactttaaattttcccattagtcctattgagactgtaccagtaaaattaaagccaggaatggatggcccaaaagttaaacaatggccattgacagaagaaaaaataaaagcattagtagaaatttgtacagaaatggaaaaggaaggaaaaatttcaaaaattgggcctgaaaatccatacaatactccagtatttgccataaagaaaaaagacagtactaaatggagaaaattagtagatttcagagaacttaataagagaactcaagatttctgggaagttcaattaggaataccacatcctgcagggttaaaacagaaaaaatcagtaacagtactggatgtgggcgatgcatatttttcagttcccttagataaagacttcaggaagtatactgcatttaccatacctagtataaacaatgagacaccagggattagatatcagtacaatgtgcttccacagggatggaaaggatcaccagcaatattccagtgtagcatgacaaaaatcttagagccttttagaaaacaaaatccagacatagtcatctatcaatacatggatgatttgtatgtaggatctgacttagaaatagggcagcatagaacaaaaatagaggaactgagacaacatctgttgaggtggggatttaccacaccagacaaaaaacatcagaaagaacctccattcctttggatgggttatgaactccatcctgataaatggacagtacagcctatagtgctgccagaaaaggacagctggactgtcaatgacatacagaaattagtgggaaaattgaattgggcaagtcagatttatgcagggattaaagtaaggcaattatgtaaacttcttaggggaaccaaagcactaacagaagtagtaccactaacagaagaagcagagctagaactggcagaaaacagggagattctaaaagaaccggtacatggagtgtattatgacccatcaaaagacttaatagcagaaatacagaagcaggggcaaggccaatggacatatcaaatttatcaagagccatttaaaaatctgaaaacaggaaagtatgcaagaatgaagggtgcccacactaatgatgtgaaacaattaacagaggcagtacaaaaaatagccacagaaagcatagtaatatggggaaagactcctaaatttaaattacccatacaaaaggaaacatgggaagcatggtggacagagtattggcaagccacctggattcctgagtgggagtttgtcaatacccctcccttagtgaagttatggtaccagttagagaaagaacccataataggagcagaaactttctatgtagatggggcagccaatagggaaactaaattaggaaaagcaggatatgtaactgacagaggaagacaaaaagttgtccccctaacggacacaacaaatcagaagactgagttacaagcaattcatctagctttgcaggattcgggattagaagtaaacatagtgacagactcacaatatgcattgggaatcattcaagcacaaccagataagagtgaatcagagttagtcagtcaaataatagagcagttaataaaaaaggaaaaagtctacctggcatgggtaccagcacacaaaggaattggaggaaatgaacaagtagataaattggtcagtgctggaatcaggaaagtactatttttagatggaatagataaggcccaagaagaacatgagaaatatcacagtaattggagagcaatggctagtgattttaacctaccacctgtagtagcaaaagaaatagtagccagctgtgataaatgtcagctaaaaggggaagccatgcatggacaagtagactgtagcccaggaatatggcagctagtttgtacacatttagaaggaaaagttatcttggtagcagttcatgtagccagtggatatatagaagcagaagtaattccagcagagacagggcaagaaacagcatacttcctcttaaaattagcaggaagatggccagtaaaaacagtacatacagacaatggcagcaatttcaccagtactacagttaaggccgcctgttggtgggcggggatcaagcaggaatttggcattccctacaatccccaaagtcaaggagtaatagaatctatgaataaagaattaaagaaaattataggacaggtaagagatcaggctgaacatcttaagacagcagtacaaatggcagtattcatccacaattttaaaagaaaaggggggattggggggtacagtgcaggggaaagaatagtagacataatagcaacagacatacaaactaaagaattacaaaaacaaattacaaaaattcaaaattttcgggtttattacagggacagcagagatccagtttggaaaggaccagcaaagctcctctggaaaggtgaaggggcagtagtaatacaagataatagtgacataaaagtagtgccaagaagaaaagcaaagatcatcagggattatggaaaacagatggcaggtgatgattgtgtggcaagtagacaggatgaggattaacacatggaattctgcaacaactgctgtttatccatttcagaattgggtgtcgacatagcagaataggcgttactcgacagaggagagcaagaaatggagccagtagatcctagactagagccctggaagcatccaggaagtcagcctaaaactgcttgtaccaattgctattgtaaaaagtgttgctttcattgccaagtttgtttcatgacaaaagccttaggcatctcctatggcaggaagaagcggagacagcgacgaagagctcatcagaacagtcagactcatcaagcttctctatcaaagcagtaagtagtacatgtaatgcaacctataatagtagcaatagtagcattagtagtagcaataataatagcaatagttgtgtggtccatagtaatcatagaatataggaaaatggccgctgatcttcagacctggaggaggagatatgagggacaattggagaagtgaattatataaatataaagtagtaaaaattgaaccattaggagtagcacccaccaaggcaaagagaagagtggtgcagagagaaaaaagagcagtgggaataggagctttgttccttgggttcttgggagcagcaggaagcactatgggcgcagcgtcaatgacgctgacggtacaggccagacaattattgtctggtatagtgcagcagcagaacaatttgctgagggctattgaggcgcaacagcatctgttgcaactcacagtctggggcatcaagcagctccaggcaagaatcctggctgtggaaagatacctaaaggatcaacagctcctggggatttggggttgctctggaaaactcatttgcaccactgctgtgccttggaatgctagttggagtaataaatctctggaacagatttggaatcacacgacctggatggagtgggacagagaaattaacaattacacaagcttaatacactccttaattgaagaatcgcaaaaccagcaagaaaagaatgaacaagaattattggaattagataaatgggcaagtttgtggaattggtttaacataacaaattggctgtggtatataaaattattcataatgatagtaggaggcttggtaggtttaagaatagtttttgctgtactttctatagtgaatagagttaggcagggatattcaccattatcgtttcagacccacctcccaaccccgaggggacccgacaggcccgaaggaatagaagaagaaggtggagagagagacagagacagatccattcgattagtgaacggatccttggcacttatctgggacgatctgcggagcctgtgcctcttcagctaccaccgcttgagagacttactcttgattgtaacgaggattgtggaacttctgggacgcagggggtgggaagccctcaaatattggtggaatctcctacaatattggagtcaggagctaaagaatagtgctgttagcttgctcaatgccacagccatagcagtagctgaggggacagatagggttatagaagtagtacaaggagcttgtagagctattcgccacatacctagaagaataagacagggcttggaaaggattttgctataagctcgaaacaaccggtacctctagaactatagctagcagatctttttccctctgccaaaaattatggggacatcatgaagccccttgagcatctgacttctggctaataaaggaaatttattttcattgcaatagtgtgttggaattttttgtgtctctcactcggaaggacatatgggagggcaaatcatttaaaacatcagaatgagtatttggtttagagtttggcaacatatgcccatatgctggctgccatgaacaaaggttggctataaagaggtcatcagtatatgaaacagccccctgctgtccattccttattccatagaaaagccttgacttgaggttagattttttttatattttgttttgtgttatttttttctttaacatccctaaaattttccttacatgttttactagccagatttttcctcctctcctgactactcccagtcatagctgtccctcttctcttatggagatccctcgacctgcagcccaagcttggcgtaatcatggtcatagctgtttcctgtgtgaaattgttatccgctcacaattccacacaacatacgagccggaagcataaagtgtaaagcctggggtgcctaatgagtgagctaactcacattaattgcgttgcgctcactgcccgctttccagtcgggaaacctgtcgtgccagcggatccggcgcgccggattcgacattgattattgactagttattaatagtaatcaattacggggtcattagttcatagcccatatatggagttccgcgttacataacttacggtaaatggcccgcctggctgaccgcccaacgacccccgcccattgacgtcaataatgacgtatgttcccatagtaacgccaatagggactttccattgacgtcaatgggtggagtatttacggtaaactgcccacttggcagtacatcaagtgtatcatatgccaagtacgccccctattgacgtcaatgacggtaaatggcccgcctggcattatgcccagtacatgaccttatgggactttcctacttggcagtacatctacgtattagtcatcgctattaccatggtcgaggtgagccccacgttctgcttcactctccccatctcccccccctccccacccccaattttgtatttatttattttttaattattttgtgcagcgatgggggcggggggggggggggggcgcgcgccaggcggggcggggcggggcgaggggcggggcggggcgaggcggagaggtgcggcggcagccaatcagagcggcgcgctccgaaagtttccttttatggcgaggcggcggcggcggcggccctataaaaagcgaagcgcgcggcgggcgggagtcgctgcgtcgcgccttcgccccgtgccccgctccgccgccgcctcgcgccgcccgccccggctctgactgaccgcgttactcccacaggtgagcgggcgggacggcccttctcctccgggctgtaattagcgcttggtttaatgacggctcgtttcttttctgtggctgcgtgaaagccttaaagggctccgggagggccctttgtgcgggggggagcggctcggggggtgcgtgcgtgtgtgtgtgcgtggggagcgccgcgtgcggcccgcgctgcccggcggctgtgagcgctgcgggcgcggcgcggggctttgtgcgctccgcgtgtgcgcgaggggagcgcggccgggggcggtgccccgcggtgcgggggggctgcgaggggaacaaaggctgcgtgcggggtgtgtgcgtgggggggtgagcagggggtgtgggcgcggcggtcgggctgtaacccccccctgcacccccctccccgagttgctgagcacggcccggcttcgggtgcggggctccgtgcggggcgtggcgcggggctcgccgtgccgggcggggggtggcggcaggtgggggtgccgggcggggcggggccgcctcgggccggggagggctcgggggaggggcgcggcggccccggagcgccggcggctgtcgaggcgcggcgagccgcagccattgccttttatggtaatcgtgcgagagggcgcagggacttcctttgtcccaaatctggcggagccgaaatctgggaggcgccgccgcaccccctctagcgggcgcgggcgaagcggtgcggcgccggcaggaaggaaatgggcggggagggccttcgtgcgtcgccgcgccgccgtccccttctccatctccagcctcggggctgccgcagggggacggctgccttcgggggggacggggcagggcggggttcggcttctggcgtgtgaccggcggctctagagcctctgctaaccatgttcatgccttcttctttttcctacagatccttaattaataatacgactcactataggggccgccaccatgggcgctagagcctctgttctgtctggcggcgaactggacagatgggagaagatcagaagcagacctggcggcaagaagaagtacaagctgaagcacatcgtgtgggccagcagagagctggaaagattcgctgtgaaccccggcctgctggaaacaagcgagggctgtagacagatcctgggccagctccagccatctctccagacaggatctgaggaactgagaagcctgtacaacaccgtggccacactgtactgcgtgcaccagagaatcgagatcaaggacaccaaagaggccctggacaagatcgaggaagaacagaacaagtctaagaagaaggcccagcaggctgccgccgatacaggccactctaatcaggtgtcccagaactaccccatcgtgcagaacatccagggccagatggtgcatcaggctatcagccccagaacactgaacgcctgggtcaaagtggtggaagagaaggctttcagccctgaagtgatccccatgttcagcgccctgtctgagggtgccacacctcaggacctgaacaccatgctgaacacagtcggcggacaccaggccgctatgcagatgctgaaagagacaatcaacgaagaggccgccgagtgggacagagtgcatcctgttcatgctggccctatcgctcccggccagatgagagaacctagaggctctgacattgccggcaccaccagcacactgcaagagcagatcggctggatgacaaacaaccctcctattcctgtgggcgagatctacaagagatggatcatcctgggactgaacaagatcgtgcggatgtacagccccaccagcatcctggacattagacagggccccaaagagcccttcagagactacgtggacagattctacaagaccctgagagccgagcaggccagccaagaagtgaagaactggatgaccgagacactgctggtgcagaacgctaaccccgactgcaagaccatcctgaaggctctgggacctgccgccacactggaagagatgatgacagcctgtcaaggcgtcggaggacctggccataaggctagagttctggccgaggccatgagccaagtgaccaacagcgccacaatcatgatgcagagaggcaacttcagaaaccagcggaagatcgtgaagtccttcaactccggcaaagagggccacaccgcccgcaattctagagcccctagaaagaaaggtggatccggcggcgtttctggatggcggctgttcaagaagatcagcggcggttccggacctgctgccaaaagagtgaaactggactccggactgcaactgcctccactggaaagactgacactgggagctgccccagccgccaagaagaaaaagctggactacaaggacgacgacgacaagggcggagctagccccgggggcggatccggtggaaccgagagacaggccaacttcctgggcaagatctggcctagctacaagggcagacccggcaacttcctccagagcagaccagagcctaccgctcctcctgaggaatccttcagatccggcgtggaaaccaccacacctccacagaagcaagagcccatcgacaaagagctgtaccctctgaccagcctgagatccctgttcggcaacgaccctagctctcaaggcggaggcggctctggtggcggaggatctaagacaatcgtgctgtctgtgggcgaagccaccagaacactgaccgagatccagagcacagccgacagacagatcttcgaggaaaaagtgggccctctcgtgggcagactgagactgacagcttccctgagacagaacggcgccaagaccgcctacagagtgaacctgaagctggaccaggccgacgtggtggattctggccttcctaaagtgcggtacacccaagtgtggtcccacgacgtgaccatcgtggccaattctaccgaggccagcagaaagagcctgtacgacctgaccaagagcctggtggccacaagccaggtggaagatctggtcgtgaacctggtgcctctcggacgtggcggctctggcggatctaaaaccattgtgctgagcgtcggcgaggccacaaggaccctgacagagattcagtccaccgccgaccggcagatttttgaagagaaagtggggccactcgtcggaaggcttaggctgactgcaagcctgaggcagaatggggccaaaacagcttaccgggtcaacctgaaactcgatcaggctgatgtggtcgacagcggcctgccaaaagtccgctacacacaagtttggagccatgatgtgacaatcgtcgccaacagcaccgaggcctctaggaagtccctgtacgatctcacaaagtctctggtggcaacctctcaggtcgaggatctggtggtcaatctcgtgcccctgggcagataaacgcgtaaatgattgcagatccactagttctagagctcgctgatcagcctcgactgtgccttctagttgccagccatctgttgtttgcccctcccccgtgccttccttgaccctggaaggtgccactcccactgtcctttcctaataaaatgaggaaattgcatcgcattgtctgagtaggtgtcattctattctggggggtggggtggggcaggacagcaagggggaggattgggaagacaatagcaggcatgctggggatgcggtgggctctatggcttctgaggcggaaagaaccagctggggctcgagatccactagttctagcctcgaggctagagcggccgcgcatctcaattagtcagcaaccatagtcccgcccctaactccgcccatcccgcccctaactccgcccagttccgcccattctccgccccatggctgactaattttttttatttatgcagaggccgaggccgcctcggcctctgagctattccagaagtagtgaggaggcttttttggaggcctaggcttttgcaaaaagctaacttgtttattgcagcttataatggttacaaataaagcaatagcatcacaaatttcacaaataaagcatttttttcactgcattctagttgtggtttgtccaaactcatcaatgtatcttatcatgtctggatccgctgcattaatgaatcggccaacgcgcggggagaggcggtttgcgtattgggcgctcttccgcttcctcgctcactgactcgctgcgctcggtcgttcggctgcggcgagcggtatcagctcactcaaaggcggtaatacggttatccacagaatcaggggataacgcaggaaagaacatgtgagcaaaaggccagcaaaaggccaggaaccgtaaaaaggccgcgttgctggcgtttttccataggctccgcccccctgacgagcatcacaaaaatcgacgctcaagtcagaggtggcgaaacccgacaggactataaagataccaggcgtttccccctggaagctccctcgtgcgctctcctgttccgaccctgccgcttaccggatacctgtccgcctttctcccttcgggaagcgtggcgctttctcatagctcacgctgtaggtatctcagttcggtgtaggtcgttcgctccaagctgggctgtgtgcacgaaccccccgttcagcccgaccgctgcgccttatccggtaactatcgtcttgagtccaacccggtaagacacgacttatcgccactggcagcagccactggtaacaggattagcagagcgaggtatgtaggcggtgctacagagttcttgaagtggtggcctaactacggctacactagaagaacagtatttggtatctgcgctctgctgaagccagttaccttcggaaaaagagttggtagctcttgatccggcaaacaaaccaccgctggtagcggtggtttttttgtttgcaagcagcagattacgcgcagaaaaaaaggatctcaagaagatcctttgatcttttctacggggtctgacgctcagtggaacgaaaactcacgttaagggattttggtcatgagattatcaaaaaggatcttcacctagatccttttaaattaaaaatgaagttttaaatcaatctaaagtatatatgagtaaacttggtctgacagttaccaatgcttaatcagtgaggcacctatctcagcgatctgtctatttcgttcatccatagttgcctgactccccgtcgtgtagataactacgatacgggagggcttaccatctggccccagtgctgcaatgataccgcgagacccacgctcaccggctccagatttatcagcaataaaccagccagccggaagggccgagcgcagaagtggtcctgcaactttatccgcctccatccagtctattaattgttgccgggaagctagagtaagtagttcgccagttaatagtttgcgcaacgttgttgccattgctacaggcatcgtggtgtcacgctcgtcgtttggtatggcttcattcagctccggttcccaacgatcaaggcgagttacatgatcccccatgttgtgcaaaaaagcggttagctccttcggtcctccgatcgttgtcagaagtaagttggccgcagtgttatcactcatggttatggcagcactgcataattctcttactgtcatgccatccgtaagatgcttttctgtgactggtgagtactcaaccaagtcattctgagaatagtgtatgcggcgaccgagttgctcttgcccggcgtcaatacgggataataccgcgccacatagcagaactttaaaagtgctcatcattggaaaacgttcttcggggcgaaaactctcaaggatcttaccgctgttgagatccagttcgatgtaacccactcgtgcacccaactgatcttcagcatcttttactttcaccagcgtttctgggtgagcaaaaacaggaaggcaaaatgccgcaaaaaagggaataagggcgacacggaaatgttgaatactcatactcttcctttttcaatattattgaagcatttatcagggttattgtctcatgagcggatacatatttgaatgtatttagaaaaataaacaaataggggttccgcgcacatttccccgaaaagtgccacctgggtcgacattgattattgactagttattaatagtaatcaattacggggtcattagttcatagcccatatatggagttccgcgttacataacttacggtaaatggcccgcctggctgaccgcccaacgacccccgcccattgacgtcaataatgacgtatgttcccatagtaacgccaatagggactttccattgacgtcaatgggtggagtatttacggtaaactgcccacttggcagtacatcaagtgtatcatatgccaagtacgccccctattgacgtcaatgacggtaaatggcccgcctggcattatgcccagtacatgaccttatgggactttcctacttggcagtacatctacgtattagtcatcgctattaccatggtcgaggtgagccccacgttctgcttcactctccccatctcccccccctccccacccccaattttgtatttatttattttttaattattttgtgcagggcgaggcggagaggtgcggcggcagccaatcagagcggcgcgctccgaaagtttccttttatggcgaggcggcggcggcggcggccctataaaaagcgaagcgcgcggcgggcgggagtcgctgcgcgctgccttcgccccgtgccccgctccgccgccgcctcgcgccgcccgccccggctctgactgaccgcgttactcccacaggtgagcgggcgggacggcccttctcctccgggctgtaattagcgcttggtttaatgacggcttgtttcttttctgtggctgcgtgaaagccttgaggggctccgggagggccctttgtgcggggggagcggctcggggggtgcgtgcgtgtgtgtgtgcgtggggagcgccgcgtgcggctccgcgctgcccggcggctgtgagcgctgcgggcgcggcgcggggctttgtgcgctccgcagtgtgcgcgaggggagcgcggccgggggcggtgccccgcggtgcggggggggctgcgaggggaacaaaggctgcgtgcggggtgtgtgcgtgggggggtgagcagggggtgtgggcgcgtcggtcgggctgcaaccccccctgcacccccctccccgagttgctgagcacggcccggcttcgggtgcggggctccgtacggggcgtggcgcggggctcgccgtgccgggcggggggtggcggcaggtgggggtgccgggcggggcggggccgcctcgggccggggagggctcgggggaggggcgcggcggcccccggagcgccggcggctgtcgaggcgcggcgagccgcagccattgccttttatggtaatcgtgcgagagggcgcagggacttcctttgtcccaaatctgtgcggagccgaaatctgggaggcgccgccgcaccccctctagcgggcgcggggcgaagcggtgcggcgccggcaggaaggaaatgggcggggagggccttcgtgcgtcgccgcgccgccgtccccttctccctctccagcctcggggctgtccgcggggggacggctgccttcgggggggacggggcagggcggggttcggcttctggcgtgtgaccggcggctctagagcctctgctaaccatgttcatgccttcttctttttcctacagctcctgggcaacgtgctggttattgtgctgtctcatcattttggcaaagaattcgggccgcgttgacgcgcacggcaagaggcgaggggcggcgactggtgagagatgggtgcgagagcgtcagtattaagcgggggagaattagatcgatgggaaaaaattcggttaaggccagggggaaagaaaaaatataaattaaaacatatagtatgggcaagcagggagctagaacgattcgcagttaatcctggcctgttagaaacatcagaaggctgtagacaaatactgggacagctacaaccatcccttcagacaggatcagaagaacttagatcattatataatacagtagcaaccctctattgtgtgcatcaaaggatagagataaaagacaccaaggaagctttagacaagatagaggaagagcaaaacaaaagtaagaaaaaagcacagcaagcagcagctgacacaggacacagcaatcaggtcagccaaaattaccctatagtgcagaacatccaggggcaaatggtacatcaggccatatcacctagaactttaaatgcatgggtaaaagtagtagaagagaaggctttcagcccagaagtgatacccatgttttcagcattatcagaaggagccaccccacaagatttaaacaccatgctaaacacagtggggggacatcaagcagccatgcaaatgttaaaagagaccatcaatgaggaagctgcagaatgggatagagtgcatccagtgcatgcagggcctattgcaccaggccagatgagagaaccaaggggaagtgacatagcaggaactactagtacccttcaggaacaaataggatggatgacacataatccacctatcccagtaggagaaatctataaaagatggataatcctgggattaaataaaatagtaagaatgtatagccctaccagcattctggacataagacaaggaccaaaggaaccctttagagactatgtagaccgattctataaaactctaagagccgagcaagcttcacaagaggtaaaaaattggatgacaga

SEQ ID NO: 313 - DNA, 14782 bp, Synthetic construct
  source 1..14782: mol_type = other DNA
aaccttgttggtccaaaatgcgaacccagattgtaagactattttaaaagcattgggaccaggagcgacactagaagaaatgatgacagcatgtcagggagtggggggacccggccataaagcaagagttttggctgaagcaatgagccaagtaacaaatccagctaccataatgatacagaaaggcaattttaggaaccaaagaaagactgttaagtgtttcaattgtggcaaagaagggcacatagccaaaaattgcagggcccctaggaaaaagggctgttggaaatgtggaaaggaaggacaccaaatgaaagattgtactgagagacaggctaattttttagggaagatctggccttcccacaagggaaggccagggaattttcttcagagcagaccagagccaacagccccaccagaagagagcttcaggtttggggaagagacaacaactccctctcagaagcaggagccgatagacaaggaactgtatcctttagcttccctcagatcactctttggcagcgacccctcgtcacaataaagataggggggcaattaaaggaagctctattagatacaggagcagatgatacagtattagaagaaatgaatttgccaggaagatggaaaccaaaaatgatagggggaattggaggttttatcaaagtaagacagtatgatcagatactcatagaaatctgcggacataaagctataggtacagtattagtaggacctacacctgtcaacataattggaagaaatctgttgactcagattggctgcactttaaattttcccattagtcctattgagactgtaccagtaaaattaaagccaggaatggatggcccaaaagttaaacaatggccattgacagaagaaaaaataaaagcattagtagaaatttgtacagaaatggaaaaggaaggaaaaatttcaaaaattgggcctgaaaatccatacaatactccagtatttgccataaagaaaaaagacagtactaaatggagaaaattagtagatttcagagaacttaataagagaactcaagatttctgggaagttcaattaggaataccacatcctgcagggttaaaacagaaaaaatcagtaacagtactggatgtgggcgatgcatatttttcagttcccttagataaagacttcaggaagtatactgcatttaccatacctagtataaacaatgagacaccagggattagatatcagtacaatgtgcttccacagggatggaaaggatcaccagcaatattccagtgtagcatgacaaaaatcttagagccttttagaaaacaaaatccagacatagtcatctatcaatacatggatgatttgtatgtaggatctgacttagaaatagggcagcatagaacaaaaatagaggaactgagacaacatctgttgaggtggggatttaccacaccagacaaaaaacatcagaaagaacctccattcctttggatgggttatgaactccatcctgataaatggacagtacagcctatagtgctgccagaaaaggacagctggactgtcaatgacatacagaaattagtgggaaaattgaattgggcaagtcagatttatgcagggattaaagtaaggcaattatgtaaacttcttaggggaaccaaagcactaacagaagtagtaccactaacagaagaagcagagctagaactggcagaaaacagggagattctaaaagaaccggtacatggagtgtattatgacccatcaaaagacttaatagcagaaatacagaagcaggggcaaggccaatggacatatcaaatttatcaagagccatttaaaaatctgaaaacaggaaagtatgcaagaatgaagggtgcccacactaatgatgtgaaacaattaacagaggcagtacaaaaaatagccacagaaagcatagtaatatggggaaagactcctaaatttaaattacccatacaaaaggaaacatgggaagcatggtggacagagtattggcaagccacctggattcctgagtgggagtttgtcaatacccctcccttagtgaagttatggtaccagttagagaaagaacccataataggagcagaaactttctatgtagatggggcagccaatagggaaactaaattaggaaaagcaggatatgtaactgacagaggaagacaaaaagttgtccccctaacggacacaacaaatcagaagactgagttacaagcaattcatctagctttgcaggattcgggattagaagtaaacatagtgacagactcacaatatgcattgggaatcattcaagcacaaccagataagagtgaatcagagttagtcagtcaaataatagagcagttaataaaaaaggaaaaagtctacctggcatgggtaccagcacacaaaggaattggaggaaatgaacaagtagataaattggtcagtgctggaatcaggaaagtactatttttagatggaatagataaggcccaagaagaacatgagaaatatcacagtaattggagagcaatggctagtgattttaacctaccacctgtagtagcaaaagaaatagtagccagctgtgataaatgtcagctaaaaggggaagccatgcatggacaagtagactgtagcccaggaatatggcagctagtttgtacacatttagaaggaaaagttatcttggtagcagttcatgtagccagtggatatatagaagcagaagtaattccagcagagacagggcaagaaacagcatacttcctcttaaaattagcaggaagatggccagtaaaaacagtacatacagacaatggcagcaatttcaccagtactacagttaaggccgcctgttggtgggcggggatcaagcaggaatttggcattccctacaatccccaaagtcaaggagtaatagaatctatgaataaagaattaaagaaaattataggacaggtaagagatcaggctgaacatcttaagacagcagtacaaatggcagtattcatccacaattttaaaagaaaaggggggattggggggtacagtgcaggggaaagaatagtagacataatagcaacagacatacaaactaaagaattacaaaaacaaattacaaaaattcaaaattttcgggtttattacagggacagcagagatccagtttggaaaggaccagcaaagctcctctggaaaggtgaaggggcagtagtaatacaagataatagtgacataaaagtagtgccaagaagaaaagcaaagatcatcagggattatggaaaacagatggcaggtgatgattgtgtggcaagtagacaggatgaggattaacacatggaattctgcaacaactgctgtttatccatttcagaattgggtgtcgacatagcagaataggcgttactcgacagaggagagcaagaaatggagccagtagatcctagactagagccctggaagcatccaggaagtcagcctaaaactgcttgtaccaattgctattgtaaaaagtgttgctttcattgccaagtttgtttcatgacaaaagccttaggcatctcctatggcaggaagaagcggagacagcgacgaagagctcatcagaacagtcagactcatcaagcttctctatcaaagcagtaagtagtacatgtaatgcaacctataatagtagcaatagtagcattagtagtagcaataataatagcaatagttgtgtggtccatagtaatcatagaatataggaaaatggccgctgatcttcagacctggaggaggagatatgagggacaattggagaagtgaattatataaatataaagtagtaaaaattgaaccattaggagtagcacccaccaaggcaaagagaagagtggtgcagagagaaaaaagagcagtgggaataggagctttgttccttgggttcttgggagcagcaggaagcactatgggcgcagcgtcaatgacgctgacggtacaggccagacaattattgtctggtatagtgcagcagcagaacaatttgctgagggctattgaggcgcaacagcatctgttgcaactcacagtctggggcatcaagcagctccaggcaagaatcctggctgtggaaagatacctaaaggatcaacagctcctggggatttggggttgctctggaaaactcatttgcaccactgctgtgccttggaatgctagttggagtaataaatctctggaacagatttggaatcacacgacctggatggagtgggacagagaaattaacaattacacaagcttaatacactccttaattgaagaatcgcaaaaccagcaagaaaagaatgaacaagaattattggaattagataaatgggcaagtttgtggaattggtttaacataacaaattggctgtggtatataaaattattcataatgatagtaggaggcttggtaggtttaagaatagtttttgctgtactttctatagtgaatagagttaggcagggatattcaccattatcgtttcagacccacctcccaaccccgaggggacccgacaggcccgaaggaatagaagaagaaggtggagagagagacagagacagatccattcgattagtgaacggatccttggcacttatctgggacgatctgcggagcctgtgcctcttcagctaccaccgcttgagagacttactcttgattgtaacgaggattgtggaacttctgggacgcagggggtgggaagccctcaaatattggtggaatctcctacaatattggagtcaggagctaaagaatagtgctgttagcttgctcaatgccacagccatagcagtagctgaggggacagatagggttatagaagtagtacaaggagcttgtagagctattcgccacatacctagaagaataagacagggcttggaaaggattttgctataagctcgaaacaaccggtacctctagaactatagctagcagatctttttccctctgccaaaaattatggggacatcatgaagccccttgagcatctgacttctggctaataaaggaaatttattttcattgcaatagtgtgttggaattttttgtgtctctcactcggaaggacatatgggagggcaaatcatttaaaacatcagaatgagtatttggtttagagtttggcaacatatgcccatatgctggctgccatgaacaaaggttggctataaagaggtcatcagtatatgaaacagccccctgctgtccattccttattccatagaaaagccttgacttgaggttagattttttttatattttgttttgtgttatttttttctttaacatccctaaaattttccttacatgttttactagccagatttttcctcctctcctgactactcccagtcatagctgtccctcttctcttatggagatccctcgacctgcagcccaagcttggcgtaatcatggtcatagctgtttcctgtgtgaaattgttatccgctcacaattccacacaacatacgagccggaagcataaagtgtaaagcctggggtgcctaatgagtgagctaactcacattaattgcgttgcgctcactgcccgctttccagtcgggaaacctgtcgtgccagcggatccggcgcgccggattcgacattgattattgactagttattaatagtaatcaattacggggtcattagttcatagcccatatatggagttccgcgttacataacttacggtaaatggcccgcctggctgaccgcccaacgacccccgcccattgacgtcaataatgacgtatgttcccatagtaacgccaatagggactttccattgacgtcaatgggtggagtatttacggtaaactgcccacttggcagtacatcaagtgtatcatatgccaagtacgccccctattgacgtcaatgacggtaaatggcccgcctggcattatgcccagtacatgaccttatgggactttcctacttggcagtacatctacgtattagtcatcgctattaccatggtcgaggtgagccccacgttctgcttcactctccccatctcccccccctccccacccccaattttgtatttatttattttttaattattttgtgcagcgatgggggcggggggggggggggggcgcgcgccaggcggggcggggcggggcgaggggcggggcggggcgaggcggagaggtgcggcggcagccaatcagagcggcgcgctccgaaagtttccttttatggcgaggcggcggcggcggcggccctataaaaagcgaagcgcgcggcgggcgggagtcgctgcgtcgcgccttcgccccgtgccccgctccgccgccgcctcgcgccgcccgccccggctctgactgaccgcgttactcccacaggtgagcgggcgggacggcccttctcctccgggctgtaattagcgcttggtttaatgacggctcgtttcttttctgtggctgcgtgaaagccttaaagggctccgggagggccctttgtgcgggggggagcggctcggggggtgcgtgcgtgtgtgtgtgcgtggggagcgccgcgtgcggcccgcgctgcccggcggctgtgagcgctgcgggcgcggcgcggggctttgtgcgctccgcgtgtgcgcgaggggagcgcggccgggggcggtgccccgcggtgcgggggggctgcgaggggaacaaaggctgcgtgcggggtgtgtgcgtgggggggtgagcagggggtgtgggcgcggcggtcgggctgtaacccccccctgcacccccctccccgagttgctgagcacggcccggcttcgggtgcggggctccgtgcggggcgtggcgcggggctcgccgtgccgggcggggggtggcggcaggtgggggtgccgggcggggcggggccgcctcgggccggggagggctcgggggaggggcgcggcggccccggagcgccggcggctgtcgaggcgcggcgagccgcagccattgccttttatggtaatcgtgcgagagggcgcagggacttcctttgtcccaaatctggcggagccgaaatctgggaggcgccgccgcaccccctctagcgggcgcgggcgaagcggtgcggcgccggcaggaaggaaatgggcggggagggccttcgtgcgtcgccgcgccgccgtccccttctccatctccagcctcggggctgccgcagggggacggctgccttcgggggggacggggcagggcggggttcggcttctggcgtgtgaccggcggctctagagcctctgctaaccatgttcatgccttcttctttttcctacagatccttaattaataatacgactcactataggggccgccaccatgggcgctagagcctctgttctgtctggcggcgaactggacagatgggagaagatcagaagcagacctggcggcaagaagaagtacaagctgaagcacatcgtgtgggccagcagagagctggaaagattcgctgtgaaccccggcctgctggaaacaagcgagggctgtagacagatcctgggccagctccagccatctctccagacaggatctgaggaactgagaagcctgtacaacaccgtggccacactgtactgcgtgcaccagagaatcgagatcaaggacaccaaagaggccctggacaagatcgaggaagaacagaacaagtctaagaagaaggcccagcaggctgccgccgatacaggccactctaatcaggtgtcccagaactaccccatcgtgcagaacatccagggccagatggtgcatcaggctatcagccccagaacactgaacgcctgggtcaaagtggtggaagagaaggctttcagccctgaagtgatccccatgttcagcgccctgtctgagggtgccacacctcaggacctgaacaccatgctgaacacagtcggcggacaccaggccgctatgcagatgctgaaagagacaatcaacgaagaggccgccgagtgggacagagtgcatcctgttcatgctggccctatcgctcccggccagatgagagaacctagaggctctgacattgccggcaccaccagcacactgcaagagcagatcggctggatgacaaacaaccctcctattcctgtgggcgagatctacaagagatggatcatcctgggactgaacaagatcgtgcggatgtacagccccaccagcatcctggacattagacagggccccaaagagcccttcagagactacgtggacagattctacaagaccctgagagccgagcaggccagccaagaagtgaagaactggatgaccgagacactgctggtgcagaacgctaaccccgactgcaagaccatcctgaaggctctgggacctgccgccacactggaagagatgatgacagcctgtcaaggcgtcggaggacctggccataaggctagagttctggccgaggccatgagccaagtgaccaacagcgccacaatcatgatgcagagaggcaacttcagaaaccagcggaagatcgtgaagtccttcaactccggcaaagagggccacaccgcccgcaattctagagcccctagaaagaaaggtggatccggcggcgtttctggatggcggctgttcaagaagatcagcggcggttccggacctgctgccaaaagagtgaaactggactccggactgcaactgcctccactggaaagactgacactgggagctgccccagccgccaagaagaaaaagctggactacaaggacgacgacgacaagggcggagctagccccgggggcggatccggtggaaccgagagacaggccaacttcctgggcaagatctggcctagctacaagggcagacccggcaacttcctccagagcagaccagagcctaccgctcctcctgaggaatccttcagatccggcgtggaaaccaccacacctccacagaagcaagagcccatcgacaaagagctgtaccctctgaccagcctgagatccctgttcggcaacgaccctagctctcaaggcggaggcggctctggtggcggaggatctaagacaatcgtgctgtctgtgggcgaagccaccagaacactgaccgagatccagagcacagccgacagacagatcttcgaggaaaaagtgggccctctcgtgggcagactgagactgacagcttccctgagacagaacggcgccaagaccgcctacagagtgaacctgaagctggaccaggccgacgtggtggattctggccttcctaaagtgcggtacacccaagtgtggtcccacgacgtgaccatcgtggccaattctaccgaggccagcagaaagagcctgtacgacctgaccaagagcctggtggccacaagccaggtggaagatctggtcgtgaacctggtgcctctcggacgttaaacgcgtaaatgattgcagatccactagttctagagctcgctgatcagcctcgactgtgccttctagttgccagccatctgttgtttgcccctcccccgtgccttccttgaccctggaaggtgccactcccactgtcctttcctaataaaatgaggaaattgcatcgcattgtctgagtaggtgtcattctattctggggggtggggtggggcaggacagcaagggggaggattgggaagacaatagcaggcatgctggggatgcggtgggctctatggcttctgaggcggaaagaaccagctggggctcgagatccactagttctagcctcgaggctagagcggccgcgcatctcaattagtcagcaaccatagtcccgcccctaactccgcccatcccgcccctaactccgcccagttccgcccattctccgccccatggctgactaattttttttatttatgcagaggccgaggccgcctcggcctctgagctattccagaagtagtgaggaggcttttttggaggcctaggcttttgcaaaaagctaacttgtttattgcagcttataatggttacaaataaagcaatagcatcacaaatttcacaaataaagcatttttttcactgcattctagttgtggtttgtccaaactcatcaatgtatcttatcatgtctggatccgctgcattaatgaatcggccaacgcgcggggagaggcggtttgcgtattgggcgctcttccgcttcctcgctcactgactcgctgcgctcggtcgttcggctgcggcgagcggtatcagctcactcaaaggcggtaatacggttatccacagaatcaggggataacgcaggaaagaacatgtgagcaaaaggccagcaaaaggccaggaaccgtaaaaaggccgcgttgctggcgtttttccataggctccgcccccctgacgagcatcacaaaaatcgacgctcaagtcagaggtggcgaaacccgacaggactataaagataccaggcgtttccccctggaagctccctcgtgcgctctcctgttccgaccctgccgcttaccggatacctgtccgcctttctcccttcgggaagcgtggcgctttctcatagctcacgctgtaggtatctcagttcggtgtaggtcgttcgctccaagctgggctgtgtgcacgaaccccccgttcagcccgaccgctgcgccttatccggtaactatcgtcttgagtccaacccggtaagacacgacttatcgccactggcagcagccactggtaacaggattagcagagcgaggtatgtaggcggtgctacagagttcttgaagtggtggcctaactacggctacactagaagaacagtatttggtatctgcgctctgctgaagccagttaccttcggaaaaagagttggtagctcttgatccggcaaacaaaccaccgctggtagcggtggtttttttgtttgcaagcagcagattacgcgcagaaaaaaaggatctcaagaagatcctttgatcttttctacggggtctgacgctcagtggaacgaaaactcacgttaagggattttggtcatgagattatcaaaaaggatcttcacctagatccttttaaattaaaaatgaagttttaaatcaatctaaagtatatatgagtaaacttggtctgacagttaccaatgcttaatcagtgaggcacctatctcagcgatctgtctatttcgttcatccatagttgcctgactccccgtcgtgtagataactacgatacgggagggcttaccatctggccccagtgctgcaatgataccgcgagacccacgctcaccggctccagatttatcagcaataaaccagccagccggaagggccgagcgcagaagtggtcctgcaactttatccgcctccatccagtctattaattgttgccgggaagctagagtaagtagttcgccagttaatagtttgcgcaacgttgttgccattgctacaggcatcgtggtgtcacgctcgtcgtttggtatggcttcattcagctccggttcccaacgatcaaggcgagttacatgatcccccatgttgtgcaaaaaagcggttagctccttcggtcctccgatcgttgtcagaagtaagttggccgcagtgttatcactcatggttatggcagcactgcataattctcttactgtcatgccatccgtaagatgcttttctgtgactggtgagtactcaaccaagtcattctgagaatagtgtatgcggcgaccgagttgctcttgcccggcgtcaatacgggataataccgcgccacatagcagaactttaaaagtgctcatcattggaaaacgttcttcggggcgaaaactctcaaggatcttaccgctgttgagatccagttcgatgtaacccactcgtgcacccaactgatcttcagcatcttttactttcaccagcgtttctgggtgagcaaaaacaggaaggcaaaatgccgcaaaaaagggaataagggcgacacggaaatgttgaatactcatactcttcctttttcaatattattgaagcatttatcagggttattgtctcatgagcggatacatatttgaatgtatttagaaaaataaacaaataggggttccgcgcacatttccccgaaaagtgccacctgggtcgacattgattattgactagttattaatagtaatcaattacggggtcattagttcatagcccatatatggagttccgcgttacataacttacggtaaatggcccgcctggctgaccgcccaacgacccccgcccattgacgtcaataatgacgtatgttcccatagtaacgccaatagggactttccattgacgtcaatgggtggagtatttacggtaaactgcccacttggcagtacatcaagtgtatcatatgccaagtacgccccctattgacgtcaatgacggtaaatggcccgcctggcattatgcccagtacatgaccttatgggactttcctacttggcagtacatctacgtattagtcatcgctattaccatggtcgaggtgagccccacgttctgcttcactctccccatctcccccccctccccacccccaattttgtatttatttattttttaattattttgtgcagggcgaggcggagaggtgcggcggcagccaatcagagcggcgcgctccgaaagtttccttttatggcgaggcggcggcggcggcggccctataaaaagcgaagcgcgcggcgggcgggagtcgctgcgcgctgccttcgccccgtgccccgctccgccgccgcctcgcgccgcccgccccggctctgactgaccgcgttactcccacaggtgagcgggcgggacggcccttctcctccgggctgtaattagcgcttggtttaatgacggcttgtttcttttctgtggctgcgtgaaagccttgaggggctccgggagggccctttgtgcggggggagcggctcggggggtgcgtgcgtgtgtgtgtgcgtggggagcgccgcgtgcggctccgcgctgcccggcggctgtgagcgctgcgggcgcggcgcggggctttgtgcgctccgcagtgtgcgcgaggggagcgcggccgggggcggtgccccgcggtgcggggggggctgcgaggggaacaaaggctgcgtgcggggtgtgtgcgtgggggggtgagcagggggtgtgggcgcgtcggtcgggctgcaaccccccctgcacccccctccccgagttgctgagcacggcccggcttcgggtgcggggctccgtacggggcgtggcgcggggctcgccgtgccgggcggggggtggcggcaggtgggggtgccgggcggggcggggccgcctcgggccggggagggctcgggggaggggcgcggcggcccccggagcgccggcggctgtcgaggcgcggcgagccgcagccattgccttttatggtaatcgtgcgagagggcgcagggacttcctttgtcccaaatctgtgcggagccgaaatctgggaggcgccgccgcaccccctctagcgggcgcggggcgaagcggtgcggcgccggcaggaaggaaatgggcggggagggccttcgtgcgtcgccgcgccgccgtccccttctccctctccagcctcggggctgtccgcggggggacggctgccttcgggggggacggggcagggcggggttcggcttctggcgtgtgaccggcggctctagagcctctgctaaccatgttcatgccttcttctttttcctacagctcctgggcaacgtgctggttattgtgctgtctcatcattttggcaaagaattcgggccgcgttgacgcgcacggcaagaggcgaggggcggcgactggtgagagatgggtgcgagagcgtcagtattaagcgggggagaattagatcgatgggaaaaaattcggttaaggccagggggaaagaaaaaatataaattaaaacatatagtatgggcaagcagggagctagaacgattcgcagttaatcctggcctgttagaaacatcagaaggctgtagacaaatactgggacagctacaaccatcccttcagacaggatcagaagaacttagatcattatataatacagtagcaaccctctattgtgtgcatcaaaggatagagataaaagacaccaaggaagctttagacaagatagaggaagagcaaaacaaaagtaagaaaaaagcacagcaagcagcagctgacacaggacacagcaatcaggtcagccaaaattaccctatagtgcagaacatccaggggcaaatggtacatcaggccatatcacctagaactttaaatgcatgggtaaaagtagtagaagagaaggctttcagcccagaagtgatacccatgttttcagcattatcagaaggagccaccccacaagatttaaacaccatgctaaacacagtggggggacatcaagcagccatgcaaatgttaaaagagaccatcaatgaggaagctgcagaatgggatagagtgcatccagtgcatgcagggcctattgcaccaggccagatgagagaaccaaggggaagtgacatagcaggaactactagtacccttcaggaacaaataggatggatgacacataatccacctatcccagtaggagaaatctataaaagatggataatcctgggattaaataaaatagtaagaatgtatagccctaccagcattctggacataagacaaggaccaaaggaaccctttagagactatgtagaccgattctataaaactctaagagccgagcaagcttcacaagaggtaaaaaattggatgacaga

SEQ ID NO: 314 - DNA, 14968 bp, Synthetic construct
  source 1..14968: mol_type = other DNA
aaccttgttggtccaaaatgcgaacccagattgtaagactattttaaaagcattgggaccaggagcgacactagaagaaatgatgacagcatgtcagggagtggggggacccggccataaagcaagagttttggctgaagcaatgagccaagtaacaaatccagctaccataatgatacagaaaggcaattttaggaaccaaagaaagactgttaagtgtttcaattgtggcaaagaagggcacatagccaaaaattgcagggcccctaggaaaaagggctgttggaaatgtggaaaggaaggacaccaaatgaaagattgtactgagagacaggctaattttttagggaagatctggccttcccacaagggaaggccagggaattttcttcagagcagaccagagccaacagccccaccagaagagagcttcaggtttggggaagagacaacaactccctctcagaagcaggagccgatagacaaggaactgtatcctttagcttccctcagatcactctttggcagcgacccctcgtcacaataaagataggggggcaattaaaggaagctctattagatacaggagcagatgatacagtattagaagaaatgaatttgccaggaagatggaaaccaaaaatgatagggggaattggaggttttatcaaagtaagacagtatgatcagatactcatagaaatctgcggacataaagctataggtacagtattagtaggacctacacctgtcaacataattggaagaaatctgttgactcagattggctgcactttaaattttcccattagtcctattgagactgtaccagtaaaattaaagccaggaatggatggcccaaaagttaaacaatggccattgacagaagaaaaaataaaagcattagtagaaatttgtacagaaatggaaaaggaaggaaaaatttcaaaaattgggcctgaaaatccatacaatactccagtatttgccataaagaaaaaagacagtactaaatggagaaaattagtagatttcagagaacttaataagagaactcaagatttctgggaagttcaattaggaataccacatcctgcagggttaaaacagaaaaaatcagtaacagtactggatgtgggcgatgcatatttttcagttcccttagataaagacttcaggaagtatactgcatttaccatacctagtataaacaatgagacaccagggattagatatcagtacaatgtgcttccacagggatggaaaggatcaccagcaatattccagtgtagcatgacaaaaatcttagagccttttagaaaacaaaatccagacatagtcatctatcaatacatggatgatttgtatgtaggatctgacttagaaatagggcagcatagaacaaaaatagaggaactgagacaacatctgttgaggtggggatttaccacaccagacaaaaaacatcagaaagaacctccattcctttggatgggttatgaactccatcctgataaatggacagtacagcctatagtgctgccagaaaaggacagctggactgtcaatgacatacagaaattagtgggaaaattgaattgggcaagtcagatttatgcagggattaaagtaaggcaattatgtaaacttcttaggggaaccaaagcactaacagaagtagtaccactaacagaagaagcagagctagaactggcagaaaacagggagattctaaaagaaccggtacatggagtgtattatgacccatcaaaagacttaatagcagaaatacagaagcaggggcaaggccaatggacatatcaaatttatcaagagccatttaaaaatctgaaaacaggaaagtatgcaagaatgaagggtgcccacactaatgatgtgaaacaattaacagaggcagtacaaaaaatagccacagaaagcatagtaatatggggaaagactcctaaatttaaattacccatacaaaaggaaacatgggaagcatggtggacagagtattggcaagccacctggattcctgagtgggagtttgtcaatacccctcccttagtgaagttatggtaccagttagagaaagaacccataataggagcagaaactttctatgtagatggggcagccaatagggaaactaaattaggaaaagcaggatatgtaactgacagaggaagacaaaaagttgtccccctaacggacacaacaaatcagaagactgagttacaagcaattcatctagctttgcaggattcgggattagaagtaaacatagtgacagactcacaatatgcattgggaatcattcaagcacaaccagataagagtgaatcagagttagtcagtcaaataatagagcagttaataaaaaaggaaaaagtctacctggcatgggtaccagcacacaaaggaattggaggaaatgaacaagtagataaattggtcagtgctggaatcaggaaagtactatttttagatggaatagataaggcccaagaagaacatgagaaatatcacagtaattggagagcaatggctagtgattttaacctaccacctgtagtagcaaaagaaatagtagccagctgtgataaatgtcagctaaaaggggaagccatgcatggacaagtagactgtagcccaggaatatggcagctagtttgtacacatttagaaggaaaagttatcttggtagcagttcatgtagccagtggatatatagaagcagaagtaattccagcagagacagggcaagaaacagcatacttcctcttaaaattagcaggaagatggccagtaaaaacagtacatacagacaatggcagcaatttcaccagtactacagttaaggccgcctgttggtgggcggggatcaagcaggaatttggcattccctacaatccccaaagtcaaggagtaatagaatctatgaataaagaattaaagaaaattataggacaggtaagagatcaggctgaacatcttaagacagcagtacaaatggcagtattcatccacaattttaaaagaaaaggggggattggggggtacagtgcaggggaaagaatagtagacataatagcaacagacatacaaactaaagaattacaaaaacaaattacaaaaattcaaaattttcgggtttattacagggacagcagagatccagtttggaaaggaccagcaaagctcctctggaaaggtgaaggggcagtagtaatacaagataatagtgacataaaagtagtgccaagaagaaaagcaaagatcatcagggattatggaaaacagatggcaggtgatgattgtgtggcaagtagacaggatgaggattaacacatggaattctgcaacaactgctgtttatccatttcagaattgggtgtcgacatagcagaataggcgttactcgacagaggagagcaagaaatggagccagtagatcctagactagagccctggaagcatccaggaagtcagcctaaaactgcttgtaccaattgctattgtaaaaagtgttgctttcattgccaagtttgtttcatgacaaaagccttaggcatctcctatggcaggaagaagcggagacagcgacgaagagctcatcagaacagtcagactcatcaagcttctctatcaaagcagtaagtagtacatgtaatgcaacctataatagtagcaatagtagcattagtagtagcaataataatagcaatagttgtgtggtccatagtaatcatagaatataggaaaatggccgctgatcttcagacctggaggaggagatatgagggacaattggagaagtgaattatataaatataaagtagtaaaaattgaaccattaggagtagcacccaccaaggcaaagagaagagtggtgcagagagaaaaaagagcagtgggaataggagctttgttccttgggttcttgggagcagcaggaagcactatgggcgcagcgtcaatgacgctgacggtacaggccagacaattattgtctggtatagtgcagcagcagaacaatttgctgagggctattgaggcgcaacagcatctgttgcaactcacagtctggggcatcaagcagctccaggcaagaatcctggctgtggaaagatacctaaaggatcaacagctcctggggatttggggttgctctggaaaactcatttgcaccactgctgtgccttggaatgctagttggagtaataaatctctggaacagatttggaatcacacgacctggatggagtgggacagagaaattaacaattacacaagcttaatacactccttaattgaagaatcgcaaaaccagcaagaaaagaatgaacaagaattattggaattagataaatgggcaagtttgtggaattggtttaacataacaaattggctgtggtatataaaattattcataatgatagtaggaggcttggtaggtttaagaatagtttttgctgtactttctatagtgaatagagttaggcagggatattcaccattatcgtttcagacccacctcccaaccccgaggggacccgacaggcccgaaggaatagaagaagaaggtggagagagagacagagacagatccattcgattagtgaacggatccttggcacttatctgggacgatctgcggagcctgtgcctcttcagctaccaccgcttgagagacttactcttgattgtaacgaggattgtggaacttctgggacgcagggggtgggaagccctcaaatattggtggaatctcctacaatattggagtcaggagctaaagaatagtgctgttagcttgctcaatgccacagccatagcagtagctgaggggacagatagggttatagaagtagtacaaggagcttgtagagctattcgccacatacctagaagaataagacagggcttggaaaggattttgctataagctcgaaacaaccggtacctctagaactatagctagcagatctttttccctctgccaaaaattatggggacatcatgaagccccttgagcatctgacttctggctaataaaggaaatttattttcattgcaatagtgtgttggaattttttgtgtctctcactcggaaggacatatgggagggcaaatcatttaaaacatcagaatgagtatttggtttagagtttggcaacatatgcccatatgctggctgccatgaacaaaggttggctataaagaggtcatcagtatatgaaacagccccctgctgtccattccttattccatagaaaagccttgacttgaggttagattttttttatattttgttttgtgttatttttttctttaacatccctaaaattttccttacatgttttactagccagatttttcctcctctcctgactactcccagtcatagctgtccctcttctcttatggagatccctcgacctgcagcccaagcttggcgtaatcatggtcatagctgtttcctgtgtgaaattgttatccgctcacaattccacacaacatacgagccggaagcataaagtgtaaagcctggggtgcctaatgagtgagctaactcacattaattgcgttgcgctcactgcccgctttccagtcgggaaacctgtcgtgccagcggatccggcgcgccggattcgacattgattattgactagttattaatagtaatcaattacggggtcattagttcatagcccatatatggagttccgcgttacataacttacggtaaatggcccgcctggctgaccgcccaacgacccccgcccattgacgtcaataatgacgtatgttcccatagtaacgccaatagggactttccattgacgtcaatgggtggagtatttacggtaaactgcccacttggcagtacatcaagtgtatcatatgccaagtacgccccctattgacgtcaatgacggtaaatggcccgcctggcattatgcccagtacatgaccttatgggactttcctacttggcagtacatctacgtattagtcatcgctattaccatggtcgaggtgagccccacgttctgcttcactctccccatctcccccccctccccacccccaattttgtatttatttattttttaattattttgtgcagcgatgggggcggggggggggggggggcgcgcgccaggcggggcggggcggggcgaggggcggggcggggcgaggcggagaggtgcggcggcagccaatcagagcggcgcgctccgaaagtttccttttatggcgaggcggcggcggcggcggccctataaaaagcgaagcgcgcggcgggcgggagtcgctgcgtcgcgccttcgccccgtgccccgctccgccgccgcctcgcgccgcccgccccggctctgactgaccgcgttactcccacaggtgagcgggcgggacggcccttctcctccgggctgtaattagcgcttggtttaatgacggctcgtttcttttctgtggctgcgtgaaagccttaaagggctccgggagggccctttgtgcgggggggagcggctcggggggtgcgtgcgtgtgtgtgtgcgtggggagcgccgcgtgcggcccgcgctgcccggcggctgtgagcgctgcgggcgcggcgcggggctttgtgcgctccgcgtgtgcgcgaggggagcgcggccgggggcggtgccccgcggtgcgggggggctgcgaggggaacaaaggctgcgtgcggggtgtgtgcgtgggggggtgagcagggggtgtgggcgcggcggtcgggctgtaacccccccctgcacccccctccccgagttgctgagcacggcccggcttcgggtgcggggctccgtgcggggcgtggcgcggggctcgccgtgccgggcggggggtggcggcaggtgggggtgccgggcggggcggggccgcctcgggccggggagggctcgggggaggggcgcggcggccccggagcgccggcggctgtcgaggcgcggcgagccgcagccattgccttttatggtaatcgtgcgagagggcgcagggacttcctttgtcccaaatctggcggagccgaaatctgggaggcgccgccgcaccccctctagcgggcgcgggcgaagcggtgcggcgccggcaggaaggaaatgggcggggagggccttcgtgcgtcgccgcgccgccgtccccttctccatctccagcctcggggctgccgcagggggacggctgccttcgggggggacggggcagggcggggttcggcttctggcgtgtgaccggcggctctagagcctctgctaaccatgttcatgccttcttctttttcctacagatccttaattaataatacgactcactataggggccgccaccatgggcgctagagcctctgttctgtctggcggcgaactggacagatgggagaagatcagaagcagacctggcggcaagaagaagtacaagctgaagcacatcgtgtgggccagcagagagctggaaagattcgctgtgaaccccggcctgctggaaacaagcgagggctgtagacagatcctgggccagctccagccatctctccagacaggatctgaggaactgagaagcctgtacaacaccgtggccacactgtactgcgtgcaccagagaatcgagatcaaggacaccaaagaggccctggacaagatcgaggaagaacagaacaagtctaagaagaaggcccagcaggctgccgccgatacaggccactctaatcaggtgtcccagaactaccccatcgtgcagaacatccagggccagatggtgcatcaggctatcagccccagaacactgaacgcctgggtcaaagtggtggaagagaaggctttcagccctgaagtgatccccatgttcagcgccctgtctgagggtgccacacctcaggacctgaacaccatgctgaacacagtcggcggacaccaggccgctatgcagatgctgaaagagacaatcaacgaagaggccgccgagtgggacagagtgcatcctgttcatgctggccctatcgctcccggccagatgagagaacctagaggctctgacattgccggcaccaccagcacactgcaagagcagatcggctggatgacaaacaaccctcctattcctgtgggcgagatctacaagagatggatcatcctgggactgaacaagatcgtgcggatgtacagccccaccagcatcctggacattagacagggccccaaagagcccttcagagactacgtggacagattctacaagaccctgagagccgagcaggccagccaagaagtgaagaactggatgaccgagacactgctggtgcagaacgctaaccccgactgcaagaccatcctgaaggctctgggacctgccgccacactggaagagatgatgacagcctgtcaaggcgtcggaggacctggccataaggctagagttctggccgaggccatgagccaagtgaccaacagcgccacaatcatgatgcagagaggcaacttcagaaaccagcggaagatcgtgaagtccttcaactccggcaaagagggccacaccgcccgcaattctagagcccctagaaagaaaggtggatccggcggcgtttctggatggcggctgttcaagaagatcagcggcggttccggacctgctgccaaaagagtgaaactggactccggactgcaactgcctccactggaaagactgacactgggagctgccccagccgccaagaagaaaaagctggactacaaggacgacgacgacaagggcggagctagccccgggggcggatccggtggaaccgagagacaggccaacttcctgggcaagatctggcctagctacaagggcagacccggcaacttcctccagagcagaccagagcctaccgctcctcctgaggaatccttcagatccggcgtggaaaccaccacacctccacagaagcaagagcccatcgacaaagagctgtaccctctgaccagcctgagatccctgttcggcaacgaccctagctctcaaggcggaggaggtggtatggaccactacctggacatcagactgcggcccgatcctgagtttcctccagctcagctgatgagcgtgctgttcggcaaactgcaccaggctctggttgcccaaggcggcgatagaatcggagtgtcattccccgacctggacgagagcagaagcagactgggagagagactgagaatccacgccagcgccgatgatctgagagccctgcttgctagaccttggctggaaggcctgagagatcacctccagtttggagagcctgccgtggtgcctcatccaacaccatatagacaggtgtccagagtgcaggccaagagcaaccccgaaagactgcggagaaggctgatgcggagacacgacctgtctgaggaagaggcccggaagagaatccccgacacagtggctagagccctggacctgcctttcgtgacactgagaagccagagcaccggccagcacttccggctgtttatcagacacggccctctgcaagtgaccgccgaagaaggcggctttacctgttacggcctgagcaaaggcggattcgtgccctggttttgaacgcgtaaatgattgcagatccactagttctagagctcgctgatcagcctcgactgtgccttctagttgccagccatctgttgtttgcccctcccccgtgccttccttgaccctggaaggtgccactcccactgtcctttcctaataaaatgaggaaattgcatcgcattgtctgagtaggtgtcattctattctggggggtggggtggggcaggacagcaagggggaggattgggaagacaatagcaggcatgctggggatgcggtgggctctatggcttctgaggcggaaagaaccagctggggctcgagatccactagttctagcctcgaggctagagcggccgcgcatctcaattagtcagcaaccatagtcccgcccctaactccgcccatcccgcccctaactccgcccagttccgcccattctccgccccatggctgactaattttttttatttatgcagaggccgaggccgcctcggcctctgagctattccagaagtagtgaggaggcttttttggaggcctaggcttttgcaaaaagctaacttgtttattgcagcttataatggttacaaataaagcaatagcatcacaaatttcacaaataaagcatttttttcactgcattctagttgtggtttgtccaaactcatcaatgtatcttatcatgtctggatccgctgcattaatgaatcggccaacgcgcggggagaggcggtttgcgtattgggcgctcttccgcttcctcgctcactgactcgctgcgctcggtcgttcggctgcggcgagcggtatcagctcactcaaaggcggtaatacggttatccacagaatcaggggataacgcaggaaagaacatgtgagcaaaaggccagcaaaaggccaggaaccgtaaaaaggccgcgttgctggcgtttttccataggctccgcccccctgacgagcatcacaaaaatcgacgctcaagtcagaggtggcgaaacccgacaggactataaagataccaggcgtttccccctggaagctccctcgtgcgctctcctgttccgaccctgccgcttaccggatacctgtccgcctttctcccttcgggaagcgtggcgctttctcatagctcacgctgtaggtatctcagttcggtgtaggtcgttcgctccaagctgggctgtgtgcacgaaccccccgttcagcccgaccgctgcgccttatccggtaactatcgtcttgagtccaacccggtaagacacgacttatcgccactggcagcagccactggtaacaggattagcagagcgaggtatgtaggcggtgctacagagttcttgaagtggtggcctaactacggctacactagaagaacagtatttggtatctgcgctctgctgaagccagttaccttcggaaaaagagttggtagctcttgatccggcaaacaaaccaccgctggtagcggtggtttttttgtttgcaagcagcagattacgcgcagaaaaaaaggatctcaagaagatcctttgatcttttctacggggtctgacgctcagtggaacgaaaactcacgttaagggattttggtcatgagattatcaaaaaggatcttcacctagatccttttaaattaaaaatgaagttttaaatcaatctaaagtatatatgagtaaacttggtctgacagttaccaatgcttaatcagtgaggcacctatctcagcgatctgtctatttcgttcatccatagttgcctgactccccgtcgtgtagataactacgatacgggagggcttaccatctggccccagtgctgcaatgataccgcgagacccacgctcaccggctccagatttatcagcaataaaccagccagccggaagggccgagcgcagaagtggtcctgcaactttatccgcctccatccagtctattaattgttgccgggaagctagagtaagtagttcgccagttaatagtttgcgcaacgttgttgccattgctacaggcatcgtggtgtcacgctcgtcgtttggtatggcttcattcagctccggttcccaacgatcaaggcgagttacatgatcccccatgttgtgcaaaaaagcggttagctccttcggtcctccgatcgttgtcagaagtaagttggccgcagtgttatcactcatggttatggcagcactgcataattctcttactgtcatgccatccgtaagatgcttttctgtgactggtgagtactcaaccaagtcattctgagaatagtgtatgcggcgaccgagttgctcttgcccggcgtcaatacgggataataccgcgccacatagcagaactttaaaagtgctcatcattggaaaacgttcttcggggcgaaaactctcaaggatcttaccgctgttgagatccagttcgatgtaacccactcgtgcacccaactgatcttcagcatcttttactttcaccagcgtttctgggtgagcaaaaacaggaaggcaaaatgccgcaaaaaagggaataagggcgacacggaaatgttgaatactcatactcttcctttttcaatattattgaagcatttatcagggttattgtctcatgagcggatacatatttgaatgtatttagaaaaataaacaaataggggttccgcgcacatttccccgaaaagtgccacctgggtcgacattgattattgactagttattaatagtaatcaattacggggtcattagttcatagcccatatatggagttccgcgttacataacttacggtaaatggcccgcctggctgaccgcccaacgacccccgcccattgacgtcaataatgacgtatgttcccatagtaacgccaatagggactttccattgacgtcaatgggtggagtatttacggtaaactgcccacttggcagtacatcaagtgtatcatatgccaagtacgccccctattgacgtcaatgacggtaaatggcccgcctggcattatgcccagtacatgaccttatgggactttcctacttggcagtacatctacgtattagtcatcgctattaccatggtcgaggtgagccccacgttctgcttcactctccccatctcccccccctccccacccccaattttgtatttatttattttttaattattttgtgcagggcgaggcggagaggtgcggcggcagccaatcagagcggcgcgctccgaaagtttccttttatggcgaggcggcggcggcggcggccctataaaaagcgaagcgcgcggcgggcgggagtcgctgcgcgctgccttcgccccgtgccccgctccgccgccgcctcgcgccgcccgccccggctctgactgaccgcgttactcccacaggtgagcgggcgggacggcccttctcctccgggctgtaattagcgcttggtttaatgacggcttgtttcttttctgtggctgcgtgaaagccttgaggggctccgggagggccctttgtgcggggggagcggctcggggggtgcgtgcgtgtgtgtgtgcgtggggagcgccgcgtgcggctccgcgctgcccggcggctgtgagcgctgcgggcgcggcgcggggctttgtgcgctccgcagtgtgcgcgaggggagcgcggccgggggcggtgccccgcggtgcggggggggctgcgaggggaacaaaggctgcgtgcggggtgtgtgcgtgggggggtgagcagggggtgtgggcgcgtcggtcgggctgcaaccccccctgcacccccctccccgagttgctgagcacggcccggcttcgggtgcggggctccgtacggggcgtggcgcggggctcgccgtgccgggcggggggtggcggcaggtgggggtgccgggcggggcggggccgcctcgggccggggagggctcgggggaggggcgcggcggcccccggagcgccggcggctgtcgaggcgcggcgagccgcagccattgccttttatggtaatcgtgcgagagggcgcagggacttcctttgtcccaaatctgtgcggagccgaaatctgggaggcgccgccgcaccccctctagcgggcgcggggcgaagcggtgcggcgccggcaggaaggaaatgggcggggagggccttcgtgcgtcgccgcgccgccgtccccttctccctctccagcctcggggctgtccgcggggggacggctgccttcgggggggacggggcagggcggggttcggcttctggcgtgtgaccggcggctctagagcctctgctaaccatgttcatgccttcttctttttcctacagctcctgggcaacgtgctggttattgtgctgtctcatcattttggcaaagaattcgggccgcgttgacgcgcacggcaagaggcgaggggcggcgactggtgagagatgggtgcgagagcgtcagtattaagcgggggagaattagatcgatgggaaaaaattcggttaaggccagggggaaagaaaaaatataaattaaaacatatagtatgggcaagcagggagctagaacgattcgcagttaatcctggcctgttagaaacatcagaaggctgtagacaaatactgggacagctacaaccatcccttcagacaggatcagaagaacttagatcattatataatacagtagcaaccctctattgtgtgcatcaaaggatagagataaaagacaccaaggaagctttagacaagatagaggaagagcaaaacaaaagtaagaaaaaagcacagcaagcagcagctgacacaggacacagcaatcaggtcagccaaaattaccctatagtgcagaacatccaggggcaaatggtacatcaggccatatcacctagaactttaaatgcatgggtaaaagtagtagaagagaaggctttcagcccagaagtgatacccatgttttcagcattatcagaaggagccaccccacaagatttaaacaccatgctaaacacagtggggggacatcaagcagccatgcaaatgttaaaagagaccatcaatgaggaagctgcagaatgggatagagtgcatccagtgcatgcagggcctattgcaccaggccagatgagagaaccaaggggaagtgacatagcaggaactactagtacccttcaggaacaaataggatggatgacacataatccacctatcccagtaggagaaatctataaaagatggataatcctgggattaaataaaatagtaagaatgtatagccctaccagcattctggacataagacaaggaccaaaggaaccctttagagactatgtagaccgattctataaaactctaagagccgagcaagcttcacaagaggtaaaaaattggatgacaga

SEQ ID NO: 315 - DNA, 14962 bp, Synthetic construct
  source 1..14962: mol_type = other DNA
aaccttgttggtccaaaatgcgaacccagattgtaagactattttaaaagcattgggaccaggagcgacactagaagaaatgatgacagcatgtcagggagtggggggacccggccataaagcaagagttttggctgaagcaatgagccaagtaacaaatccagctaccataatgatacagaaaggcaattttaggaaccaaagaaagactgttaagtgtttcaattgtggcaaagaagggcacatagccaaaaattgcagggcccctaggaaaaagggctgttggaaatgtggaaaggaaggacaccaaatgaaagattgtactgagagacaggctaattttttagggaagatctggccttcccacaagggaaggccagggaattttcttcagagcagaccagagccaacagccccaccagaagagagcttcaggtttggggaagagacaacaactccctctcagaagcaggagccgatagacaaggaactgtatcctttagcttccctcagatcactctttggcagcgacccctcgtcacaataaagataggggggcaattaaaggaagctctattagatacaggagcagatgatacagtattagaagaaatgaatttgccaggaagatggaaaccaaaaatgatagggggaattggaggttttatcaaagtaagacagtatgatcagatactcatagaaatctgcggacataaagctataggtacagtattagtaggacctacacctgtcaacataattggaagaaatctgttgactcagattggctgcactttaaattttcccattagtcctattgagactgtaccagtaaaattaaagccaggaatggatggcccaaaagttaaacaatggccattgacagaagaaaaaataaaagcattagtagaaatttgtacagaaatggaaaaggaaggaaaaatttcaaaaattgggcctgaaaatccatacaatactccagtatttgccataaagaaaaaagacagtactaaatggagaaaattagtagatttcagagaacttaataagagaactcaagatttctgggaagttcaattaggaataccacatcctgcagggttaaaacagaaaaaatcagtaacagtactggatgtgggcgatgcatatttttcagttcccttagataaagacttcaggaagtatactgcatttaccatacctagtataaacaatgagacaccagggattagatatcagtacaatgtgcttccacagggatggaaaggatcaccagcaatattccagtgtagcatgacaaaaatcttagagccttttagaaaacaaaatccagacatagtcatctatcaatacatggatgatttgtatgtaggatctgacttagaaatagggcagcatagaacaaaaatagaggaactgagacaacatctgttgaggtggggatttaccacaccagacaaaaaacatcagaaagaacctccattcctttggatgggttatgaactccatcctgataaatggacagtacagcctatagtgctgccagaaaaggacagctggactgtcaatgacatacagaaattagtgggaaaattgaattgggcaagtcagatttatgcagggattaaagtaaggcaattatgtaaacttcttaggggaaccaaagcactaacagaagtagtaccactaacagaagaagcagagctagaactggcagaaaacagggagattctaaaagaaccggtacatggagtgtattatgacccatcaaaagacttaatagcagaaatacagaagcaggggcaaggccaatggacatatcaaatttatcaagagccatttaaaaatctgaaaacaggaaagtatgcaagaatgaagggtgcccacactaatgatgtgaaacaattaacagaggcagtacaaaaaatagccacagaaagcatagtaatatggggaaagactcctaaatttaaattacccatacaaaaggaaacatgggaagcatggtggacagagtattggcaagccacctggattcctgagtgggagtttgtcaatacccctcccttagtgaagttatggtaccagttagagaaagaacccataataggagcagaaactttctatgtagatggggcagccaatagggaaactaaattaggaaaagcaggatatgtaactgacagaggaagacaaaaagttgtccccctaacggacacaacaaatcagaagactgagttacaagcaattcatctagctttgcaggattcgggattagaagtaaacatagtgacagactcacaatatgcattgggaatcattcaagcacaaccagataagagtgaatcagagttagtcagtcaaataatagagcagttaataaaaaaggaaaaagtctacctggcatgggtaccagcacacaaaggaattggaggaaatgaacaagtagataaattggtcagtgctggaatcaggaaagtactatttttagatggaatagataaggcccaagaagaacatgagaaatatcacagtaattggagagcaatggctagtgattttaacctaccacctgtagtagcaaaagaaatagtagccagctgtgataaatgtcagctaaaaggggaagccatgcatggacaagtagactgtagcccaggaatatggcagctagtttgtacacatttagaaggaaaagttatcttggtagcagttcatgtagccagtggatatatagaagcagaagtaattccagcagagacagggcaagaaacagcatacttcctcttaaaattagcaggaagatggccagtaaaaacagtacatacagacaatggcagcaatttcaccagtactacagttaaggccgcctgttggtgggcggggatcaagcaggaatttggcattccctacaatccccaaagtcaaggagtaatagaatctatgaataaagaattaaagaaaattataggacaggtaagagatcaggctgaacatcttaagacagcagtacaaatggcagtattcatccacaattttaaaagaaaaggggggattggggggtacagtgcaggggaaagaatagtagacataatagcaacagacatacaaactaaagaattacaaaaacaaattacaaaaattcaaaattttcgggtttattacagggacagcagagatccagtttggaaaggaccagcaaagctcctctggaaaggtgaaggggcagtagtaatacaagataatagtgacataaaagtagtgccaagaagaaaagcaaagatcatcagggattatggaaaacagatggcaggtgatgattgtgtggcaagtagacaggatgaggattaacacatggaattctgcaacaactgctgtttatccatttcagaattgggtgtcgacatagcagaataggcgttactcgacagaggagagcaagaaatggagccagtagatcctagactagagccctggaagcatccaggaagtcagcctaaaactgcttgtaccaattgctattgtaaaaagtgttgctttcattgccaagtttgtttcatgacaaaagccttaggcatctcctatggcaggaagaagcggagacagcgacgaagagctcatcagaacagtcagactcatcaagcttctctatcaaagcagtaagtagtacatgtaatgcaacctataatagtagcaatagtagcattagtagtagcaataataatagcaatagttgtgtggtccatagtaatcatagaatataggaaaatggccgctgatcttcagacctggaggaggagatatgagggacaattggagaagtgaattatataaatataaagtagtaaaaattgaaccattaggagtagcacccaccaaggcaaagagaagagtggtgcagagagaaaaaagagcagtgggaataggagctttgttccttgggttcttgggagcagcaggaagcactatgggcgcagcgtcaatgacgctgacggtacaggccagacaattattgtctggtatagtgcagcagcagaacaatttgctgagggctattgaggcgcaacagcatctgttgcaactcacagtctggggcatcaagcagctccaggcaagaatcctggctgtggaaagatacctaaaggatcaacagctcctggggatttggggttgctctggaaaactcatttgcaccactgctgtgccttggaatgctagttggagtaataaatctctggaacagatttggaatcacacgacctggatggagtgggacagagaaattaacaattacacaagcttaatacactccttaattgaagaatcgcaaaaccagcaagaaaagaatgaacaagaattattggaattagataaatgggcaagtttgtggaattggtttaacataacaaattggctgtggtatataaaattattcataatgatagtaggaggcttggtaggtttaagaatagtttttgctgtactttctatagtgaatagagttaggcagggatattcaccattatcgtttcagacccacctcccaaccccgaggggacccgacaggcccgaaggaatagaagaagaaggtggagagagagacagagacagatccattcgattagtgaacggatccttggcacttatctgggacgatctgcggagcctgtgcctcttcagctaccaccgcttgagagacttactcttgattgtaacgaggattgtggaacttctgggacgcagggggtgggaagccctcaaatattggtggaatctcctacaatattggagtcaggagctaaagaatagtgctgttagcttgctcaatgccacagccatagcagtagctgaggggacagatagggttatagaagtagtacaaggagcttgtagagctattcgccacatacctagaagaataagacagggcttggaaaggattttgctataagctcgaaacaaccggtacctctagaactatagctagcagatctttttccctctgccaaaaattatggggacatcatgaagccccttgagcatctgacttctggctaataaaggaaatttattttcattgcaatagtgtgttggaattttttgtgtctctcactcggaaggacatatgggagggcaaatcatttaaaacatcagaatgagtatttggtttagagtttggcaacatatgcccatatgctggctgccatgaacaaaggttggctataaagaggtcatcagtatatgaaacagccccctgctgtccattccttattccatagaaaagccttgacttgaggttagattttttttatattttgttttgtgttatttttttctttaacatccctaaaattttccttacatgttttactagccagatttttcctcctctcctgactactcccagtcatagctgtccctcttctcttatggagatccctcgacctgcagcccaagcttggcgtaatcatggtcatagctgtttcctgtgtgaaattgttatccgctcacaattccacacaacatacgagccggaagcataaagtgtaaagcctggggtgcctaatgagtgagctaactcacattaattgcgttgcgctcactgcccgctttccagtcgggaaacctgtcgtgccagcggatccggcgcgccggattcgacattgattattgactagttattaatagtaatcaattacggggtcattagttcatagcccatatatggagttccgcgttacataacttacggtaaatggcccgcctggctgaccgcccaacgacccccgcccattgacgtcaataatgacgtatgttcccatagtaacgccaatagggactttccattgacgtcaatgggtggagtatttacggtaaactgcccacttggcagtacatcaagtgtatcatatgccaagtacgccccctattgacgtcaatgacggtaaatggcccgcctggcattatgcccagtacatgaccttatgggactttcctacttggcagtacatctacgtattagtcatcgctattaccatggtcgaggtgagccccacgttctgcttcactctccccatctcccccccctccccacccccaattttgtatttatttattttttaattattttgtgcagcgatgggggcggggggggggggggggcgcgcgccaggcggggcggggcggggcgaggggcggggcggggcgaggcggagaggtgcggcggcagccaatcagagcggcgcgctccgaaagtttccttttatggcgaggcggcggcggcggcggccctataaaaagcgaagcgcgcggcgggcgggagtcgctgcgtcgcgccttcgccccgtgccccgctccgccgccgcctcgcgccgcccgccccggctctgactgaccgcgttactcccacaggtgagcgggcgggacggcccttctcctccgggctgtaattagcgcttggtttaatgacggctcgtttcttttctgtggctgcgtgaaagccttaaagggctccgggagggccctttgtgcgggggggagcggctcggggggtgcgtgcgtgtgtgtgtgcgtggggagcgccgcgtgcggcccgcgctgcccggcggctgtgagcgctgcgggcgcggcgcggggctttgtgcgctccgcgtgtgcgcgaggggagcgcggccgggggcggtgccccgcggtgcgggggggctgcgaggggaacaaaggctgcgtgcggggtgtgtgcgtgggggggtgagcagggggtgtgggcgcggcggtcgggctgtaacccccccctgcacccccctccccgagttgctgagcacggcccggcttcgggtgcggggctccgtgcggggcgtggcgcggggctcgccgtgccgggcggggggtggcggcaggtgggggtgccgggcggggcggggccgcctcgggccggggagggctcgggggaggggcgcggcggccccggagcgccggcggctgtcgaggcgcggcgagccgcagccattgccttttatggtaatcgtgcgagagggcgcagggacttcctttgtcccaaatctggcggagccgaaatctgggaggcgccgccgcaccccctctagcgggcgcgggcgaagcggtgcggcgccggcaggaaggaaatgggcggggagggccttcgtgcgtcgccgcgccgccgtccccttctccatctccagcctcggggctgccgcagggggacggctgccttcgggggggacggggcagggcggggttcggcttctggcgtgtgaccggcggctctagagcctctgctaaccatgttcatgccttcttctttttcctacagatccttaattaataatacgactcactataggggccgccaccatgggcgctagagcctctgttctgtctggcggcgaactggacagatgggagaagatcagaagcagacctggcggcaagaagaagtacaagctgaagcacatcgtgtgggccagcagagagctggaaagattcgctgtgaaccccggcctgctggaaacaagcgagggctgtagacagatcctgggccagctccagccatctctccagacaggatctgaggaactgagaagcctgtacaacaccgtggccacactgtactgcgtgcaccagagaatcgagatcaaggacaccaaagaggccctggacaagatcgaggaagaacagaacaagtctaagaagaaggcccagcaggctgccgccgatacaggccactctaatcaggtgtcccagaactaccccatcgtgcagaacatccagggccagatggtgcatcaggctatcagccccagaacactgaacgcctgggtcaaagtggtggaagagaaggctttcagccctgaagtgatccccatgttcagcgccctgtctgagggtgccacacctcaggacctgaacaccatgctgaacacagtcggcggacaccaggccgctatgcagatgctgaaagagacaatcaacgaagaggccgccgagtgggacagagtgcatcctgttcatgctggccctatcgctcccggccagatgagagaacctagaggctctgacattgccggcaccaccagcacactgcaagagcagatcggctggatgacaaacaaccctcctattcctgtgggcgagatctacaagagatggatcatcctgggactgaacaagatcgtgcggatgtacagccccaccagcatcctggacattagacagggccccaaagagcccttcagagactacgtggacagattctacaagaccctgagagccgagcaggccagccaagaagtgaagaactggatgaccgagacactgctggtgcagaacgctaaccccgactgcaagaccatcctgaaggctctgggacctgccgccacactggaagagatgatgacagcctgtcaaggcgtcggaggacctggccataaggctagagttctggccgaggccatgagccaagtgaccaacagcgccacaatcatgatgcagagaggcaacttcagaaaccagcggaagatcgtgaagtccttcaactccggcaaagagggccacaccgcccgcaattctagagcccctagaaagaaaggtggatccggcggcgtttctggatggcggctgttcaagaagatcagcggcggttccggacctgctgccaaaagagtgaaactggactccggactgcaactgcctccactggaaagactgacactgggagctgccccagccgccaagaagaaaaagctggactacaaggacgacgacgacaagggcggagctagccccgggggcggtggtatggaccactacctggacatcagactgcggcccgatcctgagtttcctccagctcagctgatgagcgtgctgttcggcaaactgcaccaggctctggttgcccaaggcggcgatagaatcggagtgtcattccccgacctggacgagagcagaagcagactgggagagagactgagaatccacgccagcgccgatgatctgagagccctgcttgctagaccttggctggaaggcctgagagatcacctccagtttggagagcctgccgtggtgcctcatccaacaccatatagacaggtgtccagagtgcaggccaagagcaaccccgaaagactgcggagaaggctgatgcggagacacgacctgtctgaggaagaggcccggaagagaatccccgacacagtggctagagccctggacctgcctttcgtgacactgagaagccagagcaccggccagcacttccggctgtttatcagacacggccctctgcaagtgaccgccgaagaaggcggctttacctgttacggcctgagcaaaggcggattcgtgccctggtttggcggatccggtggaaccgagagacaggccaacttcctgggcaagatctggcctagctacaagggcagacccggcaacttcctccagagcagaccagagcctaccgctcctcctgaggaatccttcagatccggcgtggaaaccaccacacctccacagaagcaagagcccatcgacaaagagctgtaccctctgaccagcctgagatccctgttcggcaacgaccctagctctcaatgaacgcgtaaatgattgcagatccactagttctagagctcgctgatcagcctcgactgtgccttctagttgccagccatctgttgtttgcccctcccccgtgccttccttgaccctggaaggtgccactcccactgtcctttcctaataaaatgaggaaattgcatcgcattgtctgagtaggtgtcattctattctggggggtggggtggggcaggacagcaagggggaggattgggaagacaatagcaggcatgctggggatgcggtgggctctatggcttctgaggcggaaagaaccagctggggctcgagatccactagttctagcctcgaggctagagcggccgcgcatctcaattagtcagcaaccatagtcccgcccctaactccgcccatcccgcccctaactccgcccagttccgcccattctccgccccatggctgactaattttttttatttatgcagaggccgaggccgcctcggcctctgagctattccagaagtagtgaggaggcttttttggaggcctaggcttttgcaaaaagctaacttgtttattgcagcttataatggttacaaataaagcaatagcatcacaaatttcacaaataaagcatttttttcactgcattctagttgtggtttgtccaaactcatcaatgtatcttatcatgtctggatccgctgcattaatgaatcggccaacgcgcggggagaggcggtttgcgtattgggcgctcttccgcttcctcgctcactgactcgctgcgctcggtcgttcggctgcggcgagcggtatcagctcactcaaaggcggtaatacggttatccacagaatcaggggataacgcaggaaagaacatgtgagcaaaaggccagcaaaaggccaggaaccgtaaaaaggccgcgttgctggcgtttttccataggctccgcccccctgacgagcatcacaaaaatcgacgctcaagtcagaggtggcgaaacccgacaggactataaagataccaggcgtttccccctggaagctccctcgtgcgctctcctgttccgaccctgccgcttaccggatacctgtccgcctttctcccttcgggaagcgtggcgctttctcatagctcacgctgtaggtatctcagttcggtgtaggtcgttcgctccaagctgggctgtgtgcacgaaccccccgttcagcccgaccgctgcgccttatccggtaactatcgtcttgagtccaacccggtaagacacgacttatcgccactggcagcagccactggtaacaggattagcagagcgaggtatgtaggcggtgctacagagttcttgaagtggtggcctaactacggctacactagaagaacagtatttggtatctgcgctctgctgaagccagttaccttcggaaaaagagttggtagctcttgatccggcaaacaaaccaccgctggtagcggtggtttttttgtttgcaagcagcagattacgcgcagaaaaaaaggatctcaagaagatcctttgatcttttctacggggtctgacgctcagtggaacgaaaactcacgttaagggattttggtcatgagattatcaaaaaggatcttcacctagatccttttaaattaaaaatgaagttttaaatcaatctaaagtatatatgagtaaacttggtctgacagttaccaatgcttaatcagtgaggcacctatctcagcgatctgtctatttcgttcatccatagttgcctgactccccgtcgtgtagataactacgatacgggagggcttaccatctggccccagtgctgcaatgataccgcgagacccacgctcaccggctccagatttatcagcaataaaccagccagccggaagggccgagcgcagaagtggtcctgcaactttatccgcctccatccagtctattaattgttgccgggaagctagagtaagtagttcgccagttaatagtttgcgcaacgttgttgccattgctacaggcatcgtggtgtcacgctcgtcgtttggtatggcttcattcagctccggttcccaacgatcaaggcgagttacatgatcccccatgttgtgcaaaaaagcggttagctccttcggtcctccgatcgttgtcagaagtaagttggccgcagtgttatcactcatggttatggcagcactgcataattctcttactgtcatgccatccgtaagatgcttttctgtgactggtgagtactcaaccaagtcattctgagaatagtgtatgcggcgaccgagttgctcttgcccggcgtcaatacgggataataccgcgccacatagcagaactttaaaagtgctcatcattggaaaacgttcttcggggcgaaaactctcaaggatcttaccgctgttgagatccagttcgatgtaacccactcgtgcacccaactgatcttcagcatcttttactttcaccagcgtttctgggtgagcaaaaacaggaaggcaaaatgccgcaaaaaagggaataagggcgacacggaaatgttgaatactcatactcttcctttttcaatattattgaagcatttatcagggttattgtctcatgagcggatacatatttgaatgtatttagaaaaataaacaaataggggttccgcgcacatttccccgaaaagtgccacctgggtcgacattgattattgactagttattaatagtaatcaattacggggtcattagttcatagcccatatatggagttccgcgttacataacttacggtaaatggcccgcctggctgaccgcccaacgacccccgcccattgacgtcaataatgacgtatgttcccatagtaacgccaatagggactttccattgacgtcaatgggtggagtatttacggtaaactgcccacttggcagtacatcaagtgtatcatatgccaagtacgccccctattgacgtcaatgacggtaaatggcccgcctggcattatgcccagtacatgaccttatgggactttcctacttggcagtacatctacgtattagtcatcgctattaccatggtcgaggtgagccccacgttctgcttcactctccccatctcccccccctccccacccccaattttgtatttatttattttttaattattttgtgcagggcgaggcggagaggtgcggcggcagccaatcagagcggcgcgctccgaaagtttccttttatggcgaggcggcggcggcggcggccctataaaaagcgaagcgcgcggcgggcgggagtcgctgcgcgctgccttcgccccgtgccccgctccgccgccgcctcgcgccgcccgccccggctctgactgaccgcgttactcccacaggtgagcgggcgggacggcccttctcctccgggctgtaattagcgcttggtttaatgacggcttgtttcttttctgtggctgcgtgaaagccttgaggggctccgggagggccctttgtgcggggggagcggctcggggggtgcgtgcgtgtgtgtgtgcgtggggagcgccgcgtgcggctccgcgctgcccggcggctgtgagcgctgcgggcgcggcgcggggctttgtgcgctccgcagtgtgcgcgaggggagcgcggccgggggcggtgccccgcggtgcggggggggctgcgaggggaacaaaggctgcgtgcggggtgtgtgcgtgggggggtgagcagggggtgtgggcgcgtcggtcgggctgcaaccccccctgcacccccctccccgagttgctgagcacggcccggcttcgggtgcggggctccgtacggggcgtggcgcggggctcgccgtgccgggcggggggtggcggcaggtgggggtgccgggcggggcggggccgcctcgggccggggagggctcgggggaggggcgcggcggcccccggagcgccggcggctgtcgaggcgcggcgagccgcagccattgccttttatggtaatcgtgcgagagggcgcagggacttcctttgtcccaaatctgtgcggagccgaaatctgggaggcgccgccgcaccccctctagcgggcgcggggcgaagcggtgcggcgccggcaggaaggaaatgggcggggagggccttcgtgcgtcgccgcgccgccgtccccttctccctctccagcctcggggctgtccgcggggggacggctgccttcgggggggacggggcagggcggggttcggcttctggcgtgtgaccggcggctctagagcctctgctaaccatgttcatgccttcttctttttcctacagctcctgggcaacgtgctggttattgtgctgtctcatcattttggcaaagaattcgggccgcgttgacgcgcacggcaagaggcgaggggcggcgactggtgagagatgggtgcgagagcgtcagtattaagcgggggagaattagatcgatgggaaaaaattcggttaaggccagggggaaagaaaaaatataaattaaaacatatagtatgggcaagcagggagctagaacgattcgcagttaatcctggcctgttagaaacatcagaaggctgtagacaaatactgggacagctacaaccatcccttcagacaggatcagaagaacttagatcattatataatacagtagcaaccctctattgtgtgcatcaaaggatagagataaaagacaccaaggaagctttagacaagatagaggaagagcaaaacaaaagtaagaaaaaagcacagcaagcagcagctgacacaggacacagcaatcaggtcagccaaaattaccctatagtgcagaacatccaggggcaaatggtacatcaggccatatcacctagaactttaaatgcatgggtaaaagtagtagaagagaaggctttcagcccagaagtgatacccatgttttcagcattatcagaaggagccaccccacaagatttaaacaccatgctaaacacagtggggggacatcaagcagccatgcaaatgttaaaagagaccatcaatgaggaagctgcagaatgggatagagtgcatccagtgcatgcagggcctattgcaccaggccagatgagagaaccaaggggaagtgacatagcaggaactactagtacccttcaggaacaaataggatggatgacacataatccacctatcccagtaggagaaatctataaaagatggataatcctgggattaaataaaatagtaagaatgtatagccctaccagcattctggacataagacaaggaccaaaggaaccctttagagactatgtagaccgattctataaaactctaagagccgagcaagcttcacaagaggtaaaaaattggatgacaga

SEQ ID NO: 316 - DNA, 10644 bp, Synthetic construct; identical to SEQ ID NO: 267
  source 1..10644: mol_type = other DNA

SEQ ID NO: 317 - DNA, 6268 bp, Synthetic construct
  source 1..6268: mol_type = other DNA
acgcgcgtgtagtcttatgcaatactcttgtagtcttgcaacatggtaacgatgagttagcaacatgccttacaaggagagaaaaagcaccgtgcatgccgattggtggaagtaaggtggtacgatcgtgccttattaggaaggcaacagacgggtctgacatggattggacgaaccactgaattgccgcattgcagagatattgtatttaagtgcctagctcgatacataaacgggtctctctggttagaccagatctgagcctgggagctctctggctaactagggaacccactgcttaagcctcaataaagcttgccttgagtgcttcaagtagtgtgtgcccgtctgttgtgtgactctggtaactagagatccctcagacccttttagtcagtgtggaaaatctctagcagtggcgcccgaacagggacttgaaagcgaaagggaaaccagaggagctctctcgacgcaggactcggcttgctgaagcgcgcacggcaagaggcgaggggcggcgactggtgagtacgccaaaaattttgactagcggaggctagaaggagagagatgggtgcgagagcgtcagtattaagcgggggagaattagatcgcgatgggaaaaaattcggttaaggccagggggaaagaaaaaatataaattaaaacatatagtatgggcaagcagggagctagaacgattcgcagttaatcctggcctgttagaaacatcagaaggctgtagacaaatactgggacagctacaaccatcccttcagacaggatcagaagaacttagatcattatataatacagtagcaaccctctattgtgtgcatcaaaggatagagataaaagacaccaaggaagctttagacaagatagaggaagagcaaaacaaaagtaagaccaccgcacagcaagcggccactgatcttcagacctggaggaggagatatgagggacaattggagaagtgaattatataaatataaagtagtaaaaattgaaccattaggagtagcacccaccaaggcaaagagaagagtggtgcagagagaaaaaagagcagtgggaataggagctttgttccttgggttcttgggagcagcaggaagcactatgggcgcagcgtcaatgacgctgacggtacaggccagacaattattgtctggtatagtgcagcagcagaacaatttgctgagggctattgaggcgcaacagcatctgttgcaactcacagtctggggcatcaagcagctccaggcaagaatcctggctgtggaaagatacctaaaggatcaacagctcctggggatttggggttgctctggaaaactcatttgcaccactgctgtgccttggaatgctagttggagtaataaatctctggaacagatttggaatcacacgacctggatggagtgggacagagaaattaacaattacacaagcttaatacactccttaattgaagaatcgcaaaaccagcaagaaaagaatgaacaagaattattggaattagataaatgggcaagtttgtggaattggtttaacataacaaattggctgtggtatataaaattattcataatgatagtaggaggcttggtaggtttaagaatagtttttgctgtactttctatagtgaatagagttaggcagggatattcaccattatcgtttcagacccacctcccaaccccgaggggacccgacaggcccgaaggaatagaagaagaaggtggagagagagacagagacagatccattcgattagtgaacggatctcgacggtatcggttaacttttaaaagaaaaggggggattggggggtacagtgcaggggaaagaatagtagacataatagcaacagacatacaaactaaagaattacaaaaacaaattacaaaattcaaaattttatcgatactagtaagccatagagcccaccgcatccccagcatgcctgctattgtcttcccaatcctcccccttgctgtcctgccccaccccaccccccagaatagaatgacacctactcagacaatgcgatgcaatttcctcattttattaggaaaggacagtgggagtggcaccttccagggtcaaggaaggcacgggggaggggcaaacaacagatggctggcaactagaaggcacagtcgaggctgatcagcgagctctagaactagtggatctgcaatcatttacgcgtctacttgtacagctcgtccatgtcatgtgtaatcccggcggcggtcaccctctccttcaggaccatgtgatcgcgcttctcgttggggtctttgctcagtttggactgatggctcaggtagtggttgtcgggcagcagcacggggccgtcgccgatgggggtgttctgctggtagtggtcggcgagctgcacgccgccgtcctcaacgttgtggcgggtcttgaagttagccttgatgccgttcttctgcttgtcggccgtgatatagaccttgtggctgttgaagttgtactccagcttgtgccccaggatgttgccgtcctccttgaagtcgatgcccttcagcacgatgcggttcaccagggtgtcgccctcgaacttcacctcggcgcgggtcttgtaggtgccgtcgtccttgaaagagatggtgcgctcctggacgtagccttcgggcatggcggacttgaagaagtcgtgctgcttcatgtggtcggggtagcgggcgaagcaggccacgccgtagcctaaggtggtcacgagggtgggccagggcacgggcagcttgccggtggtgcagatgaacttcagggtcagcttgccgttggtggcatcgccctcgccctcgccgcggacgctgaacttgtggccgtttacgtcgccgtccagctcgaccaggatgggcaccaccccggtgaacagctcctcgcccttgctcaccaggtacctttaagaccaatgacttacaaggcagctgtagatcttagccactttttaaaagaaaaggggggactggaagggctaattcactcccaacgaagataagatctgctttttgcttgtactgggtctctctggttagaccagatctgagcctgggagctctctggctaactagggaacccactgcttaagcctcaataaagcttgccttgagtgcttcaagtagtgtgtgcccgtctgttgtgtgactctggtaactagagatccctcagacccttttagtcagtgtggaaaatctctagcagtagtagttcatgtcatcttattattcagtatttataacttgcaaagaaatgaatatcagagagtgagaggaacttgtttattgcagcttataatggttacaaataaagcaatagcatcacaaatttcacaaataaagcatttttttcactgcattctagttgtggtttgtccaaactcatcaatgtatcttatcatgtctggctctagctatcccgcccctaactccgcccatcccgcccctaactccgcccagttccgcccattctccgccccatggctgactaattttttttatttatgcagaggccgaggccgcctcggcctctgagctattccagaagtagtgaggaggcttttttggaggcctagacttttgcagagaccaaattcgtaatcatgtcatagctgtttcctgtgtgaaattgttatccgctcacaattccacacaacatacgagccggaagcataaagtgtaaagcctggggtgcctaatgagtgagctaactcacattaattgcgttgcgctcactgcccgctttccagtcgggaaacctgtcgtgccagctgcattaatgaatcggccaacgcgcggggagaggcggtttgcgtattgggcgctcttccgcttcctcgctcactgactcgctgcgctcggtcgttcggctgcggcgagcggtatcagctcactcaaaggcggtaatacggttatccacagaatcaggggataacgcaggaaagaacatgtgagcaaaaggccagcaaaaggccaggaaccgtaaaaaggccgcgttgctggcgtttttccataggctccgcccccctgacgagcatcacaaaaatcgacgctcaagtcagaggtggcgaaacccgacaggactataaagataccaggcgtttccccctggaagctccctcgtgcgctctcctgttccgaccctgccgcttaccggatacctgtccgcctttctcccttcgggaagcgtggcgctttctcatagctcacgctgtaggtatctcagttcggtgtaggtcgttcgctccaagctgggctgtgtgcacgaaccccccgttcagcccgaccgctgcgccttatccggtaactatcgtcttgagtccaacccggtaagacacgacttatcgccactggcagcagccactggtaacaggattagcagagcgaggtatgtaggcggtgctacagagttcttgaagtggtggcctaactacggctacactagaaggacagtatttggtatctgcgctctgctgaagccagttaccttcggaaaaagagttggtagctcttgatccggcaaacaaaccaccgctggtagcggtggtttttttgtttgcaagcagcagattacgcgcagaaaaaaaggatctcaagaagatcctttgatcttttctacggggtctgacgctcagtggaacgaaaactcacgttaagggattttggtcatgagattatcaaaaaggatcttcacctagatccttttaaattaaaaatgaagttttaaatcaatctaaagtatatatgagtaaacttggtctgacagttaccaatgcttaatcagtgaggcacctatctcagcgatctgtctatttcgttcatccatagttgcctgactccccgtcgtgtagataactacgatacgggagggcttaccatctggccccagtgctgcaatgataccgcgagacccacgctcaccggctccagatttatcagcaataaaccagccagccggaagggccgagcgcagaagtggtcctgcaactttatccgcctccatccagtctattaattgttgccgggaagctagagtaagtagttcgccagttaatagtttgcgcaacgttgttgccattgctacaggcatcgtggtgtcacgctcgtcgtttggtatggcttcattcagctccggttcccaacgatcaaggcgagttacatgatcccccatgttgtgcaaaaaagcggttagctccttcggtcctccgatcgttgtcagaagtaagttggccgcagtgttatcactcatggttatggcagcactgcataattctcttactgtcatgccatccgtaagatgcttttctgtgactggtgagtactcaaccaagtcattctgagaatagtgtatgcggcgaccgagttgctcttgcccggcgtcaatacgggataataccgcgccacatagcagaactttaaaagtgctcatcattggaaaacgttcttcggggcgaaaactctcaaggatcttaccgctgttgagatccagttcgatgtaacccactcgtgcacccaactgatcttcagcatcttttactttcaccagcgtttctgggtgagcaaaaacaggaaggcaaaatgccgcaaaaaagggaataagggcgacacggaaatgttgaatactcatactcttcctttttcaatattattgaagcatttatcagggttattgtctcatgagcggatacatatttgaatgtatttagaaaaataaacaaataggggttccgcgcacatttccccgaaaagtgccacctgacgtctaagaaaccattattatcatgacattaacctataaaaataggcgtatcacgaggccctttcgtctcgcgcgtttcggtgatgacggtgaaaacctctgacacatgcagctcccggagacggtcacagcttgtctgtaagcggatgccgggagcagacaagcccgtcagggcgcgtcagcgggtgttggcgggtgtcggggctggcttaactatgcggcatcagagcagattgtactgagagtgcaccatatgcggtgtgaaataccgcacagatgcgtaaggagaaaataccgcatcaggcgccattcgccattcaggctgcgcaactgttgggaagggcgatcggtgcgggcctcttcgctattacgccagctggcgaaagggggatgtgctgcaaggcgattaagttgggtaacgccagggttttcccagtcacgacgttgtaaaacgacggccagtgccaagctg

SEQ ID NO: 318 - DNA, 6838 bp, Synthetic construct
  source 1..6838: mol_type = other DNA
acgcgcgtgtagtcttatgcaatactcttgtagtcttgcaacatggtaacgatgagttagcaacatgccttacaaggagagaaaaagcaccgtgcatgccgattggtggaagtaaggtggtacgatcgtgccttattaggaaggcaacagacgggtctgacatggattggacgaaccactgaattgccgcattgcagagatattgtatttaagtgcctagctcgatacataaacgggtctctctggttagaccagatctgagcctgggagctctctggctaactagggaacccactgcttaagcctcaataaagcttgccttgagtgcttcaagtagtgtgtgcccgtctgttgtgtgactctggtaactagagatccctcagacccttttagtcagtgtggaaaatctctagcagtggcgcccgaacagggacttgaaagcgaaagggaaaccagaggagctctctcgacgcaggactcggcttgctgaagcgcgcacggcaagaggcgaggggcggcgactggtgagtacgccaaaaattttgactagcggaggctagaaggagagagatgggtgcgagagcgtcagtattaagcgggggagaattagatcgcgatgggaaaaaattcggttaaggccagggggaaagaaaaaatataaattaaaacatatagtatgggcaagcagggagctagaacgattcgcagttaatcctggcctgttagaaacatcagaaggctgtagacaaatactgggacagctacaaccatcccttcagacaggatcagaagaacttagatcattatataatacagtagcaaccctctattgtgtgcatcaaaggatagagataaaagacaccaaggaagctttagacaagatagaggaagagcaaaacaaaagtaagaccaccgcacagcaagcggccactgatcttcagacctggaggaggagatatgagggacaattggagaagtgaattatataaatataaagtagtaaaaattgaaccattaggagtagcacccaccaaggcaaagagaagagtggtgcagagagaaaaaagagcagtgggaataggagctttgttccttgggttcttgggagcagcaggaagcactatgggcgcagcgtcaatgacgctgacggtacaggccagacaattattgtctggtatagtgcagcagcagaacaatttgctgagggctattgaggcgcaacagcatctgttgcaactcacagtctggggcatcaagcagctccaggcaagaatcctggctgtggaaagatacctaaaggatcaacagctcctggggatttggggttgctctggaaaactcatttgcaccactgctgtgccttggaatgctagttggagtaataaatctctggaacagatttggaatcacacgacctggatggagtgggacagagaaattaacaattacacaagcttaatacactccttaattgaagaatcgcaaaaccagcaagaaaagaatgaacaagaattattggaattagataaatgggcaagtttgtggaattggtttaacataacaaattggctgtggtatataaaattattcataatgatagtaggaggcttggtaggtttaagaatagtttttgctgtactttctatagtgaatagagttaggcagggatattcaccattatcgtttcagacccacctcccaaccccgaggggacccgacaggcccgaaggaatagaagaagaaggtggagagagagacagagacagatccattcgattagtgaacggatctcgacggtatcggttaacttttaaaagaaaaggggggattggggggtacagtgcaggggaaagaatagtagacataatagcaacagacatacaaactaaagaattacaaaaacaaattacaaaattcaaaattttatcgatactagtaagccatagagcccaccgcatccccagcatgcctgctattgtcttcccaatcctcccccttgctgtcctgccccaccccaccccccagaatagaatgacacctactcagacaatgcgatgcaatttcctcattttattaggaaaggacagtgggagtggcaccttccagggtcaaggaaggcacgggggaggggcaaacaacagatggctggcaactagaaggcacagtcgaggctgatcagcgagctctagaactagtggatctgcaatcatttacgcgtctacttgtacagctcgtccatgtcatgtgtaatcccggcggcggtcaccctctccttcaggaccatgtgatcgcgcttctcgttggggtctttgctcagtttggactgatggctcaggtagtggttgtcgggcagcagcacggggccgtcgccgatgggggtgttctgctggtagtggtcggcgagctgcacgccgccgtcctcaacgttgtggcgggtcttgaagttagccttgatgccgttcttctgcttgtcggccgtgatatagaccttgtggctgttgaagttgtactccagcttgtgccccaggatgttgccgtcctccttgaagtcgatgcccttcagcacgatgcggttcaccagggtgtcgccctcgaacttcacctcggcgcgggtcttgtaggtgccgtcgtccttgaaagagatggtgcgctcctggacgtagccttcgggcatggcggacttgaagaagtcgtgctgcttcatgtggtcggggtagcgggcgaagcaggccacgccgtagcctaaggtggtcacgagggtgggccagggcacgggcagcttgccggtggtgcagatgaacttcagggtcagcttgccgttggtggcatcgccctcgccctcgccgcggacgctgaacttgtggccgtttacgtcgccgtccagctcgaccaggatgggcaccaccccggtgaacagctcctcgcccttgctcaccatggtggcggcccctatagtgagtcgtattattaattaaggatctgtaggaaaaagaagaaggcatgaacatggttagcagaggctctagagccgccggtcacacgccagaagccgaaccccgccctgccccgtcccccccgaaggcagccgtccccccgcggacagccccgaggctggagagggagaaggggacggcggcgcggcgacgcacgaaggccctccccgcccatttccttcctgccggcgccgcaccgcttcgccccgcgcccgctagagggggtgcggcggcgcctcccagatttcggctccgcacagatttgggacaaaggaagtccctgcgccctctcgcacgattaccataaaaggcaatggctgcggctcgccgcgcctcgacagccgccggcgctccgggggccgccgcgcccctcccccgagccctccccggcccgaggcggccccgccccgcccggcacccccacctgccgccaccccccgcccggcacggcgagccccgcgccacgccccgtacggagccccgcacccgaagccgggccgtgctcagcaactcgggtacctttaagaccaatgacttacaaggcagctgtagatcttagccactttttaaaagaaaaggggggactggaagggctaattcactcccaacgaagataagatctgctttttgcttgtactgggtctctctggttagaccagatctgagcctgggagctctctggctaactagggaacccactgcttaagcctcaataaagcttgccttgagtgcttcaagtagtgtgtgcccgtctgttgtgtgactctggtaactagagatccctcagacccttttagtcagtgtggaaaatctctagcagtagtagttcatgtcatcttattattcagtatttataacttgcaaagaaatgaatatcagagagtgagaggaacttgtttattgcagcttataatggttacaaataaagcaatagcatcacaaatttcacaaataaagcatttttttcactgcattctagttgtggtttgtccaaactcatcaatgtatcttatcatgtctggctctagctatcccgcccctaactccgcccatcccgcccctaactccgcccagttccgcccattctccgccccatggctgactaattttttttatttatgcagaggccgaggccgcctcggcctctgagctattccagaagtagtgaggaggcttttttggaggcctagacttttgcagagaccaaattcgtaatcatgtcatagctgtttcctgtgtgaaattgttatccgctcacaattccacacaacatacgagccggaagcataaagtgtaaagcctggggtgcctaatgagtgagctaactcacattaattgcgttgcgctcactgcccgctttccagtcgggaaacctgtcgtgccagctgcattaatgaatcggccaacgcgcggggagaggcggtttgcgtattgggcgctcttccgcttcctcgctcactgactcgctgcgctcggtcgttcggctgcggcgagcggtatcagctcactcaaaggcggtaatacggttatccacagaatcaggggataacgcaggaaagaacatgtgagcaaaaggccagcaaaaggccaggaaccgtaaaaaggccgcgttgctggcgtttttccataggctccgcccccctgacgagcatcacaaaaatcgacgctcaagtcagaggtggcgaaacccgacaggactataaagataccaggcgtttccccctggaagctccctcgtgcgctctcctgttccgaccctgccgcttaccggatacctgtccgcctttctcccttcgggaagcgtggcgctttctcatagctcacgctgtaggtatctcagttcggtgtaggtcgttcgctccaagctgggctgtgtgcacgaaccccccgttcagcccgaccgctgcgccttatccggtaactatcgtcttgagtccaacccggtaagacacgacttatcgccactggcagcagccactggtaacaggattagcagagcgaggtatgtaggcggtgctacagagttcttgaagtggtggcctaactacggctacactagaaggacagtatttggtatctgcgctctgctgaagccagttaccttcggaaaaagagttggtagctcttgatccggcaaacaaaccaccgctggtagcggtggtttttttgtttgcaagcagcagattacgcgcagaaaaaaaggatctcaagaagatcctttgatcttttctacggggtctgacgctcagtggaacgaaaactcacgttaagggattttggtcatgagattatcaaaaaggatcttcacctagatccttttaaattaaaaatgaagttttaaatcaatctaaagtatatatgagtaaacttggtctgacagttaccaatgcttaatcagtgaggcacctatctcagcgatctgtctatttcgttcatccatagttgcctgactccccgtcgtgtagataactacgatacgggagggcttaccatctggccccagtgctgcaatgataccgcgagacccacgctcaccggctccagatttatcagcaataaaccagccagccggaagggccgagcgcagaagtggtcctgcaactttatccgcctccatccagtctattaattgttgccgggaagctagagtaagtagttcgccagttaatagtttgcgcaacgttgttgccattgctacaggcatcgtggtgtcacgctcgtcgtttggtatggcttcattcagctccggttcccaacgatcaaggcgagttacatgatcccccatgttgtgcaaaaaagcggttagctccttcggtcctccgatcgttgtcagaagtaagttggccgcagtgttatcactcatggttatggcagcactgcataattctcttactgtcatgccatccgtaagatgcttttctgtgactggtgagtactcaaccaagtcattctgagaatagtgtatgcggcgaccgagttgctcttgcccggcgtcaatacgggataataccgcgccacatagcagaactttaaaagtgctcatcattggaaaacgttcttcggggcgaaaactctcaaggatcttaccgctgttgagatccagttcgatgtaacccactcgtgcacccaactgatcttcagcatcttttactttcaccagcgtttctgggtgagcaaaaacaggaaggcaaaatgccgcaaaaaagggaataagggcgacacggaaatgttgaatactcatactcttcctttttcaatattattgaagcatttatcagggttattgtctcatgagcggatacatatttgaatgtatttagaaaaataaacaaataggggttccgcgcacatttccccgaaaagtgccacctgacgtctaagaaaccattattatcatgacattaacctataaaaataggcgtatcacgaggccctttcgtctcgcgcgtttcggtgatgacggtgaaaacctctgacacatgcagctcccggagacggtcacagcttgtctgtaagcggatgccgggagcagacaagcccgtcagggcgcgtcagcgggtgttggcgggtgtcggggctggcttaactatgcggcatcagagcagattgtactgagagtgcaccatatgcggtgtgaaataccgcacagatgcgtaaggagaaaataccgcatcaggcgccattcgccattcaggctgcgcaactgttgggaagggcgatcggtgcgggcctcttcgctattacgccagctggcgaaagggggatgtgctgcaaggcgattaagttgggtaacgccagggttttcccagtcacgacgttgtaaaacgacggccagtgccaagctg

SEQ ID NO: 319 - DNA, 6236 bp, Synthetic construct
  source 1..6236: mol_type = other DNA
ttatttctgaatattttactaaaaagggaatgtgggaggtcagtgcatttaaaacataaagaaatgaagagctagttcaaaccttgggaaaatacactatatcttaaactccatgaaagaaggtgaggctgcaaacagctaatgcacattggcaacagcccctgatgcctatgccttattcatccctcagaaaaggattcaagtagaggcttgatttggaggttaaagttttgctatgctgtattttacattacttattgttttagctgtcctcatgaatgtcttttcactacccatttgcttatcctgcatctctcagccttgactccactcagttctcttgcttagagataccacctttcccctgaagtgttccttccatgttttacggcgagatggtttctcctcgcctggccactcagccttagttgtctctgttgtcttatagaggtctacttgaagaaggaaaaacagggggcatggtttgactgtcctgtgagcccttcttccctgcctcccccactcacagtgacccggaatccctcgacatggcagtctagcactagtgcggccgcagatctgcttcctcgctcactgactcgctgcgctcggtcgttcggctgcggcgagcggtatcagctcactcaaaggcggtaatacggttatccacagaatcaggggataacgcaggaaagaacatgtgagcaaaaggccagcaaaaggccaggaaccgtaaaaaggccgcgttgctggcgtttttccataggctccgcccccctgacgagcatcacaaaaatcgacgctcaagtcagaggtggcgaaacccgacaggactataaagataccaggcgtttccccctggaagctccctcgtgcgctctcctgttccgaccctgccgcttaccggatacctgtccgcctttctcccttcgggaagcgtggcgctttctcatagctcacgctgtaggtatctcagttcggtgtaggtcgttcgctccaagctgggctgtgtgcacgaaccccccgttcagcccgaccgctgcgccttatccggtaactatcgtcttgagtccaacccggtaagacacgacttatcgccactggcagcagccactggtaacaggattagcagagcgaggtatgtaggcggtgctacagagttcttgaagtggtggcctaactacggctacactagaagaacagtatttggtatctgcgctctgctgaagccagttaccttcggaaaaagagttggtagctcttgatccggcaaacaaaccaccgctggtagcggtggtttttttgtttgcaagcagcagattacgcgcagaaaaaaaggatctcaagaagatcctttgatcttttctacggggtctgacgctcagtggaacgaaaactcacgttaagggattttggtcatgagattatcaaaaaggatcttcacctagatccttttaaattaaaaatgaagttttaaatcaatctaaagtatatatgagtaaacttggtctgacagttaccaatgcttaatcagtgaggcacctatctcagcgatctgtctatttcgttcatccatagttgcctgactccccgtcgtgtagataactacgatacgggagggcttaccatctggccccagtgctgcaatgataccgcgagacccacgctcaccggctccagatttatcagcaataaaccagccagccggaagggccgagcgcagaagtggtcctgcaactttatccgcctccatccagtctattaattgttgccgggaagctagagtaagtagttcgccagttaatagtttgcgcaacgttgttgccattgctacaggcatcgtggtgtcacgctcgtcgtttggtatggcttcattcagctccggttcccaacgatcaaggcgagttacatgatcccccatgttgtgcaaaaaagcggttagctccttcggtcctccgatcgttgtcagaagtaagttggccgcagtgttatcactcatggttatggcagcactgcataattctcttactgtcatgccatccgtaagatgcttttctgtgactggtgagtactcaaccaagtcattctgagaatagtgtatgcggcgaccgagttgctcttgcccggcgtcaatacgggataataccgcgccacatagcagaactttaaaagtgctcatcattggaaaacgttcttcggggcgaaaactctcaaggatcttaccgctgttgagatccagttcgatgtaacccactcgtgcacccaactgatcttcagcatcttttactttcaccagcgtttctgggtgagcaaaaacaggaaggcaaaatgccgcaaaaaagggaataagggcgacacggaaatgttgaatactcatactcttcctttttcaatattattgaagcatttatcagggttattgtctcatgagcggatacatatttgaatgtatttagaaaaataaacaaataggggttccgcgcacatttccccgaaaagtgccacctgacgtggatcccctgagggggcccccatgggctagaggatccggcctcggcctctgcataaataaaaaaaattagtcagccatgagcttggcccattgcatacgttgtatccatatcataatatgtacatttatattggctcatgtccaacattaccgccatgttgacattgattattgactagttattaatagtaatcaattacggggtcattagttcatagcccatatatggagttccgcgttacataacttacggtaaatggcccgcctggctgaccgcccaacgacccccgcccattgacgtcaataatgacgtatgttcccatagtaacgccaatagggactttccattgacgtcaatgggtggagtatttacggtaaactgcccacttggcagtacatcaagtgtatcatatgccaagtacgccccctattgacgtcaatgacggtaaatggcccgcctggcattatgcccagtacatgaccttatgggactttcctacttggcagtacatctacgtattagtcatcgctattaccatggtgatgcggttttggcagtacatcaatgggcgtggatagcggtttgactcacggggatttccaagtctccaccccattgacgtcaatgggagtttgttttggcaccaaaatcaacgggactttccaaaatgtcgtaacaactccgccccattgacgcaaatgggcggtaggcgtgtacggtgggaggtctatataagcagagctcgtttagtgaaccgtcagatcgcctggagacgccatccacgctgttttgacctccatagaagacaccgggaccgatccagcctcccctcgaagcttacatgtggtaccgagctcggatcctgagaacttcagggtgagtctatgggacccttgatgttttctttccccttcttttctatggttaagttcatgtcataggaaggggagaagtaacagggtacacatattgaccaaatcagggtaattttgcatttgtaattttaaaaaatgctttcttcttttaatatacttttttgtttatcttatttctaatactttccctaatctctttctttcagggcaataatgatacaatgtatcatgcctctttgcaccattctaaagaataacagtgataatttctgggttaaggcaatagcaatatttctgcatataaatatttctgcatataaattgtaactgatgtaagaggtttcatattgctaatagcagctacaatccagctaccattctgcttttattttatggttgggataaggctggattattctgagtccaagctaggcccttttgctaatcatgttcatacctcttatcttcctcccacagctcctgggcaacgtgctggtctgtgtgctggcccatcactttggcaaagcacgtgagatctgaattctgacactatggcgcgttcaacgctctcaaaaccccttaaaaataaggttaacccgcgaggccccctaatccccttaattcttctgatgctcagaggggtcagtactgcttcgcccggctccagtcctcatcaagtctataatatcacctgggaggtaaccaatggagatcgggagacggtatgggcaacttctggcaaccaccctctgtggacctggtggcctgaccttaccccagatttatgtatgttagcccaccatggaccatcttattgggggctagaatatcaatcccctttttcttctcccccggggcccccttgttgctcagggggcagcagcccaggctgttccagagactgcgaagaacctttaacctccctcacccctcggtgcaacactgcctggaacagactcaagctagaccagacaactcataaatcaaatgagggattttatgtttgccccgggccccaccgcccccgagaatccaagtcatgtgggggtccagactccttctactgtgcctattggggctgtgagacaaccggtagagcttactggaagccctcctcatcatgggatttcatcacagtaaacaacaatctcacctctgaccaggctgtccaggtatgcaaagataataagtggtgcaaccccttagttattcggtttacagacgccgggagacgggttacttcctggaccacaggacattactggggcttacgtttgtatgtctccggacaagatccagggcttacatttgggatccgactcagataccaaaatctaggaccccgcgtcccaatagggccaaaccccgttctggcagaccaacagccactctccaagcccaaacctgttaagtcgccttcagtcaccaaaccacccagtgggactcctctctcccctacccaacttccaccggcgggaacggaaaataggctgctaaacttagtagacggagcctaccaagccctcaacctcaccagtcctgacaaaacccaagagtgctggttgtgtctagtagcgggacccccctactacgaaggggttgccgtcctgggtacctactccaaccatacctctgctccagccaactgctccgtggcctcccaacacaagttgaccctgtccgaagtgaccggacagggactctgcataggagcagttcccaaaacacatcaggccctatgtaataccacccagacaagcagtcgagggtcctattatctagttgcccctacaggtaccatgtgggcttgtagtaccgggcttactccatgcatctccaccaccatactgaaccttaccactgattattgtgttcttgtcgaactctggccaagagtcacctatcattcccccagctatgtttacggcctgtttgagagatccaaccgacacaaaagagaaccggtgtcgttaaccctggccctattattgggtggactaaccatggggggaattgccgctggaataggaacagggactactgctctaatggccactcagcaattccagcagctccaagccgcagtacaggatgatctcagggaggttgaaaaatcaatctctaacctagaaaagtctctcacttccctgtctgaagttgtcctacagaatcgaaggggcctagacttgttatttctaaaagaaggagggctgtgtgctgctctaaaagaagaatgttgcttctatgcggaccacacaggactagtgagagacagcatggccaaattgagagagaggcttaatcagagacagaaactgtttgagtcaactcaaggatggtttgagggactgtttaacagatccccttggtttaccaccttgatatctaccattatgggacccctcattgtactcctaatgattttgctcttcggaccctgcattcttaatcgattagtccaatttgttaaagacaggatatcagtggtccaggctctatagctcaaatcctgcacaacagattcttcatgtttggaccaaatcaacttgtgataccatgctcaaagaggcctcaattatatttgagtttttaatttttatgaaaaaaaaaaaaaaaaacggaattcaccccaccagtgcaggctgcctatcagaaagtggtggctggtgtggctaatgccctggcccacaagtatcactaagctcgctttcttgctgtccaatttctattaaaggttcctttgttccctaagtccaactactaaactgggggatattatgaagggccttgagcatctggattctgcctaataaaaaacatttattttcattgcaatgatgtatttaaa

SEQ ID NO: 320 - DNA, 3345 bp, Synthetic construct
  source 1..3345: mol_type = other DNA
ataaaacctgcaggcatgcaagcgatcgcggggccgcccccttcaccgagggcctatttcccatgattccttcatatttgcatatacgatacaaggctgttagagagataattggaattaatttgactgtaaacacaaagatattagtacaaaatacgtgacgtagaaagtaataatttcttgggtagtttgcagttttaaaattatgttttaaaatggactatcatatgcttaccgtaacttgaaagtatttcgatttcttggctttatatatcttgtggaaaggacgaaacaccggccacgccgtggcttaagggtttcagagccaccagaagatatggcttcggtggcaagttgaaataaggctagtccgttatcaacttgaaaaagtggcaccgagtcggtgctttttttactagttctagagcggccccaattcgccctatagtgagtcgtattacgcgcgctcactggccgtcgttttacaacgtcgtgactgggaaaaccctggcgttacccaacttaatcgccttgcagcacatccccctttcgccagctggcgtaatagcgaagaggcccgcaccgatcgcccttcccaacagttgcgcagcctgaatggcgaatgggacgcgccctgtagcggcgcattaagcgcggcgggtgtggtggttacgcgcagcgtgaccgctacacttgccagcgccctagcgcccgctcctttcgctttcttcccttcctttctcgccacgttcgccggctttccccgtcaagctctaaatcgggggctccctttagggttccgatttagtgctttacggcacctcgaccccaaaaaacttgattagggtgatggttcacgtagtgggccatcgccctgatagacggtttttcgccctttgacgttggagtccacgttctttaatagtggactcttgttccaaactggaacaacactcaaccctatctcggtctattcttttgatttataagggattttgccgatttcggcctattggttaaaaaatgagctgatttaacaaaaatttaacgcgaattttaacaaaatattaacgcttacaatttaggtggcacttttcggggaaatgtgcgcggaacccctatttgtttatttttctaaatacattcaaatatgtatccgctcatgagacaataaccctgataaatgcttcaataatattgaaaaaggaagagtatgagtattcaacatttccgtgtcgcccttattcccttttttgcggcattttgccttcctgtttttgctcacccagaaacgctggtgaaagtaaaagatgctgaagatcagttgggtgcacgagtgggttacatcgaactggatctcaacagcggtaagatccttgagagttttcgccccgaagaacgttttccaatgatgagcacttttaaagttctgctatgtggcgcggtattatcccgtattgacgccgggcaagagcaactcggtcgccgcatacactattctcagaatgacttggttgagtactcaccagtcacagaaaagcatcttacggatggcatgacagtaagagaattatgcagtgctgccataaccatgagtgataacactgcggccaacttacttctgacaacgatcggaggaccgaaggagctaaccgcttttttgcacaacatgggggatcatgtaactcgccttgatcgttgggaaccggagctgaatgaagccataccaaacgacgagcgtgacaccacgatgcctgtagcaatggcaacaacgttgcgcaaactattaactggcgaactacttactctagcttcccggcaacaattaatagactggatggaggcggataaagttgcaggaccacttctgcgctcggcccttccggctggctggtttattgctgataaatctggagccggtgagcgtgggtctcgcggtatcattgcagcactggggccagatggtaagccctcccgtatcgtagttatctacacgacggggagtcaggcaactatggatgaacgaaatagacagatcgctgagataggtgcctcactgattaagcattggtaactgtcagaccaagtttactcatatatactttagattgatttaaaacttcatttttaatttaaaaggatctaggtgaagatcctttttgataatctcatgaccaaaatcccttaacgtgagttttcgttccactgagcgtcagaccccgtagaaaagatcaaaggatcttcttgagatcctttttttctgcgcgtaatctgctgcttgcaaacaaaaaaaccaccgctaccagcggtggtttgtttgccggatcaagagctaccaactctttttccgaaggtaactggcttcagcagagcgcagataccaaatactgtccttctagtgtagccgtagttaggccaccacttcaagaactctgtagcaccgcctacatacctcgctctgctaatcctgttaccagtggctgctgccagtggcgataagtcgtgtcttaccgggttggactcaagacgatagttaccggataaggcgcagcggtcgggctgaacggggggttcgtgcacacagcccagcttggagcgaacgacctacaccgaactgagatacctacagcgtgagctatgagaaagcgccacgcttcccgaagggagaaaggcggacaggtatccggtaagcggcagggtcggaacaggagagcgcacgagggagcttccagggggaaacgcctggtatctttatagtcctgtcgggtttcgccacctctgacttgagcgtcgatttttgtgatgctcgtcaggggggcggagcctatggaaaaacgccagcaacgcggcctttttacggttcctggccttttgctggccttttgctcacatgttctttcctgcgttatcccctgattctgtggataaccgtattaccgcctttgagtgagctgataccgctcgccgcagccgaacgaccgagcgcagcgagtcagtgagcgaggaagcggaagagcgcccaatacgcaaaccgcctctccccgcgcgttggccgattcattaatgcagctggcacgacaggtttcccgactggaaagcgggcagtgagcgcaacgcaattaatgtgagttagctcactcattaggcaccccaggctttacactttatgcttccggctcgtatgttgtgtggaattgtgagcggataacaatttcacacaggaaacagctatgaccatgattacgccaagcgcgcaattaaccctcactaaagggaacaaaagctggaaacatgcatgaagttcctattccgaagttcctattctctagaaagtataggaacttc

SEQ ID NO: 321 - protein, 2345 aa, Synthetic construct
MDKKYSIGLDIGTNSVGWAVITDEYKVPSKKFKVLGNTDRHSIKKNLIGALLFDSGETAEATRLKRTARRRYTRRKNRICYLQEIFSNEMAKVDDSFFHRLEESFLVEEDKKHERHPIFGNIVDEVAYHEKYPTIYHLRKKLVDSTDKADLRLIYLALAHMIKFRGHFLIEGDLNPDNSDVDKLFIQLVQTYNQLFEENPINASGVDAKAILSARLSKSRRLENLIAQLPGEKKNGLFGNLIALSLGLTPNFKSNFDLAEDAKLQLSKDTYDDDLDNLLAQIGDQYADLFLAAKNLSDAILLSDILRVNTEITKAPLSASMIKRYDEHHQDLTLLKALVRQQLPEKYKEIFFDQSKNGYAGYIDGGASQEEFYKFIKPILEKMDGTEELLVKLNREDLLRKQRTFDNGSIPHQIHLGELHAILRRQEDFYPFLKDNREKIEKILTFRIPYYVGPLARGNSRFAWMTRKSEETITPWNFEEVVDKGASAQSFIERMTNFDKNLPNEKVLPKHSLLYEYFTVYNELTKVKYVTEGMRKPAFLSGEQKKAIVDLLFKTNRKVTVKQLKEDYFKKIECFDSVEISGVEDRFNASLGTYHDLLKIIKDKDFLDNEENEDILEDIVLTLTLFEDREMIEERLKTYAHLFDDKVMKQLKRRRYTGWGRLSRKLINGIRDKQSGKTILDFLKSDGFANRNFMQLIHDDSLTFKEDIQKAQVSGQGDSLHEHIANLAGSPAIKKGILQTVKVVDELVKVMGRHKPENIVIEMARENQTTQKGQKNSRERMKRIEEGIKELGSQILKEHPVENTQLQNEKLYLYYLQNGRDMYVDQELDINRLSDYDVDHIVPQSFLKDDSIDNKVLTRSDKARGKSDNVPSEEVVKKMKNYWRQLLNAKLITQRKFDNLTKAERGGLSELDKAGFIKRQLVETRQITKHVAQILDSRMNTKYDENDKLIREVKVITLKSKLVSDFRKDFQFYKVREINNYHHAHDAYLNAVVGTALIKKYPKLESEFVYGDYKVYDVRKMIAKSEQEIGKATAKYFFYSNIMNFFKTEITLANGEIRKRPLIETNGETGEIVWDKGRDFATVRKVLSMPQVNIVKKTEVQTGGFSKESILPKRNSDKLIARKKDWDPKKYGGFDSPTVAYSVLVVAKVEKGKSKKLKSVKELLGITIMERSSFEKNPIDFLEAKGYKEVKKDLIIKLPKYSLFELENGRKRMLASAGELQKGNELALPSKYVNFLYLASHYEKLKGSPEDNEQKQLFVEQHKHYLDEIIEQISEFSKRVILADANLDKVLSAYNKHRDKPIREQAENIIHLFTLTNLGAPAAFKYFDTTIDRKRYTSTKEVLDATLIHQSITGLYETRIDLSQLGGDAYPYDVPDYASLGSGSPKKKRKVEDGEGPAAKRVKLDSGAAPAAKKKKLDTGGPGSEPATSGSETPGTSESATPESGPGASTLNIEDEYRLHETSKEPDVSLGSTWLSDFPQAWAETGGMGLAVRQAPLIIPLKATSTPVSIKQYPMSQEARLGIKPHIQRLLDQGILVPCQSPWNTPLLPVKKPGTNDYRPVQDLREVNKRVEDIHPTVPNPYNLLSGLPPSHQWYTVLDLKDAFFCLRLHPTSQPLFAFEWRDPEMGISGQLTWTRLPQGFKNSPTLFNEALHRDLADFRIQHPDLILLQYVDDLLLAATSELDCQQGTRALLQTLGNLGYRASAKKAQICQKQVKYLGYLLKEGQRWLTEARKETVMGQPTPKTPRQLREFLGKAGFCRLFIPGFAEMAAPLYPLTKPGTLFNWGPDQQKAYQEIKQALLTAPALGLPDLTKPFELFVDEKQGYAKGVLTQKLGPWRRPVAYLSKKLDPVAAGWPPCLRMVAAIAVLTKDAGKLTMGQPLVILAPHAVEALVKQPPDRWLSNARMTHYQALLLDTDRVQFGPVVALNPATLLPLPEEGLQHNCLDILAEAHGTRPDLTDQPLPDADHTWYTDGSSLLQEGQRKAGAAVTTETEVIWAKALPAGTSAQRAELIALTQALKMAEGKKLNVYTDSRYAFATAHIHGEIYRRRGWLTSEGKEIKNKDEILALLKALFLPKRLSIIHCPGHQKGHSAEARGNRMADQAARKAAITETPDTSTLLIENSSPGTPKKKRKVDGSGATNFSLLKQAGDVEENPGPMDHYLDIRLRPDPEFPPAQLMSVLFGKLHQALVAQGGDRIGVSFPDLDESRSRLGERLRIHASADDLRALLARPWLEGLRDHLQFGEPAVVPHPTPYRQVSRVQAKSNPERLRRRLMRRHDLSEEEARKRIPDTVARALDLPFVTLRSQSTGQHFRLFIRHGPLQVTAEEGGFTCYGLSKGGFVPWF

SEQ ID NO: 322 - DNA, 7038 bp, Synthetic construct
  source 1..7038: mol_type = other DNA
atggacaagaagtacagcatcggcctggacatcggcaccaactctgtgggctgggccgtgatcaccgacgagtacaaggtgcccagcaagaaattcaaggtgctgggcaacaccgaccggcacagcatcaagaagaacctgatcggagccctgctgttcgacagcggcgaaacagccgaggccacccggctgaagagaaccgccagaagaagatacaccagacggaagaaccggatctgctatctgcaagagatcttcagcaacgagatggccaaggtggacgacagcttcttccacagactggaagagtccttcctggtggaagaggataagaagcacgagcggcaccccatcttcggcaacatcgtggacgaggtggcctaccacgagaagtaccccaccatctaccacctgagaaagaaactggtggacagcaccgacaaggccgacctgcggctgatctatctggccctggcccacatgatcaagttccggggccacttcctgatcgagggcgacctgaaccccgacaacagcgacgtggacaagctgttcatccagctggtgcagacctacaaccagctgttcgaggaaaaccccatcaacgccagcggcgtggacgccaaggccatcctgtctgccagactgagcaagagcagacggctggaaaatctgatcgcccagctgcccggcgagaagaagaatggcctgttcggcaacctgattgccctgagcctgggcctgacccccaacttcaagagcaacttcgacctggccgaggatgccaaactgcagctgagcaaggacacctacgacgacgacctggacaacctgctggcccagatcggcgaccagtacgccgacctgtttctggccgccaagaacctgtccgacgccatcctgctgagcgacatcctgagagtgaacaccgagatcaccaaggcccccctgagcgcctctatgatcaagagatacgacgagcaccaccaggacctgaccctgctgaaagctctcgtgcggcagcagctgcctgagaagtacaaagagattttcttcgaccagagcaagaacggctacgccggctacattgacggcggagccagccaggaagagttctacaagttcatcaagcccatcctggaaaagatggacggcaccgaggaactgctcgtgaagctgaacagagaggacctgctgcggaagcagcggaccttcgacaacggcagcatcccccaccagatccacctgggagagctgcacgccattctgcggcggcaggaagatttttacccattcctgaaggacaaccgggaaaagatcgagaagatcctgaccttccgcatcccctactacgtgggccctctggccaggggaaacagcagattcgcctggatgaccagaaagagcgaggaaaccatcaccccctggaacttcgaggaagtggtggacaagggcgcttccgcccagagcttcatcgagcggatgaccaacttcgataagaacctgcccaacgagaaggtgctgcccaagcacagcctgctgtacgagtacttcaccgtgtataacgagctgaccaaagtgaaatacgtgaccgagggaatgagaaagcccgccttcctgagcggcgagcagaaaaaggccatcgtggacctgctgttcaagaccaaccggaaagtgaccgtgaagcagctgaaagaggactacttcaagaaaatcgagtgcttcgactccgtggaaatctccggcgtggaagatcggttcaacgcctccctgggcacataccacgatctgctgaaaattatcaaggacaaggacttcctggacaatgaggaaaacgaggacattctggaagatatcgtgctgaccctgacactgtttgaggacagagagatgatcgaggaacggctgaaaacctatgcccacctgttcgacgacaaagtgatgaagcagctgaagcggcggagatacaccggctggggcaggctgagccggaagctgatcaacggcatccgggacaagcagtccggcaagacaatcctggatttcctgaagtccgacggcttcgccaacagaaacttcatgcagctgatccacgacgacagcctgacctttaaagaggacatccagaaagcccaggtgtccggccagggcgatagcctgcacgagcacattgccaatctggccggcagccccgccattaagaagggcatcctgcagacagtgaaggtggtggacgagctcgtgaaagtgatgggccggcacaagcccgagaacatcgtgatcgaaatggccagagagaaccagaccacccagaagggacagaagaacagccgcgagagaatgaagcggatcgaagagggcatcaaagagctgggcagccagatcctgaaagaacaccccgtggaaaacacccagctgcagaacgagaagctgtacctgtactacctgcagaatgggcgggatatgtacgtggaccaggaactggacatcaaccggctgtccgactacgatgtggaccatatcgtgcctcagagctttctgaaggacgactccatcgacaacaaggtgctgaccagaagcgacaaggcccggggcaagagcgacaacgtgccctccgaagaggtcgtgaagaagatgaagaactactggcggcagctgctgaacgccaagctgattacccagagaaagttcgacaatctgaccaaggccgagagaggcggcctgagcgaactggataaggccggcttcatcaagagacagctggtggaaacccggcagatcacaaagcacgtggcacagatcctggactcccggatgaacactaagtacgacgagaatgacaagctgatccgggaagtgaaagtgatcaccctgaagtccaagctggtgtccgatttccggaaggatttccagttttacaaagtgcgcgagatcaacaactaccaccacgcccacgacgcctacctgaacgccgtcgtgggaaccgccctgatcaaaaagtaccctaagctggaaagcgagttcgtgtacggcgactacaaggtgtacgacgtgcggaagatgatcgccaagagcgagcaggaaatcggcaaggctaccgccaagtacttcttctacagcaacatcatgaactttttcaagaccgagattaccctggccaacggcgagatccggaagcggcctctgatcgagacaaacggcgaaaccggggagatcgtgtgggataagggccgggattttgccaccgtgcggaaagtgctgagcatgccccaagtgaatatcgtgaaaaagaccgaggtgcagacaggcggcttcagcaaagagtctatcctgcccaagaggaacagcgataagctgatcgccagaaagaaggactgggaccctaagaagtacggcggcttcgacagccccaccgtggcctattctgtgctggtggtggccaaagtggaaaagggcaagtccaagaaactgaagagtgtgaaagagctgctggggatcaccatcatggaaagaagcagcttcgagaagaatcccatcgactttctggaagccaagggctacaaagaagtgaaaaaggacctgatcatcaagctgcctaagtactccctgttcgagctggaaaacggccggaagagaatgctggcctctgccggcgaactgcagaagggaaacgaactggccctgccctccaaatatgtgaacttcctgtacctggccagccactatgagaagctgaagggctcccccgaggataatgagcagaaacagctgtttgtggaacagcacaagcactacctggacgagatcatcgagcagatcagcgagttctccaagagagtgatcctggccgacgctaatctggacaaagtgctgtccgcctacaacaagcaccgggataagcccatcagagagcaggccgagaatatcatccacctgtttaccctgaccaatctgggagcccctgccgccttcaagtactttgacaccaccatcgaccggaagaggtacaccagcaccaaagaggtgctggacgccaccctgatccaccagagcatcaccggcctgtacgagacacggatcgacctgtctcagctgggaggcgacgcctatccctatgacgtgcccgattatgccagcctgggctccggatcccccaagaagaaacgcaaggtggaagatggcgagggcccagccgctaagagagtgaaactggattccggagctgctcctgccgccaagaagaagaaactcgacaccggtggacctggaagcgagcctgctacatctggctctgagacacctggcacctccgagtctgctacacctgaatctggacctggcgctagcaccctgaacatcgaggacgagtaccggctgcacgagacaagcaaagaacccgatgtgtccctgggcagcacctggcttagtgatttccctcaggcctgggccgagacaggcggaatgggacttgctgttagacaggcccctctgatcatccctctgaaggccacaagcacccctgtgtccatcaagcagtaccccatgagccaagaggcccggctgggaatcaagccccacattcagagactgctggaccagggcatcctggtgccttgtcagagcccttggaatacccctctgctgcccgtgaagaagcccggcaccaacgattacagacccgtgcaggacctgcgggaagtgaacaagagagtggaagatattcaccccaccgtgccgaatccttacaacctgctgtctggcctgcctcctagccaccagtggtacacagtgctggacctgaaggacgccttcttctgtctgcggctgcaccctacaagccagcctctgtttgcctttgagtggcgggaccctgagatgggcattagcggacagctgacctggaccagactgccccagggcttcaagaacagccccacactgttcaacgaggccctgcatagggacctcgccgacttcagaatccagcatcctgacctgatcctgctccagtacgtggacgatctgctgctggccgctacaagcgagctggattgtcagcagggaacaagagccctgctgcaaaccctgggcaacctgggctatagagcctctgccaagaaggcccagatttgccagaaacaagtgaagtatctgggctacctgctgaaagagggccagcgttggctgaccgaggccagaaaagaaaccgtgatgggccagcctacacctaagacacccagacagctgagagagttcctgggcaaagccggattctgtcggctgttcatccctggctttgccgagatggctgcccctctgtacccactgacaaagcccggaactctgttcaactggggcccagatcagcagaaggcctaccaagagatcaagcaggctctgctgacagcccctgctctgggactgcctgatctgaccaagcctttcgagctgttcgtggacgagaagcagggctatgccaaaggcgtgctgacacagaagctcggcccttggagaaggcctgtggcctacctgagcaagaaactggaccctgtggctgccggatggcctccttgtctgagaatggtggccgccattgccgtgctgaccaaggatgccggaaagctgacaatgggacagcctctggtcattctggcccctcatgccgtggaagccctcgtgaaacagcctcctgatcggtggctgagcaacgccaggatgacacactatcaggcactgctgctcgacaccgacagagtgcagtttggacctgtggtggccctgaatcctgccacacttctgcctctgcctgaggaaggcctccagcacaattgcctggacatcctggccgaggctcacggcacaagacccgatctgacagatcagccactgcctgacgccgaccacacctggtatacagatggcagctctctgctgcaagaaggacagagaaaagccggggctgccgtgaccaccgagacagaagtgatttgggccaaagctctgcccgctggcacatctgctcagagagccgaactgatcgccctgacacaggccctgaaaatggccgagggcaagaagctgaacgtctacaccgactccagatacgccttcgccaccgctcacatccacggcgaaatctatcggcggagaggatggctgaccagcgagggcaaagagattaagaacaaggacgagattctcgccctgctcaaggccctgttcctgcctaagcggctgagcatcatccactgtccaggccaccagaagggccactctgctgaagctagaggcaacagaatggccgaccaggctgccagaaaggccgccatcacagagacacccgataccagcacactgctgatcgagaacagcagccctggtacccctaagaagaagcggaaagtggacggatccggcgccaccaatttcagcctgctgaaacaggctggcgacgtggaagaaaatcccgggcctatggaccactacctggacatcagactgcggcccgatcctgagtttcctccagctcagctgatgagcgtgctgttcggcaaactgcaccaggctctggttgcccaaggcggcgatagaatcggagtgtcattccccgacctggacgagagcagaagcagactgggagagagactgagaatccacgccagcgccgatgatctgagagccctgcttgctagaccttggctggaaggcctgagagatcacctccagtttggagagcctgccgtggtgcctcatccaacaccatatagacaggtgtccagagtgcaggccaagagcaaccccgaaagactgcggagaaggctgatgcggagacacgacctgtctgaggaagaggcccggaagagaatccccgacacagtggctagagccctggacctgcctttcgtgacactgagaagccagagcaccggccagcacttccggctgtttatcagacacggccctctgcaagtgaccgccgaagaaggcggctttacctgttacggcctgagcaaaggcggattcgtgccctggttttga

SEQ ID NO: 323 - protein, 162 aa, Synthetic construct
MLKMESTQQMAVSIINSSFEAAVVAATSALENMGIEYDYQDIYSRVKNKFDFVMDDSGVKNNPIGKAITIDQALNNKFGSAIRNRNWLADTSRPAKLDEDVNKLRMMLSSKGIDQKMRVLNACFSVKRIPGKSSSIIKCTKLMRDKLERGEVEVDDSFVDEK

SEQ ID NO: 324 - DNA, 486 bp, Synthetic construct
  source 1..486: mol_type = other DNA
atgcttaagatggaaagcacccagcagatggccgtgtccatcatcaacagcagctttgaggccgccgtggtggccgctacatctgcccttgagaatatgggcatcgagtacgactaccaggacatctacagccgcgtgaagaacaagttcgacttcgtgatggacgacagcggggtcaagaacaaccctatcggcaaggccatcaccatcgatcaggccctgaacaacaagtttggcagcgccatcagaaaccggaactggctggccgatacaagcagacccgccaagctggacgaggacgtgaacaagctgcggatgatgctgagcagcaagggcatcgaccagaaaatgcgggtgctgaacgcctgcttcagcgtgaagagaatccccggcaagagcagctctatcatcaagtgcaccaagctgatgcgggacaagctggaacggggcgaagtggaagtggacgactcctttgtcgacgagaag